European Patent Application EP 4 378 305 A1, published June 5, 2024. Title: METHOD FOR DETECTING CROSS COMPATIBILITY AMONG OLIVE TREES. Applicant: Centre national de la recherche scientifique. Application EP. The sequence listing filed with the application follows.

SEQUENCE LISTING (19 sequences)

SEQ ID NO: 1 - DNA, 696 bp, Olea europaea
  source 1..696: mol_type = genomic DNA
  misc_feature 1..696: note = DSI-A Allele S subspecies europaea
ggcctccacttaccttggcattcaggggttccatccacgatttgaggagatcaaagaattaatagagaggatgaaaattactcctgcacaagttgctgaagaactaatgaagagtgatgatcctcatacttctcttgaaggtctagttaattttttgaagtgcagaaggatcgaaagcaacctatcaaaggataaaggaaacgaagaaaatgaagtcgagaatataaaaagacttccatctgacagtgatattgaagtcgtgacagactaaaatttatgtgaatttgatcatgcttattatgattttaaattagaatttgaaattgtggttcttgattaaagatccaagactctacctattgaacaaacaatgagcttgtatttcttaatataaaactatttctagaattttgtctcattacagtaatttctagagaagaagagcgacctctatcaccatgttatttattatctccatcagttgtacgtgaaataattggagtggaaggagcatgacatatgctactaaaaaatagcttttcagttaagaaaaattattatccgttggtaaaagtaatttacttttaactatgataatcagcaacggatttttcgttggtaacaatgatatccttttaccaatgaatattctgtgtctaatgtaaccgtttaacatttgaatctttcacacgtacc

SEQ ID NO: 2 - DNA, 731 bp, Olea europaea
  source 1..731: mol_type = genomic DNA
  misc_feature 1..731: note = DSI-A Allele S subspecies laperrinei
ggcctccacttaccttggcattcaggggttccatccgcgatttgaggagatcaaagaattaatagagattatgaaaattactcctgcacaagttgctgaagaactaatgaagagtgatgatcctcatacttctcttgaaggtctagttaattttttgaagtgcagaaggatcgaaagcaacctatcaaaggataaaggaaacgaagaaaatgaagtcgagaataaaaaaagacttccatctgacagtgatattgaagtcgtgacagactaaaatttatgtgaatttgatcatgcttattatgattttaaattagaatttgaaattgcggttcttgattaaagatccaagactctacctatcgaacaaacaatgagcttgtatttcttaatataaaactatttctagaattttgtctcattacagtaatttctagagaagaagagtgacctctatcaccatgttatttattatctccatcagttgtacgtgaaataattggagtggaaggagcatgacatacgctactaaaaaatagcttttcagctaaggaaaattaccaacggatacaatccgtcggtaattagaaacgaattatccattggtaaaagtaatttacttttaactatgataatcagcaacgaatttttcattggtaacaatgatatccttttaccaatgaatattctgtgtctaatgtaaccgtttaacatttgaatctttcacacgtacc

SEQ ID NO: 3 - DNA, 1160 bp, Olea europaea
  source 1..1160: mol_type = genomic DNA
  misc_difference 1..1160: note = DSI-B Allele S subspecies europaea
ttaaattgatgcgatgaccagtcacagttttctaatgaaaagagtgcacatcatagagtcatattgtttcaaattgaatgtgagtattcaaaaatctacattacgaaaagtcatgacctttttacaggtgcaatatagaccattaaatataaaattatgtgatttaataatcctcattaatttatgtcaaaagatccaatcatcccaaaaatacaatggtaaatctatagataggaacccctaattccatatttactctaaaatcagttcaagaaattttggtttctaaattctmttattttttcaaaataatctgttttttattattttagtgaaattaaattccatccaattattattaggaataaaattcagaccgaacaattttaattcgttcctatcctattagtgaagaatactatcatcacttaaatttgctgagaaaagtattttcttgctttaataattttgaaagtgtgttgtattttaggagacaaacatccatttaatatgttaagacctgtgggcaaaatttgtcttaagaagctgtacactcacatacgtcattttatttcatgtccatctaattttagcgtttcagtaaatcccattttgtgtacattttgatgcacatatgttgatttcgataatttgaaactgtatccaatattttgcatcagtgaatcacgattttatcatatttttatgcatgatttttttatttatccaacaattttaacacagtggcatccaatgattgcacatagagtctctcaagacttgtttatttggggatagtgactcttatgactactactagagagacacacatgcatcgtacgtgtagcgtagatataaaaataaattatttgtgttaagcattagttacttcaaatttaaacatatgttgctaaatkttttaaggcaacaacattgcaaaaatgatgtattcagaaccatacacaacaaacaattagggatcaaattcttgataaaaaaaaaaaaaaaaaantgtaatattactttgtgaatgagaccgtcatcgattattgagctgcttattttcttaaatatttcatacagtgcctcaacttcagttacggtgactgcatgacaatgttttcaatgaaactgcattagtccattccttgtctaggatc

SEQ ID NO: 4 - DNA, 1153 bp, Olea europaea
  source 1..1153: mol_type = genomic DNA
  misc_feature 1..1153: note = DSI-B Allele S subspecies laperrinei
ttaaattgatgcgatgaccagtcacagttttctaatgaaaagagtgcacatcatagagtcatattgtttcaaattgaatgtgagtattcaaaaatctacattacgaaaagtcatgacctttttacaggtgcaatttagaccattaaatataaaattatgtgatttaataatcctcattaatttatgtcaaaagatccaatcatcccaaaaatacaatcgtaaatctatagataggaacccctaattccatatttactctaaaatcagttcaagaaattttggtttctaaattctcttattttttcaaaataatctgttttttattattttagtgaaattaaattccatccaattattattagaaataaaattcagaccgaacaattttaattcgttcctatcctattagtgaagaatactatcatcacttaaatttgctgacaaaagtattttcttgctttaataattttgaaagtgtgttgtattttaggagacaaacatccatttaatatgttaagacctgtgggcaaaatttgtcttaagaagctgtacactcacatacgtcattttatttcgtgtccatctaattttagcgtttcagtaaatcccattttgtgtacattttgatgcacatatgttgatttcgataatttgaaactgtatccaatattttgcatcagtgaatcacgattttatcatatttttatgcatgatttttttatttatccaacaattttaacacagtggcatccaatgattgcacacagagtctctcaagacttgtttatttggggatagtgactcttatgactactactagagagacacacatgcatcgtacgtgtagcgtagatataaaaataaattatttgtgttaagcattagttacttcaaatttaaacatatgttgctaaatgttttaaggcaacaacattgcaaaaatgatgtattcagaaccatacacaacaaataattagggatcaaattcttgataaaaaaaaaaaatgtaatattactttgtgaatgagaccgtcatcgattattgggctgcttattttcttaaatatttcatacagtgcctcaacttcagttacggtgactgcatgacaatgttttcaatgaaactgcattagtccattccttgtctaggatc

SEQ ID NO: 5 - DNA, 967 bp, Olea europaea
  source 1..967: mol_type = genomic DNA
  misc_feature 1..967: note = DSI-A Allele s subspecies europaea
ggcctccacttaccttggcattcaggggttccatccgcgatttgaggagatcaaagaattaatagagagtatgaaaattactcctgcacaagttgctgaagaactaatgaagagtgatgatcctcaaacttctcttgaaggtctagttaattttttgaagtgcagaaggatcgaaagcaacatatcaaaagataaaggaaacgaagaaaatraagtcgagaatataaaaagacttccatctgacagtgatgttgaaggcgtgacagactaaaatttatgtgaattcgatcatgcttattatgattttaaattagaatttgaaattgcagttcttgattaaagatcgaagactctacctattgaacaaacaatgagcttgtatttcttaatataaaactatttctaggatttgtctcattacgtgctttcttcattgtaaaatgtagcgccccgaaaatttaataaaataaaactatttgtgctacttgttatagtttcatatttttggaaagttaatgtactagggtaaaattgcgttattgggtcaaatatgcagatttcgataggacgaagataagtataacaatattgagattgttggatagctcgtaattaattatgtatattaagttggagaaaaagttaattcggataaactaaacctaaattattgaagtttaaagttgtcaataaatattattttcttagtgattatttatttatttatttatttattattattaatttttttaatttgtgaaagtgggcagcaacgtggaattgttgggatgaaattaaaatgggttgctttattttgtactagatagaagttttgggtaaattggactttcactttctataagacacttgtcctatattttcatttatgaaaccaatttccccaaagaaaaattcagattttctttcaccatatagtataagtttataaacacagtagcatgctgaa

SEQ ID NO: 6 - DNA, 963 bp, Olea europaea
  source 1..963: mol_type = genomic DNA
  misc_feature 1..963: note = DSI-A Allele s subspecies laperrinei
ggcctccacttaccttggcattcaggggttccatccgcgatttgaggagatcaaagaattaatagagagtatgaaaattactcctgcacaagttgctgaagaactaatgaagagtgatgatcctcaaacttctcttgaaggtctagttaattttttgaagtgcagaaggatcgaaagcaacatatcaaaggataaaggaaacgaagaaaatgaagtcgagaatataaaaagacttccatctgacagtgatgttgaaggcgtgacagactaaaatttatgtgaattcgatcatgcttattatgattttaaattagaatttgaaattgcagttcttgattaaagatcgaagactctacctattgaacaaacaatgagcttgtatttcttaatataaaactatttctaggatttgtctcattacgtgctttcttcattgtaaaatgtagcgccccgaaaatttaataaaataaaactatttgtgctacttgttatagtttcatatttttggaaagttaatgtactagggtaaaattgcgttattgggtcaaatatgcagatttcgataggacgaagataagtataacaatattgagcttgttggatagctcgtaattaattatgtatattaagttggagaaaaagttaattcggataaactaaacctaaattattgaagtttaaagttgtcaataaatattattttcttagtgattatttatttatttatttattattattaatttttttaatttgtgaaagtgggcagcaacgtggaattgttgggatgaaattaaaatgggttgctttattttgtactagatagaagttttgggtaaattggactttcactttctataagacacttgtcctatattttcatttatgaaaccaatttccccaaagaaaaattcagattttctttcaccatatagtataagtttataaacagagtagcatgctgaa

SEQ ID NO: 7 - DNA, 1201 bp, Olea europaea
  source 1..1201: mol_type = genomic DNA
  misc_feature 1..1201: note = DSI-B Allele s subspecies europaea
ttaaatttatgcgatgagtagtcacgatttttcaaatgaatatggtgcatatcaaagagtcaaattgctttgaattgaatgtgagtattcaaaaatcaacattatgaaaagtcatgaagtttttacaggtatagtctagactattaaatataaaaatgtgtgatctaatgatccacattaattttagtcaaaagatccaatcattccaaaacgacactcataaatctatagataagaatccctaattctttatttcttacgccaaacaagtttaagaaagattgatttccaaattctctcatctttttagactaattttttttttaattattctagtataattaaattccatccgtattattactagaaataaaattcggcctgttggtgaagattactatcatcaaatcacctttgatttgccgacaaaattatttttgtggttcattaattttgaaagaagcattgtattctattttaggagacaaacatccaattgattatattaacacctgtgcagtgaccaaaatctgtcttaaggagctgtacatttgcatacattgttttatttcatctccatctaaatttaatgttccaataaatcgcatttttgtgtacatttgatgcacatatgttgatttcgataatttgaaactttatcctatattttgtttcaatacacaattttatcatagctgtatataaaagatacagtagaagataatggagaatggtatatttcattcattctaatggcagtatttatacaggtattcagcatgtgttaatcctataattaagccctatgatataggagaaattaagggcatattacgagaaatattacaggaaaatatttagagtaaacatcctaaaattttgtctgtcatcctagaatattgcacatgatgatcatattttgtcatgcccccgcaagattatgcttctatcatggatgccaatcttggatcgatgaagaagaaatggtatgcgagatagagccttggtgagtgaatctgccagttggtcattggtgtggacatgagatacacgtagtctgttattgagaacttgatctcgaacaaaatgaaagtcaatgtcgtcatgcttcatggaagaatggaagatcggatttttgctcaagtaagtagcatcaatattatcgcagaagatagttggaatagtggatgagtgaaacccc

SEQ ID NO: 8 - DNA, 1201 bp, Olea europaea
  source 1..1201: mol_type = genomic DNA
  misc_feature 1..1201: note = DSI-B Allele s subspecies laperrinei
ttaaatttatgcgatgagtagtcacgatttttcaaatgaatatggtgcatatcaaagagtcaaattgctttgaattgaatgtgagtattcaaaaatcaacattatgaaaagtcatgaactttttacaggtatagtctagactattaaatataaaaatgtgtgatctaatgatccacattaattttagtcaaaagatccaatcattccaaaacgacactcataaatctatagataagaatcccaaattctttatttcttacgccaaacaagtttaagaaagattgatttccaaattctctcatctttttagactaattttttttttaattattctagtataattaaattccatccgtattattactagaaataaaattcggcctgttggtgaagattactatcatcaaatcaactttgatttgccgacaaaattatttttgtggttcattaattttgaaagaagcattgtattctattttaggagacaaacatccaattgattatattaacacctgtgcagtgaccaaaatctgtcttaaggagctgtacatttgcatacattgttttatttcatctccatctaaatttaatgttccaataaatcgcatttttgtgtacatttgatgcacatatgttgatttcgataatttgaaactttatcctatattttgtttcaatacacaattttatcatagctgtatataaaagatacagtagaagataatggagaatggtatatttcattcattctaatggcagtatttatacaggtattcagcatgtgttaatcctataattaagccctatgatataggagaaattaagggcatattacgagaaatattacaggaaaatatttagagtaaacatcctaaaattttgtctgtcatcctagaatattgcacatgatgatcatattttgtcatgcccccgcaagattatgcttctatcatggatgccaatcttggatcgatgaagaagaaatggtttgcgagatagagccttggtgagtgaatctgccagttggtcattggtgtggacatgagatacacgtagtctgttattgagaacttgatctcgaacaaaatgaaagtcaatgtcgtcatgcttcatggaagaatggaagaccggatttttgctcaagtaagtagcatcaatattatcacagaagatagttggaatagtggatgagtgaaacccc

SEQ ID NO: 9 - DNA, 24 bp, synthetic construct
  source 1..24: mol_type = other DNA
gaacaaacaatgagcttgtatttc

SEQ ID NO: 10 - DNA, 42 bp, synthetic construct
  source 1..42: mol_type = other DNA
tgtaaaacgacggccagtgaacaaacaatgagcttgtatttc

SEQ ID NO: 11 - DNA, 24 bp, synthetic construct
  source 1..24: mol_type = other DNA
tggtaaaaggatatcattgttacc

SEQ ID NO: 12 - DNA, 20 bp, synthetic construct
  source 1..20: mol_type = other DNA
cccaacaattccacgttgct

SEQ ID NO: 13 - DNA, 24 bp, synthetic construct
  source 1..24: mol_type = other DNA
ttaccctagtacattaactttcca

SEQ ID NO: 14 - DNA, 23 bp, synthetic construct
  source 1..23: mol_type = other DNA
stattttaggagacaaacatcca

SEQ ID NO: 15 - DNA, 41 bp, synthetic construct
  source 1..41: mol_type = other DNA
tgtaaaacgacggccagtstattttaggagacaaacatcca

SEQ ID NO: 16 - DNA, 25 bp, synthetic construct
  source 1..25: mol_type = other DNA
atcgaaatcaacatatgtgcatcaa

SEQ ID NO: 17 - DNA, 24 bp, synthetic construct
  source 1..24: mol_type = other DNA
tgcaagcccatttcaascayyttc

SEQ ID NO: 18 - DNA, 25 bp, synthetic construct
  source 1..25: mol_type = other DNA
cttawtggcttcacattccaatcta

SEQ ID NO: 19 - DNA, 935722 bp, Olea europaea
  source 1..935722: mol_type = genomic DNA
  misc_feature 100501..835222: note = DSI locus - 0.7 Mb insertion-deletion sequence
caacaaattctaccattcgctagatatatccgacgatgactactccaagttatgtgaagtgggagttgaacttgacgtattactttgtacacttactcgcaaagaaacagaatggaaatagtctaccaatgatgtgagtaactttcttgccttcagttaaacaattaattgtaaagtttggcaccactttatattatccaaactagttttgaacggcaatatcagtgacgtaacaaaggaataagttccattgaatcatacaattcaaaggggttactatattgatattagcaaggtcattcggaatagtatcctatacatcctagtgaggttagccactagtagtatgggatgcccctctgtataatgcacccatgggaaaaaaactaagtttggggatgtgtgaatcccaccagtggaaaaatgaagtaattgacttttaaagtaagaaattgaattaacttatgattgtacatcgttgtacttgattcttcacacacacacacacacacacactcattttgcattggaaaggttacaattttgtttttcactataactttgaagtatttcatgaattcgttatcatattctcaatcctgagccataaaaacaagtgattagctaaattttgtaattgagtctttcggttgtgtgttttatctatgtatttgttaagtatattagagtgttgttttgtgtttgttcgaggacaaataaagaattaagtttgggggtttttgatgagtgcgtttcactcattaaaatggcacttctaaagcataatttcaatttatttttgagcacttttgagcattttgatgtgtttgatcttgttattttgtagtttaggtaacttggtaaaaatggcataatttggagcctagaatagagtaaaagtgttgatcatggaagtgagtatagagtgcagatgaaagaagaaaaaaataaagcaggaaagagataagaaaatgaggccaaaagtgaaggaaacatatgggaaccatggtgcccatgaaaagactagaaaaaccaatagaatgtcgggtgctgcaattccctgccataacaaaagaggagcagaattaggggttctgaggagccagcaaggtattcattgcagtgttgtggtaccaataatggtcatcgcgattccccccaaggtttaaaaatcagatttttttggaaagttttttaccaaatccagtcccaaatcgtcttaaaacattgaaggactataaatacaaatatgaagacctacaattgttggagaagaccacctaagtggcaagaaatcacgaggttaattgagagcaaggaagacaacaattagttgaagaattcaagcgccagcttagtttttctcattttttccttctccatgttcttaatattagattgtattattcattttcttatccataaacttatttctagatctagagttcgatgtaaactaacttgagacatatttagattctaatatagcaatttcttttgattttttcacgagtttatttgtgttgattcttgcacattgcttttaattacctgattaatagtagttgaatgatttgacattttaaatctcgatactcaagagagggagatttaggtacatctgagaataaaataacctagattttgtaggtattgagagaaaatatgaaatctttgaggcttattccatttaggaaccacatttttgataatttctagatttttaattcgaaaaagagatattagaattaaaatagagatatgttctatttggtactcaagagattgaatagaattaatttagggttctttcctataaaattaggaaaaattgatagaagtaactgtaaaagttgagaaacattgttaatagactggtaaaatctttccctaggctttctcaagctgataaatctcgtataatttgccttgttttacttgagattgtcaccacttctactttagattagaacaaagacattgattttaacttgattttctagataaagtgaaagttaaaataatcatagtacttagtaggaattaaatattaatccttgtaggttcgatactctaatttcattcatttattataaaacttgatactgtacacatgctgtatgatttacgtcgtcgaaaaagcgtaacaaatttttaattcaaccttccaaaaagatttttgatatttttggactcttttatttgcccaatccgagcccaaaacttctaagacttcaagatactataaatacaaatctaatgttcaattttgaaggagaattgaagggacaagattcaagaaatcatgaaggaggaaaaggcagcttcgagaagtgtagaaccccaaataattctagacaccttagtggcactaagacatgaatattggatgactaaagtatacttcagatttttagtctcatttgagacccattttcgacataggaaaggaaaatgatatctcaataaaagttgtaactctttgagttagctttcaaacgcattttgaattacctcaattggatatcgggagaagaagttatgatagaaacactgaaagctgtgcagtgtcaaccggactacaaccggtcgaccgaagctgcctgaaatgaaaattctcgtttttctctagaatttaaatatttattttcatcaattattttctcaaaggaccacccacatttttgacaataaaaaccccactaaattgaagcatttaacctcaaacttaaatgacacctatgttttctttcttaaatgaaatttgacccttcatttgctttaaattatgggatatttacctgtaaatagagacctcatttcactcattttgtctcacaccaaaagtaagagcttttacatattaaagaaagagtttccaagagagaaaaagagagggaggaaaactatttttcctagaagtttaagaagtgttttcaagcatcaattctcaacgattttcaaacatccaaggagttcatttcttccaacgtccaagtttcatcgaagttttcaatccaagttttcaaatattcaaaagcatcaattaaggtaggtagaggtgcaatgtgtttaatcgtgttaagttataagtttcgattcatgttattgtttgtatgtcaaatggtactccgttacgacatatccctttatgttaatggttgtatgtcaaatggtactcaggtacggcatacccctctatgttgaagaaatgttcgtatgtcaaatggtgccctcgggtatggcatatccctttatgtcaaatggtgcctccggatacggatacggcatgtatgaaaagttataaagttaatattttgaaatgtatagcttgatcacgaatgcacctatgacacctattgagtttttcaactcacgggtttaatcccatctctacagattgaaggaattctacctcgggtatggatggaggagaagatagagagtgatgcaacgagcccatggaaatccggtgaataagtgatttggatttatttttatgaaatgttttacaatgttatttctttaaagttttgaataacgcagaatgcgagaacaagttatgttttcttcaaataaattacattttgttgttttgaaaaatgattcagtgtttttgtttaaagtatttgaagtatttttatttaaattattatccgaagatgtaagcttccgctaaaacgtatacacttgttactaaaccaccgattaagctaagtaaagtaagtagcgttctggtccactaggggtcggagcgttacagcgtggtatcagagtaaggtttagccggttctgtagaccaagtatattttttttaaaaacaaaaggaaaatgaaaagtttaaggtattccatggcatcgtgcatccatccatcaatctcatcctatggtccaggtatgttcatgtttaaagttaatgattatgtttatgttatgatattttgatatgatttagagatgtgttatttaaagttatgtaatggacttgggcaaaagctaagggcttaaagggaattgcatgatatgaaagtttaaatatttgcatgttttctttaaacaaataaaaagtatgatgtatgtgaaaatgcaacagatatggcttgtagaacagctagggcatatagagaagcattgaaccgtagaattgctatccattcctatgaaaactatgtaactgatccgacctaaccgcttagcaaacatgtgtatgacatctatgagagatgcatgatggcggttaatgctggaatggagatcacgcatatcgaggccataaataacatcacacactccctcccacctcaatggggagatatgggagtcacagttcgagatgaaatgttagaaggcaacctaaacctgttcgagtttaagaggtattgccatgccttgattgatttgtgggatgatgtaatccatgaggagcctgaggaggaacctttggctgaggaagaagatcccgaagaagaacccgaggatgatttagagaataatcctgagcctgagccacaggttgagatggacatagagtccggacctaaggcggaagacttctccgaagatgaaactccactaaagaagatccgtagaacttatagggattagatttaaatccttataatagcttcccttatgtcaagaaataaaatactatcttctttgctttagtattcgaagaatgaaactaataagaaccatatgttttgtctaaaggaaatggcccgcgcaaaccagaacttgataagagacctcctccaagcggttcaagacctaggcaggcaaaacccgaaccatgttcaacccctaccactagctcctaatgttccaaaccatgcttcagtggtcgagcaatttcgaaggcacaagccccctaccttcaacggagcagctgatccacttacagccgaggagtggcttcgtaagttggagcatatattccgattgatagggtgcacgaacgcttagaaagtccagtgtgctgagttcatgttctccggtgatgcaagtcattggtgggactcaatgtcaaggacaaggacccctgagcaacaagcagaattgacttgggaacaattcaaaggggaagtaatggacaagtactttccccagtccttgagggatcacaaagaaagtgaattcctccaactcaagcaaaagactatgtccttgactgagtatgagaggaagtttgatcaactttcaaggtatgctccacatctgatggatacggaagataagaaggtacgaaagtttgaacaagggctgaactcagatataagcatgatacttatgtcccatcgcttcactacataccatgaaatgctggaaagagctcatgctatttggtaccagaaaactagcgccgaacaacatggtcaattgttcaatcaaccggacaatagtaacatgggaaagaggaatggaatggccaggacaagggaaaaggcaagtggcataacaagaaagctaatggaggagccaatgccagcaaaagcattgtgccggttattgcgccctgttctaagtgcgaaaggacacatcgtgacgagtacttacaagcaaaaaatgtatgttttcgatgtggcaagccaggacatatcattagggattgtcccacacatgcccagaagaaggatgataacaacgaccagaactagaaaggaaaagcacgagttttttcattgactcaacaggatgcagaggaaaactctaatgtcatagcaggtactctactgatagccaatacacctgcttatgtattgtttgatgcaggagctacacactcctttgcttcaacaacttttatggctaaatctagtattacctgtgataagtcgaaaggtacattagaaattagtattccttcgggcaaccctttgaatactgatagaatagctaagtcaataagtatcgaagttgagggaaaaccaattgaagcgaacctatacatgataaaaatgaaggattttgatgtaatactaggcatggattggttaggttgtaattacgccaccatccgatgtaaggaaatggaagtatcatttcagaaactaggaaatgaaccattttctttcttggaatgaagacaaaaccccttattcgactagtatcggctttacaagctgagaagatgttgagaaaagaaacatgtcaatgatatctagtaagtatctcaggagagaaacaagagacgataagggttgaagatgtaccagtagtacggaaatttgtagaagtgtttttagaagatctatctagtattccatccgatagacaaatggaattcaccatagacctaattcccaggacggcaccagtatctaaggtcccatatcgaatggccccaaaagaactacaagaattaaagaagcagttgcaagaactcctagatatgggcttcatacgaccaagcgtatctccatggggtgcgccggtgttgtttgtaaagaagaaagatggaagcatgaggatgtggatcgattatagggagataaatcgattaaccatcaagaataagtacccactcccgaggatcgaggatctgttagatcaactgaaaggaactaaggtattttccaagatcgacttacgatcaggataccatcaactgaaagtagagacaaaggaatacctaagacagcttttagaactcgatatggacactacgagtttacgatgatgtcgtttgggctaaccaatgcacctgcagtgttcatggacctgatgaatcgagtgtttcatcaatacttggataagtttgtcatagtcttcatcgatgacattctgatatattccaagagtaaggagcaacatgaagagcacttgagaataaccttagaggtattactcaaggagaagctgtatgccaaattcaagaagtgcgagttttggcttgaacgagttgaatttcttggacatgtagttactgcacaagggattgaagtagatccagcaaaagtaaaagcagtaaccaactagaaagcaacaacaaatgctggcgaagtacgaagttttctaggattggctggatattatcggagattcatagaaagattttccaaaatagaccaatgattcagcttacaaggaagggagtaaaattccaatggacggaaaaatgcgaacaaagtttccaagaacttaagcagaagttgatattagcaattgtattaacaatgcctgaaggtacagaagggtttgttatatacatcgatgcatccaagcgaggattgggatgtgtactaatgtagaatggaaaagtgatagcctatgcttcaaggcaattaaagaaacatgagcagaactacccgacgcatgatttagaacttgcagctgtagtacacactttgaagatatggcgacactacttgtatggatggaagtgtgatatctacatagatcaaaaaagtctcaagtatttcttcacatagaaggaattgaatatgcaacgaagatgattgttggacttggtgaacgattaagattgcactattcactaccatccgggtaaggctaatgttgtggccgacgctctaagtagaaaatcaattggacaattgacgtcactacccacctctcaagtggagttagtcaaggacttgaaaaagttgcagatcgaagtggttaccacaccaggacaagtcactgctcatctagcagctttaataattcgacctactcttagagatccaattatagaagcacaaaataaagactcatttttgcagaagattaagaatgaagttggtaccgataaaaaaaaggactttggaatagctgaggatcagacactgatatttagaggaagaatttgagtgcctaaggatgaagccttgagaaacgagatattaaaagaagctctttccacaatgtacactgcatatcccggtggtacgaaaatatatcgagatcttcgagatacattttggtggagaaatatgaaaagaattatagggctgtacatgcagaagtgcatggtatgtcaacaggttaaggcagaacaccaaaaaccagctggattgttaaatcgactagatatacctgaatggaaatgggaaaatatgacgatggactttgtggttagattcgcgaagtcagcaagaggaaataatgctatataggtagtagtggattgactaacgaagtcagctcatttttttccagtgaaaatgacattcagtttagaccaattggcacagttgtacattaaagaggttgtgagattacacggtgtacctatatccattttgtctgacagagatccaaggttcacgtccaaattttggaaaagtctacaaggagctatgggaacgaagctgaactttagtacagcatatcaccctcagtccgatggtcagtctgaaaggaccatccaaactttggaagacatgctgagaatatgtgttttggatctaggaggtaattgggagtcattcttacctctagtagagttcgcttataataatagtttccaagcaactattggaatgacaccatacgaagctctctatggtagaagatgtagatcccctattcattaggatgaagtcggagagaagagagttttaggactagaaatagttgaaaggatggtcgaggtaatcgataatatccgtgcaagaataaaggcagcacatgatcgaaaaaagagctatgcagatacaaggaggaaggatttagaatttcaagttggggataaagtgtttctgaaagaagcaccgatgaaaggtgtacttagatttggaaagaaatgcaagctacgaccccggtatatcggacctttcgagatacttgatagagtcggaaatgtggtttaccgactagctttgccacctgaattatcggcagtgcacaatgtgttccatatatcgatgacaaagaagtatgtacatgatcctaatcatgtagtgagttatcaaaccttgaaggtacagaaagatttttcgtacgatgaactactgatcaagatattggatcgaaaagtgcataaactaaggaataaagagattcagctggttaagatacagtggaatcatcacggcgtagaagaagccactttggaaaaagaagaagaagtcaaagataagtatccaacactattcgcataatcagaaggtaaatttcgaggatgaaattttaattaaggtgtgggggatgtagaaccccaaataattttagacaccttagtgacactaagacatgaatattggatgactaaaatatacttcagatttttagtctcatttgagacccattttcgacataggaaatattcgatttggaaaacgatacataaataaaagttgtaactctttgagttatctttccaacacactttgaattacctcaatcggatatcgggaaaagaagttatgatagaaacacagaaagatgtgcatgtcaactggactacaaccggtcgaccgaagctgcatgaaatgaaaattctcgtttttctctagaatttaaatacttattttcatcaattattttctcaaaggaccacccacgtttttggcaataaaaaccccactaaattgaagcatttaacctcaaacttaaatggcacctatgttttctctcttaaatgaaatttgacccttcatttgctttaagttatgggatatttacctataaatagagactcatttcactcattttgtctcaagccaaaagcaagagcttttacatactaaaaaaagagtttccaagagagaaaatgagaggaaggaaaactatttttcctagaagtttaagaagtgttttcaagcatcaattctcaacgattttcaaacatccaaggagtgcatttcttccaacgtccaagtttcatcgaagttttcaatccaagttttcaaagtttcaaaagcatcaatcaaggtaggtagatgtgcaatgtatttaatcgtgttaagttataagtttcgattcatgttaatgttggtatgtcaaatggtactccggtacggcatatccctctatgttaatggttgtatgtcaaatggtactccggtacgccatacccctctatgttgaagaaatgttcgtatgtcaaatggtgcccttgggtatggcataccccttcatgtcaaatgatgcctccaggtacggcatgtatgaaaagttataaaattaatgttttgaaatgtataacttgatcacgaatgcatctatgacacctattgagtttttcaactcacgggtttaatcccacctctacagattgaaggaattctatctcggacatggatggaggaaaagatggagagtgatgcaacgagcccatagaaatccggtgaataagtgatttggatttatttttatgaaatgttttccaatgttatacctttaaagtttttaataacgcagaatgcgagaacaagttatgttttcttcaaataaattacattttgttgttttgaaaaatgattcagtgtttttgtttaaagtatttgaagtattgttatttaaattattatccgaagatgtaagcttctgctaaaatgtatacacttattactaaaccatcggttaagttaagtaaagtaagtagcgttccggtccactaggggtcggagtttcttcactttaaattgtatagatttcacatctcatctcgtgaatcaaataattcttctaggatttgattagccaaaactagaggatatgatttgattttgttttagttatttctatggaaattttcaattccatttatttgtgttgttgatttattattttcaattaattagtcactaattgaatgattaaatgctagtcaattttgacactcaagagaggggaattgaggcacgaccacaacaataacacaacctatattttacgggtttcgatagaaagtatagaatctatgaagcttgatccatttaagaaccacaatcttgataaatcttgatttcaatttggaataatgatattggaattaatttttatccggcactcaagagagaaggcaaaattacattaggattcttacttataaacatggaaaattgatttgagataactagatttttgaaaatcatatttgatagttaggtgaaatcatactctaggctctcctatattgattaattcatatggcttgcatttattcattgaatttgtcacaatcgtctctagtttagataaaacattgattcaaaaattaattcatctagataaaataaaggctacataattataattcttagtataaaattaaattacaattcccgtggtttcgacactctccgttcatatattacaaaaccttaataccatacagttgcgttatagttcacgttgtagaaaacatgtagcaagttttagcttttggctaatcatgacataaaagacatagaattgatttaaaaaattaaaagctgaatttaaaatggacttaggccctgttagaaaattatgggtattgaaattaagagaaaacatattaagtctgagtcagaaacaatatatgttgaaactattggaaaattttactatgtccaaatcaaaaagtgtcaatttgcctttagcaaatcattttacactttcaaatgatcaatgtcctaaatctaaaaaagagtttgagagaatggagagagtgccatactctaatgcaattaggtatgtcatgtacttagtggtctgcgccatacttgacttggcatattccgtaagtgttttgagtatatatatgtccagtccaagtaaagcacactgggaagctatgcaatggcttcttagatattaatgaaacttttgatttagaaattcagtttagaaaataattgagggtattttttaagaggctataatgattttgatattgtttaattcatgtataagctggaagtctcaactttaaaaattattgccttattctgaggcaaaatatatagttgccacaaatgctataaaagaaggaatatgactaaaaggcttattacatgaatttggttttattaaagaagttctttatttagatagtagatcttgttatacatttaagtgaaaatcttgttttacataatagatctaaacacgttgatattagatttcattttattagagattatatttcacaaggtgttgtggaacttgaagaagtttttgctaattttaatccttctgatgtaagagagaaaatgatgtcatgccttggaggaaccattgtaagagaaactggaaccactgaactaaggtggaaattgttggatgagtggcataatgatttgacattcaccaaatgatgtggctgctaactggattatttgaatagttgattgttgactgaattattagttcacaaagagaaaacgtgtttctaccttggtaatacttttgtggcttaaagcgttctaaccattttcactcatttgttaatgggatagattaatgagatgctgccaaaagtgtcctccaaaagtgtcctctaacaacgttggattggatgaccttctggttgcttccataatacatctggattgaaggtttttttggatagatacatggtattgtctccttacgtttaggctctgcaaatattctctctctaaaatttgttttgttgacctttaaaggatatttcatcttctatattgtgtaccggttttttattattgagagttaatctataaatctagcactgagtgctgattaaatcgttcttaagtgaatagttgatacgaagttagaataatgtaaatcttgagtgatttcggttcttggctccctgaagttgtacctttggtcgatttggctctaggtagtgcaatagtttcttccagtgatgagagctcaaaagggaattagaaactttgctccgaacattttgccttaaggcgaaaattcttgtgttatatttctctttttacacttttttatctattgttgtgtttgtttaaaatcgcctaatagttggatttaatcatgatagtgacttacgtgttcatttttatgactcaaatatggttaggagtcttgtgagattgcgtatttgatttttacttggaaaggaagtttgtatccaagttgaataaggaaaagaaattctctcttggtcaaagttctatgcacaattgtaacctaattttaatagattttcttaccttttagaactcttctaaggtatggaacgtggcctataaatacaaggctcttctgtcaattttgtttaaacattattgttatgtctgtaatttttccatattttcagttaatagacatcattcatctacgattaactctctttgttcttctttacttttaatattgcttttttttgtgatctttattagtttctattgtgtcatcaatctcattcattacaatccctccgggtctaacaagtggtatcagagcttggttcttcttctgtgaattggttgaggttttctcagagatgactaccatgaagtatacacttcgctgctagatcgcaatacaagattttctttgtggcaagtaaagatgagggctattctgggtcaattggattttgatgatgcgttgctaattttgagaagatgccaattaattagacaacggaagagaaacaatgaagggatcagaaggctctatcgtagatccatcttcatttatccaaatatattttgcaaggtgtcttgaaggagaaaacaatggctactttgtgtcttgaaggagaaaacaatggctactttgtggttgaaactggaacacttatgtatcactaaaagtctcatgagtgaattggctctaaagcagaagctatattcccattacatggcagaaggagggtcactggaggaacatattgtcgtgttcaatgaaaataattgtagatctggagatgttggaggttaagtacgaagaagaggatttggctttaatcctgttatgttcgctacctggctcttatgcatctttcaggacaccattttgtatagtcgagatactttgattatagacagcgtctatgaagctttacagtcaaaggagaagttggagttacatagagagatgatggggtcttgtatcgcatggtggtcgacagaggggcagatcgaagaataacaacaagttgttttgcttctactacatacgtaagtgacatattcggaatgattgtgataagtagtaggctaaggtgatttattcacaaatcgtggagtgcaacttttaactttagatgaaacaaatgtagttgaggatttttcagacggtggagacatgatgtggaccatgttatctaacgtggaatctagacctgacgaggagtagattttcaatttggcatgtttgcatcatatgtgttccaatcgaaatttctttcaaacatatgaagccattcaacaaggtggagttgtaatgggaaacaactagtcttgtagtattactaagatcggtcgagtaagatttaggctgtggtatgggacggtgagaacaattgatcaggttcgacatgttccaattctgaaaaggaatctcatctcgcttagtactctggatgcaaaagggtataaattctctggtagaggtggagtcttgaagatccgaaagggttttcgggttgtactagagggacggaacgggtctcaattgtacatgttgtagggaaacgcagaactagttaggagatatctggacaagtttggtgctatggtggatattcagtttggtacagtacctcttgtgacgggctctggttcggttcagaacattgctctagggagcgttggtgattcagctttgtcatcaatttcagcagttgcactgcatttagttactagggttggatccattgagcgttggtatcgtggtgtcagtgatgtctgtaattcttttgaggatgttgaaggcgacagttctagcaaggggctttttgttcagacattttgtatggtttctcctataaggtttccttcaaccttgtttggtaaacattaattccctggtggaattttgggaactcgggagtaggattcaggtgttacttgtggacaccgtgcagaggacaatggtttatatagagagttttggttattgtgttgaggagattggccatttcattttaatgcaaacgggtttatttctcaggcggagaaattttttggaggtctactcgttgcactgaaattcaagtcaaggtgaagattgttaggtttttgtgactcaaatatgttaggagtcttgtgatattacatatttgatttttacttgaaaaggaagattgtatccaagttgaataaggaaaagaaatcctctttgggtcaaaattctatgcgcaattgtaacctaattttaacatattttctcacattttaggactcttctaggatttggaacttggcctataaatacaaggctcctctatcagttttgtttaaacattattgccatgtctgtaacttctctccatattgtctgttaatataaatcgttcctctgcaattaaatttctttgttctttcttactttcaattttgtttcttgctgtgatctttattacttcatattatgtcattaatctcattcattacaatctatcatcatccaatattacggtgttaaattgctatgtgtaattggaaattactgttggagtgttctattaggagacattatatttgccaaaacaagtatcaatttcatggagctttagaattacataaaacaatttgaatacttcagaatgatgcttggtttttagttttgtactttccggtgaggattttaaatgtcgtttgaatgatgcattttacccatttttcttttcaatcaagtttgcaacgatgattaatcatccatctaaatcaagttattacacagaatctgaacaaggtgttgctcaggtcattgtacgagggaaagtaaactttgagagggaaccatggctaagcatttgagaaagagccaagagtcttgtacgacagatgtaggagcgtcatcctaagcttcgactcactgcaaaacaagttttgggaaaaatattgttctcgttcgctatgttatttaatgaatatacatcctttttcattatgctataaatttgttttgttcagacaaccacaattctttaatctcctatttcatgccgtgtacaatttacgtatttcttgggcctaggataactggggaatcaaatatgggagattgtggccgaggacaattcactcgtcgtactcatattttcattcctacattaaccgcttcgaagctaacaagaatgcagtattgactatggagatcaatcattgctataaaaaaaatgagcccctcaatattaggaaagattatttccttctgtggaagcaatatacaactgacaatgtattgttaacttcttcgttcggctggaaatgaatatttattttttatataatattaaactaagaaaccaaatttagagcctaaataaattcaattgtgttaagaatatatttgttatctatttcttattcttttatttcatggttctaaattttccagattcaactaaaagtacttaagtacacaggtaatagtcttttatacttttatacttcatatttattgtgtttatatttcaagccttgttacatatgcatgtatatacgatcattttttttctttttctttgaaataaacatcaataatatgaatatctgacagccttcattcctagtatctctaatctgcaaacttttattacccattactttcgtcatgctctttcattatgaaaatattaatgaaaataatggactcaagtatttactataatatcaatgcaagtaccatgaatttttttccaacttcttttatgagctaatctcattctttgatctacagcttaataggcagaagaaattccatgatactaagtgcttgcatgctattgtattgacggtggtgtttgttgggaatctacggatgatgcgcaacgaaaataaaaacaattttcaattttcaccaaagatctactttctgtttagatagaaactgtgatggagattatacattttacaagatctgcaaactcctttgctattctttcgttccaacgatctcaattcgccaaccgcagctgtttaattgttcaatctctcagaaaacatgattataggattatgatttttttcttcttgtgctagcaaaaatgaattctctacaaattttgaaaaccctagtcatatttatataagtccaaacgggcttgacctgacccgatctaatatttaattaacccatttaaataaattcggtccgtgaattaattaatccagttaattaattcaggcctataaatagtaatctaattaattaatttatccaacgttggttaaattaattaattgataaattacaatattctaattttctttttgtgtgcgacccatcaggttctctatcatgatgactaacaacgtgaaatattattttgacctaatcaaaattgataaattaaaacaccctttgatttatcacgaattcacactgatcgtcccagataaatatctagcaatgtatcagaacaatacatgtgaaggaaaatgttacgtggtatgacaaaaccaaactcgttcatttatcgaaaaaaccaaactcgttcatttatcgtgaaattataattctttcgtcaatatgatctgatcaattacgagatatggaagcatgtcaatctcgattatcgatcatatctttcacgtcattattaaatcaatattgtcgaaaacttcttttcgacttctaagtacatcttgatcaaggatttcgttatcaacttaattgaataaaatgcagattataatttcttactatctaagagtgacgaatcctctattagtcattcacaaccttgatacaattcttgacatacccgaacgatgctgtattagtaacccttggcagagcaacattcaatactatcaaagcatgactatcctcatataagacattataacgacctcaagtcaaagtacaatccactaccaaatgttagagattaactactgacaatcaaatagttatccatgtggaatctctcggcgggtctccaatattttgttctataacaaaacatccacgtactcattcaagtgtcaccacactttaacttgtgagatcagctacttacttcacaagtaaaaaatacaatacatgattgtctacctgtaataacgatatccgtatctcatcattacttatgaccatggatgatttaagattcaatcatatctaatttatatctgacaatcacaactctttgtgattaataaattatcaagtttgaatctacggactctactatttaatttaactgaataataattaaataatagatctactataaaattgtatcaattatatattaaaagtatttatattcaaggttgattggatttagggcataacacttacagtgtttccacaaaatctttgctacagtaaatatgtgtatatctcctttcatgaaatctgtcctcgtgagataaaacttcttaccccagacaagtatattaaaaaaataaataaataaacaacttgtttgtattcactagaataaagattgtagtattcatttagtttaattagaagtcccaactagaaacatcatttcactcccaattgaagataaattgtggctctaattgggctagaaccatagtccatcttcaaaaaaaaaaaaaataaataaaataaaaaaaaaaaaaaattggaaacactcagtaacagtacatttgaaattaccaacacaattttcttcatctttaaccacagcaataagatttctaccttgctaaatttcagcaagcatagacaaccataaaggtcaaacaggtaaagcatttccacaaatttccttcccaaacggtccataaattcaattctttaattacaacattattacccattgtgattaaagttacacattcagattaataatttcagtgcagaaacgcagtacaacgagtaaagactggaaaaaaaaaataaagattacaaaaaggtgcctgtactttaaatcaacatcttcattccaacaagcatattatccaaaaaataattcttcctcatacataattgcacattttctttatgaaagcaccacaaaattgcatcattacgaactttcatacaaatttgttctttttttatttttttatttatttttattaaaaagttatgacaatgcatcataaaaaaatagtttttagaacaaacacctaggggctgtttgagccatattttttgtcccataaaataagaaatcctactgttgcaaacagtatctctcttgacaactccctgatttagctgtaccatgtgctacatatttacaccattctttcacatttgcccttcattcaaaccacaagaaaaggacaataggggcacaaatgaaaattagcattgtctgaaagcttaattggcaacaagtcatgtgctttgggtcccactatgatgtgacagaaaaatgcattcttgggaaaaaaggtggatcaaacaggggcctatatgcaattgtattaacaatcttttcttagaattaagaagttccacttccacgtacttaatcaaatgaactttcttgcacattcttcctcatttccttgcagtaacacttgcgattacagacttttcaactctaaaacaacttctcagagagatttttctaattataaagtaactaatcatctcattgcctgcattgacatatccttcttcaccgctagatattttatagcacatagttgcatgcattggtaattgcacttacttttctaaatgtatggttgaaaattaaaacaagtggaaattacactagatgtcaaaattcgggtttacatttacaaaaatgtcacttttttaaagtgcttgcaaaattgtcatttttgggcatttctgccctcagaataatttcaatgccttatatatctttcattaatgagacatgactagatgaaaaattgtcacatagtcaacctccgttttttttaaacactatttcaaaaatcacgagaggtaaggccgttcttttagtgcccatttttcccctttctacattccttcatgcaaaagaccactctttctcccccatccattgaatcaagcccgaaataaagccaagtaaaatcccaaagaggggagtaaagtaatttttactgtacaaaaaagtctcccagcgccaatatctccactgtctacgtggtcatcttcgtctccaccactgctgtcatcctcctcctctgtacccttcggtaccatcatggccagctccctgctgccattagccgcagtagccagctctggaattcttaatgcttatcattaattctcgtccccgttaactccataaactctagtccccactttctctcacttttcgttgttctctaatagctcagattaaaactttcttgacccagatgagtgatggaattttgttttattttttgccaatttcttatgttttattctgtttactgttcttgactaaacctactaacgtggttaactggatttcatctgggatttgggtattttctatttttcaacatgatcttgaccttaataaattgggttttgataaagcttccaaatgtggtgtcaaaaaatgttggatttataatacttaaaaaaaaaaaaaaaaggttgaaccccaagcttaggggctcccaccgaccctgccctgggccattgtggagaaggtaaatcgcaggatgtgcctcccaggagccagggtggagagcacatggataggccaaggttgttaacccatatggtaactcccgcttgcaacaaagccaattccaccttacggggaatcgaactctgcacactgccgcgctgagccctatccgccctcccctttgccactgggagatatgccctgggggcggatttataatacttactttaccaatagttgttgtgaacacaatattgctcgagatgatcaggaactccgaacaattcaatagcgctacgtgagtggggtgtggtggttccatttttggtgctagtgtaagtttgttgcgatgattggtaaaactattttgatgataattataaatcctaagcttgttgatacttgtttgattctaagtatcaagtataatggttttctaaaagattatgaatccttgaatcatagatttaacaaaaaatcctattttagtcacaagttacaggcagcaccaataaggcttcacaagttcttaatgtgaaaaattacattatttattgagatctatatcttaattttcgaaaagaagatttgttgttgtagttttttatgactcacttatcagtttgtgatgatttttggtagaagatggtggtgacaataataagacagtgtaagtcacaattttatataaattacacacactttatcagaatttaatatcatcacttagccaaaaaaaaaaaagtgattattcttgctgggcttttttttatactcgcccgaagggatgcatatagaaaaatcttgtgcgattttgggtcctttttatcaaattgaattttcattgaattttggtggataaatttctaaatatgtggcaatttttggtgcagcaaattcctgtgactatgaaaagtcaattttctgtggtaagttataaagaagatgaattgtatctaagcagatccgaaaatcgaaaacaaggacaaggcagtgattaagatcattgtggagggttttttttgcttatagaggtataattttaatgctatctatgaggttaagcccttatggtgttttacttttcatcttgagagttgtcgtctttcaatacgaatcatgtttgatcatttatttctgaactctaaagatgatcgtcacattacaaaaggattatggatgttcgctatatttatcattggcttatgtgttcatgtttttccacatcatgatgcaaagttggctgttaaattgttactcctcttggtaccacataaattctgtcctcctagaagagattttgtgaggcagtcataacagaaatcaaacttcgtgcagaagattggaagtatgttctatgaacagattgtccttgcaaaattcgtaatacattatcttacatttcagtagttggctttatatttctaccttcttggggctaatttatagcatttatatgaatagtcgttgcaaaaatatgagctccatcagatgaggtgtggtggccttacatgtatagaaaggcgggtaggcaaaaagcacaacattgcactgtcgaacgaagcaaatagctacaaaacatgcaacagataaagtgcgggcctacatacagtcaggggcagtgcatggatgaacttgtatattattcgttactgtgcatatttctgtcgactggtgaattttctataatgttatttcttgaaaattgagcagactgtcgttaaagcttttagccaaactccattatgagacatcgggccattggataccgtttgaaaaaattgtacttttgcacccgcctaacatgttggcaatattatccatgtgctttaagttggtctactatttcttaaggaagccaatagttacgacttatgcaatggagcttagcttgcattaaatttgttttcatggcgtcaggggcttattgcacatgaatgtataatgtttctgactgttggaaattcgatgaaaaacttcaacgatttacgtacggtgaaatgttggtattgttatccatgctggtgcaggcgggtaaattttacgtggtttgaatgttgtaacacgatacgtgaatattcgggtagtgtcatgagttgacgcccccattcatggtgttcgtatccattcaatggttatgtacaacttgaagtagtctattatgaaacatacgtctcactttataatgttttataaaatgattgaattatgattctgagccataaaaatatgacaaagccatgacaatataacttactattaagtcacaaaaatagttatgagacttgtaggaaacttgaagataaattgtacccatcattgaagagtcacaatttactagtaaaggtatacttaagctacaagaaccatcacaccaattgtctttggaatttagatgagattggacttggtggttgggtgataaatgattataattgcttcctcccttgatgccctgttacaaatagccatcattctcatgggttcgtcatgagcagcaacaaagacttcgacttgaacgagcctctaccagttctcggttcatccccattatttccaattaacatttcatcaaatgaggatgaagctaaccctcacattggtggggaagccattttctctgttccattttccaacttggatgaagtcgtgactgaagataaatccaacgacaatgattggttggtgtatatgccatcatctaaggtaattctcatcttatctgatgattatgatgatgaaaatgggggagaaggtttaatcgttgacgaagaatgaattgggcagaaatgaattgtagttatctatgtaataagttatgtatagtctatcttttttaggaatctgaatttggtattgtctttatcaaaacttcagcataagcatgtcccaatctgtacctatgtgtttttttttatatttcggaccaagtgttgagcatgacaaaacaatctgtcgggaacgtcagatgtaatgtcgagctgtcatgcaatatgttgtctatggatcaatatttatcttgtaaagttgaacatttatttcacttattgttcaataatggaatgagaatgccaatgtaagccgaagacaaaaatgtaagttgagaatgtgttggaaaacactggaagttgagactacctttatgcaaggtatgaatgccacaatgaaattaaaaggttataagcatgatgaaaaggaatgaagataatgaaactaataaattgtcgaaatttgtaaaaattacaaaaagcactccacctctaatattttgcttataattgagtccaagttttttaattgcgctcctcttttgcttcgtagtaatactgaggaacattgatgttgctacaatagttatgtgttttctattgagtttttaaaaatcgttttttcacctttgtgcttatcattattttaaaaaatcggctatttacctttgtccttatctttcatgttgtttaccaaccgtttcagtgaaattgtcaactttgcagccgtttgtcgagaatgacagaagacatttgatgtgaccaacaatttatttgttgagatgttgtacaggtcatcaacatgaggatccttattttttatgccaacataagagcaataacagtcgcaaacgatagtgacaataaaagcatactataacttgacaatgtactatgtagtaggggaacattggacattcaacgtcaacaatgaaatcgagtggttgtttaagaattgcattgggggttaaacatgtggttcagttataacctactcgaccacagagtgtacttcctaaggcgtgtggcatattcatatcttgatcatttatgtcgtgtcgatagtctacctagaggacgacgtacaatgggaggtaaaacaggagtacgaattaagcaaggaacaacccaatctacttcttgcgaaagatgatatattgcttcactataggcatcccagtattgaggtaatcatattgtacgttttggggaacatcctctaaggtaatcaagttcgctgcacagtttgcatccattcccatattgacactcaggaggttggttttcaaaatactaatgcagagtgcagtttccttatgaacatatatgtaccaatttaagttttcatcttcacttatttctaccggaggtatattcaagttcaggactttgaacttcaattcaattttagtgcagggttgaacaataccaagtttatcattcaaccgtaacataagtttagctgtgataatacttctcggctctaaaatacaagtggatttgtcctctctccacttccattcgtcatcaatgtgaacaaactttctctcatgtgatacgatgaatctcaaatgacactcatacctgaaatgttgggattgcaattatgagaattctttacatttcatgtgtcaacatttaataccatcaaattggagttttcaaatattcagatacctgcaatagcagaaagggatataaagggtttcaacaattttcaagtgccgaaatcgacagttaaattgtctatcctgacatgtagtaaatgttgagtttgatagttcaaatgtctaacccaatatttggttttttggaagaaattattgaagacattaatggtgataattagttctcaattataacatcacaatatcttcccaaaactgaataaggaataaatcaatacttcatttaaataaggaataactcaatgctttattacaatatgttggtatttttccccttcaaaaaatatatcaaaaataaaatacgtcaatgaataataaatcaaaaaagttcaattaattatgaccatgtcgtattaaacatttaaagtagtaagctatgtgatgaaaatataaacaatttctagtagctcacatttaagacggatgatcaatccaatagtttttccttgttgaggattgaatggagagggtgaagaagaaggtaggttctctattcatacgtgtttgtgtgtgtgtgtgtgtgtgtgtattttttttaactgttcacccccttttttaacaaaaattcatattatctatataataatcatatctcaaatgtttaaaacatacaaaaacaaatcatcacatcacatcattaattgcattcaaatcaagcatttattgctcctaaaaaggtgtcataagggtaaaatgttttgcaacaaaaaggtgacattttttgaagaaattagtgcaaaagggaattttttgtgcattttcaattttagtgacatttatgaaaattcaccttaaaacaagtattaaactattactctttcccaaatttatgtctatatatacctaaacttactcccttaacgtgggtagacccacgtggggtcatctggggtcaagtgatcatatatatataatttttttcttttaaattagtgtagctgcagaaattcttcttcaaaatcaaactttctagattgaatacattttacatcatactctaattgttgtttgttatattagcttttacaattgaaaggggaagtcgtaaatggagtttgataatgtcatcttttatgaaggatctagattttatagttgttattctaggggctttggattcttcaagtgtatctacacatttgtttgatgtatgctttgcctaaaagagtgtttagaaaagttgaaggcattaatttaatcaatatgagctagctcttggtttaaatgatgattccaatcaataaagcttaccaattttcatcaaattgtaggagttaaaacttcataacatttaagtaatagtaaattattaatgaaagggacaactaatcctgacccattcagttcctttccatttgcaggtaatcgctatcctttttactttctcctcctcctcctctttgttcccattcttctattagggtttaccaaatcctcttccacatataattgatattagcatgaatctatgtataataatttatgacaatctgaactttctctctattttggtagttagattgtagaatatacgaagaacaacatcgtatgtgaggctagtttagtatttgataacagaagaacgaggatttcacacttccacatcgaagaataacaattataaaatcgtagcattcaaaaaactcccaattattgttcccaaaattgaccatgttgcaatgataagaatagcaaaattttcatacgtttctctttaacttttttttttatttcagattacacaatacagattgtagagatggttgtaactactttacagaaaagggaagtgctatggaatacactgtcgtggtatggagaatgtggtcagaaatccataataaagtctgaccacaacgaatgaattgattacctttatgcataaggaaattttttttcttccattgttttctacgataaacaagaaaaaaatggattttgacagcattaatgtgatcttattccattatgtagaaatgtgatcttccattaatgttatgctattttttcttttaaaaaaatcatttttatttttgtcctcacaatacaaaacatcctgctttgtcccattacttaacgttaaacgtgaaaactggatatagattacaaattcacagttgctagttgtatctaccaagagttcaagaatcatttcttatttttcttttggccaattctgtaaaacgtgcttgcatgcttataaccgagttccaagtagtgatacttacttgaaatcacaaaatcgaggttgaattacttgcctttgatttacttgctttccacaccgtcttgtacccgtttcttggtcagaaattcaatgacaaaggtaggaatttatagtcacaatccaagaatcaaatttgagatgttattattccaaaatcaagccacaacactcatgttgttttctctcattctggaaatcctagtttcaccatgtgtgttttcagtttttggtagaaaggaagttatatggaagaagttgactgatggaggttaagtttcaaatttaatttccaaattctcattccaaaatttatctccatgcaaactgggtaggttcaatccacatgagcgttttgttttctttcaacatctctcactcgcacacgatgagcttgacttgattatgatataattcaattatattaacctcaacatctccaagttcatactaataaatggatcgtgcgactagcgagttaatttaagagcacacaacaatatacacctgttagggatatatagcagctctagaagaggaattatatttctcgctataccttaaacatattttgtaataccaatttgagtatttctgacccctcaatttattttagaacatactcaactttctcatttataatgtattcacaattgtgtcacaatactcaaatgattaacacaattatttggccggtaaatacaagctgaggtgttagttaaatagtctttttttcctggttaaatcccttcatttcaagtcagttgctttcttagacatgtcccatcaaatcgaatcaaccgtagttattaaagtagcaacactgaattaaaattttgagaaacgatcgaaagtcataagggtatataaatgaggtcaaatgtgcctcagattctcatacaatgaagaaatagggatcaattatttcatttctcattggttgttaaagcacacgtggtatgaaacaggtgttatgatattttctctctttcttaggtgtatgtctaatcttacaaattgaacatatcgtacagatcatagttcaaatatttctcaatacctaacctgagttcttctcatatttattcctccaggtaatctcaaattgaaaactcgatctggctataaaattggtctaatggatagcaaaataattcataccgattacttgttgtaatctcttcttaatatctcatcaaggcgattggattatgtacacgatatgatcactgtgtctcatctcaagacacctcaaagtatctgaggtgattgttcatatgagtgaaccaatctcaacctgtttgacatactttatgtgtgcatatacaatggtaatctaaaaatcacaataaaagattacttttaacatgtgaactcaaaacattatttattgatagacatatatgaaaaagtttacatagtgtacaattcaaattttacgcaatctcagagatttaacatgagtcataaaaatatctcgagggatatgtaatgcctcaacccgctagtatgaaagcgtcactcaaacaattgtacattagctttagacttagaaattagctaaaaaaattcatatatatatatattaaataactaccaatgaatttcccattaaaatctacttttagatagtaatataatattaacataatttcaaaggtatttattaaagaagaaaagagtcaagcgaatccatgcatatgcctattttattacgtgaatagtggcaagtaaatatctaccgaacaaataaaaggtatgatagttttccatgtgtgaactactttaggaagtaagaaagagagtaatttgttttgatttcccattttcgcacggtaagttttaaaataaactcgtttgcatagttatcaatgttgaaatttcataaaattttaaggaaaagtaagaaacatcttataatatgacgtatccaaaatttggcttctgtcggtgacatatgaggcattaacatatttcccaaaatcccgttaacactaactaaacaagctgtattctttttctatctcgtaaggtaagtgtcaaaataaattgtttgcatagctatcgacctcaaaacttcatcaaaatttaatgtaaattagaaaactccttataacatggaatagtcaaaaattagcttctgtcgacatcatttgaggtataaaaatatttttcaaaacccaacagcgacccagttgaaaggtaaattggtgtagttcacttaaaataacatataaaatttcacagacatcaaaacctcatgatttccaatttattcagtagttaatccatgagactatcaaatacaattggtttcatccaaaaattccaagtaacggttgagttataaatttttgcagtcaaggcggaagctagaaaacagcaacactagctagtgcagtttaccttaagtgacataaaatgctacaaacattggattgacatgattccaagtttattcagtagctactctatgtggttatccagtgccattggttttgtctaaaaattccatgtagcgagtgagctatgaatttctaaaatcaagacaaaaactgaaatttttaaaagacagcaatactttaatttgctaacacttttttttttctttctttttgtaaacgatgttttgtaaattgacttctataatatatatacataattttaaacataacttattcatgaagaaatattcttaaaatagttcaacatatgacgtccatagaaatccatataaaaagaaacaaacttaaatattttatgattgaactaaaattattaaatcaccggctttctccatagcatgttgcatcatcctctatcatcatccacgttccatgaaaatccattcaacctgtacgaagggaattaatccatgagtttgaaactctatacatatcatcggtgtatttcgttatcaaattagaaatttcaaactatagattcataccgtcacacgtaaatggatttccggcaaaattcaattactatagcattatcataacacatagagccagagaatgatcattcaaactattgtagtgccgaagcaccatagctggaggtatcatttcattcaaaaatttattgaaaaatcataatttgaaaaccaaaaaaacacttgcacatctacctacctcgaattttcttggatataaagaacaaaatgtgtagaaagtctttcttcttcttactcttgttatttcttaagcttaacttgacatgaaatatatttttttgagagaaaataagagtaaattcggattgaggaggagtgtagtgaaaaattgacattcctcttcttgtaaccttcctttttaatgaaaaactaaatgggggagttgtattaccattaaatttgttaaatttgatctttaactaagaattcgaagagtttccaattcgaagagtttctaaaccataaaaaaatgattcatataaaaagttctagaaaaaatctacatggtgatttgaacatgggttgcctatatgaaataccatgtagatgaccattaaggaaacccgtttattcattaaatctttgtattcaaatttacttaaacttaatctcttaaattattgggcttttaattaatttatggcttgggttttcataattttaaatgggttgagcttctatagctcgtttcttaaatgtgctaggctcgtagtgctatatcatcaaaaaataattgtctatttcattttatttcttgggcttctacaggataggttttgtaaatggacaactaccatttggtacgtagaaatattttgtaaactcacttccttcttgcctatgatttctcttacaaaattatattttgtatcaatgtgtttggttatgctgtcttgggatccttgatagatgcaatagctacctaactgtcacagtagatcaacataggtctcacatcactactaacgacttaaatgctataagattctccttaaacaaatagcttcttgtaccgttgaagcacatgctacaaattctgcttccattattgttgttgattatgattttgtgaatctattggatttttttttgtcatttttttttattccttgtgattttttggaagacgaagataaaaaagtttgataaagatgaggccggtataaaagatctaatatcacatatccgtttcttgctactccaagagatagtgtcattattaagaaagaatacatatcccgaagttgatttgcgctcatctaggtctccacccaatcagtatccgtgtattcttttaagcacaaatcatttccttgatggcacagggagtaattagcaatatacccttcaggtatttccttgatagcatagggagtaattagcaatacccttcaagtatttcaatatccttttaacagctttctaatgccatcttctaatattggattgataactactagggatgtcaaaaaggctcggtggcttgggcggcccgttgctcggctcgtgaaaagcccgagctggctcggctcgtggctcggaccaaccgagccaaagctcgggccgagccccaaaagggggcaatcgcccgagcccgggccagcccgtttaatttaaaaaaaaaagtaaaaataagggctgtcggcagctttatagctgcctattggcagcagttaacctgctgccaacaggcagcagatttgctaccgaattggcagcaaatttgctgccagttcggcagcagtctagctgccaacaagtagctttaattataaagctgcctgttggcagcaattacgaaggaaaaaaaagacaccaaaacacgagccggctcggtaatgcccgagccaaaagctcgggtcgagctttattttttttagtcgagccggctcggctcggcttgttcaaaaaaaagcccgcattgaaaaagctcgagccgagcacgagctagaagtttcggctcgcgagccggctcggctcggctcgtttacacccctaataattactaaccagacctagggcataaaaaatgtcgggatgagtacacatcatagcatacatcaacctcccaactgcagtggagtatggaactttggacatttcttcttttttctcgagagttttaagatagatatgaagacttagagtttcactttttgatacaggagtgtcaatgggattgcaattctccattttgaaatgttcaagaattttcttttatggctcttctgacagagcaagaagcctctttgaacgatctttatggattttaacacctaatatgtaatcaacttcacccatgtccttcatttcaaaatttgcgaacaaccatttcttaacggttttaatatattccttttcattcccagcaataagatatcatctatgtagagagacaaaattacaaatttctcgttggaccctttcaaataaatacagtgatcttaatccatcatgacaaaattgtacgagataaccgctatgtcactgtctagaagactgctttaggccatagatttatctattcaatttacaaacttttttctcttgacctattttactaaaacctactggttgttgcgtgtagattttttcatccaattctccattaagaaatgagttttcatgtccatttgatataattctaaatctaacaggccaagatagttaagagtatgttaattgaagtaaatctcgctactggtgaaaaggtattttcataatctataccctcctgttgagtataatctttgctatcaaaagagccttataactttctataatcccatcagctcttcgctttattttgaggacccatttgtttccaatggcttttcgactagatggaagatcaaccaagtcccagacctgattcaatttcatagactccatctcttctaccattacattcttctatttttcctttgcagggacatgatagagcttcttatactgaacttggttctttatcatctttaggagatactaggaaacttgccattcaatctcaaaatgacatttaagcatacattttatagtactcttacgaagtaaaagctccaatatacattttatacttggagttggagataaactattctcatttggattaaaaagaagtgcttcctcttgcacctcaattgatccatcaactacaactctatcatctaattcatacaaaggttctccctttttaatttctcctctactaggaaaatcactctcaagaaatgttacctcacgtgagtctatttcaattatagtctcatcttgatttttacctatgaacacatatcctttggactggtctgtgtatcttataaagacacacttcttgccttgagcacctaattttccaaacttacttgaggaatcatggatataggcagttgatcaccgagatctaagagaattaaatcagtagatctacctgtccaaagctgatatgttatagtaggtaccgatttagaaggaactctattcagaatataggtcacagttaacaaagcatctccccaacaggaaataggtaagttagcctgcaccatcatggacctcatcatttctagcaatgttctattccttctctgagcaacaccattttgttgaggtatactgggaataattaactacctaatgattctcttatccatcacatagttttttgaactcttcggatagatattcacaccctcagtcagttcttaaggctttcacctttctatctatttgattttctaccacatttaaatattgtctaaagcattctgatgcactcgacttatgagaaatcaaatagacataactataccacgtgaaatcatctataaaagtaatgaaataggaagctccagtcttgccctcacattcattggccacatatatctgaatagactaactgtaatggatgttcggttcttaaggctttaccaaatggtttccatgttatttttccaattagggaatgttcacaagtaggtaacaaaaccttagagattgaacctagctagccttctttggccaacctattcattctctcttgtccaatatgtcctaatctagcatgcatattgatgtatcaacattcaaatctttagaaaagaagaagatatattcatagaaaaacaacgatcaacataacaattataagtgtttggatcacaatccaacactacaaatccactttctacatgtctagatccataaaatatattaccattgtttgtgcgaacagaattagcacaaaagtttaaactgaaacctaatcttaaaagaacaacaatgaaaattaagctccttcgtatccccggtgcaaacaggacatcatgaaggagaatagtatagccaccatgtaaatgtaacttgcatgtaccaatctctttcacctccactctatcatcattgccgatatatattcactttgtaccacttggaaattgacggactgcacagacgcttctcaatccctagttacatggtctgtcgttcttaagtctaaaatccacataggataagatttagttagcttaacagtgcttgaaacataaacaacactaaaagaagtatttataagagctatcttctttagtttaggacattctcgagcaaagtgacccagcacctaacagttgaagcatttcagcttgcttttatttttctcctatccaaaccatttatccttcttattgtgcttgtgtttgttctttttaggtccctgtccagttttttcccctccactttctcgtctttgaaccagttcttcttacacttaaagcttgaaacttttgtaaaattagattcagcccctaaagcttgtcccatagatttagccatactaaggtgctcattctctagctctacatggcgggcagcatcggtaaatgctttgacactatcattgtgagtcagatcgacttcagatattctaaattattaggaagggagaggatcaaagcctgaacttgttgctcataagagagtatgtgaccagctgaattcagttccctaatcatagtagacatgatcctcacatgccatgtgatgtttttattagaaaatttcttgtaagtgtcaaatttaatagtcagctatctcaatctagtcaaactagtaccgctatatttctctctcaaatatgtgtggatgtcatgagtagtctggaattgttcacacacatgtatgagatcgtccatcacgaaacttaccaaaaattgcacgaacagtggaatctctgttttttcatgtttggtaagtttgtcaatcccttatccactgaacagtttgacctaccactgtgtcatgtgattaatgccctcaaggaagtcctgttcctccagtacataccaaatttcatggcgctaagtgttatagttgtcatcattcaatttgtcacccttatttaggttagttatgacactcttagatgctaggtccatcaaactattagagacaatcatataaatgtccatttatgtaaagatcattttgctctcatgcaaattaagtttcgtgataattttacactagacatggagttgaaagttcactaagttcccagtcatcatccatttttctaatgttatattatcaaaaaattaattttatagagcaaaatcacaagttctaagtcagaataactcaaactttttcaaccttagaactcctactaaattaaaagattaatcatgtacaaaatagcaagacattttgaataaatctgataaatatgaaacatatacattaatatcaaaatatcaaatatgtacatgcaatcgtattaaacatctttaaataaatactaaacatgagaaataaaatttcacattgttggataattttgaactaatcacacgtatctaaattaatcataaaattctcattttctaaattccatttcctcttcaagatcctgatcaaataactatagcatagaggtaatgaattatccacaacttcaatagcaacaccatggcaatatttagggagtgtcttcattagatgatacatattgtccacctcacatatacgttgtcccaaatgtattacttctcgatgcatcacttcagatgttttatgtgttgtactagattattttgttgatccatttcatagtttttataagtacgtaatttttcaatacattccacagcccgtgctctagtagcttttcctctaaggatgctaaaagtgcatgttgactcagccatatctgacaagcacaagagttgaaaaccagccacaatggatcctgtaacctaatcaagacctacacagcttatgaacgtatagaaaatatgatatattaaatactttcgaagtatttttcatttaaaaaaaatgagagcacaaaaaaactcccactaagcaaataccatttaaaaaaaaatattcttgatttaaaaaaaatatatatattcaaaatttaatcaagttcaaaaattatatatacaaatattttttattatcttaaaattattttaattgcacaaaaaatcaagaatatttgatggaccaatttcaaatcttctaaattgaatttggaataatcaatttccaaattgattatatatatatatatatatatatatatatatatatatatatatatatatatatatatatatatatatatatatatatatatatatatattaggaccaacttacaacttttcaaattgatattggaataaacaacatttaaaagtgttgggactgacatgcaattttccgaattgcgatttgtaataattgagggatgaatatgcaatttttcaaattaaatttggaatatttaacattcgaaagtgaggagaccaacatgcaaattttcaaattgcatttggaatattcaacattcaaaagtgtgaggaccaacatgtaatttttcaaatttcacttgcaatgtttaagggaccaacatgcaatttttttaaaaatggactttggaattcccaccttcactgcaatagtttcatttcagtgttttttctcaggtactcttcatcttcccaaaaaagcatatttctcagatttctgtcaaaacttcataaggctataacttcttcaattcatggacaaaaattatgttttttatatcgttgaaaaggtctcaagaagatatatccaaccatataaaatgggtagcgttgaacataacgtacaagcaattatcatacgatggaatctcaactttctcaactagggtttgatttttttttttctaaaatacaaatccaaatgaaatgaaatttttcagatatgttatacataatatcattaacatacagtataaatttcatgaattcatatgaagtatatcaaaagttgtcattaatgacattcaagcttggaaacaaaatcggaattcttgcatttcaattattctaaaacatttttagtgtgtttaagcaagaaaacaacgtacttaggctctaatgccaatgtaaactgttcttgcatgcttataaccgagttctaagtagtgatgcttacttgaaatcacaaaatcaaggttgaataacttgcttttgatttgcttgcttgacacaccgtcttgtacctacttcttggttaaaatttcgatcacaaagaaaggcatttgatagccacaatccaagaaccaaatttgagatgttattattccaaaatcaagccacaacactcatgttgttttctctcattctggaaatccaagtttcaccatgtgtgttttcagtttttggtgaaaatgaagttatatggaagaagttgattgtgggagattaagtttcaaatttaatttccaactcctccctccaaaattcatctccatgcaaatcgagttgggtcaacccacaagggcggcccattttcttccaacaagttttaatcacaccattcctttctcatgtattatagtaattaacttatagtgaacaatcgataactctcccataaaaaagacactttgaaaatcagatgactattaaattgtctattactcttttacattagcaaacttcttaccattttcccacaaaattgtatcatagtaataacatttacaaccattttcgctctaacttcgtcttcaaatgaatttcagatatcaaacataactggaatatataatcttatctcatagatttctacggcagaaaaaattggcccgaaaactcattgttgcaggaaaataggcatcgaaaactgctagtaatattgctcgccgatacaaatatctttttctaatggactaggaagtaaatgtgcattcataataagtacaaatgttctctttttttaatttatatgtatttcttttattaatatcgttatttacttctgcccttcacacaggcaactatgaatttataatctatctccagtcacagtcgcattatacgacacaaatgttacgacacttgaagatcaactaaagattggaaagacatatatattgttcaatgcaacaacagagacaatagaagaaattttagaacctcactaaagacaaaacttggagcattacaagtaaaacaaaaatagaagaactgaatgaggataatttaaactttttgttctcgacatatgagcttacactattttacgaactggaaaaacatgtggataatagaaaaaacataaccatactttttctattcatcacagttgttatctgagttgctatggacatttgccaaaaacaagttatccaaacccactttgggacacaagcctgtcttcaagatgttatatagacaaatatttctaaattgtcatcctaacactatggtgtaggcctgagttgtctgcagaaggattaaatgagcaaattaagagatgtaaattccaacattatggggtcaatagaatcaattaagagccaaaattatctatatattaaagcaagatatgtgtataccaaaatagtaatgtttactttatataccatcaccgctgtaaagaaaatcaatgaaaaaaaatctgaattctttctttaaaataacatggtatcagagcagttgtttccatatcctctacaatccgaaaccctataaagcagagacaagaacatttcacttgttgagaatctacttattatgtgcagcgaaaaataaaacaaatttatattcccaccaaggatctattttgtgattaggtagaaattgtacctttccatgattctgcaaactcctttgcgtttcttttgttcccacaatcttgatctgtcatccataactatccaattatccggcctccaatagaaattcacacagggaacaagaatgagagagaaccagggtttacttttcttgtgctagcaataagaatgaaaaatccaaatcaattccaatccctagccacttatttatataagcccaaatgggcttgacccatctcctgacctagtccattaattaattaattcacttaattaaatccgatccatgagttaattaatccaattaattaattcaggcctataaataagtaatccaattaattaatttatcaaatgcttgttaagttaattaatcagtaaatctcaatcttcgagttctctttttgtgtgtaacccattaggttctcaatcacgatgcctaaagaagtgaaatattattttgatctaattaaaattaataaattagaatggccttttaatttatcaccaattcacattcatcgtcccagattgacgtttagtaatgtgtcacggtaatacatataaccagaaatgtcagtggtatgataaaaccaaactcgttcatttaccatgaaactataatcccttcgtcaatatgatctgatcagttacaagatatggaagtgtgtcaatcatgattattgatcatatctttcattccactattaagtaaatacaagtcgaaaacttcttttcgacttctgggtacaccttgaccaagaatttcattatcgacttaattgaattaaatacggatcataatcttttactatctaagagtggcgaattctctattggtcattcacaactttcatacaattcttgatatacttaaacgatgccgtattagcggcccttggcaaagcaacattcaacaccatcaaagcatgactgtcctcatataaggcattatgatgacctcaagtcaaaggaccaattccactaccgaatgttaaagattaattactgacactcagatagttatctatgtggaatatcccagcgggtctccaatattttgttctataacaaaacatccacgtgttcatttaagtgtcaccacactttagcttgtgagtttagctacttacttcacaagtaagaaatgccacacgtgatagtctatccgtaataacgatatccatatcttgtcattatttacgaccatggatgatttaagattcaatcatatgtaatttgtatttcacaatcacaactccttgtgattaacaaattactaatatttgaatctatgggctccattatttaattcaattgaatattaattaattaaataatagatctgtcgtaaatcgcattaactatatattaaaagtgtctatgtccaaagtcgattggacctagggtataaaatttacatcaccatggtcgaagtaggctcacatttggaagagtctccttcatcatctatcatgtccgaacttactacaaaaatggctaaggtactgtccaaaaccttagctctaaccccaaacaattgacatggccaccgcatcaatcgaaattaagctggataggaccatttacgcacattggtctcaagtggtggaaatgtacgtatccgataaagacgagttggggtatatcaatggtaatcttcccaagcctccatcgactgacctaaccttccaaagatggcataccaacaatgccatagtgaaaggctggttgatcaattccatggatctatcaatgattggaaatttcattagattttcaatggaaaaaaaggtgtgggacgccatagcaacaacctatttcgaagggagtgatacctccaagtgtatgatctatggtgttgagtaacacatctaaaacggataggtggctcattagagaactactgcaatgacctgcagagattatggagagaaattggcttccaaacgttgaatctgatgcagttatgtagatattcagaaatataacagtgtggtacaagaagaccgagtgtatatctttatgaatgccctagatgatagtctagatggcactcaaataggtgttttacaaatgaaaccatttcccatcatggagcaagggtacacctatgttcgacgaaaggcggcacaataattagtgacaatatagggcaactctattcacattgatctattatgatgtgtgaggtccatccccaaaacttactatgcttgggtatcgatgattgtactagtatgacgtgattataattgttaagatacaaagatgaagtttttgatacatttcaatccttttacgagattatttttacccaatattgcccaaacctagggttctttactccaataatggtggcaaatatgtgaatacttagtttcgtgatttctgtcaccaacatggaatattcatgagacgacattcccgagaccctgaagtaaatagggttgccgagtggaaaaattatcacatccttgaggcttcttgaccccttcttcttccagctaatatgcagtcattattgggtagatgcaatcacaatgatcttttatgttattaacagaatgccatcacaagtccttgaaatgtagacttctctccaagctttattcacatttgttaccttatcttcagttttgataattcctccacatgtcttaggatatgccgccttcggtcacctttacaaggatcaatgcactaaaattgatcctcatgcaatttaatgcattttcttgtaatatggcatacataaaaaattgtatagatgctacgatcccgctcattggcttacgtatgtgtcaatagatgtcactgtaacgccctgacctgcatatatgtgtgtgtgtgtgtatatctatctttaaaaaaaacaaataattcagtactaaaacataacctctattgacgtgaaagaaaaactttaaaaataatgttgttgttttagtttttatctcaaacggaaattggcaaaataaattcgttcatagctatcgaccttgaaactttgtgagattttaatgtaaagtggaaagctccttataatatgaaatatccaaaaattggcttctgttggcagcatatagggtattaaaatatttttcaaagccctgcagggactcaggttggaaagtaatagcatactttatgtgtcatataaaattctacacaagttgaattgacatgatttcaactatattcagtagctaacccttgagattatcaaacccaatttgtttcatcgaaagatcttgagtaacaagtgagttatgaatttttgaaatcaagggcagaagttgaaaaatagtaacactacccagcgcagtttactttaagtgttaaataaaattctaccgacattgaattgacatgattctaagtttgttcagtagctaacctgtgaggctatctaacaccactagttttgtctaaaaattccaagtaacgaatgagttaagaatttttaaaatcaaggcagaaaccaaattttaaagaaatgacagactttaaatcactaacactatttgtttggtaaacggagattggtaaataaatttttagaacacatatttactttaaaacatagcttattcgtaaagaatgttcgtagaatagatccacacatgacaccataggaatcttatttaaagaaaacatgaacatttcataatcaaactgaagatattaaatcaccggcttctcaatgacatgttgcatatccatctgctatcatccacaccccaacctagtcaaatcaatttgtagaaagggaattaacccatgagtttgaaactcgatatatgtcatcggcgcatttcgttatccaaactagaaatttcgaactatagattcataccatcgcacgtagatggattttcggcaaaattcaatcactatagcattatcataacacgtagagctagagaatggttattcaaactattgtagtactgaagtaccataaccggaggtaccatttcattcaaaacatttaatgaaaaatcataatttgaaaatttaataacacttgcacttctaccgatcttgaattttcttgaatataaaagaataaaatgtgtagaaggcctttcttcttctcacccctgttattcggttaagtttaacttgacatgaaatatatttttttgagagaaaataagagtaaattcggatttgaggagggatgtagtgaaaaagtggccttccttttcttgtaaccttcatttttaatgaaaaactaaatggagttgtattattattaaatttgttaaatttgatctttaactaagaatttgaagagttcctaagccataaaaaaataattcatataaatttttttataaaaacatctacatggtgattcaaacttgggttgcctatattgtagacgaccattgaggtaacccagttattcattaaatctttgtaatcaaatttacttaaacttaatctcttaaattgttgggcttttaattaacttatgacttgcgctttcataatcttaaatgggcttgtggtgttagatcatcacaaaataatagcctagtttcattttgtttcttgggcttctacaattacatttctagaatctgagactttgtttacttttcaaacaccaacttctcatcttaaggaaagaatcatgattaagagatgaattggctgtggtttgattgaccaaggtttattcacccgaatatacctactccgactgagattgaaggcattgcagagaaagaaagaaatcctcccattgatcctcctcactcttcagtatccattgtcttatctccagagaatatcattgagatacactctgtttgctctccaattacaccttaaatttctaaaatgataaatgccactacccctattagctatgggtttcctttcaggtataatcatggtaagccactaaattgatactctcctgaggtgaaacaagaatggtcaaaacatcttattgccagttatatatccgttaataagttctctaatccaatgaagagttttgttgacgatctttcatctcatcacattcctaccaatgttaaagatacgttaaaggatcatagatgggtccaagctatgaagaaagagatagaggccctactaaaaatagacatgggtactcgtcttactatccaaaggaaagaaaactgtaggatgcaaatgggccttctccatcaatacaaagcaaatgggtccatagaatgatacaagacaagattagttgcaaaaggtcatacccaaatatatagaattgattgttgaaaaaccttttaaccaatggctaaactgaacatcggttaaagtcctattatctcttgtcacaaatcttgactggccattacatcagctcgatgtgaaaaacgcattccgtcatggtgatctcgaagaaaaatttatatggatatccctttcggatatatgctaagtttagaagcaaaggtcatgtgcaaattttagaatactatatgttggagacaatttccttgagctttttctaggagtctaagttaagcaatgaagaaatatggctttcgacagagcaattctgattacactctattttttgaaacatgagaaggtaatattatagcactaattgtctactttcacaatataagcattgtccaagtgaagatcatatgaatattgtaatgcaaattctctaagatgttggttagacaggaaatttgcttcaggctatttctcatttattagaggaagcctagttatttagaggaataagaaatattaggtaatggcgttatcaagtgcagagatagaatttcagggaatgaccaaaggactatgagagcttctttgactcaagagacttttatctgagattgggtttgctcccaattgtgagatgaatctattttgtgttaatagaatggctattgacatttcataaaatccagctcagcatgatcagaccaagcatgtagaaatttaacggcattttatcaaatggaatctcgaagctaagataattttttttccttttgtgtagtctgaagaccaactagcagatatgctaacaaaggctgtatgtagtaggagttttcacaactcacttggcaagatgggcatgatagacatatagactcggacatgggagtgttgatatgggttgtctgcagatggattaaagaaacaaattaagggatataaattcctttgttatagggtaaacaaaatcaatcaagagccaagattatctacagactatagcaagatgtgtgtataacaaaatagaagtattgtttactgtatctataccatcaccgttgtaaagaaaatcaatgaaataaaaatttgaattctttctccaaaataacatatgggatagctttgttgaaagagaatctctcactatactagaaaaccttgcaaagaaacctatcatatgagctacaaaccagagtttcatcattcaatggtacatatatatatagaacatacaatttcctattcaataatattacaagaaaatgaacttatgtatgttctaattcttctctttgtaggggttacacttactgctaaagtgaaaatcactttcttcattaatcgtgacatattaacagctatagatcgtagagaatggtctcaacacacaactatagaaactctttaccatccacttcttttctctttggatttggaaacaaattagttccagaaaataactcctcctgttcgtgtgctattcttctatagggtataaacaaataaatacaaactcgacgagttaatagaaaattaatcattgccacaaaaaatttcgcctcccgttgaacattaattcatatgaatcgcaaacttattaggagtttacgtagggataatttctaaaacattttactaaatatataatacagctatatagttattatcatgtcatgactattgtaacaagaaaaaaatatttccaatatctttttgacatctaaaatagcatgcatattcccctccagaagaaattctattaggtgaaagctcgatcataaattatttcaaacacaacagagattctggtatatggcttgtagtaattgtaacaaaaatactcaaccacaattattatattgtagaaccctaatggaaaactgaatgatgtgataagaactgagactgatgaagaaatgctattctacctcaaagtggagcacaaaaaaatctatcagagtatcgacacaaaatcatatttctattcacaatgacggatgcaaatatttagagttagtagaggcacaatctgacttataaaaaatttacaaaaaattaatgtgttcgatatcttattacaatttttctctgtacattttcatactttgataatatcccataattacatcatttttaatactgcaaatacatccttctcatacatgcaataaaactatcattcaaataatttttggcaatggatacactttcttatttaattttcgcaaccaatttttgtgcaagatcactgaggccttgtcatcctttcaaatcttcgtcaatgtacatgttaagaatctatgtatctaattgattatcaagttcgaagatatctcttgctttaaaatttgttggataatactcacatagtcgaattactttgttcttgtcaaaagtagcgaatgaattatttggaaacaaacacgcaacatagaggagtaagtcactattcacctctaaaaaaaagttcattcaattcttgaagttgcatttcaatgatggtataaaacattttcacaagaaagtgatgcaaatttgtcactgtagcacgtcatgaacggtctagaattatgcgcatatcatccatatttggaatattgatctcacgagcttcacagaatgaacaaaccattcgaaaaaaagaattccatttataatctcttatggtttgaaactgtactttacataatttcttcaatctcatgtcatttacaatatcttgctctttcctttgtaattctttcgacaattcatttgaacttctcgacatctttctaatgaaatgtagattaaatgcaaattcaaattttaatattgtccccaataaaatgtctacattaccttacaatcaagttaatcaaaaaactgtaatgagaatcccaacatttatcactacaaagctttagagtagtttcttgattgagacccgttctgcttgatattttaccaagtgcttcaagaattttgagtctttgtttcttttgaataagatcactccccttagccaatcctccaacaatattcaccaatccatgcatggaagtgaagaatgcttcaatttttcggatgtttctgtgtaacggctacaagagcaagtagaagttgaaaagtaaagcaacgaatgtaataagcactgtgtactaagagtgtgcaaaccgcaagtggacaggttgtgctcaagtgataaagtagacttttttagtccgagctgttgatccctcaaggaacgttttctttcgattacacaactttaattaatttaattctaacaataaaaagaaatacatacaattagaattataattttgaaaatgataataattaaaaactatatgaaaataacaaaacataaaactctcggaaattttaaaggaaaacatgttgggatcatggtttcactatattttctcctaattaatttttccataagctaatttacaaattactcaattatgatgttaaaccagacttttcaagtttagttaattacctctctcgagtgaaattaaccctaattgattggtttaatatactatatatttgtgtcgattaaaatcaaacaaccgtattaaatctttgtgaaaacagcccaatggatcactcagggttagacgtatatctctatcacttactcttagtgttactactatttggtctaaaatgtataatcttctcttgaatttgtacaattaactacacacaatcatctattggtcatataaatgaaaatgtagtaacaataatagtgaaaacacatgaacataagtaatttaaaatcaaagagcaaatattgaaaatcaattaaatctgggtcaagctactaccataaatcacaatgcaaataactagtccattttatacaaatgataaaagcaaaatgtttatagcaatacattacaaatatggcaaaataattgagaaaaaacaaggtaatagataaaacccttttttgagcttggtcttgactttccccaatttattttttttttttaaacattttctttgaatttatcccctttgtttgctttgatgtttcctccaattaccaagaaaatgaaagagaaaatgaagaaaagaaaatgaatatgaaaagggaaagggaaagggaaaggggaaaatgtaggaaagaaaaagaccccaagttgctgttttattattatttttttcacttaataacctggaaaaccatccatatttgcaaccgaagtccccagaatttgggacaaacaaacgtccatgatttttagagtgttgcctaggtgccaactctatgttaaaaaaccaaacaaaatggttttattttgcagccaaagtccctaaatattgcacgccaagtccctcaactttgatctttacaatttggtcctcatattttcactttcatatcaatcatggcctccaaaaattacagcctcaagtcctcgaattttttgcccttgtgcaatttcctctccaactccacaattttgtacacttttttggtcttttctcacttccttttacattgttctattttcttgggtgattttctctacaaaagctcttaaatttgatatacttaagctatgtgtggagaataattgatcaactgtagccttaagtgcaatatctatggtactagaaacatacgtgataccaataaaatgttccaatacacgcccattcttcacatatcaaatgataattaacctttgctccttcattgacatatctcgagattcatcaactagaataggaaacaagctattatcaatatctttgacaatcacatttagagttttagaaacaatagcactcacaatatctttctgaacttttggtaatgttaatttgtttttcatttcatgtatattcatcaaagaaatagccttaatctcaaaattatgatgacaaaaccaatgatatagttcgagaaagtttccttgattgtgtgaatatttagattcatcatatgcatgaaagccattccttatcgtagaagaaatcgaacacaatcaattgatgtattcaaacaaattcgatactctattcgagcttgatgcgatttcttaaagagactttgatcttgttttttgaatgattcattttggactagagcctgattgtgtgcactactaatgcccttacgtgttttctgataatttcctacaatttccaatttaagaacctatcattaacaaatgaaccaccacttgagctgaaaagatagcaatataagcaaaataaaacatcttttggtatactgcgtttcaaccagttaggatgctcattataccatgaaacacaaaatcgcctatctttattagccattcttataggtggaaatacataattgcgaggttgatacagaccttttcggacataaactcttcgaattaaatctctaatattagcatcataattttgtattggactctcaatctacgattcgaaagaagctgtgcacatcaacttcaagcccttcatccccaacatccctaacattagttttaataaggacgtctccaagtttggttccatcattttcattcatttcatcaccaagttcgtcatcctttttatttcaaacatcattttcatcccttttatcttgaacatttctttcattaacattttgttcatcacaaggaaacgtagatttacgtttatatcacttttccataactaatacaaagatataatggaaagtgtcaattcaagtgaaaaaaatagtccttctatcaataattccaaaataaatctcacaattgccttaagatgtaagttatgtataatggtttcataaatcaaaatctcctaatagtgttatatctattttgaattttttataaagtccccaacaaaatcttagaaattacaaatcacaattcataaatcaattatccatcatagatttaaaatttacaaatcacatatttacaaatccaaatttgataaaatttagaaatttacatattacaagtataagataaacttgaaattgatcggagccactaaacgttaagtaaaattagaacattatactaatcttgacactctagaaatgctaaataggataagataaccttaatttgtatgatgatcacccacgcccaaataaataagtttgaatattttattgaattgtgtggttttgcttcaaagtctagaattgggagccatcatacagggagttttctctcgtgatagaattgaattgggattgggacggtttgttgcattagaaaagttcggcaatggccaatgggggggaggttgatttggaatttagacgggttcaggtctcattgaattggaatttagaaggattctttaaataccccattttaactttattaaaaaaaataacttttcggttggtgagtccgccaatgtctattcagttcttcaaccacaatgcctaacaccaatttatcaaccatcatgacttaaataaaattttcaactccaattgctgatctcaacgtttcaattggaatgaatgatggctcagacaagaccatcacaaaggtaaaaataagatgtacatgatagactgtgaggtttcacaaatgccaacaaagtgacaacaccaactgcaaataggttactcttccaaacaacagatgaagcaactgagactcattcaggcaagaaattgaacattgacatggaccaatcaaccgatgaacaaattgatatcatggcctttgaggaaaagaatgaaggaaaaatccctgtatcttttttgactatagtcgattaagcaagacatcctaatctatatatgcacagcgataaactgctaaaagtttacatagttggacatagtgaggtcactttgaatatattggtgcctttttcataatcgaaaatgtatatattctaaagtgctaacgagcactacttgtgtgtgtgtgtgtgtgtgtgtgtatatatatatatatatattctcttgtcgaacctgtttcttgaaatacagaaactcaataccaagtgtaaaagcacgtgaaatggaaacagtaaataaaacaaggaataatgcgtatgtcattagccagattaagaagcaatagtaatgtaagtcaaaaacaccaaaaacatacatcaatattgctaaaacatcaaaaacttaatctagccattgaatagatacaaaaccacagttatatcacaattaatcaaaaaatgagatctacctatctatcatatatctactccccctttttgtcacaaatgacaaaggagcaaaaacaaaaactacgctgcagcaccacccgcactcaaagactcatcaacagtctcgtcactcgtgctctcatccaagcgatcacggatccaacgtaactgacgctgacacacagctaaagcacgtcgaaatatagaaagctcaacagactgatgctgacacacagccaaagcacgctgaaatatagaaagctcagcagactgatgctccgaagcagcacgtaactgcatgatctcggccatcatacgagcctgctgctcgaccaaagtagacatctgtcccataagtgtcaccatggggtcaatgtgcaaggaagccacccctggagcggaagtagacgtcgaaggaaggtcggcctgagacggaggagccggaggaatatccaaacaaggaggaagaaagacacgggaacccccagaaaggatgtcactaataggatcaaggtgctccgaaaagtcaaaaatatcaactggctcatcatgagctgcagcatgagtagaagaagaggatgggacgtgggatcgaatctggtggatggtctgctgtcctatcggatgacctatacgactagacgacctctcagggaaagaagcaccaagagataggacaaccctatgaatcagacaggcataaggcaaacctatatgacccccaggagtacgaaacgaagccagaatctgctggcacacaaaactagaaaggtctatagagtccccatgaagaagggcatagataaaacgggaccgcaccataggtaaagaaggcaacgggccacaggtttgtgcacacgatgcacaacaagacctgtctatcagtaggtaaggaacccgtggccatcgccgtaggccccctagcagacggggtgttcaaaagagtcgaccgaacaagggcatcgatcgaaagagaagcatgaagaatgtaaggataagtcagatgggaaatctgaggtatacctaacgcaagagctaccgtagacggaataactcgaaaagaatgaccctaagaaaaaccctaaacgacgagctgtccacatcatgaatattagcataaaactcctgaacgaggagtggaggtggtggtgtaagaccaataagaaggggcttccaaccccgggaaacaaagatagcgacgatgtcaataggaaggttagacaaaattacctcacgccccatgagaacggggtgtaaggagaactgagaagtgaagaccttctgagctgtagcagaaataaacctggatctactataagacgtcgaaccactagcgggctgtgcaaagggacgagaatgcttacgggccatctggcacacgcggagatgaaaagaataagtaccatggaaaatgcacgtaccacgatgcaatatgacatgagaagatgcacacataaacacacagatgaggcataaagaaaatgcatcgaaccacgtaaacgacacgcagaacaaaacaagcatgaccgagtgagagtccaaaaatatgatcaaaccacataaacttgaaagaagacacacacggcatgttacgacatgccaacaaataggaaaggacgaaggaaaaaagaagaaaaacaaagaaaaccataacacacataagaggtgaactttcatcgaacacgtgacgggcgcgacttcggcaccaaattccaagcacatataggacccaatcacaaatccaaactacactccatggactttacaaccatccaagccacacagcaaaccgattaacgaaacacaagaacgactccaatgaaaatggaccaaaagtgtgaaaaacatatgaagaaaaactatagtaatgcacaattcatggaaattggtgatgcaaacatgtttaagaacaatagaaacagccaaggaatgcacaaaacaacaatataacgaagcaatgagagaaataaattaaaaaaaaaaagaaacagtaaaaaaaaaacaaaaaatcgaaactgtgaattacccaaaaatgtgaagccaagagttgaaacttcggatcaagaaccgtgttaaagttgtcaaattgaggcaaacgttaatgggaagtgaataatattgatagaagaaaagaaagaaaggaagaatgagataaaaagatcgaatcgcgtgaaaaaaaaatgaaacagggcttttttaaaaggaattgtcgctcgagcgagacctgggcgaaactcgagcaacatccattctaattttgtcgcttgagcgaagtccaggcgaaactcgagtgaaaatcaaatgtcaaaaatagcaccaaaaatttgaaatttaagaaaaatagcacaattttcagaaaataacaaaaatagctccaaaaacgtttatttttattttcattttgaatttttgttatatcaaaacaatccaaaaatcgaagatgaagcacgtacccaaatatgtagacgatgcgaacaataagcacaaaatcacaaactcaacgttcagaacacatagagaaatcttaagtccacacatagttcaaaatcccgtggagtaaactgtatacagaacatcaaagtgaaatgtgccaggtagtccatgcaagttagactcaaaaccttaaattagtgagaaatgacacgtgaaagcaactgtaaaggagtgtatatcgaccaagtgacagtcaaatccaattccacacggacttatatcaaacagtttattgtcacaattttactccccctaactgtattccatatatatatatatataacataagaacttaggtgtaattctaccctcattaggcgacagacatgaccctggtaacgaactttgggccagtgactcccaagccagacgaccatagggcaccaagttagaaacccctaaggcttaattgttcgagtcaaataggccccgaagacagacataagttcagagaataacatagaaaatggggaaagatagaattgagtaggttacactcgtcacagatcaagtcaaatggacaaacaaccccaatcacagaagaataccatcgcaagtctcacccatgcggttaagactcatcacctacaggtgtgctgtgcgaaaatgcatgacgagccatataccaagaactccacaaaaaatgagaactacgatggaaccccagactcgtacatatgatgaaagatagagtttgatcctaaatgcaaacgtcataaagtcacacaagaggcacacaaaaagaaaatccccttttttttttttggtaaaacatgcaaactaagtaaacaaaataaaactaaaagacgaaccaacaatcaaaatgcagcacacacacattgatcacatacaagatatgaagtgaataagtgcagatgtgataaatgcatgaatatgcatgaatccatgatcagataggcaaacaaataccaacagccgttcgaagcgactcaaacctcaacccatctagtggtttcctaagtagatcggtcaattggttgtcagtagagacataatctagggagacaacatgtgtttcaacaagttcacgaataaaatgatgttgtatgtcaatatgtttcgttcgagaatgttgaataggattcttagatatatttatagcactagtattgtcacagaaaacagtcatggtcccttaattaatcccataatcactcagcatctgcttcatccagagaagctgagtgcagcaactcctagctgctatgtattcgacctctactgtggatagggatatggaattttgtttcttacttaaccaggctacgagattgctacgcatgtagaaatagcccccagacgtactttttctatcatctgcattctcggcccaatcggcgtcagagtagctagccaaatcaagattagaatctctagaatagaaaatgcctagatcaacggtaccactcacatatctaatgatgcgtgtaaccgagcttaagtgtgattctttgggatctgcctgaaattgagcacacactccaacactgaaagcaatgtcaagtctagtagctgtgagatagagaagactacctatcatacttcgatatagtgaaggatctacactcttacctgaaggatcacgacctaacttcaagctagtactcataggtgtcctagtatgcttcttactgtctaacccaaagcgcttaactaaatcctttggacactcagactatgaaataaacaacccatcctcagtctgtttcacctgaagtccaaggaagtaactcaactcaccaaccatactcatcttaaattcttgcttcaaacactcggcgaactcatacgctagagactcaatgggagaaccaaaaatgatgtcatcgacgtaaatttgggcagtagtgatagtttcttcaatatgtctaataaataaggtcctatcagcaccacctcgagagaacccatgttcctcaagatatgacgtaggtctttcataccaagctctaggagcttgtttcaaaccatagagtgctttgtggagtttatagacatagtggggaaactttggatcaacaaatccttttggttgttcaacatagacttcttttgaagaagtccattcaagaaggcactcttaacatccattcgatgaagcttggaccctagggtacaggcaacagcaagcagaatccgaatggactcaagttgtgcaacaggagcaaaagtctcataaaaatcaattccctcaacttgagtataaccctgaacaactaatctggccttatttctggttatagtaccttggtcatttgtcttgttcttaaagatccacttagtaccaataacattacagttttcaggtctaggaactaaaatccacacattgtttctagcaaattgatttagtttctcatgcatcgcattcacccaacactcatcactaagagcctcttcgactttcttgggctcaacctatgaaacatagctagtatatgctagattgttcagtaccctcttacgaagcctcataccttgatctagatccccaatgatattatccgtaggatgattggacttgaccctagacgatggttccttaggatttttgtctcgatcttgtggatgtgtttcattttcaggtgtttcaggtattctaagagatgattcaaacataggtggttcagtaggatcactagaccttataagatcaccatttctatcgtccatcctatcacaattttcaacattctccccctcactcacagcatcatatatcacaacattgactgactccattacaacacgagtacgtgagttatatactcggaatgctcggctatttctagagtcccctaagaaaattccttcgtcactcttagattaaaacttactcaagttctctctatcacgcaaaatgtagcacttactcccaaacatacgaaagtatttaacagtaggctttttaccctttagaatctcatatggagtctaatcggttttgggtctaaggtagactctattgattatgtggcatgcagtattaacagcttctccccaaaaatgtaaggctagtcccttgccatgaagcatggctctagccatatcctgaagaacacgattcttcctttcaacaaccccattttgttgaggagtgataagggaagaaaactcatttagtatcccttcatccatgcagaaactctcaagattaaaattttcaaactcttttccctgatcactacgcattcttgacactttgagattgagttcattactaagccgtttacacaaataagatcacatgcatcaaatttttccctaagcaattctatccatgtgaacctcgagaaatcatctaccacatccaaaatataccgcttacctcctagactctcagtcctaggtgatcccattaaatccatgtatatcaattccaagggtcttttggtcagaattttagaagtctttctatggcttcatttaagttgtttacctagttgacatggtccacacacaacattttcactaggacctattttaggcaaatcatctaccaactcctttttagccagctgtactagactcttatagtttaaatgacccaatcttctgtgccagagttcacttaaatcaatttttgcactcctacacacatagttagaattaggtaggactccataacagttatcagacgttctaaccccttcaaggaccaccccaccggatgaatcatacacggtacatctcttttacacaaagctaacctcaaaatcagcatcacaaatctgactaatacttaacaagttcgactttaaaccttccacataaagtacatttgaaatcacaggtaatccatgcatttgtacagtacctttgccaagaataggtgcagaacccccatctccaaagataaccatatccccattgcattcatcaagagtagtgaataaagccttgttaccacacatatgcctagaacatgcactatcaaggtacaacatattgtaattttgggcttttaatgcaacatgagcaacataacaatttatctgacctgaatgtccagctagatccccccttttaacccaaactttcttagacgacgaggtactcctagttagcttagtaagcatctcagtcaaatgactaacctgattagacagaaagctgacctgactaggaatattttgatttctatgctcattgcctaacttataacatctaggcctagtgtgtcctagagctccacagtggtgacaggtgggaatgaacctaggctcaaaggtacgtgtctgtgggtatctgggcatgatattcctacgtgattgatgactctgttccctcggaacattcttacccttatttggattgctgacaacgttagacttcttagaggcagaaacaaatacagtcttagatggaccagcaacatgtgtattatcctcaacatatcctagacctttcctatctcccgcaggcctattcattcctaaaatatcatccaatttcttagtcccacttatgaacgtctgaagatgagcattagatttctccaattcactagtcaatgtcttaaccttgtcttctaacttctcattgacacattttaactcactaacactcttaagtaaattttgaagattactagcaagtctctctttttctctttcaagttcatcaacctttttaagtagggctttattgacctttttgattttaagactctccttgaacaagagttgataggcctcttgtatgtctatatcatcctcatcctcattactagaattatcgttgagaagttcttcctcaacttgtcactctccttatcagattcactcttaatagtcgacacaaatgccatatagttcccttcatcttcactactagatgattcctgcctattactagacttagattcgttatctgtaagtgaaacaactaaggccttacctttcccttttctttgattcttcttataactaggacactcattcctattgtgacctatactttgacattcatggcacctaaccaaacgtggtttatcactagaacctttattgttgaacctttcaatttttttcctttgagaatctgctaggggctccactttttctatcctgaggctttctcctattcttgagaactttttgaaatttcttaacaaaatatgcaatttcatcgtccctaagagactcagtatcagaagattcatcctctttgatagattttaaagcaatggactttcctttcttaggttgtgtgacagtgagttcataagtttgcagggatcctacaagttcttcaatcttaacttcatctagatccttactttcctcaatggcggtaactttaggcctaaatctcttgggcaaggacctaagtacttttctaacaattttagactcgagaattctctcacctagattgaaactagaattaacaatatcattcagttttgcataaaattcatcaaaggtttcatcatccttcatcctcacttcttcaaacctagaagctagcatttgtaatttcaagttctttaccattttagttccctcatgtgtagtttcaagaatgtcccaaacctctttagcagtttcgcacattgacactctcctaaactcttcgggagatacggccataaacaaggcatgaagtcccttgctattccaattacactcagctatctcatccttagtccatagtgatatatcagtaagattaacagttcttgatatgctagtggagggaggtttccagccattttgcacactcacccaaacatgctcatctagagacttaagaaacgcacgcattctaaccttccagtaagcataattacttccgtcaaaatacggaggcacaaaaagtgattgactcatctagacaactatgggtcaagactcgagatttgactctgataccacttgaaaagactatagttcgacccaaacaacacctagaggggggtgaatagatgtttatgcgaattttaacaattcaatcaccttatgcaacaagtcacataaattaaactttgtccagattcattcacatgatttaactacctatgttgaatttccaattgaattaaaaatgatagaaagcaataaataactcaacaaattgttgatggagaaaatccaactgggtaaaaactccaggcacaagccagtagggattcactatagaagacttcaacttacagtacgccagacatgactgtatctaacaacactctaacctcctgactgtatcaaccaaagctctcttagattctgtagatctgtacaaaaatcctagccttgttcttcttctatttctcgtgaatcagcaagaactccagttcttcaatcaatctctttcccggatcttcaatcagtcaatcttctggaagtagtgagaatttttgaaaggtgttttgttttaagaggtgtttgatgtttttcttcaataagacatatgatgaaaagaaggaattatgaagttgatcctttggttgagaggaaaaatcttttaattgtgtttttccaaaggttgtgtatgaaaaacgggacttttgaatatatatgaggtcgtttttggttgtatggaacatctaaaaattgcaaggaaggaaaattaccaaaagtcggatagcactgtcgctcgagcgaagtgccggcgaaactctagcgacgtactttcgctcgagcgaagcagtggcgaaactctagcgagataggttctgttatttaggctcgagcgaggtcagggcgaaactctagcatgatcttgcgccgttttcatcttcaaggcacccaactttaccctagacctataccataatttttgctaaattgcaacacaagtccctaaacttttagacctttacaaattagtccttgactttacaaacttgaaaaattggtccttttggtcacagattgccaattacaacattttcctaatagaccccaaaggtcttacgacctagatgatgataatgacaatctacccttgagcttagactttgaaactaaatagatgaacttgaagaggaaagaataattgctatactttggggatgcatagagaggagagcaaagaggagttagaaatgaaaatgaaggcttgctccttcaaaataaggtagctacgacgggatattatgccgattaaacatattctgattgtgatacagttccattgtctgttcctattctaggtttgaaactcggtctatttgctcttacaaaactcagtcccagacctttttttatcacgaagctcgccaagtatgattgaaaaagcaatcgagccaagcaccttgaaagttataaaacccatatgagtttgagaaattcttcttatgtcatgaggtgtagaaccttttacttggcattgaatggaaaagcacaagtctggtatagcaggtaagacattggagtatcataagctagtcgaacttccaaggcctttcctaaagtgttttgcaaccaataaagagggagaggcacatgtgcagcgcctccagagtatgagacggcaaccaaaggagtttttgaaaagctttttatcccaatttacggatgaggtgacctattttgtgcaagtcactaataggaaagcattttctgacttaaaagaaggtcttgatatgaattactcctttggagagatgtgcaaaatagagatcccaccaactatgacactttgttggaaatgataaggcctcaggttaacagtttcaataaaagacttccatatcctcaatggcaaagggaaagaggacctacccccatctgctggactatcatgtcgaccattcaatcgtcttgaattcaggacaagcattagctattgctatgctaaatgtggtacacaaaggggtgaatccaagctttaatatacaacgaaagagatcaaggcagtggactcctcaaaggaaaaaagcttgtggacaatacatcaaacttgaaaatagggatgatgtatccctctattgttcttatcaccactcatgcaacacaacacagctgattgtaggttacatcctcaacaagacattcaaggaaataatcaatgaccacaagaaaatgtatcctcacctatgtaggctcagcagcctatgtaaaaggaggaaagatgatctcattaggcaagataacaatgggaataggcccaatgatagtctaaggtaaattagaaaccactcaactaatgtgggccatgaaactattcaagagattaacataatttttggaggtctctatgttggaggagagactagaaaagctaaaggaattatgcaatggaggccaaggacaccccatggcaagctttatagtcaacaacaaactcaattaggcaagaaagtgtagcctgttactttacccaagatgacacgataggtttgcactgtccccacacaataacctagtgataagggtcatattagcacaaaatggtcttaaaaagaatgctagtgggtaatggaagctcaaccaatatcatattcggagctatttttgacaaaatggtggtagaccacaagctgacccccatgagctccctttgtatggttgtactatcaacaacatcatcctaagaaggaaaaacaccctagctagacaagagaactatatctcaagctgcccaccacttgatagaattcttgatagtggacaacatatctgcttatcatatagtgctagaaagattgctttgaaggaattgtaggctgtcatctccatttaccacctatacatgaaatttcaacctaaaatagcatcaccatagttacaggtgatcaaatgtgggcaagtgaatgttatctaaactctttaaggtaggcaaaaccacgagatgttaatgtaatattggtggatgtcgagatggataaggttccaaaagtagtacagaccctgcacaatgagaggatgttgaaatgttggatgtctctgaagaagaaatgatctttagaattgttgatgcttcttcagaaggatagccgtaaacaaagggctaagtttgatgaactagatccttgggtcattggttgtgaaccacgaaccgctcctgtaaaagacctggaaagtttcacagtggatccctatgaccccaccaagaccttgtaggtggagatagactagccatcgatagctaaggagaagctaaagtacttcttatacaagaacatggatgtctttacttggaagcatgaagatatggtgggcattgacccaagagtcagttgtcaccacctgaaaattgatcctaaggttaacttgcataaataaaagaaaaagagccttcaacccagaaaggaatagagctaaaggaagaagtacataagttgataaacaatggcttcattagggaggccacttatccaaggtggatttccaacccagtgttggtcaacatcgcagtggtaagtggagattgtgtactgacttctccaacctcaaccaagtttgtcccaaagatagttttcctttatcaagaatagaccaacttgtagattccacagttgggtatgagttcttgagcttcttggatgcctacttaagctagaaccaaattcttatacacccaactaatgaaaagcacacatcctttatcactgatagaggtctttactactataaagtaatgctcttttagtttaagaacatcgaggctacctatcgatgcttgtcaacaagatgtctatcgacctcattggtaaaaccatagaggtctatgttgatgatatgttcatgaaatgtttgaaagttaaagaccttgtaaaccatatgggtgaaactttcaaaattttaaggaaatacatgaagaagttgaatcctttaagtgcatatataatgtcgctttcaaccaaaggctaatcttaaaaagataaaagccttgattaaaatgaggtcctcttaaaaattgaaagagatacaaagtctaattagttgagtggcaattttgagccactttcttttaaaggccacagataaatgcctcattttctttaaattttcaaataaggaaagaacttccaacggatgaatgagtgagaaaaggccttctaagagttgaacaagctcctatgacaggccccctcctctcaaaacctaagctgataagccaatgtaactttatttggatgtatctaataaggccatctgctcagttctcataagagaaaaaggcacccaccacctatctatctattatgtaagtaagatattttttatggcggagacccactacccagatatagaaaagttaactatccttcctagttaccacttctaggaagttgaggccatacttctaggcttaagtgtatatgtgctaaccaacttcttactcaaacaagtgtttaaaaagcctaaggattcaggaaggttgatgaagtggactagggagcttagtaaatttgacattgtcatcaaggaaagaaccactatcaaaggtcaaatcattgtagattttgtggaaaactttgctaatgtcctagagatggaagaagtattggagtctacagaacctttcgtgtagaacctatttgtggatggctcttttgggaagataagttcactgccaatggtggttctagtcagcctaaaaggccataactcaactgtgcaatgggactcgaatttaaagctaccaataatgtggtagagtatggggctatcctagccatcctcaagttggctagagaaatgtaaatgaagtagctacttatcagtagcgatttccagctggtagtcggccaagtcagtggtaactttaccgttagggataaaggtatggctacatatctcaagatggtatttgaccatatcccaccttttgaaaagtttgagttagcttaaatctcacacatggagaatgtacatgttatcattctgtcaaaactagcagtaaggatttcgagctactgatccctggcatccattaagcacctttctaggtcttcaactgccaaggaggaaaaggtaatatggatagaagcctcctagatacagcctatcgtatcatttcttaaggatgaaacccttcccactaacaaggaaaaatgccaaaagcttaggataacgatagcaaactttgtcttccaagagaaggtattgtacaaaagatgtttctcattgcctttcttccaatacgtagaaggcaaacatgtcacctacgtccttcgagagatctaagaagggtttgctttggtacagaaagttttaagatagcgatactatttgcctaccttgaaaaaggatgcggaacagtttgtaagaaagtgcgataaatgccaacgattctcaacaatacaaaggcaagccttccaagagctaacagtggtagagcctttggtcattagccaaatgggggattgacctcatagttcccctacctaaagaaagatgaggtgcaagctttttcgttgtagtcgttcatcacttcaccaaatggtagctaaaacaactatagctaacacattctaagttctaatgaaagatcattatatgctaatttgacatttcttactcaattgcatcagataatggatgacaatttaacaacaaagaggttagagacctatgtgtagaacttgggatcaaaaaatacttctttactcccatcaccccaagtgaatggtcaagtagagactgtcgacaaaaatatcaaatataccctataaaggaaacttgatggctcaaaaggggcttgggtcgatgaacttccacaagtgttgtgggcaatccaaaccactagctaaattgccacatgaggaacgccattttgtacagtatattatgccgaggctatgagctctgttgaagtaggtctaccctcacctcatcacctatatttcaacgatatatctaatgatgagttgagtatatatgcgctcaattttctagatgaaagaaggaatgagtcccaagtaaaacttgctatgtatcaacaaaaaatgacacggtactacaattcgaaggtcaagaaaaagtcatttcctattgttgatttggtgctacgaagagtttttttctcttcgaaagaatcaggagtagtgataagagatagaatgtcatattttaaatccattcatacttgcatttttgtgattaattaacacttaaatatactcaatatccttgtattttgatttaggttgtaaatggatggaaaatatagagtttggaacaaaagagcgaaaaaggatcaaaatggaagaaagtgaagctcagggtccaagttacaaacaatccatggatgagacgggctatggaatgaagattcaagagtgttgaaggtcaattggacgaagaaagaagccaaagaagtgaaatatagtcgaaatattatcaagtaacaactttcaggcgaaaaatctatgctcaagatttttagtctctactttagacccatttttggcatagtaagcttccgaatttggaaaatcctatttctaccaaaattgtagatcttcgagttagcttcctaacacactttaaatcacctcaatgagatgtcagaagagaaaattatgaccaaaatactaaaaactagccaacgaaaaacgattgaacaatgcggtcgcatagttcaaaatcaatgcagtcgcatagcgacctccaaagaacttcagagtataatcaatgctattgtatcgtgacctctagcaagtcttgatgacttgttactggttcttagtgagttgtgctaacatgttccgttttctggtggtcaaggtgagttgtcgtaactcgccctggtttttggcgattcttggtgattcattactagctcttggtaagttgggatatcttagtctggtttttggcgattctttgggactcgctcttgtttccttctgagttgtgtgacacgttctattattgaacaaatgcttaaattatttttcttattctgatttcttgtatacatctccttgaaagcaagggttccaagttttgtgaattctaatcctactctcttattttttagttaaatatatacttttctcacgtgaggttatttagataattagcttactggtgtttttctttgtccaagatctcatgtaaggatctgaaaatttgagggaacgcttgataaaagtgttttctgtcgttaaacattactcaactgctatttctatcagttacattgcttatattcgatatcagctagaatcttgatactaattatatattcattgctatggatacattgatataatctcctacattgtgcaaattaatgatcagtgagagtgtgtttaattgagtaaaatctctttgctcggaattttgcaaatattgatgttcattaattttctccaagtttaaatttcaccatgtggcataaacttgtttttgtgactttatttgcaaacatgagttctgtacaaaagtttaaggtagacatgtgaaatggtattagagactttagaatctagcactaataaaaaagaggactttattattaaaatattttaaattaaaatataagttgtgtaacactatacttttcaacgtaagcacccaacttaaatagttacaagtaattatagccacttaaatttgcatactcaataaaaacttaatataatacataaataaaacaacaatttaattattataaaatgttattttatcacagcaaaatataaaatatggtcatacacccaacaatgccagatgtatttctaagagaacaagtaagattgtttgaggtacggtggtctatgttgggcaaattgttgtcaaacaacctcctgggccataatgtaaactcggtttaattatcagtcggctttgttcaattgattgataaatcaccaactcctcgtaattatatgactcaaccctaaaaccaattttgggccattagtagcgacctaatttcattagagtcgctcatgctggaaactaggattgtacgattaagtacttatttaaataaattatctcattattctctgtgatataattgccgttattgtaagtgaaatcttttttgattggacatatctatttgttgcatagtcaattccgttgcgcctttaattccgttagaatatctagatcttacccgttcaaacattctcttgatctaagattgcaagtcttacgaaaccctgaaaatttagaacaaaatatgttcaatttttctctcactactacttgtgcttatgaataggtgtccattgatgtgtcaattaattattagtgaacagcaagttggatagcagaccttaactcaattcgaccatctctaaactattatcataaatagatatttcattgatcatttcatcataggaatttaatatcataaattactgtaggatgtcgaacttattataactgattatatacacattttactttaattaaaattagccttaatcaagaaaaaacacaatcaattcttcgaccattcatggcttgtatgattctcgttaaatattgagaaaatgaggcaaatttttctttcaaaacagaaaaatattagacccaaaaaatgaaagtacctgtaatagagaaatgttaatttggacatattattttccctaagtgaaagagaattaatgttgaaaagtcggttgtgttgtctttgtaagtgttatgacctaggttcaatcaattttggacataaacacttttaatatataataatgcaattttatgaaagacttattatttaattaatactcaattaaattaaataatagagtccatagattttagtaatttcttaaaggagttgtgattgtgagatacaaattacatataattgaattttaaattatctgtgatcgtaagcaataacgagataagaagatcgtttttactgataaatcatcacttgtgacttttcttacttatgaagtaaataattaatctcacaaactaaattgtggtgacactcaaatgaatatgtgaatgtttcttcatagaacaaaatattggagacctgctagaaagataactacctgattgttaatggttaatctctaatgttcaataatgaaattggtcatttgacttgaggtcaacatagtgccttatacaaggacggtcatacttaagtaatgttggatgttgcaatgccaaaggtcatactttgacttgaggtctacaacgatcaatagaggattcatcactcttagttagtaagaaattatgatctacatttcatttagttaaattgataatgaaatgcatggccaagccgtacacataagtcgaaaactcattttcgaaatacattgacttaacaatggaatgaaagatataactaataattgagattagcacatatttataactcgtaattgatcggatcatattgatgaaaagattatagtttcacggtaaaaaaaaaaacaagtttgcttttgtcataccacgtgacattttcgtcagatgtgttgtcctgatactttgctatatgtcaatctaggatgacggatgtgaattgatgataaattagaaagggatgttttaatttatcagttttgattgtatcaaaatactgattcacgttgctatgcattgtaatcgagaacctaatgggtcacacacaaaaggaaaactagaagaatgagatttatcaattaaattaattgacaagtgttagacaattaattaattagattgcttgttaataggttcgaattaattaattggattaattaatttatggaccaaacttaattaattggattaattaaatattggatcggattaaggtaaaagatggactaaatccacttggacttatattaatagtttgctagggtttgaaaaatcataacaaaatacaatttcatattcttgttagtacaagaaaagagaaaccctagttctcttaatcaattttcctatgtggattttcattggaggctagaaaaatggattgctataaattgttttaagattagtaaaggagtttgcagaatctaccaaagatattattctatcatagtttctatctaagcgcaaagaagatcattgatcataattgaaatttttgtttaaatttcattatgcatgctaagtaaattcccaatagtggtatcgaagcctactttgtatttgaagaaattgttttgcatgatagaacaatcaaagattgttcatatttttcttgaatctagtaatttagaaaattaattttcatcttcaaaaatctatttttggaaaaaaaaaagtaatttttgattgacaaaaaaaaaagatcagacaagaggacaactgtgaaggtcaccaccgtcgcactggcggagagttcgatggcgcagtagctgcacgaaggagcgtgctgtctagcacacgctgcatgtctggcagtggtagtagacgccactacaaagtgcaccgccctcctttatccaaaaagaaaaaatatgccactacaaaatgcaatgacatctactgtaacatgacgtcgcaacaacaacacacaaatccactgcagcatgactgcaatagcagcgcgcagtagaggcgttcgatcgacgagatgctgcctctgagagtggtgactcttaccgtagaaggaaaaagtgaagacaatagccgttgccacccaaatcttttgtgcttttaagttttcgattgaggtgttggaggtgggggcatggtgtgcaatttgtgaaattgtaagcccccgcccacaattaaaggaaaatggtcaattttgcaatattaaataaagaaactgctatgcaattttcaaaattgaaagacctacttttgattttaaacctaggtcaaattgcaattttcaaaagggagtttagaatttgaataataaaatggatttaaaattgtattttaaatgagtttgacctatatattaattttgacccatatttaaaattgacgactttgatgttatagttagaattgggttttaatttaaacattaaactctaaccctaaattgaattttattttatttagaatttttttcttaatttaacatgttaattcaactataattagagttagaccctaatttgatattttattaatatttgattttaattaaattatccacactaatatgttattgaaattagagttggactcaaatttgacatttaattgtaattcgattttaattaaattgttaagccctaaattttttcttggaattagagttagactttaatttggtatttaattaaataaattcgccctataattgtggaattagggttgtactctatttcgacatttacttacaatttgattttaattaaataaagctgctaattagattaattaattatttaaatgtttgacttttataatcatgaaattcgtttgcatataatattagatattatatatgagtgcatttatttgatgaatgttttatttagtagatgattatggactcaaccatgtcgttgtgttgaatgcttagtcttattcttgttgcattatgggcctatgagctctttacttattttagatatatgagtccgttgtaattattatgggcttgcatgtccaattatttaggcctgcatgccaaccagtataagatatatgttataactagactaattgaagatacaagaagatgaggagactatagagatgaagcattgtatgagtccatgcaatgtcccctacgaaatgaccaactagtctttcttatggctggggacgattagatagtaaaagtccataatcatccatactatatttgtatgttagatgtataataaaatatatagaattattacaatgagacctttgcatacaaaacccctcgttaaaatattaagtcatttatattgggtttctatcattattgtgaaaaactagagtcctcgattgatcttaacttgttgattacactcaaggttggtttattaagaatatgtttgacactatgaaatattagatatttctgaatgatgggtttgacttaactaaaatttattttttgttgagtgcactaaaaaagatatattttagaggctagttaagctaacacataaaatgtatgaagacaaagagttgttagcttaatgatttgggagttgtatagagatacaattgataatagtatttattcaaattttctattaagacttgtttagtaaattcaaggtcttaataataacaaatgggatcccggctcactgggagtcaagaatggattccataaatttatgtgagagggtcatatatttgagttaaatagttagagcataattgatttaacgaaatatcatgttcaattaattgatgcattgtgtatattattcttttacttttcatcatttacatttcttgaatcatgagtaaccatatgtatttgagcggcatactggatgccaaccaccaaacaaaatttttagattggcatagaataatctgagtattgctctcaggtatgagaaaattggttacgtcctttagtagccctttccaaagaatctgctaatgactcgattaaggaagatgtggttgctatgataaacacagtgatgacgatagtagtgcaatatgtgagatgcttgcattatgccacctgaattacaaaagcaacatgatggtacaaatgataacacatgatttttatctcaaagagttatatgatgaataatcacgtggggaaggatatgagagttctaagcaaccatactggtgcaaaatgatagagggatcttcagtcaatgctcatgtactgaagataatgggtattgagaagttgtctcaattgggatcaatcatgaaccgtgaactaaatattgacttagttctacaatttttgtcaaaaagagctattcacaatttattatacatttaacatgaataaactcgaatgcacactcattaagttgctgaatatgctcaagactgtgaagcctaacatcaaaatttgtagtgggcaaatcttagtcatttatttctttaagggtaaagaaagtttaaaagatgctttaaaaaagtatcaaggacggttaaaacagtcaaagcaaagaaggacaacacccaatctaataaccattgttatcattttagaatgaaaggtcattgaaaggggaattgcaaggcttatatctacttcattggcttcttgtgtattagatgctagatatggatctcatatttgtacaaacatgtggaaattagatacaagtagaccacagtaaaagaatgaagttgatccatacgttgaagatgagcaaatgttgttgcattgcctgtaggagcatactcattgccattgcctttgcggttaatattagaattagagaaactttattttgttctcaccattattgagagcattatttgaatttcatgtttgtacatcaattattttaatgttaaggacaattattattcctttttatcttgaaaagatcttaatggttatggtaaattacaaaatgacatttatatagaagttgaaaggcttaacaatgataatctgaataacacctatatcttacattatagactagtcacataaatgagaatgcaattacaaaattacaaatagatgtatatttggagctaattgattttgaatcatttgacaaatgtgaattatgcctgttagacacaataaccaaatctctttttacttgaaaaggtgaaaaatctacacaattactaggtctaatacatagtgatgtatgtggcaacatttcaattaatgttatatgagatttctcttatttcatcacatttactattgactattttagaaattgttatgtatacttaatgaaattcaagcatgaagctcttgaaaggttcaagggattcaagttagaagtagagaaataaaaaggtaaagatattctaacgctaagatccgatcaaagtggagaatctcaaagatgaaattttagattacctaaaatagaatgagtttatcttatagtggactcctcctcatacactgcagcataatggtgtatttgaaagtacgaatcgtaaactattggttatagtgcaattaataacaaaccatgcaatcttctcaaaatcattttggggtcatgtactaattgccgtgtgctacacactaaatagtgttccattcaaatcgatcaacaaaacttaatatgaattatagaaaggaaaaagactcaactaatctcatataaaagtttggggctgtgacgcttatgtgaagtgtaatgaatctaataagcttgagattaaattcaataaatgtatatttgtaggatatccaaaattagaaaattggatttcaattctacaatcctgttgagaagaatgtgttcatctcaagacatttatattcttagaaaaagagttcattctaggagatgatagtaggaacaacatagaacttgaaggagttcaagaatctacaaatatagttgaccaagtatataaacctaagtctaatcccacacctcttgagggacatgcccttgattaggaaatagagactttgatgtgaacccatgtagcaatagtagatccaaaacccaaaaaagattgaatcgaacccaagattcaagaatatcatgaggattatttgaatgctacaacaaaataattcttggtaagttcgaaatttagttcaatgaagaacaagaaattgaaaacaaaaattgctcacaaaatagtctctcttattgaatgaatgaatgtttacaacaaaataatgagtcctatttataaaaaaaacccataaaacctagttaaaatggaataaaagtctaaaaattatgtaagttaccaaaaattagagtttcaatacaaataaaagatttcgtaaaatttggaaaattcgcgaccagaagttgaactatgtggtcatatagttgccttggatgtaaccgcgtagaagcctgaatcatccagcttcactcgctacttgtttacatgtgaccacatggtttatataactatgctatcgcatagttatatgatttactcacttcgtccattgctcgaatcaaatagatccaacgtgttttttcttttgaacccaacatgaaaattgttcttttatttgccaaaatcgatgtttcgtccattgtagcttgcaaaagtaatcacattgcttctttgatccttttctctcgcaacctcatcatccacccttcttcaacgattaacggatccttgcccgaacttgccttcgttgcattcattccatgaataacttcatccattccctcttctaaaggattcaacctcgactatatacctacatcaaagagaaaaaaaaatcaaacacattaaaagtagctaaaatattatactcaccaggaagatataatttcaaggtatcgtagtcaatcctttcaaggacttgaaatagaccattcccttgactgcaactttgatttttgttgttctagacaatgctcttttctcaagtatacccaaacgtaatctctgggttcaaatctaatgctcttctaacctttgtttggctgagacaaatagtgcttgttcttcttttcaatttgcattcttaccttctatggattgatttcactaagtcgaccatcttctttccatctaaattacctcgttcattaataggtgaaggaattaaatccaaatatgttagcggattacaaccatatacaatttcaaaaggcgaacataaagtagtagaatgcacaaccctattgtatgcagattcaataaatggtaagcaccctttcaagctcttcaaattcttattaactatagtgtatatcaattatatcatgattctattaactaccacagtttgcccatcggtttgtaggtgacaagttgtagaaaacaataactttgtgcctaacttattccgcaaaaccctccaaaagtaacaaaggaatttgacatccctatccgatacaatacttctaggaatttgatgtaatcgcactacttctcaaattagcaatgttagtggcatcgtccattttatgacatggaataaaatgtaccatcttgctaaatttatctccttccacaattatggaatctattcttttttttagtcaaaggtaaatctaatacaaaatcatagaaatatcaacccaaggtttactaagaataggtaaaggtgtatataagccttgagataaaaccttagacttagcctttttgtaagggacgtatctactacaaacctgatcaacatcaattctcatttaaggccaataaaaatgttcgctgacatttctaagatattgttaacctcaaaatgtcccattaaacctctactatgtgcttctagtactaacaattctttcattgactacttaagaacacaatacttgttttcctgaaatagatatccatcatgcctaaagaatttatcaatagctcctttatcacatgattcgtatttattagaaaattttaggtcattagcatacgtgtccttaacatattcaaaacccaacaattttgtacttaaagaagttaaaagcacatgccttctcgataatgcatctgctaccacattttctttaccttgtttataccgaatgatgtatagaaatgtctatataaactccatccaccttgtatgcctcttttttagcttaccttgacctctcagatgctttaaagattcatggtagatgtgaatcatgaactcctttggctataggtagtgctgccatgtctcgaaagtttgaactagtgcatacaacgttttgtcatatatagtataattgagagatgcctcacatagattttcactaaaataagctatcagtcttctatcctgcattaaaacaactctagtatctatccctgaggcattatattcaatctcaaaaattttctcaaagtcaggaagagctaaaatttgtgtcttacacaacctatctttaatagtattaaatgaatgttattggtcaacgccccattgaaaccctatactcttcttgaaaatttttgtgagtggtgtggcaattatgctaaagtttttgacaaaacgcctagttctcccaatcttgttcactgtgtgaatttctattggagcttgtacaattgaataatcgtggattgtgaattgcaattgttcatgctctaaaattagcgaaggagtttgcagaattcatcaaaggtattattgcatcacagcttctatctaaacacaaagaagatccttagtggaaattaaatttttgtttaaattttactgtgcatgttaagtaaattatcagcagtcttttctaaaaaatcaactagtctctaacacgtctctcatatacttgaatttgtggcctctgttttaatattaactaatctgcagtaatagctaatctacttttattgctttatgttaaaatcagaattttctcttaataaaagcaactaattaggaacataaagagtctaccctttctttctttttttgagcatcatagccttcaagttttaaatgtgcaaatcaaacacactagttattgaaatcccaaatttaatgtctaatgtttagttagagcatatccaagatattctttaaacataagatgttttctcttttaaagagttaacttttaaaattatgcttcaaaagactcttgaaattaacatctataaatagagagagagtttggctcttcaaatttagagagttaaacccaccctctatcattaaatgcaaacaaaatatttcaatattcaatggataaaaataatataataatttgaagggaatttagagaaaataaaagataagaaagaataataatttttctttgaaattaatagaattaagtgtcaaatggaatataaaatttttttactttatgaatttatatatgctccttaaattgcaaaatatgttctttaaaaatgaagagtctcatggagatactctctggcctgtagtgtttcaagctcttgcttttatccatatttaacactttcattctttctaatttttgaaatatttatttggttctcacattgatatcttttagaggtagctttgcaatgtgacaacttttttcctctttgccatgactagtacaatgctttttttaaattaatagttaggattaattccctaacataaggtcaagaaattaatattagccttaatcaagaaaaatacacaataaattctttgattttggttttagctatatttactaaaatgaaaaattaggcatagacaaacaaggtcttggaattaatcaaatcacaaaaggcagtggaatccaaaatccaccattattaactttctttagtcacaaaaaaaagcatttatggcttgtatggatctcgttatggatggagaaaatgaggcaaaattttgtttcaaaatcagagaaaattggaccaataaaaatgaaacctctatgttactatcttgtttcaccattcttgttgaagtggctgcctgcaatggagacattaacttgcagtgagagaatcaatgccggaaagcccgtagtaatgtcttttctggaagatcagccggtctctatgacttctctcatatccttgaatttgtggctctgatttaatatttactaatccgctttaatagcaaatctacttttagtgctgtaaaataacaaattcagttctttctcttatgaagatccgcatggcctatctaggatactcttactccactttctgaatcaaagtctgttgattaaagtaagactttcgttccatcaggaatacgtacaatctaagccacttcctctttattttctctaggtcatctttatctttgcatttggaattgtcattttctctccaccataatgcaaacttcttgctttaaggattgatttctgactgtcaaggaagcaaaattaaataatcttagattaattagagtgttcttgatgcatgcactggaagtatttgacaattcttagatagaatcggtctgttcagatggcaaatgccaataaataaatatgggataaaagtgaaaatggtaaaaagtgctggtagtttttttctttattggataatcctgcatttttggaatgaaaagccagtcatttatccaatgaatgaggacctgaagtagctttacacttgttatatatctaacctttatcttctcctatctgccttctgttttcttgtctccattaagtaaatttctgagagtctactattgtagcagaatagtacttctccattattgttggcattatgcttctttggtttttaatttaattatcaaaaccatttgagtcatcatttgtttactagatatcttgcaagatatgtaaaaaaaagaactcgtgtaatcaaccatttgaatcatcatttattgtcattttgcattttttttttttttttttttttttttgataacccaggtgtcccagcttagccggactaaatcctggacctctagcccccggcccctcagtgactagtggaggtaaatcgcaggttgtgcccttgttggttcccaggttcccacatggcttttactccttccccaaagggaccctcctccatggttattacatcaccaaactgctccaacccttcctctggttattacatcacttggctgctccaaccaggaatcgaactccccacacttggttccagagccccccaatgtgattgttttgcatttccttctacggacagtggaccttgcttttccttgttctgtcgtgtaacactttgtaaagtatagttgtacatgtgctcacaaccccacaatacttttgcctttatgaagaaattagattgaattttgtcaatttgattcttggaagtagatgtcgtatcgatggatagattagaatattttagtacttgaaactatgtattacattggatattataaatggaaccatttaagttcacgtaattattggaaccaaactcaaactcaaatgagtttggttctatccataacaattttttgaatatttagcaaaatatgtcgtagaataacattcaatatgtaacaaaacataaacaataaattaataaaccaaaaattacaaactaacaataaggaagtactacgttctacaaatgctaaaaataacataaatttattcatctgaaaatagcataacaatcaagattgtcaatttttcttttcatttcattgttttctttgcatcccattgggtcaaggtgaataaattgtaaaatataagaaacttataaaaagaacaactaggtattcacgattttgattcaacccaatttctaaaaatttgtttaattggcccagagatgtcaaaagaaaaaagaagggatttttttattctatccaagaaaaggggaatgcacatttgcttgaaacaattcccaaataactattttacgcttttgagcacgtaaagaatcgtctaagatccggtcgattctcaattctcaattttagttcctacttccttttttttttccgtaaaatcaaacctgaatattggattccaattccaattaaaatgcccaccttactttgaggttctaatggttagtctgatgattcgttgaatgataagccttagttgtcatgatcaaacctcctccccatactcctcatacagtaatagtcgctccttatttcttaaataatgaaatttgaaatgtttgggaaatatttgatacaatgaataaggcaggttgtttaaatcagattagtccgatagcacccttaacttttttatgccctttatcgatgaggacaaatccctatagatgaaagaaatgagcatgtgaaatattttctcccgtcaatttatatcaattatcattttttttaatagaatatgttttagataagattaggcttacaaattcgtcttcaatgccataagaggtattattccacattcctcaaatgtgcagctgccttttaaaatggattagattaccgttagattggcacaatcactttatgaatacaagtttcgattaaagaaaaaggaatactgagcacacccactcccacggccacccccacccccacggccaccccaacttgatttgtccatgtgaagtgccactctaactcttttttcgagcttactatttaatgaacaaacaatgtacttcgtatatcttagtacaaatctgttctcaggattttgtctccctgctttccatgcagaattatactcattcaaaacatgcatatatttaaatattatgaagtaagaccatgtttgaaggaacttatcccctatttgatccccaatatctataaaatctttttcaaccatatattatttaaataaaataattttacacatgaattcaaaatttttacctactttttaaacatatattctatactgtcacaaaattcttatattttacaaacaccaatgctaaatgtgcagaaaaggagttcacagaacccttccaaatgtgacacatggggtgagttccatgtaattaaaatattgtcaaaaaaatctcacccacaccacctgttgcatctaatctggtggggttctgtgagcctcaccctgtacgtgtatcatctctcttttacaaaagcttaaaacaagctttttagcaaattcctgtttgacaattcaatataaaattaaaatattaagaaaaacggcccccaccctgattcagaatatgagacatccaatgaccttatcccccaacttttgggttttcattttcagcctatatttataggttgaaaagacaaaaacgcccttgacataatttccccccaacaattcattgaattagcctacttgtacaaattattttgtacaaagaggttgacaatccctgaaattaaaatcaaagtatagatatatgtgcgttcatttgtcaacatatctgcatgtaattctatatatgtagcagagttacaatccatcttaacaatagatccccacgtgttgtctcatgaaggcacgaattggtaaatattataagacattttattgccttgtaggacccactacacgatttatttatttatttttttcaagtgattttatcatttaatagggctaaactaacactagagtggttgtctagagagaatttaaaagagatctctatcaccactttacaatttgctaattttaaaagtagtaaattgaatgagactctaattagctatcaaaatacatcactttacgataatgccacgataattgttaactcgggaattgagaaaattgtcatgaacattgtgaagtacaccacgaagtcatgactatttgtgggatcccatgtttcattcttgtgaatgtgattaaatttgggagagcttcaagcgaaaggtcaaaacattgtcaaactctaatagtagtggagttatattttggcaatcaagcgtatatttgacagcattcattgcctcaatctccatctagaatacaaaaaagaaaattatcttagtcgaatggttgatcagtaaaatatgtatataatcagtcaagatcaaatttcatttccacaataccctatccaattggagccaagcttgttaattcttaagaaaggaatttgaaatgcctgggacatatttgatatactgaatagaacatgttatttttggcaaaattagtttcacaacacatttaacctttaatttattatcatcatcatcatcatcttgtgttgattcaataaatcgtattaaacatatcctctgcaacgaaatcaaggtctttttactaattccttaaatgtgcaactgcctttccaattgtttagatgacaatgagtatgtacaatcactttatgaaatagtagtttcagtgcatgtagatataattgttggtatgcggaacataaattatttgcaaaaataaaaaatttctctaattcgagaattcaagatcctaattaaatattcatgtgtatactttacttaaaaataataatcgctaatcaaatattgatacgttaaatctcctatggtattccacgatctcccaaattcaacccatagagaataattaatgtctttgattttggttctatctaatctctttttataaatataaaagagttccaaataatgtgcaataaaaatttcaaataaagtagtcccaattgaaattagccctaaaacttcaattacaaagatagttaaatttacaatgtttatagtaattacttttatcgtaacaacaattaagctaaaacatttagggttcgtttaattgcaaaaattgaaatttgggtggaaagaaaacgaaatccaaggaattgaattgtatagagcttgttttcctgagaattttttcaattaatgtgtttgattggtataattttttacctgaaaagtgttgaaattttctatcttttggtgttcgtttggctttgtttttcatagaaattgtcaaagaacaaaatttgttacaattggagatagaatttactccaattgtttaaaaaaaattaataaaaaaaaccgcctagaaaaccaattcccacaggtttggtgggaattggttttccacaaaaccaaagaaattgcacatgtgtagggagaggaaggaaaatgaattccataaaaaattattataatcaaacaagcccaaagatggaaaatggaaaatgattttcacgaaaaatttggccctatcaaatagggccttatagtaattgcaaatattttacaatgctttataaatctactgcagtgacttgttcaaacatataattccaagctttaataattagatactgtgtagtgaaccctaggttatcaaatctaattattagtctttgttttctccattaaaggcaaaagactgcatgaaatatataaaatcacaaaagttaatagatctgtaatactttctttaaccagtcatatctgtattttatttttgtccgagatttgataattggatataagcacaaatggctggtttgtccctttaattattcacaccaacttaagttatattttcttcaacggccttatgaattaatccctgacgtcaaagtttggtcattatgaacattgagctcaaatttacaatcgttcattagaaaatacttagataatcactctagctattttttaggacgatggttctagacatgacttcatgttctctgctttgcttattctcaatttttcgatcaatagaaatatttgattaattaaattgatgtcactcactgatgacctaaagaactatcaaagtcagaaaaagatctatgcaactatgtcaaagattcagataaatattcgacgatcaaataaaatttaattctttacacaatcatactataaagtaattctctatatgcatggggttagcctcgctacccaggacacctctatgatttgtagagccaaaataaggagttgacaaagaaaatctaagcctctgcatgcctagagaaggagctaggaaaagctaagtctcatgtagaaaagtctaaattgaagaggatgcaggtggaggtaaaactggaatcgatttaatgtgaagtaagccacttgaaaaaagagctacatgagccggagtgctagatggcaactctcgtaaaatggttcgatcaatcaaacaatcataagcgggtcactattgaggctttggaaacctatactaaagaaagatagctgaggtcgtaggtcggagcccgaaaagaagaaactaaacatttaaaagtagagacaactataatcgacgaggtggcaatctagaactttattaataacttcaaaaaaaaatgaacaaatatgacgacttcgtcagtattgagcgtccttgagtgcataagaaatgatgactcggatgagggaggttcattcggaacgggacatcaacttcttagaagaggaggacagtgggccaatcatgagttatccacacattgaggctaatatcaatgaagctcatccttgagatgaagcaaaagttgtcaaggtgaaccaagctgaagcaacaatcatagtagatgtagtggtaaacccctagactaattttgttttcaaaagattataagggcttcaacctctcctttcatactcaacttttattgaatgaaaatatttttcttcctattatttttgcctcttatttttccacatatgtttgttattacctcgttgcattgctaacaacgtcttgtcttcatgtaatgaactagcctactaactcctcaacgtgacctcaaataggttaagtctatgaataatatcacctcaggttctcataataaaaattgtaaatccaaatgttagtgcatcggtcacttgtagttgattttataagacatgcaagtgttgatgcctcgagtgtaatgagaaattcataagcttttttaagtaagtacttcttggcatggtgtatagtgtgtccatgccaaaggataatgaggttggtttggtagattttagggtcgcctccctttggtatgcttcacacttctcttgtcgaggtaacaaaaggcttccttgcatgtggatggttcatacatgttaagagctttttacatggtagatggtatatccatacaggagatagtaaagtcggcttcgtaggtttcaaggtaggcttctttcgggatgcttcacatctctcacaccgaggtgagtacatccataaagggataatgaggccagccttatggttttaaggtgggctctctttaggatactttacacctcttctatcctgcatacatggcgaatgtttcatctatgccaagggcttcctagatggagaatactgcatctatgcatggataatgatgtctttatgagttgaggaaagatattgctttcgagaacttgtcccttacgtggattaatatgatctataatacttgtcttgaaatttgttccatcgatgaaatttttttacatgagcaagataagatcattcagttaaaaagatgagccaagttcgttggtgatatttttcatagatgttctatattctatgttctaggttgtagttctttcttgatgtaatggggaatctcttaattggggccaagtatgcttatgcttggttcttttgacaagaaaaatatcgtccataagactagatttcctatgcgaaatgacctctttttaactttagcaatatagtgtaggtcatcttttgttggtacaaaggcgagctttacctgtgaatgatcctttcttaaaggacaacgagcgtataccttctcaactaaccatacgtaatttcactgaagtgttagcaacaaggtaaaggtatttctaccttagttgggatcatatcttggctccataggccataaagaaaaggactcttctagtgacaattctatttgtggttcaaatagtccacaaaacttgaaagagttcgtcaacccattctactttggaagcatcaaattttcttttcaaggtgtacttaatgattttgttaactggatcaacttggacgtttggcttgaggatggtaagatatagagaagtgcttattgattcctaactctttgcaaaattctttggcctttttgttatcaacttcttgcccattatcagataaaattgaatggaaatgtgaaactggcaaatgatgttcttctaagagaacttgaaagtgtaggattctatgatttttcagcccttggatcagcttatatccacttcgtgaaataatctatggcaacattatatagcatgcactacctcttccttttggtgacaacatatgaggtcaattcctaacccagcaaagggctaagggctagatacaactatgagctcttgtgaggtcacctttgtatagttgcaaagcattgacattttttgcacttttgtacaaattacaggacatcattttcaagttgggtacctaagcagcttcagtacgagaatggatcctccgatgcgatttccacatatacccttataaaattctctgaggacgtacatcgcctcttttcctcctgtgtatcgaagaaagagtggtgaaaattgttatttatatagcatatcatcttgaagaatgaaacgtgtttctcctatcctaagcttttgcgcttcatccttgttaccaggaaggacctgatctttaaaaaaggctatgattgtttacatccaagatgggttgcctccaacccatatcacatactctcccttggatattgatggcttggggaagtgtttgatcctttgaaaatttgcaagtacatgggatcgtaataaagtaatataatggtaaattaagtatcaaatgtttaatcaagataaagttattaatacacttaatcgaatagcaatattgagttataattaatctacgtcttaagttattaatgcacttaatcgaatagcaatattgagttataattaatctatatctaatttatcaactaactacagagcaaagtagaaactcgtcaaatttgtgagatgtattgctaagatgaagaatcgcccttattattctatttttagtccaacaatgcgagttggtcaatgttcctaatttatgtaaaagcttccctagattagcaattaaatctaatcctacatgtgatctttttatatctctatgaaagatacatgtatgtaagaaaccattaaacatgctagaatatctataaaaatcatgtcaagcatagagatatatctctattctctatcaaacctcataatgcttattactacgtgctaatgatcttattacttctttcgatgacaataaaacccacaagcaattcaactagaggccaattaatagaaaagcaagataaaccataataaacatcaaagcattcaaacatgataatgtcaaactaattgttcaaatgaaaaatctcataacaaggatttatcttatcctagtaatgtaaaaatctaacttagcatattgaaattagaaaaaatattctaaaatcaataaacatcacccagaaaaattgaacaattgaggagaaatcttaaattcttgaataacttcgatgaattcttgatatctcttgaattatcctcccaatccttgtcaattttctatgtgaattttatttgataattttcttgcaattccataattgaaacctctcacaaatattatttttccctcttcttccaatagatttctcaaagaacctcgatgttcctgtgttgtttttgcgcaaaagaggctctccctaagtgtaggagatattgtaatatttatattgctcaagttttggtcaaagatatcgtccaaagtcttgccaatttgagttttaatcatataaggaaacttgagattcaactaaattttataactatgtgacagcatagttcaaaaggttgggaccgcatagttcaaaggttgaacacgatattttcctatatagtgccatgcactggcattcaaaatgcactatgtggctgcatagtttaacttttggctgccttcttcaattctttcacattttggtccctgaacatctacgcattgtctttttcctcattctcttagcttcctagtgcatccaattgaacccttagtattttcattcttcgattcatcaattcaactattgaattgctgccactttcatcccgtcttttgaatttcactatttttcaggatttttaatttgttttttccaattttttgttcaacaattgagtaatacctatttagcacaaaatacaataatttagcatatattttatcgaaagaacaactaaatatcactattttaggccctatgtataaaatacacttatgagtgctcaattggcactatcttgagcagtttaaaatcactgctaatggtgagctttgatattgcatttgcataagaatttttaaggcatgggatttgcaccaattcaaaattttcgaaagatgaaattaaatccgtaacctgttggagatatgctactgtgctattatctctaatggtgaaattttcattgaccttgctcatcattagatgggagtcactgcacatgagtagctttttcacttgcattttataagccagtctgtagccaactaggagggcattatattcttcaatattgttggaggctttgaatccaaatcatgctacgcaattgagcttatggccttctaagctgactaagaccattcttgtcttggaacctatatctctagataagccatcactgaagcagtaacgaggaaggggatgaatttttccatattcgggtagtgaggctttgcttgtaggagtgtatatctcatatagtaatggaaaattcgtggttttactcttttcttagacgaaccgagctggtgacttctttagatacaaccaaagatagtactaggggctcatcatcttggggcttgaaaaggatggaagcctaactgaagtgtttcttcaattcctggaaattatcatttgggcaagctttgttaaggttcaaaaggagttaatagactcttcacttgccactatgcttctttctgaagaatggattggtgattcacctcagatatagggctttctgataaagcaattggttatcagcttgtcaacctataccttcaaggatttatacttctctagactctaggctctccgttttttactatgagctatgagcgtaggataaattttgagatggtggcatctcaaatttgggtcgaagccattcatatcttcatgcttccaagcgaagatatccaagttcttgcacaaaaaacttttgagcttttcatttgctccttgtggtcgatcttttcccctacttgtagtgacttggtaaaatcttggagatctacgtggaagctttccaactcttttatcgaagatatttgtgtatcaaactcgatcatacgagagtccaatttatcatatgttgaccttttctcaaggatcctccattcttcagagcatctatcatctcgacgtcttttccttattttggaatttgcccttttttagggatgttgatcattttgaagccaatagtaacatttcctagcccctatcttaacatgtctagcgattacaatgacattccttgttaaaagattcacgtataagatatgtatggaagtaaaggctcataattctttcaaagcatgtcttcctaaaactctgtggtaagttgattttttatccaccacaagaactccatgtaatggctggccacttaggaatgctatctcatatctaccataagaatgattgtccttgtgagataatattattgcctatgaatctatagagtgggaaagtcatggaattaactcaagatccactagtatcttatcataagttgctccaaatataatgttaactgtgctcccattgtctactagaatgcgcttcaatttattacatgctgcgattgtccttaccaccaggccatcacaatgaggatagtgtagtcctaccatatctttctaagtgaagatgataggttcaatccttattattctataagggtagttgtctatttagctggtcattagagagtctttagcctttctgtcagaattcctttgagcattacttgaatcttctcccacataaagccctcaaaagattgtatcaatctcccaaattagtgcattatccatatccgttggaggtcttttctttatctttatacatttcttggccttttcttttcctcttctcttttgtgacgatgcaaatcttttctagaaggtcaacttgcaagtcttattttaggctgttgagcataacttggtgggaaccaatttccttataaggacgattctctttctcagggtatgggagttacttcgttctatggagactagcacatttctacactcattggtattgtggccatgagaattgatgataagtatcgaagggttaagtatctttagggcctcctaggtctatttctttggtcctcttgcatggccatgattggcatggcatttagtgtggcagaggtgtatgactgacctaagaagggggaaatttgacgtcctacttaagaccgatggtgatttaccaaatggaagatgggacctttacctctttgcctatgagggaaatgggaatccaatagccacactattatagtattcgaacatctcttcatcgatgatgtcattttccatcatctctaccaatttttcataggaggtagtgttattgttatgaacacctctctagaatatgatgttcacattgaggcctctttttaagatagaaagaattttacatcatagatcatcccacaaaaaatcatttcattgataaaagaggctaagtaattgttcaacgttttatcgatgacttacttcatatcttggaggtgctaaactggggcctctctttcctacttggataggaatttattcaagatttggtcttttagattcaaccaaatcttaatattcatagggtagagctcattgtaccaactctgttatcctgcatatagtaaagtagaaggctcttcacttcagcactaggaaggctcatttcaaggtcatgtgagtcatgtaagtatttaggtgcttttctaagtcacatcttccatcatacaatggtattttgaggatggaaatggtttgatacctaagtattccaaatctcctggaacaagtgaaggttgtcattgtcatcgtcgagctcataggatctgtatgcccattctttatcaatttggtagtgagacgatggaaagttcattgttttatacattgtggcctagactagtcttctttctcgcgtatttctaggttgtaggtcattttgaagcccattcctttgcgttcgtcctagggcctaaatataatatgctaatgtcgtgccctatttctaggcgctttggtgtctaaccaatcaaagatgttggtaaacctttcaaatcttcactctcattcatcgccaagcagataggcacaaagccagttaagggcctgagtccaagcatagagctatactgcaagctgatactgaaaagatccttttcttaggtaatggagatactctaagaattccattagttatgtatcaacgttctcgagttggtattcagtgagccaacattgactctgaagccagtgatttcaattgcagttgtgggttcagaacgaacttaggagggagaaaagggggccgggcctagcacgttctttttggtttgggacataggctattatattatagacgcatcattaaagacttttcgaagcgtagaggttttccctgactttgtccgtgtcaacaaccaagccttgggtcggggtcacaatgacttattgtagtgaatcagaatcagaatgcgctcttcatataccgaatggaaattgtcttctccattgaaaggatcatcgcttgtctcagccactattactttcctttcaataaggctgatttctctcgtgtcaatagaaatggaccctattactttgcacctcatctttttcttgttggttctcccattggacttgttggccttggaatagatccgattgaggcatatcttagggcatttgcatactcacttgccagtaaatttgttgtcgtagttgtggcattatgaagtcctacttcataatattcctcatgttaatggccatgactactacttctctggtaagacgagctgctacccgaccacctctacgatgatgctatcaacgatcaagtgaataggtttaggggggctcttctatagagacttcctgggtctctttagatttttattttctgcaatcacactcatggtgggtagacatctcatttattcaaaaaagagtcttttaagtagatatttcttttcacaaatctcctttttcaaggaaaacgtgaaacgccaaagagtggagaacaattggaatattctttctctgaaactttcacttattcttttcaagaacaaaatatttttcaagggaaaatttgaagcatttcgacaagttgtttccatggtttagtaatgtggctttctagagacagtgctaatttgttggcctcgattttctgaatggatgacatggccaacatatctcgtttccacttacgcccatgtagcctttcttctccaaacttagacaaatcattgggatgagtagaagtcatgagctagaatatagttcggcactggggctatataaaagagcaaatatgaagcaatattacttagagtgtgtaaaattacattatcctcaaatgatattaagtgtaagtttttatagtagaagtggtgaaatggttactcttggatgaagagatatgtggcatcatcttgaaagtcgaggcatcttctcctatgtgtcaatacgtcattcctaggttcacaggcatttaatatttatgaaaaatagccaccctatagcctaggttaaatctttgaaaaatatattaatagttgaccataaggcgtttattgtagagatgtcatatcaatcaatcataggaagattttggacaaaaaatctctagaaagaggtgaaatgggaaatgtcttctcttattaaaaggctaattgccttatattcactctgcaactggttatacaaccttcacaaggccataggaggtgtcggcctctacatggaacctcggctgaagtgattcatcaatttggttacctcagtatattgctttggttagatcattaagatagtgatgtggagtatgtgcttgattgagcttgctagttgcctgccacatgatcgtagtttggattctcatttgaagatgtgtaatagtattcttagagtcttagatggaatccgtcagtggggatgacaagagccattaaacagagttgggataaaagagaaaatggtaaaaaattgggggtggtggttgcaagttttcttttctaatggtttgtcaattatcatccgtttagttttaactgaacttaatttaatttttactgtcattgtactggcagtattattgtcaacatgctgatagttgttttcggtattttgatagtcctgtatttttggaaattatgaaagccagtcatatccaatgaatgaggacctgaagaagctttacacttgttatatatgtaacctttatcttattctatctgccttttgttttctggtcttcattaagtaaatttctgagagtctactattgtagcagaatagtacttctctattattgttggcattatgcttcttttggtttttaatttaattatcaaaacaatttgaatctgcatttgtttactagttatctagcaagatatggaagaactcatataatgaatcatttgaatcatcaattattgtcatttagtatttcgttcgattgacagtggacctggaaaagtatggtttcacatgtgctgacagccccacaatacttttgcctctatgaagaaagcagattgaattttttgaagagacattgcatcgagtgatcgattcggatattataatacttaaaactatcaataacctttagggtattttgtaaatggaaccattcgagatcatgtaattattagaatcaaactcaaaatcgaactagaaccatccattatgctgcttttttattttttataaatcatgagtttattatccagtatatcttttcaatatccaccagaaattgaagaaataaaatatgctatctaatacataaaaaaaaaaaaaaaaaaaaaggttgaaccccaacctgagggcccccaccgccccgcccctagagttttgtgagggaggtaaatcacgggatgtgccccaacaggttagagaacaagagctgcttatacactgcgcctacaaggagtccaattccatgtttcaggaatcgaacccccacactgcggctgccagcaagacgtgaaataacatcactcatgtcctttgcaccgctagactatacccccgggggctatgctatctaatacatattttgacacttcagtgcttcagccccgtgattaatcctaccaccatttggaaaatcatttctcttgccctccttgacgttgaggacatcctcgaagagcaggagatttcatgacatttcgaattggctgtcttgtaagctattcatctcctcgaacgcatgtggaagcatatcacctgcaattaggagccactactggatctgggcgagtttgtttcagccagcctcaatccttcccaccatacctgcctttcctgggaaaagacctagaacatacttcttaaaaagggctccaaaaaacaaccaacagttacccactctatcgcagaagctgaatactatctagataatgaccatgccaccaagtgtaatcagtatcctaatgtagacttcagagagtctttatcagtctggaagtttgaagtgttataataaaccaaatcaatattttggtgatgaccatatgatttattggtctccaaaggtaattaagggtatgctttagaaccaagtatcattttcttcaatggtccagtgaactatcacatatgccgaaatttaaacgtcactaaaattgaggtcaaacttataaccatttcatagaagacacttagatagtcattctacccatttttcaaagggatggttacgaatttgtattttctactcagctcattttcaagttctcaacctattgacatatttgatcaattaaattgatctctcccgttagtaaataaacaaagccaaataaagtaacgaaaacatatacaaaaatgtcaaaaagatttagataaaatatccaattattaaatgatttattttttcatacgatcatgctaactatttctgcgataaggacaaattgcaaaattgaataatgaatctaccaatactacaatcttctagtacaaagtctcagttcttatacattgattataaacgagttatttatgatgacaatataagttatattatcataatgtgcttctccactcaagcacatggcttatattatcacaaatgatattatgaactttaatttggatactcaatattaaataattataataagcccttgtttgattcctattattttcaaaaaaacaattttctccatcttcttttcaattacaaatttttcaataaaataatatgacgtgcaaattcaaaacttttctttattgtttaaccacacattctccaataatccattttcccaaaattcattctacattaaaaatagggtaatgctacgtaatcccactgaggttgcaatcacaatttaggtgacattagatgataggttaaatgcgaggtgaaattaaatatcacctctcaattaatgtcatattagcgtcacttagatctaggttgcaacccccaataaggattaatagcattactcttaaaaataatgctgaaataggacctaaataaataaaataaaatatttatttatttattacaagatattatctcagaacgacaaattatttcaacacacaacacaacaataatttgctccaatacatgataatgtaacgtgcttgaagtaccaagttgcatccaacgaggtccccacaccctgttatagtcgaactaatttctccacgtgcaatgccactccaaatcctttttaaggctttttatttttattattatttttatttatttttattttctttaaataatatcctatcattcatcacagaggcactagatatctatttaaagatcctcttaagattttctctctttcctctttggtccaaccatacaaaaagttaaaaattcacagtgctacttaatttatggcacactttcccagttggggtcttcataaaaggtctactttacaattgccatttttcaaaaaattgaatatatggtgatataggacaagtgtcgatattaaaatgcattgatatatcattttttttaatcctatggtgcaaagtataccagcacacctggtgcttctgtttaaaatgtctattttaaaacaaagttgtttgtattttttaggtttctcttttcatgtttaatgacgtcgaaaggaaaaagcagtgagagaagtgttggcactgtctctccacatacaattccttaaaaacaagatttttttattggtaagcgtaaaattttattaattaaaatttcatgtataagtacatcgagcatacttgtgtaagacaaaacaaacgtttaatacaattactccgggcaaaccctggcaaaataaaaggaacgaaaaaaataacaaaaatcaatgacccaacattaaggactcataatgaatcaagacatacggatacaaagagaacatgactttgtatacgtgcgtattaattctattctcaatacaattcaagtgtggtctaatgtcttcaaaaatctttccgttccgagctaaccaaatgtaataaacagtacttgcaagagcaatcatcttagccttgctaagccatgatgtccacgagcatccttttttatccacttcaatgcactaacgagtgtagatatagatctttttatgccaagccacatcctcttattaccttttttttttttttttgatatccagttatccgccttacagtgactaaatcctggagtctacaccttgacccctcaagctgcagacaggttaaaccccaggttgtgccccaaactaacaagtgttcaagagccccccaactgatctgccaaagtaccaaacaagtcgtttcccatctttgcaccttgccttctaatagagctcctgcctttcagaataaatcctgaattccaggagaatatctgcgtttcaagagtctttcaggaatcgaacttacgacctctgatctgtcagtcttgaagcgccctcacatcctcttattactttacttctatgtagtgtacactacgcattaggaaaaaagcacacatcaggaatgctttcttctattatatatgtcacacttctctatatcatatccaagtaaagatacacaatctctctctctctctctctttctctctctctcgggttgaacaagagctaaaattttgtaacaatgttggtgaatttctttgggatgccttcggcatcgtcgatttttgcagcgtatgcctcgttatcgacatttattatgctgcttcaaactgtgttgaatcaactcatgccccatcaagtgcaacattacatttggtccttaattcagctctttttaaagaccgcaacctctaaagccaccatagtcattgaagaaagggatggtatgtcgagcaacgaagtgtacaatgctggtgaaatctatctgtccacaaagatcagacaaaatatcgatctccttaaggtttgcaagcctcataatgagaacaatatcagtgtgaagtttgctcaatgtgagaaaattatcgacttctttgaaggcattgagcttgaatggaaatatgtttacgaagatagaaaaaatagtaccaaggtaattgatgaagatactgacaatcttgttttcatatccgagaaaaaatacttcgagctgagtttcgataagaagtacaaggaaaaggtactcgaccattacttgcctttcatgcttgaaaaagccaagtccattcgagcagaaaagaaggttatcaagttgcatactttaggtccttattcgtccacaaacgtatgggattctgttaccttccaacatccctcaacttttgacacccttgcaatggatacaaagattaagacgagtctcattgacgatttggacaggtttctccaaaggaaagatttctacaagaaagtgggcaaagcttggaaaagggggtacttgttgtatggtcctccaggaacaggcaaatctagcctgattgcagcaatggctaattacctcaaatttgatgtttatgatttggagcttactaatataaagcgtgattcggatttgagaaaattgttactgagaacttcaaatagatccgtacttgtgatcgaagatatcgactgcagcgttgaattgccggacagaaatgggcctatttatgcagatggacatggacaggctcgtgatattcaggtacttgaaattctagttattctaatctgtttgacagttggttgagctcttgatctccctcgtcctccccttctttctatgtcatatattattaactagattaaatcaagcccaactatcagacaaacaaaatgctagatagtttaaatactagctggattaaaactgacaaaattatgatgttgacttatgtttttttctcctgaggttgttcaaaaagcttcgtgcaagcttctttgtatttgcatcagatgactctcgtgaaatagctttgttttgacacacaataaagcattatagaatttaatttttgttgcactaatgtatataatggtttacatatacatgatgtgtggttaggtatgatttgaccagaattttttcaatcaaatatatatggattatgctacttgtacataagttattacataaaataatgtggaaagaaaagattggataaaaaagttgattatgttttaaagtggcaaatgatagaatgacatgtgacattatatgactcattatgtaaaatttaatgtgtgtatatatatatatatatatatatatatatatatatatatatatatatatatataggaaaatgctgtgtgtacacacacaccccttcatgtgaggggagtgtaaagctgtgtgtttatatatatatatatatatatatatatatatatataaaaagatatttcatttgaatgtaaactattatttactgtcattaagtacaagcagctttattctttaatttgcgagacagaaaattctctatttgttttgcagttcacgctctctggactattgaacttcatagatggtttgtggtctagctgtggggatcagcgaattatcgtgttcactaccaacaacagaggaaaactagatccagctttgctgcgccccgggcgcatggacatgcacattcatatgtcctatctcacaccagatggttttaagcttttggcctccacttaccttggcattcaggggttccatccgcgatttgaggagatcaaagaattaatagagattatgaaaattactcctgcacaagttgctgaagaactaatgaagagtgatgatcctcatacttctcttgaaggtctagttaattttttgaagtgcagaaggatcgaaagcaacctatcaaaggataaaggaaacgaagaaaatgaagtcgagaataaaaaaagacttccatctgacagtgatattgaagtcgtgacagactaaaatttatgtgaatttgatcatgcttattatgattttaaattagaatttgaaattgcggttcttgattaaagatccaagactctacctatcgaacaaacaatgagcttgtatttcttaatataaaactatttctagaattttgtctcattacagtaatttctagagaagaagagtgacctctatcaccatgttatttattatctccatcagttgtacgtgaaataattggagtggaaggagcatgacatacgctactaaaaaatagcttttcagctaaggaaaattaccaacggatacaatccgtcggtaattagaaacgaattatccattggtaaaagtaatttacttttaactatgataatcagcaacgaatttttcattggtaacaatgatatccttttaccaatgaatattctgtgtctaatgtaaccgtttaacatttgaatctttcacacgtaccaaatattaccaacggaaacaatttgttggtaattagaaacggattatccgttggtaaaagtaattcacttttaactacgataatcagcaacgaattttccattggtgatgataatatctctttaccaacggatattttgtgcctaatataaccgtttaacatttgaatctttcacctacggatattccgttggtaattaaaaacgaattatccgttgataaaagtaattcaattatctcacattggaagtttacaataaagtctttggagttttcctctataaatttgtggtccaataagtggttaaacaatatttttggcttttcaattcaattgtttaaaagttttaaaaaaattataattattaaataaataataataacaataataaaaaaataagtcaataatttttttttttttttttttatcatacctcacatctatacgattatttacaacattaatttttaccaattgtaatgttagacatttacaaacggaaagtcagttagtattggttaagatttttaccaacgaaaatttcgttggtaaaaaattcacacattaccaacgaaatttctgttggtaaaatgcttactctttacctacaacacaatccgttggtaattatcagcgaccttcaaattaacaatggatttgtggttgcaaatattccgttggtaaagagtaatagtaacagatatcaagattataggaactgaaaatctgtgtccgaagctatattttttagtagtgatattatactccctagtccctattaatcatatcattcagctcaccatcttaaagcatcaaaaatcctgcgttagaatattaacatataaatggattttataatttttgtgcattaactagaatatttattcaaaatgaaacatagaggtattttagggatatgcgtactttacaaaaatcctattgtgctctctctttgttcctccagattccaccttgaagctctagagtacttctcggtgttcttaaagatgaaaaagaattgcagcaattttttatgcgtgatcactataattaaaaaaaataaataaatgaacaaataaaaaatcactagacattaacacaaatacacacatttatggtcgcgcgcgcaaatatacaagggacacaaaccctgatgcgcatgcccccccccccccccccgccatgtgtccagtttaaatggcacgtcattgtcttattgaatttagttacttgcactacagtccctgataaattatatctcttatcataaagttataatttatctcaattcttattttgaagccactaaaagatcttgatcggacccggttaaactaaatttaagtaaattaatcttgaatggataccattccattaagaacaagattgcactcacaaataatcaacaattatattctctgacttgtctttcatacgtattacccatgacaatcatttataatatttaaaataaggttaaaataaccaaaacattattttcaaatatacttaaatcctcaaattcctttttatatctcacattttcatgtgattgttggagaaaaatcaccgagttagagtagagatcacaaaatatgaataaaaaaggccaataacaagataatcacgaacttgtatcaatgaatggcttgaacacgatatcgttgtcctcaaacgatatttgtccattcttctataaatttgagatgtttcgaaagttgttagcaaatggtttgcaggattataacaagccttgcaaggatttaagcaccaaaacacaagtgcaaatcctagaaaacttgaaaaacataaatgatgaatatgaatgacttttaaaaactttgatctttgattttggaagtaatatggaaccttgattttttttgtgatgatagtgccttcaacatggatctaatatatataggcatacaccacattcacgaaatggtaccaaactttaagccaaaagtcaccaattttgaatttacaacgggagaaaacggtctccaacgatcaaataattgtaccatgcaaccgcatggtacaaattcatgcggtcccatgatttgcccatgccgagaccatttggtctaggcataaggctatgcggtcgcatggaccaaatatatatatttttaatttattgttgttgtttattttgaacaacaaatcacagcagtgatcacatcataatattaattcaacaatcaacaatgaattattgagctcatatttaagtatccaacataaaatcctttgagatcataatcgcgcctttgtaatatgtgatgtattccatatttgcaaatatatgttcctcattatttcactttcatttcaaaggcaccaaggtattgaccaacacctttatctcatctattgatatctcaaagaacttcaggacgtgatggatgaggaatcaccgtaaggtctatcaccgtataaagtaataggacgtgatgcatgaggaattaacttaaggtctaccaaaaacttcgtaagacacacctttaccttattcgtctcacaagctacaatgtgccttcaaggtgaaattaacaatagctcttgatgcttatctaaacaatggacctgccacttactatgaacactggtttggatatgcacttgcatcttatcaatttgaaaatcaaaatccatataacctagtagggaccaaatttggagctaaataaactaagcatattctctagttctacatatattgccccccaaggcatatcccagtggtgcaaaggataagggtgaggtatactcagctttgctggcagccgcaatgcgaggattcgattcctaaaacatggattgagactctttatggacaccagtgtataggcagctcttgttccttgccctgttggggcacattccgcaactaatctctctcattgtgctccaggggtgggacggggcggtgggggattcttaaagttagggttcaaactttttttagttctacatagatatttgagtatatgcttaatagctgtcaagtgacccggtcctacatttgattgatatctatttaaaatcccaacaatatagcaaatatcaaactgtaagcacaacacagaatatatgaggcttcaaacataagagagatataagaaacttgcatcatgaatggcacttcacaacccaaggttcattaggatttagtcttattagtttgattaaacctaatgttccaagttctagatgtctgctaaagtctataaatggacattttcagatagtagagtttatgctcttggcccttttaaataaaactatgtggttacattaagatgattcttatatacttatgcttaattgtgggtgaggaggtctcatcataattgatgccttcttgttatgtaaaactcttaaaaccaattagatttaaaggtctctaccttttcgtttgcccctctttttctcttatgggcccatttccaccctatggattttaccctattagttacatctagtagattctacaatggctagtgtacatagatttcatttctgagtcaataaaactcctccaatggtcaacgtctatctcctccatagattctttatataaaatataatcctcatcttgcttagttgagactaccatataatactctccatagagcaagtattgggatgctgagtagttcccccactacattaattgttggagcttcttagttgaatggaaattgaaattgttctcttactactcctttaccatgctcctcttctttagtctcactactatgtggtgccttaatagttgggacttgatcctttgacacctctagtgtttgcaagttaatgggtattgcaagtaaaacctccaattgtgtcccattatgtcaaggcactattggcgatagaggtgttatcttattcggttcaatgcaaatctctagaatagatgatctttttctttactctttctaaaaagaaccttaatctaggattcacgttcttttatacgtgtttcctaagaaggttgcatttgtactatgaagcacattcttggtaatattctccctttaggatattgtataacatgcatacttgtactctcgattcaatcttatttgtcttttcgttgaacacgtgttctgatatttgcactatctaaatatgtcataaattaggcttgtgctcattttcctacttgagttgtgtcttagggatagacttaggtgaaaccatattcaaataaggatattacagtttgcacaacatatcctcataaggattttataagagtcaagaagccaacagagatatgataatgtccaacaaagtcttggttctccttttggagacaccattttgtttgaggtgtacctgatgcactcaatcgggattattgggaatttacttatcatgcacagtggaatttaaaaattaattcccatcaaagatcttctttgtgtttatatgaaaattgtgataaaagttatacttttttttagatctacaagcttctttgcttttcctttgttccagcaaccttgatcagccacccacaactgtccaattgtccagcctccaatgaaatttcacagaaaacaagattgtaggtaccggggttttctcctcttatgctagcaagaatgaattctctacaaaactgtaaaccttagctacttatttatataatcccaaacgagcttagcttgacccagtccaatatttaattaacctatttaattaaatctggtccatgaattaattaatccaggctaataagtaaaccaaattattcatttatccaacgcctgttaaattaattaattgataaatcacaatcttccaattctccttttgtgtgtgacaaattagatttccgatcacgatgcctaaggatatgaaatattattttgatctaatcaaaattgataaattaaaatactcttttaatttatcaacaattcacactcgccgtcccaaattaacatctaacaatgtatcaggacaatacattgtgaccgaaaatgtcacttagtatgagaaaatcaaacttgttcgtttatcgagaaattataatcttttcgtcgatatgatccaataaattacgaaatatggaagtgtgtcaatcccgatcatcaatcatatttttcattccactattaagtcaatataagtcgaaaactccttttcgatttctgagtacacatttgccaaggatttcgttatcgatttaatcgaatgaattgtggatcataatctcttactatctaagagtgacgaatcctttattggtcattcacaatcttcatataattcttgacatacccgaacgatgtagtattagcgttccttagtggagtaacatccaacgccgtcaaagtataactgtcctcatataaggtactatgatgacctcaagttaaatgataaattccactatcgaacgttagagattaaccattaacactcggatagttatccatgtagaatttcttagtgggtctccaatgttttgttttataacaaaatatccacacgttcatttaattgtcacaacactttaacttgtgagatcaggtacttacttcacaagtaagaaatatcatacgtgatggtttaaccgtaataatgatataagtatatcgttattacttacgactatttaaaatccaatcatatgtaatttgtattttacaatcataacccttttgattaacaaattactgaaaacttgaattttcagactctattatttaatattatgcatcagaatattaatttaaataaataatagatcttcccaaaaataaatgcattaaatatattaaaaatgtttacaatctaaatcggttggatctagggataacacattacagggataaaatctcattcttttataaatatgttctaaagtcgtaggatatataccttctaccttaatttgatcgaattgttataatgttcttacccaatttcttttccacttcaatcatatttccttgatctttttaggggtttcagacttgcaagccatcagacacacacacacacacacacacacacacacacacacacatatatatatatatatagcccatgtttggctcctattttgtggaaaaattgatgggtggaatagtatttttttgaaaaataagtggttgaaaaataagagagagaaaaatgtaatgacatgaaaattaatgggggccaaacgggggcatatatatatatatatatatataccctcctctagtaaggacaataattggtccccatacatcaaagtgtactaattataagacttcctgggccatattctccttagatgtaaaaggtctcatggttatcttatcctgtaaataggatttacaaattagtagggattctatccatacttcacttaaaggatcatcccttactactctttgaattctattaaggttaatgtaacagagtctatggtgacacaaatatgtctcactagagagagaacatttttatgcatttattaggtttagtaatgttgggtgtaaagccaacaacgcaatctgaaatatataaattattaaacgagtgtctatgtttttcgatatcaagcataaactgcacaaaaagaaaagaatatccatgctgaaatatttgagctatggaaattaaatttcgttttaacattaggaacaaaataaaaatttctcaaaagtaaatgttaattttgctggagaaataggaaaatagatccaatggctcaactagacactagttctcatgtgtaatctctgagaaataactctctttgttgaactccatagttatttgaaaaccctgcaatgaattgtaaatatgattggtggctccagaatatgatattttggtattagtagaatcaactactaagcatgactcaatatatgatatattaccattacctagctttttggaaactaggtattctaggtagttcctcttctagttacacttctgtccacattaatgcattttccattaggtttacatccatcttcgctttcttagcctactattgtgggtccttcatggtggaattcttcatctttttctttccactttaggcttggaaatgatagtccagtagaagaaacaatgaaggttacaccactcttggtcttcagaatagcctcaatattttggagctccttcttcaacttgttcgaggatagcttcagctttttcatgttataattaaccttgaactatgaatacatctcaaggaaagtctaaaacgattttaacctgcatgttcgatttgatttcattcgttaaattgagtgatcaatgtaagcatgcgatctcacatgcatcccttgttccatgtaaatgcttataatagacctaatgacattctgttgagcctggcaagcttgaggtccaaatgtatcctgaagtctttccatatcttgagctagagtgtcaatgttttgatatttctactacaacacttttgacttgaaaaccaaggagttgtgtatagtaatatgaaaactgctaaggagttgtggcagtcgttggacagaaaatataaaactgaagatgccgaggctaaaaattttattgtcgacggatttttagactataaaatggtggactccaaaaaagttatcagtcaagtgcaagaactccaaatgattcttcacgaaattcatgtcaaagggatgattttgagtgaaacttttcaagtggttacaattattgaaaaatttcccccgtgtggaaagatttcaagaattatttgaagcaaaaacgaaagaaaatgaacgtcgatgaactaattgttagacttcaaattgaaaaagacaacaagagttctgaaaagaagtggttcaatcctggtgtagctaaagcctatgttatagaccttaatcaaagtagtaaaacctacaaaaacaaaatttgaccatctggtggcaaaaggactaagcaaggaccaaaaggtgaaatttctaagaaaaatttcaagagaaatgcttcaattgtgacaaagaagaccacaagtctttgaagtggagattgccaaagaagaagaaagaatcaaatgtggttgatgacgtgacacaagatgtgtcggagttgaatctctcagccgtcatttctgaagtgaacatggtggaatcaaatcctaaagagtggtggattaacaccggggttacgaggtgtgtgcactttgataaagagctgtttgaagcgttcagcaattgaaaatggggagaagttgtttatgaaaaattcaacaacttctgaaatcatgggtcaaggaaacgttgttctgaagatgacttcgagacagaagctgactcttaaaaatgtgctttatgtgccaaagttttgcaacaacttagtgtctgggtcgcttttgaataagcatgattttcgcactgtatttgagtcagacaaagttattttgtcgaaaagtgaaatgtttgtcgaaaaaggttatgtttccgatgatatgtttaaactcaatgtaatgattgttaatccaaaaatgaataaaacaaactcttctgcttatttgcttgagtcttccaatttgtagcatggtagactaggacatgttaaccatgatactttacaaagactaattaacttgaattacatacccgagtttcatattgattacaaatataaatgaaaaacttgtgttgagacaaaattgacaaggtcatcgtttaaatcaattgaacggaatataaaaccacttgattcaattcacagtgacatatgtgacttaaaacttgtaaaaacaagatgtggtaacaaatatttcattacttttgtcgacaatagcgcaaaacactatcatgtgtatctgcttaaaagcaaatatgaaactatagagaaatttgttttcaataagaatgaagttgaaactcaacataataagaaaattaaggtattaagaagcgattgaggtggtgactattaagcacaatttcctgaattttgtgtacaacacggaatcatacatgaaaccatcacaccttattcaccgcaacaaaatggtgatgatgaacgaaaaattgtactttaaaagaaatgatgaatgcaatgctagtaagtttcagattacctcaaaacatgtggagggaagctgcgttatcaacaaagtaccttttaagtaatgtgcctcgaaagaaaatgaaaaagaccccttatgagctatggaaatgaagaaagtcttcctataaatacttacgagtgcaggggtgttttgcaaaagtggttgttccaacaccaaagaaggtaagaataggaccaaaaatagtagattgtatcttcattggctatacacacaatagtggtgcttatctgtttcttgtgtatgattctaaaattgtagatagacacaaaaaacacgttattggaattaagaaatgcttcattctttgaacatgtattttcgtacaagttcaaagaggaaacaagctcttccaaacaaacatatgagactatgactgaaaatagtcttaacgaaaaactagaaaaagagactgagattggacgtagcaaacgggaaaggacaaaaaatcgtatggtcatgattttcttacttatatgctaaaaaatgaacctcgaaattatcaagaagctgtgaattcttcataaggacctaaatgaaaggatgtcattaaaagtgaaatagattccatactgcaaaatcatacatgggaactagtggaccttcctctaggaagcaagccactagactacaaatggattttcgaaaagaaaataaaagcagatggaactatcgaaaagtacaagaccagatatgtaataaaaggttacaaacaaagaaaaggccttgattattttgatacatattcttcagtgacaaaaataacatctattaggataatacttgtgattgccgctttttaaaatcttgaagtataacaaatggatgttaaaactgcattttcaaatggagatttagaagaagaaatctatatggaacaacccaaggagttttcattaccagggcaggaaaagaaagtttgtaaattgataagtcactatatggcttgaaacaagtgcccaaacaatgacatgaaaaattcgataatattacgatagagagtggatttagaatcaatgagtgtgacaaatgtgtttacgtcaaagacattaaagatggttatgttattttatgtctttacgttgacggcatgcttattgttggtagtgacaataagatgattgaatccactaaaaatatgttaaattcgaaatttgacatgaaagatatgggtttagctgatgttatacttggagtcaaaacctcaagaacataaaatgggcttgttctaagtcagtcacattatgtggacaaaattttagaaaagttcaataagaaaccgatagataaaagccatcatctatctaaaaataaaggtgaaagcatctctcaaatataatattcaagagttattggaagtccaaagtgtgcttaatgagttgtacaagaccaaacacagcctacacaatcagtaaactgagtagatacacaaataatccaagagttgatcactggaaaggaatagtaagagtactaaggtacttaaaatatacttgtgactatagactacattataccagatatccaacggtcattgagggatacggtgatgctaattggatatctgatataaaagactcaatgtccactggtggacttgtgttcacattgaaaggtgctaccatatcgtagaaattctctaagcaaacagttatagccagacctacgataaaatctgagtttatagctctggataaatgtggcgaagaggccaaatggctactcaacttcttagaggatattccaagatggtcaaaatctgtgccagcaatttgcatatattgtgacagtcaatcagcaataaaaaggacatagagtaacatgtacaatggtaagtctagacatatacgtcgtagatatagagtaacatgtacaatggtaagtctagacatatacgtcgtagatacaatatcataagacaactactctcaactggagttatcactatcgaatatgtaaggttaaaagataacattgcgaatccgttaaccaaaggattaaatagagagctagttggaaaatcatcgacaggaatgagacttaagcccttgaacagataagtcattacaaaggaaatccaacctaattgactagagatcccaagatctagattcaaagagacaatctaattgtaaagacttaataaaatcactgtgggggtgttacctcctatccattcccatgatgtaacagtgatgcccataaggatgaaggataagcaatagacttttaataatttttatgcatcgaaaatcgagccaagtaatgcgggttacttgtaataagaaatcacctatgtgagatagaagtgagaccacttctaagagaattttgtggggctcaattcttaagaactctcacagaactagacatatgttcatggtcaaaacgaaaataataatgagaattgaattgtgtgacaaagaatcctatatggagtatatcaacatttacataaacgatagaacagttcaagaataacacgtctactcgtcaactagtaaagtaaatatactttcacatggaaaggctcaaagggtaatacctatcaatcctatacaggcttcaaccattgaactttatcaccaagtcttatctctctcggtctcgtgtctcttccaatttcattcacataggggattgttggaaaaaaaatgaataaatgactcacttttggcacaattttcgatgcgaccctttgttctaatttggaatatcaaaattgatccatgctctcctccgtgagagtatcaaaaccgtatatttacttgccaaaattgatgaaggggtgaatgagaaattggagctcaaaattgaccattggaaaatagtttatgtgagaaaattagatttgtaccacataggaaaaagaagaaagtatgaaccactttatattggctacacattagaaaggtataatcatgtgtagcatagaggctctctccacgtgcgtgcacagggggggttcaaatcatggatcaaaatagccttcgaactttgaatttgtgtgtgggcataacctgcgtacatgaatgtcgaaccgaataaagcaaaaattggcccatctggaatgtccacattttgtaatttttttgctttctccaattgacttttgaatttctgtaactgctaaaactccagcagaaactgaagtgactccaatatttattgccagagttaatgtcatatttatcttatattaagactcattttctagcaattatgatacactagaaaacacaaaaaaatacagtctgcatacacgaaaatatattgcatattattgttctgttttcattcgtcttggtggtgatattgttcaaatgttaactcagttcgtcggagtagtttctacaatgctcagattctattggtttacaattgtatcctgggaaacaatgctcagattaaatctcaagcatttacagtgaggaggcgaatctgttttaaggaagctgtgctcgcataggccttgggttgaaaattcattttttatttatttcctgaatttttatcttatttgttcgacttgcagattcatatgcagttatattctttttgtacttcatatattttaaagtttattttctgtttatattaaaataaaaatctgaaaaaattttaatgacattcggttgggtaagtacatatacgatgttctgcaatttcggtatttgtaaataaaaatcgatatatgaaaatacgatatctaaattggtaaagataatatatgcaaatacggtcaaatgcatatacggtaggcagcatatacaataagctgcaaataagataagctgcctgcaaatacggcaagctacatatacgacatgtttaaaatcggtatctaaattacatatacggtatgtgttaatccggtttcatctattaacaccgctaaattccaacagatttagctaagtcgagcttgaacttgtaacttttctttgtaataaacaaagccattttattgataatacttcttaaatgttcaccactccagggatgttttagagtttcaccattttggtcgtccaatttttatgttcttagccttatacttcaactacactatatgatccttcctagtttaggcctaacgaacttgaccccatatccttatccgcaacaaaaaatttctttattaccaggtcaccaactttaaaggttttactgtgaaccttgaagttaaaatacatttccatcattctttcatacactacgaattttatttgggaggcatcctatttttcctccatggaatctagacttgcattcaaggcttcttcattctgttcatcgtcaaagtttagttccttgtggaaacgcaagcctatttgacgtagtgaaaatattatagggaagatgaacaatcacaaattgagaaacttctcaaggaagattttattgaatttaagaactactgcctccaagggcttacaaccgattaaatagaagaaaaacctaggaaaatccagaaaataaaaaaaaataaaataaagatatttttttccaaaaatggaaaatatgagataattactaagatggaaaatacttatcttcaggatcatcctccaacaaacggaatctaaatccgaatttcatggaaagagatattgtaaaaatgaaaattaccataaatagaaaaaacgattaaacgagggccttaacgatagattttgcccgaaattggccttgcgtcagggccgaaggtgctgagttttattccttgactcgactccaatcaaattagactagcgatttgctaaaaatgagcaaacttaaagtcatcatgaaatcatttgccatttttgccaacttttgccttgtgatggtcccattttgccatgaattctaatcccttatgcacttcatcattctccccagtatggaaaaattcgccctcgaatttgacgagaaaggagtttcatcatcatcatcagaattatcaccatgaaatggcaccaaatgcttgatattgaacacgtcggaggtacgaatatggctgggcagctttaaacagtaagcattcggattgatcttctcaatgacctccaatggaccaatcttcttcacagtaagcttgttgtattcatgagcaggaacacgatcctttgttaacaccgcccaaacgaagtcacctacctcaaactcaacatgtcaacgtttgagatccgcagcacgcttatactcagcgacagcagcctgcaactgatcatgagcctgtgagtgaacctgctgcagttgttgaataaagtcttcagccttaccatgcatttaacagaagtagaaactagaaccagatcaagaggaccacgaggaacaaggccatacaccacttggaacggactaaaacatgtacttcagttaacagcatgattgtgagcgaattctgcttgacacaacttctgatcccaagacttgatgtgatcactaaccaaacaacgtagtaaatcaccaaaggaatggttaacaacctctgtttgaccatctgtttgagggtgatatgcactgctgaagtccagctgtgtattcacagagccccatatgctgcgctagaagtggctgaggaaacgagtatcccgatcagacacaatagatgtaggcagtccatgaaggcgataaacttcacgaaaatacagtaatgctacattgacagcatctgtagtcttcttgcaggggatgaaatgtaccatttttgaaaactgatcaaccactacgaagattgaatcaaaaccacgctgggtcctgggaagtcccacaacgaaatccatgctcacatctgtccaaggctgggttgggataggtaggggcatttacaagcccgcattggtcgccttgcccttggccaagtgacaaacctgacaatgttccacaaacttgttgacatctttgcgcaatgatggccaaaagtaagaagcagcaacaagatgcaatgttcggtcacgacccacatggccctcattatgcaactcttgaatgatcttcaacctcaaactgccctctggaacacacaactgattgccatgaaatagaaaaccattaacccatgtaaactctgactgcacaccctctgcaacttctggacaacatgggaaaagtatggatcagtagcatataagtcacacaacctgtcaaaacctggaacctccactcgcatttctataaggagcatttggcgcctactcaatgcatccgcaattttattaagggcacctgccttgtgcttaatcacaaaagtaaactgctgtagataagcaatccaagaggcatgtcgagcagaaaccttatcctgagtaccaaggtgtttaagggcatcatgatctgtatacaaaatgaactccttatggaacaaatagtgacgccaatgtcgaacggcctggaccattgcatagaactccacatcataagtactataccgagacttcgggccagaaagcgtctcattgaaatatgcaacagggcagttgttttgactcagcacaccaccaatacccactttcgaagcatcacaatgcagctcaaatggttgggtaaagtcaggcaacaccaaaactggagcagtagtcaacttctgtttaatcaattggaaagacgactctgcctcgtgagtccactgaaacctaccatccttcatgcaatctgtaattggtgccatgatgctactgaaatgcggtatgaacttgcgatagaaggaagcaaggccatgaaaaccccgtacctcagtgatagtcttgggctgtggccactgacttatcgcctctactttagatgtatcaactgctaaccccaccttcgacaccacataacccaggaataccacactatcagtgagaaatgaacacttcttcactgcagcatagaattttctccctgagaagaactgaaagaacttcccgaaggtgccgaccatgttcatcatcgttagcactataaattaaaatatcatcaaagtagaccacaacaaatttaccgatgaatgggcgaagagcctgatttataacccgcataaaggtactgggcacatttgagaggccgaagggcatgactaaccactcgtacaatccttccctcatcttaaatgcgatcttccactcatccccacgtctgatccgaatatgatagtacccactcttcaaatcaagcttgctaaacacacaagcaccggtaagctaatccaacaaatcatctaggctgggaataggaaagcggtaacgcacaattttattgattgccctactatccacgcacatgcgccacgtgccatcctttttcggtgtaagaagagcaggaacagcacaaggactaagactctccctgatgtgtccttttgccagaagctcctcaacttgcttgcacaactcttcatgctcagtggggctaattctgtaatgcgttcggttaggtagggcagttccaagtaccaagtcaatctgatgctgaatatccctcagtggtggtagtccatcaggaagctcttccaggaaaacttcatgaaactcctttagcaatggctaaactacgagagggacttcatgctcactgtcaaccgactttccaatcagcacatacactatcccagactcctccatctctgtctcgaacttctttctggtcagtaaattggtattgttcccaactgtctgtactgaacccttatctggtagtatcacaattttctttctcccaaacagaaagttgtacgtgttggtatatccagcatgcagtgagtgcctgtcaaactgccacggcctccctaatagtatatgacacgcatctatctctactacatcacataagacctgatccttgtaggtaggtccgatgaagaagctgattctagcacattgagacacttctacgtcattgcctcttttcagccaggctaagttataaggtttgggatgtttctcaatttgcaaacccagcttcttaacgacctcctcagccaccacattctcgcaactaccagaatcaataacaaatttacacaccttccctccaacagtacatgttgattgaaagatattattacgcaaccaatcactgttattctccaaaggagtcaggaaactcctcctcaccaccagtgcctgacccacatcaccaacaacaaactctttctcttctgttgcttcttcttcgccctcaccatcaaatacaggcggtccttcataatcgccattttcctcatcaacaaagagtcccctgcgcggattctttgggcacttagactgcctgtggcctgtgactccgcatccaaaacaacgaataccaaccccaggacgtgttagttgttgagcaggatttgttctaggaggaccaaattgagcaggattaccaggacgtgccacctgctgttgtgggttactagaagaactccctgcaatggaaggactagtagttttcctggactgttgcttctttatctgtactgccctctgatgtgtttcagaaactgttacaggatcaaacatattgagagtatcctgtatttggggatgaagaccacccacgtaccgtaacaccaactactcctccgtctccatcatctcgctcctcgtaatcaacatataaaaatccgtggtatagtcactaaccgttttcccaccttgacgcagattttgcagttgttagtacatggtccgcacataattgtaagacagaaattgtttcttcatatgtttcttcaatttatcccacaatgcaagcttaggtttcctcagcctggatcttgtcaccttagtctgctgccactacgccgttgctcgcccacgaagcctcattgcaatgagaggcacacatttatcggcaggaacctctttaaactccaagacctcctccactacagtcacccaatccaagaattcctctggactcaacccaccatgaaattctggaatatctaccttaaatcctgattcccaacgtcggttgtcctcctgaccacctcttctccagtgaactggcaaatccaatggtttttgaagcggtgcaaacggattctcatcattggaatccctaagctgttggcctacaggcgcaggctgctgcggcaaaatcgcaacgatctaccgtgtcagcaattccacttgttgacatagctgtgcgacttcatcacgtctaggtacctcctctaccgggcatcacgggcttcaggacgtctctttggcggcatggtgaaggaacgatttcggttctgataccaactgacatagcgaaaatattatagggacgatgaacaatcacaaattgagaaaattctcaaggaagattttattgaattcaagaactactgcctctaagggcttacaactgattaaatagaagaaaaacctaggaaaatccagaaaataaaataaaataaaataaaagatatttttttccaaaaatgaaaaatatgagataattactaagatgaaaaatacttatcttcaggatcatcctccaacaacggaatctaaatccgaatttcatggaaagagatattgcaaaaatgaaaattaccataaatagaaaaaacgattaaacgagggcttaaacgatggattttgcccaaaattggccttgcgtcagggccaaaggcgctgagttttactccttggctcgactccaatcaaattagactagcgatttgccaaaaacgagcaaacccaaagtcatcatgaaatcatttgccctttttcccaacttttgccttgtgatggtcccattttgccatgaactctaatcccttatgcacttcatcactatttctactaaaatcatggctttagctctataagctaaacaaaaagaaatttctcctgtggtattcctggttgtagtacaatataaccataagatttgtgataacattgtcagtccataatcccttcacaatatcaagctttcttttcaagatgcttttcaaggttttatttacttctttcacttgtctattagcttaaggataatatggattagaaaaatacctatggatccttaattcttcacatatagatttcaacatttttccttagtattgtgtcccattttctgaaataatcgactatagaattccgagacgacaaataatattcttttagatgaacttacaggtattagttttatgatgttggcgagagcttctgcttcaacccatttagttaagtaacctacttctacaataataaacctcacgttaactctttatttagttaagggtccaacaaactcattacccacttcgcaaaaggcgtagggctattcgcagtaaccaactgacgtgaaggatgttgaggtatagctgtacacctttggcatttcatatttttcgataaaatccacggcatcctttctcatagttcttatagttggccaataatacccatttttcaatgctttctgtaccagggaatgttagccaacatgatctccacacgtcttcatagaattctctcattacatatatcactttcttattacctaaacatcttaacaaagagattgtgtagcttcgcttaatcaggaaaccttctcgtaatacatatctcgctgcctttatacatagttttcttgttgagaaaatcgaggaggttattgacacaatatgaagtatatgatcgcacaaataataacaagattaaaagttaaaaaaataaaattggcagaggaatagaatgttttattgacaatcaatgggaaagaataatacaacttcagcaataatgtttctcctaaattgaatagaagagtcacatatttataggggcatattcaaactctaataataccatgaagatggaaataatataaaaataatgtgagataaagaaaataatatttttccaataaaataacatgaaataaaggaaacaatatttttcaataaaatcacgtgaaaataaggaaataatattttccaaaaaattcaacataatttggatcacaaaatctaataatcttcaccttgacccaaattccagtgcaacaaacgaaattccaaaatttctctatctggagaaataaatctgactataacaaaattaacaaatttctttattcagaacaaaaaacctccacctaaaaaaaaagctctatgcaatcctttttaatgtgttatttcctcttacaatagaagcaacctggttgctgaagttcatcatcgacttacctctccgtcgatcattatgagtaaccagagcttcctcatctcgagatccagctccaacgagatgcttcattttctctttgaaaataaagcatcataaacatcatcaatggtgagtgtgtcacaactgtacagaatcgtgtccttgaacaacgaatatgaagcgagcagtgaggacaacaagatcaaggccaaatccttttcatcacactttacctctaacatttacagatcagcgacgatttccttgaaaacagtcaaatggtcctcccaagatcaccattctgtcatgcgatgagaatatagcctctgcttcagatgcaacttgcttgtcaaactttttgtgtcatgtacagtttcaaccataatccagcagttgtcttcctcttcaatacgttctgaagaatgttgttagaaagataaagatgtatttgtgaaagagccttttgatctcttcgttgagtctcctctgttgtccaagttgtggacattttatcaaaccccaacaacgcatcatccaagtccatttacgccaacattgctctcgtctttacttgccataacgaaaatcttgtattgtaatctaaaagctgaatttcatactttatgactgccatcgataataaaaacctcaaataaaattttcaaccatagctctgataccacttattgggaaaattagggagtttattgacacaatatgatgtgtatgattgcacagataagaacaagattaaagtaaagaaagaaattggtagaggaacaataagagagaagaataaaatcacgtgaagtaaaggaaacaatatttttcaataaaatcacatgaaaataaggaaatgatattttctaaaaaatccaacctaatttgggttacaaaatctaacatttcttgattctttttattctctgaaagggttgcatcgcttaggtaggatataatatcttgaatccatgggttctctcctttggatccataggctctattcctttttttggctgaatgatagatttggtaataatcgtactactatggctttaaataattcagcatcattagtgatgctagcttggacagtgcataagtttatccattttcttctcttggtatttgtggaagttcaaacttactgaaatctcatgtaacctccggcaagtataaggccattgttttgtccttagtggcgaactttccattaacctcattcactacaagttacaaatcattgtttaattagattctttgtgcatacagttctttagctagtcaaaggtctactgacaaagctttatattcctctacattatttgtttctttaaatatgaacctcatcgtaccatctaatttatacccatctggactagttaagattatttcaactccgacaccactttacctgatgaaccatcgataaataatttcaaaatttcttcatgttcagggttcttttaagaatgggaaagtttgaaagttcggcaataaaatctaccaatgcctaagctttaatcgcagattgccttttttagtttatttcgaactgttctaatttcattacccacttcatcaatcatcctgatgcatcgagtttttataatactttagcaaaagttagtcaacacattaatgatatggctttgaaagtgacacgcccctttcctcgtaacactactggacttggaatgtaacgtgattcgatgatagttatcaactaaaggtcggcccaccatcaaggctacaataatatacaaccttttataattttttaatagaatttcggcatcatttcccttataaatagggctaacggacctataattcactatgcacaaatcccagcattattaaaacacaatagggataagagctgtgcttgttgtacactctcgtgtacagcaagggtcacagactcccacatgaaggggacccgccttggtgtggggccccctcttgtgaggaggctataaatgtaaaatcctagcttgactgtacaagcaacttaaccccagggataaaccaaagtctcaacttttactactaaaataacatgaaaggtatatatggatgcaaaaatacatagtgagcctcattgttatctactaagtaacattcaaaaatgaacatgtattccaaaacactgactacgtgctctataaaatgagttatactagtaaactttttagtgtagctttgactctagaatcaaaggctcaactccaaaagatagctagaaacttagttgctacttgataagaaaaatcgtgggaaaatatatgagttggtaactcataaatagaaaaatttgaaaatacaaatactttttcatttatacaattcatcgaaaatagaatttacatcctttaagaattcacagtattacagtatataataataatcaagatgtgagacatccttataatactgaaaattatcatctcatcatcgttatataatcatcaactgaaatatatatattcatctcatcacatcaaatgtactcaaaaatccacaaaaacaagtaccctctgactcaagtatgtaatcttgtcatatgagcgtttactatcccttaggttaatcactcctgacacggacataaaatcccctcagtgagcgaaagcaagtctcaaagacttctcataatcgattttaaaatacagctaaggctgcttggtgtattatatgtacacggtcttgacccctcagtgtagtaattaacacggccaaggcctctcaatgaactaaaaaaaacataatcatggatacttttctggttgatctcaatatcacatacatctcacattccaaatcacaaatacaccatacgatctttgaaattccacatatatcataataaaataaatttctcataataataataatcatataatcgaacacataattgtgcataattacacataatgtaatagtataattaatttatcagtacatgaaaatatttaagttttttccactcaattatgtacaaaaaatcaactcggttggtatgttgtcccaattcctgtatcgctgcttgaaatatgatataatatttagattaaaaattaactattttaataaattctgataattaaatggggataccaaatcctaatcttttttatgcttaagcaattttgtcgattcctttaatcaattaagctattttttcttccttttaacttaattacatagcatattatacttaatttaataattttccttcaatgaaaatgaatttaaactaacaattcgacaaccttaaagtttaagataacttttcaataagtaactttttacttacccttgaatttgaagaattcaagcttaatagtaaaaagcaattattttccaacaacgttggcgcacttgcctattttctgtttcttcttcttcttcttcttcttcttctctctctctctctctctctctctctctctctctctctctctctctctctctctctctctctcttttaaagtagtgcaaaatggatttggacccaaaattggattgatataaaacaaataaatatattgcctagccactgaatgattattttattgttttttcttagcttgacacatttgaaaagagtttttattttagccatttaaagttattttataattttataattttaacttggtatttaaaaaacttaccccgtttaaagaattccatcatcgaaattcaattgattaaatatgaaaaaaccttggatatcgagaacacatttgctcttcactttcccatgtcacttttcctatagcatgattctttcataagattttaactaaaagaataatcttactacacgagacttgttcctttctgtccaatatctgaattggttcttcttcatatataagattttctttcaactctattgattgtgattccaaaacatgagacggatctggaatatacttacgaatcatggaaatatgaaatatatcttgaattttggacaattccgttggcaaagccaatcgataagcaaccagaccaatgcatacaataatctcatatggaacattatatctcggactcaattttctagtttaaaaacctaataatacctctccatggcgataatcataggaaaactctatctccaactgtaaattcaagatttattttacgtctatctacatagttcttcggtctatcttgggctgtatttaactttttttttaattatacttactttctcgacaataatctgaacatattcaggctctaatgacttcatttcgcccactttatccaatatactggagttctgcatttcctatcagacactgtttcaaaaggagtcatttctatgcttgaataataattgttattataagcaaactccttaaaaggaatatgattatcctaattctctttaaactacatagtacacaagcgcgtagcatgtcttccaaaatctatataattcttttcgattgagcatatgtcgatgcatgaaaagctgtactgaaatgaagtttagtacccatagcttcctacgaactaggtcaaaatttagaagtgaaacgaaaatctccatctaaaacaatagatactagtaccctatataaactgactaccttatcaacatatatttttgacaatttatctagcgaataagtgactttaataggcaaaaatctggcagtcttcatcaatctgtatactataatccatatatcatcatgaccactctgagtacgcggaagctcaaattagaaatccatagtgatgtgctctcatttccactcaagaataggcaatgtttgtaataatcctgctgcttctgacgatctagttttatttactggcgaatgagaaatctagatacatactcagctatttctctcttcattccatgacatcaatagtgttctttaagtctacgatacacttagtactacttggatgcatttcataagctaaactatatgccttttctagaatccctttcttcgattttgaatcatctaggaacacataatctgctttcggtaactaaagctccgtcatctcgaatagtataatttgtatgcttatccttattaacttcttctttcaatttgctcaacattagatcttgagtttgaacttttctaactgtatcaatcaaactagacctcactaggaaattggcaaacaatgctcctataccattaactgacagttgaacatgtgaaactttgaactcaccaaacaaggaaatacgtactacattagtttgtgtcatagaactagatgtctttccactgagagcacaagcaattacattggccttccttggatgataatcaatattgcaatcataatcttttaccaactataactatcttctttgcctcaagttcaactagaaggtccaaaaatagctaaccaagaggggatgaattggtaatttaacaactttttcaaaaataatcgcaatttcaaacaaataataaataaattaactacataagtaaataagtaaaagtgaagagaatgcacaagccatgcgattatggaggttagatccaatcaacgatctacgtctcccattaccaaactctctgtcatgagcaaagccatttttattattgttgattgacttatggtgcaatccaacccttacaaccggtgacttacaaccaaggatcacagatccttttacaatgttgaaattttcgggacttcaacacgacctacaaccaaacaagaaaaagctattacaaggaaaagcttctctcttaataaatgatatgatcaattaagtctcaagagagagataggctaacacttcaataaatagcaataagtatagctcaagtgttagttgttaaaaaatttgatgagataaaagattttcacaaatttggtcactcaaaaagtttttcaaaaaataaatgttttgatttcctagagatttaaacaatgtagttgagattaataaatgctcaaaagaaggttgttgcaaatggaaagagaaatagtatttatggcactcaaatgggcaaaaaatctgtccaaacagacatgtgatcgggagatttagttgggatccagacgagttaaaaactagccatttaagttagaggcaaaacggtaaaaaacaatgactgttggacgtctggacgttcggttgggcggaaatgcccccgtacgtttttccttcatgatgaatttgatcaatgtagtttcttaaaggactttctcacttatgttgtaaagataagtattttagtaaaaatttgatcgtcaagttgaaatacttgccttttttaaaatttaatttttatacatatatcttttgtcacatgaatttttcctcgtgcataaaaacttttttgtgctgtaatcgatgctaagaattgaagtttttacctttacatataagttcaaagcatctacatctattgttttgatgtttgatgatcgatcttttctacaggatgattttttacgtgaaggctcaattttcgtctctacgtttgtcaattgccaattttgtttccatgttgatcttcaaacgtcaatttcatttgtattaaatatgcacgtttcttgatcttcattttcgtgtcttcatttttgtcaattttgcaataatcaccatcaacaatcaaattcaatttgtgagaaataaatgcaatttgtttacgataatcaaaacgagaagtcaaccatttaggtcaacaatttctccctttttgattatgacaaacaagatgatttgcaatataaacattaaacaaattgatgaggcaaggaacataaattctgaattttacatatatatgttcccctattcttttacatatattccccctgtcaacatgcatataaaattttataagttcaacataagttcctccttacaatgttcctctttccccctattttacataattatctacctatcttctcccttttggtaaaaacaaaaagaagtaataccatatggtaataatattttcatatcgtgcatggaaataaattgaagaacaaaagttatagtgcaaaaacatataacaaatggaaacacgacaccttaaaaataaactaaggtgctgaaagcggtgtgagtgggaaagcgagcatagaagtcagcaaaaaatgcattctgttgtgcctgcatcttagcctgtcggtcttggattgtggtctgctgaaggtgagagaatcgatgcgcccatgaaggagattatactattccacgatgaatgtaaaatggcctcttgaaggacgagttgcattggagtcgggaatgtcagaaccggaagttgtggctttaggatcgtcttcgggctcatcttgggcttcctcttcgaaagctaaagtggaagaaccggagccagggttgaatcctttcgtgtgcgccacccattacccgtgttctttgactatcttcattcatttaagggtttggatgttgatagtatctgtatggtgtaatttaacaaaggtttcaccatcgagagagacgtgaaaatgtttaaaaaattttgtgagaagcatcccgtgaggcaaagtttttacatgttgtgaagaatgcacaagtttcataagtcccaatgcaatggtaggaaagtcaagttagcgcccgtccaaaagtatatgtaaaataaaaagatcgaagtgattaacttcatcctgatggccctttcggggaaaaattacatgggtgataatattttgtaaaaactttgcatggaagaattaattaattagcacttaattttgtaatattctcaaggtccttcccggtgacttggcaacatgctttggaaggatcatagccttccaaggtaggtggaattttgtgtagacaaatttcctagtcacatagctcgagttcgagaatatcacaaattaatgcttttgttatcataatgcgtacatttttaatcatgtaatcatcccattctttcaaaatattcttcaatatgaaaaatggaagcttctatagtaaatttagtgaaatcaacgttcttaccaataagaatgggtgaatttttgaagagattcagtagcacctcgggctccaaatctatttttcgtcggaagagagaggaggagatcgtctcacgatttgtttaagtctttttctagccctttttcctacttgagaccccaacatattagaatttgatgaagtatttgagaatggcaagctagggcacgatattagagcaaaaaggaaggaattttgaatgaaagttaccaaattttgggattttgagaactttagtcttgtgggtttttagattagatgggagattggtgtttttacaaaaaaaaaaatttttagtaatttctagtggatttagggagaaaaagtggtgaaaatcgatgagaaatgaatcaagtagccatttttatatattttgactcgtgcatatccgaacgctcggttcaccatccagacgtcgtgattgacagacttgaaatcttctatcaaatcggacaatgaagtctggacatccgaatgagtctttgacttgtccggatcctttctctaggtgaaattaattaaccacatcattttcatcaatgagtcataaacctcttcaaaaatgtgaaaatcgattgtgcattagagtttggtgaagatgtcagccaattgttctttgttttatgaattctaacatagtatctccctttgtacatgatttctaagaaaacagcgtcgaattttaatgcgcttagttcgagagtgtaaaacgagatttttaaacaaattgatggcactggtgttatcacacattataggtacgtgattataagataggtgataatcactaagggtttgtttcatccagagtacttgtacacaactacttgcggccgaaatatattcagcctcgacagtagaaaatgcaatggaattttatttcttgctagaccaagacacaagtgcaaagcctaaaaagtgacaatttccactagtgctcttacgatcagtagtgcatccaatcaatcaacatctgagtaacttaataagtcaatgtgacttccagtgggataccaaagtcctaaggttctaattctactaagatatcgaaaatttcttttctcgaaaagtgaatgtaactccttaggatttgattgaaatctagcacataaacatatactaaacattatattgggtctattagcagttaagtgaagaaggaatctgatcataccttgatattttgtgatgtcgactggagtaacttgctcatcttcgtcaagctttaaaattgtactcattgggggtgttcattggctttagatcatccatatcgaatatgttaagcatgcctaatatgtatttattttgatttatgaaaattctgtatttgtttgtttaatttgaaggtcgaggaagaatttcatctctcccatgatgctcatttcaaatttcttactcatgcattttgaaaattcgtcaaaagaaaggatatttgttacaccaaaaatagtatcatcaacataaatttgaacaacaagcatatctctcttatgagttttgacaaaaagtgcctattgagaaaccatttgaaagtaaaaatttgctcaaacattcataccaagctcttagaacttgcttcaaaccgtaaagagcttttctaagtttacaaacatgatctggatacttgtgatctttaaaatcaggaggtagctcaacaaaaacttcctctttaataaatccgttaaaaaatgcacttttaatatccatttgataaagtgtaaaacctttatagcatgcaaaggtaagaagcatacagatggattctaatttagctatcggtgcaaatgtttttttcaaaattgataccttcttcttgattataatattgggcactaatctagccttattacacacaattattctattttcatctagtttgtttccaaaaacccattttcccaactacggtttggttgtttggtctaatgactaaatcccaaacatgatttctttcaaattgatttagttcctcttgcatcgctagaatccaaaaacttattaaactcagctttttgaaatttttaggtttgatttgagacatgaatgcacagctactgagatgatttttgaatgaggttttagtagtgatacctttggatggatcacctatcattagctctttgggattagatggaaaaaacttccattttttggtagtgggagatcactttgagcttcggttgatttttcaacacattcttgaacgtagggctcctcattttgtttttcgttgggagtttccttatgttgttcttaaatattcatttgttcgaatggagcttccaaacctacattgtctccaataactttctcgcaatcaagagagttagtctcatcaaatataacatgtaatgattcgtcaacaactagagttcatttgttaaatactctacaaactttgctagtcaatgaatatcctatgaaaattctaatatcggattttgaatcgaaattttccaaattatcttctgtgtttgaaataaaacacttgcatccgaaaaaatttataataactaatattgggaattctatttttctaaagctcataaggagttttagttttctttctacttactaagactccattgacaatgtagcaagcgatactgacggcttcggaagaaaaatacttcggtaagttgttttcatttagtatggtcctagccatttcttgcaatgtaagattctttctttccactatatcattttgttgaggagttctaatagccaagaaattatgttcatatccattttcattgcaaaaatcatcaaaatcgacattatcaaattctccaccatggtcatttctaatagttgtaaatcttgaagtgtttaaaaactttttcataagagctgagaaattatgttcataccctttttcattttcaactttcttacaaaagtgtttaaaaacttttaaggcttcatcctttaaacttaaaaacatgacccaagcaaatcttgaaaaatcattgatgataacaaaggagtaatgtttaccgcctaagatagctgttctagatggtcaaaaaagattcatgtggagaagttgtaatggttttgtagttgaagagtaaagtttggacttgaaagaattttttacttattttccgaattgacacgcatcacaaattttatattttttaaatttcaaatttggcaatcctttcacaaaacagtttttggaattttggaaataagatccacgctaacatgacctgatctcctatgccacagccatgttttatctttcaagctaagtaaacaatttttattattttcaaattcaatatttatgatataaacatctttgcattggcttcctatgaaaattacctctttcgatgtagcccttatcacataattgattaatactaaataaattatgtttgagtttatcaactaataaaacattttcaatcgagggagatgagtgattaccaatgtttccaatgccgataatttttcctttagcgttgtctttgaatgtgacatgacctccatccttccttttgaagtttaatagtaacgtttgatctctggtcatgtgtttcgaacattcgttatccaagaacttcacttcttgttttcttcggtacatcgtcttccatcgccatgaagcacatgtttggaatttcatcttggctacattttcattgttgtcctcattgtcactatcatcccacgtagcttggagtgcctttttcttgatataattctttttgtttgggcacttgattctattgtgaaccgacttgtcataatcatagcaaatgattttcttacatctttcttcgcctttttccttcttttgaaatattcaattattatgaagacctctcatttttttacaagaatgactaaatcatcgagctcttcattgctcaagttgtcatgtgtagttccttcctcaattgccgactttaaggcaatttaatgcttagactcctttgattcttcctcactttttcttgattttctccttaacctcggcatggttgagttataggtcattaatgttccatatagatcttccaaaggatacgtattaatatccttagtatcctctatcaacattctcaataaactccattcttttgataacgacgtaagcatttccctaacaagttcaccgttagtaaatttatgatcaaaacctttaaggctgtttacactatcagtaaaatgagtaatcatatcaacaatgggttcatcttgttttatgaaaaaaatttcaaattctttaactaacaagttgatttttgtttctttaactttgctagtgccaacatgagtaacttcaagtgcatgccaaatatcatatatggattcacacgtgctaatctaagtaaatacatttttatctaatgcacaataaagtaaattcttagcccttgcattcaaagattattttttcttatcttcttcatcatattcttccttgggcttaggaataattaggtcggattggccatctatgttaatggtcttagtaggtttataaggataatattcaactacttcccaaatgttgtaatctatatattgaatgtcaatcatcctagccttccaataattataatgtactccatgaaagacaagtgattggtttgtggaatgtcccttgagagtttgaagagtgggtagccattgctcaagattgtgaaatcttaaagagaattaagaccttgctctgataccaattgaaggcccaagaacagctaaccaatagaggggtgaattggttatttaacaactttttcaaaaataattgcaatctcaaataaaaaaaatttaattgcacaagtaaaataagtaaaaggaagagaatgcgcaaacgatggaattatggagatttgatctaattaacgatctatgtccaacgttaccaagctctccatcacgagcaatgcctttttcactattgttgattgacttatggcgcaatccaacccttacaacacttccagtaacttacaaccaatgagcaccgatcctttacaacgatgaaatttttgggacttcaacataacccacaatcaaacaaaagaaagatattacaactaaaagcttctctcttaataaatgatatgatcaattaaatgtcaagagaaaggtaggctaacacttcactaaatagcaatgagtatagttcaagtgttatttgttgaaaaactttgatgagataaaaaatattttcacaaatttgatcactcaaattttttttcaagaaataaatgttttgatctactaaagattgaaatagagtagttgagattaatgaaagacttactcaaatgctcaaaagaaggttgttgcaaatgaggaaaagaagtagtattttagcacgcaggtgaggaaaaaaaccatccatccatacgcgtgatcctaacatccagttggggtccgaatgggttaaactagccgtttgagtagaggcagaatggtaaaaacagtgaccgttggacgtctagacatccagttggacagaaatgcccctggacgttttttcttcatgatgaatttgatcaatgtagtttctcgaaggactttttcacttatgttgtaaagataagtattttgtaaatatttgattgttgagtcgaaatacttaccctttttaaaattcagtttttatgcaaatatcttttgtaacaggaattcgttctcgtgcataaaaattctattgagctataatcaatgctaagaattgaagtgttttatctttatatataagttcaaagcatctacatctaatgtcttgaagtttgatgatcgatcttttctctcagatgatttttgatgtgacggctcgatttctatcactacattcgtcaatcgccaaatttgtttccatgttgatcttcaaacgccaatgtgcacgtttcttgatcttgattttcgtttcttcatttttgtcgattttacaataatcactatcaatacttgaattcaatttgttagaaataaacgcaatttatttgtgataatcaaaatgagaagtcaaccatttaagtcaacgcagctctttctgatcgaaaatatactttaaactcttatgatctatacatatctaacatctcttgtcatacaagtaatgtctccaaattttcaaggctagaacatttgtggctaactctaagtcatgtataggataactcaattcatatttcttcgactgtctgaaagtatatgctataatctatccaattctgcattaaaacacaatcaagaccctgatgtgaagtatcactatatataacaaactcttcaatggggatgtaagggtaagaacaggagtcgaaattaattaatttttcaattctaaggaactattttcacaatcttcattccaaacaaatttaacattctttctagtcaaattggtcaatggtagagcaattttaggaaacccctttacaaaacgacagtaataacctactaagccaagaaaatttcgtacttctgtcacatgtaggcctttctcatttcactattttttcagttttctgcaggtcaacataaatttcctctgttggtataacatatcccaaaaacacaaatctatcatgccaaaattcacatttattgaatttagcatacaactgcttaccacgttcagtctgtaaaataattcttagatgcttgtgtgctcatcatgatcttaagagtacactaatatatcatcatacaatcacaaatttgtctaaataagggcaaaacactctattcatcatatccataaatgttgttggtgcattagtcaacctaaacgacatcacgagaacacataatgaccatatattgttctgaaagcagtcttccactcaccgctatttctgattttaagttgatgatatccagaatgaaaatcaatctttgaaaatactgcagcgccacgaagttgatcaagcatatcatcaatacatggcaagtgatatttattacaaattgtcactttgttcaactatctataatctatacacactcatacggtgccatctttcttcttcacaaacaaaactaatactttctatggagatacactaggttggataaaagcccttgtctacaaactcttgcacctgaaatttcagctctttcaattctgttgaagccattctataaggtgcccgtgaaataggtatagttcctgaaattagatctaccgtgaaataggtatagttcctgaaattagatcaagtagatcattaatacgtagcaagggatattttattttgctaacatctgtatcaatcacatgagccaataagcatgacaacccttattgagtaatcttccagcatcaatagcggatatcgtgcaagatggtaaatttctatactgtccattgaatataataatgtcaggatgtcctagttgtctaaacacaacctcatttcgaaaataattaaactaaaactcgatttataactaaaacgttcattcctgaataacatcaaaatcatgtatgccaaaaggcatcaaattcactttctactcgtgctcctttaccttagtcgtacaatctcaatatatactctctggtaatagtgattcacctactagcgtacccactaccaaacaactgcctatggtttatagcttttggtttgcatataacgcaagtgcaaatgaaataaaagaatgtgtagatccaggatcaatcaaaacacaagtatctctacaaaaaatagaaaacatacctataataacatctggtgactcctttgctgcctttctgagtcataacaaaaactttgccttggatctttgatcgcccttcctggccttttgctttagtaccactatcacttgcaatattggactagatcatattgtttgtacctactttgttagctgagacatcttcctgtatctgattctatcttttattaacaccacttgctgggaagatattatttgggacataacactttccagtaataaaactggacaaattattccaatgtgttcatcttggccacaatgataacagacaccatcccctttgaactttgaactttgaacatgtaccaagatgaggtctttcacataaccgacaatagggaaatctaatactagtagaactctcattttgtctcgaagtaaataatctttggggaaaaccctgagcatgagtatggctagccaatggctgctgcacagtactgtgactaagctaggaccctaacttccccgtgacctaggctagaaatagcctgaactagacacattagttcgaaatcctctactgtacctctgtggtcgtctatagttagaactacccactaatgattgactactgcttatttagaacattatttgttctctactaattggttaaccaaaggtgctcttttctagtctcaaagccaatttaaccaatttattaaatgcattccaacctgcgactatcactatggacctgatctattctcttaacttatttttaaattgtctatatttatcaatttcattgctaacaaaacttgagcatactttgaaagttcaatgaatttaacctaatattctgcaacagccacctgcctttgtattaaattcaaaaattcttcttgctttgcatctttatatgaacaacagtaataggcatcataaaagatacatctgaaatctgcccaagtgacgatctcgatatgtactctgtactaactgccattaatcatatgcatcctcatctaataaaaaattggcaagatgcatctttcgatcatctaggcaacccataacatcaaatatcctttctatcttgatcatccatgcctgagtaactacagattgactatgcctatgaaaacttcagcccctgattttgtagccctctcaatattgaaatctctttatgtattatgcatagcagtagcaattctttcaacagccataggataattccaaaccacatttcactgttcccgttgatcaggaggttggtgaaccaattcatctactctctcgaactctataagtttatctctactaggaacaatgtaagactggggcaacatatcttggagccttcgagttctgccaccacgagacatgactcaactacaattatgcacgatatgctaaatatcagaatgcatgtatgtacaatgcaagtcaatggactctaaagcatgctctgattccaaactaacaccccccgctccatgtaacgctattggacccaaaacgtaaagcgtgtcgatgatggatactaactaaaggtcgtacccacatcaaggaaactacgatatgcaactttttaaaaaatttaaatagaatttcgacattattttccctgcaaataggacttgtaattcactatgcacaaatcctaatagtaatacaatacaatagggataaaaaaaaattctcagctttactactaaaataaagtgaaaggtacatatggatgcaaaaataaatagtgagcctcatagctatctactaagttatatccaaaaataaacttgtatcccaaaacactgattacatgctctataaaatgggtcatactagtaaactttgtcgtgtggctttgactccaaaatcaaaggctcaactcaaaatatgctcagaaatttgactgttacctgataagaaagatagtgcaataatatatgagttgatagctcagtcagtgaagagttcgaaaatacacttacttttcatttatacattttattgaaaatcgaatttacatcctttaacagttcacaatgtaatagcatataataataattaagatatgagacatccttataatactgaaaaatattgactgggggggtctcattaaaaatttcatgcaaagtgggcggtattttttctatgggtagattgtgtgatcgcatgaccacaataccttacgacgaactgccagggaatcttttatgtgatcgcaggctatagtgtcgtgcgatcacatggcaatacgggtcgggattcttggcgcgtgctagacttctcttgaatgattgaatatgcgataaactgatttgggtaaacttctttagattaaaatgaggttagaaaatcattccattgatagttggatcaaaataaaaaaacaatcaaatttttcctcttcttgacacccatatgcgtacatgtgtatatgacttgcccgctcatgtatatgccactttaggctcagttttattgcaagaaggccttgaacacacgtggaaatttttactatacacgtgcatggttatgtcctagagagtttatcaatatttttgtcatatttttctctcccaatgattcgttcaaggagattcaaagtatattgaaaagccaacttataagctagaattcttcttgagaattattttttcaattagaactttgactataaggaaaatgggtcttagtctaagactggaaatctcaagcataacttgttcgactaaaaattgatgtgtgagaatattttgattatattttacccatttgacttcttttctcatccaattgaccctaacactctcaaatcttcgttgtgaggtcctataagacttttgagtatttgtacttcaatccctgggctttggatctcttgcaattgagccatttttcattcttttttcccaattccaccattttgtcaatctttatctaacatgcataatataaataaaattaagacatagttcattaaatatctaagaaatactctaatttaaaggtctaaacaagtgcacaaaatacactaattagcatcatcgccaaattgaagaaatgggcttagttctaatggcacgttataatcttccaacactggagacatttttcttacatcgacctatatcataaatcatttgcccactaaaagtctagaaagtaaatcgccttttgaaataatcgttaaacaaaaactaaattataggttcacacacatgtttgggtgtgcccgctagccaaacttacgagcctatgttgtcattttagtttcgcaagtgtacgaaccgtagcaagtaatatggacctaagagtctagattatcaatcccacaaagactattttctagaacttaattcaattttttttaactactatttgatgaattcaaattaaaagatgtaggacttaaattttaatctaaattctagaaaataaaggatgcacacacaattatttggaaaatcaaataataaatggatgttggggcaaaataacttcacctattgatcatcttaacatctcaaattaagactaaattctaatgtagtgtttggccgaattttcctattgtattcaatttaccctctcgagttctcattgaacctattcaactaattaaatttcatatctctatgaaaattcaactaagttaaacgagttctttgttcaaaaaatcaattatgaccgcaataattggcatagatatctctactcattatactaatttaccagattttactacatagtctaaatcctaaactaatatctctattcgtaaaggatctaggaaactcatcaaaccattgatcaagtaatttaatgtattcaattcatagtaaaaatcaacacatggaagaattaaaaaccaagaatcttaataagaaaatataaaagatctcaaatggttatattattcgccctagcactggatttagctacgtgtaataaaagaagaaaaacaacaaattgtcttagaatacatcactagattttgtattaaagatgtagaagaaaaagtagatcttgcaccaagaatttctttctcttccaattgataccttacgcgatgaatttgtcgatgttttctccctttgaatttctccttttctcataagatgtgtttctttacctctcaatgtgtgtagaatatcagatttttaggtcaaaaagaagctttttttcgttctgggttgtttaggtatatatatgatgtcaaaatattgtttccatgtagaatttcatcagaataagaaaactggcccgtcacagaaaatttggcccttgctcctgcgccatatatttcattgcacgcactagtcaaagattttgctctcgggttggagaaaaagaggtggtgcgcgcacgccatttcttgcccccgcgcgcgccgtgttacaagcacgttcgtgtatagctcttggtaaattgatcataactttatcatctgaactctgattgaggtgattcaaagtgtgttggaaagatgactcaaagagctacaattcttcttgaatatatattttccaattcgattgtttgctactcaaaaatggatctcaaatggagacttaaaatctagaacacaacttcttcgactggaaattgatttgtgaaattgcttcaactctatttcactcatttgacctccaattgcatccaactgatgtcatatgatctccaatcatcgttttgtgatttgaatcaactattggatatttacactttggtccccaaactttgtaattcctttgttttcccatgtttttgttcctttcttccaaatccaccaattttcattgatttcaacctaacaaacataattaaaacgaaattagtctatcactcattcaaatcactaacaaataccctaatttaatggcctaaatatgtgtataaaatacacttatcaaacacctccaaacttgaatatttgtttgtcctcaaacaaaagtataacctaaataataacaaacgcacaatcatgaaaaaaaaaagtaataatatttggttgaacaatctagcctctcatatcaggattcaagatttaagtattaatttcacaaacatgcttcaaagttataaaaccaaactaatattcactcttccagtgcaaaatcgacgtgtgtgtgcgaagaatcaagcaatcaaccatgactgcacaagttgtttcaactcccaaccctctgtagtcaaataaatccttacatttctcgtttgattcatccacccccaaacttattcttttttactcttttctcagcttgtgatcgaaggttgaatttttcattactatcatcacctctctagtttaggtgaacttcactagttacaagtcaatacttcaatgaacaggaattctccaattatttgattgcttcgaccttcaaaactcaactaggctaatatccttcatcaaagatcaaatttccttaaataagtgttggggcttaaccaaggtatttcgtgcctttgctcttttcatgcacctacttttttctggtttttcataagttattttattttaatttttgagcaccaaattttttttttttatttattttttatttttttattttttggcattctccccattaaactttctagataatccctatagtaggcatgactcccaaaatagattattatagggcactaagtagggatgtcaaccggctcaatggcttgggtggctcgaagctcggatggagcaagcctaggctcgggccaagccccattttggggcgttcactggagctcgagctcgcccgtgtggctctccgagccacatgggccaaaatggcctgtgacaaggcccgcccgaaattcaaagttcaaagttcaaaaaaaattaataataataataataataatatatttgaaaaaggtcaagctgccattacaggcagctttatagctgtctgtaacggtagcatctactgccttaaggcagcctagttgactgataaaaaaatacgttaaattgtatgattttctactgtattttataattcaatttacgaggttcatatttgaaactcaatttcaaatttcaaatttcaatttcaaatttggaggtaaaattgttttttttttttttgctataagtacgaagtaaatttttaagtttcaaatcaatttgtctcaatcgattttaacttgcagtattatagattcaagtttcaactccaatttctttgctctcaatctcatattcaatttctttcactctcatatagtcatattctaatattctatattttatactatactagttatagatgaattttactagtgatgagtttaatcaatttaagggtagcttgagtactccatccggttacgacgatgcatctcaaaatgttccaattgatttggagaataatgatgaggaagaagtacttgagattaaaaggtcgaaaaaagagtcctcggattgttggcaacatatgatacgtaaaaaagttggtgttcaaaatggagtggatatttggaaagcatattgaaattgatgtggcaaagaacttagttggaagcccagatcgagcacaacacatttgaataaacacatattaaggagttgcaaagcgaaaccagtcgatctcgactcgaaacagaccgaactactgtttggcggttcttgttctactctttccacctttgtatattcacaggaaagatttcataaaggaatggctacatacgtagctgcaatagagatgccgcttacgatgatagactcagtacattttacccgactcgtgctgaaatatttccaacccaggtattcttcttattgtagaaatactcttcgttcatatactataaaagtatacaacaaaagaaaacaagttgctattgaaagtctaaaaacttttaatagtgttacatcatttacatttgatttttgaaccggtggtaatagaaaaggttatattgctgctatggctcattatattgatcacctgtgacttttacataaaagaattattgcatttagatgagtaaaatatcctcataatgccactaacatatatatggttttaaaagatatcatacaggaatatggtattcaagatataattcgaagttttacttttgataatgctagtgtgaacaaaggtgttatcgaaagatttattaatgatcttaacccttcatttggaactttattttttcatcaacattgtatatgtcatattatcaatttaattgtaaatctggattagaacatataagttctcctttagataaaattagacaagcaataaattttatcactgtgtcaccagcaagaaaacaagcatttaatagtttgtgtgcagagtatagcttacaggagaaatcatttgccactgatataacacatagatagaactctacatatcttatgttaaacttatgtggaaattatgataaagtgatttcattatattataatggtaggcatacatacgacccgaacataatttagaagattgtgaatggtctcttaaatttcacgcggaaaaaaatttaaaatctgttttcaatgctacaaaggaatgtagcggagtttattaccctatatcttcacttgttttacaacatttttctacatttcacaaatatttcataaatatagaaatttgccattttttgacttagtttgctctatagagttaaaatttcgtaaatattgggaagaattgcgctttttatttattttagcttcactaatggaccatcgacttaatttgaatagtagaatagccactgtaaagggatttcaaatttcatgaatgtgggattatcacatgtgaatataaaatctacgttatctgaaatgtataattattatgctgataaagaaagctagtgtagttctacttcccaaagttcttcttcaagaaatatttcaacaaatttagataatttatgaaatttttgggaaagcaatacaagtgtttcctcatttagttctagttcatcaatgtctagagcgataaatgtcggtggtacatatatgtgcgtggacattcgcaatgtgttacctaaaaagaattacaggaatttaatcttctaaattggtggaggtgtaatgaaagacagtgtccaattgtatcaaaaattgcacgtgatctactgacaactccggtgtctacagtagcatcggaggctgtattcaatttaggtggtcgaattttatcacacgagcgttcaagactaaaataagatatattggaggctttaatatgcttgaaggattgagaatgtgcagaattacatgttcaagaacatgttgacagtatactagttgaagagttgcagcagatccaaatataaaatgttgtaagtttttaaaataatttatttcaaaacaatatgtaatttttaaatttattttttttaagaaaaaaattgtacatgaaatattttatttgtgtacaattttaactccgcctacgtcatgtaaccggtcccaagcccgaaaaaaggaggagggttgtaagttgtaatttttatttaatttgtaatgcaatttcataagttgtaatttttatttgatttgtaactcgtataaattatgcaatttttaattttttttaagaaaatgttagattcgtaatcttgtataataaaaaaaatcgagccggcccggcttgactcgacaaggcctgagcctaaagcttgagcagagccttgttttttcggtcgagcttttgctcggctcaaatcagactcaaaaaaagctcgatttaaaaaagctcaagtcgagcacgagcctcgagtttcggctcaactcgttgacatccctagcaccaggttttaaacgcccttacagacttattgaccagagtaaaaaatgcttcgaagagaactttttttttcaaatgcaatttcgtctccattaaactttctaaatgacccctgtagcgagctttaggtcgataactctcaagtcaaacgacttcagggcaccagattttaagatacccttgcagacttaatcacttaagtcaaaaaggcttcagagagaagtttaaatttttcaaatgtatatgtcttgattagtgcaatactccttatcacatacacattcaaacaagccgacctcaaacttaagactttcgtagagttttatcatgttagtctaagacaatccacacataagttttcacacatggaatccacattcacatccgcaacttcctacaactataaaatcacccccaaactatgctaagtttggtctaaggatagataatttaatatggcttagttaaagcatctatgtccaactagatcaacctatcaaaagcaagaaagaactcatttaatcacaatgtcaaactcaattctagcgcacttgtaatatcaaattttgtaaggtcgagcttcaattagtctagcatgcatcctatccaccgttcacaaatcaacaccaaatctcaaattaaatcatcatcgtttgccagactatctaacccacacaagcacaaactaaataaaagagatttttttttaattctttaaatttttcaatttttttcttttatttaaacaaacacacaaaaacataaaaaatacgaaaaacaaaaatttaaagttattttacccccaaacttaaaattgccattgttctcaatgtcatatagcataatataaacacaaaaggggtagggaagaaaaggaagaaggtactccccaaatttttccattgaatgtatgaggcactgtgtgtcacgactggaaaatcttcttcatcgtgctttcccttgggcctttgagtgttacacgacatcatgttcctaaaaaggaaaatttcacaaataaataaatggaatacgggttacttaactcaagcaatcaaaataagtaacaataaattcaagtgcttacgggcagaagggatacgggtgatgactcctaaataaactaataaataaacttaactatcctataacttgaaaacaaaataaataaaggaaaaaaagcttgggttgcctcccaagaagcacttcttttaagtcattagctggactttgtactgctattattctggaacagcaagttagagactctctttagtggtgggaaactcctccacgtaatgtttgatgcgttgtccattaaccttgaaagttccctttgtttagtggtataatttaacatagggaaacacctgggagacagtgaaagggctggaccatgtagatttcaattttcctgggaagagcttaagtctggagttgtataaaaggacttgatctcctactctgaaaattcgttgcttgatgtttttgtcatgccattgcttcgtcctttccttgtagatggatgcattctcatatgcttctcttctgaattcttccaattcatgtagctgcagtattcttgtttctccagccttctctagatccatgtttaactacttcagtgcctagtatgctttatgttcaaactcgactagtaggtggcatgttttcccaaagactattcgatatggtgacattctaatgggcatcttatacgctgtgcgataggcccacaaggcatcatctaatactttggaccaatcttttcgagatgaattcacagtaaattctagaattcttttcaactgtcgattagaagttttaacctgtccacttgtttgaggatgatatggtatggctattcgatgttgtaccccatatttgtgcagcactgcctggaataatcgattacgaaaatgagttccattatcacttataatggccctgggtgatccgtggtggttaacgatttctttctttatgaagtctaccactatccttacatcatttgtagacaatgctttggcttccacccatttggaggcgtagtccactgccattagaatataccagttgttgtaagatgatggaaaaggagccataaaatcagtcccccagacatcaaatattttcgcctccaaaatgttgttaagtggcatctcgtgatgagctgatatattacctgttctctgacacttatcacatgatctgtggaaaatgtggcaatgcttcaacaatgtaggccaaaagaaaccacattgaagcacctttgccgctattttagttggatcaaagtgtccttcataagccgaagcatgaacttgtgaaaggatcgattttatctcatcctttggcacacatatccggatactctagtctattcttctcctatataaatttgaattatcgcaatgatagaattttgcttcatgaagcagatttttcttctgtgataggtgagatctggatccttatagtcactagccaagtaattaacaatatcagcataccacagggccttttctacccgcaatagctgctcatctgggaaaacctcattgatatccatatcatctgaatcctgcagttgctctagccttgataagtgattcgttacctaattttctatacccttttttatggcgaatttcaatgtcaaactcttgcagtaacagaacccatcgaatcggcctaggtttagcatttttcttctcaaacagatatttcaaggttgcatgatcagtgcaggctatcacttttgaaccaatcagataggaacgaaatttgtcgaaggcaaagaccatcgctagcatctctttttccgttgttgcatagctgatctgaacatccatcaaggttttgctggcatagtagatggcatgtaacagttttcccttgcgttcaccaagtaccgctcccactgcaaactcactaaattacacataagttcgaaaggtagatcccaatcaggtgctcctatcacaggtgcagaagttaaattttctttcaaagtattaaaggcatttaaacactcattagaaaagtgaaatggcacatccttctccagtagattacacaaaggttttgtaatttttgagaaatcttgaatgaaccttctgtaaaaccctgcatgtcttaagaagcttctgatccccttaactaaattaggaggctgcaatttttcgttcacttctatcttggctttgtcaacttcaatgccctttaaggaaatcctatagcctagcactatcccctccttcaccataaagtggtactttttccaattgagcaccaaattcttctcttcacaccattgtaatacaagcaatagtcattccaagcaatcatcaaaataatccccaaacactgagaaatcatccatgaataccttgatatatttttccaccatgttagagaatatagccatcatacactgttgaaaggttgcagatgcgttgcatagaccaaatggcattcttctaaatgcaaatgtaccataggggcatgtgaaagttgtttttttctagtcctctggagtaatggctatctaattgtaccctaaataccgatacagaaagcaataatgagaatgtcctgccaacttctaacatctgatcataaagtgcaatgggaagtgatcctttctggtagcattattcaacttccaataatctatacatactctccatcctgttactaaccgtgttggtatcagctcattgttcttattcttctctacagtaattctatccattttaggcaccacatgtactggactcaccgaagaactattagacatgggatagataatacctgcatctagcaatttcaacacttcttttctcaccacttccttcaaagttggatttaacctgcattatccttctggtgatggctttgacttgttcttcattaaaattttgtacatacacaaagtaggaccgattcctcttatgttggcaattgtccttccaattgcagttttatactccccaagtacttccaatagcttgttctctttctcctttgtcataccatttgcaatgatcactggaagtattgtagattctcccaaatatacataacataggtgtaaaggcaacaactttagttcaagagtaggtgcattttccactaagggtaccagggtaaagggttatcaccaagagattcatactgtcaatttctccttcctattggttgttcgaccaagttgacatcacctttagtattttctacacttgttgcttccaattgtgtattttctgcttcacaaaaaattgtttgatgctctgtctcaaatgtatctgccaccaactcttcaagaacatctatttggaaacaggtgtttgaagccagtggatgtttcatcttcttgaacatgttgaatatgacttgctcattgtctacccgaagaatcatctttccatcgtaaacatcaatcaacactctttcggtagcaagaagggtcttcccaagattggagggatgtttgaatcctcctccatgtccaaaatgatgaagtcaatcgaaaaaatgaatttatcaactttgactagcacatcttcaataatccccttcgatcgtttgatctatctgttagccagttgcaaaaagatggttgtaggttttgctttccctaatccaagaaacctgtaaatagaaagagacgtcaaattaacactggcacctaaatcgcataaagaatgttcaaaataattagaacaaattgtgcaaagtatcgtgaaactccctgtatcttttagtttagggagtagcttcttcatagaattgcactgcactcctcgttcaggcagataggctcatgttcttccaacttccattgttagacaagatatctttcaagaattttgcatagctaagcacttgggctattgtatctgcaaacgggatatttatgtgcagtttcttgaaaatctctacaaacttggaaaactgcttgtccagcttctttatctgtaacctttaaggaaagggaattggtgacacataagctttcaaggggctcggtgctctcactgtggatgtttctttcctttcatcttcctcgtaagttagtggttcaaactctacttctttctcagcctctttaaccattacttctttatcttttctctttggtctcttcacatgtatctctgaaagttgtaccccacatctggttgtaatagcttgcacttactcttttggattgatcattttgttgctcggcaatgtcccttatgtgcgttctgcaagctgttgagctatctgaccaatttgtatttttagcttcttgatggatacttgttgattctgaaagttagtgtcaatctgttgaaacaccttgtctatcttctgcatgtactagttgaacatctccccaaacttggtttttctcctgttaggcattgtttgaactgttcctttgctgattatccgaccatatgaagtttgggtgttgtctctatcctgggttgtatgtttaagcaaatggattaaaattttgacaaccattctgaatgaagttgactattcctctggaaatgccatagatgagcagttttcgcatgatggatcggctatcactgcatgtgcttcatttgtttgtgacttcaccaacaactctacatattttgttaatgctgctatttgggtgttggtagatattgtgctatttaattcatatattatcgctgcttttggaggcaccactctttctgatgaaaacataaagtgagtagtagcgaccaactcaagtagatccatacattgttgcactgatttccctatgatcgatccacctgtagaggaatctacttgagatttggacagtggtgaaagtcccgtgtagaaatattgcacttgattttcgatagtaatcccatgatttggacacttccttatcaactccttaaatctgtttcgtgcctcgtgatagctctccccatctttctgtttgaatttcagtctaatttttgctactttagctggttgaaagatttgttggaaaatttcatggttagtttccatcaggttcggcatccggccattctaatgctgcatctcttagcatgtaaggaaataatcgcaggttgatagtgtcctcattaaccctaggagcatgactactccggcaattcctaagaaacctggagatatgtgtttggattctcatgagatagcctgtagaattgtagagtgttgctgatcaaattaatccagtcagctcatatttggttgtttactccaaaatctggatgcacaatacttgatcgtgcagatgctgctataggcgttagaacattgacactggcaagtccccttcatttacttcttttttctcttgctgttgatctctcacagccatttgtccaattggctgtatagggataaagtagtttagattgtcagccatttcatgttgttgtttttgtttgtgctccatgtgtcttcgtctgaaggtacgttctattttcgaatcaaacaattcaagatcgtcaccttggacgcgaagcatacaacgaacacgattttctgtaaataaaagaaaataaacaaatcaaataatggttaaaaataaaaatacattaagactaaaagttatagtcccccgacaacggtgccaaaaacttgttatcaaatttagattcgcaagtgtacgaaccgtagcaaataatagtggacctaagagtacgggtcatcaatcccaaaaggactattttctggcacttaattcaatttttctttaactactatttgatgaaaacaaattaaacgttgtaggatttgagttctaatctaaattctagaaaataaaaggatgcacacacaattgtttggaaaataaaataataaatggacgttagggcagaataatttcacctattgatcacctttacatctcagattaagactcaattctaatgtaatgttcggtcgaattctcctattgtattcaatttaccctctcttgagttctcattgagcctaatcaactaattaaattccacatctctatacaaattaaacttagttaaacgagttttttatcctgggaattcaattatgactgcaataattggcataagtatctttactcattatactaatttaccgaattttacgatatggtctaaatcctaaactcatctctctattggtaaaggatccatgaaaattgtcgaaccattgatcaggtaatttaatgtattcaattcatagtaaaaatcaacacatgaaagaattaaaaaccaagaatcttaataagaaatataaaggatctcaaatggttacattattcgccctaacactacatttggctatgtataataaaagaagaaaaataacaaattgtcttagaatacatcaccggattttgtattaaagatgtagaagaaaaagtagatcttgcaccaagaatttcttcctattccaattgatgccttacactatgaattgtcgatattttcttcctttgaatttctcctttttcttccaagatgtgtttctttgcctcttaatgtgtgtagaatatcatattttttggtcaaaagggagttttttttttcgttctgagcgtgtttaggtatatattgatgtcaaaatattgtttctatgtaaaatttcatcaaaataaagaaattggcccatcacagaaaatttggtccatggttgtgtgccatatattttattgcgtatgcaccgatcaataatttttctctcgggttggagaaaaagaggtagtgcgcgcgccatgttacacttgtgtccctggacaactctcggtaaattaatcataacattctcttccgaatttcgattgaggtgattcaaagtgcgttggaaagatgactcaaagtgctacaattcttcttaaaatacatattttccaatttgattattttctacttgaaaaatgggtctcaaattgagacttaaaatttggagcacaacttcttcggctggaaattgatttgtgaaattgcttcaactctatttcattcctttgacctccaattgcatccaattgatgtcatatgattttcaatcatcgttttgttatttgaatcaactattgaatgtttacactttggtccccaaactctggaattcctttgtttttgcatgtttttgttcctttcttccaaatccaccaattttcattgatttcaacccaacaaacataattaacacgaaattaggctataattcattcaaatcactaacaaataccttaatttaatggcctaaataagtatataaaatgcacttatcatcatataacaaacataaaattgattttcgctccaaaacctacatttttattggttacagtctctcacatcagggctacaaatgtttggatttatgtgtaggcaaaatctttgtttcacgatgttgtcttcaaggaatcttgttttctttgttggaccctacaatcaaatctacctgggactccaactcatgcgctttgcctttaactattcatgataatatatatcttaagtccaccatctaacaatgtaggtacaaatcctacacaaactggaaatgatcattccacctctactttcaagtcttgaacattcctaacgaagttgtttttccagatgatatgctaccgtaatagccaggcatgctattcaaaattcaatttttgctcaagatatttcatacaaacccactactacacaaagtcagacattaaatggtttcaaacacagtccctcaatagaagagtgttggaataattctaatgtggacttccaatttgattgtagattttacgtgttagatatatagttcataatgatattgtagttgggccaaatttattaagtgatcaattggccgttttaccccttatagtctatatttagtatgatgtggaattttaagtatgtgggttggaaatatatgtaaaccccaattagagtttaaattataatgagacagtttaataatttcctatataaaggttaaatctcatctcctctccatattgttttattaatttgccacattgacagctaatactttatgatgagcaatgagaggaagatctattattcatatcaaccatggtttccgtaggtatgaattcaatttattaatttattattttgtgattcttgattcttagaacgaatatcattaaattcaacaattggtatctgagcctacatgctaaaatcaaattcctttataaaaataaaatagcattctttttcaattcctaccttcgattattaacacattattcaagttattagtcgtcatcatgtttcgtattttattataaaaaaaaaataaataaataaataaaaagcttaattaagcccaactacatccaccacaactcagaattctctcttaccacaatctttgcatgtgtctctctctcaaaaatcaagcacatggagaccgttttatgtatctacgtatgtatatgtatgtatagctcactgtaggtgaatgtgagcccacagtccaatgtagaaatctattgaacttgttatagaagagaagaacattggaaagtaaacttaatttttaagtttatttggatcgcatctgctaccgccgggcactctgctgcttttgtggcagcaggatcgacaggtgtggcgcgcaaagaataaaaattcatggtttctgtcaattttagagataggggaaaactgggactcttgttgtaaatagctaactttcaagcccctatctgcaattaagtgattggagtcatatttcaatttttaaaaagagggacttttagcaatttgggaaatttgtaggatctattttgtaatatgaaccagggtcatattgcaaatttcaatattttgtaaaggcattttaagtttggaaatttaaatatttgaccctaaaatttcaattttgacccaattaaataataataataataataataataataataattgacggtttttatattttcgttaaaatgtttatgcatttaaaagatttctattatttgcatacttaaatttcactttttttatatattgaaattttgttaccaatttcatctctcaatcacatatgagttttttcgttcatcgattgacgattatgatttgttacataattattgttttgtcattaaatttttcatgggctttgaaacggaccttattttcccactgagataaatattttgaaatgaaaataggtgatagctgtcaaagtggcacactcattgttattattctatcttttgtaccaatatatatatatatatatatatatatatatatatatatatatatatatatatatatatatatatatatatatatatatatatatatatatatatttgtgccgcaattttgatttattgcatataatatcttgcccaaaaggtgttatcatatgtgatgttttggaaaatggcataaggcagttaacgagtttaccttgatctagaaatttccttctatccaaaggtgttggtatttcgagaaccaatgtaattttgttgatcagctacatgatgtgttttaaaaataccttatagcatgttgtattgtcagcacaaagaagattttataatgatgcatctaggctctaatgtaataagattcatatggttctgactttaattacgaattatctaattaatagcccatgttaattagatggatattttatcatccacagaccgcatgcattatgtgtggattatattatatgtttccacaattttaaatgcctcatctctttcaagtcaattgtctactattaaaatcttgactaataataattatgtgaaatgaaaatgaggcatagaaataacacttggtcttctgggcttggattttgtaatagagaaaatgcttgcgaaacccacagataagagcactgttgaatatgtagttgagtataaaaagtgggaaagggccaacaaactctgtttgtaaataatttagcgctctatatccaattccactatgggtgctatcccagaaaatgaaaatgtcaaaggttttatggatgccataggagataaatttgttgcgtctgataaaatcgaaattggggatctgatgataaattgatgaatatgagatatgatagtacaagtggtgtcagggagttatgaagatgataaatatatcatctaagctaaatgctcttaaaatccctattctggaggctttcctgatcaattatgttttaaattgctttcctaactagtttaatcagcttaaggttgcctacaacgctaagcgggataaatgagatttgaatgaccttattgcaatatatgcccaagaggagtattggatgcggtgtgggattattaaaactatgcaattagtttttcagtcatcacagaacaagaagtcttctcataaccataagtctaagttccgtaaggataataagtcacatcgaaatcagtagaataaacattttggccgtgccaaaggaattataaagaaaaataaccaatgtaagttgtgcaaaaagaaaatgtctctaatccatgaatcatcctctatgttgtggcataaacgattgtgtcagatttcaagggataaaatggaaagaatggtaaaagttgagatactttcttctctagacttatttgattttgacacttgtatcgattgtacaagaggaaacctagctaagtctacaaggaaagattccactaggagtaatggtattttggacttaataatactgatatcagtggaactttaccttccaccacacgtggaaacaaatacttcacaactttcattgatgatttctcacaatatggatatgtttacctgattaataataaatctcatacacttgagaatttcatgatttaaaaaatgaaagtaaagaaacaatgtggaaaaattatcaaaattgtaagatttgatcgtggtagtgagtattatggaaaatatgacgagtctgatcaaaacatgagtgattttgcaaaatttttacaagagtgtggaatagtgtcctaatacaccatgctagggacacataagcataatgattttaatgataatgggagttctacattgagagaactttttgttgaaccaaatcaagttattgttctaattcctgctatacggaaagagttggttctcaactagttgaagttgttaatgaagaattgatgaatcaagaggaacttccaattcctccaacaacaattgggtcagtttttgagccacaagttacgagatcgcaaaggtaaaagagatctgcattgcccagtgattacgttatctatttattggagagtgatttcaatattaggcatattgttgatcttgtaacttataatcaagcatttacaagtcttggggtagataaatagataaatgctatgggagatgaaatgaattccatagaacggaataaagtttgagaacttgttaaacttcctctaaatgctaaagctattgataacaagtagatctttaaaagagtaaattggattcaaaagggaatgttgaacgaaagaaagcaagatttgttgaaaaaggtttcactcagcgagaaggcattgattatgttgaaatcttctcacctgttttgttgaaaaattcttttcgaattattatgacacttgtgatatactataatttggagcttcatcagagggatattacaacagcatttttgaatggagatctttctgaaaaggtttacattagacaatttcaaagctttgttgtgaaggtaaaagaaaatttggtatgcaaggtaaacaaatccttatatggcctcaagcaagcatcacgacagtggtatttgaagtttgatgaggttgtcaattcttttggttctatcgaaatatagttgatcaatgcatttatctagaataaacaattacaaatacaattatattgttactaaatttcacttctttatccaaaaataaatttgatatttttccgactttatccatagacaaaggatactcatgcaaaatcatcattttcgaaagactatatcgatacttatctggatcgaaagagtaagtacccattgtgaccttgccactcgtggcatcctttttgaaacttaatgttgcttggtgagtattatccttataacggaatacacatctcttcaaatgatcatgcaaatgctttgtaccattttttgtgtcacccctaactgtttattgcaatgattgcatatagtcttccatttctcactaattttttgtcttttgtagtgctcccaaacagatgaagtcaattttctctttcctaaagattgatctccaatgtcacgctcctcgtcacttaggtttattggcctttcatctgcattcggtaacggtttagctggatcttcttgcgggacattactcgtgggtatattggtcgtgctatcgtcctcgcatattagtcctcatctaatacttccagtactactggaccagacataacttgaatgcactacagaagacaagaaacaaataaacaatcattaaaattaatttgactagtaactcaaaagtcatgataattccaagataaaagaaaaaaaaggttttcaggatttggtctgagatctgtcaaattgaaaaacctagatggattatttgtccatataaacattaagaaatgcaataacatgaaattacatgacaaggtgaaccataaaaaaaacgattacacggtatttcaattagaagaaaatcagcattcgacaagatcaaacaagctaatatttacaacaatcacattgcaacttattcaagatcgacttttgatcaggctagagatctaagcttctatttctggtttatgtaatatttagaaacactatcatttgtatgtttattttccaaatgcagaaaacactaacaatatgtttctaagctcctgtcttggaacaactaaataacccgaaataaatataaatttactccaaaatccaaatacacagttacaagaaattatttcaaatccgtgacggtatccattatgcatttaataaacaccacaaattatcgaaataaatcaaatgatttccttgtatgttcggcacttcggctgcatttaaaatcatttttatgaaatgagtaataatgaaacatgtacaataatatgcacctgttgttccataaacagtgaaaaaactttgtaaaaacttattctaattgaaattgaagtagacccccattgacttattttacaaaagcgaacacagtaaatgccctcaagacaatggattatttgtgaagtactaaagttgttacatcctatttcgtactagtcaaaggtcaatactatttattcaaagtcaaatatttgactggtcaaagtcaaagtcaaacaaggacttaaatgaagtaaatcattttaatgggacttgaattgaccaaattatttttgggagtttattttacaaattgacaacatttaaaggtttaagatgaatggaatttaattttgaggattttgaatgactaaatatcatatttaattgaagaagagggacttcctttgcaaaaatgggttagggcagtacaagtggcaagttattcactaatatcccatttttcttcatatgatacatacacacgagagagagagagagagagctggacgggtggcatgttcttaagtaatatccatttttcatatgataaaagagagagagagagctggaagggcagaagtaagaaaaaaacaagaaagaggaaggaaaaggagaaagaaaagaaaagagaaaagggaagaaaaagaaactaagtgaaaaaggagggggagcgagggggggggggggggggggacccttgagtcccattattcaatttcttcaatttttagagaggaaaagaggtaaatattttgtggtataatttatattaaattttctaggcttctaagtagttgggctaatttgatagtttcattttcggattgatggaaagattatgatttcaagctgatttgtgaaagatttttgtatcaaagtaagaaatactaattttggtaaatcctagagtttttaattgagtttttgaataggtatgattagtggaatgatggtaattgataaacataaacattatacatatctatccatttctcacttttggggaatgtagggactgaaggaatagaaaagggcagatacataaatcgagttgagtggataaatatatgtgtaattgtgttttgattagtagaaattccaatggaaatggaattagttgaacaaggatcccatgaaaggaaaatgaaattggttgtacagggcttaattggaaggaaatgaaattgttactttttagcatcaaattgtagccaaaaatgaaaaaggacttccttgcatttggcaaccatagtagcgatcgaggaagaagggtaatcaaattaagactattggtcttataatgtgatcatcaatgggaaattagaaagctgaaatatttactggctattattatgttggcatgaatcagtgggatatattatcaattaattttaactgactttgttatgtatattaatcttgagacgggttggattgtaattttatcaaataattatgttactattccaggaggcaatgtagacattggaatagcttaccagctgaacgaatcatcacgtaaatagctttttgagtggaaaaacttaaatttttttaaagtgtttctaaataaagtatatgttcaactatgtgtttgattttatgattattatataagtttcgtttattatgatccacgtagaatttcaaggattatttatggtatgtttgtgacgttgtatgtgaaacatgtgatattgagatttgtttggtatgtgagatatgtgatattgagatcgatctgaaaaaagtaccatgattatatatttcttctaattcaatgaggggccgtggccgtgttctatactatactgaggggtcttagaccagggatgaaggggttttgaccgtgtacatatagtttactgaggggctttaaccgtgttctagaattgattatcagaagtcttgagacctgtggcgaaagtgcttggcttgatggacgaatttcatattttagtcagaatgtatatttttggtggatcatatgtgatgtgatgagatgatggtatatatatcagctaatgactatattgtgattaagagatgatatttacagtattacgagaatgtttcactttttgtttataattgtatgaggctatcatgtgaaatattaaatgatatgaatttgatgtttgataaaaatatttaaaggagaaaatatgattatttttgaactattccactcactgagctgtcaactcatatttttctaaaattatttttataggtaatgttggttcttgatagcttgaggagtctagtgatttcagagttagagacacacgacatattgaatgatatgagtcaatttgataaaccatgaagtaatttttgagcccattgcactatgtttttataaacatttgatttaggcgtatatgttgcaataactcatagtctaccttggtggtagatatgacatctaatcagcatctatcatcaacgcacatcacgtttcgggtctatagggtaattcgggattggtcatgtcaaaagtagacatgatgcgactttaaaaagaatctagttatttacttataataaataaatgtaattacaggtgaattttatcttggccaaacatggactctaaagcttaagaatcaacttaatgaagaccaaagtccgtaagaaattaatggtgcagacacaattaaacaaactcagcttgtgttgacacaacgaatttattgattattgacgtgaatgtctgaaccctttttttagagtttctgaggaattatagagctctttcttgaagtaactgacgcacaacaaaataaatagcaatttacaacaaacccacatacaaaaatcaatgaaagtatccattatgcatctaaagaattcaacaaattatagaatgaaatgaaatgatttcctcacttatgattggctggacatataaacatagaaaaacctccagaatttggtctgagtctgagagcaaggttgctggctggtgggtggtggctgcgtgagactcgttggcgttgctggaaatggaatgattcaatgaagatggatttttaggattgtgttgggtttggggaattgtgtgtatgtagtttattttggatttgggtttggggaaatttggaatgggttttgggtagtaggtgtccagtccagcagcaggacgaaggggggggggtggaaaaaaataatcgcggggcggggcatccccgccccgccaacccgtcgggacggattttacttccatccctaagtgtccttaataggtttcagtcaaatccaagacaagagtattgaaaagtagctaagaaagtcatgagatacttgaagaaaactgaatattatatacttacatttcagcattcaaatcatattgaggtggtaggctattcatattttgattttgatggatgtcaagatgattcgaaatcaacctgaagttatattttcatgttagctggcgtgctatctcttgaaaaaaaaaagggctaaacagactgtagtgacattttttactatgcaggttgaatttgtatcatgttatggggctacagttcaagctgttgggttaagaaatttcatttattagttgaaagttgttgattttatctcaagaccaatcactatttattatgataataacgaagcaatgttcttttcaaggaataataaaaattctggtaagtcaaaatacattgacatcaaatatttggtggttagagatagagttaaagaagtgcagacgaaaatagagcgtagcaggacaaaggcgatgatagcaaatcctttgacctgactaagggactcgctccaaaagtcgttatatatatgtgtgtgtgcgcgcgtgtgtgtaaaagaactatgacattggttagaggatggggatccatgttgataaggatgctgacatttatagttgtggaatggtatgacatcgcttaattggtgtaatgatttacatgttcggtggagtgatttcgacgtccggtgttaacattcttgttggaccggatcatgctacgtaaggtgtcatcattggaactatactttttttaccacatatgtacgttaacctggatgttaaaagttttgttataacagttaaatatttgcccaagtggaagaatattggaataattctaatatgggctttccatttgattttaaattttacggattagatgtatggttcataatgatattgtgatagacaaaatttattaagtgatcaattgagtcgttttacaccttacggactatatttaatgtgatgtgaaatttaagtatgtgggtcaaaaatatagaaaccctaattagagtttaagttataatgggacgacttaataatttcatatataaaggttaggtctcatcttctcttcatattgttttattaacttgccttattaacggctaatactttgtaaggaaaatgaggggaagatctagctgctattattcatattaacgatggctttcgcatgtatgaattcgatttattaatttattattttatgattcttaattcttagcacgactatctcattaaattaaaagagacaaaaaataaataaataaataaaagagagagagagagagcgtttttttagctttgtttgataaccctagtgatagcaacggggcagggcgacgtttctcccaccccacaccccatctcgcacctcgccctgccccaaacccgcccctcgccccgccgaagcagtgggcttgcctcgtttcttgcccccccccccttttttttaaataatttcgagttcaataaaatacagataacattcaagctgacaaagttaatatccaaaataaaacactacaaatattaaatataatggtcgctattggtacacaacattgattattaggatgaacaatattttttgtgttttttcttttgatattgtcacaaaagttataaccccacacactttaatttattataatatataaaatttcaaattttttcagttgaacatgttatatctttttatatttgttattatcaatataatatcaatttgacaaagtagcataatagtatatataaattagtcaagtttgataagacttgtacaattgaggatactagaaaatagatcacatccttatatttgaaacaagttgaaccaatgaaccctaaaaaaaaaaaaatctcggggcgagttcagggcggatttttttgctccattcggagcaggacgaagtaaattgccatcactagatatcccctgccaaagtgcgtacttgcagaatcaatctctatgcctatagtaccttgacgtttactgaagcctcaaaacaatcaaaatggcgtgaggctatgacgtggaattcactgatctattaaaaaatagtacaagggacattgtacttcctaaattaaatactaacctggtgggaaataaatgtgtattctgcattataaaaaaaacggtagatgaaggtgtagagtacttcaaagcgcttcttgtagccaaaagctaccaccaccaacctggctttgacttcaccgaaacatttagctccgtgaaaaaactatgaacaatctattttatactgtctctggctgtcacacatggatggagtatccatcagattgttattcagaattttgttttacatagaccattagaagaagtttatacgcagcagccccaaggttatgaatacccatattttctgttgcacgtctgtcgaccaaaatgagtctgtatgacttaaggcgggtaccttgggcatggttctctcgattaactgagaaattgtaacaacttggtttttattggctccaaagaagacaattccctatacacccttcatcgcattatattctcttcgtatattttaatctatgttgatatttttatcactggctcccattcacgtgaaatttaagaactgatttggctaattgcaagtgtctttccggtgaatggtttaggccgtttatccttcttcctcaatttggaagctatatttgatgatcaaaacttatttttgactcaaagaacaaacattgtagatctattgaaaagagtcaatttgcatcaagctaaaccatgttcgacaccaatgagcacgagtagtaacttatccaagtttgaagtttgtgaggattttgatgaaccccagctataccggagcacttttggagctctttattacttggcctttaccagaccagacatagactttgtattgcatcgtgttagtaagttcatgcaacaaccgaaagatatccattcatttgcaggcagtgaagtgtatccttcagtattaaaacacacgattgcctatggcctcaaactctccagtaactccaatcactctcttcaggggtatagttatgcggattgggctggtgacaaggataacaaatgaagtgtaggatcctactacatatattattcagggagcaaatataatcggttggagctgtaaacaacagtaaaccttcggaaggagtaacacagaatcggagtacaaatttctatctaacacagcagccgaactccattggttacaatcagttttgattaatcttcaacttccacctgctatttgtccaacattatggtgtgacaacattggagccacatatctctcctcaaatccggtattccatgcatgcgcaaaacacattgagatagattttcattatatacgggatcaagtcttagcaaagaaattaagagttttatttctctccactcaggatcagcttaccgattttttaataaagccactcgcttccgcgcgctttcagttgataagagataactttcatgtgcaagatttgtccctttggttgaggggacgtattggagcaaatattttttgcagtagatattatatatttgatgcaacaaaaaatgctaaaaactcagatatttgtgcaatagaaaataacaacagatattaatgtaacagaaaacaataatagcaaaggagttgaggatatcttgggatgttttgaaattagaatatgcaaccctgtttggtagttattaaaattaatttttttgtaaatttcgatagaagttaatgaaatgcattgcggaacacataaaatatgcgattagaattaattatgatttacacttagattaaaatctaaattttgattcgtaacaaacaagggcagaaaagcaccaataaaatagcagtaagttcttaaagccgtactatttaaatcatagcatgtaaacatcatttgaaatgaaaaagtgaaagaaacattcagtacatattatttccaaatttgttaagtgataaaatctcatattattgaataaagatagaaatatagaccaaattattaacaagaccgaccttttaatatagaacaccaagtcttaacatgatatcacagccaattgagttttaaagaataatttgatttgattaagattaaaaaaaatgagtagacggatttcaaaattggttaattcaaatgagttaccatcttgaggaatatattaagggatagaatttcatatttaataaagatgaaaacatagaccaatttaaaaaggttcggattactcctcttaatacgatcgacttttaaaaacgaaattccaagtcttaataaaatcctacaagggtgaatagggttttaaattcttcatcttaatttgaaaggtattgaatttatattttcttgagtaaactaatgtttgtacacaagagtaacttaaatggatgctcactaaattttagtattgattaccacttttttccaaataaataaatggttaccaaatgttccctcaactattctttaagttacccatccatcatttgggactaacctgtctgtataggtggacaataatttacacgtggatatgaaaaaatgacgtggatgatgaatcatgtccatatcatctaaaattgttatatttaaaatactcaaaattgcataattagaaatagacgtgttttttggatggagaaaatcaaatgtctaagaatcagagagagcaaaattttcatccccaaatcaccttcatcttcaaatcatatcctctggctaattcattcaattggtaatccccgatttgtaatcgatattgaagaagttctatatctacatccccattaattgaaatttacattgtgcctatacacgaaattatttctttcgatttaaaactcaccgcaggtgtacggttcgttaacaagtagtagaatggattatgagtccaagtatcgatcccataaggattgaattagttcaaatcaatctactatgaccttaaccgaaacacgaaagtaagatgcatgtattgtgatttaactaagaaaaatgttaactatgatgcaattatgagtgagaaacttatactaaatgcaaaatgacctggatgcaatctatgataatttatggaattaacgaattactaacgcactaggatcacgaattcccaagcaacacccgttcaacttttaatcatgcaaatttgacacacattcccacaattgataaatcaatattcttgtcttaatttagcaatctctctcaagtaatgtcaaacctaccccaatatgtgattcgactatatctctatgacgaatactaacatacaggaatgcattatgatttcatgaatattcaacaattcacacgaggcatagaggtatatttctatcctctatcgaaccctatgatgatttatactatgtcgagcctattttccttctctcgaatgcataaaacaggccaccaaaatcatataattacgtgcacaataataatatggacataaaaatgtataaatcattcaattccggaacacgtgcttaaatatgtcaaatatccaaataaaaaatcaaaacttgtattgcaaggttcatcgatctcctagtacatgaaaaatctagcctaacatactaaaaaaaagaaagtaaaaaaataattgaagaaacgtcatcacccgaatcaagtttcgatcaattcttcaattggcgcgatattttcctcttgttctcccttcgttttctcctttaaaatctctctttttcttctaaaatcggtgtccccttcgttctggtcgagttttcatttatataggaccccaaaaattttgtttccacaagagtttcggcgaaataaggaaactgcagattcggcctccgaactactctatgtgaccgcatagtacatttctatacggtcgcatagagtaaaaaattttgagaaattattctcggtctgcctctatgtgatcgcatagagggtagcactatgcggtcgcatagtgctaccaactatgcaaaaaatccattttggtccttgaactttcattcttctttatctcagtccctttgcaattccttcttcttccaatcatcctgtatcgcgttaaagttcatacttagcatattttcattcccgggttgctttttagttcaactttgaatatttatatacttagtccctgaactatcactttgctccatttcagtccttttcggctcttttctcctgaattccacaattttcatagaaacacctacattgcatgaattcaataagattaagtcacaatttaaatattttgctcgtaattaagtcatgtttgtgatctaaataagtgtgcaaaaatacatttatcaaaccccccaaacttgaactattgtttgtcctcaaacaagatagtgacttaattctgaataaacatggcttaataccctgtcgtggctcaggattggactaagtatttgactttattaaaaattttcagtgcaaaaatgacatcaacttttacctgttaaatgcatacttgacgtgtgtgtatgagttcatgccaacatatcaaattcatgatgggttgagtcccgaccccaagtggtcaaatgtatccttactcgctcaagagatacacaaccccccaaacttattcttttcactcaattatcccgggattgtgttttaagattaggagtttacatagctgtagtcctcaccctctcatagtttggattgatcttactatcacaagcttacatttcaacaagtgaaggttttcccaagtttgattgcttcgacactcaagattaaaataggttacttgccttacctcaaaggtatagtttcctcaaccaaatgtctaagggcttttcttcattttttgtctctcttttgtttttatatatatataattattattatttttatatgtatcatcttctcatttgctttctatataatccatgtaacgagctttaggccggtaactcctaaaccagttggctttagggcaccaagttttaaacccttgcatgcttattcactcgggttataaaggctcgatcagatgactttttattaacctctttccctcttgctttctatatgacccctttagcgagctttaggtcggtgactcccagatcagttgaccttaggacaccaaattttaaaatatccttacaggcttacttgctcgagtcataaaggcatgaaaagaagagtcttattctcacaatttaattttatgcctttactgttctagacatttagtttccaaaaccaaccctcaatttaagattttaacctaatcttcacctcgctggtctaggaaatccacacaataaaatttcatgcacggagcccccgcttatctcaatgctctctataatagctcaaccaattccaaacaatcttaaggtgatttacgtgtcaaatcaatagagggttatcattcttttcctactttatgctcaaaatgcagtcattcacccgacatgttaagcatgaacaacatgcatagataatgtcaagtattgcattacaaatattggttaatctattcagcactatattcaaagtttatgaattataccaatccaataatcacatcatagccggcaaggctatcaagcccacacaagcatgcaaaagtataattaacactcactcatcaagaattcatcgtgcaacaattagtcaataataacgatggactatgaaattgcaaaataattacatgccgactatttgttttaaattatgccaccatcccccaaacttatacagtacattgtcctcaatgtaagaattaaagttgaaatgacataatttaaaaggaaaaacaagaacacaaaatagcaaaatgaggtaaacaagactcccctgatcaatatggtggctgtgatggaaggttgggtcctgcagcatcatctccagcagggagaggaaggcgggataaaatctctctcaatatgtcagactactgggtctgctctacctgcatggcctgaaccctggtctttaagctccctaaacggtcccatgtctcattcactcaccactgtatatcatccatcctgccaacgtacattcccaagcccccatcaaaggtactcatctctcttcacattgcaagggactcactgctggcattggatgcgaagtttcttgtgattgccatatcattctgcacctgctggatagtggtactcattgctccaaaagattgctgaagagtctgcatgtcctggttgtgtcctgttatagtggcaaacatctgccttaataactgggtatcaatttcaactaggggtggaggaaattatggcatgtcaaagtcgtcagctacttgtcattcctcatcctattgctatcgacgtcgctcgtttttaacttctgttgatgtttaactctagctcggtcctgggcctctagtgtgaggggcttgatatagggacttggtttttctggtgcttctccaggctggacttgtatgtctgcagctctacatatcccacttattaaacttagaaaaatcagtgaggtgtgcctatctccccatgtgcctataatgtgtatctggttgtagatgtatgtggccaagtcaatcttgtttccccgaaccaaatgatagataaaccccgccttttgatttgtgaatgtcatcctataggatatgggctcgatgttgtggcatatgaataaccataggatagctatagatgggatgagatcaatttgataccaatttgcagtagggagaggccaagcattctcacgtcccaataataattctgcaacctcaatccagttgaaattatgtgggactgggaccacattattccaggttagttggtagtagtcatgaattacttctagtgaaaacataatccatttaccccgaacccatgtttgatgtagatgatctaatccaggcttgtcgatttctgtattgaagttggcatagaactccttcaccagattttcttacactggatgcggtctttcaattactttctcccaaccacagttgtggattaaataaactaattcaaaactgaggaaatcgtccaacttaactagccttttggggatgagtgcccactcgcggacaacattggcgtaacgggctgctgtgtctgaggatagaaatctcctgatacccccttcgggctctctagtctgggctgtgccatatatggaaccaaccttctcttttccttttgatgttctttttggaagcaacctgcaaaggtatagaaataacattcatcaaacttcttgttgaaaaacaagagaatgaatgagattagcaagacatgtattttacaaatcccccaaacttgcttcaacatgcatatataacacattggtgtgcaatcttcaaaacatgatattcaatatagtgtaaatagtgtgccaatatgaaaaactaagaaaactaggcctaaacatgcacatttgaaaaattggacctatgaccgagtgcgtatattcggccccgggcatcatcgaaaaatatcgagattttcctgggaaatctctgggcatgtgaaattattcaatgagatctagcatatactcaaatttcaaatcaattggactttgtttggtgtgtcaaatgatggtgtaaagtaggggacgtagggtgttgtgacatgccgtgacctagctatgtgcctacgtgttgcaaaatggatttgatgttttacatggcctttcatgtgtatgtgcatgtggtagtatgcaaacttctataaaacatgctcaagaactataaggaatgcaaaataacaacatacacacaagttgagctcaaaacatccaaattgtgtcaagtgacccatgatcaagtgcgcaatttcatccctggacatcatcgagaaaaatcgaatttttcccaaacaacctctgggcatatgaaagtacgtagtgtagagtgacacatattcaaatttcatacccattggatttcgtacgagtacttaactcaagggacgaagtgggtgctatgaagtgacataaacctaacatgggtgcctacatgtgtgtggttggtgagtgaatgcttccagctcaatttctatggcattcgatcacaatgtgtatgttaatttatatattcagattgtcaaatgcgagattcgacataatatacaacaaacttcacttagacaatttattgaacatgtaacatgcattccttggaaacactcaaaatcccaaaaattgaatgtgccaccaatccataacacaacccaagttcaaattacataatccatcgactacttcggttcatctcgaatcgaactaaaaaatcatagaagaaagggaatgagagaatgtaccttgaattcgcaatgaacgtgtggagtattgatttagggtgccaatgggatgaagaatgctatgtaatatgagtgtgagttgtgtgtgagtgtgttgtgtgaagtgtgtcttaccgtgtgttggtttgaaggtgcgagagatgtgtgaagagggagggaggggggaatgattgagagtgacttggtcatagcttaaatccatgaccaagtcactactatgcgatcgcatagtgatagaaatgccccaatttttcttttcgattgatgtctatgcgaccgcatagacaattttttttaaaaatctgaattatagaaaaaaaaacaatatcaaaattacaattttaacctccaaaacacaacttaattaaaattttctcccgaagttggttttcaattaaaaatttgacttggctaatatcattcctaaaaaatctagaaacttccaattcaatgggatatgtgcttgccaaaagacttagcaccaagaccaatttattgaataaacttgaaacgcattctgaaaatttttatgaagaatgactttatgcatcgaaatgcccccaaaacaacttcaatcaacttgactcatgccaccttacatgtgtaatgcttagactagtatgcgtgaaagatcgatgacctaacaaaaaaaaaattgcaaatgcgaaattaaacaactcctaaaataatgtgaaaagtaaaataaatcgaaggataaagtaggttgcctcccacctagcgctaggttatagtcgatagctcgactttaccgtattacatcattctgatggtctaagatgaacggtcgacttttcctttgagaaatcgcctctccaatagtgcttcaaatggtgtccattgaccttaaatgtttccttactatcatgagtgatctcaactgtcccatgtggaaatacctgtgtaatagtatagggaccagaccacctcaatcgtagctttcctggaaacaacttaagcctagagttgtagagtaacactttttgtcccactttaaattcacgcctctgaatatgcatatcatatcactttttggtgcgttccttgtagagtcttgaattttcgtaggcctccattctaagctcatccagctcattaagttgtaataaacgtttttcacccgcagcattcaagtccaaattaaatttctttattgcccaataagcaaggtgttctatctcaagaggtaagtggcatgccttcccgaaaatcagtcgatatgatgacatccctataggagtcttgaatgcagtcctataggcccacaaggcatcgttcaacttcttagaccaatcttttcgtgaagagcttattatgacttcaagtattcgctttaattgcttattggacacttcaacctgtccgctggtttgaggatgatatgcactggctacacgatgtttaacgccatatttagtcaacaactgttcaaattggcgattgcagaaatgtttgcccccgtcactaattatagctctcggtgtgccaaagagggtgaaaatatttttctttagaaaatcaatcaccaccttcccatcattggtaagcaatgcaacggcttctacccacttcgatatgtaatccaaagccaccaatatgtattgattagagaatgatgggggaaatggccccatgaagtcgatcccccagacgtcgaatagttccacctctaggatactgttcaaaggcatttcatttctcctggatatattatcggtgagttgacatcagtcacaccttttcacgaattcaaaggcatccttaaacaacgtaggccagtaaaaacctgactgaaggatcttcgtcgctgtttttgaagtaccaaaatgccctgcgtatgtagatgaatgacaatgttctagtattaagggtacttcttcctcaggtacgcaatgacgaatgatttgatcagctcctcgtctgtatagaatgggatcctcctaaaaataatactttaactcaacgaaaaatttcttcttctggtgattcgagtaatttggcggaatgatagacctggctaagtagttaactatgttagcatactagggtgcctcctcctcaccaaaaatctgttcatctgggaagatttcattgatttccatgatttatgtttgctctgtggtctcaaatcgagacaagtggtctactaccacgttttcattgtccttcttatccctgatttctagatcaaactcttgaagcagcagtatctaacgaatgagacatggtttagcatccttcttttccattaagtacttgatggtagcgtgatctgtgtaaacgatgacctttgaacccacaagatatgattgaaaattgtcgaaggtgtagactaagccaaggaactctttctctatcgttgcataatttaattgagcgtcgttcaaggtcttacttgcatagtagattacgtgaaatatcttatttgttcgttgtcccaatatggtcccaacagcaaaatcactggcgtcgcacattaattcaaatggcaggttccaatccggtatgatgatcacggatgctgaaatcaacttctctttcaaggtattaaaagccatcaaatactcatctgtgaactcaaatgtggattcattcatcaacaaacagcatagtggtttagtatttttgagaaattttttataaaccttctgtagaacctggcatgcctaaggaagctacgaacacctttcactgatgttggtggtgataatttttcgatcacctgaatctttgctctgtccacctcaataccctttgctgatattctatgtcctaatatgatgccctcctgtaacataaagtgacatttctcccaattcaacaccaagttggtctctgtacaccgctgtaacacaatacttagatgctccaaacactcatcaaatgaagacccaaacactgagaagtcatccttgaatatctcgatgaatttctcaatcatatcagaaaatatagcgatcatgcagcgctgaaaggtggcagcggcgttgcacaaaccaaagggcatcctacggtatgtaaaggtatcatatgggcatgtgaaagttgtcttctcttgttcgtcaagtgccactggaatctgattatactcggagtacccatcgagaaaatagtaatgtgagtgccctgctagtctcttcaacatctgatcaattaatggtagtggaaaatggtcctttcgagtagcagcatttagtttgcggtaatcgatgcaaactctccatccagtcactgttcttgtaggaatcaactcatttttctcgttctgcactactgtgatacctctcttctttggaacaacctgcattggaccaatccatgtactatctgatattgggtagatgatgcttgcatcgagcaatttcaatacctcagccctaaccacttccttcatgtttggattcaatctctgctgaccatcaatgcttggcttgaaattttcctccatgagtattttgtgcatgcatagcgacgggctgatcccctgatatctgcaattgaccatctaatggctgttttattctccctcagtacccgaagtagtctcttttcctccacttcactgacagtatttgaaataataaccgagagtgtaaaagactctcccaagtaagattatcgaaggtgtggggacaattgtttgagttccaacttgggaggttgctgaatagatggcactgacttcgtagtcctagttttcagttcttcgaagtgacgcttgcacatatatggtggattagtttccaaaaatcgtgcacatgtttcaatctcacttgaatcagtgtgagtggattgagaatgtgcaatgcatgcctcgtatgcatcggaaggatgatgtagctgaaatgtgtcttgaattattctgtcaattacctcgatctggaagcagctgtctaatccagtggaaagtttcattgccttgaacacgttgaaagagatctgttcttcaccaagcctcagtataagctgccctttctgaacatcgacaattgctcttccagtagctaagaaaggtcaacccaatatgagtggaacatccttatcttcctccatgtctaaaatgagaaaatctgctgggaatataaacttttctacttttaccaacacgtcttcaatgatccctcttggatttgtaagggatcgatctgctaactgtaaggtcagtgctatggcgttagcttttcccaaatcgattttcctaaaaatagaaagagacatcaaattaatacttgcacctaaatcacacaaagctttatcaaaatgacaattttcaatagtgcaaggtacagtaaaactccctgaatcctttagttttggaggcagctttttctggattctggcactgcattccatagttagcatcactgtttcattttcttctatctttcacttgttagagaggatatcctttaggaattttgtataactcgacatttgaacaagtgcctcagcaaatgggatattgatgtgcagtttcttgaggacttcaagaaatttactatattctggtccaatttgtactttttcaacctctgtgggaatggaataggtggctcatgagggttgatagaattggcagctgtaacccgtgatgtattggaactcttcttggcaacatcctctattgtttgtgcagtctgttccacaatctcgtcatctgaggtaggtgctgattccttgctaactaccggtctttttacacgtatctctggtagttgtactccacttctggttgttatagcttttgcgtgctccttaggattgatttcaatgttgctaggtaggtttcctggtgctctacccgtcatggagattgctatctgtcccatttgcgtctccaaatttttgattgcaacacttgatcttggagagttgtgtctgtcttttgcataaactggctgttggactccatgtaccgattagtcgttgccatgaacttctcaaacatctcttccaatggtgactttttatcctgctgctgaaattgaccttggggtctgttttgattctggttactccatgagaagtttggatgttttctccagctctgattgaaggtttccaaatgtggattgttctgttggcgttgaccccattgcacaaaatctgcatgttcgatcccctgtatgagaattggacagttgacagtattgtggtctgctccacattctttacagcttagcttcttaacttgttttacattggcggtctgtgaaatgttctcaagcttatggaacaaggagtttatctttacgaataatgttgagtaaatatctacttcataaactcccggtgttctcttctgaaccactcgatctgtagaccacatgactgaagttgtagccattctctcaaacaattcccatgctccgtcaattgttctcgtggagatcgacccttcggatgatgaatccaccatgctcttgaaggatggaagtaatccagtttagaaaaattggatttgtgtctttttatcaaagccacgctgaggacacttccttaacatatttttgaagcgattccaggcctcttcaaatgattcggacttgccttggttgaatatagatatgttcgcatttttgctaccttagttggcgagaagaacttggtgcagaatttgtgggctagcttgttccaagtggtgatgcttgcgacggaaaccgaatctagccattcaagtgctttatcccgcaaagtgtgtggaaacaatcacaatcttatagcatcgtctgagataccctggtacttaaagtgttggcacatgtccagaaatcaagatatgtgtgtatgtggattctcattagccatcctgtggtattgatgcccattctgaaatagttgaattacatttgttttcagctggaagttcggttgcccaaatggaggatacacaatgctagattgactctggacgaccaacggtgtcatgaagtccacaagtaccatattcccttcatcttcaacccctgcgccttcgttgagttgaattaccagacgattttgctcgttagccatttgttgttgttgtttttggtctttttgaatttgttgtgctgctcttgcttctctttgcgtgtgacgaaatgtgcgttcgatctctggatcaatgggaaccaaatctgatcaggtgctctttgcatacaagcactgagatagcaaaaatagcacaaaattaaattaaagtaaataataaactgagtctagtaagctaactactactaatctaggtaagttcgaattaatgtcacgatagatacaaataaactaaatttcaatctctggcaacgacgcaaaaaacttgttcacgaaattatttctttcaatttaaaacccaccgcaagtgtacggttcgttaataaatagtagaatggattatgagtccaagtatcaatcccacaaggattgaattagttcgaattaatctactataaccttaaccgaaacacgaaagtaagatgcatgtattgtgatttaactaaggaaaatgtgaactatgatgcaattatgagtgagaaacttatactaaatgcaaaatgacctggatgcaatttacgataatttatggaattaatgaattactaacgcactaggatcatgaattcacaagcaacacccgttcaacttttaatcatgcaaatttgacacacattcccacaattgatgaatcaatattcctatcttaatttagcaatctctctctagtaatgccaaacctaccccaatatgtgatttgactatatctctatgaagaatactaacatacaggaatgcattatgatttcatgaatattcaacaattcacacgaggcatagaggtatatttctatcctctatcgaaccctatgatgatttatactatgtcgagcctattttccttctctcgaatgaataaaacaggccaccaaaattatataattacatgcacaataataatatggacataaaaacgtataaatcattcaattccggaacacgtgcttaaatatgtcaaatctccaaatcaaaaatcaaaacttgtattgcaaggttcatcaatctcctagtatatgaaaaatctagccaaacatactaaaaagaagaaagtacaaaaatagttgaagaaacgtcatcacccgaatcaagtttcaattaattcttcaattggcgcgatgttttcctcttgttctctcttcgttttctccttcaaaatctctctttttcttctaaaatcggcatccgcttcgttctggttgagttttcatttatataggaccccaaaaattttgtttccataagagtttcggcgaaataaggaaactgcagattcggcctccgaactattctatgcgatcgcatagtacatttctatgcggtcgcatagagtaaaaattttggagaaattattctcggtctacctctatgcgaccgcatagagggtcgcatagtgctaccaactatgcaagaagtccattttggtccttgaactttcattcttcttcattttagtctctttgcaattctttcttcttccaatcatcttgtatcacgttcaagttcatacttagcatatttgcattcccgggttactttttagttcaactttgaatatttgcatccttagtccttgaactatcactttgctccattttagtcatttttcggctattttctcctgaattccaccattttcatagaaacacatacataaattcaacgagattaagtcacaatttaaacattttgctagtaattaagtcatgtttattatctaaataagtgtgcaaaaacatacttattagtgcacagtttattcgaaatcagtgcgaaccccacttttttctcctaaatcaattcaactaaaatttggccacaaaacatagaaacattcttgtcgtggttttaaggaacctagaagacccaagaagtatagaaatggaaggcaatgtagttatggaggaagccctttttcagagagtggaggagggaccacataaggtaaattttatactattttttggatggattcttcaattttatactataaatgtggaagacttgtcgagactaggggtgaatgcggttcggtttgggcggtttgtgctatatttttaactcaaaccattttatgcggtttgaaattttttgaaaccaaaccaaatcattttacttctcgaaccaaaccataatttgcggtttggtttagttttaatccgcggtttacctttcgacgttatagtaatgtatttaacataagttaaataaaagtttaaacgaaaactaatgatgttaaatattaaattacattcatatttaccatgaaacccatgataaattattatcaaagttggttgctgaaagatgttaatagaacaaatacatatttctttatttttatttaccttttcttgtttgacattcatatcatcgtatagcggttggtaaatgtagagttacattgtattattatagtttgtttaaaactcctttcgttttgctagttaagatgttaaataagattgaatatgatgtgtttagatgtacaaagattgatagagttttaacttattgggaattgacaaattttatcctctaactactttatgaaagtataatgtaatagtactagttagggaattttaatattttcacacaattagtgcgctccgcccttcattcttttcaaatcacaaataagttcattatcatctagacacataaacaatcatttttctatctaaactacaactcacaagtgtataataagtttaaaaaaaataaaagaaagaacaatggaaaaataacttgaataaaaatttaagacttatcgaaagagaagagaaaaagaggtgattcaagtagagattagtggactaacaggcaaagacgactggtgattcattcagcagtggcaaacaagtgtcaaatgttagggaaatgagagtttctgaaattttgtacgtgatttgcggacatagttttgttgaattataatttgaattgttgaaaatatatatatattttttcttcatttcatatgattttgggatattttagtttagtttaaatatcgggtgaggacatgtgttgtaaacccattaaattataggtcataatgatgaccctaatttactttctataattatttcaatacactggttataatttgtattgctgaattgataattttttttaaaaatgaaaactgtaaatttttaagttaataaaatttatttttaattaaaaattttaaaagcgattcggttcggttttgtgcggtttttgaaaattaaaacttaaaccaaactattttgaaacggtttggttcgatttgagggaaaataaaccacgggtccacgtggacccgaaccaacagtttcaactcagttcggtttgcgatttcgcggtttttttgtgcagtcctagtcgagatggttatttttgtccattaaacacgtgatcgttgttcattatatgcacactttggctgcaaagacatttttgttgcccatgattcattctagacatgtttgaaaccaataaaaatagataaattaagcatctaaaccatttatttgcgtaaaataccaaaaagttacatcaacagaattcgacgtaaacaaataaaaaactattatgaacgacaacacaaaggtcaagccacattatgaaaggcaatacaagggtaatgaaaactattcaaataaaatactatatgcaaactatcccaatatgtttttttgtttatatgacgtctgacccttcttacaggtcaaactcgtgcctaggaggccacagagtaatacaagaggggaattgcaacgaccagaacaaccatctgattttcagttcatgcccacacctgggattggtttagcaagtgctgcaaaatttgtgaactattaagatttggggtccatcttaataaggtcaaccttgttaagaggagtgacccaagatttatttaagttggtcaatatttcggtatttaaccgatgtgggatttattcccttaacatgtccccgcaagatggtggctttttttgagcagatcaatcttgaaatccgtgtgctcatttttgagacttaatcaaatcgaatagttcgttagagcttactgggctctgataccatgttaagacttggggtccatcttaataaggtcaaccttgttaagaggagtggcccaagatctatttaagttggtcaatatttcggtatttaaccgatgtgggatttattcccttaacatattgtcctccacttaatgagccagctaatttgcagatgccaaggacaagtatagaacttgaatccttagtggaagatttgcaagatataaagaaccaagaaaaaggattgtcggagggtcagttccatttgcaccaccaaaaaaatgcagaatacagcaactcagtagtaactatcagaattctattctagttttacaactgtgcagtagttctgtcgtacaagatagttgtatttttgtttttgtttttgtgtcaagacgctgaaactattaatgtaaatcagttccattttgcaggtggcttttcactaatgatataagactcattactgattgttttaatggatttttgtttgaacatttcagatgatttgtactagtgaatttttgctgatgtttttgtcttgatggcttattactggcaaatttattagttgattttcacttcatttgatcaatgactaaagttcttttctgtacgttgtgtatatcagctatattacgtcttggattatttgacactcttcatgttgttgctgacaacaattaggaaaaatcaccattagccccaaatgctgatgttctcattcatatattaaggctgtcggatgaacgggaaaaaccattatatcactgtgactaccaatttgataaccactgatttaacttcattgtagaagctgaatagaaataggaaataaacctttcacaaatacaatatcaaatttaagtaaaatttaagctcattacacataaatttcttaagacatgctaacaagtggggatataaattcatcactacctagaagaagatgtttcaagcattttttgtttccaattttgctcctgaagcaattgttatttctgttttagtctatctacttttaactttgatttccagaacattggatatagtacattcatcattccataactacgcagtgcatactacagaatattaaaggatttaaaataggatttatcatgaacaaaactcaagaatatccaggacttctagaaataatcaataggcacaacaacagacttaaatcagaatatttttatttttttcatttcaatcagggaaataactagtgcaatacatagtgccaatagcaacataccaaccgcactttcaaaagaacaagaatagcctagcaactacaatactaattattccctactttcaaacatcgagatcaactacatcacataaattactgtaatggtcttcactttgatcagtagccaaatccattaaacacaaaggccgattacaatgcttatcaccaggaccacctgatattgcttcatcaatttgctcttcctaaactccctctgctgcatatcatttgacctgtgaattaacccattcattacaaccttgtaccgtggatgaagaggtgggtcactacaacaaaaatggcattttgcaacacttgaaatgcaatatttgttatttgaatgttgctaactaaaaatgtctatcgcaacaaaaatgtaagtgaatattgccattggtaagcataattcacatttggtaccattttccaaaagaatgttactaatgtcgcttttttgtaacatttattgaatgttgcaaaaagttttatctttcacaatgtttattagctgttgttaaaagttcattatatagcaatactcgatcaccattgtggatacttagatatatagtttttaacaatgtttactttcaacattgtgaaaagtttctctcatttcaacatttaataaatgttgcagaaagttaaacttatcgtaacatttattaaacatagcaaaaaagagaaaattttcacaacgattaatacacattgcgaaaagttgaacttttcacacaaagtttattaaacattgcagaaagtaaaatatttcataggtgggttcgggttttgggttaagaaggtaagttgggttggattagttcatgggttggcccatgaaaatcggttgcgaacttttgggcccaaaccaaatgcccaatttatttatttatttacttttacactctagcccacattggcaatgtccaaataagaagtgaagaagcccaatacatccaagattccatcacaagacctttcgattttaacatttaaactattctttcttccacatctcgtcctcccgtctccacatccgccatttgcttttcatgaaattttttaaaaattagctatttaaaaaattcctaaagaaattcaaatttagcctttacaaaaaattcctcaattaactataatcctacttagaaagagtggacggaattgcaatgtcattttttgacctaggtattcacagtttgctggtcgggtaattggcgcaaaacatccttacctttcgaggttattgtggaaaatgtccctacctttcattttttggcatttttgcccttatttaccacctttcttgcgctgaaggtccttttcactgttttttgacgattttgccctctattcaaataaaagaaaaagaaaagaatagaaaaccaaagaattaattgcaactaatgccccaaatttttaaaaaattacaaattagtaataaatataagagttaatagtccaaatggtcactaaactttgtcaaaggtccaaagatatcattgaactttcctaaatacaaaaagaaaaaaaaaaaccaacaaaaaaaattgaagaaacgggccccaccaacaaaaaaggacaaaaaaaataataaaaaaaaataaggaaggtgaaaatggaggaaggtgaaaagtaaaccaaaaattattttttattttttcaatcgtatatttttaatcaaaatttattgaaaattttatttttagcaaaactaatctgtattttttttctttatttttaaaaataaaattttcaataaattttgattaaaaatgtacgattgaaaaaataaaaaataatttttgatttacttttcaccttcctccattttcacattccttattttatttttattattattatttttggtccttttttttgttggtggggcccgtttcttcaatttttttgttggttttgttggttttttttttttctttttgtatttaaaaaagttcaatgacctttttggacctttggcaaagtttagtaaccatttgggctattaactcctatatttattactaatttgtaattttttgaaattttggggcattagttgcaattaattcttttattttctattctattctttttcttttatttgaatagagggcaaaatcgtcaaaaaacagtgaaaaggaccttcaacgcaagaaaggtggtaaataagggcaaaaatgccaaaaaatgaaaggtagggacgttttccacaataacctcaaaaggtaaggatgttttgcgccaattaccctttgctggtcccccaaaccttattagtcgagctagcttctcaactggttcagtactgtgctacaaaactcttacactggatctgatagaaactggtctccactgttcaagaactagatccctactgttcatagcaaaaaatctttcgtatatgtacctattgtatttctaaaccttctccaatctctatctaatgaaacataagaaataagacgagccagcaacataggtagtgatatccatcggactcatccaaaagattgcgccctaactcactctcgttccattagaactcccgttttccttcatcgtagtagcaggatctctgttaggtaatattttattttattttattattattattttttttttggtgctgggatctcatttgtttcttatttttggaagaacaatgaagatcttgagttagctctggatagaatttttctctgtcgacgaatctgtgtttctgccggttattttaaatccttatatagataactgatttgccattttccttttactctacttttgtaattgaggctcgccatggtttcaacaatgtattcactttgaagttttggtcattttttcttcattgtttctctctaactttgcgggcatgttgttccttttttattctatctccctaattatcaacttatttctttgaaacttgatttctccttctacagcaaatagaatggttagtctttagggacatgataaaagggattatcttaactatagtgattggcctattgtagctgccataattgtaatattacatgtatgttttctttgtatccagtttggtaatgataatagttacttatggatcaatatgatttttttgctaagtttttatttaagatttatattttgttttctttccctttaatgttctcaacatttatatatggaaataatcacttcagcaagtattgatagaaagaaagagattaatcgtttaagtgaatggctggtcatagaaagtaggttcctacttggccatatatatatgtgggcttttatgcttgttctgtctcttgtcacgatgacattgttattgaaggtatcattggttgatttcatcatattgtctataaattgaattcgaatattatgctttcgctcatttaggattggcttaagagctcttctctgtggtgctcatattataactgatggatgtttgaaagcagctgctaagtggtatgccgtaactatattatgccttcaatctatgttatgatgttccatgttacttattatcaaaggttctagaggacttcttattcctttcccttatacttaatgaacatgatatcttcatgcaactgcaatatttgttcagtcattaaatgttagcttcaaacacggccaactatatggatgtgatttctcctttctaaaaaaatggaacagcgtagttgagattttagttctttaagcaggcaacttaccaaaatctggttataccacctctggcaagttgctttatgatgcctaattatatggattttcagccagtttggtacaatttcgtttgcattataaaaattcgaccaaatattctctatgacctctaaaaatggatgaatataatgaggaaaataaaacattcaaagattaggagaatgtgagttatatgaaaactgtaaatctttgaaatttatggttgacatgacccatgtgtaatggaatttagaatttaagggaataagaggaactttagctttattattgaatatgtgatgtgagtatataatattcaaattacgagatcaaagaaatacacattttttcctcgtcttctagttccatgttcaacagtttttgggtaaatttgagtcgaagtcctcaaccattgttaagcgtaacctttgggttcccaacgagtgtaacctttgggttcccaacctatcttttatatcatcaaacagactatcatatcattggttgattcaaagaagagaccacgtgagaaggggaggggattcattagaactctacaaatataaatctcttgaaaattgctctcttcaactttttttaacactatcattttatcaaatcccactagggcaatgagtggctctacttcttttaagaaagctttggctgccagattatctcttttcaaccattccctctcctagctgcaagtttttcttgagatgagttcttcaaagtacaaaactttgttggtaacaaatataattttggctatttttttagtaagatcttaaaggtactttggacaaaaaatattagcatataatcaagtatcacttattagtcaagattttgaaggatgctatcaataaaattccatcagctatcaataaaattcctgacgaatgagatattatgtatttctttattacatgtttgaatgcaaggaagacaaacatgataggcctccgatctagttcacctatgctagaagaaagaagaacaatgatcctaattgttttgccaagtcaattgagttagttagagaggggtagaaatgtaatagtctatgttaggaaatgcaaataaatgtggaaggtaaaggggtggggaaggcattgatgtactggtttttagttgggagtagggggagggacggggcctctctaatagccccgagcttgtatctattttgtttcttcacttgattctattaataaactactaattattctgtaaccttgagtgttagctatagttcaatcatttgttcctaacaaagccaagttatattattgtttttctctccagcaggagctcttccttccatcacagttggcctgcagtagctgggattgtatcaattagggtagaagtgagaatgttgaggccacaacgattgggccagatcgtggaactagcccaatgggtagaggatcgcaacgagtcccttaagcgagctgaagcttcagtcggccaaattagatcaagatcctctaatttggctccatcctattccagctcatttggggacaacccaaactatatgagtatttatccaagaggggtgactcgagcttcccaaatcagctagcaaactctaattacagccccctgataagtgcgcttttaaacacttattcggtccacaaagcatgactaattattgatgaaattgattggatatggcttaattctatgcaatttcttttgtaggaccatattgatggataatgaaactcaagagaaaagatacgaaaaggggccaaaacgaaagaaatcgaaagttcagggaccaaagtgtaaatatccaaaagatgacccaaaagacgaatcaagaatgcaaatgagcttttctctcatgcctttcttcgttcatagtagaaagattaatcagttatttctgattctaggggaaaaggcccgttgagttcttacagtcgtaggtccttcactttcattaaaaaaagttttttcattaattgttttcgattgttaagggttgggctaggagggatttgtcctagatccaaaatcgaaatgattcgtcccaaaaaattttttcgcggttatgcaaaaaaaccattttcttaatgaatccattcgagaattaaatcaactaagcccttttaggaatggagaaaattgcagaaaaccgaacaaataatatgggatgggataagagcgtaaaatataatattttattctcttaattattgtatttatgtgattatttgatatcaaaatgcactcattatacttatgctttgattcaggttgcattttggtagaaaatgtgaaatttataaagaaaaaaagagcgaaaagggaccaaaatgaagaaagtgaaaattcaaggactaagttacaaataatctaaagatgagacgggcgatggaatgatgattcgagtaagctaggagtccattgggtgtaattagaagtcaaaagaagttaaatatgaccataacatattcacaaatcaaatttcaaccacaaagatttttcagatttttagtcggagattgagatcaacttttgacccagtaaaagttcgaatttggaaagagctatttctagtaaaattgtagccttttgtgtttctttttaacgtactttgaattgccttaatcggacattgggagagagagtcatggccaatatactgaaagtagtcgcacatgactatttttggccgaatctttagtttcataattccgttcaaactcttgtggtaacttgatctcccacgaattttaagctctaaatcaccccaaaataggggagaacgcccccatgatctcctatctcttttctctcatcttgggcacaaaaactccacggaaggctaaatattttggtaaagccatgaaagatctcgatcggatttggggattttaacatctttccattcatgtaacatgcttttcattgttgaataattttaggatttaaatttctaccttattatacttttgaagtttgtttagcttttattaaattgttcatggattcaattatgtatttacattgaatgacgaaaatatttgttgaatttaagcttcaattgattaattgatgtgatttaattactattttatgcttgaggtatataatcgtttcctgaatcgtacttcaatgaatcaaagatgaatatgttcttaagaagcctaaattctagaattagaagtgaaatcaaattgatctaggtttttcttgatgaattggttttgaaagtggtttaattcttatttgatttttcattgaatcagtcatgctctttctatagtttgattgaatatttaatgaattccaatttcaattaatttcattggtgtgatttcttactgtcttatgattgatgtatatgatcgctttttgaatccgattttaataaattaagtgggaatatattataggaacctagatattttagtaagatacatgcatgattggtattgattgatacaatccgggagagtgaattctggtgcttcactaatctcacactttggtatttaaatttaattcaaattgataaattcttctcacaaccacaaaaaccctagtttgtcaaatcctttaaacaattcgtccatctccctgcggaatcggcaccccaaagctgtgctacaccaccgcattattctttgggcgaaatcaaattttagcgtcattgtccgggagacagtacaaataattgaaggactctcgaacaaaagggtgacttctttcctcttctactttttttagttagtttagtttattttcttagttattttgtaatttctaatctagtttcattttttttttgtgttttatgaacaggcattgagacgagcgaggacgattgattgcgaggcctcaaccagtgtttgaatcaccttcaaaccctctttttgatactacatctgttgacacgaatatcactttacataacacaatgtctaatagtgattacgatgatgcgccctataggaccttgcatgattaccttcaccccacacacacacctacaccgtcatgcatcatatttccacttaacatgccacgcatggatctaaaactgggaatgattcaacttcttcccaattttcatggtcttgaaagcgaaaattcatacgtgcatattagggagtttgaggagatggtaggaaccttccacagtcaatagggtacattggatgcaatcaggctaaaatgtttcccattttcactcaaagaacgatcaaaaagctggttgtattcactgcgatcgcgttcgatttggacttgggctgaaatgactcaagcattcgttggcaagtgctttccccaccacaaaacaactacattgaaaaagcaaatctcttcttttactcaaaaggagagtggaacttaatattaagcgtaggaaaggtataaagaattgcaagtcctctgcccccaccacgcttatgaaagctggagcattgtgagctattttttgagggattattacctagggagtgtcaatttgttgaaataatatataatggtgaatttttgcaaaaagatcctgatgaggctctaaactacttagatgacgtagctggattctcaaccaatagtcagcatcactacctatgatgctcggactcgggtgcgggtgtcggatacgggtacagatctaggagtcggattcttctcattttaaaaattaagatatggggatacggttaaaaaagatccgaattttggataccggtacggggatacgtcttataatttttttcctaaaaaaatgattcaattaaagcaaacaacaaatcatgtcatttacaataaataataaaacctttagagataacacctaatttatggcagtatgaattgttgacttttaaaccacttaattctttcatttctttcttcttcttttttttttggaaaaatacacttaatgaagggtagcccaactagttacggaaatttcttcatattattaactttttcattgggctccacttttttgcaaaatcttgaaaatgttgttgcaatccttcataaatttctacatatttttatcaaaagacgcaaaacaaatggttgttactgccacaaacgcaagctagaagcaatacttcaccgtccattgttttctcccttttccagccatgtccgagttcaaaaccgagaatccgacacatatcccatgtcggtatccatgtcatgtcgtgtcgacacgggtacttcgccatttttgaagagtccgagcatcatagatcactacatggaacaatctagcacagaagttctgcaccaagtttttcccacgtaccaagattgcaaagctaaagcatgacatatctgttttccatcaaggcgactcaaagaactttgatgaaaagcttggaatagttttaaaaacatgctatggaagtgtccacatcacaggatcagcaaaggacttcaggttcaatatttctgtgcaggattacttccagcctttaaaagcatggttgactcctcatctaataggccactaaccacaaaaactattaacgaggcactgaagctattcgaaacaatggctactacatcagctatgtggaaatcagaaagagtggttcagaaaaggacactaggagtctatgaagttgatgcatattcagccctatctacaaagattgactcgctatttcacaaagtgaaaaacatgtcaaaaagttgaacatataagagtaggcatattttgctcaatggggacaacgccagtaaaataactcgtttgggaaaacataaaatccaagctggaaaaaatgccctaatttctcttggagcaaccaaaataaaatatgccacagggtcattgtcaacaacaagagaaaaaacctcaactagaagagatgttcaaaaagttcatggaaaagaccaatcaatacatggaagccaataatcagagtcagtgccaacagtaagagaaaaagtctcaactggaagagatgttcggaaagttcatggaaaagatcaatcaatacatggaagccaacaattagtttatgagaaaaattgaagcctctattcaagattaaaatgcaaccataaaaaattcagagactaaaatcgaaaagatggcagttgctttgacttgcagagcaccaggtagtttgtcaagcaacacgaaaatcaacccaaaggatgttgagacaattacaactcgaagtggggtgcaactacctgaaatacacgtcaagaggccgactgtaaacatagaaacaacacctcctacagaaaaagaaactgtggagtaggatgaacttataaatgaatctactccaaaagaaggttcagggacatcacgggaaaaggcaatagttccagtcaacccttatgagactaccattctattgtcccaatggttaaagaagcagaagatggatcaacaatataaaaagttccttgaggtttttaagaagctctacataaatatcccattcatcgatatactagttcagatgcctagctacgccaagtttctgaaggacatcttatcaaataaacataagcttggggaacatgagacagtgatgtcaactgaagaatgcagcgcgagaattcagaaaaagctcccacctaatttgaaagatccagggtgtttcactgtcacttgtactattggtaaagtttattttgataaaactttgtgtgacttttgtgtgagtattaatttaatgcctgtctgtttcatgaaacttggattgggaaaggccaaaactactactgtaacgctgaaattagctgatagatctttgatacatccaaaagggataatagaagatgtgctaatcaaagtggaaaaatttatcttccttgctaattttcttttcttggatatggaagaagacaaggatataccattgatcctgggtagaccattcctggctatcggtagatttttaattgacgttcaggagaagcagttaattctgagactcgtagaagagtagacttcttttaatgttttcaaggcgatgaagttacccatagaatcacatatctgttcccaaataaatgaaattaaaaagatggttcagtacacattcctactgcacaacctatcagacgcttacgaagcttgcatcacacactctcaatcaacacattcagattctctagaaattgagatgtgtgcgagatttttggagaccaacccaccgtatatatgcaaaaggcattttgaggagtttggaacataacccacaaagccactaccatctattcagcagccgcctacattagaactcaagtaattgccacatctcatatatgcctacttgagggagtcatgtatattcccggccattatcttgaacacagtcagtgaggtggaggaagaaaaactgtttggggtactcgggagaacaaaacaatgattggatggactatagcagatatcaaaaggatcagccttccactgtgtatgtataagattctcattaaggagaattttcgattgagtatagagagtcaaaggaggctaaatttaaatataaagaaagtggtaagggcagaggtactcaagcttttagatgtagacatcatatatccgatatccgacagtgcatggaccaacccagtttaggttgtgccaaagaaagagcaaatcaaggttgtgccgaacgagaaaaatgagttaattcctaccagaacagtcacgggatggcgagtttgcatcgagtatcgcaaactaaatatagccacagggaaagaccatttttctctcccatttattgatcagatgctggagagattgacagaccatttacactactacttcctaggtgggtacttcggttacaatcagataccagttgctctagatgactaggggaagaccagctttatgtatccctatggtacctttacataccataggatgccctttggtctttgcaacacccctgccacatttcagaggtgcatgatgcaattttctcagacatggttgaaaagttcatagaggtgttcgtggatgacttctcagtctttcgatctttatttgatgagtgctttgaacacttgaacttggccttacaaagatgcaaggaaacgaacttggtattgaattgggaaaaattccacttcatggtacatgaagggattgtactaggacaccgtatatcagtaaagagaattgaggtggacaaagcaaaaattcaggttattaaaaaattaccgccacttacatcaatcaagggtattcctagcttcctaggacatatcagattttatagacagttcattgaggatttttcgaagataacaaagccatcatgcaatttgatgaaggatgtacagtttgagttcactgaggaatgcttgacagcttttgacattttgaaggcaaaacttacttcaacaccagtaattgtggcaccagattgggaattgccttttaagttaatgtgtgatgtcagtgattatgtcgtgggggcctttttgagacaacgaagaaacaaggtcttccatgtaatctaccacgcaagcaaaaccctgaacgacgcaagattaattatgtaattacaaagaaagaactcttagctatatagtttacgcctttgacaaattcaggtcatatctagtaaaagtcatagtatacacagatcatgccgcattgaagtactgatgacaaaaaaggatgctaaaccgagattgatctgctaggttttattgctacaagagtttgacgttgaaatcagggataagaagggtagtgaaaatattgtggtagatcatttgtctcaattggagcctagagagcctaaagagttaatagacatcaacgagatcttactagacgagtagatattcagtgtggaaggagcaccatggtacgtgggtatcgtgagttacttggacaaagccatctctctactagattactcaagtcaccaaaggaagaaattctttgcaaagttaaaatattacttctgggaggacccaattctttatggcagatcaaatcattcagtggtgtgtgccagaagaagtgcctcaaattctggaacactaccattcatttgcatatacgaggcactctggagcttcaaaaacagcagtcaagattttacagtcagggttttaccggcctacattatttagagatgcctttgaatttgtgaaaaggggtaatagatgtcaacacacaccgcgggatataatcgttgatgggaaagacatttatgcaatcaccagtttgagcaactattgagtaaatatgttctcaaacaccgtgtggctaccccatatcatcctcaaaccagcaggcaatttgaagtttctaatcagcaattgaaaaggatacttgaagttacagtaagttcttcaaggaaagactggtctaagaaattggatgacgcattgtgggcttacagaatagtattcaagacacccacatgcatgtctccataccgtctggtctttgggaaagcgtgtcacttgccatttgagttagagcatcgtgcatattaggtattgaaaaagttgaacatggatttgaaggtagtcagtgaaaagggtctgctataacttaacgaattggatgagttcaaagtggaagtatttgagaattcaaaacattacaaggatcgcaccaagaagtgacacgatttacatattcagaggctagagtttgaagtggggtagaaagttctactatataaatctagactcaagcgcttcctgggaaaactgaggtcaaggtggtcgggtcttacactattacgaagatgctaatgtatggagctatagagatcaaccatgaaaacaatggtactttcacagttaatagcaaaggcttaagcactgttggagcgatgaattttccaaggaaacgtctaccatccatctcaaggcaccagaataaaatagacatggaagagtggagctatcgactatacactagtgctggatgggaggcaacctattgtatccttttagtttattttgctttttgcattagtttatgaatttttcattttttagcatgtttgttagttgtaggtcgtcaatatccatataggtcacatggagttaaagcatggtatacacaaatcccaatgcattaaacacgagttgtgaacgttgaaatcaaattttggtggttgggtgtgagtttcacgcattttgacgcacaattaaggattttctaagtttttcaagatcaatgtgtaatttcaatcataaaattggttttgaaactaagttcacggcctacacgcttcccatatgatttaaaatgtgttctggcaagttttgagggcgatgcaaggccaattcgaatcttaattcgaaaatcgtgactcaaagatttttggaaaaagccagggatgtttctaaaatttctctacgtatgtgcactcatcacattatatgggcacgaatttctctgagaaaaaaattgaactgactaggtagtctatacaatcgcttagactaacctgttacgcggtcgcaggtcaagaatcaaattggccctgatcgataaccctatgtgactgcaccatagcactctatgcggtcgcatagaatgaataaaaacatatttcaaataaaacacacgacacatacatacccaccacacaacacgaacacattcacactccaatgccatctcacaactcacgaccgagtgcacaagcaacatcactaacacacacgacctaagagtgagtcacacaattgggacttcaatcctcaagaatccatcttcataggccgacattgattgcactccaattgcattccactgtcaagcgcacaaggtagattttctaagccctaatttatcaatttcgaaatttgggggcatcatgattctcttaggttgcttgatgaagtttagcatatgttgtgattgtggacattttgtgaggaagaagaagggtagattatcacatatgcattacaaaggataagaaaatcgcattatgcacacaaggtgtttgatagaattctaaagtgacgggtttttgtgtattcacttgaggtgattgatattgaaattgaattatgtgttgtgataaatacctatggaattgtgtggaaaacacttaacacccaagttgaacacaactaggcacaacaatggctaagacatggcatatgagctagagtagtaaggatacttttatatgcctggagattgctcaggaaaatttcgacttttctcgactatgctcagcagtgaaagtcctaggtaagtcatggatccaactaaacaaagtgcatatttaagctaagtttcgttggtgatttatatcttcatgatatgaactctatttgagacataagttatacaccttgcatgccaactttgttcacgtgcacttggaagcaagtttggaggctgtgccgtacatatgttcttctttcatatttcttcgttatccatttatactttgtggtctaatatgtacactttacgcctttggcaggatgccacctaaacgaacatccaagggaaaggaaaaagttgactcgtcattgggcactaaatgcataagagagctcaaagggggcgtaaggagatttctcaaccctgagactgcagcccaatgcttgaacattattagccattgggcgacacttccagagaggcctattaagttggatattttcccggatttgagctagttaccttgatctaaatttgtggacatgagaaagtggtagaatgacctcgcccagtctatgaaatcttagttagggagttttatgcaaatttcaatactgaaatggatactctagggtcagaacatttgcaccagacatgggtaagaggaaaatggatcatgttctcgcatgaggtcatccatgactactatcagctgagttggaataacttggttcccatcccaggcaatttaaattggcatgaggtggctgaggtattattggggtgggaaaatgcatggcccctccaaatagcagaatggcaccagattgagttcactccatctatagccattctatggctattcatgtgccacaatatcgagcccaccacacacaagacgacatttaatgatccgaaggttgggttcatatatcatctggtttgggaaaataaaattgatcttaccacctacatctacaagctgatacataaaatcgaaatttgagataacagacgatgttcattgatattcccgagccctatgatgctcggactcgggtgcgggtgtcgggtacgggtacagatctaggagtcggattcttctcattttaaaaattaagatatggggatacggttaaaaaagatccgaattttggattccggtacggggatacgtcttataatttttttcctaaaaaaatgattcaattaaagcaaaaaacaaatcatgtcatttacaataaataataaaacctttagagataacacctaatttatggcagtatgaattgttgacttttaaaccacttaattctttcatttctttcttctttttttttggaaaaatacacttaatgaagggtagcccaactagttacggaaatttcttcatattattaactttttcattgggctccacttttttgcaaaattttgaaaatgttgttgcaatccttcataaatttctacatatttttatcaaaagacgcaaaacaaatggttgttaccgccacaaacgcaagctagaagcaatacttcaccgtccattgttttctcccttttccagccatgtccgagttcaaaaccgagaatccgacacatatcccatatcggtatccatgtcatgtcgtgtcgacacgggtacttcgccatttttgaagagtccgagcatcatagcccgagcctaatcagtgggatttgcaggaatgcaggtgtcactatcccatctggggaagcacttgagaaatctagtccctttatcagacacaccaaattggaggctctagatagagctagggaaaaacattgggaaaagatggagaataagcaccacaagcagccgtaggacaggcgactgagaatgtagagatgccacaggtccctccaccagctattgatgtcgacacatatctattaaggtagatgtttgctactatgaccgggtccggccgagacattcaaagccttcagtaagcatttggggctatgagtactgaaatccaaccggtgtaggaagacatgcacatcacacgaaaactttacatcaaatgccagcagagtgtccctggcctcgagaagagaagtggacaccatgaatgggcggttgggtatgtacgtcgatcgggtagatggtttccagttgagagtaaatgagacatgggacaatttaggtagtttgaagactagggttcgagatatgcaagctgagcaggccagtagtctgagttgatgaggcagatcctgactcgactatctccaccacaggagacggcactgcgggtcccagctttccatcaccaccatattgatcagggaagtatcgaataacccatttttgtacttttattttgatattgtcctcaaattataccttttaaacttctacttattttcacattgaggacaatgtattgtataagtttgggggaggtgaatattggaatgcattaggaactatagatatggtgcagaatttgatcaacttgaacttgttgatgtgatacttgacaatttttttgcacacactcatattttacatgttaggttagtgattgagaccatgaacaaagtagaagaaaactgaaagccctccattgtattaacctataaaccaattttagtttagtttggagatggttgaacagttacaggggaactttgagataggtacgggtttcgtacatgagattttattgtgtcgattgcctagaccaataagatgaaaattaggttaaagtcttaaattggaggttagttttgaaaactgaatgatcctaatgtttttccaaatttcaagtcaagtgaattttgttaggcccccaatctggttcacctatgcttgaagaaagaagaacaatgatcctaatatttttccaagtcagttgatttagttagagagtggtagaaatgtaatagtccgtgctaggaaatgcaaataaatgtggagggaaaaaggagcagggaagacattgatgtactggttttcagttgggaataaggggaaagatagggcctctctaatagccctgagcttgtatccattttgtttcgtcaattgattccattaataaactactcattcttatgcaaccttcagtgttggcaatagttcaatcatttgttcctagcgaagccgaattataatagtgtttttctctcccgcaggagctcttccttccatcacagttggcctgcagtagctgagattgtatcaaaatattgaggcgatggatataaaaatagtacttgttagtattattgctctacatgtgtgaataattctttttgtttactatttgaatttcgaagatttgtatttgaagcatttttgtgcttacaatttttttgttgctatgtttgaattgagcatgttggacataaatagagcagaagcagctaaagtcattcttgtcattggaattatgaccattcatttttttggggagggctctagtgttggagtatcatttgctgcctcaggtaatttgtcttatttgacgttatggtagaataaatgcccaccaaattgcatgataatgtaaaacttgctaaaatgtaacagtttataaacaataaagttgggaatccaattttttctagaccttagttgataatttttatggaatgaaaactatgatgaaaaattaatgattgattcttgacaaagtaggttctccctagatagtaacaaaaagtacataatgctttgaaaaattaattattggttcttgacaaagtaggctttcttgatgcaccctagtataattttgccatcatttatatgtgttgatgcattcagcaagttcttgccatgtgctatgggatttgctgctgggtgcttgatttagatggtaaagttcaatggacttatagcatcaaaattaggaaacgatgaaggcgaaattgtccattgaacaatttacgatttttcttcttcttagatactagaaaatggagatagcaaagaagttagatgagttggatttgatcaaatttatcataagaacttgattgtgattttgtatttttgaccattgaaagtttcgtctcattttagcatgcaagaaaaccactccaaagacattatagggtttgtggaattttattattattattattattattattatcttgagaattgtattggatgtttatgtacttcacaattttggatctaggttttgtatggatatttttatgtattggagtcaatttaaatgattattggagttacttgatattgttatcttttatattgttttgtggttgatttgtataaatcgctccacaataaaaaaaaaatacaaaattaaaaaaatgtaaaatgacctatggcaacggtcaacaaaatgttgccaaaaaaaaaaaaaaaaaaagaatgtaatcatagacaatgggcaaaaaatgttgcaaaaagattatttgcaatactaaaaaatattgtgaaaaattatttgtaacacttaaaaattgttgcagaaatgttattcgcaatgtttaaaaaatgttgcaaaaagattacttgcaacattcaaaaaagttacaataactttattagcgatactcaaaaaatattgcaaaaatgttattagcgaagattcaaaaatgttgcaaaaaggttatttatagcattcataaaacgttgtaaaaatattattagcaacattcaaaaaaacgttgctgtatctttttactttatggcaacattgagatttataatatacgtccggacgttgtaaaagacctttggtaacattgtttgaacattgcaataagttgttttggtgtgatggggtccacccaagtgaaatactcgtaagcacctgagtggttgctgaatagattttcattacgaattgaaggatttgattcttcctagggtgaggtttcaactggggatttcagatttctctttctgtgatgcaattggaagtaaaggaataaatttaaaaaaaaaatgtttttttgttaaatattgcgtttttatccaccatttactgaattaaagccgttgttgccacaataattttcatcctccacgtgtaagttattgtccacctgtatagacggataaggccctagtgatggatgggtaatttaaagcatagttgagtgagcatttgataactatttattttttgatgagcaagtggtaatcaatactaaagttcagtgaacatctagccgtccaacacacttaaattggggcgaagaaaaagaaaaagagaagaatgcttcagtcggaaaaataataaggtaatgatgaatatacactaactgggttcttcaatttatgctttaacttggagaggtaaatataagaatgttgaattattttttagggtcatggagaatttgtttaaaatcaaaacttacaagaatcaaagattattgatatgtagttgaggtattaaacaagaatattgcggaaaaaaaattattttgggagattggtattggagtgaaagtaatatgaagtagatttacaaagagcttaaatatttaatttcgtagtgtgaatatggtaccaaaacatgctatttccgtgtaaaattctcacactggtactattatgaaactctatcctgaaagtgttatttttgttattcatttctgagacaatgtcaatatacagaaattggtgccaagtgtccaatgatccagtggtgctatatttgtcaatttacagtttgtatatttaaatatagaaaccaaacagccgaatcttgaggtttaggtgttgaaataacttatctaaaggtggtttcatggtttaagtaaactgcattctgaagttggaaactaagttaatttttattcttaattatagaaataatgctataggcacccatttgaaaggatgtgaattgtttgggattccgtcagtcaattgtccaatggatggattaaataataaacccaatttattttgtttctatatcaagagtttgtatggaaatcggacaagcctagcagcctacagtcggtcactttttaactttgcgtgcctggtcactttttaactttgtgtgttagttaaaaaaaaaaaaaaaaaccttatttatcaaaaattaagcagttagcccccggattgagaaccctttttgggatgtattttgaaatagtgattcttttgggagaatttgtggttaaaaatgagtgaaaagtgttggatttacgtttaaaattattttatgaaagtatgtgattgaaaataagttttgaaaaaaatgaattttaagaaaaatgagagtcaaatgggaacttaattgctttttactagctcataaagtttacataatttattgatttatatatgaattatatattgaatcatataagatgcgatggctaatcatttttgaattgtcgagttagacaaatatgattttttagaataaaatagatttataaacgagtagtccattgtcatagttaaataatttctttggcatattatataaatattgaatgtttccgcttacgtaaagttaattttataattagcaaaaagtacccaggtggagcttacccctctcttaacttcactggtgcgaatgtgtttcgactatgtatgatcagaattttagtagtcaagggaccctctctcgtacacatagactttggactgtgtactagggttcttatcctttggagctgctttacacatgtccaaccaaaattagtcgatacatgtatatggttattagggggtgacttttgttttgtttttatttttatttttatttttttattatattacatcttatcaaatttaaggttagagaattcagtttatgcaattaaagattttaagattccaacttatgcttgatattagtaaatattagatcatttattgttttacacttgcatgattagtacagagagatatgatgaataatcctatttgtacattcaaagatataccaaattgtttacctcctctcacatgcatgaggaattcgcataattaaaaaattttcaaaatgtgatctccactccctattgtgagtagtggataagggattatgttaaaaaaattgatatatatagcattttcccaatatgattccctgaaacagcaaggtataatttacaaataatatttattcgattttataacaatttattattatttaaaaaagtaaagattttgttaaaatatgtatagtaaggaaaaatataattattttgcaaactatctacccattaagttacaaactcatatatttttaacctgtgttgtgggaagaacggggattgaggtagggatggtaattgagttcatcggttcgagtcgcccctggctcggtttgaaaaaagctcgagccggcctggctagggactcgggctgagccccatttctgggagttggctcaagtcaggcaggctcaaaaaaaaaaaaaaaagaaaagaaaagaaaaagagagagagagagagagaaaggaaaacgtgtttggcaactaagagagaataaaaataataaaaaaaatttcaaaaaatcgagccagctgggctcgggcctcgggccttacaaagcttgagcctagccttaattttttagcggagccttacaaagctcgccttaaaagagcttgagccgagtctgagtcaggaatttcagtcggcgagccaactcggttcaactcattgacatccctaggcggaggtagtggggagctgggatgggctatagcccagcccaacccccagcccatatgaaaaattaagagtaatttttttcaattttggcccaaatattttttttagcgtagttttagtttaaattctaacccaaacttaatgctcaattaatcaaattttgttaaagaagccacaattattaaatactattttcatgatatttatgaaaccgaaacatctttttctaaattaggtattttatttaagcatgtttaactaaatttagttatggcaattaagtaaatttataatagaaattgatcacatctaaaaagtacttattttaatagttagaggcactatacactacatgttttgctaagctcaaaagtaattaattttttttttatttcttaaatgtttcatatattacgagttcatacttatgagaaaaaaataatttttttgaccatgaaatagatggtacgattgaaataaataacttgctctggatctgatcttatcaataaaaagaatattagttaaattttatttatttataaattaatctatatatacgtatattcttgaaactgagcaaaatatggatatgaattaaatctaatttcttaggatcctcataattcttagtcgattttttactttagatgcgattcctcactcactatgaaatgaagtgatataaataattgtcgtccatgccaaatagtaattttgagacaataacatatagtaatggattattaattgcgttctttgacaaagttttcagttgtttcaaaatgctagtcgttaaatttattagaatagtattcatttaataatttcataatttttcattggtggatatgtattatttgcttattaaaattatggttcggttagtttatattttttaaacgtaatcattgattttttatttggggtaagaaaatataaagagatttagcaggacttcttaggttgaaatatctagagttcttttatttcattgagtattgtatacactttgtcataaatgtcatgagtttagcttcttgttatgtgagttcattcgaaaattttaaatttcaacccatcctaatatcatttctcggaagaagttgagtttgagtagctttaaaagagcttgtcaatttatgagtagagcaatacgacttagataatttgtattacccaatttgttatactacgtggtcactatctttttaaggaatatgcatattgtcttgatcatgtcatcgggtctaacgacacttcaaactaatagattgagaaagatattgataccaacaaaaaaaaaaaaaaaaaaaaaaagttggaggacgttgcaacaaggtctatagttgagggattaagggtgaaaattttccatttataggattaatctccaacatattaaaagggtcgattgaggagaaacttttgaatgtcaattttacccttatatatttagctatatgacaattctaccattatatatttaatatagtaccatttaatataattttattttatttaatatccatttaagtatagtgtttaattttttatattggagcacttggaattttacattaatcaaattaagtttaagtacttaaattaaattatttaaattaagttcactacttaaaattgaagctcacatacattgatgtaattttattataattatataatatactataatttactaaatgttgcattaatataatagtggattaattaaaatataaaattatatttattatagcttttatataattatatatgtagacgtgcttcaattttaagtattaaacttaatttaactaatataaaattatgagtacttcaatatgcaaaataaactctatacttaaaaaagagtttacataaagttaaagtttaattaatctattattaatgtcacctttaacatattataatattgagaggtaaaagttgaagatgagaaaaattatccatcaatcttaaaaatcttactaattactcctaataattatgagttacttacctttcccatatttgtatccaccccactaaatacaagttttgcatctcaattacaaaaatttcactaaaatcagtataaataaaaattaatgctatgtgttctaaaaaataattaagatagtactaagtattttattcatgtttatttttgaataaacataaaaattgattgtaatcaattacttattagatataaatatataaagaaagaaaaagatttttatcatgatacatttaacgggagaatttttattcttccatatgtattaatcccattcaaaagaaaaaagaaaacttttgttctaagatttttcacttctatatctgttttgaacgtaactttggtttttaatttaaaataaatgctatggattaatatgactagcatgattagtatataaattttttttctgaatgtgtttagataagataatcttttatttttactttttacgataaaacagtttatattacagacaaaatgagtaaatttttattttgaaaatgtacgcttagtttacttgtaagtaaacattttaaatttagtcatatatacgtttcttaatttgattcttcttggtgttcgtctataccacaaagttgatcgatattggtgtaatgtttgaaaatatggtccaaccaatgtccagcacaaaacaaatgagtaaataaaatattacatttaagtttattaaacattttcacattttgtacgtaaatttcataaaactctaattcatatacatatatataacaattttaactttttctttaacattatcaattacctaactttaaaaatattactcatatcattcattcggtacataagatttgcaacacccgtgattactgttagtctcaaataaaaaacttgagcaatactaattcattctcgtcgtgaataaaattctattcttattcaagacaacaataaaggaaagaaaaacaaacaatcatgtttattcgctcaccgtgaataattaactgctcacaatctaagcctaacaaaaataaaattctcagaagagttttaaattattaagaacgattcaatacgaataaaatattcaatatatccctcggtcgaaaacagtccaactgttatctacagtgggaaaggcccattccgttgttggtttcggtttccagttattgaatttaattttgcaggtgggcaattgacagaacgacaagccatgtcatgctttactcaagttgcagatataaaatattttttcatatgttttgcagtccaaaactgaagctgattttccgtctcattaacattaattaattatgtattcaggtagttggctcactgggttttttattcttcccagtttattgtttaagattaaaaatccaacaaattcacaagccgttttaaaacctcaaatttcgaaattaaggtttaactactcgacaaaaattagtaaaaaccaaaattttatgatttgtgattgcttccaatcattgctcgggcagctcacagcatgcgttccaaatttccaactagtattaaaatgtcaaatatatattaaatctatatacataatataaatgattaaaaaaaaagatatttagttatgacaatttatttatcctctttttgtttgttatataatatattataagttctttattacaacggtcatttttcaatagatataaatatgtgcatacattcaagtatttgatttgacattacattgataacgtcttaaaagcaacttgtaacaaccaaacaagaaacactgtgtgagtctgattacagcttataacgtcataatttattaagcctattgaccattgcagttacaatccacttttaattagtcaaagtcaataatcattcggtcaaattcaataatcatttggtcaagtctaagtcaaattaaggatgagaattatttcatacatattcttgtgggctattttgtaattataggaatattggttgatgttatgccctggttgatgttatttcatccacgtgcactcgtccacactaaagcactgaatttggatgtgaaatgttaggaaaactttgttgctttcattgaaatgcttagtgtcatgcattttcttcttcccatgttaaaaatgtgcttatatttgtgcatacatgaattgtgtttatgtatacatttaatgtgcttatatttgtgcatacatgaattgtgtttatgtatacatggaaatttatacaaatgtgcgtacttgagtttgcaattcgaaacgattaagattaatagatacctgcatgaaaagttcttatttttgcctctttccttatggtttaaaatatatattattttattcatttagtaagtaaattttattttattttatttttgttcttttgtatatcaaaatttggctacttgaaaactgtcgagcaagtttcagttttcttaggacgtgcattaggatgcgaaacgagatcggacaaacgaaaaagcagagtcattttatttgcttatatttactggattgtaacatgttgttttataaagctaatttttataactaagaaatttatttataaaatataaaatcacttttgtgtacgtaatcagttgcttataaattaaaaatactattaataagataaaaaaatcacttataacatatataatattacttattgtaaaaaatcatttatgtataaaaaattgtttaaaagtacaaaattaatttgtaattttaatatttacttataaataaaaaaaattactcgtaatttaaaattttaattatatataagtattttagtttttaaattaaaaattaccttatatgcaaaaattactgataaataaaatattatttatgagtaaaaaaattcatacgaaatttacatttagtctaagtcaaccaaaatttcttagtcatttttgtatttaacacaaataatgttacagtagccacaaatgaatttgtaaccaccaactaattatggaattgaactaattcaaatgcaaattaactatagaattgactagaattgaaatctatgaattgttgttacaatttcattattattttccaacggtcccccacatgaatgaaattaacaacaatgatagatagacatgatgataaacttcactggttgaaacctgtatagaataagtaggtgttaccctttaaaccttccattgtgtaagtatatttactttactaactgattagtagacataatatccatgaattattctgccatttgtgtaaacgaagacacaatccacacaggcttctttctaatacaattcagttctcatagttcattttggcaatgaatatttccctggttctgtgagaaattctaagaactgagccctacacaatttccttagaaggggcctcacttctctctcacatagatttgcattagtttgcttggtcttcgatgcataagaaatcattaaaagcttgttgtctatccttcatccgtacagacatcactgttacatcaaaggaatggatatgagattatatcatccactatgattcaattatgttttttaccactaggttgtctctttaaacctagatcttaggatcttccatcaactaggttaggtttcctttataataactaattcgttcaagggcttaagtcacattcctttcgataatttttcaactaactttctatttacccctttggttagcggatccacaatgttgtcatttgaccttattaatcaatagagacaacttcagttgacagtagttgccttatagcattatgtctacgatatatatgtctagactcaccattatataagttattttgtgtccttcctgattgactatcatagcgtatgcaaattactttgcataggtttagaccatctcgaaatatcttctaagaagttatcctcttcaccacatttatctagagctacgaacttagaatccatggtagatatggctatcactatttgtttagaggatttccatgatatagctacacctcctaacatgaacacaaatctactggtggactctgagtcttttatatcatgtatccaattagcatcactatacctttcaatgactgctagatatatggtatagtagagtacataaaaacaagtatatcttaagtactttagtgcccttactattcctgtccagtggtcagcttctagattacttgtatatctacttagtttactaactatataggttatgcctagtattgtgcaactcatcaagtacattagacttccaataattctagaatattctacttgagagacactctcgcctttatttttagatagacgctgacttatatctattggtattctagctatgtcaatatcatcattgctaaacttttcaaaaaatttgtccatttaatgtgactagcttagaatgagtccttctaatgttctagtaattttaactccaagcatcacatcagctaaagccatattttcatgtcaaatctccaattcaacatgtttttagtagatttaataatctttattgtcgttaccaataatgagcatatcgttaacgtaaagacataaaatgacgtatgatttcccatgtctttgacataaacacatttatcaaacttgttaataagaacaatgcaatcttatcaacgtaaagcgttcaactttatgtattaattgtgaatgacatattttaatcacattacgaattatgtctcactatactcgaaccatcgattatacaacttgtgacattctatatgatcatggtaccttagataatcattgaaaattgtaacatgcgaataatcgaaagccgattcataatgtccttttacaaaatattactcgaaaatggcatcaacctaacaatctcccacttgcccttttagattatatgacatatcaagaataatcatctccttaagatgcccatcaaaaaccttagctggtaaggttttggtggacaaatccgcaagattatctgcttatgcaatcttgccaaccatcacatctcttcaatgaacaattcctataacaaggtaatattttctttcaatgtgcttaccacgttgatgactccttggttctttaacgttggcagtagctccactattatcgcaataaagtgatatgggttctattgtgaaaggtacaacgtcaatgtccaaaagaagcttcttgaaccatacaacttctttagcagctttaatagactttttaaagtcatgatcggattgaaaattggaatcaatatatccaataagattcaaatcatgtcctgaatagacaatcgtataatctctcgttctcggaaggtacttgagtatatgttttgccattatctaattttctggtcctagatttgatttacaatgactaacaatacctacagcataataaatatgcagtctagtgcaaagcataacatacatgaggctttctatagttgaagcataatgaagtgcaaagcataacatacatgaggctttcgatagttgaagcataatgaaccttctccatgtaatctatctctgttagagtctttttagaatgctccttagatagatgaactccatgtctaaaaggaagttgtaccttttcgaaatttcgcattgccagtttaaaaaatattttgctatatatgaagctcgggataatgctatccttctgtttttccaatctcgtaagatatgaattcccaaaacataactagcttctcccaagtccatcgtatcaaacttctatgataaccatttctttatagatgataatgtccctacttcatttccagtgagtagaaagtatccaaataaagaatcagaaaaattattttcttcccctgcatacgcttgtatacactgggtttaaccaattttggtcaaaaccataagtcttaatgttttgatcaaatcttatattccaagacctggacgcttgcttgagtccataaatggacctctataacttacaaacttttctttcatggttttcttttacgaacacttcaggttgcgtcacgaagatggtctcataaagacgtccatttaaaaatgctatcttgacgtccatttgcaaaacctcatagtcttaataaatggcaatggataaaaggatttgaatagataagtatggaaacccgtgagaaaatttcttcatagtcgataccttctttggttaaaatccttggttactagccttgctttaaagttttcaaccttcccatctattatagacccacttccaccctataagtttgactccattaggtacatctacaaaatcccaaacttgtgggaatatatagattccatctctgagttcatggcagatttatatgattcaaagtctacattctccactacttctttaaatgaagtgggatcttcttcttgctcagtagagatcgcctgatatgactctccataaagaaagtacctagaaggtggtctcacaaacctccgtccaagaaaagtggttaaatgtgcctgattgtccagtctgactaaaggtccttcctttcttcttaccgtttggtcctatccttggttagggccaaattcctcattatctccattttaaggggcatgcgaaggcataacaatgggtatctcattctctactatctttggttatgtttttccatgaggttctgtgggcatctctagatcacttacctcatcagcaaccactggtcctgtagagggtccaagtcatcactatttgattccatacgaaaatctggaatcgagtagtttaaaccatgttctaacatcttttccaatcgaattttactagtagacttatattcatctatatatgtatcatctaagaaggttacatttgtactaacaaatacattcttatctagaggactatagaagtaatgccctctcgttccttttggatattgtacagagagataaacctttgatcttgatttcatctaatctatcattcccttgagcatgtgtgctggatatccctatattcgaatgtggtgcaaattaggcttttgcccattctacaattcaagaggcattatgggaattgaattagatggtacaaaattaaagatgtaaatggttttttgtagcgcatatcccgaaaaggaattaggcaacgaggaataactcatcattgatcttaccatgtctaaaagagttcgatttcttctttttgagataccattgttaggaagtccttggtgcacttagttgggataatatcccattattcgataagttgacctcaaattatcgagatagatattcaccacatcaataagatcaaagggccttgatacttttacccaattgttctcaacctccatctgaaactttttgaatttctccaaagcttcaaacttgtgagacataggtatatgtatccaaatctagagtaatcatctgtgaaggtaataatgtaacgacccgagtccctgtacccaagccgttagcttacgtactgtccactttgggtggcctacttacccctcatggctttctgtcccatctcccaggattcgaactcataacatttcccttaaataagacttaagttgaatccttgtaacaacctgggtcactgtacccaagtcgttagcttacgtactgtccgatttgggtgggccttgcatccacttacccctcacgactttctgtcgcgttccccaggattcgaactcataaccttccccttaagtaagacttaaattgaaccctggtaccaatgggacaagttaccaaattggtaccagaattcaacttaagtcttacttaaggggaaggttatcagttcgaatcctgggggacaagacagaacccgtgagggataagtgggcacaagacccacccaaagcggacagtacataacctaacagcttgggtacagagacccgggtcgttacaaataaattgctcatatcctcctctagtcagagtactaatggttacacaaacataggaatgtactaattccaaaacttatttagcttttagtcccttagccttgaagggcctcttggtcatctttcatttcatatatgattcataagtttgtatggattctatctctaactcatttaaaggtctatcatttaccaatctttgaatcctatttagattaatatgacctaacctaagattccataagatagtttcattagtactagacgacttttttctttttcctagcagtagtagtattatgtatagataagacttaagacatggaggctattaatcatgtgaaccaaacatataacataattattcaactagataaccatagttgaaagggtaaaaagtaccaaataactaacacgatataaaagtgcaatgaaaaccaagtttcatgtaagttcaagatcataaaaatagttatccgaaatcgatgtccacaattttcaaaatataaagtaaaggtgccaacaactttggcagataatactacttctgtgcaaactctaagagtgtactccccttcactgaggtgcttgatttcttggaacccctgcaaagaattacgaaaatgattactaacttcagaatcgaccacaaaacataactcaatgaatagggcacaacctttattttgctttcccttagataggtgatttgggtaattcctcttccagtgaccattttgtctaccaaaaaaaaaaaaaaaacacacacacacacacactttccctttagttttccatcgatagtagttttcttcccttttgacttgctatctttcctttgtttggcctctttctcttattttctcctttgtcactaaaaggcttatgatgagaggatctgactgttacaattacaacacttccacttctggcaaatataaacaattattgaaagcccaagaatagctaactaagaggggtgaattggttatttaaaacttttttgaaaataatctcaatcttaaaaaaataacaaataagttaattgcatatctaagatagcatgaataggaaagtaataagtaaaagagaagagaatgtgcaagcgatgtaactatggaggttcgatccaatcaacgatctacatcctcgttatcaagctctctatactatttgtcgattgacttatggcgtaatccaaacctcatagcgctttcggtgacttacaaccaagaagcaccgattcttttacaacattgaaattttcgagacttcaacacaactcacaatcaaacaaaaaaattacatgtaaaagcttatctcttaataaataatatgatcagttaagtattaaaagagaggtaggctaacacttcaataaataacaatgagtacagttcaagtgttagtttttctaaaaactttaatgagataaaagattttcacaaatttgatcactcaaaaatttttcaagaaataaatattttgatcttctaatcattgaaataaaatagttgagatcaataaaagcctcacttaaatgctaaaagaaggttattgtaaataaggaagagaagtggtatttataacactcaaacaggcaaaaattttgtccatccggacgtctggttagggtctggatgtgttaaaaactagctgtttgaattagatgtagaatagtaaaaaaatgtgaccattgggtatcgagacgtctggattaccattcaagcatccgtataggaaaaaatgcccccggatatttttccttcatgatgaatttgatcaatgtagattcttgaaggcctttctcttttattttgtgaagataagtgtttttgtaaatatttgattgttgagtagaaatacttacctttaaatttaatttttatgcaaaaaaaaaacttttgtaacgtgaatttgatcttgtgcataaattattttgagctatagtcaatactaaaatttgaagtgttttacctttacatataaattcaacgcatctacatctaatatcttgaagtttgatgatcgatcttttctccaaggtgatttttgacatgaatgctcgattttcatctctacattcgtcaatcgtcaaatttggttccatgttgatcttcaagctcctatttcatttgtcaatatgcacgtttcttgatcttgattttcgtgtctacacttttgttgattttgcagtaacactatcaacaatcgaaatcaacttgttagaaataaacgtagtttgtttgtcataatcaaaaagagaagtcaaccatttaggtcaacaatttccttcttttttattattacaaacaagatgatttttaatacaaacattaaacaaattgatgtgacgcgaatttacaaggaatttaaattttgaatcttgcatgtatattccccctatctttttcatttatatttctcctatcaacatgcatttatgagttcaacatacaaattttataagttcagtataagttttccctatttagcataaccgtctacctatctttccccttttggcataagcaaaaagaagtaatatcacaaattaattttgcgaggaagtcaaccataggaaattgattcagcgtataccatgcattgacataactctaaagcttgataaaagttatattacaaaaacatatgacaaatgaaaatgcaaataaataaataaactaaggcaccgaaggcaggaaacgaacataaaaatccacaaaaaatgcgttctgatgcgcctgtatcttagcctgttggtcttggatggcggtctgctgtgcttgaatctgaaggagtaggctaccaagactatcgatgaaggaggtgagagaattgatgcgctcgtgaaggaattatactattctttggtgaatgttgtttcgcgcgggttaattcgctaacaattaaagaggatcagacgattgtgtaagggacgaaaacctcttgagacaaagtcccaaaaaggggtgttctttttattggcgatgaactttacaaattggagacggaaaacaacgtgcctctaaggggcgcaagcacacgagttacagaaagggaaatgtttaagtctaaaagctaaaggaatgaaaattacatattctctgttcgagagtttttgattcggtccttgcttctaagttctttctcccttttatacttcataggcgatccctttgtgattaactgctctaaaaaactgcttgatcgcccaataactacccactttctttgtaatggccattttgtcatacaactgtcttttaactgctgccattatcttgcatcgttcaactgctttcgattgaaccccttgagtcgtggaacgtgatgaaattactttagcaactgccttaataactgcatcataatgcattatgtttgttgataccttgggcgacttgaagatttgggcgagactttggacgaccgtttgccactccattcgttcagattctgaacgacttgcaaacttgggcgatggcattaccgcactattgggccccttatttgggcattcaccttgattcattcaattggatttcgttctttgggctatctgatttggggaccctctaattagactttactctctgggcttgttcgatttgggctgaatttttttatgtgtcaacaattaccccccaatatggcagaattaataataactattgaattttgccatattcacttcacgtcttcagcaacgttcacgatccccaaagaattttaatcattgtctccttctataacttgaaaaggtgcgtcgctttgcaaacccttataaactccaaacacgtcattttactgctacgaaatcacgtttcatatttcttacgcatccttcgcgattcactgttcatattttgcttccttgttacgtaactctgaaaagcttcgttccttcttcaatggctgctttacaatcccaagctagcgattcctttagttttgacgactttcagaaacttctgagtcgtccatacgtaaccccaagttttctttcgcccgctgatgttggacgtaatgagttttacttgggtcctttcttcaacaatgcggaagcaatcgatcaggcggcggtgggccagctgtttccttgcacccatggccctccttttctgaattctttgccgctggggccacttcgtgaaaaaggtattcgcacttggcccaaacctgacgtagcttttcgtaggtggcatgctcgtcttgtgggtcatggtcctactaaggcactttttgatagcgctaggatttctgatttgttggaagtctctattcgcccccctgcttttgattcagcactctttccgattgctttgagcttttggtcctctgagtataacacctttatctttcctcttggccccatgtctattacgttaagggatgttggggctctagtaaatttaccacctttgggtgataccgttttcccgggcatcttagtttctggtggcgcccctcagttcggtaaacactataccgattcttattcaagcctgcagacactgcacaatcactcgagtgctgaacctactcatgctgagcgagtggccttccttttactctggctttgtaaatatgtgttgtgcgtgcctagtataaagccctctctaagttatctgcctatagtgcatgaactggcccgtggcaggcctttgaatttatgttctttgtttttggctgccctttatagaggtatggcttttcttcagactcaattgaagaatggtgcatctcctactggcagtggacctctttggttcactcagctgtggttgagatcctattttccatcgcttggtgctccatccatttcttgtccttctgctagttgttacgggctagctatggagcctttaactcccgtaagtatgtccaaaagggacatttttttattcttttattctttaaattcaatctcttccttctttcctttccctccttttttgactccggactatgtacatcctccttccactctagatagcgcgagcagttctctgctcatttggattcagttcttaactgggagggagcttttccacgatatcttaaccgggaccaatgccaaagctggggtagaaatttatgttccccaattttttgctcggcagtttggtttcggccaaacttggcctgttcctctttgctattcgaagaacttaaacgatcgctttcataccattaataaggtggaagcagaggctataaacgttcgcaacctccacttatccagccatttttcattagctccttttaatccttgtcatgctactcatcctcttttcgaacaactttggccatcggtgaagcgcagattatttgcgactgaggccaaccgtgcctttcattcattagatcaaccgagtatttcttctcctcctcctgttttggcccctcctttgtctattcggaacccttctccttctcgtcgtactaaacaatctgctcgtccatcttcttccctccctgccaagccaactatggccaagagtgttccaagccgcaaacggccagcttcagcatctcccattctggaggatgatgttgatgatgatgatgatgatatccctcttatcgttaaaaggaaggtatttaaattggtctatttataagtatgctcttccctatctgaaaactttttgtgtactgatgatcttttggacttttcagaaaagctcagtttccccttcaaagcctttggcattaccaactcctattccatcatcccctgttaaggctacctcatccaaaccggttgatgatgggaccatgcttaaaggtatatcttcagtcccagattcttcatcacaactcatgaatgagccaccttcctcccagggcgtctaccccccaatcaccgaagcagaaggtagttcagttttttgatgtcttacctttgttcgtgctattggtttctgactggttgctctttgaactttgtagatactcccatgagtccgcccattgtggcaacgtcttctcgctcggacaagaggaaatcttcacaaatggacgagttattggtggccagcttggctgagggtgcaccatcttctacgatcgtcgacgaggtaacttttctctttgccccattcctatttccaacttgttcgttgcaacgaatatttttaatgttggcaatcttctttgcaggatgctgacaggattgttcgttctatccaggatttgtttgcttcttgggggcaggtccaaatgcctcgccctactccatctgatcgtcctgctgcttcttcagaagaggacttaaagttcttgaaggagttggtatttgagtacgtgtctttcatggacatggacatcggaagggctaatgttgccaaacacaaggatgaacttgaacgcttgagtgcgaaattagagcaagcactgacgcttccgtcgctcaatctttctgccgactttaaagcgacgttgaaggtcattcactccgaggtccttactatgttggccaagaatgctgaactaaaggtcaagcgtactcaatatcttcgagctgtagccgagaaagagtctctgtgcttggagatcaacaaggctaaggacgagttgcaagagatctcttccgaagtcatgattgaagactccttgatggttaacttggctgctcaaatgagggaacttcaagccaaaatggacgattgcagggcgaggatggccgctaaaaagcacaacgcttctcaggggattgagcgaactaaatctttggtcaaacaatacaagaagctggaggttgatgatgatgacatcgccgctgaattgaacatcacttcctcccgacagaacgaggattgagaaaaacttagggaacaaattcgttccttatggggtagtttgtaattaagacacatgatgtcttttttgtacatttgtcccttattaatgaacattaatttcttgtgcttttatttgatgtttattttctaatcatcaattcttcaagcatttaactgctttgcattaagaattttgtccattcccttttgatattcccactactgttcccgagacttagggccatttatttccgtctataggcagaaatgtggctgttcatattctgtctcttcatcttcgcccccttataaatgtttagcatttttcatcttctatcttcacctcctcattttcttattcgaaaccaatttgctgccatttcttggcattctggagatcaatctgatccgaagatggactgtttagtccgtccgccttacatttactttgatgtcgcctttggtatgggaggtataggaaatgttttctggcctgcagtgaagttttttcctgcaaaattcttcccatcgtctctttgttctcaacaaggagtcaatgatggaaggcaatttctaggttgctcacaggccattttgcttgctgagagtgcttctcagtttgcctgctgagagtgcttctcagcctatttgctcgctattgcagcgatgcatttagaaaggtagtgaggccagtacaccctctcactcgtcaatcccaccaccgcagcggtgcatttaggaaggcagtgtgaagcttactcagtgatcggctaggagatcatcttactttagttgtatcttgtaacaagcctattacttgtatcttttacatccttgtaatgaacgtttggtaataaagaactttacttgaacgtatttcgctctgtctttattatttttaatcgtccagaatgttcggttatgtttttatctgttcacatcccataaagaaggaacatattttttcaaatatttgccattaatgaatcttacgtgcttggtgccgtctaaatcttccaagtggtatgctccattaggcaatacattgtttattttgtatggtccttcccagttgggcgaccacttcccgtactttggatccttggtgtccaaagggagtattgtcttccaaactagttcatctaggctgaatgacttggctatgacttttttattataaaatttagccattctttgcttttgaacttgcaacctatccaagacgtccaacttcagttcatctaaacttaataaattttgaactagcgattcggcatactcatcatcattcaacttatgttgtaagcacactcgaattgattgcacgttgatttccataggcaaaacggcctcctgttcataaacaagttggaaaggagtaactctggtacttgaccgaggcgatgttctataagcccataaagccatattcaaacattcgtgccaatttctggcgttttcctttatcatctttctgatgatattttttagaatcttattagaagattccacttgtccgttggattgagcgtagtacggtgtggagtttactagtttaaccccaaattcgctcaaaaatttgtttacttgaaccccattcaaagatgttccgtgatctaccattatggtttgtggaattccaaacctataaataaggtgatcacgaataaattctataacattcttctggatgatctcttttaaaggtactgcttctacccatttagtgaaatagtcggttgcaactataacaaaagtatgttgtttggacgatggagggtagatcttccctattagatctatcgcccaacctttgaacggccaaggtttaataataggtgccatctctcgcgctggcgccctttgtattggaccatgcttttggcatgctaaacaactttttgcgtactgaacgcatagttctcccatctttggccaaaaatatccactcctaataattaaccatctcatcctttggccagcttgatgagctctacatatcccttcgtgcacttcagccatgatcgtcttggcttcttgcaaacttacacactttaataatacaccattagagcgtttcttgaataactcttcgtctattagtgtgtaattcagcgaacataactttgtcttcctactaattcttccattaggttcttgaaggaaccctttaatctctgtccgccaatccactgcatctccatcttgtatacagtgaagttcaatttttctcgcccttctttgagttacgggcaatataatcccatattcgcaagtagacttccaattcaagattttagagtaccctgaagccatttgggccaactcattcgctacatcgttatatattctattaacgcattgaagttctacttgatcgaattcctctaataattcttgggcgatctcgtattgacttataatggaatcactttggcatttaaaatcaccaatcaattgatgtatcactaattgagaatcgcccttaacaatcacgtttcttacccccatatctatcatcagttctaagcctacgattaaggcctcgtactcagcttgattattggtgcacattctgtctaaggtgaatgcaaatttatagcaaatccctaaaggattaattagtgctactcctactcctgcacctttagaggtctttgacccgtcgaaatacaatacccaaggttttagtccgaacgagttgatttctaattcgatttcttcaggcatgtcaaggcatggatgatcggctaggaagttagccaaagcctgatttttgactgccttttgaggtatatattgtatttcgaactctgataaagttaatgtccaaaggcctaccctttggtgtaaaatagggcgtgagaacatatatttgactaaatttactttagaaattaaataaacggttatgggccgtaaataagcccttaattttgtacatgtgaaatacagtgctagacacaatttttcaacagcagagtaattacattcacatttcgttaaccatctactcaaataataaattgccctttcttcaccaaattggtcttcctgtgcgaccattccagctattgattccttttcagccgatacatacactttcattggccatccctggattggtgacaccaatactggtggacttgatagatatgccttcaggctttcaaaagccttttgatgttcttctttccagacgaattcgtcctgatttttcagctttaatagtggcgaaaaaactttagttcgccctttacagttagaaatgaagcgtcttaaaaaatttacttggcctaaaaacctttgcaactcctttttattgctaggtggtttagcttctaagatggccttcactttgtttttattatcaagttcaatccctctcttgtgtactaaaaaaccaagaaagttccctgcattaacaccaaatgcacatttcaagggattcaactttagcttatattgcctcattcgttcaaacgaacattttaactgttcgaaatggtctttttctttaatagatttgactactatgtcgtctacatacacttcaacaaacttgcctatcatgtcatgaaagattaaattcattgccctttgataagttgcccctgcattttttaggccgaaaggcatgaccacccattcaaaacatcctagagacccagggcatctaaaggcagttttgtgtatgtcttcttcagctatataaatttgattgtatcctgaatacccatccatgaaagaatacatgacatgtccggcagttgaatctactaaagaatccaccgtgggcattggatactcatccttgggtgtcgctatattcaaatttctaaagtctatacacacccttagtttaccattcttttttaatactggcacaatattcgacaaccattcaacatatctggctgttcttataaaacctgctttcaataatcgctctatctctttcttaatctcggggagtacattaggagcaaaacgcctaggaggttgccaatgaggtttaaaattaggcttagtcggtaacctatgttccaccaattctctatctaaaccaggcatttgttcatattcccaagcaaaacaatctttgtactcttttaacaaagcgattaatttattactaacctcttggtcgagcatctggctgatgaacgttgggtgatcttctccttcattgccaatgtttactttgatcagagggtcttgtgcttgagcgtatccaggtttggcaatccgcatcacttcgtcgtccagttctcttgtatgtatttcctcttccaaacagtccactttgttgacttctcggccaaggctttgctctaactcgaatactgccaacttgtctttcaacgcttttagggcagtctcttcctttgctttgtcattgcattctttattgaaaaccaccagtctggctttgaaggcctgaatatcggccattcgcttttgcaattcagaatccatttaagattccttgattattcttttgccaattactggctcttctaaggccactatgtttggcctcatctgtttgaacatctcagtgagtgcgtccactgagaatggttcttcgctctgtgcgacaacttgagtttcttccccgtcttgtactactctgacaggtccatagtttccttcgtacataaacttttccactgagtttgcttctgcgacaaaaggcctatgatcggcctgcaccacttctgcttcgcctttgtcattccaaaaaatcaggcattgatggagcgacgagggtatacatcgacttccgtgtatccaatcccttcctaaaagcacgttgtaactagtaggaccatctattacaaagaagacagtggtcctagtagtcgtacctatagttatgtccaatggcataactcccttagctgaagttgctcctccattgaagctagtgaggatgacttctgtaggaatcatatcaccctctgtttttgtaagttttctcatcattctggatggaatggtgtttatagctgctccattgtcgacaagcacttttgccactgggacaccgttaactagagttttaacgtataatggcctcaggtattttgtcaacttcatggctggccgtttaaaaacaaccttttcggcagcctctatttctacctcttgtttgttttctgtcgaattatccccttgtgataggtcgacgtgtagtatgctacgctgatcctctatctcctgaatctccttcttgctttttcctaatgcttcctcatcggttacccaacctgtgggaggaggcattattttttcttcctcatcaatcatccaacttgtgggaggaggcattatttttggaggcgatccatatttctcagagcgaggcactctcttctttcttttgggtgttccgtacagtacgtagaaatcgaaaggacgcccagatggctcccccaataagtctacttcgcggactccctcttgatgtagttgctttaacagagtattacgtgatacccctctctttttcctttctgcttctagatcaatttcttcttcaatgtctgtcatcccatcgtcctcttcatcgttgtaggcctctccagaagtctggccttcatcgcataccagcatgcaggcttctccttcgctgtcctccctctcttcttctttttccttatttttgaactcattggccagtaggtaattattggccatgacaggaggcaacgtaccgaattggatagcaaggggctcatctggatattcttcttcccttttatctctttcaaaccttgatctcccagaagaggtctctggcagttctttcattgattcgtatgtaccagtttctctattacccttcaggacgttttgattggttaccttgagtagtagaggtgctttagggtgtggcattccttgttgctgcctcatcatccgcccgtaatttcgctggaaacgcctttgttgagtcctggtcatctcatcaaagggtattgctcttcttgcagtgtactggaatgaatgccatacatttggccggcgaggttgcggcctaaatgttcttccaacttctgttggtctgaactgcctttcaaaaggcggtcctctatagaatgatgcaccttgtcttttactaggctgaacgtttgggaagaaaacagggcgatgaggatgctgccatgtccctggtttctctgtgcttccatttacttcccttttacaccttgcacacaggacgctttcgtccttttttggttcttttcctttgatacgttcaaagacactgggatgtggtttaggatcttcttctccgtcatctacgactaacttgaattttggtaacttgttcttgaatccagatgttatcatgtttaccccaagtggctgtgggaaaggattctcgtccactgccatctttttcttatcgtcgaacgtaattcgtcctgactcaatagcatcctgcaataaatgacgaaaaaccaagcaattgttagtcaaatgtgaccatgcattatgccacttacaatattttttaccctttatttgttcagggtttggcaatttgtgcttatcgctcagttttatttgcttatccttatataacttatcgaatataaggtcagctttggttacatcgaacgagaacgttctagcctttatgtttccatcctttatgggttcatctttgcccgatggtctaggtttggccattatgggacaagtatatgtatccccttttactaattcggccaaacacatttcggcctgatcatacgattcgtcatcgatggtatgaacgtcaaaattcgggtctctgtaataagtccctttactagaatttttcatttgttcttcttctcttatcaatcgctcatacctaatgacattcgcacttaactggaaaaggtcgggaaattccttgtcttggaacttcttttttaaatcaaaacttaagcagccttgtgcgattttgacaaattccttttcgggcaaaggtacaaatcacttgcttcttgctgttttgaacctttggagaaaactttctgcccattcatttggcatttgacgtaaattcgtcaaatcagccaagttgacttcagattcagttttgtaaaactgagcatgaaacaactgttccaattgttgccatgtttgaacagagttcgctggcaagttaatgaaccaggggaaagctactcctgttaacgaactagggaagagtctcattttgtggtaatcggttacatcaccactttgcaacgtgaatcgccctatgtgttccagggtagacacctctcctaaaccagtaaacagtgagaattctggcactttataccctctaggccatggatatgcttggtcaacccaatcaggatatggctttgtgtaagtcggtctaatgacaggacgcaccccaaaggccatctgatcctgcacgatttccataatctgatttctcaatatgacattgggatcatatggaattcctacaggctgattaaccggttgatttgcatgaggtctgatgtttggtccttaattggcaacaaaattaccataattagggccattaccattagcctggacatctaccccctcgttaccacgtggaatattctgtccattgtttaggatattatccctcacgtttggattaccccccaagttaggcataccactactactaccttgatttggtattgtaacacctccttgatttgaagtagaggggccagctagtggttctaccccttgactcggatttgggaccgaaggattatgtcctacgatcgtcctagtttgaaagtgacttgtaagaggtatagccggctgacatatttggcctactaacttattcattgtttcattcaacgtctttagttgtttggccatattgtcatagtgtgcattaccactttgtgtaaatctttccatattatgaatacttcgaagatttacctgctcaacgacgtcttgcgtgagttttccaagcaatgcacgcatggttcgaggactcagctccgtcattggttcgtaacgactgttactgctctgattttgtccatctgttcgtggagtggcatgttgctcctcatatcgctcgattacagactggactcctccctgacttgctccttccttgtcggatctctgaggcatactgtttctctttttgcactttcaacacctaacaccactgtcccactgggcgtgccaaattgtttcgcgcgggttaattcgctaacaattaaagaggatcagacgattgtgtaagggacgaaaacctcttgagacaaagtcccaaaaaggggtgttctttttattggcgatgaactttacaaattggagacggaaaacaacgtgcctccaaggggcacaagcacacgagttacagaaagggaaatgtttaagtctaaaagctaaaggaatgaaaattacatattctctgttcgagagtttttgattcggtccttgcttctaagttctttctcccttttatacttcataggcgatccctttgtgattaactgctctaaaaaactgcttgatcgcccaataactacccactttctttgtaatggccattttgtcatacaactgtcttttaactgctgccattatcttgcatcgttcaaccgctttcgattgaaccccttgagtcgtggaacgtgatgaaattactttagcaactgccttaataactgcatcataatgcattatgtttgttgataccttgggcgacttgaagatttgggcgagactttggacgaccgtttgccactccattcgttcagattctgaacgacttgcaaacttgggcgatggcattaccgcactattgggccccttatttgggcattcaccttgattcattcaattgaatttcgttctttgggctatctgatttggggaccctctaattagactttactctctgggcttgttcgatttgggctgaatttttttatgtgtcaacaaatgtaaaactgcctcctgaaggatgaggtacgttggagtttgaaatatcataaccggaagctggggcttcaagctcgttctcggtctcatctttagcttcttcttcgaaagcaagggtagaaggaccggaggtaaggtcaaatcctttagtatgtgctatccattgacaatgttcttttttgattttcatttgtttaagtgtttgaatgtttatggtgtcagtgggttgaagtttgacagaggtctcaccatctaaggaaacgtcaaaatatttaaaaaaatttgtgagaagcatcatgtatggtaaacgtttaacatgacgtgatgaatgaactagcttcataagacctaatggaacagtgggaaaatcaaattttctgccgacaagaaaggaatcaagaatataaagatcgaatgcacttacttcattgcgatgactctttccaagtggaatgacatgtgcaataatgttatgtaagactttgcatgaaagagttaattgatttgcattaatttttgtgatactttcaaaatcctttccggtgacttgacgacaaatctcggtaggattatacccttcaaaagtgggatgtgcattgggaagaaaaatttgtgtttcacatgactcaagatttaaaatgtcacgaacgagggttttattgactttaatatgtttatttttaagtaaacataaaatgttatccgaacgatgatttataaccatgtttttatgaaatttgctacaacattaaggttgcaaaccgaagtgcaggttgaatcaagtagtaagctcggaagtccgaggtcgaaccacagggaattggaaggaaataaactagttgatgagtagtgaatggttggtgaaaatacgatggagaagaacactagagcgttgaggattcacttcggataaatgacttttgatcttttatttaactcatatgaaaatcagctaggaagtgatctcatatggaagataaaacattgatcacaaatatactaagagatagttcttgataattgtttgaaagaatatgtcaaaataagttatgggtatatagaaattatctaagcatttattgtgtaaaaattgtcaacaataaatcaaaaccatttgtagaacatctacgtcaaccaagtaagaagatcaacattgaagaacaaagtcaaagatcaaagataatactaaacatttatcaaagtatcacccctagctctatctaaaggtttagaaatacataatgaaatgttacaaagaaaatgaaagaaactagaatatgatgaagaggaattgatgctctcaaactcttggctaaggtcccattttataagtaaaggaacatccaacatgcaagaaaacaatttgcaacttgtttttctccaacttgaagacagccagaacgtgtaacttgatagcaattttcagatatgttgtacagtgaatttagacttttgatcaacagataagttgtttccacttaagctatctttctattggtataaatattaggtccattggatctctagaactcaagatacagccaaaacaatgagtgctgctcatagatagaaaagctgtggcaggtaacaacgtgtactttgcacggtaattttgacttccctttgatgataatttgacttcttggtaaacataaaaattgtagatacatatcttatctttccaacccaacttgaatcaccgtggttcgataactacagttcaagttatgaccattttaccgagacagctgcatcctactcgagatagctcatcattttttacttttcaacattttttctccacttgctctacatttgaaacacctcaaatagatactatttcaaaagtataatactcatgccgatatgtatgtaaacacatatttcgattaattgtatttttaaccatgtatttatgcaattgtgggaaaagaattgaaattagagactaacattagtgaatttataaaaaatgaatgcaagatgtctagtaaatgatatatctttgaagcacttttagacactaatcacactccccaaccaagatattgcttctctctagcaataaacattcaaatatagttcatataaatagcttgtcgcacttgtcccaggatttgaaactacttaacaaaatgcttctaaggtttgctaccaaaacatagtctaacttgtccaatgctcgaccaacgtgtttgcataatcaattcaatcacatactttttcaaattggacttaccccgaccctcaataatactattactcaccatctctagtttggttagattttactaattgtagctcaacacatcaataaatgagggttctccttatttttgactgattcaacctccaagaatcaactaagctactaatctcttatccaagatctaattctctaaaataagtgtttggcgcttaatcaaggcatgtagtgcgtcttctgttttatgaacttgtttttcaagtttgctgtgcgtattctgtttcatgcacaggcctaattttttatatatataattgtcctcattgagatcttttagggtagcttcacaacatgacagtttttttcccttttatgcaatgattagtgcaatgtccctcattaaacacccattctcgaaaatcaatctttaacttaagattttctcccaattatcatctcattggtcttaaacaattcgcacaaaatttagcacacatggaatccacatttatctcaatgtctctctactacagctcaaccaccccaaactatcctagaattggtctagtaggatttatttatttatttatttttatatttatatatatttttttgtgtttgtcatagtcaattctacatattctatccattgatccaatctaaataatatgtgatttcatgactattgtgaacaatataaattaatctaacatgtacaagcttcaacttaattaaagcggcatcccctagtcacaattcataatataaaaacaatttcaaataatatcatcattggtcggtaaggcttttttttttgaacttcttacttttttacctcccaacctaaatgaaacattgtcctcaatgtgaaaattaaacatgaaaaatgtatgaagaatagtaaggagcaaaatttttgaacaaaggcacgggtttcgagctttacttggagagtctgtataaacttggtcttctagaaccttcaatttcattagagaaaaaaatcacataaaagaaacacacctaaaacaaacacacaacattacaaaattgaaatgaaacctacaaaataaaataatgagaaaatgatatcaatatttaggatcatgcaaagcaatggactcttctaatctcgagaaattctcaaaaaatggtttcaaatgatgtccattaactttaaaagtattttcattacttggattttcaatatctatagctccatgtgggtaaacagttttgacaataaaaggttcactctacttggagcataattttctaggaaataaatgtaactttgagttgtacaaaagaactttttgagatggctcaaaagtttttctacattatttttatatggaataccttcattctttccttgtaaatttgagagttcttataaacttcattctttatttcttccaactcattcaattaaagtttccttagtgaacatgtcttatctaaattgaaattaaatattttaataacccaaaatgctttgtgttccaattcaataggtaaatgacaaggctttccaaaaagaagtcgataaggtgacataccaaaaggtgttttgaaagctgtacgataagcccaaagtgcatcagttaatcgtaaagaccaatcttttctatttggattcactgttttttccaaaatgcatttaatctttctatttgcaagttcagcttgaccactggtatttggatgataaggagtagacactttatgaataatctcatattttttcattagggccttaaaaggtctattacaaaagtgtaaacccccatcacttataatggcttgaggtattccaaatcttaacaaaatattttctttcaaaaattttaaaacaattttgtgatcatagtgtttacaaggaattgcctctacccatctagaaacatagtcaagttctagcaagatgtataaataaccaaaaaatgatggacccatgaaatcaatacctcaaaaatcaaatatttcaataactaatatgggtgccagtggcattatatttctacgagttatcccacctaatttttgacaatattcacaagatttacaaaattcatgtgtctctgaaaagagttggccaataaaattcaaattgcaagatttgaagaaaaggaattgcctctacccatttagaaacataatcaagtcctaccaagatgtataaataaccaaaaaatgatgggaataaacccatgaaatcaataccccaaaaatcaaatatttcaataactaatatgggagccagtggcatcatatttctacgagttatcccacctaatttttgacaatatttacaagatttacaaaattcacgtgtctctgaaaagagttggccaataaaatccagacttcaagatttttgcagtagttttctttgaagaaaagtgaccgctacatgcttcagaatgacaaaatgaaatgatctttttaatttcattatttgggacacatcttcttattatttggtccgaaaaatatttgaataggtgaggatcatcccaaaagaaatttcttacctctttgaagaatttctttttgacttgggcattccagtgaaattgtatttgacttgttacaataaaattagcaatatttgaaaactaaggcaaatcagaaacactaaaaagttgttcattggagaagtatccttgatcgatgttgacaagtaagcataaacaagtaatcagctgcaacattctctactcatttctttcttgaatggtgatgtcaaattcttggagtaaaagaatccacctaatcaacctaggtttggcatcgttcttagagagaagatattttaaagctgcatgatctctaaaattaacaattggtgagccaacaagatatgatcgaaatttatccaaagcaaacactacaacaagcaattctttttcagtggtgtaataattcatttgagcactattcagagttttacttgcatagtgaatgacatgatgtttttttttttttatcttttctttggcctaagacagctccaacagtataatcactagcatcacacgtgatttcaaaaggtaaattgcaatctgaaggttgcatgatacgagcacaagtaagcatgttcttaagttcaacaaaagctttttgacaagacttagtccattcaaagacatgtctttagataggagattacacaatggtttagatatagcactaaagtttttgataaaccttctataaaaaccagaatgtcctaaaaaagatcttacctctttaacactatttggagtaggcaaattagaaatcaattctttagacttgtctatcccaattccgttagatgatacaatatgaccaagtacgataccactagtgaccataaaatgacatttttcccaattgaactcaagattcttttcttcaaaattagttaaacaatcatcaaatgaatccccacaaatagtaaaatcatccatataaacttccaaagatctttcaatcatgtcgttaaaaatactaagcatgcatatttgaaatgtagtcggtgcattacataatccaaaaggcattctacaataagcaaaagtaccaaagggacatgtgaaagtggtattttcctggtcttcaagtgcaatttcaatttgattatacctagaatatccatctagaaaacaatagaattcatgtcctgccactctttccaacatttgatccataaaagataaaggaaaattatctttccgagtcattgagttgagtatcctatagtcgatacacatacgccaaccagtaacagttctagttggaattaacttattttcttcatttttaactacagtaacaccagatttttttggtacaacttgggttggacttacccatctactatcagaaataggataaatgctttcattatctaagagtttaatgacttcatttcttaccacctcttttaaaatagattaagccttcgttgcatttctcttgtaggtttagcatattcctccaaataaattttatgtgtgcaaatcaaaggactaatctcctttataccatctatggtctatcctaaaatgtttttatgcattttcaaattttgtaacaacttaccttcttagtgtgcattgatttgggaagaaattattacccgaaaagtttcattttcactcaaaaatgagaattttcaattagacggtaatggcttcaactaaagttttggcatttgaacacttgaaatcatggacatattgaactgaacttcgatttccaatcacttgtctttttctcctaaaaagaattcaacaaagaaattatatgcgattttaaaattatcgttgaattcaaattctagcacatcgaatggagacgtagcgataaactaatcatcaacatgttgttcaatgaaatctacttcatgcagatcatctttatctccatgctgcttgaaaatgttaaaaacattcatttccactgtcatattttcaaaaaagtttcaaaataccatttctacaatttatcaacgcatttgaagtagcaagaaagggacgtcctaaaatgacaggtatttgtgcatttgaatttaaaacaatatgtgtctccaaaactataaagtcaaaaggataatagaatttatcaatttgaactagaatattctctacaaccacttttggaacttttattgaatgatcagcaagttaaagtgttgttgttgttggcttaagctttcccaacccaagttgcttacacagaaaaaggcaatacattaacactagtgccaagatcaaacaaagcacactctatcctattatttccaatcacacaagaaattgttggacaaccagggtctttgaacataggtggagtgttttgttgaatgattgagctcacattctctgtcaaaaaatgccttttcacgaacattaagtttcatcttgacaatgcacaagtcttttataaattttgcatatgaaggaacttatttgattgcatccaataatggtatgtaaattttgacttgtttgaaaggttaaaaaatttcaaaattatggttgagttttgaaattggttgcaatcattgaggaaatggaactcgaatgggacatttttcaacattaggtttataaatgaatttttcctcagttttgaaaacatcattttcttgctttgaagtcccatccggttttagttcttttgaaggaatgattttgtcgataatttttccactacgcagagacatgatggagttggaattttcttgttgactttcagaggtactagaagcatttacattaaatttcctagaaggatttggttgagttgagcacgaaatttacctctcttgagaatgcaaagaagaggtcaacgaagaaagagtgttcttgatttcattgatggcttgtgaagtttgattattaatgtttgcttgtccttgcatgaatgactacaatgtttcctcaatagtttttgattacggtggtgggtaagaaggaaattttgaaagcccttgaggttgtgatatatgaacacgattattatctctccaactaaagttgggatgatttctcgattgttgattatatgtttctgagaatagagaaggaaaaagctttttgaaagtgttcatagaattggcttgatcatgtaaagtttctttgaaaactggaatgtttggacaatcatgtgttggatgtcgaaaagtttcacaaatgctacaaatttcatcattttacacgggtttaacttcatttacgttccttaattccatagcttcaacctttctagacaaattgacaatcctggcatttagatcagcctcttgactcaattgatattttccaccgctagaactaacaagactagatctgattgagttttcgattgattttactgtttgccaagattgagaattttcatctagatgatctagaaattctaaagcgtcatcaaggatctttatctaaaaatccaccattgcacatcgtttctacaaattgttttgtttcaggagttaagccctcatgaaagaaacttatagtactccatttttcaaaacaattatgtgagcaagtatttaacaagtctttaaatctttctaaatactgaaaatatacttcattggtttttctaaacatgagatactatgaactttacttttcatacttggctaatataattcatgcattacgtgctatttacattgacattgcatttgcatcaatagttagaaattgttttatcttattatggtttacttgatcattgaggttttaagatcttcacatggtgttagtcatcgtcttcccgacctaggtggtgaatctagcattgggctatggtagaaatttaagttaatctagatgttggatattgaatttttaaacaactgtagtctttaaagagtcgaagtcattatcgagaaagttacatgcttttaaattggttaatcatggttaccctaaatcctaattaaatctttaccatacttgggacattagacatgaagttccatgacaataaataatataaggttcatgcaacattataaatattgaggtccgaattgtttaagtcgatcgagaatcgggcacgaattacgtaagaaatcgattgaatggttaagtaactaactttataaattattttgggatcttacgaaaattaaattaggttgtagacacactaagataggtcaaagatatttttttaattccaaggatgggtgtaaacctagatttttactacaaaaccacatgcttggaaagacctcatgcttgaagctaccttttatagaaaatttcttcattcctaagcattatgcaaaactcagctccctaaagatttcatatctatctcctacataagaaatttgctccttcaactcatccttatttgattccaagtgaaaagaaagcaaaagagctaaagagaactagaaaacaagaaactggaattgaagggtgcgtttggtttgcatttccattttctgttatcagttttgaattcatttttagttttctgttttgaaggactatttttgaattacagaaaatgtgtttggtttgtcattttcaaaaacaatttctcaaaataaaaaaactagaaaatgtgtttggcttaaaatttttggaaattgttttatgaaatttattcaattgatttgattatttagtaaaacataataattttatgctaatgttatctacatttaccattttttatgttcataatcagcaccaaacagtagtcttaagaagataatagaaaggggattcatagatttgagtagttgacctaaattttagggcataaggcttagatttttgtaataattccattttgtagtcgaacctaagtttattgggaaaaaaatgtcaaagttatcggttttttagtaagcccatgtttgattcccattaaattaaattacattacatttcatttttctctttcttattttcaaccacacaatcttctataaaataatattacacgtaaatcgaaaacttttccttctttttcaaccactcatttttctaaaaaatactattccccccattttcattttcaggtaatgggcatcaaacgtaggctaaataaggacacttttaatatgcactgtaaatatgcaaacattaaactcagtgaatggaggagagtttagaagaattgcaaatggttacatcaacaatgaaatcatcattactagacactgaaactattacacaatatcactactacaatttcaaaacaaaatacaaatatacgaaattgaagcgggaaagcgaacctcaccataatcattcaagaatttcttgtggcaatcgaatgcgtttaggccacatatatccgattgatactgcctgggtgtagaacaaataaaaatcaatcagcacaattcaagaacaaaaaattatgcaggcatagagacgggggagagaaaagagaatacggcgtgttttgagcgttttccgtgttttgagtttttttaactaaaaacactcaaaacggaaaacaatcgttttgaattttcagtaatgaatgctttcttgtttttggaaatgcataatttcctttgagataagatataatctctttttaacttcatttaccaataccagaatactttaaaagaatattaggaattatttctcaacttgatcagaattgatttctttttttttttccaggacgcttcatatgaaattgtcgaggtctacagatttgtctgcctcaaaatctacgtaagctcagatatctatctcctatggactaatatggttattttatcgagaattttgtctttcctttgccatctacgacccacaaccttaagttctaacctaatacatgtcttttaaataactcattttttttttcaaactacttttatctttgcatacaagatatacataaagcaaaatgtaaaacatagtgaaatatggaaaacataactttagaatcataaccatttcataacaagaatttagaccttgcttagttaaacatacatgtgtgtaatatgaggtcgattgatagatgtgagatgccatggagtgccttaaatgtttcattttctcatctttaatttttccactttatagttaagtatttttttatataaacaaaatgcagtaagtgtatagaatctactaaactcgtactctaataccatgctgtaacatcctgacctgcatgtatagaaacaatactaaattaattgtgctttagctgcaaacttaataaataactatacttcagcagaaagcataaaaatttaatttaagaatttgtataattctaacaacatcatttcaaattaagcgatcatctaattgtttcttagaagtaacatcacatttggacagtaggaaaaataatgaaatgatattgaaaattttgaacaaagtccgtgcaagttctattgtttatgtgaatgaaggcatgcaccaaaaaactaggtaaagaaatctttttttttttcaaaagataacataattcaataataaaagaaacaaattcaaaaaaaaaatgtgtctttagaatggttaccattcatttatctattattgacgtgaaattctaggcaaaaattttaataaataaatgttattgttttgctttctatctaaagtggcaattgtcaaaatatattcgtttacatagctatcaatcccgaaacttcatgaaatttaaatggaaagtagaaaactctttataatatcacatattcgaaaatgggcttccgtcagcaacatataaagtattaaaatatttttcagctccccatagcgactcgggtttgaagataacctagcgcagtttacttaacgtgatatataaaattctacaaatatcaaatagacatgattttatgtttgttcagtaactattccatgagactatcaaatcccactggttttgtcctaatatcccaagaaagattgagttatgaatgtttgaaggcaagggcagaagctggaatttttagaaaacagcaacacccagtttacttaaaatgatatataaaaattttatcgatatcgaattgacatgattccaagtttcttcagtaactaacttatgaggctatcaaacgccactagttttattcaaaaatttcaagtgacgattgagttgtgtatttttttaaagtcaaggcaacggttaaatttttaacaaatagcaacattaaatcgctaacccttttttgcgataacgtgacttgtaaggtaatttctataacacatatctacttttaaaaataacttaaccatttaaatgttcatagaaatgtaccacatataatttcataggaatctatttatttaaagaaaattacgtaaatgtttcataatcaaataaaacatcaagtcacggatttctccatagcatgttacatcttcatctaccatcgtcgcacgtagatggattttcgacaaaatccaatttagaattatcatgatacatagagctggagaatgataattcatactatagtagtgcttcaagcttttaatgaaaaatcataatttgaaaacaaaagaaccacttgtactgctacctaccttgatttgaagttttgaaatggatgaaattggatagtgaatattgttttccgatggcacccgaagcgttaagaaatttgctcctctcttattttttttctttcttttgaaaatctatttccttgatcaaagtgtgcactttttttgacagaacttgtatgcttcccaatggcaccggaagctttaagaaatatttaggagaaaacgaaaagtctagacttttgttttgtcaaaaaaatggtggcaacatttaaaagtgagatttaagttacatttcttgccttttttatgctatttaatggaataatgttggtagtcattcattcacccattaaagcaatgtttatgtttcattacatgcctttaatttgggatttcatttcttgcatttttatatgcttcttttgtaacctttaacattttaaattcttttgcacaaatatatgtacatctatatatttaaatttgaggaaaatgaagtgggtcattaaataaattttattcttgtccctatttatttacttaacaagttaagaaaatatcaacatttaccctcaaacagaagcttataagttctcttttatgtctcgtttttaaaatttataatttagcccttttaaaaaaaattatgcatacgaaaatcaaatcttagaaatatttactatacgtgaaataaacttttcaacgtcgggtcaaatctttgggaaaattagaattttgtcctactttatattttatagaaaatatgcttgattgcgtatgaacttccatgatattaaaattattttaaagcatatcaaactaatagtgggctttcatttcttacgtgggccgagcataagttcatctataagctaggctcatggtgctagattattgcattaaactaacatgtgagcctaattatttattattattattttttggcttctacactctacatttcagcgttacttgatagtcattttctctgatatggtggaaaaaatcatagaagtctttatggatgatttctcaatcttcgactcttcatctaatgagtgcctagagcacttaaattggtcttgcagcgatgtaaggaaacaaatctggttctaaaagggaaaaagtcactcatgataaaagagagtatagtattgggacatttgatttcagctaaagggattgaattagacaaggcaaagattcaggttattgagaaattactactacctaccttagtttagggtgctcgcaatttctttggtcgtgccgagttttattactccttcaccaaggacttctctaagatcactaaacaattttgcaattagctaattaaaaagatgtttcttttgacttatctaaggagttattttatttatttattattattttttagctttgaacaatctaaaggagagattaatttcagtgccagtaataattgcaccagattggggcttaccatttgaaataatgtgcgagtcaagttactgcgtggtgagactagtattggggctgtgaagagaacatttttcatgtgatctactatgcagacaagatattgaatgatacatagttaaactatgccgccactgagaaagaacttttagctgtagtctaagcttttgataaatttcaatcctcttgttggatcaaatgtaatagtccatacaacattaaagtatctggcggctaagaaggatgctaaactaagactaaacatatggctgctactcctccagaaatttgatttgaaaataagagacaaaaatggaagtaaaaatttagcagccaaccatttatccctaattgagcaagggaaacagacaaagtggatatcaatgatgtcttctcagatgaacaaatattaaacttggagactgcaccatagtatgctaatatagtgaactatttagccaaatctatcattccactagattattcaagttatcaaaagaagaaattcttttttgactttaaatactattttttgaaggatcagattctctgcagacagggtctatatcagtttatcaggtggtgtgttcctaaaggaaaagttccttctgtactcgagcaatggtattcttcttcctgtacgggacactttagcagcaacaatcttacaatttaggttctacatttttgttcttgaatctatgattttactgtttttagatagcaatttgtttcatggaattttgaccaaaatttaactttgaatctccgaataatcttttgagtagtatattcagagttattatcttgataaacaaagaaatcacaacagaatatccatgagactctcatattgaaggcaaaaattggaacaaaacattttcttgaggctttaaaaatgtttttgcctctcttttgaagtgttcgaatccttgaagagtgagtgtaatgccccgtactctagtgatacgttgggttaccaacatttgtccttttaggttaacttcccaatgcaaaattagtgatttattttaaaatcaacagcaagttgaaaacagtttctccattttatgcagtgattttacaaaaattatttgatcaagcaaaccttgacgaaacttcatgaaattttacccgatgataaaaaacccatataagtatgacatataaaaacttgagatctcgaagacgtcgtttgaagtaccaaattatttttcgaataggctggtctgaaatcctggatttaactgtcacagcttacaaaaaaatgctacgaaaagttctatgggacttcaattgacatattttcaattgcatatgataaataactcataaaggattattttccaccttgaaatatgcaaaaattcattatttacaaatcagagtaaaaatttcaaaacagtggcagaagttgggatttaacgaaagacacattttcccagtttcaaactttaaggttttttagtcttcaaaagtaaacccaaactgaagtttattagactccacaaggattattgaccaaaaaaggggacaatctgaaatttgggtaactctctccataataaaatatgacatcaatgtcgagccactgcaagatctccgatcattctgaaaaagttaaataggaatgagcatttcaagaatactcagtaggcttcacaatttatatggacataataatcatgcatgtattcttacatattgcatttgttaataattaaatcgatgatcaaacgctctacttaagggtactgatgagcctctgcgatgatcagttaagcatatcaaattagagttctgatgagcttctacgaccatcagttgaacatataaaattaaggttctaatgagcctctgcgaccatcagttaaacatataacttttccatcatttactttcaagaagaaccattaaggaacttcacatactttcataagcgaatacgaagaataatatgtatgaatgaaaattaaatccataaaatgatcacttagtgtagaaatcctaccttagttcgaaatgatatagtggcaactacctcaaatgatgtttcttttcaaatattgaatatgagaatgctctcctttgtaactataatggcgtgagtagggtagtaatattacatatataaactatcccttatgaaaaagacaaagaaaatatgattagggactctccagattaggtgttgaaatgaattggtctcaccaaaatgtttatcaatctcattaacgaaaattggttgttaccttgataggagtgaaattctcttaattaaggttccaataatggacacgtgatttaagtgtaaaagagttaattaggttgttcacagaattcaaatgtaatgcaaattaactaattcaacatatctaattttaaatcaatagatcaatttattatgtctaatgacatgtggtgatcaaacctgtgaacatgcctaattaatattagttaaatatgtattcctttgagctacaaaaacaagaacctaacatattaaaaataattttttctcgagtctaaaattcttcatttaatatgagctttgaaactagtctaatcttgacatggaaattctcattaaatggatgcttgattattctaccgaataaggtaacaacgttgaaacatattttactttagtctctctatttcaaaacataaaaatatagcatataaaacataaaaatgttattttataaaattttcggggcgttacaatgagattgggtaaaatcttctctccaattccaaaacatttgaaccatgtttgaaaccattttgaaaaacttggattgcaattttgaagaaataaaatgaactgagaatgtgttactggtctaaagtaaaatatattactccaggcacccttgtaatcaaagtaattgaaatgagattcgaatgattcgtctgtagagagatgcattcgcttctcattccatagttgttgtccccaatcatcacatgacaacacctttcaaatgctaatttttgacaaatctattctttttggatttttgttggtttggtgtatgagtaatgatacctgatccaatttttgtgaggatagattgataatactctatgaatttttgatattctaaggcatgaaacagaattttggaggaaaaaagtctaaaatacatttatctaaatttgaaaatctattgatccaagatgtttccatctcgaatatagagctacaagatgctttgaggtagtgttgaaaggtgtttggagggattatttgagggagtttaccagaaccttgaacagctttttcgaaatttgaaggttttggttgttctggattgtttttattttggttgggttttttgaatactaggatttaaagggtagtattttggatggatgaagaagcttgttcttcatttcttgaggatgtcctttgaagtaatcatccattgaaaataatgatataatagtctttttttcaactactcttctttgaaaataatggtatagtagtcttttgaaaataatggtatagtagtccattgaaaataatggaatagtagtcttttgaaatggagcttctgaagaagccattgaagttttttctgtttttgaattttttctctctattacttcctgaatatctagccaattcattaactcttttctctcaatatttgatttctcactactctcctttttctgtatgaccctcttgtaaggaagttagcaagaatgtttgatttaccttgtatatatagaatttcaaaatcaaaacaggacaaaatagcctgccatcttacaaagatttggtttgaaacaagattttttttcatctttttgtaaatgtctttggatgctttacagtttgttttcaaaataatgttttattaattttgaaattttgaaatacatagtactatagataaaatcttttttttttatagtggaataattcttttaagagcggtccacacatcactgtgatacctaaccaactattcttgatttcactcttttggaatatgttttatcactccaccatattctatgtcagatgtacctgtctcaacaataatagaagcagtggggtcaaaaattgatagacgatgaaaattttttatagcttttttgacttttggatagttattgtatgctcatgacttcattggtcagggttttttgtagcctattgaaaagaagggaatagatttgatgtattgacaaaatcgacaacataattgacatagcctaattaatactgcaaactaattttatctagaatttcatcaggaaatttatcaacaaattctagaattctttgaattggagtaataaagtttgaaagaggattaaaaatatcattcataattttttgaaaatcagaatgagcatttttaaaccaaatggcataatattctattcatattgaccaaaagggatattgaaagcaattttgtatctatcttcttctttaatttgaatttgccagaatcctaactccatatcaaattttgagaagataacaactttgtaaagtctattcaaaagatctttcttttgaggtcagggatatctaatccactgaagagatttgttaagaagtttacaattgataacaagacatggaacgccccgttcaatttcagcagaattattggcatagaatgctgagcaactccaaggagatttgctcgaacaaataagacctttatcaagtaaatccttaacttccttgatacaacgatctaaagttctttattcatttgaatatgacaagattttgtaggaatatttgattcatggaaattagaattataaggaagagaaatagcatgtttcttcctatcacataaagcatttggaatagtagaacaaatttctttttcaatttctttttgaaaatttaaaattttctcttgaattaaagaattttgtaattgttctttaattcttgaaatttaatttcttctttaagaaacttaatatgattctttttaaaatttatattattaataattttttatataaatacttttttaaggaattaatatcctcataagaaagaggatttatgaatttaaaacaaatttcttcaccaattatgtttgtggtttgagccttttgaattagattgaaaatcatagatttgaacaataaaaagagtaacaagaataacttcttggtttaaatctttaaaaagataaaatatatttttgaaacaaatatttaaattacaaacatgagcgtttgaaagtttatattgaatattaagcttcttaccattggcaccataaagacacttagtggttttttcaaaatattttgtaggtattaatcattccctaatacaattttgatcagctctataatcaataaggactctagatgtgaatttaaattctttgttgactacaatagttatattgcagtaccattttttacaccgaattcagttaataacgttaacattttcttcttcagattgaggatttgaaggaatgcctttatggataaattcttcatcagaagaatcagaagaggataaaactctagattttttctttaaatcttgagttttaagaaatgaaacttccatacaaacatctttcatttgaaattcaagattggaaattgggatttcatagaattgattttttactttgaattagaactagaaattttttatgtttcttttgtaaaacaatttaaaacattttgcatattgaaaggttcaaaagtaggttttgaatttgaaggtaaagggtactaaacttatttttgacagttaaagaagtgttaaaaatcaagcaaattgaaaaggaatatctctagatctatgctcagatctagaggaataaattctttgaaatctagataaagatgaagacgatcctttaaaaatcatcgtaatatttccatcggaaaaagtaataatttgatttggagtagtttgaataggagcaagaattagattttgaacattttcaaaattcctttcaagtcttctggattgtagatttcaagaaactctcttgggaatcagagtttctgaatgaaaatggttgacttttacccaaagatgaaagatggatgaatgaagagcactaatattgagttaagtactcataagcttgtaatatattctatatattacaccaaaagcatacaaaataaagatttttttgtttgaatatgaagatttggaacattaagaatagccccataatcaaaattgatagaaaaatttggataacagtttgagaacactggaccactatatagatttgactctagaacatataaagaatttttaaatttgaggagtctcttatctctgagagttaagttaagagaatagaaatgtctaaaccaagtcgaaacaatggtttgacagcaatttgaactaatccaacatgaagatatttaaatttcttcttatggcattccatagcatcttttgaaaataaattgatgtatgcattttgacttttgataggtaatgtttgttcaaaagttttgataacataattttgagtaaaatcaaactttcctatttcatagatagagtttttctctacctttggaatagtccatttatgcaatctttgttcaatttaaacaatttgaagttcataactattgaaattatttgatgctgatgcaaatgcttgatctaattcttcttcattttgaaaaatatttgaaatattttcatatttatttctagatctccttaactaacttgaaattgaagacataatcaaataaaatgaaattataataacttgccattgtagacacaatactacaggataaactgactttcaacaagcctacattgagaccacctaaatatgcctacaccggcttaacacgggctaaccaatactcttcagcggacatctaggttgaactaggttttcctataacacaatatctaaaatgaaaattattataacctcacttcactcagttatggctctgataccaaataagtctaggggatatatatatatatatatatatatatatatatatatatatatatatatatatatatatatatatatatacgatataactacctaaatacgaaggacaataaatttgaatgagaaaagaattcacttaaatgtgctaagcaattagggggtaaaaagtcgaagatgagaaaaattatccatcaatcttaaaaatctttattcttccatttgtgttaatccattcaaaagaaaaagaaaacttttcttttaagatttttcacttctgatgagggtcgtgtggaagaacaggtgcttgcgtacatggaacgcttggattgtcgacgtttgaagaaattggcataactttcgcatacggtgtccgttttgggcccataaccccattttggaaaactcgcgacaattttgaatgaactcacatgttcgccgtgacgtatgatggattttgtcagtttgaatttgtttactaattcaaaatagcatttaaatttcttgttttgttattttcaatattccttattttcgttttgtagcccagcccattaaggaactactggcccagtaggttatttgttcttttcgtatttaaggcttgaaaaatgcctcccatgttttctttggttgttcttgaaataagaaaattgttggtttcttgagttcaatccatttgtgttattgttattgcgtggttgtagattcaatctacatcatttgacatcagagcatggttcgcggaagaggacatgcttgtcgtggtggctagattgacgaagttacagatctgcgtaaccaagtcacggcattgacagttcgatttgatcaatttatgacgtgggcagcagaggtggagtagaacgaaacaactcctgctccccaacgtcgtgtcccagtgagtgatggggaaggtggatatgaatcaggtgagaggtctgatgaggagaccttattggaggcatgtagcgatcgcgttcaggaaccttgtatgtcatagcaggacgcattccagcattgggaatctagaatcaaggttgatatacttgagtttcacggtgggatcgaggtggatgaattccttgattggctagcagcagtagaggagattttagattacaaagaagtgcccgataataagaggtatccttggtgacaacctatttatgtggtcgcgctgctgcttcgtggtagcaactgaagcagaattggatccgtcagggtaaggtgaaaatctagtagtgggaaaaaatgaagaaataatggaaggcagctttttttttgctttaattatgccaggaccttgtatcaacgcttatagaatttaaggcaagacagtcgttctgtagatgcgtattctacaaagttttactaactaatagcgcgaaatgatgtgggagaattagaagaccagttggtagcacactacattggtacactacagttgaatttgcaagatgttcttaatatgttttcgccggtgtctatttcagagactcatcagcgtggacttcaagttgaaaatcaacaattatgccattctatagttggcgtttctggcggtccatctagaggtaggggttgaccatttgcccccaaatcccaaatttggtccgtcccaatcctttacatctaggaatcggggcgctgattgaaacacttggccagcggtccctccaaccgttagtctgggtggctgggctccttctggtggatgagggtgtagtggtctgtgctttgggtgtggttgttttggtcatttgaggaaggactatccatcccaaggacagtcacgcccaggcttgttcgtcggatgggcaacaaaagccgatgttattcatgtggtgaatgaagaagaagagaccgaagttgtgcatataggtgacacggggcctcttttggtggtgggacgggcgtgccttacacctaaagggtcatctgaggaccagcagcgaaacaacatttttctgtccacatgtaccattagaggaaaggtttgcaggttcatcattgattcggacagttgtgagaatgtgatttctgaagccactgtgcagaagctacagtaccaaacctcaccttgttccttacagcttggcatggttgagatgaggtaatgaaatttgtgttactagacgtgtgttggtatctttttctattggcaatgtgtattgtgatagcatttggtgtgatgtggtgcctatggacgcgtgtcatctattgttgggtcatccctggcaatttgatagggatgtgtgtcatgaaggacgtcgaaatgcatacacgttcaccttttcaggtaaaaagattatactactacactctaaagatactcattgtatgtcttcggtaggggaaagtagtaatctactttctaggtccttgtttgtgtctgagatgttggcagaagatgttgtattggtgttagtggaaactggggcaacgggagtgtcgataattcctatggtagccgagggatgggtcttcatcccaaagctacctccttggtgtctgaatttcacgatgtgttcccagatgaccttccataaggtcttccacctttgagtaccaggcatcccacattatcgaatgagcccagcagaacatgaagagttgaggaaacaggtagaggagttggtgcagaagggttacatcagagaaagcctcagcccgtgtgcagtccctgcacttctagtgccaaagaaagatgggagttatcggatgtatatagacagcagagccatcaacaaaataacaattcgttaccgcttttcgatactgagattagatgacttacttgatcaattggctggagcaacagtatttaccaagctggacttaaaaagtggttaccatcatatcaaattccgccctagtgatgagtggaagacagcgtttaagacatgggagggattgttcgagttgctagttatgcccttcggattatccaatgcaccgagcacattcatgcgggtgatgaaccaagcactctggctgtttatttgtaagtgtgttgttgtatactttgatgacatattagtgtacagtgagttggaggaatctcatggtgagcatctaagggaagtcctcactgttctgcgcaaggaggaattctttgcagccccaaaaaatgtgtattctataccgatagttttttgtttttggggtatgttgtgttagccagtggggtgacaatggattcagctaaggttgatgcgatccggcagtggccgtcgccataattagtttctaatgtgcggagtttccatggcttggtgtcgttttatcgacaatttattcagcactttagtagcatcacgtcttccattactgattacatgaaggagagtaagtttcagtggactcccgaggtagagaaggcgtttgtgaccattaaggaacgcttgacttcagtcccgatacttgcgttgcctgatttcacaaagcctttcgcattacattgtgatgcctccaaactgggcatcagagctttccttaggaaggaaaaccagtaacttatttcagtcagaaattagcatgggctcgtgggaggtataacacttatgatgcagaactttatgctgttgttcaggcaatttaccattggcaacattatctatttgagcgaatttgtcttatacagtgatcatgaagccctcaaacatttgtccagtcaagagtctgtgtctgcctgtcatgcatcgtaggttgcctttttacaacaattcaactttgtcattaagcatcaggctggttcatctaatcgtgtggcagacgcactcagtcggtgtcatgggttattagcacatctacaggtggcagttatcgggtttgacacctttgcctctctttatgctgatgatccttattttggccccattttccacaatttactgcaggaattccattccccctttctattagagaatggttatgtgttttgaggcgttcagttgtgtataccagattgcagtctttgtctgaaatcgattgaggagtttcacggcgagggtcgtgttgggcgagatcgcactttggctctggttagtgcttcatttttctggcctactatgcgccacaaagtggagaagtttgtttcacggtgcagggtatgccacgtggcaaaaagaaaagccacgaatgctagcctttatcaaccaatgtttcttaatttgattcttcttggtgttcgtctataccacaaagttgatcgatattggtgtaatgtttgaaaatatggtccaaccaatgtccagcacaaaacaaatgagtaaataaaatattacatttaagtttattaaacattttcacattttgtacgaaaatttcataaaactctaattcatatacatatatataacaattttaactttttctttaacattatcaattacctaactttaaaaatattactcatatcattcattcggtacataagatttgcaacacccgtgattactgttagtctcaaataaaaaacttgagcaatactaattcattctcgtcgtgaataaaattctattcttattcaagacaacaataaaggaaagaaaaacaagcaatcatgtttattcgctcaccgtgaataattaactgctcacaatctaagcctaacaaaaataaaattctcagaagagttttaaattattaagaacgattcaatacgaataaaatattcaatatatccctcggtcgaaaacagtccaactgttatctacagtgggaaaggcccattccgttgttggtttcggtttccagttattgaatttaattttgcaggtgggcaattgacagaacgacaagccatgtcatgctttactcaagttgcagatataaaatattttttcacatgttttgcagtccaaaactgaagctgattttccgtctcattaacattaattaattatgtattcaggtagttggctcactgggttttttattcttcccagtttattgtttaagattaaaaatccaacaaattcacaagccgttttaaaacctcaaatttcgaaattaaggtttaactactcgacaaaaattagtaaaaaccaaaattttatgatttgtgattgcttccaatcattgctcgggcagctcacagcatgcgttccaaatttccaactagtattaaaatgtcaaatatatattaaatctatatacataatataaatgattaaaaaaaaagatatttagttatgacaatttatttatcctctttttgtttgttatataatatattataagttctttattacaatggtcatttttcaatagatataaatatgtgcatacattcaagtatttgatttgacattacattgataacgtcttaaaagcaacttgtaacaaccaaacaagaaacactgtgtgagtctgattacagcttataacgtcacaatttattaagcctattgaccattgcagttacaatccacttttaattagtcaaagtcaataatcattcggtcaaattcaataatcatttggtcaagtctaagtcaaattaaggatgagaattatttcatacatattcttgtgggctattttgtaattataggaatattggttgatgttatgccctggttgatgttatttcatccacgtgcactcgtccacactaaagcactgaatttggatgtgaaatgttaggaaaactttgttgctttcattgaaatgcttagtgtcatgcattttcttcttcccatgttaaaaatgtgcttatatttgtgcatacatgaattgtgtttatgtatacatttaatgtgcttatatttgtgcatacatgaattgtgtttatgtatacatggaaatttatacaaatgtgcgtacttgagtttgcaattcgaaacgattaagattaatagatacctgcatgaaaagttcttatttttgcctctttccttatggtttaaaatatatattattttattcatttagtaagtaaattttattttattttatttttgttcttttgtatatcaaaatttggctacttgaaaactgtcgagcaagtttcagttttcttaggacgtgcattaggatgcgaaacgagatcggacaaacgaaaaagcagagtcattttatttgcttatatttactggattgtaacatgttgttttataaagctaatttttataactaagaaatttatttataaaatataaaatcacttttgtgtacgtaatcagttgcttataaattaaaaatactattaataagataaaaaaatcacttataacatatataatattacttattgtaaaaaatcatttatgtataaaaaattgtttaaaagtacaaaattaatatgtaattttaatatttacttataaataaaaaaaattactcataattaaatttttttattataaataagtaatttaatttttaaattaaaaattagttataaataaaatattatttatcagtaaaagaatttcatacaaaattgacgctaagtctaagtcgaccaagaattatgtaactttgacaattcaaataatcgagaaattatttggtaaatgattcaactttctaaaatctctcgagatgacaagaagaccagattggaagagggtttttctcaagatttctctttagataatcccactttacttgaagttagaactgatgaaaaagttgaaagctcattgattggattccagttgagtttattctgcctgagcaatcgcacgccatcatcacaggtttaattgaatattctaaggtattaaagttctcaaagcagtacaacaaaattagcctttcatagtattgatttacggcttgcatattgttatatatttataccataaatataaaatgtgaaagaaataatcagtttagataaagtgttcaagtgttgggaaatgtagcatttgtgtgggacgtcgggggtttgggtcactctcatgcaattattaaaaagttttttattgggttctggagcaggctcttgggtttccttgactaaaattatttattttcttaattatttaatgggtcaaactagtcagtattttgtgaccttttgtaacgatccactactcacaaaatcattaaaatattgcataattctctagtcatggaggagatatttaaacccagtttgcctatatatactcacctctcgttttgggaaaaatacacatgaaaggaaacagaaaatcatttgaaacgaaatcttatttatcatattcttaaatttttttttttttttggatttttacatatattttggaatacacttgagggttctgaaaaccattcggaattactgcacaagttgtttatgattgttgtatcataggagtgattgtccacaaaggtcgcagcaataatcgacgggcaatttcactttaggacatcgtgctgtcatgagattcaatcggacgataagttttatttttgcattttactattctgcaactgattatttttccaacacataaaatataccactaaagtagaccatttaagtagagtgccttgatggaggagaccagtatgagaacaacatgaaaggggcctgctttattcatttccttcttaaaaataaggaccaagtaaaaattctccaatgaaagatatgtttttgttttggttgactgacatatccccttgatcaaatgtgttattatcgattgcttggtataataatatggttcgttaaaagtttacaatatgttttagctgattttgaagtgaccgttttgcttgtagttcccagtaatacgaatttttctgactcgattattttacagtaaaatcacaaaatataaatgaaaagaaaataaagaaatacaaaggaatttttcagccaaaaggccccgaggttcagcgaccatctaacgcctacatcctcgttgagcatccatatggattaagctcgaatccactatcacagtccccaaaatcgggtaaaatcaagttacaaaggatgaaaatgttctgccgtttttagtcacagaaagccctcagaaatcatacactaatctcactaagagatgtaactcatcacttttattacactactacaagatttcactcagaaatcacacacaagaatcatccagaagatgaagagaacgaagaagaaaagcggcaattgaaagagattagggttccacaaaaaatcttctaaccctatttatatgagacgcatccaacagattgatccaacggtcacagttctgccaggtgtaaggaatctagtgtgggacgcgtttaggttagagttgtatttccaaaaacacgatttccttaaatctggaaccttcagttaaaatataccggtcattgggtcgggtctaacatttaattgcagatcatcaactgggctcaagaatttcagcagtccaaatcttacaatctccaccttactagaattttgagactgattaagcggattcgaacataaattgttttcatttgctcttattacctgttaacaaaataaaagaattagtaaacttcaagattcaataattttaacgaaccaaaaaatttactaagtattatcttggtacctaaatctgcaggattaaacttagtaggaattttaactagtttaatatcacctttttcaacaatatctctaataaaatgaaacttaacatctatatgttttgttctatcacgaaagacaagatttctactcaaaaaaattgcactctgattatcaaaacaaagctccacctgatttccaataatatctaattcatttaacagacccattaatcatattcatttaacagacccattactgcttctgtagcagcaatatattttgcctcagtagaagatagggtcactagtttctataattgcgctttccaactaatgcaagtgtcatttatcacatagaaaaatgcagtggttgattttctattatcaggatttctagccaaatcagagtccacatagcctttcaaatttagaccatttttattagttttaaacataagtcctaaattctgtgtgctctttaagtatctgattaagtttttcatggcttcccagtaaagttcacctgggttgctcataaacctgcttaaaacactcacaccataagctatatcaggcctagaacatagcataatatacataacaaatccaactgcattagcatatggtacatgcggcattcttttaagttcagtttcatttttaggtgattgatcaatggacaatttaatacttgcagacaaaggtaagctaacaagtttggcttcatgcaaagaaaatagtttaataaccttttcaatgtaccatttttaagttaaaaataattttccattgtgtctatccctttttatttccattcctaaaatcttcctagcaagtcctaagtctttcatctcgaattcaaactttaattttccttttatagggttcagtgcatcagaatcattaccagctagaagcatatcatccacatacaaaagcatataaaagaatgcagatttttcatttcttttgaaataaaaacaaggatcaaactcagattttctgaacttaagtccttgtataaaagagtcaaaccttttataccattgtcttggggcctgttttaggccatataaggacttgtttaatagacacactaagtgttctttatttttaacttcaaaaccttttggttgtgacatgtatatagtttcatctatagagccatacaaaaagatagtttttacatctaattgctctagctctaaatcaaattgtgctacaagggcaagtaatatcctaatggaagtatacttcactacaggtgagaatatttcagtgtagtctataccctctctctgtgtaaaccctttagcaatcagcctagccttgtatcttttgtcatttgaattgtattttccttcttttattttgtaaaactatttacaatcaattagtttgcagtctttaggtttgactactaaatttcaagttttatttttatacagagaactcatctcttcttgcattgctgcaacccatttagtagagtccttagaggtaatagccacttcataacattgaagttctttatctaaggattctggttctatctgtccagacacataatatgcaaactggtacctagaaggaggtctaattgttcatctttctctatctctggccaattgatagtcctgcatgtcatgtacaggttgaggattatctaaattttcatcattggtatcaagttgaatcttagtctgaggtgtctccacctcaatttatatttgttcaggggtattttggctttcaaagtcaatttcagtcataataaaatcattgtctattattttatcttcattattgtcaccaagacatgggaaaacatcttcactaaaaatcacaaatctacttatgaccaccttaaatcctttagtttcttttagccagagcctatagccttttaccccttccccataaactaagaaaacacatttcagagatcttgggtcaagcttagaatcagtttggtgagcataggcagcacgcccaaatgttttcaaatgagaataatcaggaacagagcctgaccctatttgttgtggtaccttgttatttagagaggtggaaggacacaaatttatcagataacaggcagttttttctgcctctccctagaaaatttttggtaatcctgaactaatcagcatgcacttagttctttcaaggatggttctattcattctctcagctacaccattttgctgaggggtatagggcactgtcctatgtctaaatatgccatttgtggtgtaatactgatcaaattcagtattgtagaactccaatccattgccagctcttaaaactttgatcttcctacttgtttaattttccactagagtcttccactccttaaaaactgagaaggtgtcagattttgattttaacaagaagattcaaacctttctagagtagtcatcaatagtaaggagataatatctatatccagatgcagtagatacaggtgcaggcccccacaagtcactatgaatgtattcaagtatatattgggacttatgtataccatgattaaagggcattctgttttgttttcacataatacaatgttcacagaaggttaacttctgaacattgtcattcccaaaagcaccagcctttgaaagaacctttaggcctttctcacttagatgacctagtcttttgtgccacaatttagaattatcagtttgtgtgactaagttcactgtagtattctgaatgacaaaatcatgatttagagtatagatgctattaattttgggtgatttgaatataagtgactcatttctgtttattttttttaaaaccatcattaatttcaatttgatacccttcgtcatctaatatccccaaggatataagattcctcctaagtgctggaacatacttggtatggtttagccttaggagttgaccattcttcaattttaaaacaatatttccaattccttttacttgacaagaatcattattccccagttttacacgcccaccactaaggtttgtgaaatcagtaaaccaattaatattggggctcatgcgaaaggagcatcctgaatctagaacccaatcatattcaggtttttctaatgagagcacataagccaccccaatgtcagcatcttcatcccttttataggaagcagcaacggttgaagtgccattatcacgcttcgggccatttcctaggtccttagctttcttgaaacaatcttttataaaatgatcatttttaccgtagtaatagcacttcttattgttagcctttcccttgtatactttcttatcatttcctttattatttccccatttttatttagagaaatttttatacctattgtaattagcttgaccgaaattatttaagcctttactagggaattttggattggacatggatttttcaacatgtaaggctaccttatgttcagatttgagttctagatctctattcttgagtgagtcatgaatgatttcaacagttaaatcactcctaccatattttagggcattcttaatgtccttatacttatcacccagagcatttaatagaccaactactttatggtcatctaaaattttttccccaaatttggttaaaacttatgtgatcttattaaatctatcaatattttcttccagatctgcagcaggatcaaatttattactgaaaaattgtttccaaagaaagaacttatttggcagggacttagaaacatattgtttttctaaggcagtccataattcagtagcagtagtggtggttcctatctttctagtcacagaatcagataagtgatgaaatatggtgctccatgctaattcatcttgctgaattttcctaacttctgataaagtttatggccaagattcatcaattgctttaacacatcttaattgcattaaaagagctttaatattctagctccagagagtaaaatctcctttgccatcccaatgttgaatatcaattttagtggacatattgtgcaagtgtgtcacaataatgttcaaaatgattcaggcaagatttaatctcagctaaacagatcactcaatatgaaatacacagcggaggtatgtagcataaaaatagtccacactcagtaaacttaacaattgacagattaattcttgaaataacaaataatgcactttcttgccaaattatgcaaacgtgagtaatgacatagaaatcaattgaataatgtcaactgcagatagatgattagtattgtcaaccatatacgcaagaattaggttaagcaaggacaataacataaattgcagagcaaaaagtaataaacccctaatgaattttcttcatcgttccttaatttcctcagattctagggttctcatatgaaaccctagacaaaggtaaattaaagggggttcaaaaaatccctaaacttaattcctaatcaagattcgacaagtattgaaatttgggccaggtatagatttcaccagatttacagcttatgccaaaagtaccaaaccgataccacagatctactaaagattcagaacgaagactgattcctgtacaacaaaagtagatctatcaattttggcaatttatagtccaaccgagtcacggaaaaattcgaactattatattttggaaaaaaaaaattaatagtggctttgataccattgtagttcccagtaatacgaatttttgtgactcgattattttacagtaaaatcacaaaatataaatgaaaagaaagtaaagaaacacgaaggaatttttcggccaaaaggccatgaggttcgacgaccatctaacgcctacattcccgttgagcgtccatacggattaagcgcgaatccactattacagccccaaaaatcgggcaaaatcaagttacaaaggatgaaaatgttctgctatttttaatcacagaaagccctcaaaaatcatacactaatctcactaagagatgaatctaatcacttctattacactattacaagatttcattcaaaaatcacacacaagaatcatccagaagatgaagagaatgaagaagaaaagcggcagttgaacgagattagggttccacagaaaatcttctaaccctatttatatgagacgcgtccaacagattaatccaacagtcacagttctgccaggtgtaaggaatccagtgtgggacacgtttaggttagagttgtatttccaaaaacacgatttccttaaatctggaaccttcaatcaaaatataccaatcattgggccgagtctaacatttaattgcagatcatcaactgggctcaagaatttcagcagcccaaatcttacactgcccaataagattacagttgatatagctacggtccatgcaaggacaaaaaagcggtttatgccttttttaattgaagcttatctcttatgctattgtacaaaatttaggacactatgagaagaaaattgagttagcgttttaatgacattgttctgtttttcgttgacagcaagataaactatgaggtcctatggaataaggcctaatgaaaagattgcgttttcagtcagggtaataaatatcatgcttgagaaaagatatgattcatgaattgaagggtggaactaaaaaagacaaaagtaatcacaagagtaagcgtctgtttgctccacctttttccaggtgtggaatgaaaatttgtgaccgttgctcgtactatattctgccaacccgagtccaccttgctgtaccatatgttgcactttcccatccacttttccataattgcccatccaaaaacggctgttgcatgttttgatataattgaatatggacaaaacgagaaattggttggaatttaaataaatatggcaggatgacacatgcaacgggtcccaccatgattggacgtgcaaaatgcattttgtggataaaaatggggatcaaacaagggctaaattcagttcctttgaataataaatccaaatagactatagattatatgtctactttgatattgaatttcattttaaaatcttcacacatatgctgaaaacataattatagaagatcttttaacagccttctagctcctagtcaagacttcctcgcttagatcttctctcttgttctcccctttagatgcgttcttttctaggaaataagagaatatggttaaccctaatatctcgagagatgagtccataaatgacattgttataatactcaattagagtttcataattgcaaaattttcattgaactttattgttgtaagacaattaaggctcacatcgatgttagagctaagagatagacctaatcgaactcacaaaactagaatttcaacagatatttctaatttggtcaactcttggacaatcaaaatacatgtattaatcttgactcatttgatcgtcaacatgttaagacatacaaaatgattgttttgcccttttaacatgtataacctttagagttcaatttcataagacaaatccgttgggaacaaatcacaacattgggtccaaatgtctataaagtgcaccggagtgacgtttgtcttatcgtaataattagttcctctatttaaaatttataatctttaattgtttcgctccaattccaaattaccattatcgatcttttgaagacttcaatcattggcaccttaaagaatttgaactagcaatcagatgtacattacttgctcgggatttaagtgacttgtttgatgatcgagtagaatcttatttctagcggtcacaaataagtcatttatgggttcatgttcaataggcatcaaatacatcattgcattcttattctcaagtcatatattccaataagaacaatgcaatcttattaacataaagcatccagctttatgtaccgatcgtgaatgatatgatttgatcacatcacatattgtgtcttactatactcgacatcttgtatgatcgtggaacattacattatggttgcaaatggtcaaatcataactcgtaacatagttcgcaaaatattgctcaaagggcatcaaactaacagtaactccttgaaagtgggttgaggattaaggaatatgagccattgaggaggaattttagtgaaactagttgttttggctttgtatttcggaacacattgatcttggaatcaagcaaatatgatactaggtcagtgcagattcttctaaatttaattgagttcactgtttttagtaccatggaagtgtaatttttttagctattgtttgaaccattgcgaatctacttagtacatcatgattatatttctattagaacatttgactttaatttttttgtagaatctccataagatttgtgttgttaagttgacacaatgtttcgtttgttagttgcactatgttatgcatactcaacaaagcatgtaaattcatgcttgtgaagcgtatcaactttatgctcctctcagccacactaagtctctaaagttcagttttcatccccatattgtttatttgtgaactttaatcatgccttttctgttatttttttaatggaaaaatcataaatataactacttttcgaccttttaaaattaatattaatttttgtgatgggtagagagttgattgatttggagataactaagttgttgtttcaagaataaaacttgtttatatatggatcaattatttaataatattataatcaattgttttggaatagtagtctatgttttcaataataaaattgtagaataatatgattttatttaacacagcaagaatataaataaatagggaataaaactcctaagatatatttttcgctgagaatagtgtaaatctgcaacccgagacctctgtgtacacagttttcttaaaacagattcgcttcctcatcgtaggtgcttgagctttagtttgaacgtttgtatcctaggatacaacagaataatcggtagaatctgagcacttcaatttctatgccagtgaaaggaattcgtgttaaaatagtaccataaagacttagacagaaatggaatcgaactagaaattacacaaagatttggaactgaaaatgataaagaataattttttggtggtgaacagtggaaaaacgggctcagttataaccttgatccccatgaatggcgagtaaatttgttcattagctcaatattgtaatgacaataaccattggagttttaacagttttgtaagctaaaaagtcagttggagaaagcaaaaaaatagcaaaatgtagacactcctaaggggcaaattttgctctgttcagtccgatattcgtgtatacagatcgcacccacaaacaaactcaaagcttgatgtacaattttggtccttaatttacaccccctgcacgcacacgtggagagaacccctatactacatatgattatattcttcaaaaatgtaatcatttataaagtggtctttcctttcatcaacttccttgtggcataaaaataaatgtagttttccctccaatcataaaccatcttccaatggtccacactaaactccaatttctcattcacccgaacatcatttttggcgagtaaatatattatttcgatattctcatggaagagaagacaaatcaatcttgatcttccaaaataaacaaacacgtcctattcaaaatttatgccaaagtcagcccttcaattcattatttttccaacaatcctccacataaatgaaaattgagagagacagagaaataggagacacaaagatttggtgatatatttcaatggttgaaacatgcataggataggtagctattactttttgaacctttcattatgaaagtatatttactttattagctgaccagtagacactatgtcattgaactgatctgccttttatgtaaaagatgatatactatacacataattcttccttgtataatatagttttcattgttatgctcattatggccataagcatcctggttttgtgagagttcattaggattgagcccaacacaatttccttagaagcagcctcacttctttctcacataggtgacttcttatacaagtaactctcattactttgctcgattatcagcgcttaagaatcattaaaagtctattgcttatccttcattcttacgggcattagtgttatatcataggagtggacatgagatattactccccacagtggtttagttaagtctttacaattagattgtccctttgaacttagatcttgggatctttagtcaaccaggttaggtttcctttgtattaattaattcattcaaggacttaagtctaatttcttttgatgatttttgaactaagtctctatttaaccatttggttagcgaattcgcaatattatcctttcaccatacatagtcaaaagtgataactctagttgagagtagttgccttatggtattgtgtctatgatgtatatgtctagacttatcattgtacatgttattttgtgtccttccaattactgattgactatcacaatatatgcaaattgctagcacaggttttgaccatcttagaatatcttctaaaaagttgcataactattcaacttcttcactacatttatttagagctataaactcagattccataatagatatgctataactgtttgtttagaggatttttaggatatagccgcacctcccaatgtgaacaaaaaattcattagtgaactttgagtctttcatatcaaatatcaaattagtatcactatattcttcagtgattgttgaatatctggtatagtacaatccaaaattacaagtatattttaggtacctcggtactcttattatttctttccaatgatcagttctttgattactcgtgtatctactcagtctactaactatataggctatgtctggtcttgtacaactcatcaagcattagactttcaataatcctcgagaattctacttgagagacactttcacctttatttttagatgaatgtttgacttgtatctattggcgctacataatgtgactgacttagaacgagcacatctgacgttcttgaaattttgattccaaatattacattagctaaacctatatttttcatgtcaaatctcgaatttatcatatttttagtggatttaatcattttattggcgctaccaacaataagaatgtcgttaatgtaaagacacaaaatggcataaccattttccctctctttgatgtaaacacatttgtcatactcgttaattttaaattcacactatatcatgacattatcaaatttttcatgccactgtttgggggcttgtttcaagccatataatgatttcaccaatttaatgactttattttcctatcttgataatgaaaacccctcgaatagtttcatatagattttttcctctaaatctccatttagaaaggcagttttaacacccatttgatatacttcaaaacttcgtagagcggcaatcgcaagtataatcctattagatgtcattctcaccattggagaatatgtattaaagtaatcaaggcatttccgttgtttgtaaccttttatgactaatcagaccttatactttttgatagtttcatatgttttcatttttcctttgaaaatccatttgcagccttgtagtttatttcctagagggagatccactagcttccacgtatgattttgaaaatggaatctatttcacttttaatggtatctttccattgacgtccttctgaagagttcacagcttcttaatagctttaagattcgctttctaacatataggtcagaaaattaagaccataagatttttctgtctttccccttttgctacgtcttggttcagcctcaacgttctcttctatttcttggtcttgactattttcaaccgcagtctcatgtatccatttagaagagtttccttcatttttgaatatgtatgaaattatatgctcaaagaatgaagcatttgtcaatttcattatcatgttattgtgtatgtctaagattttagattcatgcaaaaaaatttgataagcactagtattatgtgcatagccaatgaagatgcaatctacagtttttgacctatctttaccttctttggtgttagaatagccactttagcaagataccccactctcgtaagtatttataagaagactttcttcatttccataatttataaggggtcttttccatcttcttttgggatacttcatttaaaaggtaatttactgataacacaactttcttctgcatgttctgaggtaactcagaatttattaacattgcattcatcatttcttttaatgtacgatttttttcgttaggctacatcattttgttgcggtgaataaggtacctaatttcatgtatgattccgttgtgcacaaaattcaataaatggtgcttcatagacaccaccacgaccactttacaacaccttacttttctttttaagcaatgtgcttaaaatcatactagcccgactggttggactgggaaagtcgaaaattggtcttagaaccgggccgatcatggattaataatcgtatattaagaaacccgtttggataccactaaaccggccggttaaaccactaaaccagaaatcagtctcgatttttgcgagttctaaaattccttttaggaacaaacttttactccactattaggccaaccatgcaaatgaagggcccatactgagatgggtgtgtcatgttcctgctactttaatagagtcagtgcctttaacatgttgcactgatttctgatgtgggattccactcaattcccataacactatgttccaaagtttacatgttaaaacttaaactttcaaattttaaatagaatttttcatcttttaatattttcatttattcattttttaaactcaatctaaaattcactttattattagcataataatgttagacatcattttcaaataagcctgtacgattacaattttaacagagtaaaaattatttcaatatatagattattagccttaaagtatcgagaataattatataataataaatttaattagttaaaatagacttgtatttactttgaattattagtatgaaaattaaaaaaataattaatgttatggtatttttgtgttcggtttgaccccgattgaaccttttgaccattgaccttttccgggtcgatacccgggtcggttttcaaaacattttttttaagttgattttaaattttatttttatagagagttctctatggctttatccttacttaagcaaatacatataacaatattttgtgctatcgttgataaaagtaataaagtacttgttgccgcctcttgtttgatttaaatcacataggtcattatgaattaactaaagtggttatgtattctatttaattgatttaaaaaatgaccttgtcaattttaactcaacacaagtttcgtacttatgtttggaatcaataaggaaagcgggtatgcaattcaagttaactagcctacgtaaaatatcataattaacatgttctaatctaccatgccacaaattaaaaaactcaagcacgtaagtagaagagtttactttattcattttcggcttaacaaccattatatttaacttaaacataccattgaaaatataacattttcagataaacattccactttttgataaattaactttgtttgactcaaatacaatacgaacatcgtgcttattcagaagcgacccagacactaggtttttgtagatttctggcatatacagcacattgttaagagtcagctctttccccgaattcatcttcagaatcacctttccttgacccttgattttaggcgttgctgaacttttcataaacaacttctctccattttcaattgcttcaaaagtagtaaacagctttttatcagagcacacatgccttgtagctcccatgtcaatttacctctcttttgggtttaaacccaccttattcacgtcagaaatgacagctatgagattaatctctgacacataatatgacatgtaatcaaccacatttgcttctttctttttctttggcaatctgcactccaaagacttatataacccatttcatcacaattgaagcattaaacttcttttagaaattccatcttttagtcctagcttgattcgtttgctaccagattgtccacacttgtttttgtaggtcttattactgtgaccatgctccacaacattggctttagcaacatcaagattgaaccacttcttttcttaactcttgttatctttttcaatttgaagtctaacaatcagttattcgacgttcatttcctttctcttatacttaagataattcttgaaatctttccatgcccaaggtagcttttcaataattactaccacttgaaaagtatcactcaagatcatcccctcggcatgaatctcatgaagaatcacttgaagttctttcatttgactgattacaacttttgagtccaccattttataatttaagaatctattgacaatgaacttttttgcccctgtatccttagttttatatttttggtccaaagacttccacaagtcctttgcagttttcattgtactatatagttgtataatgaatctactaggctattcatgatatagtttcgacatagaaaattcgaatagttccaagcatcaagtgtactattgcttgaacatctctttcacccttattgagttttataacaccttccatcaagaatctcgcatgtttcaaggtcatagggtaaaataacatttttagatgccaccttttgaaattcatgccatcgaatttctttgatttttttccatgattaaccagaacagtaatgttatggacaattgttcgagccacaatttgactcatagcaagaatgtaaataaacaaagtataaaactgcagagatatattttttgctaagaatattgtaaatatgcaacccgaggcctgtgtatacacaatttccttggcatggaatggtgaataaattcgtctattaatttaatattgtaatggcaaaaaccattggagtttcaacagtttcagaagctcaaaatttgttgaagaaagcaaaaaaataaaaatatagcaaaacatggacatgtttgtatacgtagttgtgctcgtatacaagtttaaggctcgatatagaatcttggtccttgatttgcaccccctacgagcgtacgtggagagaatatttatgctacacatgattatactcttctaaagtttaaccatattctaaagtggtctttgctttcatcaatttcctatgtgggataaacataaatgtagttttccctccaattaccatcttctaatggtccactttgaacttcaatttctcattcacccaagtatacgatttcaatgttctcacggaggagaacacaaatcaatattgatcttccaaaataaacaaatgggtcccatttaaaatttatgccaaaattagcccttcaattcattatttctcgaacaatatatactttagcattgtgatatctactatatgagtaggatgttttcagtaattatttaaacacattctatttttttggtaggttgtattcaacagtactcaatactttttattttccaaactatggaaaacatgattatatttatggtgacattcaatgcatgccacatacgaaagttgtaatatagaattaattaacgatatgccttcaatgtatgtcgtaaaaagagacatctgcatcactgtgtgcgtatggaagccgtaataaagttagtcaacggtatgcctccaatgtatttcataaaaagagacatttattttatggcgtgcatatggagatcataataaagttaattagcagtactctttgatgtatgctgtaaaaggagacatcttttttatcgtgtgcataagtgaaccataataaatttagttatcaacgctctttccatttattatagtagcagtcaatgtgtgccgtaaaaagaggtgactatttacattgttgctttatacggcatttaaatatacatcataaaaagcaaactatggcgtagtactaagatttagaaatttaattcaattcctagcatttttgtatcgttgaatacattttgttttataacacttcatttcattgatattattgttgattacatcaacttatttttttattattacaatattgcacattttcaagtttggaattttcattgttgtaaagcttttagcgataagcatatttaaaatcacatttaaaaaagaaatttgaatttccttgtcattaaatcttttaatctatcactaaaatactttcaaaaataaaatttcagaacttaaaaatacacaacataaattaataataaaataatttaacttaattacaatgaaatcaactagatgttaaacaaaatgtagtcaaagatacatttaactagcaatcaaataaaagttctgactctggaaaactgtaatatctgttgcaaatttacttaattatgcacagctaaaaataaaaatatatttaaattcccactaaagatttactttgtgtttagatagaaattgcgattgaaaatatagctttgatgaattccttgaagagcaatcttgattagcaattcacagctatctaattgtccaacttccaatgaaaatctacatagggaagaatattgagagaactatgataattctttttcttgtgatagcaagaatataattgtattgtattataaattttcaaaccttagtagccgattaataaaagttcaagtgggcttagctcgtcttttaaacttaactcggtctaatatttaattaattcatttaattaaatttggtccatgaattaattaatccaattcaagcttattaacaagcaacccaattaattaattattcaacacttgtcaattaattaattggtaaatcattcttctagttctcttttttatgtgtgacccattaggtttctcatcacgatgcccaattacttgaattattattttgatataatcaaaatcgataaaataaaatacccatcttaatttatcatcaattcacatcaacgtcctagattgacatccagcagtgtgttagagcaatatatgcgaaggaaaatgttacatggtataacaaaacaaaacttgttcatttatcatgaaactataatcattcgtcaatatgatccgataaatttttagatatggaagtgtgtcaaccttgataatcaatcatttctttcatcctactattaagttaatttaagtcgaagattctttttgacttatgagtacacttggccaatgatttaattatttacttaattgaacgaaatgtaaaccataatctcttactattaaaaagtgacgaatcgtctattgatcatttacaaccttcaaatgattcttgatatacccaaatgatgtcatattactgactcttagtagagcaacacccattatcaccaaagtatgactgtcttcatataaggcactatgatgacatcaaatcaaatgaccaatttcactactgaatgttagagattaaccactaatattcaaatagttatctatgtgaaatctatgcagtgggtctccaatttcttgttctttaacaaaacatctacattttcatttaaatgtcattgtaatttgcctctgacaatcacaactctttattattaacaatttattaagacttgaatttttggattctattagtttaatatattcaattaaataacagatgttactaatatataaaatatattaatcatattaagcccccgtttgatctccattaaattcaattaaattacattctatttttctctctcttattttcaaccacacaatcttccataaaataatattacacaaatcaaaaactttttcttctttttcaaccactcatttataaaatactattttccttattttcattttcaggtaatggaggtcaaacaagggctaaaagtgcttacaacttaaatccattgaatctggagtataatacttacaatatcccaattttttttttctagaagccaggaatgatggcgcattgggtttctcaggccaaggaaactaaagatgaaattcaaaaagaaattgaagaagaatcctgtcaataaactttttatcttttccatctcaaatctaagcaggggtaaacatagcttcgtttggacgattttcgacctaatttcaaattataccattttaatagtttgtaaaaaattattatttaacgaagaccatgtatttaatccaagaacaatcaattctaactatagtcaaatggccaattttgattgccaaatctatgctaatttatctaactaaaaaattattctaatgcgcaaattatgagagcttttgtaaaagtatgtggaacaattattaatacttcggatctccattattatttcacttaaatacaaattaatattgtcacaacccccattcacaaaggtaaccatacctaacaatacattaacctatgtaggaatgaaattgaagactcgacttggatataaaatttcataaatacattttttttcacttgataaaatgaaataaacatcttcacaattatgtcactgtttgttaactcctaatcacatgtgacgatcatatagtatatcaaaatcaaagatcatacagccataatccaacggatatgttctaagattataaacatatctacgggccatttcaaaatgtatacaacacaggatcccaaaatataacacaataaactgtaaactcaaaacaatagcccacaaaataaccctacgggttttcatccatgtacatcaaaccctgaaatccgataagagctctacaactagccatgatttctacgtagttccatgctcacctacaatgcaaaaactacataagctaatgcttagtaaacaaaaatcatgcatgtcatgagtatgagtaacaatgatatatgataccttgtcattcattttaaacattatgctaaagatgcatcatatttcaatattcatcaaagtcaactcaaaatcatttcatttgaaatctttcatttcattaagctcttgatccacttactatgcactggatagaacactgaataatatcaatatcaataatcaaatggtcaatataaaatcgacactggcgagtggaccatccactcgtgaccactagaggcccattccctaactacctctatgatcactcaagaagtattccaccccgacagtgccaatagtcataatatcacaaggacacagtcgagtggtccatcctttcgtgatcacccaaggcccatcccctgtctacctttgcagtcacccaagaagtatcacccacgatgccaaaacatatcacataatccggcctcacatgtcttagtgccccagttgtggtcaataaaacatttataaggaaaactcaatttgaaatcatgtttcgcatacaaagttttcaaatatgatcatatgtcgtgcatgtcgataaaaatgctcgtgaatgacatgcttaatgaaagtcgatgtcaatgagtttcacaactgcatactcaatgatcataaccatcatatgatatgcaatgagcctcttatgaaagttatgtaaatattccaacgttactataccataaatactaggttcttacattgtagctgcaaatgaatttttacttacctttcgctcttgtgtgtgcaagctcctatggagtgcatatcaattttgttttttgctcaaactcaaaaaatcacctgtattaccatctaatattaaagacaatcctcaatttagtaatcttaatacacacaacccaaaaatacgtccattcacgcattacaaactacccccataaatctcgctatttctcgagtccagtcatggacgtcaacgtcatccagctgttgtcaacaacctagtacaccttagaatctattttctaggctcaagaggtcattaatggacatgtaaaggttgaaactatgtaaaccaccaaaatggacagaatctgttttttggtctccatcaccatccaattatttttcaaattcgttttcacgcccttaactatatccgacgactcccaaatttttaccgcacttctataatatatatgtgaaggtaatcttgtcataaatctatgataaatgaagggttttcagccttaaaaccagtccattttccatgaaaccaaatcaggcagttttcattgtgacagtttttcaattttccattgtattagcatgcgaccaatagaattctcagtcattaaaaatcatttctatacttcatgcttccatgtgtaaatgttcatattgatagatataagttctactctaagaattatccaacatcaaggtttaaattattcaactcaacaacctacatcgctatccaagttgttttctcccaagttcttgtaattcattacccttattttgccatcataaaatcattaacaacactagcacctaatcataggaaagttcacatgttcaaaagatcgcaaatcaaatttcgagaataaagttgtaccttgaagttgatcaaacaagtcataatccttggtagtggatgtttattcttaattattaccttattcagttctcgataatctatacacaatctcattgtaccattatttttccaaacaaataatactggtgtaccccatggtgaaaagctagatctaataaaaccttttatccaacaacacttgcaattgtaactttaactctttcaattcaattagggccattcaatatggacctttggaaattggaggtgttcgtagaattaaatcattcacaaactctatctcatgatctggtggtaccccatgtagctcatcaggaaataactctgaaaattcttgtgccacgggtacattactaagcttcggattgtattgtgcttcactagctataacactaaccaaataccctatacacctactaactagtaacctctatgctctcaatactgatataactggaaatctgaaacctttcccaatcccactgagtgtgaatggttcatttcctaaaagttgaaaagttactaactttctcttacaatctatagtagtttgatatttcgataatcaatccatacccaaaattatatcgtcatctctcatatccaacacaattaaatatgcatagagttctctattttttataaggatcacacatgctcttaaaatcagattggtttgttgtacatctccaaatggaatagtcacgctataattgacctcttttacattagttatcctacctaatctcctcatatactatatagaaacaaatgaacgtgtagctctagaatcaaatagtacaagtgctggaatgccaaagatagaaaatttacctgtcacaattgatagatttgcctcagcatctgatctagtaattgtaaatatcctagctggtaccttcttctactctataggatttggatcacttgggcatggtctagcaagatgtcccacctttccacaaatataacatgtcttggtctctgtaagacatgctccagtatgctgtctaccaaacttggagcaagatggttgtgtcgtcgaggcttttcctggatctatctttggacacttgccctaatcccactattattgtccttgtcttggttgaaacttaggcttcttactctgtccctgaaatgctctcttcttatcactcttaggccaacgctgtccatgaccttgtctaaactataatcaagcttcttgagcgcgactaattctttgttctgcttgctctgcaatttgaaaatgctttctctgcaatttgaaaatatgagacaccgtgagttcctgtcatgcgtacatctatataaagttctagtgttagcccttcaagaaatctttctacttttagctcatcaatattaaccatgtgggtggcaaacgtggatagttgctcaaacttacgaatatactctcctattgtcatccctccttatcttagctgtataaattcattcattttcatggctcgaactggggttgtaaaatatttattatgaaataactctttaaatctatcacaagtcatagcatttacatcttcaatgctactcatcatatcccatcagtgtccagccctgcttcatagcataaaggatgcacaaactactttttctacttctaaaactctcatatacctaaacatattctccaaacttctcaaccaatcctccgcagctgttaggtctaattcatcctcaaatattggaaggtttatttttctaaatctttcccccaactacctcaatatgttcagccttttttttgtggttgtatgaattcggccctttgctattctctcctttctttttgttgaattaattgctgaatttgatgagaatggcgctcaactaatttcgtcccaactatcatttaaacagacgtttcttgtcttagagtgctagctctattgttactggcatttctggttctcaccatggctgcataaagattggccaatatcattcataaagtatgcaaaatataatgcaacaaaataaaacttactagcttagctctagtctttcgtactccaagatcatgtacatagacaatctacagaattctaaccttgctatgataccgctctctgccacaacccccattcacataggtaaccatacataaccatatattaacttgtgtgggaatgaaattgatgactcgaacttgacatagaatgtcacgtatacctttttttcacatgataaaatgaaataagcattttcaaaattgtgtccatattagttaactcctaatcacctgtgatgatcatatagtatatcgaaatcaaagatcatatacccataatccagcacatattttctaaggttataaacatatctacgtaccatttcaaaactatacaatacaggatctccaaaatataatacaatagactgtaagctcaaattaacaacccacaaaataaccctataggtcatcatccatgtacatcaaactctagaatcccgtaagagctctacagctagccatgatctcaacgtagttcaatgctagcctacaatgcaagacctacataagctaaagattagtacgcaaaaatcatgcatatcatgagtatgagcaacaatgatatatgacaccatgtcattcattttaaacattatgctaaagatgcaccatattctaatattcatcaaagtcaactcgaaatcattttatttgaaatcttttatttcattggaccattggctcacctactatgcatcggatagagctctgcataatatcaatatcaataataaaatggccaatatgaaatcgacacgaagaagatattagaaaccaacctatttggactttatatagttgatttaaaacagatggcaaggactaagagaacatgcaggaagacatgttcattgatgcctcatcgatatgagatagtgggctagtatgaagagtatcagtgaaattcagcacatgatattagccagcatattagagagatgttagtaaggtggagagaggtgaggcaactaggtcatatggtcactggtcgtcagggcaaccacttccttattgatacattgcaaaacaatggctagatatggccgaatcaatttacaattatttgtggagagttgtcatacccactctgccccgagagattaactatgaggcattctgcgtagagctgacggtacaatgggaggaagcacgagatgatgcacttgtatatcccgaaggtgatagagtgcctattaagatgtacatttaggaagatgcacctccacctatatcagatgatgagtcacaaccttttaagaaaaactgggtttcatggaggctggattaatgccaatgatggcaatgaggaatagtggcatagatttttagtagattttatttggtttaggtcaagttaacattaagtagcatttcctttcttctttttggttgattagcatcaaacgttctttcaagattgtttttcccataaaggatttagttaataataaaatatgttatctccaaattatggttcccatttattgtgcaatgtttgattactatgattttccaaaagattacaaacccattccatttgtatgaaggaaaatggcaccaacatcgcacgtgagagcaatcagagaactgcaataagcagtggaggaaatgagacgggtcttaatggcacaagttacttttgaaaacctaagaacaactaactaagaggggatgaattggttatttgatactttttcgaaaataaacgcaaatttaagcaaataactatgaataaagaagataaaacaaaattaatgagaggaaaggaaaagagagtgcaaacgatgtaataaggaggttcgatccaatcacgaactacgtctcccattaccaagctattcgtcacgaacaaggcctttttcactatattgattgacttatggtgcaatccaaccttcttacaacgctttcgatgacttacaagcaaggagcactgttcctttacagtgttgaaattttcgggacttcaactcgacctacaagtttgaaaaataaggagtacacaagtgaagacttctcttgcaataaatgatataattgaagttgaatacaacaagagaaggtggctaacactttagtaaatagcaatgattgaagctcaagtgttagataagaaaaacactttaataaaaatgatttccaaaagttgaatcaatcaaaggtttttctaatgtaaataagttgaagaaatagatatatataaagatgattgagtagatagattagtaatatctcactttaaatgctcataaaagtctctatattgaatgtaaagtgatctggtatttatagcaacaaaaacggtcaaaagtttctgttctaccggacaaggaaaccggactccgctattttatcggatggtcaaataatcattttttgttcagaagtcagaacgttcgatttcttgaccgttggacaaacctgtcatattggacgtccgctagaattaacgaacttgtccgctagacctaccggatgcatcatctagctaccggatgcgtcctttagatcagcacgtttttggaattttccttctttaaataatgtaacaagatgtaaattcatgaaggatgtttataacatgttttatggactttttgacttttcttaaagtatataataggttcttgcttttctttctgcaaaaatcgtgtttgtcatgtgaagaaacgtttcttgagcttcaaaggacgtatatgccaaatactaaagtgttttaccttagcatttgaaatcaaggtgtccaaatttattttcttctaatttcttctttgtttgacttgatgaagtgatcgttgtcttgatgtatagcttggtttctactttgtccaatcttgcaagagctccgaaagcatccttttgtccacgcttgtgataaacttctataatcacttaaatacaattgttaaataaaatacgtttgttataatcaaaatgagaagtcaaccgtaggccaacaattttccccattttgattatgacaaacaggagatgagggacattaaaaaataagtaacgaaataatttcccccatcttttatacgtgtattcctcccttacttaagcattcctatcatgcatatcgtctcatttatatcataataaatcatgtatatcatctcataataaatcatgcatattattcatgtatattatctcataattgataaatcatgcatattattaatgtatatcatcacaaaatttttccccttttggcattatcaaaaaattgacaaacaagagaagtgacataagttcacaatatcataaccaaaatgccaaaagataaagtcataatgagttcgagagtacacaaaaagatgcataagataaatgataaaactaaaagctaaggctccggagaaggtggtggaggaaaatgtgcgtaaaagtgagcatagagcgcattctgctaagcttgtattttagcttgttgtgcaagaatggcatcctgccgagcttggattgcggcctgttgtgactggacattatgaagaacaccactaagcccatcaaccgaagtcgtgagagagtcgagacgcccggtgagtaaattatactgatcctcagtaaaagtgaatcctcgggaagaagaggaagaagtactaattggtggtggatgcgagagtaatgggacgtcttcttcatcctcaaatggtaatgtagaaagtcccgaggcggggtcaaaccctttagtgtaagccacccattttccttgagttttagagattttcatacgcttgagggtttgaatattgattgtatcagtggcacaaggtttgatgacggcttccccctcaagagagacattgaagtgtttgaaaatttttgttaaaagcataccaaagggcaaagctttggaataacgagaagtatagataagtttcataagacctaaagcaattgttgggaaatctaactttcagccaacgagaaatgaatcgagaatgaacaaatcaaaataattaacctcatctcgatgcccttttctaggtaagataatatttgcgatgatattttgcaatattttgcaaggtaaagtgagttggttagcactaatttttgtgatgttttcaaaatctttccccgtcacacgatgacatacgtcactagggttataaccttctaaggtcgggtgagctttatgaacaaaaactttcgtatcacatggttcaagcctaagaatttcctgaataggagctttagtaacggtgaaccttacatttttaattaaataagagatactatcagaacgtggtgtaataaccatttttgtataaaaagttttcatgagttgaggataagcattttcttccaatgaacataccgaaatccatcccatattttcaaagaattcttgaatgtgaaaagcagatgcttcaacagaaaaagttgaaaaatcaacatttttacctagtagaatgggagatttttcaaatgggtcaacacctcttcgggttcaaaatccatttctttgtcggaggagggtgttggaggccgatgttccgtagtttttaccctttttccagcttgctttgttctcgacattgattgaattgaagcaaaatgatgaaaatccagagttagggcacaaatttgggaaatgagaaattttgaaaacaaacgcaaaatctgtgagggatagatgaagaagatgaagtgtgttaatggattttatgttaatttgtaacaaattagacgagtggaagaaggcttttgagtgaagagaggaggagagttcgaaagaaaacggagaaggtgggaaaatgaaaagaaaaagaccctgtcacatttttaaaattcagaggtttcagtgtatgggacgtccgataagatttgccgaatcatccggtacggtagaaaaaaatttctgttgagccggatgatttaacggacgcgtccggtataattgtccgatatgtatcggacgcgtcagataaactagtccgaaaacatttttttttaaaaatagaatagagaaattaaagaaataaaaaaaagtcatgcaaaaaatgatttaacacttaattaacttcattttcgtcaagaatacctaaacctcttcgaatataaaaaaatcgatcatgcgctagaggttttgtaaaaatatcaaccaattagtcttcggtctttataaattctaattcaatatctcctttttgggtatgatcacgaaggaaatgatgtcgaatctcaatatgcttagttcgtgaatgtgaaatgggatttttagacaaatttatggcactagtattatcacataaaataggtatatgatcataagtcaaatgataatcacataatgtttgtttcatccaaagtgtttgtgcacaacaactagcggccaagatatattctacctcggtggtggatagtgcaacggaattttatttcttactagaccaagacacaagtgcaaagcctagaaagtgacaatttcctctagtgcttttacgatcaacattacatccggcccaatcggcatccgaataattaattaagtcaatatgagtgccttttggataccaaagtcctaaagttcttgtaccacttagttaacgaaaaattcgttttactgcctttaagtatgattctttaggattagattgaaagcgagtacataggcaaacactaaacataatatcaggcctactagcagttaaataaagaagggattcaatcatacctcgatattttgtgacgtccatggatgtaccttgctcatccttatcaagctttagagatgtgctcattggtgtgttcataggcttgatatcatgcatgtcaaatttcttaagcatgtctaatatgtatttattttgatttatgaaaatttcttctttcatttgtttaatttgaaggccaagaaaaaattttaactcacccatcatgctcatttcaaattctttactcatgcattttgaaaattcttcacaaagataaatatttgtagcaccaaaaataatatcgtcaacataaatttgaacaatgagcatatcatctttatgagtttttataaaaagtgtagtatccgcttttccaatcgaaaaatcatttgagagaagaaatttgctcaaccattcgtaccaagctctaagagcttgttttaaaccgtaaagagctttttgaagtttaaatacatgaaccggatacttgtgatctttaaaattgggaggttactcaacaaaaacttcttcttgaatgaaaccatttaaaaaagtacttttaacatccatttgataaagtgcaaaatctttgtaacatgcaaatgcaagaagcatacggatggattctaatcttgctaagggtgcaaatatttcttcaaaatcgataccttcttcttgattgtaaccttgggccactaatctagccttgttacacaaaattattccattttcatctcttttatttctaagaacacattttgttccaataacggtttgattgtttggtctagcgactaagtcccaaacatggtttctttcaaattgatttaattcttattgcatcgctagaactcaaaactcatcaaactcggcttctttgaaattcttaggttcgatttgagaaataaatgcacaactaccaaaatgatttttgtaagaggttctagtagtgataccttttgatggatcgccaattattagctctttgggatgagatggaacaaacctccattcttttggtaacgagggatcactttattctccggtttgtctttcttcattttcttgagcatttgacttttctatgtctccatttggtacctccttattttagtcttgaattttcatttgttcgaaaggagcttccaaacctacatcatcataactatctttctctcgatcaaatgagttagtttcatcaaaagtaacatgcatggattctttaacgactagagttcgtttgttaaaaactctatatgctttgctagtcgataaatatcctaagaaaattccaatattggatttggagtcaaatttccccaaagtgtcttttgtattcaaaataaaacatttacatccaaaaactttgaaataacaaatatttggaattctatttttccaaagttcgtaaatagttttagttttccttttgcttactaatactctattgataatgttgcaagcagtattaacggcttcggcccaaaaatatttaggtaagttattttcatttaacatagttcgagccatttcttgcaatgtacgattcttcctttctactacaccattttgttgaggtgttctaggaaccgaaaaattatgttcatatccatattctttaaaaaaattatcaaacccaacattatcaaattctccaccatggtcacttctaatagttgaaatagaatagcatttttcattttcaactttcttacaaaaatgtttaaaagttttcaaagcttctttttttaagcttaaaaatataacccaagtaaatcttgaaaaatcatcgaaataataaaagcataatgtttacctcctaagctagctgtcctataaggtcccaaaagatctatatggagaagttgtaatggctttgtggttgaagtataaagttttggtttgaaagaactttttacttgttttccaaattgacaagcatcacaaattttatctttttcaaatttcaaattcggtaaaccttttacaaaacaatttttggaaatttttgaaagaagatctatgtttacatgtccaagtcttatatgccataaccatgattcttctttcaagctaagtaaacattttttattattttccatttcaatgtttataatataaacatctttacttcggcttcctataaaaatcacctatttcaatgtagcatccttaataagacatttggaagaatagaattttatgttataacctttgtcacataattgactaatgtttagtaaattatgtttaagattatcaacgagtaaaacattttcgatagagggggatgagtggttaccaatgtttccaatgccgattattttacctttggcattatctccaaaggttatatggccttcatcattctcttgaaagtttgataataatgatcggtctccagtcatatgcttcgagcatccactatccaagaaccatttactttttattttctttggtacctacaaagacaaattacattttgacttttgatacccacacaaatttgggtcctcgatagttagtttttgtagattcttgtatccacttgtatttgttttcaaagaataatttctttttagttacacaattaaaagcaatatgtccacttttattacaaaaactacatgaaatatttgaagccttaaaaaacatatttttgagtgatttttgttttagagagggtttgtatccaattcctcctttatcaaaaacatacttttgactaccgagcattaaatcaaaatttttcttactttcggtaaacttatggataatttgtgttaaatcattaactttttttttcaaagaaatgttttcttttatcaaaaggtcatgatcaatactttctttttgtttttcgaaattttttttaatttcgtctttcaaaacagagtttttctttttaagaatagcatgatttaaagcgagtttttcaaaattttcaagcatttcatcataagaaattgaaagctcatcataagaacatacctcgtcttcggttgccatgaagcacatatttgccactttatcttgactatcatttccattttgtttttcgtcgtcactatcatcccatgtggcttggagtgcctttttcttgaaatttttctttttgtttggacactcggttctcttgtgacccaacttgtcacaatcatagcaaacaatttttttgttcctatcttcccctttttcttctttcttttggaatattcgattattacgaaaacctctccattttttgacaagaatgaccaaatcatcaagttcttcatcgctcatattttcatttgatgttccttcttcaattgccgattttaatgcaatttgtcatttaggaggctcctttgattcctccttgctttttctcattttctccttaacctcgacattgtttagctcatatgtcattaatgtgctgtagagctcttccaaaggatatgcatttacatccttagtgttctcgatcaacatcctcaatggactccattcctccgataagaacctaaacattttagtcacaagttcaccgttagtaaatttacgatcaaaacctttaagaccatttacaatattggtaaaacgagtaatcatgtcaacaataggctcattttgtttcataaagaaattttcaaattctttaactagcatatttatctttgtttccttaactttacttatgccaacatgagtaacttcaagagcatgtcaaatatcatatgccgaatcacatttactaattcgattaaattcatttctatcaagtgcacaataaagtagatcttttgccttggcatttaatgatgttttctcttatcttcatcatcgtattcttctctagatttggggagagtttggtccggtctaccatctactttaatagtcttagtgggagtatatggaccatattctataacttcccaaatattgtaatcaatagattgaacatatatcatcatcctagccttccaatagttataatgtgtaccatcaaagaaaggaggcgggtttgtagagtgcccctcactattttgaaatacttggttagccattactcaagattgtagaatctcaaaaaaaaagagtaccaaactctaataccagtggaaagcccaagaataactaaccaagaggagggtgaattggttatttgatacttttttgaaaataaacgcaaatttaagaaaataattatgaataaacgagataacacaaaaataatgagaggaagggaaaagagagtgcaaatgatgtaataagaaggttcgatccaatcacgatctacgtcccccattactaagcactccgtcatgagcaaggcctttttcactatattgattgacttatggtgtaatccaaccttcttacaatgcttttgatgacttacaagcaaggagcaccgttcctttacaatgttgaaattttcgggacttcaactcgacccacaagtttgaaaaataaggagtatacaagtgaagacttctcttgcaataaatgatataattgaagttgaatagaataagagaagatggctaacactttagtagatagcaatgattgaagatcaagtgttagataagaaagacactttgataaaaataatttccaaaagttgaatcaattaaaggtttttctaatgtaaataagttgaaaaaatagatatatataaagatgattgagtagatagattagtaatatctcactttaaatgctcataaaagtctctatgttgaatgcaaagtgatctggtatttatagcaacaaaaacggtcaaaagttctgttctaccgaacgaggataccggacgtccgctatattaccggacggtcaaataatcattttttgttcagaagtcagaacgttcgatttcttaactgttggacaaacctatcataccagacgtccgctagaattactggactcgtccgctagacctattggatgcgtcctctagctaccggatgcgtcttctagatcagcatgtttttggaattttccttctttaaataatgtaacaagatgtaaattcatgaaggatgtttctaacatgttttacggactttttgacatttcttaaagtatataatatgttcatgcttttctttatgcaaaaatcgtgtttgtcgtgcgaagaaacgtttcttgagcttcaaatgacgtatatgccaaatactaaagtgttttaccttaacatttgaaatcaaggtatctaaatttattttcttctaatttcttctttgtttgacttgatgaagtgatcgttgtcttgatgtgtagcttggtttctactttatccaatcttgcgtgagctccgaaagcatccttttgtccacgcttgtcgtaaacttctataatcacttaaatacaattgttaaataaaatatgtttgttataatcaaaacgagaagtcaactgtaggccaacaactttagcagtaccaatggctctaacaagaaaaaatgtacagatagtgccaacttgttgcgatataaactacacatataccacccattacttcagtagcaaccactactccaactatgccgatcatggagcagctacaatatccctttggcagtagaggaatggctccacacaattaaaaaaatcttttgacacatatcttgtccagaaaattagagggtgttgtgtaggttggaggagccgtacattgatgggagtccacatcatatacatggacagaagaagaacaatgtgatatgacatggacccaattcaaggtagagttgactgagaaatatcttctgcaaacccttcgtgaccataaggaggcagagtttttacaattgatatagggagacaatgacatcactggttacaagaggaaatttgagaaattatcccattatgccccacattttatgaatacggagtttatgaaaataaaccgatttgagaagggactgtgccccaagattaggtagataatgatttcacatgaactcaccatttatcgagaaattgtaaaaaaggcccaaatcttatcattctcaagttacaaactttgaagttagggactacagaatgatactggaaaaagtaagtggcatgatcagggtaaggataagagctctggatagttcaagaagtagaataacgggcttactagcagacaatcaaacaatcattttcttccatgccctaagtgcaagaaatctcatagagtgaatgttggtttggcaagaatgtctattacaagtacgtccagtcaactcactatgcttttggttgtcgggcaatgctgtctaaggatgttgaattggtgaagaaaggaaaggcaagaatttttaccatgatatatgatggggccacctaggagccagacgtaattataggtattttaactgttcgtaatattttcgtttacgtccttattgactctactgcgacacattcatttatatgtgtggtatgtctagcgaagatcaatgttttatgtgagagaactagtatcatactagaagttagtatgccatcagaaggaatcattagtacaaataagattgctaatacggcaataatagattttgatgggctaatccctgaggcagatttacatgtcatagagttaaaggattttgacattattttgggtatggacttgttgaggatatcttgttagccttgcgggcatgccattagaagagttaacattggataaagtggctttgtacaggattacactgacgtatttccttatgacctaggggtgcccatttgatagataagtagaatttacaatagatttggtacctggagccacattggtgtttaaggttttatatttgatgacacaaaaagaactacaagaattaaagatgcagtcgaatgaacttaaaaaaaaaggtcttatcaggccaagtgtgtctccatagggagctctggtactttctgttaaaaagaatgatagaacaataagaatgtgcattgactattgagagttgaacaagctgaaagtcaagaataagtatcctctcccaagaattaaggatttatttaattaattgaatggtgtaactgtattttcaaagattgatttgaggtcaggctaccataaactaaatatcaagccaagtgatatacttgagacatcatttagaacttgctatggacattacgagtttacaattatgccattgggacttactaatgcccttgcagtatttatggatttgatgaatagagtatttcagtacaaggacaatttaatttattaataacaaactggtgtattcgagagattctcagcagcatgaatatcatttgaggacaatttttaggaactttacataatgaaaaattctacaccaaatttaataagtgcgaattttgacttgatttaataggatttttggacacgttgtgacagctagtggtatgagatagactcgaggaagtatttactaaccggcaaagacttgtgaatattggggacatgaggacctttctaggtttggctagatactattgctgatttatagtaggtttttctaggacaacaggtcgtttgactaacttgaaagaatgtgaagtttgtatggtccgaaaaatgggaacaaagctttcaataattgaaagataaactagtattttctccagtgttagcaatccaagaggaatcgaggagatttgttactatagtgaagcatctaagctagttttgggttgtattttgatgtaatatggaaggaatgatagcctatgcatcaagaaaattaaagcagtatgagaaaaattgtccgacgcatgatttaaaacttgcagtgacagtttacgttctcaagatttggcatcattacttgtattgaaagaagtatgaaatttacagtgaccataatagcctcaagtacttttttgcccaaaaagtattaaatatgagacaatgatgattgttggaatcagtaaaagattatgattttaatatcctttaccacccaagtaacgctaatgtagtagcagatgctctaagcaagaaaaatcttgatcatttatctgtgctatgtacacagcagagccagttaatcaaggactttgaaaattcgagaatagaagtgctaacaatactagctccaatacaggattatagcagtacaaagagatgaccctttattggagaagatcgaggccaatgttggaaccgagaaaaggaaaggatttgagataagcagtgataaggtacttatgtttaaaggccgactatatgtacctaaggatgaaggactaagaaaggagataatggctgaggctcattccgctccttatgttgcacatttaggctccaaaaatgtacaaagacttacataatactttttggaggagaaatatgaaaggaagaataactttgttcatatcaaagtgtatatttttgtagcaaatgaaagcagagcatcagaggccatcagggttattaaatccaattgacatactagaatagaagtggaaaaagatttcgatagattttgtagtaggttttcttaggttggcaaaaggtcatgatgtcatttagttcgtagtagaccgacttacaaaatttgcccattttctatcggttcgtatgactttcagtctggaacggtattcacgattatatgtaagagaaatcatttgacttcattggggtaccaacgtccattgtgtcggacagagacccaagattcaccttaaaattttggaagagtctttagatagctatggattcaagattgtctttcagcactgtatatcatctcagtccgatgggtagctagaacgaactatctaagtactagaagatatgttcagagcatgtatactagacttgggtggtaaatgtgagaaccttttgccactagttgagtttgcttacaataattattttcaagctattatcgatacgtcaccattcaaggcattgtatggccgaagatgtcgttcattgatatgctgggatgaggtcagcgagaggggaatttcaagtctagaacttattgagaagattgtggaggctatcggtaacatcagaatgaggattcaaatagctcaagatcaaaaatagagttatgcagatgagaggagaaaagaactagaatttgatgttagagagaaaatatttctcaaggttgccccaacaaatgatactatgatttgaaaagagagagaaattgaaaccgagatttatcggcccatttgagatctttgagaagattggaaaagtggcatatcgtttagcactgctacctgagtatcggcaatgtgtgacgtattttacttttctatgttgaggaagtaaatccacgttccaagtcatgtggttaacgtttagtcgtaggacgtgaagaatgataagacttacgaagaagcaactgcaataattttagataggaaggtgcacattttgagtaatcactaagtgccatcagtcaaagtctagtgaggtaaacatgggaaagatgggactacttaggagagagaagcagatcttttagctaggtacccagtctcctcaaccaagagtgttaaatttcgaggacgaaattattttaagtatgaaggatttgtagcgagcaaaaaataaaattgcatttaattcattttggtacgttttgttatatttaggatgttgtggaatgtgaaaataaatttcaacatcattatttttattcggtagaataatcaagcatttatttaatgaaaatttccccgtcaatattagacctattttgaagctcacattaaactcgaattttagactcaagacgaagttagataagttagtttcatgtttttgtagctcaaagaaatccatatttaactaatattagttaagcgtgttaacaaattttcaaccacgtgtgtcactagacaagtgaattgatgtattgatttaaatataagatactttgaattagtttgttttccatttgaattctatgtagtaccagttgacccatttacaacttaatttacgtgtggctattccacaattaagaccataactaagagacaggaacagatttagggcctcgctggactgggctgtagcccagtgcagtcttgggccaaataccatttttgtgtggaaaatttctggaaaaaaaaagttacagaaaagttcataattcaggagtattctttataccaattcaagaatgagctagattatttaaaaattcaaaaatcaggtatatatttaattaaaaataatgatgtcacagagacatcattataggtcacattttatttatttttagtcaaatattactttgaggtcacaaatcaaaagttttatatatcacaaattgtcaaattaattagtcacatattatttcgaggtcacaaatcaaaagttgtataggtcacaatttatttctttgatcacaaatctaaaaatttataggtcataaattatttcgagatcacattaattggtcacagattatcaaatttttaggtcacatagtcacaaataattaaatggtttgtcacatacgtcaaatagtggtcacagaccaccaccaccaacactatcgcaccgtcactagcatcacgatggtcacaaattaccaaatttttaggtcacatggtcacaaaaaaataaatggttggtcacatatggtcacagaccactatcgcatcgccactgccatcacggccacttgcaaccacccttaccccatcaccgacgtcaacatcaacaccaacaaaaatcaagaccaccactgaaaaccatcacagcaaccaaattcaacaaaaatcaccccagtcgttagattcaccaccaccaacaaaaatcacagccaaccgttagatccaccaccacatccaacgaaaacactgccaccgcctcaaattccacaaaaaaatctccaaatccgtcggttggcaccaccaccaccatctcaaatcacaacccataaattacatacaaccacaaactttgtctactcttaaccacgaacatcggaaaagtggttgttgggagtggaggtagttcgccactcactgtcagaagacggggaagcgacgatctgtactgcaaacatccgacgatattcgccgccagcctctgttgaataggaaaatggggaaaatgtgctagattcaagggaagcgacgatctggtgttgcgaatggaggtggttcatcgctggcatgaactggttcgtggggaaaaatgaggtgaatgaaggggtaagtgaatgaagaggtggtttgtcgccgctgctaatggaggtggtggttctggcgcaacttgagggagtgaggagagagagtgtggtgagtgcgtgcggggtgagaagagagagagagagggtggtgtgaatgaagaggtgagtgaatttattagggtttgccatacttgatttgtgaaaaaattaaacttctgccttgatttttgatttgcaatctttaaacaccagttattaggtaattttctcaaaaagttatagctcagcccaaaattataattagctcattgtttccattccaaagtccaacctggtaacccacctaatacattagcccactgtttgactccattaaatcattaaatccaatcccagtccaaaatcaaaattatcccacaaattaactccattccataatttccattgaatccattccaaagtccaaaccagtaacccacctaatcattaaatcatgcattcatactcctcaaattctcaaatctcaaattcttcccgttgattctggaaacgtccaaaggcccaagcttctgcaagttagagagaaaacgatactggcggcaacgtgttctttagatcacagttcatctctaactccgattctttagctcgacggacacaacttcagtcggtcatgtcttgatgaaactttatttcatatactttataaaaatttatgtatatatattttaaattttagcccccctaacatgattttctggttccgcccctgcttgcattactattaaggtaaaaaccaatttacattgctatgattgatatatatttatggcagcccaaatcatcttttttaataagaaattggttatacaataaactatcctgtccacgctattattcgatataccattttcatatgtaagatttgaaaagagataccatttgaggtagtcattgctatatcatttcgaactaaggtaggatttctacactaagttgatcgttatatggatttaattgtcatttttgcatgctattttttacatttgtaagctgtgacaatcagatccggaattacagataagcatattagaaaaataatttagtgcttcgaacgttgttgtcatgatcccaaatttttctatgttatacttctatgagttttatgctatccaataaaatttcataaattttcatcaaggtttgctcgatcaaataatttttgcaaactcactgcacagatggagaaactgtttcagcttgctgtttacctttgaaaaagatataattttttttattaattttatgcttggagattaaccttaaaggattcatgtttggtaacccgccttattattaaaattcagggtgttattattgatatgattacttgttttatcaatattattaatggccttaaaggctttgatcaaaagtttactaacagtgaacttaggagtaaagtgattaggtttctctctgaggattgcagctcattaaaaatgttgatagaaaacactaaaatgtcaacacatactcattggagaagttccatggtaaattgatgacatatcacatatgagttagatcacgtcaaaacaaaggagaaaaaaaagaaaaaacaaagagctttgataaaggaatttcctaggcgttaaattgctttgaaattggaaaaagatgaaggcaaattgagtgaaaacatgaataacgaaaaatttaatgacctagttcttctttcaaaaagtggggcagggggtttgcaacaaatgtctgctccaaaagaaaaatgtaaaaggggaaggaaaaagtaaaaagattgtttgttatgattgtgacaaacttaatcacgaaaaaatcgaatgttctaacaagagaagattcatgaaaaagaaagtactccaagtaatatgagatgagagggatgatgaagaccagaaaatgagagttaagagaaagttgtcaacatgtgctttcatggccatggaaaatgaggtaagatcagatgacaattctttatatgatgaagtatctacctaatatgccccccggggcacagctcaactagtggatcaatcaacattgtcttacttccagcgacagggcggagagttcgattcttggtgggaacctgcggccaaatatttggtatggagcaatcactgtagaggagggtctcttgtgcgcagaagtgtacaggcaatggggggaacctgtgatccagttgaggcatgacccgcgatttaccccctccaaggtaggagcaagggtcttcggggtccaggatttagtctagtgtaagttgggatacctggatatcaaaaaaaaaaaaggtatctacctaatatgatgtggtggtgggagtgggaggaagatggggtaggtggaagagaaagtgattttttttaatttatttattttggattcgtttgtactcttttaaaaaatttgggactatatctcaaattagtttctttattttttccttcttttctttttgttttatttaaacaagcgagtatattcgttatttcacaaggctttattgagaacatatgatgaaagagggtcttctgcgtctgaaagtcattataaaaagattgggtgtattccactatgggttcaaagaatagggggttttgagccaatatacctttatataacctttagtcctttgctcccaatgcttgagtaagatttccaacgcttggtataataatatggttcgttaaaagtttacaagatgttttagctgattctgaagtcaccgctctgctcaataagttgattttatagtgaatatagcttgggtccatgcaaggaccaaaaagcttttatgcctctttttattgaagctcatctctttcgcttttgtacaaaaacttaggacaatatgtgaagaaaattgagttaccattttattgacattgttttgttttggttgacagcaatataaactctgagatcctatggagtaagacctaatgaaaagatagcgtttacagtcacagcaatgaggcaatggtttttagaagtaattacaagaagaaattggttcttttttaatattaaatccaaatagatatctcgtttgatattgatttttcttttttcttttcaaatcttaacacgtatgatgtgatcataattttagaacagattttattggccttctaccccacaagccaaggcttccttatatcttctgtcttgctctctcctttaggtgcttcctttttaggaattaagggtccgttggattgcaaagatggaattaaattgaattgaaaacgaattttaggaaattgaattacctaaaaattattttcttgagaatagtaaattattgtgtttgattagtataatttttcacacgaaaaatgttaaaataaaagtcttttttgatgctcgtttgactttgttttacatgaaaattgttaattaaaatgatagaatttattagaattgggtatggaatttgtttccattgtcaacaaaaaaaaaatcaagaaaatcatctatcttttggtgtttatttgactttgttttacatgaaaattgtcagttaaatggaaattttctttttacaataattcttagaatttatttccattgtcaaaaaaaaaaaaaattaaaaatgctataataaccgagaattccaattctcaccaaaatggtgaaaattggaattcaaggatttgatgaaaaatgctgacgtgaccaagaaaggagaaattcttttttcatggaaaatttcacctatcaaacactacaaaagttgaaaaatagtattgattttccattttccattttccatggaaaagggtgtgctatcaaacacaccctaagagaatgtagttaatatctctagaaatgtgcccataaatgacatatttaaaatactagaattttataattgcacaatttacctggaattttattgtagcaaatcaattaagtctcacacctaaattagagctaagagccgacttacaattaaaactcgagctccaataaatatttctaattgagtcaactcttgaacaattaagatacatacattaattacatccataaatttgaaacttaatcacaatcttcgatttaagctaatttaacagtctagatttattaaaacctttattaggaagtgtttggatgtgagtctatgaattttaaaatattttaattgatctaaaccactgaattagtttaaattaaatgtaatgattatttgtcaaagtcatttgttagattagcagtctcctaaaaagaaatacttaatatgaacggaataaaaaactttcaagttgcaaaccaccaattcaaaggtcgtagaagatttcttcattctcaaatagttttttcttttaaaaagatggaaatcataaatttacataaagaactgaaaatttgtaagatgtcattaattgcatcgtagatgttgatagtatgaattgaattaaatgattttattgatgaacaattacatttgaataacaatatgaatacaatcaacactctcacctaactatgagttccacctcctaaatttacaaatccagatgcttcaactagaataaaaggagaaatagatatttgaaagggaaatatttgaattgcatgtcttcttcttcaaacgagagaggggcatctgtaaatttccctccaagcattgttttgtcatttcttcgttatgccaggtagcaactttttgttggctatcttctaaccaattgtgttatcaatcatgcttatccacctatccacttgccttatattgatggcctataactagcttggatatgaagaatggtttgtggtttttaggcaaactttttgcctctgaattccccttgcacttcactaataactagatgggttcgttgactgttttttgtaagttaacaatagattatagatgtacaattaaacctaataaaattgcattctagcgcttcatttatcaactaaaatcttcctaagaaaatttccttatcaaaaatagaaacaaagaaaaatatgatttttaaataaaatttcaccgaaccataaatatatggagaatggctcgtggtttttatgcaaaacttttgcttcttaattccccatactcttcactgatttggatagtttgctaactgctttttgtaagttaacaagtagtcccccaagtctggttttaatatttatattaaatctagaaatttatttattatatcatcgatgccattaagggttcatcactttatctaatcgttccttttgacaggggaaacgtggggaacatattggcaaccattaccattttatgcccacaggggggctttatttgcatttttactgtttagtgactcctaactcttttggatacacgtttgcacatgacttgcttcttttaccttcggattcgaatggccacccattcattttcaacgattatgattgttactggcatgtttcaacgactaatatcttctgtcagaatctataaatatgtcattatttcagttggtcttcttcattttgccaccttgcttttcctaagtaatttttcttttcttctctttttttttttttttttttaaatctttgtgctcactatttttccacaattctttccacactgactcttagtgcatctggcgattttgatttgaagagttctaattccagaggtgatacttcaggcgactcttcttatactgtggaaaatttatactttgatgtgctctcctataaagctataaccaattttagtatatttgttaacctgagcattttggtcaagtcggaagtttttgtcctgaggacaagacacataatgtggcaagcggacactaatatacccgttgatcttaatgaagacgctgtaagcatttttgaggcttcaagaatctttagctatcttattgaacaagacacggccgaaattaagttttgttccaacattcctaacaatatagagcttttatgtcctaggccatttgaaacatggatcgtccattgctaggtctcacagctatccacaaacattcattagacatgggacccagagtcctcttttacccttgttttagggatgtgctttcctcattaaacatggaaccttctcaacttgctccgggtgggtggcccaattgtctagcttttttgctataaggtacaataggcctgatagggaaactttcttcgaatatatttcataggctttatcaccctaagtcattggggaatactgcaaacccatagaaaaaaggtatgatactttttccctcacttttccatagcatgtctagcgtaggtaattcctcttgcccaagagtcttcttggaaggagggctttttcttcgtccaaggtaactaaaagtttcaactcaatttcctctatagacatgccttaacttatggtgagtatttatgaatgttggtgacacgacttgtcccaaatcaacctaatggactcgacacgtgtcatgtgccgatggtagataccagctaagtgccggaccttggtccaaggcaactttgactgtgacatatttttattttgacagagtttccaaaggactaaaccaacctaaaaatcaacaagacctcatctagacatttaaaccaaaaattttgggatccaccaattctgccaataccaccacaactaaaacaaaatacaactaaactcgactgggtacttctactgtaaaacatcatgtctacatacaatcattacattaattataaacccttctatgaagtgaaaatcaaacaaaatattagacaaagtgtcaataaacatgagtccccaactatacattacatactatgatacggttaagatcatgcgctaaatgacgggtaaccaggctcttggcttcagcaggctttcctagatatctcaaaatcagcggtctcctgataggaaaaacatgacaatatatatgagcttgtaactcagtgaatgaatagtttataaataagtatactttcccgtttatgcatattttctaaaaatttttgcactactaaaacttctagaaattcgaaaatctggtaatacttttaaaatcaaacatgaatgcatcataaaattctttgttcttctttcaagataggcagctgtaagctataataaatataaataatctgatagcagtaaatataagtgaaaatatcctgtcacaatactataaactgaaatcattactctaaaaattgaagaaactaaattttgtagtttgaaatctgataagctttatatattgaaagtcacaccacaaaggtacccagtgaatagccttactcatgtacaaagtaatcccgatgtacaaggcaaagccattcacatctgataatctggtcatacgtacgtagagttgtctcaaagtctaatcaccctaatacacggtccaaagcctatgtgtctacgagagtgggtcctaaagacatctgataatctggtcatacactatggaaacacattcatagtagtgcagagcgagtaaaatgaccttaattagccatacactgtggaacacattcacaccagtgcagactagagtaaaatcacttggtacttttatgtggtttttagaaaataactttagctatactaaaacatgcaatacgaatggaacatgctattgaaatgatttaactgaactagatcaaattttaaaaacaattatttacatatcaactttattctgaaaatcacgctgtcaaatcaactatatgaaataatacattttctgatttaatataaattgaataaatacttattgctgaaaataatattttttaaccgctcacgaagtgtgagctacaagctagactgcctaataaatgtttccaatctcttcggaaccacctgaaatacattataaaataaatatttaaacactgccaaaacaagaaattgtttatctttaatgatagtacttaaattaaatttctcgatacttgaataaatttttcgaattttcctttgatcaagtggagctaattctactttctaataccttcacaaatgtatactacatccaaatttaccttcacccactcataaaaaaattatactttccaatctaatgaaaactaggaaccataattccacccatttaaactttcatcttgtttttcaaattcgtgctttcatgtgggtattccatcaatataaccattcccattaacaataattaatcaaaaatcccaaatagaaatatggggtttgccaaaaattatattgcttaccttcattgaactaaaaattaatccatcaagtaatttaaacaaggattcatactcctttcactaaacctacaagtaaaacccacaaatttaaccaactaattaaaccttagaaatttaacatcataaaaccatagaacatttacttcttaatttcatgaagaaatgaagtaaatgaacccaaacatgaagaaataaatacttacttcccccttcttcttcttcttttctttcttcttttccttttctcctttctctttctcggcctttctgcttctccgtcggtttttctagttagtgtgtgtgtgtgtgtgtgttttgagagaaaaatgggtcagaggttgtaatataaaggcccacttacaaaaaattgcaagggaagtccctcaactccatttatataacatttactccttctaaattccattaatataaaagtaaattcacaactttaaattgtatccaatttaaccctcatatattttcaattataaaataaaccccaataaaatatttaatttcattttagtccttaattgactttgaccttgactagtcaatttttgatttttgactaataaaattttaattgtaacagttggtctattatttgtcttttaatgtaaattaatatgccctaattgttacacccatttcatgctagtcaaaagtcaatattatttattcaaagtcaaaggttcgactagtcaaagccaaggtcaattagggacttaaatgaaattaattattttattgagggttcattttatgatttaagatatatgaatgtttaagatggacatcatttaaatttggggaatacttattaattattagaagttagatgacttaataagatatcatgtgaagtttagaggacttgatagcaaaagggtttagttggtggattacaagtggcaccttgcaagccatttctttcatttttcatatcacatgcatacacataaagaaggtgaaaactggtgcagaaacagggagaaaaaccggcagaagaaagagaaaaagagaagggggaaaaaaaaggaagaaagaaagaaaagaagaaagaaaaggaggaagaggaaaaggaaaaaggacggaaaagaggtaaggttggctttttcaattttatcttcaatttgtctaatttctttaagagatatggtatattttatgcctaattgttagggttttgatttattggtttaattttcagattgtacgaaggaatatgttttgaagccaatatttttgaattgggacggcatatttacactaaggtaagaaataccaattttgggcaaaacccttgaattttatttgagttcttgaacaagtataattagtgaaaatgattatggcaatgatatattaattggaagaatggttttatggaacaacatgtaaatttaattggttgagttatggttattagctttactagattggaaggtggaataattatttttaagattagaataaaggttattgtgatgaattagccattagaaaatggactagaaagtggaattagcttgaagtggattaaaggaaattggagaaaattattcaagtctcgagaaatcaagttttagattccgtcatcaatatttaaaactacttagcaggatagtggttaaattagttattttacattgtctttcaggtggtagcgaagagatgggaaaaacttatccactaccataaagagtagcctgtttggagttagtggatataaaacttattttttcagaaattagtatttattaaatttatattaagtcgaaaaatttattatttcatatagttgatttgacagcataattttcagaatgaagttgatttataaatagttgttttttttaaggttaaattcactttagttaaatcattttattgccatactatttcggtattaaatattttagcatatttaaatttattttctaaaaaccaccagaaagtgcacaggtgattttaccctagtctgcactagtgcaaatgtctttccacagtgtatgaccagtaatggtgattttacccgctctgtactattgtgaatgtgttttcatagtgtatgatcagattattagaggtctttaggacccactctcggacacacataggccttgggtcatgtactagggtgattagcctttggggcagctctgcatacgtatgacctgctgcatacgtatgacctgattatcagattttcagattatcagatttgaatgtctttgccttgtacattgagattactctatacatgagtaaggctattcattgggtacctttttagtgtgatatttcaatatttctacagtttatcagttttcatattatagaattcaggtaatttaatttttagaataaagctttcagcttataatattgagcaggagcaatattttatagattttcatgaatatcaaattatttatagtcattatattttacagttgtttttctagaattaagaatctttaattttatgatgcaataatgtttagttttaaaagtgttactaaattcagaatttttcaaagtttaatataataagaattttcaaaaaatatgcataaaagaaaaggtatacttatttgcaaattatccactcactgaactttaagctcatatatttttttcacctttttcctttatcaaatagatagcagtcgaattgagttggagcctgtcgaaccaccgaatttagccatgcatcataggttgtatgatgtcctttattagattatacattatgtgttcttttaggatatatgtagtttaaatcagaaaagttcattatggtctcattagatatttggtatttttaatatatttgagaattgttggttgtaaagcaagtaaatattgaatagccagcattttatttgaataatttgtattttgagggactggcgtaccctaatttatattataggtattgatttgaggaaaattggttattgttcaggtgattttatttcatattttagggaaaactatgttaaaattttgttaaaaatatttttcagtcaaataagtcaagattgccttggtggtggggccgacaattagttggtatctaccatcggcacacgacacatgccggatccattaaggtgattcgggatgggccgtgtcactaatagtgatgatttactaaccacattttgttgttcttagtcgtattcttgaagagttttgtaacctattggcccttattttctatttaccttctgaagcccacgaagctaagagattgctctatcccatcaatcccaacttctacaaccttggcattcaaaccattactgataagatgttttaatggctgctccacttcttattataagcatttaactagatatttttgtcattttgttctaatgtctattttcttttgtgttttcagtgtggaatgattttggtgcatgttgatctatgattgacttatcgttttgattataaaaaacaaattgagtttatttttaacaaattgtattcaaatattgatagagaatattgcaaaccaaacttaaagaggcaaagttcaaaacaaagcgactatcgacatggaagtaaaattgatgttgtgaaaattgctatgacagcacaagtctagcatgcatgtcatcacaaagaaccttattgaagatagtagatttagattttttgatcaaatatgtaaagataatatgcttcaattttttacaatgaatcttaaaaagcccgagtgtcgattttatactcaagaaaaattatttcaccaaatacttgcataaagtatttttcaagataatgaattcaatcttacattataaaagtgccacttatcttgaaaaatctagtaaaaaacgttcttcgaagtattacctttgtcaaaatcattggagaaatttttcacaaataaaattgttatagcgaatgcctgttagggctggcagacatgcggtaggcttacggttaaatttttaaccattctaaaatgcaacagctagtgaactgtttggtacgatgatggacgtccggtatgacttgtttagtgggacagattttttgacggttctactgttataaatatcccaatctcttgcattcatatcatcacttctaaaagcattaaattgagatacttttaagctttaacttttattctctttatttatctctatcaattcattcacttttgaaaaatattgattgagtttacttttgaaaatcatttcatttatcaaaatttttcaaatctaacacttgagctttactcattgccatttattattaaagtgttaacctacttatctccttggtacacaactttaaataattttcattaagggagaaaatttctaatgtaaagtttactcttgattgaattgtgggtcgtgttgaggtttcggaaagctcaacggttgtaaaaggatcgatgctccttgattatgagtcatcgaaagcgttctaagggttggattgcaccataagccaaccaaattagtgaaaaaggacttgcttgtgacggggagtttggcaacggagaatgtagatcattgctttggatcaaacctccataacatatcgttgtgcactttcttttccttttctgttattatctttcaagttatcttgcttgcttgcttattatcttatttgttaattgattaaatttgctttattttcaaaaatgttttcgataaccaattcacctccctcttggttcgccattcttgggcttttaattggtatcagagtgaggtactcactttcaaaagattttacaattttgagtaatggctaaccaagtttttcaaaatattgtgagacattccacaaacagaccccattcttcgacggtacacattataattattggaaggctagaatgatgatatatatgcaatctactgattataatatttgggaagttattgactatggtccatatgttcctaccaagactattaaaatagatggtagactggatcaaattttacctaaatctagggaagagtatgatgaagaagataagagaaaattatctttaaattccaaggctaaaaacttattttattgtgcactagatagaaatgaatttaattgaataagcacatgtgaatcggcatatgatatttgacatgcacttgaagttacccatgttggcacaagtaaagttaaggaacaaaaataaattttttaattaaagaatttgaattttttttcataaaacaagattagcctattgttgatatgattatagatttaaccgatattgtaaatggtcttaaaggttttgatggtaaatttactaacggtgaacttgtttgcaaaatgcttaggtccttatcagacaaatggagcccgttgaggatgttgatcaagaatacctaggatattaatacatattctttggaggagctctatggcacattaataacctacaagctaaataatgtcgaaattaaggagaagataagaaaaagcaaggaggaatcaaaggagcctcccaaatgaaaaattgtcttaaaatcgaaaattgaagaaggaacctgaaaagaaaataagagtgatgaagagcttgatgactttgttcttctcgtcaagaaatggaaaggtcttcgtaataatcgaaaattttaaaaggaggaggaaaaaggcgaagaaagaagcaaaaagattatttgctatgattatgataagcccggccacaagagaatcgagtgcccgaacaaaaagaaaaatttcaagaaaaaggcactccaaaccacatgggatgataatgacgatgaaaaataaaatgggaacgatagtcaagacaaagtggcaagtatgtgttttatggcaataaaaatgaggtatatttaaatgagaagtgttcttatgttgagctttcaaattcatacaataaatgcttgaaaattttgaaaattttgccttaagtcatgctattcttgaaaggaaaaattatttgttaaaagaagaattaaaggatattttcgaaaagaaaaaagaaaatgttgatcatgattttgtagtaaaggagaactttgccttgaaagaaaaagtggatgacttatcgaaaattattcataaattcactgagggtaagaaaaattttgattcaatgctcgattgtcaaaaatgcatatttgataaagggggaattggatataaatcctttttaatacaaaaatctctctcaaaaatatgtttgttagagcttcaaacactacatgtagtttttgcaataaaagtggacatattgctttaattgcctagctaaaaggaaaactatattttgaaaacaagtggattcaagaatccccaaaaactaactaccaaggacccaagtttgtatggataccaaaagtcaaaacttgaatttttcttgtaggaaccaaagaaaactaaaagcaaatggttcttggataacggttgctcaaagcgtatgaccggagatcgatccttgctatcgaacttcaaaaagaagaatggaggacacgtaacctttagagacaacaccaaaggtacaattattggtattggaaacattggtattcactcatttccctcaattgaaaatgttttactagttgataaccttaaacaaaatttactaagcattagtcaattgtgtgataaaggttacaatataaaattcgattattccaaatgccttattaaggggctacatcaaaagaggtatttttcataggaaatcgaagtaaagacgtttatatcataagcatagaatttgaagataatgaaaattgtttacttagcgtgaaagaagaatcatggctatataatagaaaattaggacatgttaacatcaattttctttcaaaaatttccaaaaattattttgtaaaaggtttaacaaatttgaactttgaaaaatgtaaaatttgtgttgcatgtcaatttgaaaaacaagtgaaaaactccttcaaaccaaaactatatgcttcaactacaaaatcattacaacttctccacatggatctttttggaccttctaggatggctagcttcggtggtaaacattatgtcttcattatagttgacgattttctaagatttactttggttataattttaagtttgaaaagagaagccttaaatgctcttaaacacttttgtaagaaaattgaaaacaaaagaggctattctatctcaactattagaagtgaccatggtggagaattcgataatgttggttttgatgacatttgtaatgaatatggatatgaacataactttttggctcctagaactcctcaacaaaatggtgtagtagaaaagaagtatcgtacattgcaagaaatggctcggaccatgttgaatgaaaacaatttgccaacatatttttgggttgaggttgtttaccaccgcttgctacatcataaatatttaggaagtaaaaaagaaaattaaaactccttatgaactttggaaaaatagaatttcaaatattagttatttcaaagtttttggatgcaaatgctttattttaaatacaaaagataatttgggaaaattcgactcaaagtctaatatttgaattttcctatgatagttatcgactaacaaaacatatagagtttttaacaaacgaactctagtcgttgacgaatccatgcgtgttacctttgatgaaacaaactcatttgatcaagagaaaggtagtgacgacgatgtaggtttggaagctctatttgaacaaatgaagattcaagatcaaagtaaggaggcaccaaatgaaaaacaaaatgtggactcaaataaagaaaaacaaaccgagacacaaaatgatcctccactaccaatagaatggaggtttgtttcatctcatcctatggagcttatcataggtgacctatcaaaagttataactactagaacctcttataaaagtcatctcagtagttgtgtatttatttctcaaataaaacctaaaaatttcaaagaagccgagattgatgagttttgattctagcgatgtaagaataattaaatcaatttgaaagaaatcatgtttgggatttagtcgctagaccaaaccatcaaaccgttataagtactaaatgagtttttataaacaaataggatgaaaatagaataattgtgcataaaaaggttagattagtggcccaaggttacaatcaagaagaaggtatcgattttgaagatatatttgcacccgtagcaagattataatccattcgcatgcttcttgtatttgcatgttttaaaaattttacactttatcaaatggatgttaaaagtgcatttttaaatggatttattcaagaaaaagtatttgttgagaaatcttcgaattttaaagagcacaagtatccagatcatgtgtttaacctaagaaaaaactctttacggtttgaaacaagctccaagagcttggacgaatgatcgaggaaatttcttcattcaaatgatttttcaattggaaaagtggatgctacactttttgtaaaaactcataaggaggatatgcttattattcaaatttatgttgacgacattatttttgacgcaacaaatactcatctttgtgaagaattttcaaattgtatgagcaaagatttcgaaataagcatgatgggagaactaaaattcttcattggacttcaaattaaacaaacaaaagatagaatatttataaaccaaaataaatacattttagatatgctcaaaagatttgatatgcgagacattaagcatatgaacacaccaatgaacacgtctttaaagcttgacaacgaggaacaagggacaccagtcgacataatgaaatatcgaagtatgatcggttcccttctttatttgactgctagtagagtcgatattatgtttagtgtatgtttatgtgctagatttcaatctaatcctaaggaattgcatttacatgccataaaaagaattttccaatatcttagtggaactagaaccttagactttggtatcgaaaggacactcacattgacctaattaattcttcggatgccgattgggccggatgtaatattgatcgtaaaagtactagcggaaattgtcactttctaggctttgcacttgtgtcgtagtctattaagaaataaaattccgttgcactttccaccgtcaaggcggaataaatttcggccacaagttattgtgcacaaacacttcggatgaaacaaactcattgtgattatcacttatcttgcgatcatgttcctattttgtgtgataacactagtgccatcaacttgtctaagaatcccgtcttgcattcacgaacaaaaaatattgaaattcgacaccactttcttcgtgaccatgcacaaaaaggtgatatcatgttagaattcataaaaatcgaggaccaattagctgatattttcaccaaacctctagcgcgtgatcgattttctcatattcgaagaggtttaggcattattgatgagttcgatataaatggctaagattaaattatatttatttttatttgttttagttatacatctacctacccctaaaaaaaaattctttccggacgagtcaaacagaccgtccgatagaataatcttgtatcggacaagtccaagtggactatatgggataagcattcgatttggcagaaatttttggtctttgacctactagatgtccgataggtgtactagacatccagtacactatgtgttcagaatttaaaaacatgaacatatgctatgtcttccaaccttcttcaattccttcgaaaccctcttccatattacactcgattttcatcatttcactcttctggttcatcatttgaacaccaaatccataggtccacttattatacatctttttctcttccaaatatttgaaatttctcttactattttgaaatccccaaatttgtgccctaaatcaaactatccatattttcttcaaattgcataatgatgaaataaaaacgggttgcaaagagcccgaagcgccgacaaacccgtttgagaaatctcccattttaataggtaagagtgtagattttactgatttcactattgaagcacccacatttcactttgaagaatttttagaaaacatggattggtttcggtttgcatcttagaagaacacgcctatccccgtcttataaaagaattttatcaccaaatgataatcagtccttgaatggatgaaatctcttgtttgattaataatgtccgtatcacaattcccaaagctttaattcaccatattctcgagcttgatgaatgtgatatgcaaatttttgtccataaagcacatctgacaaacaaaggttactcctctgccgatacttgtcatcatgtgacgggaaaagattttgaaaacattacaaaaattagtgcaaatcaacttaccttacaatgtaaagttttacaaaacataattgcttgtatcattcttcctaggaaggggcattgagacgaagtgaactttttttgacctcttcatacttgattcattcattgttggcagaaaattagattttccaaccattgcatttggtctcatgaaacttgtacactcttcatggtatgctaaggctttaccctatggcatgttactcactaaaattttcaaacattttgacgtctcgttggatgacgaatctttcgttaaattacacccactgatactattaacacacaaacactcaaaagtatgaaaatcattaaaatgcatggtcaatgggtggctcaaacaaaagggttcgaccccacttcgggaccttccactttaccttttggaaaagagggagacgaagaagaagaagaagaggcagagaacggtccacaagttccacatactctacccaacatacccaactcaagtggctcacgtccttcgagtagttgattcacatttaccgaggaccactataatcttctaaacggtcaagttgattcttttaccactaccgttgacggacttggcgggctacttcatcaaattcaagctcaacaagcccaaattcaagctcagcaagacgccattctagtgcaacaagcagagatgcaggctcgacagaatgacttctatgctcacttctatgcccattttcctccgtccctggcaccttaggctttttttgactttttttaacttagactatttaacatgtttgacccttttttttgtgctccatagttaaatattaacttcaatgcaatcaccttggttgacttccttgttaattatatatatatatatatatatatatatatatatatatatatatatatatatatattgtttgtctttttgcttatgccgaaaaggggggagaatacttgacagtggatgattatgcaaaacaaggagtacatttggttatgcatgttgacaggggaattatatatgtctcaatattactgttcctcgattattactgtgcctcgtcaacttgttcaaaatttatattgcaaatcatcttgtttgtcataatcaaaagggaaaaactattgatctatggttgacatctcgttttgattatcacaaacaaattgagtttatttctaaaaaattgtatttgaatattgatagagaatattgcaaaccaagcttgcaaaaggcaaagtacaaaacaaagtgacaatcgacctggaagtaaaattgatgttgtgaaaattgctatgaaagcagagtctagcatgcacgtcatgacgaagaaccttattgaagattgtagatttagattttttgatcttatgtgtaaaggtaatatgcttcaatttttggcaatgaatcttaaaaggctcgagtgtggattttatactcaagaaaaattatttcatcaaatacttgcacaaaatatttttcaagatagtgatttcaatcttacattataaaagtgctacttatcttgaaaactctagttaaaaatattcttcaaagtattacttttgtcaaaatcattggagaaatttttcataaataaaactgttgtggcggacatttggtagggctggtggacgtccggtagactaacgatcaaattttttaaccgttctgaaagacaacggctagtgaaccatccgatatgatagtggacgtcttgtacgactcgtccggcaggacagattttctgatggttcaacgctataaataccccaatctcttgcattcatatcatcacttcgaagagcattaaattgagatgcttttaagctttaacttttattctctactctttatttatctctatcaattcattcacttttaaaaaacttttgattgagttgacttttgaaaatcatttcatttattaaagtttttcaaacctaacacttaagctttactcattgccattcattaaagtgtttacatacttctctcttttgtacacaactttgaatatattttcattaagggagaatatttcttttgtaaagtttactcctgattgaattgtggttttgttgaggtcctcgaaagctcaacggttgtaaaaggatcgatactccttagttgtaagtcacataaagcattgtaagggttggattgcaccataagtcaatcaaattagtaaaaaatgccttgctcgtgatggagaatttgacaacaagggatgtagatcattgctttagatcaaacctccataacacatagtttgtgcctttttctccttttctcttgttgtgtttcaagttatcttgcttgcttattatcttatttgctaattgattaaatttgctttattttcgaaaaagttttagataaccaattccccccccccccccctcttggttagtcgttcttgggctttcagtgcaaacgtcctagacatcaaaggatatcctcacctacggattagtgctttggcaaacataagagggttagctccgcccttgtcaagaatttgactgttaagtcttccttccacgaagatcccgtagatccaagggatcgtagtacttcactattgatgttctggtttcagggccattactcttagaaactacatcttacgcctcacttattcatgttgaggaaaataaattggccaagtcaagtgtgtctggacaaagtttagatccaataccttcttcctcgcttgacattgagttttacttggtcgcagtcgccatgatgagtttgatgcaaaaatcttgttttctttttcccatctcactgcctggatggttaggtcatgctatgcctatctaaatctatcctggaagaaactgactaaggaccttactcccatgcaaaggagagatatgattgatgctcacttgtcgagaactgtatcttattccaagattagcagacagaacatgagttttgcattaagtgagtcaatagtttgaccaaaaaggtccagtctttggaggaagaatattatgcacttcaagtcagcctgggtgtggttggaggaggagaaatctaaatataaaggtatgtatcgaagctttgaggattatgagaaggttagagatattatttttgctgatatcgggcaattagcctccaattcaacacaaacttggttggataacatagccaactccgaacaaaagattgtgaaattgctaagctaaaggaggcacttccaccgattagaattgattacctacttgtagtaaaaaaatgtcctgacaagggctaaactaactttacttcgtagaaaattaaaaagcaacgaggctaagctttctattatggactctgcaattgttaaagaagggcttatgaggccaaacttgttgaagaatccatgcagaaagggaaaaatcgattcttaatattatcactaatttcatcctagatagaacgtagattttttagaggttcatggagaggatgtcagtaacacttaacttttcgaagtttctttatcaagcctctagtattttatgtatctttcctttttcttaagccttttggtttgcaaattctgatactattccttggtactaggtaaccataggcttccacttttggcttgcaaattttgatattagcccttagtactttgcaatgtaacttacaagatgcaaaccatataatgttgtatcatgtaacaaaacatattactaaaataacttaattgtaatttttattcataagtatgcttctgtataggtacactatattttatcatgacaatttggtatgagtagccataggtttgccctttataatttttggaatcaggaagatagacttcaattctattttcattggtcaaacatcgttggccttgatatccattcattggtgggattgaccttgccttcaaaagctattttcttagcggacagaattttcaccttcaaacatggaaattttagtaggattaacctcgctagtagttagaagatcatggtaggcagagagagactcgtctttcaaatttatttttatagagttcctgtgagcatgttttagtcctagcttcgacattacaatgctttttcgaatactaacaaaattctcttcaatggtgaatagctttttcaaccccttgttcacagcttcggacgtttgctttcctgcaagatgattttcaagcatgtttgtttcaacgatcatagttgtattgattagtggagccctttgggctgcctttctcagatagttgaaataacattcacgtgcgcggcttggtctccttttaccattgctattccttttggagtctcgaagtagagatataggtgaaggatagaagtcacagctgtgaactattttaagacgagccgtccaaggatctcgttataagcaaacctactatccatgattaagaagtccatgtatccatagaatacaattgtcactcaacagctactgcaattcgttctctagaattagagcatctacagtgaagtcataaagtagttcagatattggtacccaaggatgatcaatctgtattttgtcaaagatacttctgaataatatattgacaagactactattatccaccaacattttaacgccccgaatccgagggactcgtgacattacaaggatcttaacttcatagaattctacccagatttgtttatgaaaatgtagaaatttaactgggaccaaaaaaattatggtttcagagtccattaccaggctaagaattgttcctgtgaaattttcatttttttttattttcagcttgagccactttctgaaataaatttccttcgactactaaatgggatccaaaaattacaaaatttaaacagtagacactttacacaggagaattcatgcataaattcaatgggtagatgggtcaaatttcttatcaaaaccggatctagttattccgggatgcattctgtcagctccgggaaaaacatccataacttgagttttgcacaaccaaaatttgtgatttcaaatttgagagatatataactcatatggctatcaactctaactaaatcaactgaaaatctcaagaaatttggtctgggcgaatttttgaacgtagatcagaaactgaaggtatccaaattcctaacgttgctattcgcatggattaaataaaccaccatagaatatcctaccaaacatgaatgaatttcaatcaaacttccgtctttaagctttcaaaaacaaatactaatgcaaataattcaaatgtttaaaacatttattccaacaaaacatgattcaattgatgactcttggggttcacataaaattgatgttattttagatgaacggattgtgttgacccatagagagattcagtgctttcttgttcgttggatggatcgacctgattctgatagtacatggattcccaaagagagacttcagcggcgtgagccaaattcattggagccttttaagagtcagcaaaatcctcattcgcccaggttattttggtcagctcatatttttgcgggtaatttgcaattggcattgtcatcatttgtggaatttcaatatttagttcattagaaagatcgtcccccatggcttgacttggagtattttgggtatcagatcaactgcagccttctgtgttttatacactcgacgaatcgagtttttctcccaccccaggagagttgatgcggacatccatttactatttattttcgatttagactattagttatattctatttggattattatttatgtttctattatttggcttgtatagtgggtttggcccaagcccttctctttagggtttttgttttgctatttatttctgttttgttgcgtatttgagacagttgataaattaatgaaatgaatatgtttggttttaacgttttcattccccttcctccctaacttctccttcttctccgggtttctcccccttgctgccgttttcctcttttattctccttcttgctgagattctgcaattcttcttctttcctggtgttttcattctttgctagaatccctctttatccagcatcgttggcccttgcatttggttgaacgcctacatctttgggatctctttcttgtctctagctatgtaagatggtctccgattgagcgttcatccctgcaagttgttgcattatcctctctatggctcatcgctactgtgtttgcttcctgtccatttctccttgggattcctgaaggctctaactgccttcgaaagatgagtaattccactagtgttgtcggccatcaaaattgacagctctaataccagttgctatgtatgtaccaaagtagctaaccactttcttacacactttgaatggcttcttcaagagagcctaacctccaaaaatcgacttctttcgacaacatataaggcattaaaatatttttttaaatctacagtgactcagtttggaagatgaagtagcacagtttacttaaaataacatacaaaattttatagacattggattgataagatttaaattttattcagtagctaacccattatactatcaaattactgttttgttcaaaatttcaagtaacggttgatttatgaatttttgaagtcaaaaggatagaactgtaagtgttatgccattgctccaatcaatttaggttgtaaacacttttaatatgtttaatgcatttatttttgacaagatctattatttatttaaatcaatattctgatgaataatactaaataatagtgtccatagattcaagtttcaacaatttgataatcacaaaaagtcgtgattatgagatacaaattacgtataattggatcttaaataatccatgatcgtaaataataacgagatgcggatagaccatcaagtgtagcatttcttacttgtaaagtaaatagctaatctcacaagctaaagtgtagagccacttaaatgaacacgtgaaagttttgttatagaacaaaacattggagatccgctgaaagattccatatggataactatcagagtgtcagtggttaatctctaacgttcggtagtggaattgatcttttgacttaaggtcatcatagtgctttatataaggacactcatactttggcgatattggatgttgctctactaagggcagctaatatgacattgtttgggtatgtcaagaatcatatgaaggttgtaaatgatcaatagagtattcatcactctttgatagtagaagattatgctatacatttcattcaattaaatcgataatgaaatcattggccaaggtgtattaagaagttaaaaaggagttttcgacttatattgacttaatagtggaatgaaagatatgatcgataatcaagactgacacacttccatatcttgtaaatgatcggatcatattgacgaagggattatacttttacggtaaatgaacgagtttgattttgtaataccacgtgacattttttgcatatgtattttcctgatactttgctagatgtcaatttgggacggtgaatgtaaattggtgagaaactaaaagggtattttaatttatcaattttgattagatcaaaataataattcatatcgttaggcatcgtgattgggaacctgatgggtcacacacaaaaggagaactagaagattgtgaattgtcaattaattaatttaacaagcgttaaataaattaattaattgagttgcttgtttatagacccgaacacggactgaatttaattaaatggtctaattaaatattggattgagtcaggagatagaccaagcttgtttgtgcttatataaataagtggttagggtttacaattttgtagagaatttttattttttatttttctagcatcccacaatattgctctctatgtggaattccattggaggttaaacaattggatagttgtgagtagcagatcaaggttgctggaataaaagaagagcaaaggagtttgcaaatttcacaagaaggtataacttctatcacaatttttatataaacacaatggagatctttggtgggaattgaaaaacgttttattttttgttatgcacgataagtaaattcccgatagagccaattatgtgtttattaggaatttatttacatttcaaaagttgatttactcatgttattttcttgaatctagcaattttagaatttattttaccttcaaaaattaattttcaaaaataaaaaaataaatagatgtagcggttcaccgtcgtcgccacctcaaaagctgcaggagtggcagacgccaccgctacagcagggcctttgcagtgctgaaagtagcaagagttgccatcttcaggcgacgggctcttgctgttgttgggggtacatcgccaagcaaatgagagaaaaaaaaattaaggttttcttcgaaccatgagatccttggaggtaggggcctctaatgcactttgtgaaattgtaggcccccatctgtaattatggtttagggtcaagttgcaattttttaaatgcagggctgctatgcaattttagaaattgtaggggcctgtttctgattttaaactagggtcaatctgcaattttaaaaattggttttaaatttattttaattgggtttgaccagtattttaatttgacccaaattcaaaattttatttaaaattgatgactttatatttttgttaaaattagattttaacttaaatatttgatttcaacagtgaattgaatttttgttttatttagtagttttgtcctaaattaaaatattaatacaattttattagagcttaactctaatctaatgttaattaagatttgattttagttaatattattttcccattatatattgaaattagagtaggactctaatttgataattaattaaaattttattttaattaaattatcccaccctagaatttcaaagagttagagtggactcaaaatttagtatttaattaaaatttaattttaattaaataacttttccctataattatggaattagagttggactctaatccggaatttaattaaaatttgattttaattaaataggcccgccaattaagttaattaattaatatgattaattaattatttaattatttcgattcatttatttaaatgagttttgatgactataatggctagattcttgagacatgtctgcatataatattagatattatatagaaaacatttatgtgatgaatgtctattaatggatgattgtggactcgactatgtggatatattgaatggttgatttaattcttgtcgttttatggacctgtgagctattaatttttttggacttgcaagtccattattattattgttgttatggacttgcaagctcttgattatttttggacatgcgaatccgttgttattattatcattattataggtctacgagtccaatttcattttggcttgcgtgtcaactagcataggataaaggttgtaactggactaattgaaggcgcaaaaaaaaggaggaaaccacgaacatggtgcattgatactgattcaatgttatacctcctaggaactgaccaactagtcttcctttggcttgggaagactagatagaataagtccataatcgtccatactattatatatatatatgtgtttatttgcatatttgatgcatgattatatatattgatgagaccatatcattataaatcccttactaaaatattaagtcggtattattatttgccttccactattatagtgaaaaatgagagttctaaatcgatctcagcttattgagtacacacaaggctggtttgttagagttatgtttgacactatgaaacatttgatatttttgaatgatggattcgaataaactaaaatttatcttttcttgagtatactcaaagaaataagttttagatgcatattaaactaacatataagatgtttgaagacaaagaattgtcagtttaatgatctgaaaattgtatggagatacaattgataatagtatctacccaaatgtttttttgaggtttactgagtacattcaagatcttgatataataggcgggatcccagcccaatgggaatcaaatatggattccaataatttatgtatgagggtcatgaatttattttaaacagtgggagcacgtttaattaatgtccatgttaaatttgtgcaatacattataatatatattaattctttattttttgtcatttacaatttttgaatcatgagtaaattatatgaatttgagagagatactggatgccaacaaactaaccagaccaaattttcttgattgacaccgcaatttgagaatcattctcgggcatcagaaaatttggtatgtccttgagtaacccttttcagagatacctactgaaaaattcactaaagaagaggtgactgcttataacaaatatagtgatgacgataatactacagcatgtgtgatgcttacaattatgtcacttgaaaatttcactagaagattatcatctgtcaattaattaatttaacaagcgttgtataaattaattaattgggttccttatttataggctcgaattaattattttgattaattaattcatggatcgaatttaattagatggattaattaaatattggactaggtcgggagacaggtcaaacccgtttgaccttatataaataagtacttagagtttacaattttgtagagaattttttttttcagcacaagaggagaaaacccggttccctacaatcttgctcgcagtgtgggattccattggaggctggacaattggacagctgtgggtagcagatcaaagctgctggaacaaaagaaaagcaaaggagtttgcaaatttcgcaaaaaagtattagttctatgacaatttctatctaaatacaaaggagatcctttgtgagaattgaaatctattttatttttcgctgtgcatgataaataaatttttaacaaagacaacaatactaaatcttatcggtcacatttttctaatgaatggtaacttgtatgttaacttctataaaacataattactttcaaacataactaattcataaaaatcttcttagaatcgtatcacaaatgatgttcaaagaaatctatttatttaaagaaaaatatgtatacgtttcataattgaataaaaacattagtcatcggcttctctatagcacgttagatcttcatctatcgtcatccacgccccaagtaaagaaaatcaacctatgaaaaggaaattaacccataaatttgaaatttaatagatattatcagtgtatttcattatcaaattagaaaatttgaactatagattcatactatcgcacgtggatggatttccagtaaaattcaatttctacagaattatcataacactttaagatagagaatgatcattcaaacaatagtagtgctgaagcatcgtacccggaggtatcaattcattcatactttaaacgaaaaatcataacttaaagcacaaaataatcacttgcacctctacctaccttgatttttcttgaaatataaagaaataaaacatgtaaaaacctttctttttcacatccttgttattcctttaagcttagcttaataataatggtgtttttgagagaaaataagtgtaaattcggatttgaggagaagtgcaatgaaaatgtgactttcctctttttgtaaccttcctttttagtgaaaaattaaatggaaaagttatattatcattaacattgttaaattgagtctttagctaggaatttagagagtattaagccataaaaataatttttataaaggttttataaaacatttacataatgaaaaataaagaaaaatgaactcttcatatgatttataacttgtctcgatgattgctcactaataaggtaattatttcatctaattaacttcttaatgtgcaaaatgagtttttaactgaaaaagaaaacatctgcattatgtttcgaacctattcattaaatctttgtaatcaaatttacttaaacttaatcccttaaattattgggcttttaaataacttatggctcgggctttcattaccttttttgggcgagcttccatagctcgtttcttaaatgggctacatcaaccaacttaagaatataaaatttggaaccgtagattattagtggatgttttttctatatccaacaggctgcttatgttttgctgttcatcatgtttctatagtgcgtcaataccttcagtagttgaatgggtactaatagtcatgtctgattgtcactgcctgaatttgcaacacattttgctgaaatattttgattttctccattctattctctcaagttttgaatttcaagttcttgagataagagtaaaaatcacatgactctagctatctcttgtaatgacctttttcttctctttctatcactctacttttttcaagagttttacgagccgagaattcatgagatatgctatgttcttaatagaatctagaaaaattggcattttcaaattctttccatggtcactcataattctcataatttaatctcatcgatatatttcttctttgtcaattttagaagtgtgaatttctcaaatacgaaagacttcccccttaaaaaatctacctaagtttaccaagaaaaaatatctatacatacatagatattcctattattgctaagactattagtgtgaataagtctcattaagtccatatgtagtaattctagactatgagaggtcgcaagaaactaaacttgtttatatgtagttctagtttgtctatctttttggcatgaataacacataccttcaggcttttcagttagccttttactacattaagtttggtacgtccaacaagatcaccataattcaattatcctaattgtttatgccgtaaatctatagaatcagcctgagaagcatgacaactaatgttagagtgaaaaagatagcatttatcaccaggcctagcactacataagacacaattaccatcatgttaagacctcgcatgattatttttgtgaacataaccataagatcgtcatcacacagttatcctatagtaatcaaattagcttttaagtctacaacaaacaacacatcatttaagagatagtgtccattgataaagtatattttatacactcatttggacctaaaaatttaaacatttaatagttctttaagggaattatagtataagttattgtatatttcgttcattgggtaaaatttgatgattgaaagtggaattgaaataaataagtgaaaaataacgaagtccaaagtttgaggactaaattgcaaacattcaatagttgagtcggaccacaagacaataatgatgtaccaggggagcaaaaaaatagaaggcttacttaaatattatgaatcattttttgtatccatgtttgctacagactgttaataaaaagaacgtgagcaagtagataaagtgttatttctaaccaaatcaattaaaagatagcgaatgaagagtcgccatctatcattctttcagaaggaccaaattatcccaaagattggagaaaaatctattaatatccctaatttgaagaagaaggcatgcaattcaaatatcccactgtcaaatagttattttacttcttgctcctattttagcatctaaattagcgagtttagaaagtgaaaatcgtagataggtgagccttctttatcttcattcccattgcatgtcactttatacctcaccaatggggataactcttgtcggatgtattccttggttcaacaaatagtcctccgagtttgattttattatttatattaaattaggactaaactatttcacaatttaaaagtcacgagcttccctgacggactgacttaatttactttgcacttaatgcttcggtcagatggtgatagctggcgagtagtttcaagaaatgttctgaatttttctatccctcgtgtgttatatgcttgcttataactgttgttttgtgtcctttcgtattcaacggctaattgcatgagttctgatgaggaagtccatttagattttatggctgtgataggctcctttcagcactatatatatgcaccatattgctattaatctttatttttcctgatcatataggatgtgtttcgctaccttgtttgctgttgatttcatggagaaatttcttatccctattagacttctttttccatgttatcgttattccttcacattctttcctaattctactatattttcctgatgaatccttcttggatcttttacctttaccttaagcaataagacatagttttagaattgtcataatatttcaccagccatgctacagttgcttatctgtgagtctgatttcattgcatataatttgaaggccagcagatgatggtttggaaaccagtaggcttatcatcatactcttgcatcttcctcaagtatgcatctgcgatgatttatcatgcaaggcatagttctagatgttgtaataaacccttatgcatttcgtcccgaaaagcactcatctacttttaaatggtgcttccggcgaaaggattgaatttactctatgtctctccctcatcttttgactccaggaatctttgtgagagcaactattatatagggtgacttaattcgagaaattacttttcgacaccataatagcttttaattcgtataagatgccttttactaataatacatcattttctggtatgttgtgagctttacttgagaaccatctctatttttccctaaaaggtctaggctcacttttatcgattctttacaccaatattcattggtatatggcctctatcttgtatgctaggaagaaagagttttgtgcagtgactattttttgtggcagttcggcatgcggggatctgtaacaattcgtcagcctatactctgtgctgaatcaagtttcctttattagtattttattgatggcttttacttgcctgttgcttgaggacaatatggagtggaaaagtgtttgtggatgcccaactaatgccacagtgctttcagtcttttaccttgaattttgtttcatgatttgaaattactgagttaggtactccgaaccgacatacaatgtttttctatatgtagttacaagtgttagcctcgctaatatttacaagggtttagcttctacctacttaataaaataatcccctaccactataaaaaatctcatattggatattttcttaggcagtagtcctgtgaagtcaattctccacttgataaagggccaggtgccgctactagttaccaaatcctatacgggttgtaaatgaatggatatgaacgtttgaaacttatcatattttcctagaaaagttcattgtatcctttctcataggctaataatatatcaattttaaggttttttgtaatatggaggatcaactagcatgattaccagatatactttcaaggatttcgttcattatgcatgaagcttcatatttgttaatgcatctgagctgaggaagtgtgcaccctcatttgaataagatttcacctggcaatgtatacttagcagcttttcttctcaactttggtgctacctttttatccttagggaatactttgtccctcaaataagaaatgatgtcttccatccactaagttttgtcctgtatccataacatttcctccattttcaggcttatttatggttttggtagcaattcttttggaactattttaaacaacttcgtgtcttttgaacttgtcagctttgataaagcatttagatgctcattttcctctctagatatttggacgagttcaaacttgttgaagcattaaagtaaatttatgggttctgcaaggtatgtagtcattattttattctttgctatgaacgtaccatttatttggtttaccatcaaatgttagtcgctttttatttcaatatttggcacttgcatttcttttaccaatcataggcatgtcaataatgcttcgtactcaaccacattattggttgctttaaacgcgaacattaatacacaattaaactattctctttcaggcttatcaattattatcctgctcacgagtcggtacctcccgacaattcatccacagacaacgtccacgttcccttttcaggcttctcctctagaattggaatttctgacaattccacagtaaaatcggctaatgcctatgctttgattgcaaatcatcctttatagcttatcttaaattgccctaactacactgtccatttcattagctttctagacgcatcggtcttttggagtactttttgaatggaaattttactattcaatagtatggctttggaaatagggctgcagttttcgcgatgccatgacttagaaaagggccagctttccatatctggatactacttctctgtttcttgtagggcttagtagattggtaattgttgtcgcccttcttcttttactagtactgagttgactaccaacttggatactgctaaacatagtaataatttgtctccattttttgggtttagataatatggtattctcccaaagagatcctatagggtatggaatgtctattcacatttcctactccattcgaacttcttctcacctttcaacatttggaagaaagtgaaacactatcttttctgtatactttccccgtttccattgttgtccgtcgttttttacagattgacgaatgtattcgataatcaatattccccttttaagaagataggatttctgattattcggacgtcgaggtatttgtgtaaataggtataatccatggtattttagttgctcgatatacaaaccttcttaaggcgacgactcttcatgttgaactttacatttcttttggtttagatggaaactgcatttttatgaaggcttgaattttattgaggtttgctccaatacctaacagattgacgatgtaacctaggaatttacattgaaagcctcttccaagtgttttcagtggtcttcagcttgaaggctttttacacgcatattatcgatgtatacctccatcattttcccgatcactttgcgaacattttgttcactaatctttgatatgttgcccctcattttttagcccaaacgacattacttttttttatagtatagtcctcgatctatcacaaatgtgtaatgttcctcatcaagcccatacatacgtacttggttataccccaaatttgcatacaagaaacttaagagctcatgtccgacagtcatatcaccaggtgatcaattcttaggagcgggatgctgtctttctatcaagcttattcaagtccataaagtcctggtaggttcatcatttttcgttgctttttgatactaggaccaaattgcatatccaaactaggtaacgagcttggaaaataaacccattttccaatagtttatctacctcactttttagtacctcatattttttcgccctcattagctagggcctttgtattttaggcttgatcttaggattgagcttcaaagcgtaatagacaactttgggatcgattcctatcatgtctgcatgtttccaagtgaacaatctaggttcgcggctatggattttttagcaagcctttcataggtttgcttaactcattgtcgattttgtttcgaaattattgcttcatttcaaaaaatgtaagtacacaattcgttaataagtaataaaatgaattttgagtccaagtatcatacccacttagattgtactagtttaaattcaaatcaacttcaccttaaccgaaacaatgaaaatttgtgatttttctaaaactgaattgtcactaattattaaaaaggcaagagttgagttaatgaaattcaattcacgattgtggtaatgttagtttgatgaaaagtgcactaggatcctgaatcctcctatatcaattccctttagcccgaatcttaaaaattgacaacacaacttaattatgaagattgatattcctatactgtttgacatttctcttgaatagaattgaacatattctcacatgtgatctgattatatttctatgatggatgcaacatacaataatgtattaaggatttatgaatgcttatagatcacgtagagcatagcgatatatttctatatccttttggactctacaacaattaacactatgtctaacttattttcaatttttcaaaggtaaaacaatccacaatattcacgtaatcattgtaatagtatttgtagaaaagaattaaaccatgaaaattgtccaataattgaaaaagagttttgaatgccaaaaagaaataaagtcaagagtcaaagattcataatacaattttcatcataatcctagcactagattactttagcctaacatgttatgtacaagaaaacaaaagaaataaaaatagttcatcacctgaaattcttgaatttgaagtttgaatttcttgaattagatcttgcgttcttctccttttttgcaattaattgtccaatcctaattatctgttgataattggtatttatactagtcttcaaggaatccctaaagtctctaaaaattgcacatatcatgatccaaatgaaagtttccttgttggagtgaaaactgaacgaaactcgcgactagattgggaaatcaccagtagaaaatcgagaatttgccaggcagcaaccatttaagtccctatttttgcactttcaagttgggcagttgcctcggccattataaattggtgggtacccagttataaaaactttcaaaattcgccctttagtcattttattcattctttcttccactttgatcctccattacaaattatgtcaaatttgatccttcaacttcttctcatgagcacattagtccccaaaccttccatcctatcatcaattcatccctcgttcttttccaattacatatgaaatggtccaaaattgaaatgaaagaaatttaagctaagtaaaattttaacactttaacaacataaaggctaagtaattaaaaaaaaaaaaaaaaatttggatcaagagcacaaaacacgcttatcaaacaccttcaaactaaaaccttagtttgtgcttgaatgaaacaatacaaaacttaggcacaaaccatactatcctaaaataaaccagaaataacatactcaatattgaattgcttctcatatgcattaggttcgaatttaagaaacactttcgaaagatccaaacatgacaaataaattttcactcatccgatactcaacttagtgtgtgtgtgtgtgtgtaattagtcaacattgaactcacacccattgtagaacacaactaatctaaggttgttgatttactcataattccaatcatcttgtcgttagtttttccttacatctttgagtaaaatcacttcttatgcttttccatccaatcctgaaatatttctagcacatgtaggtttctaagaatcattattaatcattttccacacaaaagtgatcaaaattggatacttatatatccttagaaaggatatggtaagtatttttcaaagttacaccattagtttctagagttcaaatcttaaagttcttaccaagcacatctcacttttgaccatctaaatcctcattttttttacatcccttgtgcaagacttctcttcattgagctttctaaatgacccttgtagcgagcattaggccgatgattccaaagtgagatgactatagggcacctggttttagatacctttaaggcttaattactcgagtcataaaaactacaaaggaaataataggctgtatcatactttcttttcgttatctttatatctcatgtacaagccatctttccaataaactttttaaatgacccctatagtgagctttaggccgatgactccaaaatcagatgactataaggcaccgaattttagatatcgttgtaggtttaatcattcgggctatgaaagttcaacaaagagaagtatatgatgtatcacactttcttttgatatgggattcaaattctaaaaatagttagtgcatgttccagactccttaaatgaagcgccttcaaccaaacatttgattcgagaattccaagccatcaaacttctataaacaaaagcactaacctaggtttctatattaaggatttggggattctaatagctaggttaccaagactactaagtccacaaaaatcaaatcgtgtcccaacataaattataagtcaataatggctatgtactcaaaaagtcaagtctaacatggataagtactcaagtagaagcatgagatatgattttgtctagttctagctaaaactatactcagttcaaacaaataaattccatcataggtggcaagccattcaatgataaactatacattactctaggattttttattttattttattttatttttaaatttaaaattaaatagttatacagacccaattggcagttggaaaatgaacatatattctaagtatcataatacttactccatccctaaacaaaagtattacattattcgaaatgtaaaagtaaaaaattaacaaagtaaaagagtaaaggatcaaaaaatccccatggtagatgtggatgagtagaagtgtcaaccaggtccacttggccggcagaagtggcaggcctcaaggactcgacgttcctaatatctggaccatgtttctatcaatcgtttctagttgactcccaaagcatagcatttgatcaagcacctcattgtaagcttatgtgatggttctttgatcgtgtcacattctatcattacattgctggaacccacgtacattgtcactctctcttacaagcttcctttgtatgtttacctgcatccgctgcatctccaataacatattttgcatgtagcctactgatctaccaagctctacctaatttacctaaatatgaaacaactgtctacccaggtatgtctcgatgtatgaggctagatgaggtgatggaggtgcctgtttgggatcctggactctctctctaatcctttaaacctggcttcgaaattttctacattcttctgctgatcatatcaagggagtaatttcttcatttggcaaaagtaggatcccaacagtcaaacagatcctactgataaggtacgaaaacatgatactgtgctgactgatcaatacagccaactcttgcataaaagtgaagacataggacactaaataaattttatgcccctatgcctgatagagtagttgagccgtttcttcgttgaacttccttcgctgggatgtaggatagatgctggtggagacgaagatgtgcaggagtctcatctcagagttgaatgtctcatctcagagttgaactgattattcatgaaccgagatgtaagaagttgccatgcattacatctattatataagcaccggacaatcaataccatatcctggctagttggtaaaggcactatatcaatgtagcccagctcgtaatatttgtcaatcaccattgggctgagtcaaaaccacttatctcttacccatgtttggttcatgtgcgatgaatcaaggatatcaatttcaatattgaagttatcacagaattccttcagaaagataggataagatagggtattattcaatagatgaagaaaatatggctcacattccccaaactaaaatataggaggtattttatgtttccatccaaaaccaaacaaggactttcataattggaaaatgtgaggaataatgattcacaagcgatctctggacatatgaaagattatatattggtcttactcatgttcaaatttgaggtcaaacagagattgtttgggttagacgagggtggacgaaattggtgacatgaagtgaagatgcctagccatgtcatgccaaatgtgccaatttgggtgtaggtattctataatagattttcaaggaattttaacagaacaatcccaaatgtatagcaacgatgtcaattgctcgaatagccctaattagtcaagaaatttcaaataggcaattgatcaaacagctaggaggcattatattttgccctaacatttgaagaaattggggttctaatcattccacaatcttcacatcacaccaccagacaatccaaccaactacaccacaatctacctaatgtccatactcctcaataatgtgcctaaatttttaagttataacaatagcacaatagttaaagagaaagtaattgacatacctttaaatcctttgtagattgatgtggagtaatgaaaatcaatacaatggaatgcaattcctagtgatggattcttaatggttttggaagatgatcgtgaaggtgaagtcaaagaatcgtgaaggtgctgtgagttcttgggttagaaagaagtgaaggaccgtgtatttccaagtgtcgtgatgtttgaaattataggtgccataattatgtgcttctttggtttaaaatgtgtcagaaagtgtcatttttcattaacactaggcagtcgcccagtgtattactgggcacccgtccagttcacctatcgaatcagaaaaactacataaaatgtgattaaaatacatgtaaatgcacaaattcataactaaaactctaaattactagtgtaatacctagctttatgtaatgcaataagcaataaaaataaaagataacagataggaaaatgggttgtcttccactaagcactcaatttatattctagaggttgactttttgagagatttactctggtgttgcaaggtgaaaggtggacttttctttcgagaatcttccgccctaatatggctttaacctttgtccattaactttaaaagcgccttggcttttgtgagtaatctcaatagttccatatggaaaaatttgattaatggtgtacatcccccaccacattgacctcaatttgcctgggaaaagctttagtcttgaattgcatagcaagacttgttgtccaacctcaaacttccttcattgaatacaagtatcatgtcacttcttggttgctccttgtgtaacttagcattctcatatgcttctaaatgaaactaagccatctcatttagttgaagtagtcttttttcactgtctgccttcaaatcaaaattcaggctcttgattgccacaaaagcttgatgctccaactcaactatcaattagcatgccttcccaaaaacaagatgatatggagacatacttataggggtcttgaaagctatttagtagacccgtaaggtatcatcaagctttttagactaattttttcttaaagaactcatcatcacctcaagtatctcctttaactcccgattggagatttagacttgcccactggtttgtggatgaaaagagacacctatatgatcccagacgacctattttgccaacacggactcaaattgatgattatataaatatttacaccataactaatgattgcatggggtataccataacgagtgaaggtatacatttcaagaaacttaccaccactcgagcatcatttataggtaatgcaacttcttctacccagttagaaacatagtcaactgtaatgagaatgtatttatttgtgaagaaaggagaaatggtcacatgaaatcaattcttcacacatcaaacagctctaccttaagaatattgttcaaaggtatttcgttccttttagagatatttcctttacgctggcatctatcatacctctttacaaaaatatgtgcatctctaaatatcaaaggctagcagaacctaaactgtaagatttttgttgctaaagtatccagtatgagtagaagaataccattgctcgagtgcataagggactttttctttaggaacacaccacctaataaattgatatagaccctgtccatagagaatatggacttcaaaaaatagtatttcaagtcaaaaaaaatttcttcttttgataacttgaataatctagtgaatgatagatttggctaaatagttcactatatcagcataccatagtgcagtctccaagttaaatagttcatctgggaagacatcattgacatcaactaactttctctatttcccttgctcaattcaggataaatggttggttattgaatttttacttccattcttatctcttattttcaaatcaaatttctataggagtaacacccatctgttcagttttagtttagcatccttcttagcagccaaatactttaatgttgtatggactattacatttgatccaagaagataggattgaaatttatcaaaagcttagactacagctaaaagtttcttctcagtggtggcatagtttagctatgtatcattcaatatcttgtttgcatagtagatcacatgaaaaatgttatctctttgcaactccaatactgctctcagattgcaataacttgtgtcacattagatcaaatggtaagctccaatatggtacaattattactagcgctgaaaataatgtctcctttagattgttcaaagctcaaagctaaaaaacactctttagataagtcaaaagaaacattttcgattagcaggtagcaaaatggtttagtgatcttagagaagtccttgatgaagagtaataaaactcggcaggaccaaagaaattgcgagcacccaaaactgaggtcgataatagtaatttctcaatagcctaaatctttgccttgtctacttcaatccctttagctgaaaaattaaatgtcttgatactctactctcttgtaccatgagtgagttttccctttttagactcggatttgtttccttacatcactacaagatcaattttaagtgctctaggcactcattagatgaagagtcgaagattgagaaatcatcaataaagacttctatgattttttccaccatatcagagaagatggctatcatgtaacgctgaaatgtagagtctagaagccaaaaaagaaatgaaatttagctcactagtttaatgcaataatctagcaccatgagccgaggccatatatgacccttatgcttggcccacgaaagaaatgaaagcccaccactagtttgatattccttaaataatttgaatatcatggaagtttcccaagcaatcatgcatattttctagaaaatataaattaggatggaatttaattttttcccaaagatttcacccaacggtgaaaaatttatttcatgtatagtagagattcctaagatttgatttttgtatgtgtcatttttattaaaagggctgaattaaaatttttaaaaatgacacataaaagagaaattataacttctatttgaggataaatgttgatattttcttaacattaagtaaataaatagggaccaagaataaaatttatttaatgacccactttattttactatatgtgtgtgtgcgcgcgcgcgcgcacaatttaaactgttaaaaggttacgaaagaagcatgtaaaaatgcaagaaatgaaatcccaaattaaaggcatgaaatgaaacataaacattgctttaatgggtgaatgaatgactaccaatattatccctttaaatagcataaaaaatgcaagaaatgtaacataaatctcagaaaaaacataagagaggagcaaatttcttaaagtttcgagtgccgtcaggaaacaacattcaccatccaatctcatccatttcaaagcttcaaattaaggtaggtagatgtgcaagtggttatttcagaatgagtatttaagctccacgctttcattcttttgaattaaaattcaatcaagtagagcacacaaaattcaatgttttcaaattatgagttttcgttaaaagtttgaatgaattggtacctttgggtacggtcctttggtactactatagtttgaatgatcattctctagctctacgtgtcatgataattctacagaaattggattttgccgaaaatccatctgcatgcaatggtatgaatctataattcgaattttctaatttgataatgaaatgcagtgatgatatctattaagtttcaaattcatggatgaattcccttcctaaatgttgatttgatttgcttggggcgtggacgatggtagatgaagatgcaacatgctatgaagaaatcggtgacttaatgttttatttgattatgaaacttttaaatattgttctttaaataaatagattcctacgaacattaagtaaactgagtgttgctgttttctgaataaacttggaatcatgtcaatctgatgttagtaaaaattttatatgccactttaactaaattgagtgttgctattttctgaaaatttcagcttctgccattgacttcaaaaatttataactcaatcattactttggatagttggacaaaaccagtgggatttgatagtctcatagattatttactaaatagactaaaatcatgtcgatctgacatttgtaaaattttatatgtcactttaagttaactgctctaggttatcttctaacccgagtcactgtacggttttgaaaaatattttaataccttatatgttgctgacggaagcccatttttgaatatgtcatattataaagagttctctactttccattaaaatttcatgaagtttcggggttgatagctatgcaaacgaatttattttgacaattgccacttgagatagaaagcaaagcggtgacatttatttttttaaattttttgcctagaatttcatgccaataatagatacatgtatggtaaccattctatatatatatatatatatatatatatatatatatatttttttttttttgaattagtttctttcagtattgaattatgttgtctttaaaaaaaaaaagattgatttaccaaggattttctttcttttttttggcatgccatcgttcacgtaattagtagaacttgcatggactttgttcgaaattttcaatatcatttcactattttttctgctgtctaaaagtgacattacttctaagaaataattagttgatcgcttagtatgaaatcatgttgttagaattatatgaattcgtaaattaaatctttatgctttcgctaaaagtatagttatttattaagtttgcggctaaagtacaattaaactagcgatatttcaatccatgcaagtcgaggcgttatagcatggtatcagagcacgagttcagtagattttgtagacttagtgtattttgtttatataaaaaaaaatacttaactatatggtgaaaaaattaaatatgagaaaatgaaacatttaaggcacttcatggtatctcgcatctatccgtcgaccttatcctatgacccacgtatgtttaactaagcaaggtttaaatacttgttatgaagtggttatgattctatagttatgctttccatatttctctacgttttacatttttctttatgtatatcttgtatgtaaagaaaaaagtagtttgaaaaaataagttatttaaaagacatattgggctagaacttaaagttgtgggtcacaaatggcaaaggaaagacaaaattctaggaaaatgaaccatattagtcaataggagatagatatccaagcttacctagattttgaaatagacaattctatagaccttgatagtcacatacgaagcgtgtattggcaaagaaaaaaaaaagaaaaagaaaaaaggaaatcaattctaatcaagttgagaaataattccctatattttttttggtattggtaaatgaagttaccgagagatattacatcttatctcaaaggaaatgtctcaagcaaacaagaacaacttgataaaggaccttttgcaagcggcttaagatcttggaaggctgaatcagagtcaaactccacctacaccaccagctcctattactttcccaacccatacctcaatagttgagttatttcgaaggcataagtctcatacttttgatggaccatctggtccactagtagttgaagaatggctccgtaagttagaacgaatttttcggctcatagattgcactgacacccaaaaggtctagtattcagagtttatgtttatcggtgatgcaaatcactggtgggattcgatgtctcgaactaggaccccagagcagcaattggcattaacttgggaacaattcaagaacaaagtaatggacaagtattttcttcagtttctaagagattttaaggaaagcgaattctgtcaactcaaacaaagtaatatgcccctgactgattacgaacgaaagtttgatcaactctcaaagtatgttccattcggggttgacacggaaattaagaagactcgaaggttcgagcaaaggttaaacccagacctaagcatgattcttatgtcacattgtttcacatcacaccgtgagaaactcgaacgagctcatgctatttggcatcggaaggctaatgtagagcaacatagttaattgtacaaccaacatgataaagggcaaattggaaagagaaagtgaaatggtcaagataaaggaaaaggtaaatggcaaaataagaaaactaatatcgaatctagtgcgaataaggccatagtagctacagtggcaccgtgccctaagtgtagtaaaacttatcgtggtgaatgattgtatggaaagaatgcctattttcgatatggtaattcaggacatattgcttaagattgtcccatatttacttagaagaatgatgataacagtgatcagaacaaaaaaaggaaagcatgagtttttacactgactcggaaagatgtagaggagagctcaaacttagtactatttgattcgggagttacttattcttttgtatcaatgtctttcattgctaaatctagtattacttgtaataagttagagaatacactagaagttagtattttctcagacagaaaattgaatacatatcaattagctaggtcgatgaatcttgaaattaagggaaaaacattagaaactaatttatatatgatagggatagagactttgatgtgattttgggcatggattgattgagatgcaattatgcaaccattcattgtggagaaagggaagcatctttaaaaccaaggaaaagaaaaaatttctttccccgaaataaaccaaacctcatgtccaactagtatcggtgttgcaagctaagatattgagaaaagaaaaatatcaagggtttctagttaacatcgcaagagagaaatagacaatgataaagattgaagatgtaccagtggtacaagaatttttagatgtgtttctagaagatctacgtggtacaccaccagatagataagtggagttcacaatggacctggtttccgaagcaactctagtacctaaagctccatctaggatggctccaaaggaacttcaggagttgaaaattcaattacaagaactattggatattagctttattcaaccaagtgtatctccatggggcgcactagtattgttcgtaaagaagaaagatagaagtatgatgatgtgtatggactatcaggatcaagaataggtatcatctcccgagaatcatcaagatcgacttacaatctagatatcatcaattgaaggataaggaaagtgatatacccaagacaactttcagaactagttatggacattacgagttcacaattataccgtctgagttgacaaatgctccgacagtgttcatgaatttaataaatcatgtattgtatcagtatttggattaatttgtcatagtctttattgatgagattttgacatactccaacagtaaagattaacatgagaaacatcttagaataatgttagagatattgtgtaaggaaaagttatacgccaaatttaaaaagttcgaattttggcttgagcgagttgaattcgtcagtcatgtaattactgtccaaggaattgaagtggatctgataaaagtgaaagcagtaactaattggaatacaccgactaacgctagtaaagttcaaagttttctaggattatctgggtactatcaaagatttattgaaggattctccaaaatagccagaccaatcactactaaaaaaggagcttcaagcatagatttttcgttcctgaaaccatgatatccgttactattactctttaccaatagaatatttgcaaccgcaaatccgttgctaatttgagggtcgctgatagttaccaatggattctgtcgtaggtaaagagtaaacattttaccaacgaatttttcgttggtaaagtgtgaatcttttaccaacgaaattttcgttggtaaaaattttaccgtttcgttggtaaaaatcttaccgataccaatcgacttttcgttggtaaatatctaccattacaattggtaaaaatcaatattgtaaatagccgaaaacgtgtgaggcatggtaaataaataaataaatttagagcatatttggtacagcttaaaatctaattaaaatcaaaattttgaccattatttcactatttcagtcgtcatttttgaattcttctctcataggtaggacccactttttctctaacggtcaaaaagtcaattaacaaaatccctaccaaacaagcacttattattgttattattatttatttaataattctaatttttttttaacttttagccaactgaattgaaaggtcaaaatattgtttaaccacaaattaatttatagaaggcaactccgataactttgttgtgaactttctatgtgagataagtgaaatactttaaccaacggataatccatttctaattaccaacaaaatatccgtaggtaaaagatccaaatgttaaaggattacatgaagtatggaatatccgttggtaaagagatatcatcgttacgaatggaaaatccattgctgattatcgtagttgaaagtgaattacttttactaacagataatccttttctaattaccaacggatgcaatccgttggtaatattcggtatgtcacctacggatattccgtaggtgaaagatctaaatgttaaacgattagatgaggcaagaaatatccgttggtaaagaaatatcatcgttaccaatgaaaaatttattgctgattatcgtaactaaaagtgaataacttttaccaacggataatccatttctaattaccaacggattgcatctgttggtaatttttcgtaggtgaaaatttattttttagtagtgaatgacacaattgataaggaaaggagtaaagtttcaacggacagataaatatgagcaaaattttcaagagctaaagcaaagattgattatagcacccatgttaaccatgcccaaaggttcggaagggtttgttgtatatagtaacgcatccaaacaagatttcggatgtctattgatgaagcatggaaaggtgattgcctatgcttcaagacaactgaaaaaacatgagctgaattatcggacacaagatctcgaacttgttgtggtagtttatacatcaaagatatggcctatcacttatatggaggaaagtgtgacatttacatggatcataagagtctcaaatatttcttcacacagaaggaattgaatatgagacagagatcatagttggagctagtaatgattatgattgtactattcattatcatcctggtaaggttgatgttgttgctgatgctctaagtagaaagtcaataggatagttggcatcagtacatactacttagatggagttaatcaaagattttgagaatttgctaatcgaaatggttgccacgccagagtaagtcactgcccgtttagcaactttggtagttcgacctacttttagagatcagatcataaaagcacaaggtaaagatccgttcctacataagatcaagaacgagattcgtactaataagaggaaggattttagaataacttcggatcaggtactgatgtttaaaggaagaatttatgtctaaggatgaagttttgaaaaaggaaatattggaagagactcgtttcacccccataaatcgcatacagtggtggtatgaaaacatatagagaccttcgaaatacattttggtaaagaaattgattagtgcattttgtgcacttatttgaaccatattactaagtttttatgtcatgaaagtgtagatttttacttaactaggtaaatttcatttgttttagtgatgtacctgtttctaagcaattggaaaagaaaaatggggaattctaaagtctaagggctaaattgcaacatttcaatagttgatttggaccaaaatgaagattaaagatgttgcgggttgaactggatgcaattaaaagtcaaaaggttgaaataacaagagaaaggatttgaaagaatcaagaattgaattcgaggactaagatgcaacattcgaaagttttataactaggcgacaacccagttgtttagagtgggcgactacccaacatcaacgaacaattaccgaggcaaaaaagatagcctgggcgattgccagtgttttgcccaagcagtccacggtgaaaaaattctagtttccttatttgattaaaattcttacagaagcaaatcttgggaggtattttaaaattctagggctgtccctaagcatggaagacgtattataacacattcataagggtttttaaagaagagaataaggcaagaacatgatggatgaatgaatgactaccaatattattccattaaatagcataaaaaatgcaagaaatgtaacttaaatatcacttttaaatgttgccaccatttttattttatttttttacaaaacaaaagtttagacttttgattttctcctaaacattttctatcctatataagtgcgcactttgatcaaggaaatagattttcaaaagaaagaaaaacataagagaggagcaaatttcttaaagcttcgagtgccattgagaaacaaaattcaccatccaatttcatccatttcaaagcttcaaattaaagtaggtagaggtgtaagtggttatttcattttcaaattatgatttttcgttaaaagtttaaatgaattggtacctttgggtacggtgttttggcactattatagtttgagtgatcattctccggctctacgtgtcatgataattctatagaaattgaattttgtcgaaaattcatctacgtgcaacggtatgaatctatagtttgaattttccaattcgataacgaaatgcaccgataatatctactggagagtaagtagtactaaaggctgttggtaggtagggtcaagttgttgagggttccaaaccttaaggattttgtgaagcaaagaattaaaatatggtccaaagaatctcgatagtagttccaacatttatgtgaaaattccaacatttatgtgaaaagtacagaagccgggaagaagcatatcctgtaccttgacctacgaagccctatgctcctgcttgcgaaagactactttccaagtgaatttcaaactcatgaattaattcccttcctacaggttgatttgattttcttgcggtgtggatgatggtagatgaagatacaacatgctatggagaagccggtgacttaatgttttatttgattatgaaacgtttacgtatttctttaaataaatagattcctatgaacattatatttggtactattctatgaacatttaaatggttaagttatttttacaagtagatatatgttatagaaattaacttacaagtcacgttaccacgaaaaaaagttagcgatttaatgttgctgtttgttaaaaattccagcttttgccttgactttaaaagaatttgcaactcaatcattacttggaattttttaatagaactagtggcatttgatagcctcataggttagctactgaacaaactttgaatcatgtcaatccgatgtcagtaaaaattttatatgtcactttaggtaaattaagtgttgctgttttatgaaaatttcagcttctgcccttgacttcagaaattcataactcaatcattacttgggatatttggacaaaaccaatgggatttgatagtctcatggaccagttactgaatagtcttaaaatcatgtctgtagaattttatatgtcattttaaataaattacactgttttaccttccaacttaaattgctgcgggtttttaaaaatattttaataccttttattttgccaatggaagccaaatatttattgtggaatttttggaatttgtgactgaatgtcaaatgggttgctttcatttgttgaatccagtgatttgaagagttgatttggttgcagtgaggcagtttcattcatcacacggttcacttaggagcagggttcttggtttggttttcattgattataactttgatgattgaattggatattggtaggcatataatatagttgtgggttggctttgtatatactcctgaggcatggcaggtgtagatatttctgctaagatttcttccaacagatagagtaaatggcaaactctaagcggtaaattctctttttgtagattttccagaatttcttgggttgaagaacaaaatgtgaaagaataactggaaaagtaaattaattatggttctggaatttctgattaaatggttccggaatacattgagattcttgaatttttattttattaaaattttgatgatgccttctactgacatgatgcaacaagaaagattaatcaggtacatcttgtgtttattttttcagggatttttttttagataattaagatctcttcaaagctcattacagaagatttaagttttcttttgaatgaaattgattaatttcaagaacgtgacattactttatggaaaaggttccaaaaacttgtaacttttagtttttaatttttaatttttaattaaatggtgaagttgtgatgaattctacagtaagctgatggggaattcatattttaattctatgtgattgttgatctctgattcggatgctctgttgatgaattctacagtaagttgttatgctgtagattatatcttttggtctcatgagaaggcagtgtgtgattgctttggtgtattttcttgtatctttacttggatttgtttcttaggcctccactgattaaaaatggtgtttgaattaggttcttggaagaaaaaaaaaaatggcgctggaagcatcatcatgattacattaggttggggatgggtaagaacttgtgtctggtagtactagatttttgaaactctagaacttttatattggatgtttcatgggtgttatccatctatgtaaacacaccaccaaaaaaaaaaaaaaaaaaaaaaaaaaaaaaaggaggaggttcttcccataattgtatgactcttaccattgaatgaatttcagttgtcttttttgttttatttaagttgtactctctaatgccaatcatatccttctcaacattacaccccagcgttgtgcatcagctgacttcttacttttgtagttgcttcattccagagcagcctggaatagacaagaaattagtttgttatatccatactttctagtgttgtatatttcacctttttgaacatgcaatcataataccttttgagcaaaactatcatattcaaaatttgttcatgaatacaacaggaatggttattaaagaaacattgagactataccctcctggtcctttgttagccccaaaataagcagggaaaaatgcacgattggtggatatgatatcccggctaatacaatagctgtaacaaatggttgggcaataggaagagatacagaaatctgggataatcctgatgtttttgaacctgagagatttagtaatatttcgactagttaatgattgaatgtgctcgatatatgtttcatccagctattgttatgtttcattatgttgcatatttttaatcgttgctcaatatatttttaacacgtacttaatgattgaatgtgctctttctaccttgttcttccaaggaaaaagatagtattgaggataatccagaagaggaatcttcacaagctggacgtgaacatgattctgaagccaagcaaattgagaattggtagagcagatactgagggtaatcagcctggtgtcccttcatctccaatgccattgtttgtgtgcaatttgtagtttagatagtttattgtagtttcgagctttatagaggatgcaatagaaactcttcaatccctactcctttttagttaggtgcctttttagttaggtggtattgtatcatattctaacattcaagtgtattgattcaaatatttgtaatgaaattatcaagttttatgcaattccaaaatttgttctccaagtgtcattttcaattttaccagtgaatttacataaattgtggtaataaaaaaaggtatctatagcaacgatcaaaaaatattgcaaaagccacttttcataacgttttttatacgttgccaaaagtcacttttcgcaacgttttttagacgttgcgaaaagtcactttttccacattgcaaaaagtttacttttcgcaacgtctaaaaaacgctgcaaaaagtcacttttcgcaatgtttaaaaaacactacaaaaagtgacttttgcaacggtgaacaaatgttgtcgtatctcttccctcaacggcaacatcgaccccgcaacacacgctaaaacgctgcaaataacattttgcagcattttttgaccactgcaaaagcctttttttggtgtagtgggttaagaatttcttcctttttgattatgacaaacataataatttgcaaagtaatatcaataagggataaagaataaagatcacacatttaaagcatatcccctaccttttacaaactaattgttatacatttaaaacatatcaaatagaagatgattcaaagtatatcatttgaagtgtgccatttagtctttcaaagcatatcatcttactcatatttcttattttcaatgcatttcaaatctatcttactcaatttcctctttttggcataaacaaaaatatagaacatatgagagcagaatatggcatacaggatcaaaattttaagtcaaatttaggaaataataatccctctcaattaagcataaaatgccaaatatatgcaattttaagcaaggggatgatcatcacatttatagcaaaatactaattagagcatgagtgatgaaatgtcaaaagcaaaatcaattgggtaaagttcatataaattccaaccaacgatgcacatagaatcaatcatgcaagaatacaattcagccactcacttcaaatttattaataattctcaaaccccttcgaatatatgaaaatctatcaagtgttagaggtttagtgaagatgtcaatcaattgattttttgtatttacgaattctaatacgttatccccctttaggtgaattcagaagtctaaagacctaatattctagtacaataaaatatctaattttttttttaattacgaaactaaggtgtgatactttagaattgtattgaaatctagcaaataagtatgcaatttaatagagaagagatctgatcattttgtatttaacaaggttctagtttacctttttgtacatttgcttcttcttcatattgatctttagtgtcttcctttttttcatcttggatgttcgtttgctcaaaaagaatctccaaacctacatcatcaacaatacttttctcttgatcaagaggattagctttatcaaaaatttcatccatggattcatcaacaaaagttcaacaacttaagttcttttgttgaagaatcgatagcctttactcctagacggataaccaagatagatttcaatatcagactttgaatcaaattttctcaacatttcttttgtgtttaagataaaacatttacaaccaaatacttcgaaataactgatattaggaactctacttttgaaagctatatagatttttgttttctttcgaataactaatattatattcataatataacaagtggtgttaacggcctcacctataagtattttggtaaaccagtttcatttagcatagtctgagtcatttcttgcaatataagattcttcttttcccctacatcattttgttgaggagttttaggagctaaacaattttgttcatattcattaatattgcaaaaatcaccgaatataatattgtcaattttccgatcatgatcactcccaatggtagtaataatgtaccccttttttgttttgaaccattttacgaaaatgtttaaatgcattcaaaacttcattatttaggttcaaaaataggacccaagcgaagtcatcaacaatcaaggtagcataatttttatcatttaagcttgtgattcttgatggtccaaaaagatttaggtagagaagttgaaagtgttttatagttgataaacgttgctttagtttaaagagcccttcccttgttttccaaaatgaacatgaatctcaaattttatctttctcaaatttcaaatttgccaaacctttaacaaaacaatttttgaattttttttgaaagtacgtatatgctaacataacctaatcttctatgccactatcaagtatcatcttttcaacttgataaacatttttcttcccttcaattcggcttcctataaatataacatcttttcatgtagtatccttaataaaaaaacatggaagaatcaaatttgatatgatatcttttatcacataattgattgatactaagtagattatatttaaggttatcagctaagataaatttttaatagaggaagacgaatgattaccaataattccaatatcaatgacttttcctttggcattatctctaaaatggcatggcacccatctttcttttgaagcttgataacgaagttggatctccaatcatgtgctttgagcatctactatccaagaatgttttgctctttgttttctttggtacctacaacaattttttttgtctttggtactcaaataactttggatgcatcactatatataacaaacccttatgaacctttgggtatgcttaacacgggtgttgtaatcaatctttactatagttcctaaaaactttgctcacatttaatagtccattaaaactttacttctttctttgtcaattgtatcattggtagagctattttggagaatccttcgattttgtacccaaccaatcctaaaaacttcgaacttcactagcattagtcagtgtatttcaattagttactagtttcacttttattagagctgctgcaattccgtggacaataactacatgaccaaggaatccaagtcgcttagcaaaaattcccactttataagtttgacgtataatttttccatacgcagtatttctaccgttattctaagatattccttgtgctaatctccactcttggattatatcaaaatgtcatctatgatgactatgataaattgatccaagtattgatgaaacacacgattcattaaatccatgaataatgttggatcattagtcaaaccgaacgcataacagtgaattcgtaatgtccattacaagttctgaaagttgtcttagatatatctcttgccttaacctttagttgatgatattcaaatcgcaagtcgatcttagaaaataccttagcccttttaattgatcaaataaatccttgattctcaaatggtctagttcccgatagtcgatacacatcctcatatttccatctttcttctttacaaacaacactagtgcgccccgtggagagatacacttggtcaaataagccactgcctaacgattcttgtttttgaattttcaactccaagagttcttttggagccattatctatgtagcttcagatattgatgctctgggaaccagatctattcgaattccacctgtctatttggtggaataccaagtagatcctcacgaaattcatctataaattcttgtaccattggtatgccctcaactttatcgccgtctgttttctcaagagattttaactaaaacatgtttattttctcaacattttctcggcttacatggtcgataccagttagagatagggtttgttctttattccgaggaaagaaaatttttcttctcctagtttctgaaaagaaactttctcttttgtacaacgaatggttacataattatattcgaaccaattcatgcccaaatcacatcaaaatctttcatctctattagatataaattagtttctaatattttttcctcaatttcaaaattcatcgacctagctaactgatgtgtattcaatcttctgcccaaggggatgtaaacttctagtgttctctttgacttactacaagtaatactagatttagtaatgaaagacgtcgatacaaaaaattgagcagctctcgaatcaaacaatatataagcaagtacatcagatatttgaaaaatacttgctattacgtttgagttctccttgacctctttctgagtcggtgatttcccatatttgctttgatcattgttgtcatctttcttctaattaaatgtgggatagtccttagtaatatgccatggcttaccacatgaaaaatgggcattcgcgattgcaactactatggctttgtcttgaccatttcactatctctttgcaaattgcactttatcctgttgattgtacaattgattatgttgctttgcattagccttccgataccaaatagcatgagctcattccagcatctcacggtatgatgtgaaatgatgtgacataagaatcattcttagatctggatgtaactctttcgcgaacctttgagtctttttaatttttgtgtcaactaggtgtggagcataccataagagtttgtcaaacttttgctcttaatcaattaggaaaatattacccggcttgagctaaaggaattcgttctccttaaaatctcttagagattgagaaaaatacttgtccattactttctctttgaattgttcccaagttaacgccaactactactcttaggtcctagttctagacatcaaatcccactagtgacttgcatcatcggtaaatataaactttgcacactggacttttttaatatcagtgtaggctatgagtcgaaaaaagtgttctaacttgtgaagccattcctcagctaatattggactagatgctccaccgaatgtaggggttttatgcctttgaaataacttaactatcgaggcatgggtccagagagtaataggagctggtggtgtaggtggagcttaattctgattcaacctgctaagatgttgaaccacttgtgaaaggtaccttgtcaagttgttttgatttgctcgaaacattttccctgaagcaagaaatattttcttttattaaacttgtatatcaatactagaatattggaatgaaaggacaaagtataatatttcacgacttgatcacatgattttttctgttaactacatgttgaaataggaaaaacaattcaataaagtttattattatggttttctttcaaatagaagattaatctccataagctctactcatttcattcttagtcttcttctgggtcctcaactagatcttcatcttcctcttcgttaatattttccacaattggttgtgcgacttagtcatctgaagtcactatcgattcggatgccgagtgagagataacatcaccaatcataatctcgcaattatggatataggcattgcaaaaatcctcatagttaagttccttaagtttactttctaaattttgagatagcatattgtcttgtataaacttctcaatacgtttctcacgagatgcaagagattctagtagataacttattgcttgtcaatcactaatactataataatcattctttgcttttagccaatgctggtatacatttcgtatgtgattgtcaagatctaaagtttcgtctacctcaaaatcaaggtaagctcaaatatctatctcctgttgactaacatgattccttctactagcaattatgtcatcccctagccatctatcattcacaacttaaatttctagacaaatacatgtcttttaatcattttctttttcaaattatatttatctttgcatataagatatacatgaagaaaaatgtagaatgtaccgcaacatggaaagcataaaatagtcgtaatatttttcataataaaaattttaattttgcttagttaaacatacatgggttgtaggacgggatcgatcaatggatgcaagatgccatggattgccgtaaatgttttattttatcattttaatttcccacttgtacttaaagtatttatatattttttttttttgaaaaataatgagtctacagaatcgactacactgtgctttgacactatattgtaacacttcaactcttatagatcgaaacaccatagaagaacatttgtaatttaggtcatatttagaaattttttttgaaataatttaattaaacatatatatttcttattttaaaaaaaacgtaaaatttcatattaagaaaaacaaactatcaaataatttctcataagtgaagccacttcttggacaacagcataacaataaattattccagtagaaacgaataaaaagatatgtaatcccgaataattctccatgcatatattaattattaatttgtgtagtgcatgcagagctttttggtaataccgaattaagcaacctgtttcgttatgaatctcggaacttcatgaaattttaaagaaacgtaggaaacttcttataatatgatatgtccaaaaatcggcttccatcaacaacatatgagatactaaaatattatccaaaccccacagtgactatgtttagaagataaatcagtacagtttattaaagtgacataaaattatacaaatgtcaaattgacaagatttcaagtttattctataattaacccatgaggctatcaaaccctgaaataatcgcttgcacctttacctatcttaatttgaagcttttgaatggataaagttgtacgataaatgttgtttccttgatggcacccaatgctttaagaaatctgcttctctcaagtttttcttttctttttttcaaaattttttcttgtttcaaagtgtgtaaactatacatagatatatagtagaaaggttggggttcaacctttatagtagaaagtaatatgatttatatgggaaatgaaaatttagtcctacagtgaataaacgtttgtatattaatcacaattgatgaggattaaaggaaatgtttaatagggaaaatgatgggttaatcacgtgtaggaattgtcggtactcatctccattttaaggtgaattaaaagtggcctttttatgctttaattcatgcatatctctctctctctctctctctctctctctctccccccccccccccccccggaatttgaggaagatgaaatattgtcattaaataaattttattcttggtccctacatttatttaatgaataaattaaggaaaacaaccgcacaaattcacaaagaaaaaatttaaatcctcttttacatataaattggtcctttttacaaaataacgtgtacaaaacatttagtattagaaacgtttactatttttaaaataaattttcactacctggtccaatctttgggaaacattaaatttagtcctactttatttaaataatttttcttttaaccaaaacatgcatgattgctcattgaaccttcgtgagattaaatttgtttagggcatatcaaactaatattggactttcatttctcatataggccgagcataagactctttaatgggctaggctcatggtgctagctcatcatattaaaatatgagcctaattttattttattcattttttttttttggaaatctacataaaacaatatcaattaggatattatttgtgtcaacatccatatatgacttacatgctcatcaaatgaatatcaaaacatcattgttaatgaggaacttgatgaggtttatatggaacaattgaaaggatttttctactcgataatgaacataagatgtgcacatgagtaaaattattatatggtctaaaacaagcaccaaataaatggcatgaaaaatttgacttcgcaataatttctttttgcttcatgcataatagtatggataaatgtttatattttaaagtatacgacaaatatgttgtatttatttgtttatatgtcgatgacatgttgattataagtaatcacaagaaagagataaaagaaacaaagaggtttctatctttcacatacaagatgaaggattttgtacaagtggataccatatgggatgtcaaagttacaaaacttagtagaagttattatttgagtcaatcacattaaagaatgtgaaatataagttcaaagacttgaccataaaagagtttagtacccctcttgatcctagttccaaacttataaaattgatggaagagctattgctcaattagagtatgcaagttctatagatagtcttatatatacagttcaatgcaagatcggacgcagcatttgcaattagcaaacttggtaggtttattagtaatttgagcaaggaacattggaaggccattaagaaagttcttggttatttatagaaaataaaaactttggtctacaatattttcctaattttcagctatattgaaaggatttattgatgttagttggatatgtgaatacaaatctatttcgaattgggtgttcattcttgcagaatttgtcgtttctttgaaggctaagaaataagcatgcatatcaaatttaatcatggaatctaaatttgtggcattagccgagatcgagaaagaaactaagtggcttaaggatcttctatatgagatacctttgagattgatgaatacatcttcgatatttatcatatgtgatagtcaagccacattaacaagataatacaatgagaagtctagatctatgagcctaagacacaactacacgaaaaaattaatcaagagtggaatgattttcctaaattacgttaagtcaaataagaatttagcgaatcccttaactaaacctcttaataaagatttagtaatatctacatggattagaatggggtcgaacctccttaattactttaagtcaaataagaatttagctaatcccttaactaaacctcttaatagagatttagtaatgtcgacgtcaattagaatgaggttgaaattcctaaattaaaaagattcaccgatgatggaaaccaaacttttcattactaaaatagtaattcatgggttagaaggataacattaagtcattcaataagtggatagttttagtatttatcatttctgcaaaaacctaatcctaagctaaaaatgccggttgttacttgaaggatggctgagctttaagctcctaatatagttcggtattaagtacatctaaaagtaacaacaaaactagaagaatttcaactagattaccttagaggtggtgctgcctcaacgaaaagttagagtttctcttttaaaagtcctactaataggataaatgtaaggtcataaatgtgctaagctaatttaaggaacttgtgaaacacatgacccttgtttctatttttttcacctgtatcatcacgaggaataattggttcaaagctatcatgatatctgaaaaattccaatgatacttcgtgaaaattacactatggttaagttcaaatagcaagagatctaatccttatgagtcgggttgcataagtgagccatataattttgaacaagtgaaggattattgtaattttgttcaagaactataatggaaggaagaattggacaatggacatgtgctgtacgttgaggacaagaaaaaattaagccatcgcccgatgttttaatgatgttgtaaagaggttttgatttccactgggctgtcacctggtttacaactgtgcgatcacctaggatatcaaaactagccattaggcagtttcccaattttgatttttggtgactttacatgaaaaaattcaacattttcatgaatgattggcattatttcatggtgatgtttagaaaaccattaataggtgatagtttttcataatctatttttttatttatttttattttttttaataaaaatataaaagaaccataaaatgtgttctcaattcaattttctatcacaaacaaactttctaatgttcttaaattctttgaagaaaaacacaaatttttaagtgtttccttcttaaatgctggttataatcctaaaaatcatttgtcggtgaatcctttaagcacttaaataatcctagaagaggtaaatattgtttgaagatagttattacatgttcaagtctattacttcattttcggtgtttttgttgtcatctccttctccattctcttgatggtcgatttttcttttgctattattttcccaatggatttttaatgggttgatagcattccacactttatttcacctatcggcttgggtgatttcaagaaaatcaatttctcttaaaaaaaataaaaataaaaattacatggacctttctaaagtttataacaattacatagaaacccctattgttttaaaatttacagaaatctccaatctcagtaaaaactttccatttagcaaatataaaattataattgtttttttcacttatttaaatttagataaaaataatattttcaatgttaaaaaaattaatttttttatcttttgtacaatgtgatttaattatagtcatacttttttgaaaagtatatttcccattttaaaaaatgaataaattaatattgacttaaatatttattacaaaaagaaaattcaaaattctaatattcttatgccatttttagttatgataatattacttaattttcaaaacttaataattaagaaaataaaattagggaaaatgctactaaatcaagcatatttaattatttttagttatgttactaaattgctagcgatctcattaatattagacaataaataaatgtaaatcaatcaatgtagtattgccacctcatcatctataatgctttttgttcattttatctatataaggagtttgattctattttgagatctagctttttgttgatttttgacaatttttagtaattttaggatgtgattgtgaagaaaaatagtgaaaattcaacattgcagggatcaccttcttctgttgataaatttggttcgaagtttcatgggattgcaatgagtataggcaagttcgcgacgatcctccccacaaagttttaaaataagtatttaattaaatagcataaaataaaaaataaataaaaagattcagggtgggattgggaaatttgggatacgggaatgataagtatagttgtactattatttggatgatcaaaagtgaataattttagaagaaacacgagattcaattgttttaaaatgagcaaaaaataaaaaataaaaaatgaaagaaagaaagaaagaaagaaaaattgcaccaaaaaatcttaaattgagtaaattataaaatatggactagagtttcaaaattggaaagattaagcacttctaaatgaaagctctagaggactctctgtacaaaagagggaaggtgaggaccggactggatagaaaaataaaatgtgtgaatttatttcttatttccctctaccaatttcgtttcccaccaatttcacaattcacgtatcaagaaaactcatcccacaatgacaaagccctctttctcacaattttttcaatctccaattttgcattgcggctttcgattatggctgtctaaacaatcaaaataaaattctctgtatcaaaaggtatgtatcttttctcaaaaccatcgattataactttccatgtctgtctcaagaatcaattattattgtcattgatgtcgtgtatgctgtcaagaaatgttaataattttggactatctcacattattcttggcctgttgggcctctttacattgggccaaatctgcttcaccgggttgctgttttttaaagtgataaaatgtgttttcagttataacgcctttttaaggaatgaagatcatccgtacacgtggctgctcttctgcactctgattgtgtcgattgaaatggatagatattacactgggtcttggcattattctcattctagatgattctttcagtctcttcgtctctctctcccttttctgagtgaaaattagggtttagttactgtaatgtgagatcgatctttgtgattgatagttttctgttctttgtgaagagagatgattgttttgtacgatctgtgagagtgaaaacagttttgtgttgttgtttttagagaggcaagaaaactctctttacatttgtatactgatttttgttcgatattagtggatctagagcctaatctcttgggagatgctcaacgggtgattagattgaaaaatcgaacatccgggcccttttaaaaggataaaacatatttggtgttggtttttcgattttctgcactttttattaattcttgaatttatcgatcctttaagatttgtagtttagaacgtaacaaaaagtaaggccacactctctatggttcggtagatagtgtattacggtgtgagcggctcaaatttctgaagttagattctcaatttttagcctgttattaaaaggttaaatcctaaccttaagggtcccccatcacccctgtcctgaagtatcgtgagggaggtaaatcgcaggttatgcctccaagggtacagggtggaaggctgcttgtacacttgcacttacccaagagtcaaatccatatttcaggattcgaactcttgacgcagcagtttcaagcaaagctggatttctggcctgttattgctcgtacttggggttgtttttgagaaaaggaaagacctttcaggaagcgctaaatggagagtattcataaaaccctcaggaaaccttttaaacagtctaaagacctaatataatattcatagagaaatatttaattctttaggcattaaaacttgaagaatatttctgttgtactacataataggcaaatgcatacaattctgttatgaatgtatatcggtatgtaatgtgtatctatatggatgttcattaattttccattggataaaaacaacagaaaaaaaaacaaaaaaatataacctctccgagatggtctttagcaataaaaaattcaaatgttgactagtcaaggtcaaagtcaattaagaactaaaatgaaattaaatattttattggggtttattttacaattgacaatatatgagggttaaattggatacaatttaaagttgggaatttacttatatatttttggaagtttaggattaaatgtgataaaaaaaaatggagttgagggattttctttgcaattttttgtaaatgggatttatattcaacctttgaccatctttttctctcaaaactcacatcaacacctactagaaaacaggcagagagcaaaaaggccgagaaagagagaaaaactaaggaaagagggaagaaaaaagtgaaagaaggaagaaaggaagaaaagggaagaaaaggaagcaaggtaaggttaatctcttcaagtttggatttaattttttccatttgttacaagtgataaaagtatgatttatgttaaaattctacagttttaacttgtagtaaaaattttcaaatttaggtgtgataagtacgaattggagctcaagcttggggattacttcatttccaatttcagttaagtaaggaatattatttttaacaaaccctagaaatttcatttgggatttttggatgaaaataatgatgatgaggaaataattatttggaagtatgaattgatggaacaagaggaaaatttaattggtcgaagcattgtgacaagtatgaagtggtagttacattaatgcttggaatgaaggttatgttgataaattagttactagaaaggtatcataaagtgtgattagctccaattaataaaagaaaatttgggaatttaatcaagtatcaagaaatttaattttaagttctatcattagataataaggtttcttgatttaatagtggataaattggttattaatatcgtatttcaggtcacgaggagattggaaatgtttatcaggcagtctagcttgtagctcatactttgtgagtggatagaaacttatttttcataaattagtatttattaaatttatattataatagaaaatttattaattcatacagatgaattgacaacatgattcttagaataaagtggattttatagtttcttttaagttaaattcaattcagttaaatcatttgattagcaaggtatatgaatattaaatatttcagcataattaaagttagttttaaaaccaccagaaagtacttaggtgattttaccctaatccgcactgttgtgaatgtgtttctacaatgtatgatcagttatggtgattttacccgctctgcactatggtaaatgtgttttcatagtgtatgaccagattatcagaggcctttgaaagccattctcgtacacacataggctttgggccgtgtactagggtgattagcctttggagcagctccacgtacgtataatcagattatcatatgtgaatggacttgctttgtacattgagattactctgtacatgagtaaggctattcatagactatttggtgtaatttttcagtatttctatagcttatcagatttcagattatagattttcatgaatatcaaattctttagattcattataccttacagatagaacaaagaattttataatgtaatcatgtttagtttttaaagtattactagattcaaaatttctcaaagatttaataaagttagaatttttagaaaatatgcataaatggaaaagtatacttatttgcaaactgtccactcactgagttacaaacttatatattttgtcatgtttttcttatcaggagaccgttgattttgagatacttggaaaagcctacctaagtcaaagagaccgtttcatagtaagtaatgaatagttggggactcatgtttattaagtactttgtctattattttctttgacgtgtattttgtagaagggtttgtaattgatgtaatgcttgcttgtagacatgatgctaatgtagaagtactcagtcgagtttagttgtattttgttttagttgtggtggtattagtggaagtggtggtttgaatgtttatatgaggttttgttgattttttaggttgattttgtccatgtctaaggggaaactctatcaaattttttatagaaatatgtcacagtcaaagtaggtcaagtttgccttggtggtgggttcgacatttagctgacatctaccatcggcgcacgatacgtgtcgagtcaattaggttgattggggttggtcgtgtcaagacaggttttctttgtccactaaatgctttgtgatttttatcattacaccaatttttacatttgatatctgggaggttatatcaaacttgatatggatgtttttgggtgcaattagaactggtttgatttatgataattttgtgatactaacatgtatactctctctctctctctctcatttgctagcacattgtacaatgaataaccaccaccttgttaggaatgaattttgttggaactctaatctggcaagtgtccttgacacaacccgtcccgaatcactttaatggactcgacatgtgtcgtgcgctgatggtaaatactagctaaacgtcgaacctaccactaagttaactttgacttacttgacttaaaaatatttttaacagaattttgacagagtttcccctgaaatacgaactaaaaccacctgaaaaattaccaattttctcaaatcaatacatataatataaatcagggtacgtcaatccctcaaaatacaaactattcaaataaaatgttggcaaattaatatttacttgctttacaaccaacaatcctcaaatatattaaagataccaaatatctaatgagcccataatgaacttttcttatttatactacatatattccaaaataacacataatgtataatctgataaaggatgtcatacaacctatgacgcgtgactcaattcggtagttcgacaggctccaaagctactcaattcgattgctttttgtctgataaagaaaaagatgaaaaatatatgagattaaagctcagtgagtggataatttacaaataagtaaacttttctcatttatgcatatcttctgaaaattctaattctattaaaactttgagaaattttgaaatttagtaacagttttaaaaccaaacatgaatacatcataaaattcttttttttttttttaattctagttcaaaactgtaaaatataacgaatataaatactatgaaaattcgtgaaatattgatgttgctcaatatataagctagacgctttattctgagaactgaatagacagaattctatattgaaaaatcacaccaaaaaggtacccgatgaatagctttactcatgtacagagtaatctcgatgtacaaggcaaagtcagtcaaatatgataatatgatattttattcataatgaaataacgtcaataaaataatttggtcaattcatgtcccaataaaatgatttgcttcattttagttcttgtttgacttagattttgacaagtcaacctttgatttttgacttattagaatgagttgtaacagtcctgcctgttgacttgagagagaatgagactgcgtaccaagcatatgctatttattgaatgcttttgcattattacttctagttgaggctgtgggcttacattatttgtaataattaaactagaaactgaactcagcaagtgtgaggggggaatgttggcagtgcaagtgttatgctggtctgatgtgtccgtgctgcatctgggaaggaaaagctgttttatcaatattttcaattccatgttcttgacaatagaagcaataatgtcaaaacatagttatctctctttttgaaaattgtaaaactattttctgaggtttacttttcttggattcatgggttgacaaattggcatagactgagaaatggaagtttaattaaataaaagagttctagcaaataatacaactacagaaaatgggaattgcaatttagcagaattaaataaatagattgatagattagatataagatgaatataattaaaattagaaacaggatttaaacaatataacacgaaagctaaaaactattttagggtgtgatgaaggtaggagaagtgttacatagcctctttaaactcatgaaagcatattttgatggcccatactccacattttactcgatgccataacccgtaaaagatggtttatgggatcgatttctggtaattgttatttattataattgcttcctttgctatttattatgtttacagttaattttttattaatttacaaggataaatatgtatggctattggagaatactatcgatgtgtatgacacatgaaagacggcgaatgatagatataaaaatatgatgaatggtgctcgcgaaaaaccgaatgtacaagtcaatttgataaacctatcgattggaaatgacgtggtccgcattgaataagggcacagcactggaatgtcttgtaaattattgaaatacctagaagtgacaaagcaacgcgaagattgcaagtgagaatcgccttacacaaggacatgatggtaaaatgaagaaacatactactactattggtagtctcttttgtgactacaaggaagagatcggtaattttttctcattttatttatattttgtattttaaagttcatttatttttttaactgattgtgattaataaattgcttattttttaggagaaggatatggatcttcaaatgtctgaattagagtttttcaatcatatccacaagaaaaatcacaaacttagggattttgctgataaaaaattcaaactagttcatctaagtacaattagagtttaggtacttcatagtttgttcatataatgagtatgacaagcattttttttttccacatgatacttaaaaggcttcaatagagtccaaatttgatactgttagagatgattagcctgagctagatcacaacttatggatgtatgttgtcaatggtccatctaagggccgtgtttatgggtttggtcctcgaaaacctactttgcatgttcttggtgcacccggggctggccgtgaaattttagatgtcctgtgcgacattttaaaatggtgcccctttcgtgtaatataaaatatattataaaaaaaataattcaataacatcatttcatcccaaaaatatgacattatatatatatatatatatatatatatatatatatatatatatatataacttcatcaaaattcatatgtcatcaataaagaatcatccaaactactaacctcttggtacaatttcacatgagcaaactttgaaatcaaaaatagcaagtaccacatgtaaatcttgaaatgcaacaaatcatgtaaaaatatttgtcctcgcatttttagagagaaactcattaattaaaccttcgtaatcaatatgttttagcaaatctttttcaagaaatatcaaaactagtcattcatcatttttataacatggttgatcacaaataagtttttaatagctttagttttgaagaacatttttcgacaaatgcaacaataacaataattatcaatagtattatataagcaataaatatattcgaaaaacaatataatcttctcaaataagtcaatatattaaaagctatttttgtttcttttcgtaaaaaaaaaatccaaaaattgaatgtaatcaactatcagttatcacctaacaaaaacttacccttctagaaccaaaataataataatagtaatcatgaaatagcaattcgactcgttcttgtgacttggttgaatgcaaataatattttaatagctttagttttgaagaacatttttcgaaaaatgcttcaataacaataattgtcaatagtattttataagcaataaatatattcgaaaagcaatccaatcttcttaaataagtcaatatatcaaaagctatttttgtttcttttggtaaaaaaattctcaaaaattgaatgtaatcaactatcagttttcacccaacaaaaacttacccttcaaaaaattaaaaaattaaaaatcatgaaatagcaattcacaaatggaaaacgggctccaacaaatagattctactattatggagtaagtaataaagattggcaataaagtctcttttattctttatttgactattctttgtaggttaaaggatgagaatgagagaattgataaaagtggatctagtattagcttttcactctccattttaatcatttgaattttgggcttcttattttctttttagatttgtaattgatcaatgaagctaattggacaattgatataaggactagtaaaatagatagtttataatatttttgaaagcaagatattttagaattataaaaatatttttttcaatatatgttaaattaaacatttattttcaataatatattaaattaaacaattattaacataatataatttttttattcttttttcataaatattttgccctttaacttaatataataataaaaattttaaatctttaaattaataaagtaatatgtaccattataattatgtacttctacatatatacagacttacaaaaaaaaaaaaatttggtacccctataatgctgaggccctgtgcggtcgctcaactcgcacgcccttaggaccgcctttgggtacacccacttcacctagacattcaatactttcacgtgatgaagagctaaataatttaaagtctgagctggctagtgcaggaaatacaatagaaaaaacaatgaaaggattgacgatttcactatacatcttgaaagagttgaaaaaatcataggatcgagttgtcgagatgggagaaacatggcagagcatgtttagggaacaaaatattctatactttcaatttccttctaacttgggatgatgaaatgatgatgtgtaagacatgatcttcatacattggaattttcaatttccatgtaataacttcatttattgaagttttagtgcattttgacggttttgattatttatttagcgggtatttgataatattaattatcacttagcaagtttcataaatttttagtaatttttattgaagtatgaataaattaagcttcacctacgcagaaaagttaccgacagaaattttgtttttaatgataaagtttttagatttttaccaatgaaaatttgattggtaaaggtaggcttttatcaacggaatttttggtaatggtaattttttatcaacaaaaattcggttggaaaataataagtatctagagttttatcaatgggaaatcaattggtcaaggtagacgtttacatacggaaacacggttggtaatggtagatatttacccaccaaatgtccgatggtaatggtaatatttttatcaatgaaaattccgtaagtaaaaggtagatttttaccagcgactttgccctttttattgaaaatattcttctcaaatcactccagtatgatggaaaggggacgttcccaaaatcagtactatcgggtcgagtgaatttaataatagatgcctagcggcagcacgggaataagttgcaattggtataggtagacgtttacatacagaaacacaattggtaatggtagatatttaccaaccgaatgtcctatggtaatggtaatatttttatcaacgaaaattctataagtaaaaggtagatttttaccaatgacttagccctttttattgaaaatattcttctcaaatcactccaatacgatggaaaggggatgttcccaaaatcagtattatcgggtcgggtgaattcaataatagaagcctggtggctgtaccgaaagaagttgcccaccccaatccagatcaagaagagcgtgctgcatgcatgttacgattagatactccgttggtaatgaaaagatttttactaacagaaatttcgttggtaaaagttttacattttattatttttcttttaacttttttgcttttactcgaggtgaacatgccaattattaatgcgtaccacatgccaccaggggcggacccagacctttagtattgtggggtcaaaattttaaaaataatttttttaataaacaacataatatcaatgaaaataagtttatacgtattttgacactttgaaaacgtagtataattacatcattattatattattaaataaattttgctacttgtatagttttgtttatcattttattggcaaatgctgagctaacattgagtaaattaaattgaatatataaattaaatgaattgaaataaaattcaagtttagttcaggaagtaaataaaattcaaatttaaagtaaatataattcgaaagtaattcaaattgcatttaatccgtaacgtccctaaaaaatttacgttatatttcatgtaagacttccgaatgaaacgatataaattatattgaaaaatttatcgtgcaaaaataataattaattgaattttttaaaacaaaaaacgagttaggcgtcttttttgaggcgtacgtttgatgcatatttaactattttcgatatccatttggaccattcgatatgaaaacgatgtagttttctaaacaaatttttacatggtatagacgatttgtggatttagatagcacatgatcgcaaaagaatttttaaagttaggatattatcgaaattctcaaaatactagtttcaaacgtcatactttaacatgtcataacttttgctatagttgaccacttcgcataccattaatgagtgaaaaactaaaccatgagtacttcgaaatggtattaaaaatgcaatattttgacttcatttggcatcccgacgagtacattaaagtagattaaaaaaaatcaggggcaaaattttgtggggtcatttgaccccacatgaccccatgtgggtccgcccctgcatgccacaaacatccaaaggggtgtccaaatggtgctaggtgacaataatttcaccttaagtcctcaaatgcactaacgttgatttttccttcacgtccatcttgaaattttttgtcatgatcgttgcactcgaatccttgacccatgtaacttggacaagtcattgcataatatttttgatcctctttgctctcgatcctgttattggtccatatgaaatatgtaaagaatccttgttagcttgacctccatgattccgatcatgaattgttaaaagtaatactctagttgttgtttaatgcatatataaatcaaagtgaacatttttgggcgactatccaaagaatatttattctgtaagctttaccattttctgaatctctaataagcaccagaaccataaatttgcagtcagcaaggagttggtttttctgttccaaagaaatgggttttgaatgtagtggataagctacaaatgagaggcaagcttcatttcattttgaaagacagaataattttccattttgccaagaaatgtccacttcccagtggctcctcctttttcgtttgttgttttctttactgcttcaaaaacaaattagaagcttccatctttgatattttagtcgacggaatcagcccggaaaacgatcttcgcttgctatctttgttgttttctggtaaaagaaactgttgtcagaaaacttcatctttttccagtttgctgtctttgctcttttttcagtagaacattgtccaaaaagttcttcattttccggtgtcttttttggaatgtggtgagaaacatggttatcataccgattcctatagacagcgtcaatctgttgacttcaaaaaatgcgccaacggaatcccgacctcgttccctccaaacctgcacatggaataccttgttaggattcaaaggccgccggttgagaaaaatgtcaagcgatcgtttgcactccgacagtcaagtcaacggccagacgaaaagaaaataaagagtgccaagatgggagaggggatttggtttgggtttttagaacgtattttatgttgtgaagtgaacccatatatatatagaaatggaggtgggccaaacgggttaaagaaatgggcgaagtccaattaggcccaatatgaaatatgtataacaatattttccttttactttttctttatttttttgattgtgattggggcgaacatgccaattattgacgcgtaccaagtattctataccacatgcaaaaatcatccaaagaggtgttcaaatggtgttaagtgacaataatttcaactttaattgggctgaagccctagctctacccaaaaaaagaaaaaaaaaaaaaaaaaagaggaaatgataaaatctgttgtatttatttgtttatatgacagtggtgaatctagaaatatgggtgagttggggcggtcgttaaccattaagcgtcaaatgtctatgactgcgttaacgaaataatttattaatatttaattaagctatgttaaaaaatttcttcaatcaatgtatcaatacagtaaaacataaaaatcatatacatatgaaaatataatctaatacaacttaaaataataagaaaaaattacataatacaatctcatttcgtaaatataagctcagacaactacgttctttgggatatatattttaaaagcattacaagattgtctcattctcaaaattttcaaaaatctcactctatatacataaccaaattatcatttaccaatcatctcccattttattgcgcaagtcactcttgattaaaggtgaaaaagttgcacaggtcactcttgaattcaacccgaaacttctttgtgctatcaatggactcatgtgctcgatgagagacagtacgcacgactaaaagaattaggttgagacttttgttttagttgaaaaaattgtttcatagtctgtatgaaaaataaacgtaaattttagaaatataaatttagactatttccaaatttcaaataaaaaatcacaaaacattattacaatttgaataaatcacaaagtagagttgaaaatgtttgggtgtgggtggtatgaaatgaaagttgaggtcaattttgtgaaaaagtaaaaggtttgggactgttgctacagttatccttataatattcaatcgagcaatatactgatcattctcacaaaattaaagaaatatatatatatatatatatatatatatatatatatatatatatatatatatatatatatatatatatatatatatatatatgaaaatctttattaattatagcatgaaaaattttattaaggggaatttacacaaatgtcactaaatatgaaaatgcacaaaaaattttgtgttgcacaatttttttgcaaaaatgtcactttttccccacaaaatgtccatcttaccctttgaaacctttttaggagcaataaatgcttgatttgaatccaattaatggtgtgatgtgattatttatttatctttattgttaatattgaagaaatgaatattatattgtataatatgaatttttgattaaaaaaatgggtggaatgtgtacaaagagcacacacaagtaggaattgaaatagcttcttcttcttcatcatccccctttcattatcaacaaggcatgaaggaaagctattgatcaatttcaaaggtgaggtagtggaaaagaaatttttgcatgccatacttcagtactttaaatattcaataaaacatggtcagaattaattgtccatatttcatctcttatttattgattttttatttttggtatattttagaaagggaagaaataccaatattctcaacaaaatgtgaatcattccatatgtaattccatatttaatgaagcattgagttgtactttctttgtgtgtggggagattagttgaagttgtagttgagaattgattatgaccattaatgtgttgcaataaattcctgaaacagtaaaacacatttttttgtaggttccccgaaacttatgccgttcaagtgttgagcagtttcatagaaactgtcgggttagacatttgaactgtcgaaatcgacatttagtaactgtcgggatgggcagagaattcaatcgtcgattttgacacctgaaaagctctctttttggtactacatggatcaaagtattgtaatgcgccaatttgactgtattaaatctttcgacatattaatgtgcaaaattctgacttttgtactcccaacatttcaggtatggctcaggatctgagattcatcgtgtcgcatgggggaaactttgttcacgtggatgatgaatggaagtggagaggggacaaaacgacttccattttagcgccgagaagcattaccgtaacagaacttgtattaagattgaaggagaaacttggtattattgaaccccgcaatgaaattgagttgaagttcaaagtcccgaatttgaatatacctccggcagagatacacgatgatgaggacctaaattggtacatatctatttataaggagactgcactctgcgtcactattttggaaaccgaggtcccgagtgttgacttggcgagggaagcaaactgtgaagagaatcggttcggcctaacggaatgtccctagactttaagacatggtgaggtcaatcatgtgcatagtgggtcgaacaacgaagcacccgcaccttcaattgaccatatcgaggctagagtatacgttgagtacttagagaacctgttacatggtacgaatgatgttattattgctgaaattgaccggccagtgtcatcacattccatgagtttaggcacagatgagtggatgacagccgtcgttctcgccaaaaagcaaatattctttagcaagaaacaattgtactcgaagattcgtgtgcttgctttgcaagagaagtttcaatttcgggtgagcaggtcaagcatgaaaatgttaaccgttgtatgtgtggacgataattgcaagtggatgctacgtgcttctactgtcaagaaatctgcaatcttcatgatccgtaaattcatcaacgtgcacacatgttcccttgattttcgtcgtaacgcacatcgtcatgccactagttctgtaattgccgagcacattttaggcaaactggatactccaagtcgatcgtatgaccctaccgctattgcacgtgatatggaacgtgagttcggtatgaaaatcagttacaacaaagctcgtaggggaaagcttcatgccttaactatgctacacggtacaccggaagccagttttcaaaaattatcttcatactgccacgtcgtaggagagagtaacccatggatagtaacgcacatagaactcgattctcaaaatagatttcattacttcttcctagctttcggtgcaagcattcgtggttacacgcagtacttgagacccgttatttgtgttgatggcagttatctgaagggtccatacaaagggacacttctactggcaaactacccaagatggtaacaaacaaatatatccattagcatgggggatcgtggatgctgaaaccaataaatcctggaagtggtttatgtccaacttgaaagagcttataggggactccaaagacctcgtatttgtttcaaacagaaaaaagagcattgacaaagctattactcagttgtttctatctggcatctcgaaaagaacctaatacagcgatacagcaacgcaagtgcaatacttctattcaaatgagctgctacgacatatcgggttgaggactttgaaagactcatgggacagatccacagggtgagcacaagagcgtatgggttattcattttggtcccaagcactatttattggccaccattacaacattatgatgaacaacaacgctgagtctctgaactccatgttgagaaaagcccgttctttaccgataacctgcttggtcgaacacattcggagtactttgtagaagtggttttatgaacgtcaggaaaatgcgatcgaatgcagtacagtattgacgccgaggatggaaaacgagttacggatgacattcaaaactagaactaggcttcgacaacatttgttgacaaacaacttaactcaggttggaatatccaacgacatggacatagttgactttttcgaagacacctgcacgtgtcgtgagttccaactaaaccgtatacaatgtgttcatgcaactcgtgctgcttacttcaaaggaaagtcattgtatgaccttttctccccttattacacatctaaatactggaggggtgcctatagcgaagctatatatcctgtcggacgtgaagcggactgggttgttcccagtttagttacatttattcctattttgccaccacttgtacgtcaccctccaggtagaccaccgacccgacgtaagtgttcaagacacgagcctgcatggtcgagcaggaaatgcactcgttgtggttgtcttggtcataatcgaagcacatgttcaaaccccaatgtatcacaagttccttaaacgttgttagtgtaatcgacgttgtatgttcaatgtttttcagtgccctgcaccttatgaagttatgttataaagagtgtgataattaccgtttctggatgttcggcatccttctatgcacatacgaatttgtttcccgactgtcctgttcatcacgtacgcacatcccgacagatgtgttctagattcccgacagttgacgaatgtgtgcacaacacttaagatcagtttcacgtacatggcgacctgtagattctgtgaaagggaaacaacgtaactgtaacatgcttgaaacaaagtctttaaacacgtacaactaaccctccaagtgcacggtcaattaaaatactttaaggtagtaggcaaacgaaattgtaaattgggacgttgtccttttcttgttggactgcgcgcatcatgaaccccatttaaaatatttatgttcaatatccataaaatatattataatttgtaacatcgtcctccacggagagaaatcagctctaaataaatagcatttcataacatccaccaaacgtggtgcaaaatatagatgtaggttcatttgtcgatcccgacagatagaaatctgtaattcttaacagttcgaccgggctggactatacacaaaatacactacccggattacggcgaagcgacttgttcatgtagacattttggttctgtgttaaccaactgcatccctacaaaagagtggactgtacactacttattcactatactccacagccggcatttcacttgtcgtcgacaaccgaacttgctcccccgctatcttcacccgactcatcagacgagatgataatgacctcgttctctgggacgtgcgccagcccatcgtcgtcatcgaaatccctctcgtaggcagcgtcgaccgagagcacaacatcaagcacatcattctgtgacaaactatcgtcactcccaacatcttccaagttcgggaagggaacagggaaaatggctctcctacccgtacgaagctcaatttcctcatcgtctgacgaaatgtagattggaaataatggagaggaaccgggaactgacatcggctcatccatgttgaacggttcagtgcttcctatggacgaactcattatgcttatgtagtaaagtattgatgaaacgaaatctgtctttgagagacacaaattctcacaatgctattccactaagttgtctaagagtgagaataatgtgacactgtatttataagcaacttgaagaggaaaagcaattatggtcatcatctacccaaccaccaagtccaatctccttgttaatttgaaaagcaattggtgtgatggttcaataaatttatagtacctttatcccccatttccccataattagtaggatatttagcactctttattatctttgtataattcagtacatatacattcctgtacctgaaatgcctctgtgcaaaatattcctagcaattgtgccatcgttgtaattgtagtgcttcaaaaaaaatgagattacattatattcacgcacatggtataccgagtacagttcttaagaaatattttgaaaagtagttggaagtttctatagatgcttgagaacaatgtcaatttaacaacgatgtcaacattgagcatataagagaagaaatactgcagttattatcaaaataaaaattttaagcactataatgtctatcttcttgtacagcagagtgcagtttagttgcccttttacatgggtggactttcttggtgccctttaattgatgttcttacttggaaacaaggcgtactttaacaagaatgcaaagatcattttctaaagcgaacttcaacgagaacatagaattacaaatatgccgagaacgtatcttaaaagcgaataaacacataagccaaagtactagacatgcgagtagatgagaacgaacattgcaagaggaaaataatcaagcggttaatgtatgagtgtcagaaaaacgcttatcatgtcaatttaggttccgagtgttcacataatataagacataaaaaaggtatccgacttgtaacagtagaaccaaatgtcatgacaagtggacgcagactatgtcataactaacgacaaggcaaaatgttagacgcgcgtcaaaattccaacgcacatgtcaaatgaaaaagtcaagtgtcaatgttagaataaatgtaaaagcaagtgattaattgtactcgtctactatgttcaccatctgcatgcctctaaaggtaagttaaaaccaaaaacaaccccatcgtcctgggatcccgccacttcattcacaattacttcttcaatgtctttcccctccccctcgtgtacggagtcctcgtcgcaggagcgggacgtcgtagccgagcgaagcgccgtcttgtcgtacaaactctgcctccttcttctggtacaggggcgggaacaagtacgtcagcaacgagaacaggtacggtagcgacaatacctacataaaaatggaaggggcccagtgagttaccgtcaatgacattcatgaaccatatgtattatacgcagtagtaaagcatgcaattaacttatcttcgccatctgtgatgttgcaaccgtcaatctctgcatcgctgacagcggccgcatctgagggctctgtggcagctccgtcttattaacagaacatacgtaaatgcatagcattcgacgaaacattaggaagcaagtgtcatgacatgaaattgtgaaaagtacttgtaatggacgcaataccttcctgatcgtcaattggagtgggcaacggctcgtgctcggcgtccgggcatggtccaatgttagctccctctgttgacaacaacagtaaaataatgtaagcacatttgttatgtcaagtttcgcaacatgagtactcgatgaaataatatgtttcgaattttgcatgaaatacccacatacctagcaagtcttcagtttcgacaagcagctccccctcgtccatgcatggaggactgtatgctctgtctgtggaaagcaacagtgacgtcatgagaggacattacatctcccctatatccaactctaccccaagggtaggaaaaaaagaagtccaggtcgtccaccattgataatggcaaatggatatcgatgttattatccggagcattgaatactccttcgacaattagaaccagccctagcttgtaacgatcagcacgggtcgtcgatggtcgggcaacaatagacagtagttgtgccaatgataccttgtcattggacttaaagtacctctctttcaacattttcctctcaatcaatcgatcgaaatcttccccctcggggaagacaccgcatcttaagcccgtcacagcagcgtactcttgtagaccgaatctcatcaggtggccctgcacattgaaccaaagctcgttcaccttttctgtgcggattgttctaaatagtagctgtaggattagttgggcagagaattgaatgtctggaatatcagccagatacccgaggggggagttgcgaaagtcctcgcgttgccgctcgtcaaaatggtccatcacggtctcaacgtacttgaggttgctgcgttgggaaatgtgggcccgcaaccgtgcgtcttctggaatcaggaattcaaagtccatatgccctgcaaggtgcgttgacaaaactcatgggattagattataaacataaacaatattgtataatgtctaacgctataaggattcaacatcatggatatggtgatctgttgagaactacagagatcatacgtcgatatcgacagactgtctgtggacatctgtcgataccgacggttgatgttgaaataggaatgataggctaactgtcaagaaaaatagagagtcaagtgtcggggtcgacagttcactgggagttgctatgcttactgcggggtgcaagttgaacatattaggtagtgccacatacaagtatgtttcagaagtaataatggggatgtgtgaaggcagacatgcatgctaggattcgtagccattccagttaccgtacttattatcaaatataggaaacaaatttatgtagtgagtatgaatggagagtcaatatgagacggtgaaggacatgtatgcaagtgacttgaacgaaacaattttacaggtcaaagtaggtaggacacagtatcatacacctcaactatttaacgaatacttaaaacaatcaatgaaaccaatttgtacacctcaacatggtcaacagtaattgagacaatcaatgacacgaaagaaaattaatatttatccatcttacgtatcccatcaaattgagcaatgaaatcctagcgtgagatagtaaccgtacttatgacacacaaatggagagtcaatatgacacagtgaaggacataaatgcaagtgatttgaacgaaacaattttagaggtcaaagtaggtaggacatagtatcatacacatcaactatttcacgaatatttaagacaatcaatgacaccattttgtacacctcatttagctcaacaatacttaaaacaatcaacgaaatggaagaaaattactattaattcattctaggcatcccatcaaattaagcatccaaatcctaccatcagatagtttatattcaaccaaatcaaatcataaaaaaccaaatcctatttataacttagcagagaaaatcgacttttgcagtcgcaggagttggttggaccaaaaattgccaccaccatcttataccagaaatcatcacaactttccagaagtgagacatataaaaccacaacaacagatctttgtcaacaaatgatcagattatactatggtattcacaacgactattggtaaagcaaatactataaattcgacatttttggacaccacatttggaagctttgtcaaaacccaattcattgagatcaagattatgctgagaaaagaaaaatacccaaatcccattgaacaaaagccctcatttattatgaaaagcatatcaaaagttgggtactgattaaacattcaactcttaaatcttcaaaaattcaacacaaatttggaatatagttcgccattggttcattcaaccctaaagtctcaattaatccaaaatttcccaagcaggttattgaacgaccacaactataatcatttcccaaaagcgcttcaaacaaagatatgtaaaggggaaaaatgttcattctatcttctaccaaagagcaagcatgaaattacagccattttatattcaaatcagccaaataaatccatacatactctacccaatacattcaaacaatgaaatcccaactatacttaaacaaactacactaatatagaaagaacccttgtgtctaataatatgaaaaatctcgaagtagaactaatttcccaagttcaatggatatatcaaactgtcatatgccgttttgtgtatatatttcctcttcttcagaaaaaatgcataaaatgaatacaacaccaacctgaagaaattagtgatggtcttcgtccacggcgaagtgattgatggcggtcgttgatggctagtggttcgacgattcgaatgtcagaggggagtctcgcttttcaccggttcgtatcacgcaacggactgctctcggtcttcgtcggcggtgaaagaaaggaaagtgcgatggaggggatgattccaatgaaagaggagaatgtgtgagagaagggatgtgtgagaaaaaaattgcataaaattactacaacaccaacctgaagaaattagtgatggtcttcgtccaccgtgaagtgacctatggcggtcattgatggctggtggttcgacgattcgaatatcagaggggattcttgcctttcgcaggttcgaatcacgcaacggagtgctctcggtcttcgtcggcggtgaaagaaggaaaagtacgatggaagagatgattccaatgaaagaggagaatgtatgagagaagggattgtgtttcaacactggtttcttcttctcctccgtcgtttcgtttggtcgtttcaccttcttccttcaccagttttgttctctcttttttttttcctctccaagtacctgacatttcaaagattttgtacaatttcaagtgttgtcatgtcatatttaaacaaggaatcagatggtattgaacttagtaagaggggcaaaatagtccaaatatgacaattttgcaattactttaaaaaagtgacatttctgtaagtgacaaggcaaaatttgactagtttgataatttccacttttattaattataaaaatacttatatatgttaggaatatatattgtgctaaaattgttaaacacgggagctactgagataaaatgccaaaatagattctagggacataaccatattatccataaaagataggggtagcattgacataaaaaggactttatcatttattgacccttctctctctctcatggtggcatcgtcggtgggtaaccaacctctctctctctctctctctctctctctctctctctctcagtgtttgttattggcattaaaaatgagaaaaaatagatacttgcataacacgaagaagataagcgaaacagcagacaaaaaaagcagccatggaacaagagcttcatttttcctactggcaaactgcttggctccaaacagtaaattcggggaagccagcacggacggctcgctgggtgccattatcgatgacaaatgtgctgtatttacactcaaattctcactgaacatttattaccaactctacccaaaaaaaaaaaaaaaaaccgatatggctccttgcccgtgaatcaacctccctactttctgctccatttgtacagcaaacatgcaatttatacgattctttgtatcttctccgtttccatcaaaagcttttgtgcccttacaaaagaaaatagtgttgaaaaaaaaaatgtgtaaatggctcattattgcacaatttttagtgggatccgttggtccaatttggaagatcaaaattgattcgtgttcttctccgtgagaatatcgaaatcatatacttacttgccaaaaatgaagcttggatgaatgagaaattggagctcaaaattgaccaatggaagatggcttatgtgagaaaattggatttgtcccacgtaggaaaataaagaaaatatgaaccactttatatatggctacacgttgaaatggtgtaatcatgtgtagcatagaggctctctcaacgtgcacgcagaggatgcaaatcacggatcgaaatagcctttcgaccttgaacttgtgtgcgggcacatcctgcatatacaaagtcaaaccgaatagagcaaaaattggcctgtttggagtgtccacatttttcaatttttttgctttctccaaccgacttttgagtttttgaaactgctaaaactccaatggttactgcagatactaaagcaactccaatgtttattgccatagagttaatggacagatttaagttatattaaatctcatttttccagcaattttacacacgcgaaaatatacagaggaaaaattgtgtctgcatattattgttctctacatctacctgcatatataatctcgagttttgtcagcgtcgtcttggtggtgatattgtttggatactaattagtttgtcggagtagtatctgtggtgctcagatcctactgattttactattgtatcttgggaaatagacactcagattaaatctcaagcacttacggtgatgagacgaatatgttttaaggaaactttgctcgcacaggcctttggttgaaagtccatccattatttatttaattcatgcaattttatctatttctacaatttattcgagtgctttatataatttgcaattttattatttttttcgttctatttatgttttaattaaaattagataaacgaaagaaaatggaatacagtttttccaaaatttttcagaatgctgcatatacgatatatgtaagacagtatatgaaaatacggtaaattgttgcatatacggtattctgtgcaaatacggtaaactgttgcaaatacgttatgctcctgcaaatatagtatgctgttacaaatacgataagctttaaatacggtaatttttatatactgtgtgcatataagggatcaatgaatccggtttcatccactacactaacactaaattctaacaaatagaagcatgggggtcacattttatactccactttcgagagttcatctcacttcataaattggggaaaacacgaaggaagctagtctctctcgagagaacactagaaatgatagtgcaagaagcgaggctgaaaaagagtagaacaagatgagagggaagcagaggagatccatcaccaccagtgccggccttgactataggtggggtaggcgatcgccaaaagccctactttggtgagggccccaaaaaaattattatattttattttacatgtgtgtgtgtgtgtctatatatatatatatatatatatatatatatatataggatcccatatttgaaattggtctaaagccccaaaaatttcaaggtcggctttgatcaccaccaagatcttccaaggcctccgcaggcacagtggctaccacctgtctcctcgtgctgataacaaccaagttctctgtcatcttgcccaaaaagctggatgggtcgtcgagcctgatggcatcacttaccgctctgccaccaccactactacaaccagcagcgtatgtattttttcatgtcatccttactatgtccttcacgacattggggtcaagttactccactatttagaatccgttatcgttgatgctaagtgctataactttgtgaatagcgaggcagcatttaattattataaaagttaagttgttactgattatactttcatttttataatcttagtcacctatgtaattaactcataaaagattaataacattaattaatttgtgtaaaattatttttataacaagatagattcttttgttgcattaaactggagatttttatgtatgtatttatttatttagtcagtgcccttgtttacactcttattcccttcagctattaaaataatctttttagtttttaccctacagttaccaaatattaaaatttttaacatattatatccacaaaattaacataacattgcaataataaaagcatctgagttcatactctgccacatcttttatcttgcaatggtttaattatgtaattgccacacgtatttggctaagttaactcacaattgttggtcacacacagaataaaattgttaataatttttttacattttttctcacatgctcttttgtgttgcaatgtgcaaaacatgtatgtactaaagttgatctggttttgacagggaattaatgtttgtcctcttcgtgctcgaggaagaaaacggactacgataatgccaaccagcagcttcgtgggagccaatgctggaattggtgctgtcgccaatggtgatggaggtgaatgtctgacagtggcctcccctcgccacatcacaaccaaaggtcccaccgcactcaaccactcctccattagcctaaccttttgcggtggatttagctcatgtagtactactattgctacaattgctagttcttcttcttgtccattgcattcactactaaagaacaaagcttcaagcatggattttccgttcctaaaacctcaatatctgttgctaataatcttcaccaacggaatatttgcaatcacaaatccgttgataatttgagggtcactgatagttaccaatggatcatgccgtaggtaaagagtaaacattttaccaacggatattccgttggtaaagtgtgaatcttttaccaatggaattttcgttggtaaaagtcttaaccaatagcaaccgactttccgttggtaaatgtctaccattacaattggtaaaaatcaatgttgtaaataactgtatggtaaaaaaattatttatttatttatttatttatttatttattattattattattattatttatgtaataattattttttttaaaatttttagccaactgaattgaaagatcaaaatattgtttaactccttattggaccacaaatttataaagggcaactacaaagatattgttataaacttccgatgtgggataagtaaattatttttaccaacggataattcgtttctaattaccaacggaatatccattactgaaatatcaaaatgttagacggttatattaggcacggaatatccgttgataaagagatatcatttttactaacggataatccatttctaattaccaacggaatatccataggtaaaacatcaaaattttaaacgattataataggcacggaatatccattggtaaagagatatcatctttatcaacgaaaaattcgttgctttattgtagctaaaagtgaattacttttaccaacggataattcgtttctaattaccaacggatgcaatccgttggtaatattcggtacatcacctatggaatatccattggaggaagatccaaatgttaaacggttacattagacatggaatatcggttggtaaagagatatcatctttaccaaaggaaaatctattgctaattatcgtagctaaaagtgaattacttttaccaaacaaataatccgtttctaatcaccaacggatgtaatccgtcgataatttttcgtaggtgaaaagttgtttttaagtagtgattgtaccgatgtagttatggctgtttatgttagtttgatgctcttattgagtagtacttggtaaaacaacatcatgaattgatgttccattttgggtgttacaatttgaaatgactatctaaggtttcatgatcatataggatgtcacaaattgtatactcgatagttcgttattgagacacaattcgtgatgtgatcaaaatatgtcgttcacaatcagtacataagttggacgctatatgttgggaagatatcattgttcttattaaaatttgtctagatttggggataagaccaatgatgtgctttttgattcacattgaacgagaccacgtagatgactcatttgtgatcgttcggaatgggctactcgattatcaaactagtcacctaaatcctgagcaactagttaattgttagttcaagttctttgaggtactaatgagtaaagtcttatttagaatattaatcttgatgcattgagaatcgagctgatacaattagagatcatatacttgtgatagtggaatccattaatcatcgagatcagatgatcgtcactctgaggtattttctataagcaattgaccctgagctcaatagtctgatgatgagattgttggactctatattgtgatttgataacaacaaattcgccttatgaaaatggaacttagagagtaatacatgttgaagggcaaaacggttcttttgtcattttcaacatgttgacgatcaaatggaggttgacttgtggaatgataatcgaaggatattattatcagatcataatttgcttttgtaacttttacttgactcgagaatgcaatctccatttttttttgtagaataagctgggataaatagatgtatctaaattggtcaagagttgacccaattagaaacatctattggagcttgagtcctatgagtccaactaggtccctctcttggctccaataaaggggtgtgacttaattggtctactacaataaagtccaaaattttttgcgtaattataaaccctaattgagtattataaatgtgccctttataggcacattttcaaatgttttttagggttagccacgcttttatttttcaaaaatggaggtacctaaggagcacaagggagaagatctaaagaatgaagtacttggttaggccagtaatagctccttcaaggttatcatctctactttatgtataaggcttaaaaacatccaatgatctcaaagtaatctaagatcctttattcatttgggtttaatcttcaaaggaaaattaatttcctattatgatgatgaaatccaacaaccaacaaatggtatcagaacaaaggttattgagagccttgagtaggattaagttctttaaatcctagtacaaaatacatttttagtatgagtggtgtaaggttatctgatttaacatgtttattgctttataagctaaaagtagatgtttatacataatcacttttggccctaaattttttgttgctttccattataattctttttattcgttgttctttactctacaaaaattataagccataaggcactaaggttttgtacatatttttcatatttctacacttgtgtattaagagaagctgatgggttttttcagggcttcatacatttttttgttgctggttgttttatggagactcgaatttttagaaataaaaaaatggcacgaagatcttattggagaaatggaaggaggtagagatagaacaaacaagatgcaaaaccattgtagaattgcaacaggcggcatagcaaccactgttactggagtggcgacagttgctgtgactagcagcaactgctgctgtttccagtcgcgatagccatagctactaaaaatgtagtagctgccattgctaccacgaaatagcagcatctgcggctgcaacaaccatgcaacggctacgactgcttgctacagcagcttgcagctactacaataagcgatcgtagtcgtttgctatcgtcactcagcgacgatggcggtggcgacctcttttgttgtcatcattgtcgatgtcctcgtcggaaatgggtggtagaagtgatacatgatggatttgctagagtttgtgaaattaggttaattttgagtttttgggctttctttgagacttggccaatcttgttggataaaggcatttgttttaaggattgagactcataaattaaattgacccaatttcagaaaattgcatgggttggacaacaaggaaattgaagaattgggtcggaatgtggcccaatagaatgctttaatctttgttgtaatttaaatttttaggacgggccctaagtgattataattcatttaattattgctttttatcgctttatagattatgaataaatgtatgattatcatatgtcgtgtaaattaaatgaaacaccatccagtgcactaaaatcatatgcattggtattggatttttttttttttatctatctaattaattagggtggttaaaacattatatttaataatttagtgccattataattgtttaccaaaatggttgacttctcgtcttgattatcacaaacaaacggtgtttatttctaacaaattaatttcgagtgttgatagtgattattgcaaaatcgataaaaatgtaaaccaaaaaaaaaatcaaaatcaagtaacgtgcacattgacaaatgaaattggtgcttgaagatcaacatggaacaaaaattggcgattgtcgaaggtagagacagaaatcgagccttcacgtcgaaaatcaccttggagaaaaaatcgatttatcaaaattcaagacattagatgtagatgcattgaatttatatacaaaggtaaattaattcaattcttagtatcaattatacatatgaacaaattcacgttacaaaagagattttcattaaaattaattttaaaggtaagtatttcgactcaacgatcaaatatttacaaaaacacttatctttacaaaaaaaatgagaaagtccttcaagaaccgacattgatcaaattcatcaagaaggaaaaatgtccgagggcatttctacccattctaacgttcggataccaatagtcacttttttgatcgttctgcctttgactcaagctgttagttttttaaccgtttggaccctaaccagatgtccagatcacacgtccgaatggacagattttttgctcattgagtgctataaataccacttctcttccgcatttgcaataaccttctttgagcatttaagtgacgttttggttgatctcaactgctttgttttcaatccttagaagatcaaaatatttatttcttgaaaaactttttgaatgatcaactttgtgaaaatcttttatcacattaaagtttttcaacaactaatacttgtgctatattcattgctatttattgaagtatttttcgtgtctctctcttaatacttaattgatcatatcatttattatgagagaaccttttacttgtaatttttctattgtttgattctaggtcgtgttgaaatcccgaaaatttgaacattgtaaaaggattggtgctccttggttgtaagtctccggaagcgttgtaaaagttggattgcaccataagtcaacaacaatattgaaaaaggccttgctcgtaacggagagcttggtaacagaggacgtggatcattgattggatcgaaccttctaattacatcgtttgtgcattctcttctcttttactttttacttacatatttgtgctattttacctgtgcaattaacttatttgttatttgtctaagattgcgattatttttgagaatgttttaaataaccagttcacctctttttgattagctattcttgggctttcaattggtatcagagcaaagtgctcattttttatctttttcttaaagattttacaatcttgagcaatggctaatcactttcttcaaactcttgtgggacatcccacaaactgactacctttcatcgatggaacacgttataattattggaaggctagaatgatgtttacattcaatccatagattacaacatttgaaaagtaattgaatatggtccatataaacctactaagaccattaagacagatggccaacccgaccaaattattcctaaacctagggaaagaatatgatgaagaagataagaaaaagttacccttgaatgctagagctaaaaatttactttattgtgcattagataaaagtgaatttaatcggactagcacgtgtgaatccacatatgatatttggcatgcacttgaaattactcatgttggcactagaaaagttaaataaataaaaatcaacttgttagttaaagaattttaaaatttcttatgaaacaagaacccattgtttatacgattactcgtttcaccaatattgtaaatggccttaagatgttgatcgtaaatttactaacgatgaacttgttagcaaaatgtttaggttaatatcagaagaatagagtccattgagaatgttaatagagaataccaagtatattaatacgtatcctttggaagaactctatggaagattaatgacctatgagctcaacaatgtcgaggtcaagaagaaaacaagaaaaagcaaagaagaagtaaaggggcctcctaagcgtcgaattgccttaaaaatcgacaataaaagaaggaactacaagtgacaacatgagcaatgaagagcttggggatttagtccttctcgtcaaaaaatggagagatcttcgtaataatcaaagatttcaaaagaaggaggaaaatggcgaagaaagaagtaagaaaatcatttgctatgattgtgacaagtctggtcacaaaaaaatcgaatgcccgaacaaaaagaagaatgccaacaaaaaggcactccaagccacgtaggacaatagtgatgatgaagaccaaaatgaaaacaatagccaagatgaaattgccaacatgtgcttcatggcaatcgtaaatgagataaattctaacgaaaaatgttcttacgatgagttatctagttcatatgatgaaatgcttgaagaattcaaaaaatttgccttaagtcattctatcattaaaaagaaaaagtctatatcgaatgataaaataaaaattctatatcgaatgataaaataaaataaaaattgtggaaaaacaaaaagaaaacattgattacgatttattagttaaggaaaacactttcctagaagaaaaaaatcgaggatttaacgaaaatcatttataaattcactaaagggaagaaaagttttgatttaatgcttgaaaatcaaaattgtgtttttgacaaatgggaaatttgatacaaacccttttcgaaacaaaagtctctcaaaaacatctttgtcaaagcttcaaatttaaacattacatgtagtttttgtaataaaagtctctaactcaaaaagtgaatgcttgagcttgagaaatgtatttcatcaatctaagtggaataaacaaactggattccgacttcactccagtcactagccctgccttcggcatccccctccttgcggttaaggtaacgacttcgggcatggccaatgataaaatcttttattttttgatcttcttgtaaacccttagacgaccttttgatttttgattttttttcgttgaagagttcacatcgacgggaaggtttggcacctcgatgtcgggtttttccttatttaattaacataacaaggaaattatctactccattcgactagttccgggttcgaatcccggtcgatagatttcttgaaataaacgaaaaggtaacgaaagatgaaacattcaagcagttccactttctcggcccgagaaatgcattgttggaactgggttggaacggattcctatttgaagaatgcataaccgcatggataagctcacactaacctttctagtgattcacatggtatcatcaaatgatacaagtctacatgttgctttcaattgcttaactaaaaagaagctacatattgaaagctaacataagtgaattcgagagtccacaaaaactaactaccaagggcccaagtttgtgtgggtatcaaaaataaaaaattaaattgttcatgtaggtaccaaagaaaaaaagaggtaaatggttcttggatcgaggatgctcaaaacatatgactggagatcgatcgttatcaaacttcaaaaagaaggatggaggtcatgtaaccttcgtagacaacactaaaggaaaaattatcaacattggaaacattggtaattactcatctccctgtattgaaaatattttattagtagataacctcaagcataattttctaagtattagtaaattatgtgataaaggttacaatataaaattcaattcttccaaatgcctcattaaggaagctacatcgaacgaggtgactttcataagaagccaaagtaaagatgttttatatcataaatattgaatttgaaaataatgaaaattgtttacttagcttgaaagatgaatcatggctatggcatatgagataagttcatattagcatgtatcttttttcaaaaatttccaaaatttcttttgtgaaagcattggaaacattggtaattactcatctccctgtattgaaaatattttattagtagataacctcaagcataattttctaagtattagtaaattatgtgataaaggttacaatataaaattcaattcttccaaatgcctcattaaggaagctacatcgaacgaggtgactttcataagaagccaaagtaaagatgttttatatcataaatattgaatttgaaaataatgaaaattgtttacttagcttgaaagatgaatcatggctatggcatatgagataagttcatattagcatgtatcttctttcaaaaatttccaaaatttcttttgtgaaaggattgctgaatttgaaattcgagaaagataaaatttgtaatgcatgccgatttggaaaacaagtaaaaaatatcttcaagcctaaactttattcttaaactacaaaaccattacaacttcttcacatggatctttttggaccatctagaacggctggcttaggtggtaaacattacatatctgttattgtcgacgatttttcaagattcacttggattatgtttttaagcttaaatgatgaggccttaaaggtttgtaagcactttagtaagaaagtcgaaaacgaaaagtgttataccattacgactattagaagtgaccatggtggagaatttgataatattggttttgatgatttttacaacgaaaatggatttgaacataatttctcggctcctagaactcctcaataaaatggtatagtggaaaggaagaatcgtatattgcaagaaatggctaagaccatactaaatgaaaataacttaccaaagtatttttaagctgatgccgtcaacactatttgttacattgtcaatagagttttagtaagttgaaagaaaactaaaactcttactaaaactctttacgagctttagaaaaatagaattcccaatatcagttatttcaaagttttcggatgctaatgctttattttaaacacaaaaaaataattttggaaaattcgattcaaaatccgatgttggaattttcctaggatattcatcgactagtaaagcttatagagtatttaaaaaataaactctagccgttgaagaatccatgcatgttacatttgatgatcttaactctcttgatcgcaagaaagatattgatgacaatataggtttgtaagctctattcgaacaaatgaatattcaagaccaaaacaaggaagctcccaacaaagaacagaaggtggagcccaatgttcaaaaaagtaaagagaaatcaaccgaggcacaaaaggatcccccactaccgaaagaatggaagtttgttctatctcaccccaaagagctaataaaaggcgatccatccaaagatgcaattactagaacctcatttaaaaatcatctcgtgtcacaccccaaatatatagataaccatacattaccctgtgtagaaatgatattgatgatttaacctagacacaggatctcacacatctttttaaagataaaatgaaataagcatcttcacaataaagtccctgtatattctcacatggtcacctatgatgtacatatggtatgttatgaccaaatactgtataatcaaattccaacatatttattttaagaattccaaaaagtatctaccatgccatttcaaaagtcttatgtactgtacaggattctccaaatataatacaatagattataagaccaaaacaatagcccacaagataaccctacaggtcattattctgtatatcgaactatagaatccgtaagagtttcgcgactagccttgacctctatgaagtccatgttcacctaaaatccaagaactacataaactaatgcttagtaagcaaaaatcatgcatgtcatgagtatgagtaataataatatatgaaactatgcaatttactttagacattatgctaataatacatcatattcaaatattcatcaaagtcaactcaaaataacttcatttgaaatctgtcattggtccattgacccacatactatgcactaaatagagttctgtacaatatcaatataaatatttataatcaataatcaaatggccaatatgaaatcgacatcggcgagtggaccaccctcttgtaaccattagaggcccatcccctaattgcccctatgatcaaacaagaagtgtcccacctgacagtgccaataattataatatcacaagggtacaatcaagtggtccactctcccgtgatcaccaaaagcccatcttctatctacctctgcaatcacctataaagtatcacccacgatgccaaaatatattacacaagcatgcctcggtgcactagtagtgatcaacaaaacatttacgagataaaaactcaattttgaaatcatgtagtgcttgctagattttcaaccatggacatatgtcgtgcatgcttatgaaaatgcttgtgaatgatatgcttaatcaataacgacgtcagcatgttttgaaatcacatactcaataattacacccatcatatgatatagaattagcttgttatcaaagctatgtaaatgtcccaacattattatctcacaaatactatgttcctgcatcgtagttgcgaatgaatttttacttaccttcttgcctttgtgtgttatctttctatggagtgtagaccaattccttttttcatctaaattcaaaaaaccacctatattacaatttaatattaaacaaaatttaccaatggcattacaaactagccccataaatctggttatttctccagtccaattatgaacgtcaacattatccacttgttgtcaacaacctagcatcttagaatctaatttctaggcccaagagataattaatggacacgtaaagtttgaaactacattaaacatgcaaatggacagaatctatttccaggttccatcactgtccaattattttttcaatcatttttcacgcccttaactatatccaacgactccaaattttttaccacactttcataacatgtatgtgaaggtaattatgtcataaagttgtgacaaatgaagggtttgtggcttcaaaacagtccctttttcactacaccaaatcaagtagtttcccagtaacgattttcggtttccattgtattagtatgccaccaataagactccaggccattaaaaaacatttctatacttattgattgcatataaaaacattcctatgatgtaacaataatgcccataaggatgaaggataaataataggtttttaatgattcttatgcgtcaaagactgaggaaactaatgcgggttacttataataagaaataacctatgtgagagagaagtgaggctccttgtaagtaaattgtgtgtggcttaattcttagaattctcacagaatcagggaaatcttcatggccaaaatgaactatgagaactgaatcatattaggaagaagcctgggtagattgtgtcatcgtttacacaaatggtagaataatccaaggatatcatgtccactaatcagctagtaaactaaatatacttaaacaaggaaaggttcaaagggcaacacctccctattctatgtaggcttcaaccactatagtttatcatcatgtctatctgtcattgttgttaatttcattcatgtgggaaattgttggaaagtaatatattaaaccaatatattcaagttgaatgaaattgtaacaacaatcataggtttcaattatagtcaattccatagttaatttgcatttgaattagttcaattccataatcaattggtggttacaaattcattcttggctactgtaacattatttgtgttaaatacaaaattaactaagattttgaaacatccttcatcttagcattttataaataggtgatctcattcttattctacacattaaaaatttgggagttctttcttcacatttgctctcgtctctttgtttcaagagtttagcttttagtaacttagtttatttttttgttgtaacttggtgatataattgtgagcattcttagttcacctaaagtagtgatgaggtactagtcagctactttcaatcgttgtataatggaagacatatgccatcaattctcttgcatcacagtggggggcgaatctattttaaagaaaccatgtataacacagtactcggctcctttcaatattgctactgcttcaacaactattttctctaattttattgttactctatttattgtaatgcttcattccatgactttatttatataattccagaagtatttctaattgtctttttgtatttttactaacatcttttacccagtaatttctcgattatatgaaatgccaaaattacataattcttggttgacttagactaagtgtaaattttgtatgaaattcttttactcataattaatattttatttataagtaatttttaatttaaaaattaaaatatttatttataattaaaattttaaattatgagtaattttttatttataagtaaattttacaaatacaaattaattttataattttaaataatttttatagatgaatatttttttacaataagtaatattacatattttataagtgatttttatcttattaataatgtttttaatttataagcaactgcttacacaaaagtgattttctattttataaaaattagcttttaaaacaacatgttacaatccagtaaatatactcaaataaaatgactccgcttttttgtttgtccggtctcatttcgcatcataatgcaagtcctaagtaaaatatttatttataattaaaattttaaattatgagtaatttttttatatttataagtaaattttacaattacaaattaattttgtacttttaaacaattttttatacataaatgattttttacaataagtcctaatctctttcaattgccgcttttcttcttcgttctcttcatcttctggatgattcttgtgtgtgatttctgagtgaaatcttgtagtagtgtaataaaagtgatgagatacatctcttagtgagattagtgtatgatttctgagggctttctgtgactaaaaacggcagaacattttcatcctttgtaacttgattttacccgattttggggactgtgatagtggattcgagcttaatccatatggatgctcaacgaggatgtaggcgttagatggtcgctgaacctcggggccttttggctgaaaaattcctttgtatttctttactttcttttcatttatattttgtgattttactgtaaaataatcgagtcagaaaaattcgtattactgggaactacaagcaaaacggtcacttcaaaatcagctaaaacatattgtaaacttttaacgaaccatattattataccaagcaatcgataataacacatttgatcaaggggatatgtcagtcaaccaaaacaaaaacatatctttcattggagaatttttacttggtccttatttttaagaaggaaatgaataaagcaggcccctttcatgttgttctcatactggtctcctccatcaaggcactctacttaaatggtctaccttagtggtatattttgtgttggaaaaataatcagttgcagaatagtaaaatgcaaaagtaaaacttatcgtccgattgaatctcatgacagcacgatgtcctaaagtgaaattgcccgtcgattattgctgcgacctttgtggacaatcactcctatgatataacaatcataaacaacttgtgcagtaattccgaatggttttcagaaccctcaagtgtattccaaaatatatgtaaaaatccaaaaaaaaaaaaaaaaatttaagaatatgataaataagatttcgtttcaaatgattttctgtttcctttcatgtgtatttttcccaaaacgagaggtgagtatatataggcaaactgggtttaaatatctcctccatgactagagaattatgcaatattttaatgattttgtgagtagtggatcgttacaaaaggtcacaaaatactgactagtttgacccattaaataattaagaaaataaataattttagtcaaggaaacccaagagcctgctccagaccccaataaaaaactttttaataattgcatgagagtgacccaaacccccgacgtcccacacaaatgccacatttcccaacacttgaacactttatctaaactgattatttctttcacattttatatttatggtataaatatataacaatatgcaagccgtaaatcaatactacgaaaggctaattttgttgtactgctttgagaactttaataccttagaatattcaattaaacctgtgatgatggcgtgcgattgctcaggcagaataaactcaactggaatccaatcaatgagctttcaactttttcatcagttctaacttcaagtaaagtgggattatctaaagagaaatcttgataaaaaccctcttccaatctggtcttcttgtcatctcgagagattttagaaagttgaatcatttaccaaataatttctcgattatttgaattgtcaaagttacataattcttggtcgacttagacttagcgtcaattttgtatgaaattcttttactgataaataatattttatttataactaatttttaatttaaaaattaaattacttatttataataaaaaaatttaattatgagtaattttttttatttataagtaaatattaaaattacaaattaattttgtacttttaaacaattttttatacataaatgattttttacaataagtaatattatatatgttataagtgatttttttatcttattaatagtatttttaatttataagcaactgattacgtacacaaaagtgattttatattttataaataaatttcttagttataaaaattagctttataaaacaacatgttacaatccagtaaatataagcaaataaaatgactctgctttttcgtttgtccgatctcgtttcgcatcctaatgcacgtcctaagaaaactgaaacttgctcgacagttttcaagtagccaaattttgatatacaaaagaacaaaaataaaataaaataaaatttacttactaaatgaataaaataatatatattttaaaccataaggaaagaggcaaaaataagaacttttcatgcaggtatctattaatcttaatcgtttcgaattgcaaactcaagtacgcacatttgtataaatttccatgtatacataaacacaattcatgtatgcacaaatataagcacattaaatgtatacataaacacaattcatgtatgcacaaatataagcacatttttaacatgggaagaagaaaatgcatgacactaagcatttcaatgaaagcaacaaagttttcctaacatttcacatccaaattcagtgctttagtgtggacgagtgcacgtggatgaaataacatcaaccagggcataacatcaaccaatattcctataattacaaaatagcccacaagaatatgtatgaaataattctcatccttaatttgacttagacttgaccaaatgattattgaatttgaccgaatgattattgactttgactaattaaaagtggattgtaactgcaatggtcaataggcttaataaattatgacgttataagctgtaatcagactcacacagtgtttcttgtttggttgttacaagttgcttttaagacgttatcaatgtaatgtcaaatcaaatacttgaatgtatgcacatatttatatctattgaaaaatgaccgttgtaataaagaacttataatatattatataacaaacaaaaagaggataaataaattgtcataactaaatatctttttttttaatcatttatattatgtatatagatttaatatatatttgacattttaatactagttggaaatttggaacgcatgctgtgagctgcccgagcaatgattggaagcaatcacaaatcataaaattttggtttttactaatttttgtcgagtagttaaaccttaatttcgaaatttgaggttttaaaacggcttgtgaatttgttggatttttaatcttaaacaataaactgggaagaataaaaaacccagtgagccaactacctgaatacataattaattaatgttaatgagacggaaaatcagcttcagttttggactgcaaaacatatgaaaaaatattttatatctgcaacttgagtaaagcatgacatggcttgtcgttctgtcaattgcccacctgcaaaattaaattcaataactggaaaccgaaaccaacaacggaatgggcctttcccactgtagataacagttggactgttttcgaccgagggatatattgaatattttattcgtattgaatcgttcttaataatttaaaactcttctgagaattttatttttgttaggcttagattgtgagcagttaattattcacggtgagcgaataaacatgattgtttgtttttctttcctttattgttgtcttgaataagaatagaattttattcacgacgagaatgaattagtattgctcaagttttttatttgagactaacagtaatcacgggtgttgcaaatcttatgtaccgaatgaatgatatgagtaatatttttaaagttaggtaattgataatgttaaagaaaaagttaaaattgttatatatatgtatatgaattagagttttatgaaatttacgtacaaaatgtttctttttgccatgtggcacaccctgcacagtgaaacaaacttctccactttgtggcgcatagtaggccatatgaatcactaaccagagtcaaagtgcgatctcacccaacatgaccctcgccgtgaaactcctcaatcaatttcagacgaagactgcaatctggtatacacaactgaacacctcgaaatacataaccatcctctaatagaaagggggaatgggatccctacagtaaactgtggaaaatggggccaaaataaggatcatcagcataaagagaggcaaaggtgtcaaacccgataaccaccacctgtagatgtgctaataacccatgccaccgactgagtgtgtctgccacacgattagaagaaccggcctgatgcttaatgacaaagttgaatttttgtaagaaggcaagcatgatgcatgacgggcagacacagactcttgactggacaaatgtttgaggacttcatgatcaatgtataagataaattctcgctcaaatagataatatcgccaatggcaaattgcctaaacaatggcataaagttctacatcataagtgttatacctcccacgagcccctgctaatttctgactgaaataagctactgattttccttcctgactaaggataggtccgatgcccagtttggaggcatcgcaatgtaatgcgaaaggctttgtgaaatcaggcaacgcaagtatcgaggctgaagtcaagcgttccttaatggtcacaaacgccttctctgcctcgagagtccattgaaacttactctccttcatgcaatcagtaatgggagatatgatgctactaaagtgctgaataaatcgtcgataaaacgacaccaagccatggaaactccgcacatcagaaactaattgtggccgcggccactgccagttcgcattaaccttagctgaatccactgtcaccccattggctaacacaacataccccaaaaacaaaaaaaactattggtatggaatacacacttttttgggacacgctagagctgctccaaaggataagaaccttagtacacggtccaaagtctgtgttgtcgattttatatccaacaaatgtacaaatcgtaacaagcaatacagtgaacataagagtccggatatcatttctacgagtactactatttaacaattggttcaattattcctaattttaatttgatagaaaacaaacaaaggattaaatgttgtaaattttaatataactatttgaaaatatgttgatgcatacaaagattgatttataatttaaataacgcatggatattagagcagaacattttcacatattgattgactttaagtctcaattcaagattcaaaagtctaatgtagtatttggtcgaatttttttattgtatttaaattttccccctcgagctctcattgaacttatttaactaattcaatcacatatctctatgtgaatcaattttagttaagtgaaatattagttttaagaattcatttataaatgcaataatcaatatatgtatctctatatgttataccaatttatcgaattttaatatatggtctagatctaaaactgacctctcgattcgtaatagattcacgaagtcattgaataattggccaaagaattagaagcattaagtacaaattaaaatcaaatcatatgcatttaaagaacttgaatcttgaataaaagaaactaagggtctcaaaagattgcactgtttgccctaacatgaatttagttactcatgatgatggaagaaaaactagtgaattgcattgagtacatcaatgagttttggactgagatgtagaaaagatgatgaatcttgtataagttcctattctcgttccaaatcttgatttcaaagccatgaattgttatttttctgctcttgaatttgctttataattctcaaattctattctctatctcttaatgtgtggaatttccttcaaaattgtggaaaacttaaatttatagttgcttcatattttgtgtcgaaattaggatttctatggacttctaaatggcctaaaaacacgcctcagacacatccaggtagtgcctcggtgccatagaagtggcgtcgccgaggcgctgtgactctaatttggtggcccctcgacgccatgacggtggcgaaagggtgctacctttcaggtaaagaatcagactgcatttcctttagtatttctatcattattttttctcttgatattcgattgagactattcaagtagggttgtaaagataattcaaagggctacaactttgtttgaaatagcctttttccaattcgaatgtttactaagtcaaaaatgagtttcaatcttaagcatcttggtgtaattgaaaattgatttgggaaaatattttggtcttatttcattccttttgacttctaattgaatctaattgaccctcagcatttctagaatcttcatcgtgaggttcaacacaatttttgagtatttacaatttagtctccaaactttggatcttgctcccccctcttttgccaatttttgcttctttctttcaattccgcttccattcatcgagtttcgcaaaataaacaattatataataaattaggttataatttcattaaataaccactaaatgtctatattttagagttcgaataagtgtataaaatacacttaattaagtgttattttttactctcatttttctcaaaattcatttttttttcaaaacttagggttcgtttgattgcaaagatagaattgaattgaattaaaagcgaatttcaagaaattgaattgtctaaaaattattttcctgagaattataaattattgtgttcgattggtataatattccacgtgaaaaatgttgaaataaaagtattttttgatattcatttgactttattttacatgataattgtcaattaaagagatagaatttattggtattgggtatgaaatttgtttccattgtcaaaaaacaaataataataaataagaaaatcatctattttttgttgttcgtttgactttgttttgcatggaaattatcaattaaagggaaatatttttttacgataattcttagaatttatttccattgcaaaaaaaaaaaaaaaaaaaattaaaaaaaatgttacagtaaccgagaattccaattctcaccaaaatggaattcaatgatttgatggaaatgatgatgtgaccaagaaaggtggaattcattttccatggaaaattccacctagcaaacaatagaaaagttgaaaaatagtattgatttttcatttttcatggaaaaagcgtgtgctatcaaacacacccttatttcctatcacattctcccataaaaaaaaaattgtaaacatagatccaacacttttcactcatttttaccatagatcctctaaaaaaaaatcactattccaaaatacatttctcaaaaaagggtctcaaacgggggctaaatgcttaatttatgataaataagttttttcactcacaaagttaaaaagtgaccgacgatacgctgctaggcttgtccgatttccttactaactcttggtatagcaacaaaatagatcgagtttattatttaatccttccaattctatccagtattctgcatgaatttaaaagctccaaatgtcaatcctagtacaattgactaacggaatcccaaacaattcaccatcctttcaaatgggtgcccatagcattattcctataattaagaataaaaattaacttagttaccaacttcaaaatgcaattaagttcacttaaaccatgaaacgccctttagataagttatttcaacaccgaaacctcaaacattctgcagtttggtttccatatataaaaataaaaacagtaaattgacaaatatagcaccactatccctggatcattggacatttggcaccaatttctgtatattgacattgtcaccgaaatgaataaaaaataaataaataaataaataacactttcagggtaaagtttcatagtagtaccagtgtgagaattttacacgaaagtagcaagtgtttggtaccatattcacaccagaaaattaaatattgacgctctaatttacaaatctatttcatattacttccacttcaataccaatcttccaaaataattttttttcttctttttagcaatattcttgtttaatacctcaattacacgtcaataatctttagttcttgctaagttttgattttaaacaaattcaacataccataaccctaaaaaataattcaacattcttatccttacctctctaaattaaagcaaaaattgaagaatcgaagatcgagttagtgtatattcttcattacctgattatttttcggaccaaaacattcttttcgtttcctttttctctgcccaatttaagtgcgttggacaacaaaatagtagtgtagacgtattggtgtattaaaaaatttaaaatttcaatacctttcaaaaatgaacaatttaaaaccccattcaacctaattcctcaaattcaaactattctaacaagcaaaaaatagaaaggggaaagaataaaaataagaggattagaaaataggttacgtcttgttaagtgcttgatacttcaacaaatctctcattgaagttcgagacaggttttaaaggtcttgcattgcttgtaattaccgacttcgtaagtgtagcacgtgcttgcatgcttataacgaaaatctaaattgtaaaggctacttgaaatcctaaaacgaggttgaatcacttgccttttgtttacttgtcttctacactattttgtactcattcctaggtcgaaaattcgatcacgaaggaaagaacttgatagccacaatccaagaacccaatttgacatgatatacttctaaaatcaagccaccaccctcaagtacttttctcccttttgttaccatacaaattaggtatgcaatatttcatattctttgatgtgggagttgtatatgggagttttgagttgtgggaagttgaggttcaaactcaatcttctcaacttcctcaacttctccctccaacaacactctcatataattcgggtcgggtcagtccacatgggcgatctattttcttctaacatatctcatttgtacatgataggtttgatttgattataatacaatatcaattatatttatctcaatatttctaagttcatacaggtaaatggattgtgcaaccaatgagttaatttaagagtacacaacactatatacttgttagggatatatagcagttctagaagaggaaatatatttcttgatataccctaaacatattttgtaacatcgaattgagtatttctgaccctctcaatttattttggaacatactcaactttctcatttatatgtatacacaattgtgccataaaactcaaataattaacacaattatccagctggtgaatacaagctgaggtgctagataaaatagtcttcatttcctacttgaatcccttcatttcaagttagctgctttcttagacatgttccatcaaaccgaatcaactgtagttattggcaacatgctaaagtagcaacattgaaataaaatttcgagaaataatcaaaagtcacaggggtatataagtgagaccttatgtgcttcagatacttactcaatgaagaagtggggaccaattctttcatttctcatcggtcgttaaagcacacatggtatgaaacacatgatacgatgtttttttttttagagcgtatgtctaatcttacaaattaaatacatcgtacatatcacagttcagatatttcttgatatctaacctgagttctccttatatttattcctctatgcaatcccaattgagaactcgatctggctatagaacaggtcttacggacagcaaaaaattatccatacctattacttgttgtagtctcatcttgatatctcatcaaggtgactggatcatgtacacaatatggtcactatgtctcatctccacacacttcaaaacgtctaaggcgattgttcgtgtgagcgaaccaatctcaacctatgtgtgcatattaaatagtaatctaaaaatcataataaaaaattattcttaacatatgaactcaaaacattattcattcacagacttatatgaaaatgattacacatagtaaacaattgaaattctacgtaatctcagagatttaacatgagtcataaagatatctctagggataggttttgtaagtggatcatctaccatttgatgcatagagatatatgcaaactcacttccttcttttctatgatgtctcttacaaaattatattttgtagcgatgtgcgtttggttttgttgtgatatttgggatcctttgtatgtgcaatagctgcctaactatcatagcaaatcaatatagttcccaaattaccacaaaggactcttagatgctgcaagaacctctttaaccaaacagcttcatgtatcgctgaagcacatgctatgaattttgtttccattgtggataaagaaatgcatgtctgtttcttgatagcacagagagtaattagcaatatttttaggtatctccttttaacagctttccaatactctcttctaggatttcattgatacctgttgacctgacctatgacataacaaatgtctggataagtacacatcatagcgtacatcaagctcccaaccgcattgtagtatgaaactctagacattttttctttttcctcaagagttttaggaaacataagaaatcttagagtttcatcttttgatataggagtgtcaatgggattgcaattctccatttcgagaagttcaagaaaaaatatatagcaaaaagcctctttgaacgatctttgtagattttaacatttaatatgtaatctacttcacccatgtccatcatttcaaaatttaggaataatcatttcttaatgatttcaacatactccttatcatttccagctagtaagatattatctacgtagagagataaaattacaaatttctcattagaccttttcaaataaatatagtgattttcgtccatcatgacaaattcgtacgagataattgatttgtcaaatctaagtaccactgtctagaagactgctttaggccatagattgatctattcaatttacaaactttgttctcttgtcctgttttaatgaaacctattggttgttgcatgtagatttttcatccaattctctattaagaaatacagtcttcacgtccatttgaggtaattttgaaactaagcatgccacgatatctaagagtagcctaattgaagtaaatctcactactggtgaaaatgcctcttcataatctataccttctattgagtatgaccctttgccaccaagccagccttatacctttttatagacccatattccatggaagatcagccaaattccatatttgattcgatttcatagacttcatctcttcttccattgcattcttctacttttcttttgtagggcatgataaagcttcttgttctgattttggttcttcatcatcttttggaaatactaggaaaatttgcccttcaatcttcaaatgatgtttaggcatactttttcttgtactcttacgaagtaaaagctttgatgtgaccctgtcacttggagttcgagataaattactcccacttggaccgataggtggaagtacttcttcttgcacttcaattgattcatcaagtacaactctatatccaattcatataaaggttctctatttttcttttttccttactagaaaaatcattctcaagaaatgtcacatcacgcgactctatctcagttacagttctatcttgatttttacctataaacacatatcctttggactgatctgagccccgagcacctaattttccaaatttactcgagaaatcatggttataggcagctgatccctaggatataaaagaactcgaattagaggatatgcttgcccaaagctgatatggtgcagttgatccccaggatataaaagaactcgaattagaggatctgcttgtccaaagctgatatggtgcagtaggtactgatttagttggaactctattcaaaatataagtcactgttaacaaaacatctccccaataggaaatatgcaagttatcatgcgccatcatggatctcatcatttttagcaacattctattcatcttctcaacgacaccattttgttggggtgtattgagaatagttaaccatttaatgattcatttatcaatgcaaagttttttgaactctttggatagatattcatgtccacgatcagttcttaaggctttcacttttctatctatttgattttctaccccatttaaatataatctaaagcattttaatgcccttgacttatgagaaatcaaatagacataactacaccacatgaaatcgtctataaatgtaatgaaataagaggctctatgtcttgccttcacattcatcgagccacatatattttaatggactaactgcaatggaaattcagctcttatggctttaccaaatgaattttgtgttgtttttctaattagacaatgttcacaagtaagtaaagaaaccttagagattatacctagcaagcattctttggccaacctattcattctctttcacccaatatgtcctaatctagcatgccataagaattaacaacattcaaatctttagaagaagaagaagaagatatattcatagaaaaacaatgatcaacataataattataagtgtttggatcataatcgaacactacaaaaccactttctacatatccagatccataaaatacatttccattgtttatatgaatagaattaccacaaaaagttcaaattgaaacctaatcttaaaagaacaacaacgaaaattaagttctttcgtatccccatgcaaacaagatttcatgaaggagaatagtacgaccacagtgcaaatgtaacttccatgcactaatcccttttacctccactctatcatcgctgtcgatgtatatttattttataccagttggaaatcgacagatctttacaaacacttgtcgagccctggttacatggtctgtcgcttctgagtctacaatctacataggataagattcagttagcataacagtacttgaaacataaaatgtactaaaagaagtatttataagagctattttctttggcttagagcattcctgaagaaatcgacccagcacttgacaattgaagcatttcaacatgctcttatcttccttctttccaaaccatttatccttcttgttgcgcttgggtttttctttttaggaccatgtccatttttttttcactttccattcccgcctttgaaccagttctttttacacttaaagattgaaaatttcccagaactagattcagccacaacaacatgtcccagagatttagctgcactaaggcatttatcctctagttcgacctggcgggcagcatcagcaaaagttttgatactatcattgtgagttagattgacttttagatgttcccaattataaggaaaggaacgaatcaaagcctgaacttactgctcatcagagagtatgtgactagctgactttagctccctaatcatagtagacatggtcctcacatgctgtgtaatgttgttattaggaagtttcttataagtatcaaacttaattgtcaactgccttgtctagtcatactagtaccaccatgtttctctctcaaatatgtctagatgtcatgagctatcgggagttgctcacactcataaattagatgacaacaaaacttaccaaaattgcgagcagcggaatctttcttttccatgtttgataagtttcctaaacccttctctgttgagcagtttgacctaccccttggtcttccatcaagtggttaatgcccttaaggcaattctgtttctctagcacataccaaattttatgacgccaagtgttatagttatcgctattcaatttgtcacctctattaatgtcagctatgatattcttagatgcaatggtctatctaaattaattataaaattctcattttctgaattctattttctgatcaaaaaactatagcgtagaggtggctaattatctaaaacttcactagcaacatcatgctaatgtttaggaagcctcctcgtaagacgatacatactttccacctcacatataggttgtcccaaatgtagcacttctcgacgcattgcttcaagtattttatgtgttgtactaggttatgtcacggatcaatttcataatttctataagcacttaatttttcaatacgtttcacagcccgtgctctactagcttcccctttaaagatgctaaaaatgtgtattgattcagccatatctgatcaagcacagtaattgaaaactagttagaatgaatcgtataacctaatcatgatccacaccacttatgaacgtatagaaaatgtggtatatcgaacactcggagtatttttcatttaagagagtgagagcacccaaaaaaaaataactctcaccaagcaaatgccacttaacaaatattcttgatttttctaaaaaaaaattagaatttaatcaactttaaaagtgtggggaccaacatgcaatttttcaaattgcatttggaatagtcaacattcaaaagtgtggagaccaacatgcaattttccaaattgcatttggaattatcaacattaacaggggaccaacatgcaatttttcaaattacactagcaatatttgagggaccaatatgcaaatttttatcacatacacggcaacaatttttgtttcaatttttaaaatttttgtttttttttaattaataggttactactcatccgcctaaaaaaaagcggtttttttttttttttttttttttttttttttttagatttttggcaaaattttggaaggccataacttcttcaattcaagaccaaaaattatgttctttaaaccgttgcaaaggtctcgaaaaaatctatccaaccatataaaatgggtaagtgaaaattaacgtgcaagaaattatcatgtgatgaagtttcgattttctcaactagggtttgatttttctcccaaaatacaagtccaaataaagtgaaattttttagatattttctgcataatatcatgaacatagagaatgaatttcaggaatttatatgaagtatatcaaaagttgccattaatgaagaaaacaacataaatgtctatttagactctaataccaatgtaaaacatgcttgcctgcttctatcgaaaataaaaattgtaaaacttacttgaaatcaccaaaacgaggttgaatcacatgccttttgtttgcttgtcttctacactattttgtactcactccttggtcgaaaattcgatcaaaaaggaaagaatttgattaccacaatcgaagaacccaatttgagatgatattcttccaaaatcaagccaccatcctcaagtatctttctctgtttggttatcatacgagttttgtatgtattatttcatattctttgatgtggaagttgtatatgggagtagtgggttgtgggaagttaagtttcaaattcaaatttctcaacttcctcaacttgtccctccaacaacactctaaaataaatcgggttgggtcagtccacatggatgacccattttcttccaacagtaagatttctctttgactctccaaattttaaattggcatttttcctttttatttttttgtattcaacgaaattttattttcattttttctttttctttttcaattcttcaccactcatcaactctctagcattcctcaaggttagttggccggtatgtgcggtgtacatagtaactactccttgatcatcttatatcctcaagattagaacatctttctcactgtcaaggttaaggctctaattgctgctatgaatcatcgatacgaaaaatactggcatactccggtcttccttgtatattcaacaaaataaaatcaattgaaaatataaatttatccaccttaatgacactatcctcaacctcctcccatcatggatgctttaatgaatttattagcaagctgcaaaggcaccgtattttctttactcttgctacaccaagtctatgtagatagaaagagccatcaaattaatgcttgcaattaaatcacgtaaagcattaaaagttcaacttttcccaatattgcaacttacttaggaaccctttgaatctttcaacattggaggcagcttgttgagcaaaacctgctgtagacgggatattgacgtgtagtttcttgaagatatcaataaacgtaataaattgcttgtcaaactaactctattcgtgctgctgaaattcatgtggtttctgacagcgttttggttttcacccaaagagaagtgaagatgatttctccggttaaaattgtaagaggaatattatgggtattactccacataattcatcttatccatagatgaatcattcgagcgtgcattgagcattctgttacgtggtgtatagcaacatctacagagatgttgctattaaaaattgagccgattgttatgaatattaaagatgagacaactaggaaaatgaaaataactatcataagaacataaagatttacctgaaaattcaagatggaaaaaaaccataatcagagcccgagaattcactttatcaaaaggagttgcaatatgtgatgtatgatctcacaagactctctcctgatctctctatcttcgagtctctctattaatcttggtccctctaatatgtgtaatacaccacatatttataatacaacataatctctaacatacttagagaattaatacagtgaagagtttaatatatgatgaaatctcaatataatagataaagtcaacaataaaatatttaggttgaaattggagtaaaaaacgtccataaagggaattagaatcccgtccggactatcaccacctctcgagcagcaatttctccaagcccgagctatagcctggtgcctctaacatccgggctccggtatagtatatttatattttagggtaaataattttcatataagggggaattggatcaacttgactatactttccaattttattgtttagcttatgaaaaatcaagtacacgtatctccaaataaaaattttagaattttcatgctctaagagttaatgaagatgctatcaagctacatttatttccttatacattgcgagatgcagctttgtaatacttctacataagactttcaccattgtcaaatctcatatggattcctcttgcaagtttccattaagaaaagctgttttgacacccatttgccatatttcataatcatgatatgcaacaattgcaagcaaaatccgaatagacttcagcatggctacatgagagaaagtttcataaaagtcaacaccttgtctttacttgtaactttttactacttgctttgctttgtatgtatggatatccccgtctacatcgacatttttcatataaacccatttacaacctatgagttttatcccatcagaagggttgactaaggtccaaaccttgttttcatacattgagtttattttcagattccatattctcctgccatctcttcgagtcaacacttgactttgcttctatgttatcagtaggttcatctttctcgactaatagtacttgaatgtaactgtgaattcatatattctagaaggtcgaatggtcaaattgatttaggtgaagtgtcctcaagaacctccatgtcctgatcaagagtttgtccttcagcaggtgtgggatcgaactcaggttcatattattagtcaacagtatctatggattcgtgaccttcttcaagttctaatttacttccactgccctctcctaataactcttttttaaggaatttagcatttcttgcaatgaacaccttcttctcaatggtattataaaattgacatccaattatctcttttggatatcccacaaatatacgtttattggatttagtctcaaaattaaccgattcaatgtgcgtcacgtgagtgtcacagttccaagctatcatagagataagttgggtctttttctcttccataactcgtttggatttttgtcgactgatttagatgggacaggatttagtgtgtagcacgtaacaattaatgcatgatcccaaaaggattttgggaggtttgcatggctcatcattgatcatgccatatctaataatgtgtggatcctccgttcagatacaccattatgctgccgtgtatatggtggagtccactgtgagagaattccattcccttttagataattttaaaacccctcttttaaatattctccaccttgatctgatcttagcgtgagaatacctttacctgtttgtttctctacttcaagcttgaattccttgaactttttaattgctttatgtctaaatttcatcagatatacagaaccatatctagaatgataatcagtaaatgtaatgaactaagagaaaccacctctagcggtgattggcgtgggtcctcatagaccagtatgtatcagccccaataattgcgctgctctttctccttctccagtaaaaggaagtttggtcatcttgcctaataggcatgattcgtacttgtccaatgattcaaaattaattgatcccaagtatacatctctatgtaattttggaattgcattctcacttatgtgacaaactctgcaatgctagatatagatgttgttcggattatcatttttatgcctttcaacttctatactcattataaaatactcggtatttaaaatataaatgttatttttgtaatttaccataaccattaagatcttatcaagataaaaaagaaacaacaattgtccttaacactaaaatagttcatgctcaaacatgaaattatttaatgttttggtaatggtatatacaaagtaacatttctctaatttcaatactaaacctaaagacaatgacaagatgtatgctcctacaagtaatgcagcaatctttgctcatctttaacgtacaggtcaacttctccctttagcagtgatccacttctacttagttttccatatttgtataaatatgagatccatgtctgatatttaatacttaagaagctaataaagtagatataaacattgcaatctttcttccaatgacctttcattctataatgatagcaatgttcattagatttggtattgtccttctttgctttgaccattttagctatattggatgcttacctaaaacatcctttagacttcatcttacaacccttcgaggaatcaaagattaagattttcccacttcaaaatttgagacaaattttgatttaagcatgtttagagactcaatgagtgttcacttgaatttattcatatcaaaattcataactcactgatagagattacagaacgaagtcaatactcatttcatggttcacgattaaacctaatttagacaacttctcaatggcaatcatattcagtacatgagcactgactaaagattcctctgtcatttaacactagtatagcagtttggaagtctcatatccttccgtacgcgattatttgtcgtacaactatttgaaattaaaaatcatgtgttagcatctaaattctcaaattgtgttgccaatgaaaaagacttggtttagttgtttgtataccaagtatgcctctcaaatacatatggttactcataattcaataaatataaatgatgaaaagtaaaagaataatatataaaatgcttcaaacaaatttaacatggtcttttattaaattaattatgctcctattgtttaactcaaatttatgaccctttgtcataaatttatgaaatccatacttaactctcagtgggctggaatctcatttgttatattaagactttgagtgtattcaacaagtcttaataaaatatttaggtagatactattattaattgtatttttatacaactcttagatcattaaactgacaaatttttgtcttcacatatattatgtgttagcttaacatgcctctaaaatttatctccttgagtgtacttaacaaaagataagttttagttaagtcaaactcatcattcagaaatatctaatattttatagtgtctaacatatccctaatagaccagtctaggtgtactcaacaagctgggattgattgaagactctaatttttcaatataatgatagaagtggaatataaatatgacttaatattttaatgagggattttgcatgcaaaggtcctatcataataagtatacatattttattatacatctaatgtgcaaataaacatatatataatacaatagtgtagatgattatggacttttactatcaagtcttctcgacccattagaaaaactagatggtcaactcctaggagggtattgcattaactcacacaatgctccatttctatggtctcctccttttcttttttcttcaattaatctagatgtaacatgtatcctatgctagtaggcacgcaagtctaaataattggacatgcagacctaccaaattacgacagagtcgtaggtccaaaataaagaagagctcgtaggctcataaaacaataagattaactaagtattcaacacattcacatggtcgaattcataatcatccactaataaaatattcatcatataaatgctttactatgtaatatataatattaaatacatgtatatttcaagtttctatcaattaaggtcatctaaactaatttagataaacggattggaacattaacctaataattaatcatattaatcaattgatttaattagcgggtatatttattttaaatcaaatttaaattaaatatcaaattagagtctagctctaatctcactattatcgcatggaactatttaattaaaatcaaattttaatttaatatcaaattagagtccaactctaatttcaaaacttaaggcggttgaaattaattaaaatcaaattgtaattaaatagcaaagttggagtccaactctaattccaagatattagggcaaatttatttaattaaaatcaaattttaattaaaataccaaattagagtccaactctaatttcaagaaaaaattgaggtcaagacaattaaattaaaatcaaattctaactaaatatcaaattagagtccaactctaatttcaagaatatattggggtaaataattaattaaaatcaaattttaatgaagtactaaattagagtccaactacatatttaaaattaaaattttaatttaggataaaactcctaaataaaattcaatttagggtcaaggtttaatacataaattaaaatctaattttaatgataatataaaagttgtcaatctcatatataatttcaaatgggtcaaaatttaaattttgggtcaaatccttctgaacttcaaatttaaaaccccttttaaagttgcgcggctgcagcgcaacaacgatgctgtcgttgcaatttcagcggcaatgtacgccgttgtaacactgcgatagctgcactgccttcgcccgcgccatcaccgtgattgccgccacctttttttttctcgatccgttttctgcacaatttattttcttttcaaaatcagattttcaagatgaaaaattatattcttaattgctagaaacaagaaaaatatgaacaatcaacttttgactattcaaagatgcaaaatagcttctaaaaaacacaaagtaaactctgatactagtattaggaatttacttaatcacccatagcggaaattaaaataaatttcaattcctgtcaaggatctactttgtgtttagatggaaattgtgatagaaattatacttttgttgaattttataaactcctttgctttttttgaactccaacaatcatgatctgcaatctgcaattgtccaattgtcacgcattcaatgaaaatccacatagggaataagattgaaagaattaggatttttactctcctagtgttagcaagaatatgatttttttctaacaattttcaaaccttggcagtttatttatataaaccaaatggcttggcccgtttcttaaacttaacacggtccaatatttaattaatcactacaaaaaataaccgatttcgtgacaaaaaaatgttatcgcaaaaattgagatcttgttgttaaagtaacttagagatgacaatatgtttgttgctggtattgtcgcgctatatgagtcacagaatacgttttgcaacgactttggaccactcattgcattaacaaaatcgcaacaatatttgtttgatgcaaaaaatatgaaatagcaacatagtatttttagcaataatgttgtcgcaaaattactattttgttgtagtgaattcaattaattaattcggacctattaataagcaacctaattaattaattatccaacacttgtcaattaattaattggtaaatctcatttttcttgttctctttttgtgtgtgacccattaggttctcagtcaggtgcctaatgacgtgaattattattttgatataaccaaaatcaataaattaaaaatgcccattttaacttatcactaattcacattcattgtcgtagattgatatgtagcaatgtgtcatggcaatatacgtgacgagaaatgtcacgtgatatgacaaaaccaaatatgatcgtttaccttgaaactataatcctttcgccaatatgatccgatcaattacgatatatggatatgtgtcactatcaattatcgattttatctttcatctcgcaattaagtcaatgtttgacttatgagtacactttagccaatgatttcattatcaatttaattggatgaaatgtagatcataatatcttattatatatcagtgacaaatcctatatagatcctttacaaccttcatatgattcttaaaatacccgaatgatgtcgtattagcggccttcggcagagcaacatctaacatcaccaaagtatgactatcatcttataaggcaatatgatgacctcaagtcaaatgaccaatttcactattagacgttagagattaaccactgacactcggataattatccttgaggaatctcctaactagtctccaatgatgtgttctataataaaacatccatgtgttcattttaatgtcaccactttttagcttgtaagatcaactacttgcttcacaataagaaatgtcacgcgtgatgtctatctgtatctcattattacttgcgatcacagatgatttaatattcaatcatatgtaattcatattaacaaattattaggatttgaatctatggattctattatttaatttaatttaatattaattaaataatggacctgccataaaattgcatcaattatatattaaaaatacttatatccaaagttgattggaactagggcataacaattacagttagtagtatgatttgaacctttaaataaaccctagaagagagctcaacaaagaactaatctgggagtgcaggaatgaataaaagatgtatttgaccatagaatgtcggaaattgaatcaacttatgattatataatatttgacttgatttttcacatacgtaacatttgataagtgaaagctaatcttggtataattattttgaagttgtttacaggttatgcatgaaattttttagcgataggttgtctaaatattgttgtattttgtgttctttatatatatgattttatttgagaagaaacaaatgttcaagtttgcgggtatttaaaaatttacacttttttgatgttggatgagctttcgagaaaaggagtgaaaattggataaaaaagacgtgtttcatacttaattctgaaaatggggaccaacttgctacaaattggttaccatgcgatcggagccatggatacggaaaaagcattttgtttcccttcttactttatccatcttttagaaagcaatttggccaatggtttaacctagtgtgagatgttaattccgacacttttaattcaagattttagagaagaaggcaaagaagatattcatgacaaaaaaatcaagattttgaagataaaagcatggaattgaagattaattgaaggcccgttcggagacattcaaggaagtgaaattgattataattcttcttcttgcaaattggatgatgaaaattcatatcttttgtttcaaattcatcgttaagtatgttaggttaaaacttgtaagtgtggggatgaatacattattttactgtttaattaaaagacgatttgttttattacgatttatataattgattgatatcatatgtttattgtttatttaaatacttgatcaccatttagataataaatagctaattttatttttgagtggtttgaaataagattagcatattgtaataagcatcatatattaaataaatgctaggaataattatttattgtttatgtaatcaaaaaaggtaatcaaatgattaaattcgtttctaagtatttgaattcggaatagggatatttcaggtgacgtttaaaaataggtttaacttaactcgagagggatacttgaatacaattggcttatcaattgccaatttatatacaaattagagtaaaggttatagttcccgaattggaatggagatcgatagactgaatcaaattccaaacaagttcttcataaagtcatacttaggtagaaattaaaatagacattagtataaagtaaaccatcgtcattatctgattcaatttgaatttgattttgaatcgatacaattcaagttaaaatctattcctcgtggaaaagataccgtaaacacactaaaattattacttactaataatctcgtacttttgcaatatttcaccgaacaatatcctgtggaagaaaaaactcgttctaaaaactatccagtggagagttggttccggaaacaacataagaatttttgaagacccgtgtctacctcgtgcaccaccttttcagccatacactggcggagaatgccaaatggatccttgataatgactaaatggggaggcaggaatagagtttactgagacatatcttgatagacaaattatacaatccatgccacttaacccaaacttgacggcggacagggtcagttagcatttcgaaccaaaagggcttatgttgggttgtgtccccacttgctatgataaaataattatttataataaataagttgtggttttaattatctcactatttattattgagcatgcgaattaaagttcctatgatcacttgagataatataagttgggtacttgtgttgagaagtacattgtgacacaacttatactttgatcataaataattagttcaaaaccaatgtataacggtcggcaccttgtactggaaagttgtagtattgaccgatttactattcaggtttgtgatttgtccttctcacagaaatagttaaaggtgacgctagtacacttgaagtatattgaacggatcacgtgtcgaatttaattctatagcatgaccgtgggagaattaaattccacgtgatcgaatttaactctatagtatgattgtgcggagaattaaattctatttgaccgttgtgtattttatctaaatccttgacaggattatatatattttttcatgattttaatggttctttgatttatcaatgggtgaaatcaatttgattggtcaaatatctcaatgagttgggagcttgagaaataagcggagtagataacatgaattcgtgccgggaactgttaccctaaaaaatgggtagagtgactactaaattttttttttttgttgaacggttaaaatctgatttttgtgtttagcgacgactaaatttctacatttgcgattagttcacaggaccgttgaaaaaaaatgatacctgagttagtgagaataattagaagggcaaatggtcatttatgttcgtacttaattatccaatcccgggcgagaataaaatacatatacgacaggttagaagaaagtattacagattttattggcttttgtgatcttatatattccaaaaatttattatttttcctttagtggaaaaaagtaaagattaataattagattggacgatctagggtcgactagacaagaagtaattattggaatttgtaaaatatatatccgatcaggtctctatactagctctataaagtattggagcttaattacggtaattataatagttttgtgtttattgtaattataataaagtgttatacttggttataattactatgaaagttgtaaacctaattataattgtaattgaagttttaggactatacatataattaaatgtaaaataattgaatttggactttaattaaaacccatactttgattttaattaaaattcttatttgaatgtgaaattattattgtacaaggattgtaactattttatctccataaaatagagattaaatgaaaattagacatcctataagattgtataacaattatacataattccataatattcagatttatagaaaaaagggaaaataattttttctcatcttattcaattgtccaattcaaaaattagtttcttgatttaattagaaagaaggtgcctacttatcggtataatcttgacttcgaagattaccatagaagacttggaggtttgaacctccaagaaatcaagttcttggaattaaaaagctgaaagttcgtgttctaaaaagttggaagttcgtgatttaaagttaattcaaaaattgattattgaatttaggtaaaaattcgaatcatttagtcttgatataatatacacgtaaataactagacgatcttgtttattgaattaaagaatattttaatttttgataatttggcttctgcaatccaacaattggtttcagagcaatctagatcgttcacttgcttgttatttctaaatcttgattgcatcttttactcgagcaatatctagaaatattttattatgtgatgattgaatgattgtataattttatatcctgttccaattattgttgccaaatcttgatataattcattgtttcgagtttgtaacaagattggtggattacgactctatcatcttgatttaattttttttgttcaattggattcaaaaattctgaacctacgagacataaaaatttatgtaattcttatagttatggaatcttgtaaattgattgagattgaagacgaaggacgaaaaagtttgaatacaaaaaaatgttgaaattttcgaactcgtcagcagatggatccatctactcagtagacagaattcaaaacaaaaattgtccgctgcaacggacaatttttttttttcctacatatggaccaatatgcactcacgtgcattagttcgggttgacttttagtgcagatttgttttcacaaatggggtcggatctggataaatcgggttcgaaaactttttgtataggtacggcagcaaactcctttactatttttggaatgttactgttggatccttgaaaaaattttcggttgaagttttagatttaatattgtcatgtcccattagttttaatttaatacttgagtttaattttatcactttatgaatgcttaaaatattgtcattcttgatatcacgatatatagatttatttatgatatcgctagtgatactatgaataggatgcagatcattaaacaccattttcacttcaattaatttaatttagatgaaatttttctggaagaaaatttcttaataattaaactgtgtattaatttgaacagttgataattatttttatgtttcctcgattcatttaatttggattaaatttttctagattgaaaaatcgtaataaatagaactttatattaatttggttagtatgaacagatcatcgttacttaaatttttctccatcaatttaattatggataaatttttctggagaaaaaattcgtaataattatactgtatattaatttaattaatgtgaatagttgttaattatttattattaaaatccattactttaaaattttatgtgagagtggatgtttatttaaataaaaattcatggtctcctttggtcaatccataagcaaagtaacatgtttgcctcgtaccgataatgtaacggactacatataggaggaccatgcagttcaagttgcttgactgaattcctttttggtaagatcatctaaataagaatataatttgtgatcttcgtgtagatggtgaaattattttcaagcatttggagatctagacaaagattatacactcaaattgagatcatttacaaatctcctatggaggctcccatttatgattttagtgaccaaataaaatgatactggacttatatagacatttgttgtcagatatggttaatcttgtgggagggtcccaacttggccagtggacacagttacctttcccataaaaagacctgttggattacatgaattgagtaattgttgcattattgcagttagatggatctacatgtgcatttatgcatcatatgctaaattgttatttgatgctcaaatttaatatgcaatatatgattaattttatgaagaatatcacttggcttgtaacaccccgacccgtatggatcgaaacggcactagattaactgtactttaaccgtaaattaattaactatatttttaatggaaggtataaagattaaattttagaatttaattcaagaattttgttcttttttttaataatatttcaatactaaagaaaacaatttcaaaaatatttttagaatgggttccatgcatgtaacgactattgacgtgaagttcttggcaaaattttaaaagtaatgttgctgttttagtttttatctcaaatggtaattgtcaaaataaattcgtttgcatagctatcgacctctaaacttcatcaagttttaatgtaaagtaggaaactccttataatatgacatagtaaaaaattagcttccgtcgacattatatgaggtattaaaatatttttcaaaacctagcagtgactcggttaaaaggcaaatcggtacagtacacttaaaatgatatataaaattccacagacatcaaaaccatctgttttttaatttattcaatagataatccatgatactatcaaatccaattggtttcatccagaaattccaagtaacggtcgagttatgaacttttgaaatcaaggtagaagctggaaaatagcaacactagtcagtgcagtttaccttaagtgacatataaaattctaccgacatcggattgacattattctaagtttattacataactgacttatgaggctatccaatgccattggctttgtataaaaataccaagtaatgaaagagttatgaatttttaaagatgaagcagaaactgaactttttgaagagacaacaaaactttaaatcgctgacatttttttgtaaatggtgatttgtaaatttatttctatgacatatatctacttacaaacataatttattcataaagaaatattcttagtagagttccacatatgacgtccatagaaatccaaaaaaattaaacgtaaacatttcatgatttaattaaaattttcaagtcaccggctttctccatggcatgtcgcatcatcttttatcatcatccacgccccaaggaaaatccattcaacctgtaggaagggaattaacccataaatttgaaagtcaatagatatcgtctgtgcatctcattatcaaattagaaatttcgaactatagattcatatcgtcgcacatagatgaattttcgacaaaatccaattacgatagcattatcataacaggttgagccagagagtgataattcaaactattgtagtgtcgaagcatcgtatccggaggtaccatttcattcaaacatttattgaaaaattataatttgaaaatgaaataaacacttgcacctctacctaccttgaattttgttggatataaaagaaccaaatgtgtaaaaagcatttcttcttcacacccttgctattccttaagcttaatttcacatgaagtatatttgagagaaattaagagtaaattcggatttgaggggagatgtaatgaaaaagtcacattccttttcttgtaaccttcatttttaatgaaaaacaaaataggaggttgtatattcattaagtttattaaatttggtctttaactaagaatttgaagagtttataagccaaaaaaaattcatataaaaggttttataaaaaatccacatgatagttcaaacctgggttgcctatatgaaataacatgtagatgaccattgaggcaacccagttattcagtaaatctttgtaatcaaatttacttaaacttaatttcttaaatttttgggcttttaattaacttatgacttgggctttcataatcttaaatgggttgagcttccataactcgtttcttacatgggctaagctcgtggtactagatcatcataaaataatagccaaatttcattttatttctcgggctactacatggctaatttttttcattattctaaaataaagccaattaatcaggaaaaattatatggattggaaacgtaattcaatgtttgtgctcaatgtggaaaaacttgattttgtgcttaacgaatatcatgatggacctactaaaactatgtgacaagtccaaaaggatgggtatgttgagtgagaaactgcagacaagatgtttagttgtttcattttgcttttgatgtcaaacgtgttacaacaaagacttgaaagtcagagtacctcccattacatactagagatcctttaggcatgtttggtcatcaaagtaggaatgctattttgaagtcatttttaccttatagaacatccgcatgaaattcagagtgcttgtgaagtttcatagtttgactatgattgtatacttcaaacatagccaagagtttggatgcaaccatttatcaagggtactcagtttttgacatggtattgaattttttacctaataatttttcatagtttactatggatcatcacttacacaagatgaagatactattgactgagttaatgatagagttgtaatgtggaaagtgatcctaatggtacaatggcgatgcccgtgcattatttgatgtctcctctggttccaatccaaaaggcatgtttagaaagacgaggaagaaagctatcaacaagcatgagagcaaataagatcaaaattagacggaaatccttgaggcaagtgttccaattatgatcgaaaaggacagtggagaaagactgccggggtgcacaggctagaaagcaaagtgcgggtgggtttttcataattgaatattatttagtggttgataatacaaattcttgagttgtaaattttggaaccactaatcatatatacatgtcaatgcgagtgctataggaaagcagaaaactcagtaaaggctagtttaaaatcatccttagcataagagcaatagtttaggcaagagcatagagtattatttttatttcaattattataagagtttgattcttagagactgttattatgtcccacaaaggaagtaaaaacttgatttccatttccggtttaatataacaaggttattctataaaatcgcttcgcattttaatgaataaatttcctattatctttggacatgtgattaatggtctttataatttatctattccacatatgaaataaaagttacttcgacaaattgtagaccttaaaatatcgcaccatactagtattacatatccatggcgtcttggataaatcaatcttaacaaaatataattttgactagagatggctctctcaacttgacgtgatccaagagccaagccagacgaaggtgagtacgagacgagacttgttgataatagaaggtggactgatgacacgatagaggacaaagcaagtaaaacaagtaatgggattgctcgtttaagaaatcattgatgggacgatgttcgggactcaaaatgagacaagtttcgtgttcaggtcgaaagccaaatcaaagtggatcaactcaatacaagcggacgaagacggaggccaaagtaacaaccatgtggccgcacaaacccatgcagggttttctcaagaggtgatagtttcttccatgcgaccgcatggtacaaaagtccgacagaattttccttttttcgcgaattttcttattttgttagaatttgatatcaattagacttctttctatattttgacgattttgcgcgattttagctaggtttttacctttagtataaatattctctccattacattttgtaaggagttttggcaattattattgaatttaagagtggcttttgctttcttccaatttgttcttctttgaacaataatttagaacttatcaaggataattccttgcggcgttcaacaccggatcgtgggttcttcaatttttaatcaaggggtccattgcatcaccattatcttttggttctttgttttatcttgttgggttcaaatccaaactggttatcaattggcgttattgggttctgcatcaatctggttatcggttttgtagtctaagttgctacagggttcgcatcagttggtatcagagctttggtcccaatttaatcaggttctatctttaattttcttgtttaggtcatagttttcttgatttccaagttgcttccttgttcttgagtcattcttcaattcattccttcaatttccttcaatccgtatttttttcgttcgtagtataatctcttatgttagaaaaaaatgttactgttcatctaaatattaaaaaattaaaagacactgctgatgttcaaaaaaaataaaatttattaattggttgatttgctaccaacaagttcacattcaaattcttaaagtccaaagttcttttttctttaattcttcaatttcgtcaattgatccgttgaaatttagtgagtccattcaaatttcattcaatttgtttccaaatcccttgaaaattattctcttcacttacattttgggttgaatccacaagttttaatccgatgagttcgttattgttcttggaagctctgggtgaaagtattaagttgtaaaaggcagagtactgagctcattagagggtaaaagccaattgtatgatttcgagtgaaatttggtgaggcagaaattgagagaatgtctgaacaagaaggttccaactcaagctgacacgactatcacaacaacgtattggaggatttgatacagtggtttgaacttgcttttggggttgttagagatagagtggatcaataggatgcttggagggctaagcaggaagcttggatgacgaggatgaatacatcagtggctaatcttagtagagagctgcgggcgaaggtatctaatgccatgaggccggaaaggtgggagcataggatggagcgaaaaacatttgatttgggcagtgaatgggatgatgaggagtataaagaagtgggaatgggacggatgaagaatagaggtggtaggcctgagcgacgggttaggaataatcacggagatgaagcggatggaaatttgggaaacataaagatgaccattccacagtttaaaaggagaagtgattcgaaagcatatttggagtgggaaagaaaggtagagttgatctttgaatattataactattaggaggagaagaaggtgaagttggtagttttatagactatgcaataacttgacaggatcaagtagttacttcacaatgtaggtgtaggggtagatcgattagctcttgggaagagttgaaggcattgatgagaaaacggtttgttcctagtcactactatagggaggtccataaaagttacaaagtttgtaccaagggtcgaagagtgtggaagattaccacaaggagatggagattcttatgattagggcaaatgtggttgaggatcgacaaactaccatggcatgattcttaaatgggctaaaccgagaaattgctaacatagtgaaattgcaacattatgtggaattagaagatatgttgcatgttgccattaaggtagataggtgattgaagaggaagggggcagctaggccacaaatgggtgctttgggttctaattcatcttgaaaatcgaggtgggacaacaacaaaggaaatggggctgtacctaaaggtagaaatgaatggcagaagggaaaagacgaaggaactagcaaatcaacaccaaaattggagtcacaaccatcaaggagtcgagatatgaagtgctttagatgtttggggtcggggcacattgcttctcagtgtccaaacaaaagggcaatggtgttgctagatagtggagagatggtgagtgaaagtgagggtgagtatgataacatgccaacattggaggggattagtgaagaagagaagattgaaggtgctgtcggtgatcttttggttgcaagaaggcctcttacttctcatgtcaaggcggatgactcagagttgcaatgggagaacatattccatactcgatgccatgtcaaggatgtggtatgtagtgtcattattgatagtggcagttgtacaaatgttgctagcatagcacttgtagagaaattaaacttagcactattgagacaccctaggccatataagttgcaatggttaaatgaaagtggagaagttagggttaatcgaagggtgttaatcaatctctcaattggaagttaccgggatgaggtagtgtccgatgtggtaccaatgcaggtgggacataacttgttagggagaccttggcagtatgttagacaggctaagcatgacggatacaagaatcgctatagttttgataaggatggaaagaccattacacttgtgccattaacttcagtgcaggtatatgaggatcaagttaagctaaggaatgaggaagagaggagaataaaagagcgagagaaaaagagagaaaactctaaggttgtgagtatgagagaaaattgtaaggtggatgttagagagaaaaagagagaagagccacaagagagaaacgaaagagagtcttccgagaaaaaagagaattcacgagcgaatttttttttttttgcaaaaatgagtgatttgaagagagcggtagttgagaagaaagaaatgattttattgttgtacaaagaaacactcctcaacttggaggagactaacctatccctccctagtttggttaagtctttattgtaggaattcaaagacatatttctggaggacgtgccttgtgagttaacacccattcgaggcattgaacaccagattgacttcatacctggagctgttattccaaatcgactagcttaccgaagcaatcccgaggagacaaaagaacttcaaaggtaggtagaggagttgatgagcaagggttatgtaagggggggcataagtccatgtacaatactagtattacttgtgccacagaaagatagatcttggagaatgtacgtggattgtagagccatcaacaacattacgataaggtatcgtcaccctatacctaggctagatgatatgcttgatgaattgcatggtgcttgtatttttagtaaaattgatcttaagagagggtaccatcaaattcacacgcgggaggttgatgaatggaaaacgacctctaaaactaaatatgggttatatgagtggttggttatgtcgtttggtctcacgaatgcaccaagcacatttattcgtttaatgaatcatgttttatgtgctttcatagggaaatttgttgtagtttactttgatggcattttaatctatagcaaggacctaggtgagcatttagaacatttaaagtgcatgcttgttgtgttaagaaaggaacaattgtatgctaattttaaaaagtgcacttttgcatggatagagttgttttcctaggatttcttgttagtgctgatggggtagaagtggatgaggaaaagattaaagctattaaagaatggccaacatctaaaagtataactaaggttaggagcttccatggtctggctagtttttataggctatttgttagagactttagttcaatcacgacaccattaactgaaatcgttaagaaaagcgtaggttttcattgggggaaaacacaagaacttgcatttaataccattgatgataaattgtgtaaagcacctgttttggcattacctaacttctgttttggcattatctaactttgataaaacattcaagattgagtgtgatgcatcagggataggtattggaacagtgttaatgtaagaaaggagacctattgcttactttagcgagaagttgagtggagctgcactgaactatcctacatatgacaaggagttgtattcccttgttcgagcattggagacttagcagtattacttgtggcctaaggaattcgtgatacacaccgatcatgagtccctaaagcacttacggggtcaaggtaagttgaacaagtgacatgtgaggtgaatggagtttatagagacgttttcgtacgtcatctggtgtaagcaaggtaatggaaacgtagttatggatgcattgtcacgaaggtgcatgcttcttaactctttaagtgggaaattacttagttttgagcatattaacagcatgtatgaaaatgacattgatttttcaaacatttacagttcatgtactaatgactgttgataaattttatagacatgaaggatatttgtttagggaaggtaggttgtgcattccaaattgttcaatgcgtaaatcagtaagggaagcacacagtgggggtctaatgggtcattttgggattcaaaagactttggacatattagggaaacacttttattggcctaaaatgcgtagtgacgtagaacgaatttgttagaagtgcatgacttgtaaacatgctaaatcaaaagttttaccccatggcttgtatacacctttacctgtgcctagtgaaccttgggtagatatttctatggatttcgtgttggggttacctaggacaaaaaaaggttgggattctatctttgtagtggttgataggtttagtaaaatggcacactttataccatgccacaaaactgatgacgccactaacattgctaatctattctttagggagatagtacgtttgcatggagtccctaggagtgttgtgtcggaccgagatgttaaatttttgagtcatttttggcatctttggtggaacaagttaggaactaaattgttattttctacaacttgtcacccacaaacagatggtcaaactgaagtagtaaataagaccatgactcagttgcttcgaacaaagattaataagaacttaagaaattgagaagattgcttgccatttattgagtttgcttataatcgtgctatacattcgactacttcgtattcaccatttgaaattgtgtgtggatttaacccactaactccattggatttattttctttgcctctgaatgaacgaggtagcatggatagtaagaggaaagctgagatggtgaaggcactttatgagaaggtctgttcgcaaattgaagagaagagcaagctcatcgtataaaatgcaaacaaagggcagaagcgtgtgacatttgaaccaggagattgggtatgggtgcatttcaggaaggaatgttttttgaagcagcgaaagtccaagttgcaaccgcggggagatggtcctttccaaatcaccgagaagatcaacgataatgcctacagagtggacttgccaggtgagtataatgtatcggctacatttaacgttgctgatctttcccttttcaatgcaggtgcagattcgaggataaatccttttgaagagggaggggatgatgtgatccaagagtcgagccaaacgaaggcgactgcgagacgagacccattaataatcgaaggtggactgatgacgcgatcatgggaaagcaagtgaaacaagtgatgggattgctcgttcaagaaaccattgatgagacgatgttcgggactcaaaatgggagaagtttcgtgttcgggtcgaaagctgaatcaaaatagatcaactcaatataagcggacgaagacggaggccaaagtaacaaccatgcgaccgcatggttttaaagtggtgtggccgcacagacccacgcagggttttctccaggggcgatagtttcttcaatatgaccgcatggaaatgtaccatgcggtcgcatggtacaaaagttcgacagaattttccttttttggcgaatttccttattttgttaaaatttgatatcaattagacttcattctatattttgatgattttgcacaattcttagctaggtttttagcattagtataaatactctctccattacattgtgtaaggacttttggcaattattattgaattcaagagaggtttttgctttcttccaatttgttcttctatgaacaataatttagaacttgttaaggataattccttgtggcgttcaacactggatcatggatttttcaatttgtaagcaaggagtccattgcatcagcatcaccgttatctttgggttctttgtttcatcttgttggattcaaatacaaactggttatcaattggcgttcttgggttccgcatcatctagttgtgggtttcgtagtctaagttgctgcagggttcgcattacaacttggttatgatcgaacaattgtcaatttgtaattcttgtttggaaggtaatataaccaagatatcttttttaacaaacgagatagaaccaaagacatacaagaactagtgcattctattatgtgtggtcctatgaatatactcgagaaggggaactataagtatttttttatagatgattactttaaattcaaacacatttacctaatggcttgaatgttaaatattcttgagaaatcaaaagagtataagactaaggtcgaaaaacatttgggtaagagtactaatacacttcgatctgatcgaggtggtaaataccacttgacagaattcagggacaacttaacagaagatggtactgtttctcaattgaataagcctgatatactcaaataaaatggtttttcagaaagaagaaatacgacgttgttagatatggtcagatcaatgaagagtttcacaactttaccgatctcatttgggatatacactagtgatggcaaaaaaatccgccccacgctgaacgggttggtaaggcaaggtggggtaccccatcgcggggcgaggatgccctgtcccatgaaggaaaaataaaaaaaaattaaaaataattttatttctacccaattcattaaaaacccattttgaatttttattttactttctaataataacataactcgaaactttgaaaatgtaaaaaaatttaaacgggcaaaaagttcagcttgccccgaacccgccccgttgccatccctaatatacactgaaaatatctggatatattcttaacttagttccttctaagtcttttctcaagactccccttgaatttcggagtgaattcaagtcttgcttgcatcacaaccaagatttgggggtctaacttacgtgctgaaagagacgacggaatagtttgagtctaggttagagatatacctatttgtgggatatcctaaagatatcaaaggataatttttatagtcctctagataggtttgttagcacaaatgcaaccttactggaggatgagtatataataactgttagtccaagaataaagtcgtgttggaataaattagtgggagcaattctacctcatcaattcctaggatacgacttgggacagacatcctacgatgtcaaatatacctggacaacatggtctgagtggaagagatgagttgtcatctaatccaatagatcaatagaacgttgaattaatgaggatgtaatggcaccacctaatgataataccagcgttgataaaaatattatgttccaaatgaagccatggtcctagatcaatcgtcccttagccaagtcaaatgattatcagtttaccatcaaggtacttgttgagtagatagtccaatttgttgatctccatagtacaagttgatgatctgactttacataaggagattatggatgatgtggatgcagcgatctatttatggatcgaagcagacatcgaaatcttggaataaagactcaaaaaagtgattaagacatttgattttgattagaaatttgatgaatcttgtatgtataaggagacataagacaaaattgtattctttctctagtccttatgaagatgatattctattcattaaaaataatgtggatgttttattatctatgaaagcataatttgcccaatagtttcatgtgaaagacttaatgatgctggctatattctaggtttagatcttgagagatcgaaagaacaatatgatagctttttgtccgaagtcttatatatcgacaagatacttgtcaaattttctatgcaagattttgccatcaagtatcgaatccaactctttaaggatcagtccgcgaagactactaaagagatttgagtacatgagtaagatatcttatgtgttggcagtaggtagtctcatgtatgctatgctgtgttatagacctgacatttgtcatactgttggtattgtgagtcaaaatctatctaaccataggatcgaaatattgaatgaggataaagcatatcgtttagtacctctagagaataaataattatatgctcctcactagatcttattttgataggttgaaaggattcacacttccagagcgatgaagactatcacatgtctacatcgttatcattgtttacacttgattgtcgggccattatttggagaaatatcaaggaatcatgcattgctaattccaccatcgatgttaagtatgtggtagcttatgaagctaccatattggttatatgacttagaaaatccttccgaacatcgaggtggtgcctgcatctgcatagccctttacactgtattgggattatagtaggattgttacaaatgctaaagaaccaagagttattagaagggcaaacacattgaacaaaaatattatctcttaagagagatagttgatagagaaaatgtggttgtcagtaagattgctattgagataatcgtgtacactcgtttactaagagcctatcggctaagtttttgaaggaatctacaaggcacgaggttgcatggcatgaaaaatatattctagggcaagtgagagaattgatggattgtgtgcccatatagtatatttttctacgataaaataattatttataataaataagttgtggttttatttatttaattatttattattgagcatgggtattaaagtgcctttgatcacttgagataatataagttaggtacttgtgttgagaagtacagtgtgacacaacttatactttgatcataaataatttgttcacaacaaatgtataagggttggcacactatacaggtttatgatttatccttatcgtagaaatagttaaaggtgacactagtacacttgaagtgtattaaacagaccacgtgtcaaatttaattctgtagcatggccgtgcgaaaatttaaattccacttgatatctgtgtatttcatctaaatctttggtaggattatgtttatcttttagtgattttaaatgttctttgattcatcaataggtgagatcaatttgattggtcgaatatcttgatgagttggaaacttgagaataagcggagtagagaacatgaatttgtgttgggagtcgtcaccttgaaaaatggatagagtgactatttaagcttttttctattaaacggttaaaatctgagcttagtgtttaatgacgggtaaacttcgacatctgtgattagttcataggaccgttgaagaacatgatacttgagttagtgagaataattagaagggtaaatggtcatttatgctaaaacttagttattggatctcgggtagggataaaacacatatactataggtcataggaaaatattacagatttattggcttttatatcttatatatttgaagagttcagtcttttgcctttagtgaaaaaacaaagactaaaaattagattgggtggtgtagggtcgactagacatgatctaattattggagtttggataatatatatctgatcaagtccttatactagctctatagagtactaagacttagttacggtaattataatactttttggcttaactgtaattataataaagtcatgtacttggttgtaattactatgaaagttgtaaagttaattataattgtaattgaagttctaaaactatacatataataaaatgtaaactaattagatttggactttaaaacacctgcttggattttaattagaactcttatctgaatgtggaattattattatacaaggattgaaactattttatctctataaatagagattaaattgaaactcacataatatgggattgtataacaattaaaatacataattccacagtgttcaaatttatagagaaaaagagagaaaatatttatttttctcttcttattcaattgtctagttcaagaactaatttcttgttttaattaaaaagaaggtgtcggcccaccaatagagtcctgactttggagaataccataaaagacttggaggtttgaagcatcaagttcttagaattaaaaagatggaagtttgtgattcagaattaattcaagaattggtcatcgaatttaggtaaaagttcgaatccattattcttgatataataaatacgtaaacatctagacgatcttgtttattggattaaagaaactttttaatttttggataattccagttccgcatttcaacagcttacatggtaaggattgttttttggggtgtggctccaagaaaattattttaagcccaagagaccgagctctaatgtcatttgaaaaagatggaaaaatagttggtaatctccaaaaatctgaatatatttgtttcaaacttaattgaattccctgcataccaatgacaacttgatgaggaatgtcccaacttctttgtgtgtccgccatcaggtatgatgtgggtaaatctatcttccttgtattactctactatccatccagcaaaatggtgtggtagctcatttgactttgggatgtgatcaaatcatgcacctgagtttccattgatgacactcttctgtagatttcacatgagatgtttctttcctgtcattggtattacgtaggcactttagagtgaaaaaaacccaatctaccatgggatggagaatgtctgctattagaatttgggtttgacctaaattctttgataaaaataattgagagttctaacttaagtgcacattaagaagaattctatttggaatgcttttggaatcctattcaaagtctattggcaaattctaattaaagttctatttggaaaccctattagtagttggaatttgtgttggacttaaatagatcaggataaggaaacttttgggtattctatttcatctatgactctttttctaaggcttggattgcccctatatatatatttgattcttcttccagtttatgaaatgctgatattgtatttttctctcattggttgtcaataataaaattactcagttcttctgccaatctttcttcttgttttaaatcttgtgtgatcaatatttcatattgtgatctacttgcctctcctttttttcccgacaagtggtataagagctattggttgtgatttttgtttgaggtttctattatcgatggcagccatgaagtatgaaataccacttttggatctcaatacaagatttttgttgtggcaagtaaagatgcaagctattttggtacagatggatttggatgatgcgttgttgaaatttgacaggtgccacaacttagacaatagaggagaagcaacataaggattagaaggcacttttgcagattcatcttcaactatctaacaacattcttcaggatgtttttatggaaaagatagcagctgcattatggttgaagttggagaaactgtgcatgaccaaaaatttgaaaagcaaatttcatttgaagtagaggctatattctcatcgcatggcagaatgatgatctttagaagaccatttggctgtgttcaaggagatcgtcactgatttgtaaacattagaggtaaagtatgattaagaagacttggccttgatcctattgtgctcactacctactttgtttttgtcatttagggatacaattttgtacaatcgtgacacactcaccattgatgatgtgtatgaagccttgttctcaaaggagaagatgaagcatctggttggagcagagtccagaggtgaaagaagctcttgtagttcatggtgataggacaaagaggtaagtcgagggtgtgtttcagcaatcaagtttctattgcaagagaaaaagacacatcaaggggaatcgcgaaaagttacaacataagggtaattcgattgcaagtcatggaaggcaatcaaatatttcggatgagactaacgtagttgaagactatttggatggcggaaatatgttgactattgctgacgtgaaatccaagcctgaagatgaatggattttggatacaacttctatgtcccaattgggatttgtttgaagcatatgaaatggtgacacaagttgaaatttacattaaaaaaacaacgaatgttgtcaagtagttggtattgccagggtcagattaaagttgatggacggcacaattagaatacttggctaggttcgacatgttctaaatttgaagaagaattttattcgaaggtttatgagttctctagaggagatggagttttgaagatctgaagtagtatctgtgttgtattggaggggcagaggaggtcccggttatacattttaaaaggtcgcatagaatcgatggagaattatcagcacgggtttagtaccgtggtgaatatatagtttggtatagtacctttgggagttgactctgggtcattattgaagaacactacttagatgagtttggaggatatggataattaaactttgccaccattgtctgtggtgtcatcatgtttaactactagggaaggacccattgaggataggtacgaggatactgatctggttgcatatgctttttgtgattttgaaggtgtcaagactagcaagaggcctttagttaaagcattttgtgtttagctacaaggtgggattcgaccctgttcgataaatcttgaattccttgtgggaattttgggaccgttgtttgggttctagtagcatttgtggataccgtggaagaaaaagatcagtttttcatgagatggaaaagtttcgttttgtttgaagagttcagtctattttgttgcaatcaacttatttttccagtggagaaatttatagctttgttcattgcaccgaattcgtatcaaggtggagattgttaaaatttgggtgcgacctaaattctaagtaaaatgcacattaagaataattctatttgaaatgcttttggaatcttattcgaaatctattggcaaattctagttaaagttctatttggaagccttattaggagttgaaatttgtgttagacttaaatagatcaagataagaaaacttttgggcattctatttcttctacaactttgcttttagggtttggattgtccctatatatatttggatcttcttccagtttatgacttactgttattgtatttttctctcaattggttgtcaataataaaattactcggttcctctgccaatctttcttcttgttttaaatcttgttcttgcttgggcaatcaatacttcatatcatgccatattgcctctcccatttttcccaacaccggttgcccttgtcattaaatcctgactctagttgtagaagcctgagaaataaaatgaaattatgctattattttgtgatgatctaatacaacgagcctaacccattttaaaaacgagctatggaggttcaacccatttaaaattatgaaagcccaagccataagttaattaaaagcccaacaatttaagagattaaatttacataaatttgattacaaaaatttaataaataattgggctgccttaatggttatttacatggtatttcatataggtaacctaggttcgaatcactatgtagatgttttataaaactttttatataaattattttttatagcttagaaactcttcaaattcttaattaaagaccaaatttaacaaatttaatgataatacaactcccccatttagtttttcattaaaaaggaatgttacaagaagaggaaggtcacctttcactaaacccctcctcaaatccgaatttattgttattttctctcaaaaaaatatatttcatgttaagttaagcttaagggaataacaagggcgagaagaagaaaggctttctacacattttgttcttttatattcaaaaaaattttaaggtaggtagaggtgcaagtgtttatttcgttttcaagttatgattttttgataaatgtttgaatgaaatggtacctccgggtacagtgctttagcactacgacagattgaatgatcattctccatctctatgtgttatgataatgttatagtaatttgattttgtcgaaaatccatttacgtgcgacagtatgaatctatagttcgaaatttctaatttgataaagaaatgcatggaaaatatctattgaattcaaattcatgggttaatttccttcctacaagttgaatggatttccttagggcatagatgatggcagaggatgatgcaacctgttttggaggaagccggtgatttaataattttaattcgatcatgaaatgtttatgtttgtttctttttatatggatttctatggatgtcatatgtggaactattctatgaatttttcttcatgaataagttatgtttaaaaatagatgtgttatagaagttaatttacaaaacaccgtttacaaaaagaaagaaaaaaaagaagtgttagcaaattaaagtattactatcttttaaaaatttcagtttctgtcttgactttaaaaaattatagcccactcgttacttggaatttttagacaaaaccaatggtgctggataaccacataggttagcttctgaataaacttggaatcgtgtcaatccgatgtcagtagaattttatatgtcacttaaggtaaactacactggctagtgttgctgttttttagcttctgccttgactttaaaaattcattactcaaccgctacttagaatttctagatgaaaccaattgaatttgatagtctcatggattgtctattgaataactttgaaatcatgtggttctaatgtctgtgaaattttatacgtcattttaagtgaactgcatcgatttatctttcaactgggtcgttgttggattttgaaaaatattttaatacctcatatgatgctgacggatgctaatttttgactatgtcatattataaggagtttcctacttacattaaaatttgatgaagttttgaggtcgatagctatgcaaacatatttattttgacacttaccctacgagatagaaaaagaagagagcttatttagttagtgttagcgggattttggaaaatattttaacacctcatatatcaccgacggaagccaaatttttgatatgtcatattacaagatgttccctactttttcataaaattttatgaaatttcgacattgataactatgcaaatgaggttattttaaaacttagcgtacgaaaatgggaaatcaaaatagattactctctttcttactttctaaagtagttcacaaatggaaaactatcataccttttatttgtttggtagatatgtacttgccactattcatgtaataaaataggcatatgcatggatttgctcaactcttttcttctttaataaatacctttggaattatgttaatattatgttactatctaaaaatagattttaatgggaaattcattagtagttattttggaattttttttaagcttaaattcttaaattaaattattattttaaataatttttaagtctaaaactaaggtacaattgtttgagtgacgcttttgtactagcgggtcggagcgttacactagtaatgtaccgctggcaagaaggttctgtcactcttattgtgtggactgctggtagtctaaagtgggaaataccacccgctcgacagttgaaattaaacacttatgtagcaatttggatggctgatggacttattgggttatgaggtattatctggggctaattgggacatgttgttgccgctattttggaaagaatgtgcgcttgggcctgaggtagcagagttcatggttttgccttttggattgcagctagtgagggaatggggagtacaggttccgaatgtttctttttgagtgatacagagcctttatctagttttaatgcgcgatcctaatgctgaaatgttaaacaacatcgtttgtcttatggttaacatcgtcattggttcttgcagccatgccctcatttgaggaacgtgggtgccaatcagggacaaagacacaaattttatccagtgcgggcacaatttaattaaggtcggactttgaatttttggggacctaaaatgaactttaaatttgagcccttaaattattgtatgcaatatgcattcaacacgttcgtaactaatctctaaacccaaagcaaaataaaataataaacaaaatgaacgatttaatctcaagtaaagttcgatcatgaatttttttttttttttttttggttaaaggagggcggtacctccaagattttattaatttgccctcacttatgacggaggaataccgtattcacatgtggaaaaatgaaagcagtaaattaggaagactacttcccttaaattaattgaaaatatttgagaaaatgtgctaagcagtaaaataggaagtactacttcccttacaataagttcgatcatgaatttaatgatagtaaagatattaaaaataacatagcttataagttaaacttgttttttgtcgatgaaaaacattattcctagaagaagaacctctaccaatcttgcaataccaggtacaatttcatgtttttattttttttaatttaatttaattttattttattttatttttgttttcaaacagaaaaatctcattctctgcttattttcttgaatatttgagttgcttttaaattttaaacacttcagtttgtttttcggaaatgggttcttaaaagtggtatttgattcaaaaatccctaaatccaatgaaattgagaattcacaaccccaaaaaccctcaagagttttgatatcttaaagactcttcgtaatgatgtgaaaaaactactgtctactggaacacccacctactcaaggtatgtgctctaacagagggaagggtgaatcatagaaaaccacagaaaacaatatctagaaacctcgacctcaaactacatcaagaattaataaacaatttttgttcccaaaaaaccatagcatttgaaccaatctttcgtcaaataaaaattcgcactaacaatctccaagcattgaagacagtaaatgtgtttagtggtggaaaaagtagcttaatttagcctagtgcaaatataaacctctatgttctagatgcctatgataatttgtcaaattcaagctaatgacgttaaaagagtgcttcttgggaggcaatccaaggtttcttcccctcatttactctattttcaagttatagaatagtttagtttattttacagtttattctggaatcatcatccatatcccttttccctttaggtccttaagtaattaagttcgttattagatgtttaaggagaaaaaaccccaaatggtcactgaactttgcccaaagccctctaggaggtcatcgaactttaaaacgtccctaaatggtcactgaactttgcaaaagttcctaggggtcattgaagtttgcaaattactaaactttgtaaagatgaatggggtcctaatttgcaaactttagtgaccccctaggaactttttacaaagttcagcgatcatttaggaacattttgaagttcgatgacctcttgggggactttgggcaaagttcagtgactacttagggatgttttgaagttcggtgacctcctgggggacttcgggcaaagttcatttggggttttaacccgacgtttgagctaagtaacccttgttccatgtatgtaatatctaaaattctatttttcttgaacatcacattgcaaaacactgaaatcaacaatgacaaggagaaaacgggataaatctcaagcttgacgagaaaatagatgaagaatccatcaatttcagtatcataaacaccaaacaccatgataatttgcaaacagttcagggaagttcttctcctttttctttaattttatattggggacaatgtttagtttaagtttgggtgtattataaattgtctaattgcctaaatttttttattattctgtgtgatttgtgtgcaatttttttttaaaattacttgttttgtttgcttgtgtgagttagatagccttgccggcattgatgtatataattaagtacattgttggtttatgaattgtggatatattgtgtttgagttgatttttttgcttattcatgtgaaatggaaaatatttatgcatgtgaattgattgtaacattgtacataaataattttatccatgtgtataagttgaaatagagaactgagatgctaaattcaaagaaccactaaacactattatattatgcaaccaaatctaggatgtttgggtacttgagctgttgtagggaaaacttggagataaatgtggattccatgtatgctaaattttgtgtggactgtttgagaccaataggatgaaaattgggtaaaaaccttaagttagaggttagttttttagaatgagtgtttataagggcattgcattaatcaatgcataaaagggaaaaagttgctttgttgtgaaactaccataaaagatcccaatgaggatagctacaataatctcattgtgaaacctctcttcgtagcctttataactcgagtgattaatcctgcaagagtttaaaacctggtgccctaaggtcatctgacttgggagtcatcggtcatttagaggtcatttagaaatcttaatgtagagacatcttcatatgatccgagataggtgccgaactaccaaggatttattgattgataaaaagagcctaaggtcaagatttgagttcaatttaagccaatgggactgagcaaattatttgattgatctatggagtacgaaatgttgaagttgacaagccaaataacttatatgttggtcatgaagatgaaatcatgtttggtgtgttggattcaaagttttggaagaaatatggaaaagcgagtagcgtggattaaaacgggcataactttcaggggcgtcgaatttttacccaagagtacaatcaagaatcatcaagaaattctgcacataaaaaagttgatgttgaaatttaagctatgcaaccaaataacttaaaagccatgcgaccgcatacccttatatcgagacaaaattgaagcctaaagaatgaactatgcgactgcatctgatataactatgcgattgcatagtacaaattccggatgaagtttccaattttcgcgagatcttttattttgactagaattcttatttttttggtaacttttggatttttaggagtttatctccttttcaactcgggtttcctataaatagagatattattccacacagtaaagaagactcttgatattgacaaataattgcaaggcttgtttgcttctagtttcttgttcttgatggaacaaaacatcgaacttatcaagatttaaaacattttatggcgttcaaaactatcgggtgtgaattacagcacgtgcactaaaggggttctaaaatcttcgttatcgtcaagtttcttgatttattgtcttgggttcaaatccgcaaatttgggtatgatttcgtagtcgtgtgattaagaggtcgtcagtttcatgtacttttagttgcttagttcactatttacaggctggatccaaaaccttggtgtatttggtgttcttgggatatgtgacaatctcctgtgggttctatagtgttcgttgctatgtgggtttgcatcacgtccacacataagattagttaaagtatatatatatacacatgaaaaagcaagttcataaaatataagatgcaccacatgccttggttaagtcccaaactcttgtttgagaggattaggcttttgatgagaatttagtgacttggttgattcttggaggttaaagcagtaaaaaataaggagaaacctcatttgttaatattctgaattgcaattactaaaattaaaccaagcatgagtgatgtaagaaattagtattgaaaatcaaccttaaaatacacattgggaagtgaaaagataacaagtttgggagtgtgcgaatcccacatgcgaactaagtagatatttgactttttaaggttgagaattggatcaacttattaatgtacagtgttgcacttgactgttcacgtacacacacattttgcattggatatgcaagaatttaccgtttgcatcatagctttgaagtggttcataattgatactatattttcaatcatgaactatgaaggcaaactatctaattaaatttatttaggtattttcttttattaaatttgtttacttaagtggttgttagttagttttttgtctagtgtttgctcgaagactagcaaagtattaagttttggggtgtttgatgagtgtatttcaatcatactttagacaccttctaaagttgatatttaaataattccaacaagttttagagtattttaatttatattttgatgttgtcatataggctgctaaaattgaaggtaataaacagaagttgacaaaattggaaagagaggcaaaattgtaagagatctaaagttcgaggactaaagtgaaaatactcaaaacttgtgtcggacttcacaatgaagattcaagagtgttaggagtcaattggataaagaaaaaagtcaaaggaatgaaatataattaaagtattatcatacatcaatttccaactgaaaaagttacgctctaaatttttagtttcacattgagaaccatttttgacatagcaaatgaacgaattggaaaacaatatcaatgcaaaattgtatctctttgagctagctttccaactcaccttgaattgcctcaatcagatatcgagagaaaaagttatgataaaatactgaatgataaacagtgctatcttctacttgaagtagacaccgcagcatctacgcccacacaactgaaaataatagaattcaaggcaccattgtactattacagtggcaccgaggcgttgccttgcagaaaaagtgtttttaatgtttttggaattttttcttggcccaatttagccctaattcgtccaaaacttcaagatgctataaatacaagcctagaaaccacttttcaagaagataaaaggggataactacccctacaactcaaaggaaaattcatagtcgaatttaatagggcaagaagcaagctatcatcaagaaatcaagaacaacatcgcaacggagattgaagatttaccaaaactagtatttctattctcttctttatgttgtttatttgaatttgactatttttatcgcttctatcatgaacttaacgtgtaattcctgttcggtgggggtaaaaataatatttttgtagatttttatagaagttgatgaaatatgtgatagaaaagttataggacccaaaaaatatgttgttaaaatgaattgttgactttgacttaaattaaaatctagattttaatcggtaccaaacaggggccatagccaaaacttgagagtatgatttcaatttatttcagttatttctatgagttatgattttaattcttttagttaattggccaataattaaatgaatagatgccagtcaattctggcattcgaaagaggagaatttaggtgcaatcataagattaatacaaagtagattttatgaatttcgagagaaagtgtagaatctatgaatcttactccataaaagaaccatgaacttgataaattctctattttagtttagaatagagatactggaatttgaattctaggattaatttctagccaacattcgagataggagatagaaattcaattgagttcttgcttataaacaagggaaagataattagagataactagataattaagaatcatatttgagagttaggtgaaatcaaattcttggctttcttatctttattaatctttcaaacttgttttgatattgttaaatttgtcactatattcaccataagattagtttaaaaccattgatctagtaatttgattttcttgataaaatatgatctactcaatcatagtacttagtataaaattaaattacaatccatgtgggctcaacactctaactccactagtatattacaaacttgcggtataaatcacgttagagaaaacatgtgacacatctcattgactcgtagcactctggaattatcattttgtagtctgaatcaactattgaaaagttgtaattaaaaatcactatttttccaagtttcgtatcattcacatcaatttatctaaactataaaacaacacgaaaacacaaatcaaaacattctaaaactatcagaattaaacaaaatataaagactacacagcattaatgtgatgagtgaaacacactcatcaaacaccctcaaacttaatactttaactatcctgaagtaaacatacaagaaaagaagaagaaactaatgaaaacatcaaaacaaaactaacaaacaaactcacctaacataagtttagttagataacttacctttatggctcgaaattaaaaacattatcaaatacatgaattactttaaagtcatagtgcaaaatcaaatacatgaattactttaaattgcaaaagctaaattttcaatatttcacatattcaatgcgaaacgtgtgattgtggagaattaagttcaacattgtacattcacaagtttatccaactcctgacctcaaaaatcaagtatttcttttcctcgttcatgggatttgcacattcccgaactcagtttcttttattctctttccaaggtgtaatataaggttgatttacaaattactactccttaaactctctagattggttagattttactaattgtagttcaacatatcaacaaatgaggattctccttattttcgactgcttcaacctccatgaattaaccaagttactaatccattatcaaagtctaatcctttaacaagtgtttggtgcttaattaaggcatgcatatatatattctgtaattaatgttatgtgcggacatctttttatcaagctttctaaagaacccccttagtgagttttaagccgataactctcaagtcagatgactttaagacattgggttttagatctttacatgcttaattactctagtcttaaggctacgaagatacatttcacaatgagattattataattgttttcattgggatcttttagggtagcttcacaataagatagtttttttcccttttatgcagtgattaatgcaatgcctattattcaacactcattctcgaaaatcgatctctaacttaaggttttcatccatttccgtcccattgatctcaaacagtctacacaaaatttagcatgcattgaatccacatttatattcaagtttccctacaaccgttcaactatccaaaatatcctaaagttggttaaaggatactagttctagtttaatggtggctggatttagcttctaaggccactaattcaacctataccatttatgaatcaacttattccagtccaatgttttactaaattcacgtccatagttatttcacgttccatatgataggcaaaaaaataaataaggcagacaacttatccacaatttataaactaacatgtgttctcaattatatatatatatatatatatatatatatatatatatatatatatatatatatatatatatatatatatattaccccaaacttaatctaaacattttccccaatgtaaaattaaagaaaaaggagaactttcctaaattgtctacattgccaattacattatggtgctatgatgttggatttgatgaattgttcttctaccttctcccctaaacttgagatttgcttcataaaaaatgaactcattaccactaaaatttgacactaatataaaaaaataatgatatagagatgaaaagtttaggttggctcccaagaagcgtttctttaacatcattaatttgacataaccgaagcacctaagtcgagtcatcatgctcccaaacttgttcctcaactttaaactcttcttccatttagcaaggccattaggattaggaatggcttcaactctactatagcctccaatacctctttttattttatgacattaggagttttcaaaggttctacaatgtagtttttctttctgtcacacggattgacttttcgagctaagatgaaatccacacttccttagtccctgtgtagcttccaatagcagctgcatcaatctttgaataactggcaagtgttgactttttttgaggatttgttcctttaaaaaattttgaatgacttgctcttcattaacccgtagtatcaattttcctccttggtaatcaatcagagctctccaagttgtcaagaagtgtaaacaaataattgatggtaattcttgatcttctatatccaaaaccacaaattttacctagaagatgaatttgtcaacttcaatgatccttctgaggtatgtgatggatttatcagctagttgtaaagtgattgtgattggtttcacttcttccaagcccaacttcttgaatacagatagtggcatcaaattgatgctagctcccaagtcaaacaatatcgtatcagaaatagaagtgctaattgtgcatggagtaatgaagttgcccaaatcttttagttttgagggagcttcttttggagaatggcactacattttcctaacagcttgactgtctcaaattctaccaacttcgttttctttgacatcactttcttctgaaattttgcataatttggcatttttcaaagcatcagcgaatggaatattgatatagatcttataatgcccaaaaaaatttagaataaaatttatatatattttatattcacattttaaatatgatgactaaaatgaaatatgttttaaattacattttatttgggtcaaataattaaattttaatagagtgagaatagatatgtaaatattgtactcgttggatgtgtcgtaattaatatgaagtctttgacttgagaaaaaattattttcgataagaattatataagttataattcaattcatcttttctctccaaaacctatgaggtgggtattgaattttaagtttatttttagtttaatattaacctattttgaatttgatgtgatagctagtatcctatttgaataactatgaatttgttattaaaatctaatccaaatatcaaaactaggttttatccaatagggtacatgttttctattataactaaaccacgtttttattactctaaatactatacaatggctccatatttcacaacaccaaaacttatatacacaagagagagagagagagatggcacttttgggaactagaagacaagaagccattttacaaccattgttcactaaagctttgaaaagattttgggcacgtgcattcaaatacctttcatatatttcaataatggggtaagataatttatgtacaagtgatttcatttccttatgcttttatattcaattaaatatgtatggattaccagtagccattcgttcggaattataagaggacctaagatgggtgtgtcactcggtcaccgatatactccataagatcagaaaggtacgaaatgtaatttttattgatatatatttgtatatggaaactgcacatatcttatgggtgttttcgaatactcactcttgcaaatcattacaggttagttcgggtcaattggatttgtggtagggtggtgatgcgggttgctaagaggatcgcagaaacaaaaaataattttttcattaagtttgtctgccttcataattattgttgacttattttaagacatgtttactattacttttcagatatgattgctatgtttactttaaatttatgtctgccacggttattatttattaaagaattttattttgatatgccaaattaaagaaaaaaatgaatttttggtaatgctccagtgttatgaaaatttggggcgttgtagcttggtatcagagcacgatttgacttttctgtagacttgtttttgaaaaaaaaaattcaactacggaatagttcacgtgaacagtaaagatatttttttataaaaaaagctttgaaaaaaatgtgaatagtgaaaattactgttcatgatgaacagtacgtgaacagaacactgttcacgtgaacattaacaaaaaaaattgaactttatgtttatattttttttcttcttttctcatatttttgagagttaaatgtttgtgtttaagtcaattttgaatgataatagtttataatttaaattattatggcttcatgactatggttcaaattttacatgtgataaatttttatgcgttttaactttagcctttgggaatgttttaaaaatcgaccaatttgaaaattcatattctaagagatttcacattcaatttattgtttgaattttgctgaattgcgtaattgcaaaattgaaagtttttgtcaaaaaaacctaaattgtctaagaagagcttcgaatttaagcagtccgtctgtgacccccctcctcatttggaagccttttaattgtgcattattcaaatcgacgaggcgaaaaataatatttcaaacaaaaaaaattataaataattataattaaagtgaaagaaaaaatgaatagaattaggagtttaaaggataatgtaattttttttagtattaaacaaataatgttatgagaacatttgggacgtggcgctcaccatttgactactctccagttgatctcaggtatgaaatgaattctttccattcttaattttctagcagggtcatgagttatatttctacatgttatgaaatgtataagtatgatcacctcgcataatttaattgtcattttttttcatttgactagaatgacgtttatgcactgagaataaaataatattgataatgcaagattaagtataattgaaaattatacttgtcacatgattaggatgactatgtatagcccaacatacctccagcgtgctgaaatgaccattgaaaactacataaattatgaagtaagatgggaaggaacttttagttgaaatcttgaagagcaaattactatatttaaggatttggaaatttatatttttaaagttcttcgtttctacaacgattattaataatattaggttgttttatctaatattcctaaattaaaattttatttgtattaagaaaatgtcaagaaaacaataaaatcaagctacgaccatctgagatttgctaagggtggtacaagatttttgtaggcaacaagcacaggctggccccaacatcaggtgaattgtggaacagttccgtcattacaaacccccaaccttcgatggcaagggagacccactagcagctgaagaatggataagaggaatggaacgaatcttcaaacatctatcttgcactgatgctgaaaaggtgttatttgctgaattcatgttggttgatgttgtaggccactggtgggagtcatcatctcgtactagaacagaagcacaacaacgtactcttacttagacacaatttaaggatgaaatgatggaaaaatacttcccataagccttgaaggatcgaaaggaggcatagttcgttcaacttaggcaaggaaagatgaagctcaaagaatataagagaaaattcgaacaactctctaggtattcaccacatcttgtagatacggaagcaaagaaagcaaggagattcgaactgggattgcatccggagattgggagaataatggcatcccaccaattcaccacctatagtcaagttttgcaaactgcccaagtaatctcaaatatgttggaaatggaccaaactcccccagcaaggggccgagtcatcaagaaagagaggaatgggtccaacgaagagaaaggagaaggatagaacaagaaggctaacttcagatcaaattttggacaagtcattgcaccctgtccaaagtgtaacaaaatgcacagggctgaatgtctgtttggaaagcatgtctgctatcgatgtggcaaaacaagtcacgtctccaaaaattgcaaagaagtccccttgaagaagaatgatgagcaagaaaaaaagggaaaaggcccgagtttttgctttaacctaggaacagacaactggggacccgaacgtagaaaatttaaaggaggaaattcttttaaggaggggagattataatgccccgaaaattttagaataaaatttatatatattttatattcacattttaaatttgagaactaaaatgaaatatgttttaaattatattttatttgtcaaataattaaattttaatagagtgagtataaatatgtcaatattttactcgttggatgggttgtaattaattagaagtctttgactcgagaaaaagttagtttggataagaacacattaagttagacccaattgaaagaaaatgggataaatagaattttatgtaagttataattcaattcatcttctctctccaaaatgtgtgaggtgggtattgaattttgagtttatttttagtttaatattaacctattttaaatttgatgtgatagctagtatcctatttggataactatgaatttgtaattaaaatataatccaaatatctaaaccaggttttatgtacatgttttctattataactcaaccactttttattactataaatactatacaatggttccatatttcaccacaccaaaagttatgcacatgtgagagagagagagagggcactttttggaactagaagacaggaagccattttgcagccattgttcactaaagctttgaaaagattttgggcacataaattcaaatacgttttatatatttcaataacgaggtaaggtgaaagtgttttcgtttccttgtacttttatattcaattaaatatgcatggattactagtagacattcatttttttaaagagatataaaatcctacgggattataaaaagatctaagatgggtgtgtcacttgatcaccgatatactccatgagatcagaatggtatgaagtgtaatttttattgatatatatttgtatatgaaaactgcacgtatcttactaggtgttttcgaatactcactcttacaaattattctaggttagttcgggtcgattgaatttgtggtagggtggcgatgcgggctgctagaggatcgtagaaacaaagaataaatttttcattaagtttttttgcctttaaaattatttgttgacttattttaagacatgtttattgttatttttcaaatacgattgctatgtttactttaaatttatgaatgccgtagttattatttattaaataattttattatttttttttttgctataccaaattaaagaaaaaatgaatttttggtaacgctccggtgttatgaaaatttggggcgttacagatcttcttgaagacttctacgaatatggaaaattgcttatcaaatttcttctttgaaaacctccttggataatacagatgtggcttcaaaatggaaggattatctgggaatgagattgagttaaccgatttttattctttcttgcctctacctcaattttttgctcttcaactaatttttctccaacattatctgaagtagatgttggaaccacaatctcgtagcttgctttcttcaagctcttttttcactcttcaatgtggtggcattgcagcatgctcctttaggttaacctccgtgtcactaagaaattttcctttttgtttggaggttattgcagttgcgagttgatcaatctgtacttctaaattctttattatggctcccatataggtcatatgagtcttaatattgtcaaatctagattcatccttgttgaatttcgcccttgtatatgaaataaatgtccttaagatatcctccaatgatggctttccttcaaaagcctaattgttgaacctaggtggtagctgtagcatgttcacattataccataagaggggatctcgtgattttacagtcctagatgatagtggtttgctgagtaattacctctttgattgaagtttcttcaattcacatacagaacttgctcattctccttctcagactcatggtatgaaataaaagcaaccataataggatatgttttttcttagttttttgtgatgtcattgcaattatttgagttgtgagagatgacatttgagctataagggctgtaatgggatctatctcataaaaaccagcaactttttttgcagttgatcgctcaatttcctccagcaattaaaggaatatctgtagtcttaaacatcaaagtaccacctattgcagcattaactattgcccgtgtctgaccatacaatcattgtagaagatcactatctgcattcaattctcataacaatgttgaggtcatcttctaagtaattatttgaatctctcgcatgcctcaaagaatggtttgaagtctaattgttagaactggccaatcttactccgcaattgagctgacttggaatggggaaaacttttgtaagaaatttctgagctaaaccctccaaagcagtgatggatccatatggcaatgattgaaaccatgctttggctttatcaaatggatagaatctaattgcctcttttatgacaccattcatcttcacagtaactaattttcaaaaaagatgctagatgagcaataggatcatcttgtagagattcctcaagttgattttgttgcaccatatggatcaaccctggcttcaactcgaaattacttgcaactattgcatagcgtgcaatataggaataattttcattgaaaattggcctgacatagtctctaatagcccgctgctgattgttctgatttgctacttattgtgcttgttctgccattgcttcgagttcttttcgtctgataccccttaaaaatctgaaagttctttcgatttcaggataacgggtagtaatccaacacttctcaaccttcaataaacctaaaacatgaaccaagcaaactagttaaaactacagaaatctaaattaaaagaaaggctacttgacaataacggtagaaaaaatcaaataaaacaatcctcgataacagtaccaattacttgtaagtattttatacaacttaaattataccacaaatgaagggtgttaagttttgtaatatatgaaaggagttaaagtctcaaacccatagggattgtaatttaattttacaccaagtactaaaattgtgtagcctctatttttgacgcaacaggtctcgaatcaccctaaccaaccaagaacgtgatgtgcttcgatggtggatgccgactagatgctagatctaccagcaaggcttactttaagttactaatttatatgcgccacataagatgcttatgagaaaaaaataatacaataggcccaaaataattatttcgtacattatcaaaatgaatcatattactcaatatgtcgtgttatcgtgactttagatcatctagctcctcaagctattaagaaccaattgctacctctaagaaaatatgttgaaaaatatatgagttgatagcttagtgagtgaaaatttttgaaaatagtaatacattcttatttatacatatttatcaaaaattgagttcataccatgtatcagtctaaagtataacaacatataatactaataatcaagatgtgagagacctcatattggtgaaaatatcatctcatagtcatgatataatcatcaacgtaaatccatatcatcatctcatcacattacatgtaatctaccaaaaatgtaccctctgactgaaatctgtaatccatccctcgggttaagtactttcgtcacgggcttttggcctactctttgaatgaaaataggtccttctggtaattaattctagaacacggccaaggtttttttgtgaactatatgtacacggttaagaccaatgtccgatcaagacactttatgtcggatataaaaacggccaaggcccctctatgaaatagaagaagtatataatcatgggtacttttctaaccgatctcgatatcacacgtctcacatcctaattcacaattaattgatatacaatcttggaattccgcgtatatcatagtgaaagaacctttcaatattaatcatgtaattgaacaaataattcacatagttgcacgtaatataattgtataagtactttatcaatatttgaaaatatattagtttttccactcacagatccatagatagatatatggctaaattggagaaactttccaagcttcacatcactacccgaaataacaatataattactcaaatggatttccagcaaataatttctctacctctatatgtattcttgcatctctacttctataatttttcttttctttaattatttaccaacaaatcatcacacatgatcaaattcattaaatcactatactttcttaaaatcactaccttatacctatacaacccctatacatgatttaatccagtacatagacatcaatatttattatttagtttcatttaaaatagtaaatctaagaaaacatggatttgacaaaaacaacactaaaattccgaagtattgaagtctggcaccagtttctatatatcgaaaactatcactaaaaccaatggcaggaatagcactttctgggattaatttcaaaaatagtacctgtgtaggattttgtccgaaagttgcttataataattgcttaaaagtggaaaaatctacctcaattccttaaatttgttgtttgacatcatatgataacaagaagtcaaagaataagtatatatttcataaatccattttaaaagtttcattatatttttaatttcaatatttattttccccttctaaatccttgaatataagcaattatccataaaccttaaaatcaaatatcattcctaaataagttagcattttgctcacctctagaaattggagagcgccaactcaattagtgtttagccatcaattcccatctctaaacaggcctttcctttcttcttcttcttcttcttcatcttttattttttattttatatatatatatattttttaccaagatcatgtaaaaatttagcactgcatatccttcagtatttatatcataacttttcctcctaatatcagattgaggtgatcaaagaatgttggaaagacaacacaaagcactacaaattactttagatggggttttccaattcaaatgtacactacttcaaatatgggtctcatctccaactaaaaatctggaacgtacttgtgtggttgaaaattgatttatgcaaatatttcactcatttttgcttcatattgcatctcattgactcctaacactcttcaattatcattttgtggtccatatcaactattaaaatgctgcaattgagttctcaaactttgaatttcaccatttttcttcgttattcactcattactttcaatttagcctctaatcattaagcttcaccaaattaacgtaaacttttcttgattcaagccaatatcactcatttctccaaatgtcgcattattcatatcaattcacttaacctataaaacaacacaaaaacacaaatcaagacgatctaaaactttaagaatcaaatgaagtgtcaagattaagcaacattaatatgataagtgaaacacactcatcacttacttaattgatacttttacattatggcattctaaattcactgtcacgcatcttctacaatgcaatatataccataagtgtacggcgttaagttttgtaacatgagatcaagtacgaatgtggaacccacagggattgatgtttaatttctgccaagtactataattatgtagccttattttatcaagacaaatgaaatttggaatcaatggttttaacaaaaacatgatgaatatggtgacgaattgaacaaataaatgcaagttagaagaataatcaagatgagaaagcctatggttatgatttcacctaactatcaaatataattctcaattatataattatttataatcaattttccaaagtttataagcaagaactcaattttatttctattccctctctagagtggcggctagaaattaatcctagatttcaattccaatatgtctattccgaattaaaaccaagaatttattaaattagtggttttttatggtgtaagcttcatagattctatactttctcttgaaacccataaaatctacatttgtctatcttatgatcgtgcctaaattttcctctcaagtgttgaatattaacatctactcattcaattagtggtcaattaattgaaagcattaaaatcataacacaaataaacagaatggaaaatttcataaaaataactaaaataaattcaaattacactctcaagttttggctaatcaaaccctagattatatgtttagttcatgataaaagtcataaaaataatcaaattcaaatacacaatatagagaatagaatagattagctaaatctcaagcttagatgacgtctaaaatatgaatgaaatacacttatcaaacacccccaaacttaatactttgctagtcctcgagcaaacactaaacaaaaaactaactaacaaccacttaagcaaacaaatttaagaaaagaaaatacataaataaatttagtatgatagttttccttcatagctcatgattgaaaacatagtatcaattatggaccacatcaaagttgtaatgcaaaagctaaattttcacttatttaatgcaaaacgggtgtgtatatgaagagtcaagtacaacattgtataataataagttgatccaattcccgaccttaaaagtcaaatattttcttacttcacccatgggattcgtacacctccaaacttgttttattttcacttttcaaggtgtaatctaaggttgatgtataaatcactactccttaccctctcttgtttggttaaattttactaattgcagttcaacaagtcaacaaatgaggattctctttattttagactgcgtcaacctccaaaaatcaaccaagttactaaccccttgtcaaaagcctaatcctatcaaacaagtgttcgaggcttaatcgaggcatgtggtgcatcttctattttttatacaccagctttttcatatatatatatatatatatatatatatatatatatatatatatatgttctttattcaactttgtgtggacatctctccattaaactttctaaatgaccacggtagtgagctttaggcagatggggcatcaggttataaatactggcagacttaatcactcgagtcataaaggctatgaagagatattttacaatgagatcattatagtagttctcattgggatcttttaggatcgctttataatacgatagcttttttccttttacacaatgattagtgcaatgtcccttattaaaaactcattctttttttttgaaaatcgacctccaacttaagattttcacccaattttcatcctattggtctcaaatagtccacacaaaatttagtacatatgaaatccacatctacatccatgtctccctgcaacaattcaaccatccaaactatcctaaagttggttaagggatatgaattttgtttagtggtcgtttggatttggcatctaagttttctatttcaacctataaacatggatctgcctagtcatgtacaatgtcacaatcaactcatgtgtataaatattttccatttcacatgaataagcaaaaaaagttaaattaatcacataacttatccacaattcatagaccaatgatgtactcaattacatacaccaatgctagtaaggccatctaactcacataagcatgaaaaacaagtaatttaaaaaaataattgcatacaaatcatgcaaaataataaaaaaaatttaagcaattagacaatttttaatacatcccaaacataaactaaacattatccccaatgtaaaattaaagaaaaatgagggaaatttccctgaattgtttgcattgccgtgatgttttgatgcttatgatgctagatttgatggatgtttcttctatcttctcctcaaacttgagatttatcccatttcgtccttgttaatgttgatttgagtgtttcacgacgtcatgttccataaaaatcaattttcaaattaaatacatagaacaagggttacttagctcaaacatctaataacgaacttaattacttaaagatctaaagggagatggatgatgattcatcaataaactgtaaaaattaactaaattgtcttataattagaaaacataataaataaaagggaaaaaatattgggttacctcccaaaaagagcttctttaatgtcattagcttgactttggcaaatgatcatgggcattaaaagaaggctttggatgtcttgtctattgttcttcccttcccttcccttcccttggctttgctttactctttattattttattaaacctcgacattgtccttttcaatgtaataggatttttcaatgccatccaattcaaactcaacaatgtggacttcaacttcctcactggacttaattacaaaattaatttctaaacaattaatgaattcggacgaatgtacgttactttcatcttcattcggtttgtttgtgatcgagttgtcattcactttaagatcttcaacaatcgttgaaatttttttggattgactaatcgatctacattctagatctacgagcaatgagaagtctttttttaacccctacgagtggattgtatttctaccttttggattcattccaataactccaatctccagtacatattttacacttttccaacttgaaaagtttattatagtactttgtaattattctctcgttcaatagaggaagaccattttccacaagtatgatgttttcatcccaatcaataggtacacaatcttccaaaggcatgtagtcttcatcaaatttgtcaatcgctcctttctgacatcttaaatattgtatgaaccctaaggccctgtttgacccacgttctttcaagaaaatacattcttaaacagtggttaaacatcatttcaactatagattcttcaataaaataatattacattcaaatccaaaacttttccttattttttagccacacattttccataaatacactattcaaaaatgcattcttatgaaaataatgtggctcaaacaagggctaaaagttttactgtatggggatcgatgcatgcatgcaaacaatgatcagtgtaatacatcccttagcaaagatgataaaagaaatattcttcaagcttgtaatttgtatccatgtcaagattacttactctgattgttctgctttcttgccaatgtctgaatcatgcatatgctattatatattacttgaaaaaatatcaaagagatcggggtgggtagccaaaattaacaaaataaaagaaaatataaattaaaacaaaagctacttggtaatagtattagtaaaaatcaaataaaacaattcccgacaacgttccaaaaacttgtcacgggttttatataacatgatttataccacaagtgtacagtgtcaattttgtaatataagatcaagtactcaaacccatagggattgatatttaatttctaccaagtactattattgtgtagctcttattttatttatatgactgaaatatggaatcaatggttttaactaaattaacgtgatgaatgtaatgatgaatcaaacaaataaatgcaagttagaaaaataattgagataagaaaacctagggttatgattttacctaactatcaaatatgattctcaattatataattatttctaatcaattttccaaattttataggcaagaactaattgcatttctatccccccatctcaagtgctggctagaaatttatcttagatttcaattccaatatctatattttgaagtaagaccaagaatttattaagttcatggttttttatggtttaagctttataaattctacactttctctcgaaacccataaaatttacatcgtattaatcttatgatcgcacctgagtgtggagaattgactaacatctacatatacaattagtggccaactaagtgaaagcattaaaatcataacacaaatataaaggaatggaaaatttcatagaaataactaaaataaattcaaatcatacttccaaattttggctaattaaaccccaaattagatgtttagttgatgataaaagccataaaattaatcaaatttagataaacaatatggaaaagagaatagaaaaactagtttcgatagatcttcaatcttctttgtgatgttattcttgatttctcattgatttcttgatgattgcctaattcttgcctagttggattatttttgaattgtaagaattgtagggttgaattatccgtttttactcctccttctattgtatcctttgcccctttcaatttcatttttgactggttcaattcatgaagaaaataggtttttgatcatgtatttatagtatttttgaacttttggacgaattagggttcagttgggccaagaaaaaagtcaaaaaaaaatcctacacgatggcgcctcaacaacactatagcagcactagggccatgaattatgatgttttacagcatggtggacgccactgcgccagcttcaagttgaaagaagagactgcacagcctttagtatttttatcataactttttctccggatatgtgattgaggtaagtcaagatgcatttcaaagctaacttaaagggctacaattcttagttagatatcattttcaattttgatatttacaatgtcaaaaatgagtctcaatatgagactaaaaattcagagcataactttttcgggttggaaattgatgtgtaataataatttgattatatttgatctctttgacatcttttttcatccaattgacccttaatactctcaaatcttcatcgtcaggtttgacacaatttttaagtattttcactttggtcccaaactttggatctcttacaatttagtcattttcttcaaatttgccaacttttgcttattttcttcaatttcatcaaaatatatcacaacataaaaaaacacattaaaatactctaaaacttataggaattatcaaaatatcaagcttagatggtgtctaaagtacgaatgaaaaacactcatcaatcacataggtgttagtactatgaaaggaatgttaaattatgatatgatttcatataatacaaataaagcatttaaatgttaaacttgtatagtatctaaaatgataaagaagcctcgtcaaagtataaattggacttcacaaattttagaacttggtcacaaggataaatgtgaattgaatgggatgttaaatgtaacgccctgacccgtactaactggaatgtcactcgaacgattgtaccttagtctagacttagtattaatataacaatttagtttaattaactatacttttttttttggctaaatacataatgaattactataaaatttacttaagtattatatatttataattcgttctaacaacacaacacaacgtaatttaatatttgaaggaaacaaattcaaaaggtctatggagtgattttcatgcatgtacaattaacgttaacattttaggtagaaaatataaatatgttgttttacttctctttctcaaatggaaaatgttaaaaataaattcgtttatatagttatcaatctcgaaagttcacaagattttaacggatggtagcaaacttcttatattatgacatgtttaaaaatcagcttctgccggcaacatatgagatgttaaaatatttttcaaactccgctaacaataactaaagcaaagctgttttctttttctatcttgtatgacaagtgccaaaataagttagtttgcatagctattgactccaaaacttcatgaaattttaatgtaaagtaggagacttcttgtgataagatatatccaaaaattgactgccatcgacaacatatgcgttattaaaataatttttcaaaccttgcagagacttggttgaaaggtaaaccagtgctgttcacttaaaatgacgtataaaatctcatagacatcggaacaacatggtttcaactttattcagtagttaatccatgatactatcaaattccattagtttcatccaaaaattccaggtaacgattgacttatgaatttttgaaaccaagggcagaagctgaaaacagcaacactgtccagtgcaatttaattttttaagtaacatagaaaattctaccgacattggattgacataattccaagtttatgcagtagctaacccatgaggctgtcaaaagccactggtattttctaaaaattcctaatagtgattgagttatgaatttttaaaattaaggcagaagctgaaattttaaagaaacagcaacattaaatcgctaacaattttttattttttatttttttgttttttgtaaacgattttcgtgaattaatttccataacacatatctacttttaaacatagcttattcataaagaaatgttcatagaatagtccacacatgacatccataaaaatctatttaaaagaaagcgtaaacatttcaatattgaattaaagacattaaatcaccagcttctccatggcatgttacatctgtagcttccatcatctacgccctcaagcaaatcaaatcaacctgtaggaagggagttaactcttgacttaataactcaatagataacatcggtgttttcgtcatcaaattagataattttaactgcatatccataccgtcgcacgtagatggatttttggcaaaattcaatttctatagcattatcataacacgtggaaccggaaattatcattcaaattatagtattatcaaagcatcgtacccagagataccatttcattcaaacttttaatgaaaaatcgtatttcgaaaacgaaataacatttgaaaatctacctaccttgaatcgcataaaaagcctttgttcttcactgtaaagtcctaaattttcgtgaaatagaattaaatttttatatgttatattttaatattttgaaaagttagggactaagatgatacataacaaatttcaattttatttgggtcaaataattagattttgaccgagcaacaataagtatatgaatattgggctcgttggatagattgaaattagtgacgcatattagactcgagaaaaagttgatttggttaagcgatgcccaaattatcgaggtcaaaagatatggtgctaaatggttttaattaagttgaattaatgaatctataaattgggggggggggcacgtgtagtggtactaattgaataataataataaaaaaaaagttatatatatatatatatatatatatatatatatatatagagagagagagagagagagagagagatggatatatatatatattttatattttcacacgttacttttcctttgagtttttctctctcccactcaaattagccacctctaagaaacttccacatacctactacattttccccactacccaactaaaatgaaagattctccacattccttcatttatctcacgttcatacggtttcttcacttcaacaattaataacttccccatcctatatttattaatcattttcttctatatttttatttcactcaaacaagaaagactttgcagtaacatttatagagcattcttcatatctcaacatttttctttgggctgaaacgcatttgaaggttaagataggatacgacatgcaagtggttgtcccgtttaatttttgttatttcatattgataaatattttcgttaatgatatgaaatgatatgatatgacatatatggccatccggtacaaatgatatgatatgattgagctcttaccggttaaagatatgatatgatggtacgatttattttaatatatgaataataaacgttatttgggattgtacgaatatttgtatcttattgagtattccccatactcacccctttttccctaccttacaggttagtacgggttgtgttggagtgcggtggtttgatggtgtggtcgtgtctcgtctaaagaacaaggatctaaaatctagcacgtaacctcatttattttaatttagttgtcatggaaatttatttacaattaaatttactgtgcatgtttattttttacatggacgtgtttaaacttacatttttaattaaatatttgaattaaatttttgttttccctttactgctatttttcattaatggtaacaaatttttacatgtaattaattatgaatagaacgtaacatatgcatgtccgaaatctcgaatcagcaagaatgtggggaaattactcattttcaccagccactaataatagtccaattcatcttgctagccatccgttattttctgtgaacacttatgataatgtcaccttgatttgtattaattttaatgattagggtgctactgttgcctttcaaattgatttatggatatatccatgcatgacaaattaatgaagaccctataatgacgtgagattaggggagttgaggccatgtttcacttactggaggaaaagagaataaagtatgcttattactattattttaacaacagtaaggaaaattgcttaataacatttatgcatttttcttgctaaaatggaatcccttatatatttttcttcaaagttcatcataacatgatttttatttcacatgtttagatttctttaggttattgacaagggataacatcattataaacccatttatttttttaaagaaacatttggtagtgacttaagtttaaaaaaaaaataaataaaattgggtcgctacagtttggtatcagagcgtaggtataatttcctgtagactcacgagtattttcataatttggtttaaaaaaaaaaaatagacgtgaactcactgttcacggtttgaacagtgacagttcactgtttacgtgaacagtttaaattaaataaaaaaatgtgattgtttaaatagtttatgtgtgtatatatttatatacttactagaaatacctttcttataataaattttatgtttagccacaataatcactaaattacttagttactagatttttttttcaaatgtgtgaaattttataatagtccatgcactagtatatggtattttctagtagctaaaatctcgatgtaattccccatgtaaaaaaataaaaataaataaataaataaataaaataataataataataataataaatactaaataaataaattttgaagatatatatatatatatatatatatatatatatatatatatatatatatatatataaacactgaattttatacgttttaaatattaggtgtgataaaatgtttatttgtctcattgcgtagtatttgttaaaggttaacactttctgaagatttatgaatttaacaataatgacaatttaaaagtattaaatatatgaatggtctttggcactcaacgaccaccctctgacgactctaaggtatgtaaaaagggtaagaacatgaatacacttgggtgttttgcataacttatatattttaaatttcctacttctatatttttaagacatgcactttgtttctccactaaattgataaaatgtattatgaaaaaaaaaaggtataacgtgatagacttatgctgaaatgtgatcgtaacttcatattaattttaggaaatggcagcacctactcatacgaatttgatgcgcgatttactacgagcggtacaagagttgagcaggcaaaatcaagcacctccaccacaaaatgcaccaccacagcagaatgtactgcattttgcccctggagctgtctcagtggttgagcagtttcgtaggtacaagccttccactttcgatggtaattctgaaccactggttgtcgaagagtggataagaggtctggagcgcatatttcgacacattgcttgtacggatgcacagaaagtgttatgtacggaatttatgttgattggagcagctggtcactggtgggaatctatttcacgtacaaggacggaagagcagcagcgtaatctgacttgggagcagtttaaagatgaagtgatggcaaaatatttcccacaggctttgagggacttcaaggaatcagaatttctgcaactcagacaggaaacatgtcacttactgattacgagaggcaatttaagcagctctcaagatatgccccacacttggtggatactgaagttaagaagattaggaggttcaagaatggactgcgaccagagattggcatgatcattatgtcccgtcgttttacttcatatcgtgaaatgttggagagggcttatgctatttcatatcaaaggactacatttgaacactatgcccagcaaagcaaggaatcattggggaaaagaaagtggagtgatcagagtaagaacaaacgtatctggcagaataaaagagcaaacacaggagttcgtatcggtgggacgagtgaaagtgttacaccttgtcctaagtgtaataaatttcatcgaggtgaatgctttttcggaaagaacatgtgttttcggtgcggtaagctgggacatattgctttacactatacagagcctccacgaaagaaagatgatgatcaagataagaacccataaggaaaggcccgagttttcacactgaatcagcatgaggcggagcaggatccgaatgtgatagcaggtatttattaatatttattttaacatacctgcctatgttctttttacctaggagtaaatatcatttcatttctgtcctttagttgctagtctaacactctaattacaaaaaaaaaaaaaaaaaaggtattctattattatccaatgtgcctgcttacgtactttttgattctggggctaccaattcttttatatctgcatccttcgtcgctaggtccaactttgcatgtgttagaatgaataatgaattagaggttagcatcccgtcaggaaaaactctttgcacgaaccagatgactaaatctatgaagttagagattgatggaaaaatattggaagcagacttatacctcttggaaatgaaagatttcgatgttattttaggcatggattggttaggacttaatcatgcaaccattctatgtcacgaaaaagaagtgctatttcatagaccaggagaggaagggttccgtttctttggagcaaagttcaagtctccacctcgccttgtatcggctttacaagcggagaagatgttgagaaaggagtcatgccagggattcttggttaacatcatcggttctcaacatacaaaaatgactgttaacgatattaacatcgtgcgagactttgcagacgtattcccagaagaattgacaggcattgcatcagataggcaagtggaatttacaattgatttggttcctggagcagcaccagtatctaaggccccataccgaatggcaccgaaagaatttcaagaattgaagttgcaattagaggatttattggagaaaggttttactcgaccaagtgtatctccttggggagcgcctgtactttttgtcaagaagaaggatgggagtatgaggatgtgcatcaactaccaggaattgaaccatctgaccataaaaaataagtacccactaccaagaatagaagatttgtttgaccagttaaggggtgcttcagtgttttcaaagatcgatttgaggtcagggtatcatcaactgaaaatcagggcaagcgatataccaaaaattgctttcagaactcgttatgggcattatgaattcactgtcatgccttttggtttgaccaatgctccagctgtatttatggatctcatgaacagagtattccatcaatacttagatcaatttgtcatagtatttattgacgacatactcgtgtactccaaagataaaaagtagcatgaggaacaactccgagtagtacttgagactttgaggaaggagaaattatatgctaaattcaagaagtgtgaattttggcttgatcgcgtaggtttccttggtcacgtggttaccgcccaatgaatcgaagtagatcctgctaaagtggaagcagtaacaaattggccaaggccgaccagtgtgggtgaagttcgcagtttcttggggttggctggctattacagaagattcattgaaggtttctcaaaaatagcagggccaatgactcagttaacaagaaagggtgtgaagtttcagtggatggaaaaatgtgaaaaatgttttcaagaactcaagcagaggctagtctcggctcctgtattgatgatacctgaagattcagagggatttgtgatctatagcgatgcctccaagcagggtttgggttgtgtactgatgcaacatggaaaagtggttgcttatgcctcgagacagttgaagcagtatgaacaaaactatccaacacacgacttggagcttgcagcggtagttcacgccttaaagatatggcgtcattatctctatggtgcgaagtgtgaaatttatacagaccacaagagtcttaaatacttcttcacacagaaggaactgaatatgagacagagaagatggttggaactagtgaaagattatgattacacgattcattaccatccgggtaaggctaacgtagttgcagatgccctaagcagaaagacaggatcacagttaacagttctatccacagtgcataaacacttgataagggactttgagaaattgagattggaagttatcacaccagcgactcaaactacagcaagagtaagagcgtttatgattcggcctactcttcgggatcgaatcaaggaggcacaaaataaggatccatttctacagaagataaaggatgaggttggtacaaacaaacgtatgggatttgaaatgtctatagataacgcgctaactttcaaaggaaggttatgtgtacctaaagatgaaagtataagaaatgagatactggaagaggctcactctgccccgtattcagcacatccaggtggcacaaaaatgtatcgagatctctgagatacattttggtggagaaatatgaagagaggaattggtcagttcattgagaaatgtattatctgtcagcaggtcaaggtagaacaccaaagaccatcaggactactgaaaccgttggatattccagaatggaagtgggaacacataacggtggacttggtggtaggcctcccaaggacagcaaaaggtcacaatgctatctgggtagtggttgatcgtttgacgaagtcagcccattttctaccaatcaaggtaaacttcaacatggaacagtttgcacagctatacatcaaagagatagtcagattgcatggagttccagtcactatcatttcagatagagatccgaggttcacatctaaattttggaaaagtttgcagacagccatggggacaaaactgaagtttagcactgcttatcatcctcaaacagatggacaatcagaaagaactatccaaactctaaaagatatgttgagggcatgtgttttggatcttggaggtagttgggagacacacctgcctttagtggagtttgcttacaacaatagcttccaggccactataggtatggccccacataaagctctttacggtaggaagtgcagatcccctatccattgggatgaggtcgaagagaatagaattttgggtcccgaaatcagtgaacgaacagttgaggcagttgacaagattagagccaaaataaagacagcacaagatcgacaaaaatgttatgcgaatagtaggagaaaggatttggaatttagtgtgggtgacaaagttttccttaaagtagcacccatgaaaagtgtattgagatttggcaagaagggaaaattaagaccgtgatttattcgacctttcgagatccttgaaaggattggtgttgtggcttaccgacttgctttacctcctgaacttgcagtagtgcataacgtgttccatgtatcgatgctcagaaaatatattcatgatcccaatcatgtggtaagctatccgacattggacgtacaaaaaaatttatcatacgaagagatcccggtaatgattttggacagaaagatacatcaactcagaaatagagaagtccccctagtgaaggttcaatggcgaaatcatggacttgatgaatcaacatgggagaaggaaaacgagcttagaaccaagtatccagaattcttcgattaatcaaggtaaattttcgaggacgaaaatcatttaaggagggaagattgtaaagtcctaaattttcgtgaaatagaattaaatttttatatgttatattttaatattttgaaaagttagggactaagatgatacatagcaaatttcaattttatttgggtcaaataattagattttgaccgagcaacaataagtatatgaatattgggctcgttggatagattgaaattagtgacgcatattagactcaagaaaaagttgatttggttaagcgatgcccaaattatcgaggtcaaaagatatggtgctaaatggttttaattaagttgaattaatgattctataaattaagggggggcatgtgtagtggtactaattgaataataataataataaaatttatatatatatatagagagagagagagagatattttatattttcacacgttacttttcctttgagtttttctctctcccactcaaattagccacctctaagaaacttccacataactactacattttcccactacccaactaaaatgaaagattctccacattccttcatttatctcacgttcatatggtttcttcacttcaacaattattaacttccctatcctatatttattaatcattttcttctatatttttatttcactcaaacaagaaagactttgcagtaacatttatagagcattcttcatatctcaacatttttctttgggctgaaacgcatttgaaggttaaggtaggatacgacatgcaagttgttgtcccgtttaatttttgttatttcatattgataaatattttcgttaatgatatgaaatgatatgatatgacatatatggccatctggtacaaatgatatgatatgattgagctcttaccggttaaagatatgatatgacggtacgatttattttgatatatgaatgataaatgttatttgggattgtacgagtatttgtatcctactgagtattccccatactcaccccgttttccctaccttacaggttagtacgggtcgtgttggagtatggtggtttgatggtgtggtcgtgtctcgtctaaggaacaaggatctaaaatctagcacgtaacctcatttattttaatttagttgttatggaaatttatttacaattaaatttactgtgcatgtttattttttacatggacgtgtttaaacttacatttttaattaaatatttgaattaaattgtttggtttccctttactgctatttttcattaatggtgacaaatttttacatgtaattaattatgaatagaacgtaacataagcatgtccgaaatctcgaatctcattttcgccagccacttataatagtccaattcatcttgctagctatccgttattttctgtgaacacttatgataatgtcaccttgatttgtattaattttaatgattagggtgctactgctgcctttcaaattgatttatggatatatccatgcatgacaaattaatgaagaccctataatgacgtgagattaggggagttgaggccatgtttcacttacgggaggaaaagagaataaagtatgcttattactattattttaacaacagtaaggaaaattgcttaataacatttacgcatatttcttgctaaaatggaaccccttatatatttttcttcaaagttcatcataacatgatttttatttcacatgtttagatttctttaggttattgacaagggataacatcattataaacccatttatttttttaaagaaacatttggtagtgacttaagttttaaaaaaataataataataaattgggttgctacattcacacccttgctattcccttaaacttaacttgacataaaatatatttttgagaaaaaataagagtaaattcgaatttgaggagaggtgtagtgaaaaagtgacttttctcttcttgtaaccttcctttttaatgaaaaactaaatggttgagttgtattatcattaaatttgttaaatatagctttaactaagaatttaaagagtttttaagccataaaaaaataattcataaaaaaagttttataaaacatacacataatgaaaataaaggaaaatgaaccattcatatgttttgtaacctatctttatcaatgcccaataataaaataattatttcatccaattaacttgatataattgctcctaacgtgcaaaatggggagtttttaactaaaaaataattttgtaaaaatattttataaaaacatctacatggtgattcgaatctaggttgcctatatgaaatacatgtagatgaccatcgtagcaacctaactattcattaaatctttgtaatcaaatttacttaaacttaatctcttaaattgttgagcatttaattaacttatggcttgggctttcataatctaaaacgggttcagcttccataactcatttcttaaatgggctacatcaactaactttagaataaaaattcgggatcttacattcctcacacctaaaaaaaaaaaaaatttcgtcctcaaaattgccttccagtttgacaaagagagtcgggtatttgtctttaacttcttcttctcttttccaagtaggttcttctactgcatgattgttccattgcactttgaccagttgaattttcttgtttcgtaatctatgtaccttttgatctagtattttaatcgataattcctcataaaataaatctttctgtacccccagagattgataattgatcacgtgattagaatcatgcatatacttcctgataatcgttatatgaaacacgttgtggattgctgatagttcaggtggcaaagctaatcgataagccacattttcgaccctgtcaagtatttcaaaaggtccgatataacgagttcatagttttctttcttgtcgaacctgagtataccctttattggtgccactttaaaaagacttgatctccaacttgaaactccaagtcctttcttctggtatcttcatagctcttttgtctatcgtgtggtacctttttcctagtacggatcttattaacggcttcgactatcctttcaatgatctttggtcctgaaactctattttctctgactttatccaatggacaagcgacctacaacttctaccatagaaggcttcatatggtaccattccaatagttgcttagaaacttttattatatgtaaattccacaaaaggtagatactattcccaactgcctcttagatccaaaacataggcccttagcatatcttccaaagtttggatggtcctttcagactcaccatcagattgaggtgatacgctgtacttaaatgcaattttgttcccatagctccttgtaagcttttccaaaactttgacgtaaatctcatatctctattaaacacaatagctaggggacaccatgcattgttaaaatctctctaatgtacaactgtgccacctgatctagactgaatgctatttttattgtaagaaaatgagtggactttgttagacaatccactattaaccatatggcattatgtcctcttgctgactttggaaatcctgtcacaaagtccattacgatattctctcacttccattcgggtatgtccaatggatttaacaaccctgccggtctttgatgttccactttaactagttgacacactatgtattttaccacaaataagcatatacttcttttcatattcctccaccaaaatgtatctcgaaggtctcgatacattttcgtaccaccaggatgtgcggtgtatgggtgaaataagccttctccaatatctccttcctcaaaacttcatccttaggtacacaaatttttcttttaaacattagttcccgatccgaatctattccaaaatcttttctcttatcagtaccaatctcattcttaatcttctacaagaatgggtctttactcagtgcttctatgatctgatctctaagaataggttgaaccaccatagcaacgagctgtgacttgctctagtgtggtaaccatttcaattcgtaaattctccaaatctttgattaactccatctaagtaataggtaatgatgctagctatcccatcgactttctacttagagcatcagcaataatattagtcttacgaggatggtaatgaatagtacgatcataatcatttactagctccaaccatcatctctgtctcatattcagttccttatgtgtgaagaaatatttgagactcttataatacgtgtaaatgtcttactttcctccatataagtaatggcgccatacctttaatgcatgaactactattgcaagttttggatcatgcgttaggtagttctactcatgctgcttcaattgccttgacgcataggcaatcacttttccatactgcatcagtacacatcccataccttgtttggatgcattactatatgtaacaaaccctttcgagccttcaagtatcaataacatgggtgttgtaaccaatcattgctctagctcctgaaaactttgcttacacttttctgcccattgaaacattattcatttccttgtcaattaggtcattggtccagctattttatagaatccaactataaatcatcgataatatccagccaatcccagaaaactttgaacttcaccagcattagtcagtgtcttccaattagttattgtttctacctttcttggatctacttcaatctcttggggaataactacatgacggaggaatctagttcggtcaaggcaaaatttgcactttttaaatttggcatataacctttccttgtgcaatatttctagtgctattctaagatgtttcttatattgatctttattcttggagtatatcaaaatgtcatcaatgaagattatgacaaattgatccaaatactaatgaaatacacaattcattagatccatgaacactaccagagcatttgtcaactcgaatagcataattgtgaactcttaatatccataacgagttctgaaagctgtcttaggtatatcgcttgtcttaaccttcaattgatgatattctgatcataaatcaatcttggaaaacaccttagcctctttcaatcaatcaatcaaatcctcgattctcgggagaggatactattcttgatggtcaaacggttcaactccctatagtcgatacacatcctcatacttccatctttcttctttacaaacaacactagtgctcccatggggatgcacttagtcgattaaagttaatgtctaacaatccttgtagctaaatttttaactcttgaagttcttttggagccattttgtatggagccttagatattggtaccaatttgggaactatatctatcatgaattccacttatctatctagtggatactaggtaaatcttttgaaaacacgtctgtaaattcttgtaccactggtacgtccttaatctttaccgtcattgcatgttttcctcctcagatgttaactagaaacccttgagatgcttcttttctcaacattttctcgacttgtaaggtcgatactagttaaagatggggtttgttctttattccaaagaaacaaaattgttcttttacttgtttttgaaaagacacttcccttctccacaacgaatggttgcataattatatcctaaccaatccatgccctaaatcacatataagtctttcatctctatcacttacgaatcaaattctaatgttttccttcaatttcaagattcaggaacctagtgagctgatttgtgttcaatgttttgctcgtggaggtgctaacttctattctactctctgacttattacaagtaatactagatttagaaatgaaagaggtcaatacaaaagaacgagtagcttatgaatcaaacaatacatagcaagtatatcagatgtagaagtccgagaaataaaatgaaattagactattatgttgtgatgatctagtacaagcagcctagctcattcaagaaacaaattatggaagctcaacccatttcaaattttgaaagcccaaatcataagttaattaaaagcccaacaaattaagagattaagtttaagtaaattttattacaaatatttaatgaataattgggcagctacaatggttatctacgtggtatttcatatagacaaagcaggttcgaatcaccatccagatgtttttataaaacttttatgaattatacttttaggcttaaaaactcttcaaattattagttaaatacccaatttaacaaacttaataatattacaaccccccccccccaatttagtttttcattaaaaagaaatgttacaagaagtggaatgtcactttttcactacacccttcctaaaatccgaatttcctcttatttatctcaaaaagaaatatattttatttcaatttaagctaaggaaataacaagggtgagaagaagaaaggcttcctacacattttgttctttgatatccaagaaaattcaagataggtagaggtgcaagtgtttatttcgttttcaaattatgattttcgataaatgtttgaatgaaatggtactctgagtatgatgcttcggcactacaacagtttgaatgatcattctctgactctacgtgttatgataatgctatagtaattggattttggcagaaatccatctacgtgcgatggtatgaatttctagttcgaaatttttaatttgacaacgaaatgcactaatgatatctattcagtttcaaactcatgggttaattcccttcctacaggttgaatgaattttccttgggacatggatgatggtaaaggatgatgcgacatgccatggaaaagtcggtgatttaatatctttagttgattatgaaatgtttacgttttctttaaattagattcctatggatgtcgtgtgtggatctattatacgaacattctttatgaataaattatgtttgaaagtagatatgtgccataggaataaatttacaaatcaatgtttacaaaaaaagggggggtttagcgatttaaagttttgcggtcacataaaaaaacattcaggtactacctcgtctttaaaaatttatagcaccttcaatacttagcattttaatacaaatcggtggcaatggacggcttcataagttagctattgaatgaacttggaatcatgtcaatccgatgtcggtagaattttacatgttgtataaagtaaactgcactagtagagtcgccgttttttcagcctctgccttgacttcaaaaatccataactcgattgttacttgaaatttctggatgaaaccaattgaatttgatagtctcaaggattagctattgagtaaatttgaaatcatgtggttttaatgtttgtagaatttcacatgttattttaagtaaactgcaccggtttacatttcaacggggtcactactgagttttgaaaattattttaatatcatgccgatggaagctgattttttactatgtcatattagaaggagtttcctactttacgttaaaatttgattaagttccgaggttgatagctatgcaaactaatttattttgacaattaccatttaagacaaatactaaaacagcaacattactttttaagttttgtcaaaaattttacgtcagtagtcgttacatgcatgaaacccattctaaaaacatttttgaaatttttttcttttagtattgaattattgttttaaaaaaattcttcaattaaattctaaaataatttaatcttcatatcttccactaaaactatagtaaaaaaataataaaaaaaaaactaaaaaaattacgactaaagtatagttaatctcattacgtttcgatctatgcgggtcgggatgttatagcgtggtatcaaagcacaagtttaatcgattctgtagacttaatgtattttatttatgaagtgagaaaaatgaaacatttaaggcactccatggcatcttgcacccattagttgacctcatccgacgaatccaagggatggaataaaatattatgttccacttcatttttcgagcatgatttataaatcatttaagcttgaatctatgaaaatgcttttgatgtttagaatgaaatatattatgtaagttatattttgtttcaatatacatgaagaaatgttaattgctcattatattaaaacttcaggagcataatgtttaagttgatttcactaacaaagatgaaacataattggacacttatgtgacaaacatggttaggacttatcagaccactagaaaggccacagcttgtagagcagcattgaaccataggtccatcattctgtcctttgagaactacgtgactgacttatctcgtccacttgtttaacactacatgatatctacaagagatgtatgatagatgtagatgcaggattggagatcatgcatatcgaagctatgaataacctcatacgttcactcctacctcaatgaggaaacatgggagtcatggttagggatgagatgctagaaggtaaccctctagagcatctatatatgattgaatttggtatatattgcctaatccttttagacaggtggagtgagagcttagaacctttataccagatccttctagacaggtagagtgagagcttagaacctcaattgaagatagtaattgagcccaatgataaggttgagcccaagcccgagcccgagcccaagccccgtgccttagcttgaatcagacccagagaaagatcccaaatgggagcatgatgatgactttggtttggaattagagaatgatcatgagcatgaacctaaaccacagattgagatggacctagagtcaggacctgaggcaaaagactcctctgaggatgaacctccaccgaagaagattcgcaagattcatagggattaaaaatttagattccatttccttgtgatatcttttcctttatgttattgaaagtaaaaaagttatcaaactattgaatatcctgatttcaaagagtactaaataaaaaaaatctgatcaagttgagatcttttcaatttctagtgctggaaaatgaaattaatgtgagatattatatcttatctcttgagaaatgtctcgagcaaactagaataatttgataagggatctctaacaagcgattcaagatcttggcaagttgactcaaaatccagcaccacctacaccaccaggtcctattattctcccaattcatacctcgatggttgagttatttcaaagacattaacccccttccttcgatggatcatctggtccactagtagttgaagaatggcttcgtaagttagagcgaaattttcaagtcatagattgcacgggcgcccaaaaggtctagtgtgcggagtttatgtttattggtaatgtaagtcattagtcagatttgatgacccaaactaggactccggaacagcaattggcgttaacaggagaataattcaaggatgaagtgatagacaggtatttttctcagtctcttaagggatttcaaggagaacgaattcctttaactcaagcaaagtaatatgtccttgactgattatgagcaaaaatttgaccaactctcaaggtatgctccacacctagtggacatgaaaattaaaaagactcgaaagtttgaccaagggttaaatccagacctaagcattattcttatgttacatcgtttcacatcataccgtgagatgctggaacgagctcatgttatttggtatcaaaaggtaaatacagagcaataccatcaattgtacaaccaggaggacaaaggacaagttggaaagaaaaaatggaatgatcaagacaaagaacaaggcaaatggcaaaataaaaaggctaatactggacctagtgctagtaagggcatagtagctatagtagcgccatgtcctaagtgtggtaagccttatcatggggaatacttgtacgagaagaatgcctatttttagtgtggtaagtcaggacatattgctaaggattgtcctatatttgctcagaagaaggatgataacaatgatcagaacaagaagggggaaagcacaagtgttcacaatgactcagaatgatgcagaggagaactcaaatgtgatagcagtatattactaatatctgatacacctgcttatgtactgtttgattcaggagctactcattcttttgtatcaacatctttcattgataaatctaatattaattacaacaagtcaaagagtacactagaagttagcattttctcaggcagaacattgaacacagattagttcgctaggtcgatgaatcttcaaattgaggaaaaagtatttgaagaaaatttgtatgtgatagagataaaagactttgatatgattttgggcatggattggttaggatataattatgcaaccatttattgtagataaagggaagtgtcttttcagaaaccaggagaagaacaattttctttccttagaatgaagaccaaaccccacctctaactagtatcgacctcacaagctgagaaaatgttgagaaggaaacatctcaaggatttctagttaatatctctggagaaaaattggcaacggtaaagattgaggatgtaccagtggtacaagaatttatggatgtgtttccagaagatctacctggtattccaccagatagacaagtggaattcacaatatatttggttcccagagtggcaccagtatctaaagctccatacaggatggccccaaaagaactttaggagttgaaaattcagttacaagaactgttagacattggctttattcaaccaagtgtatcaccaaggggcgcaccggtattgtttataaagaagaaagatggaagtatgcagatgtgtattgactatcgggaattgaactgtttgaccatcaagaatagggatcatctcctaagagtcgaggatttgtttgatcaattgaaaggggctaaggtattttccaagatcgatttactatctggatatcatcaattgaagtttaaggaaagtgatatacctaagatagctttcagaactcgttatggacattacgagttcacagttatgccattcggattgacaaatgctccgatagtgtttatggatctgatgaatagagtatttcattagtatttggataaatttgttattgtcttcattgatgacattccaatttactccaatagtaaagatcaacatgaagaacatcttagaatagcattagaaacattgcataaggataagttataggccaaatttaaaaagtacgaattttatcttaaacgaattggattcctctgtcatgtagttactgcctaaggaattgaaatagatccggtaaaggtagaagtggtaactaattggaagacgccgactaatgctgatgaagttcgaagttttctgggattggctggatactatcaaagatttatagaaggattctccaaaatagctggaccaatgacacaattgacaaggaaaggagtaaagtttcaatggacagataagtgtaagcaaagctttcaagagctaaaacagcaattgattacagcacctgtattaaccatacctgagaattcagaagggtttgttatatatagtgatgcatccaaacaaggtttgggatctgtacagatgcagcatagaaaagtaattgcctatgtgtcaagataattgaagcaacatgagcagacctacccgacgcatgatctagaacttacagcggtggttcatgcattaaagatatggcgctattacttatatggagggaagtgtgacatttacacagatcataagagtcttaaatatttctttacacaaaaggaattcaatatgagatagagatgatggttggagttagtaaatgattatgattgtactattcattaccatcctggtaaggctaatgttgttgatgatgctttaagcacaaagtcgaagggatagtgggcatcattacctactattccgatggagttgatcaaagacttggaaaatttgcagaccaaagtgattactataccagaacaaatcactgctcatttaacaactttgatggttcaacccactcttagagattggatcatagaagcacggggtaaagacctatttttgtagaaaatcaagaacgagattggtactgataagagaaaggattttgaaatagcttctgatcaggcactaatgtttaaaggaagaatttgtgtacctagggatgaagttttaaggaaggagatataggaggaagctcattccaccccatataccgcacatcctagtggtacgaaaatgtatcgagaccttcgagatacattttggtggaggaacatgaaagggtataaactcatttttggcaaaatgcatagtgtgtcaacaagttaaagcagaacatcaaaaaccagcagggttattaaatccattggacatacttgaatggaagtggaaaaatatcccaatggactttgtggtaggattttcaaggtcagcaagaggacacaatgctatatgagtaatagtagatcttctaacaaagtccgctcattttcttcctgtaaaactggcgtttagtctagatcagttggcgcagttgtacattagagagattgtaagattgtatggtgtccttgtgtccattatgtctgatagagatccaagacttacgtcaaagtttttggaagagcttacaagaagctgtggggacattcaaactttggaagatatggtaaggcctgtgttctagatctaggagatagttgggaattgtatctacctttagtggaatttgcatataataacagtttccaagtaactattgaaatggcatcatatgaagctctttgtggtagaaagtatagatcacgtgttcattaggatgatgttggagaaaagagagtttcgtgatcaaagatcattgaaagaatagttgaagccattgataagatccgtaccaggataaaggctgctcaagatagacaaaagagctatacagatactaggagaaaagacttggaatttgaggttggagagaaagtttttcttaaggtggcaccaataaagggtgtacttaggtttggcaagaaagacaaactacgactttgttatattagaccttttgaaatacttgacagggtcgaaaatatggcttattgactggctttaccacctgaactatcagtcgttcacaacgtgtttcatatatcgatgatcaagaagtatgtgcatgaccctaattgcgtggtgaattatcaacccctggaagtacagaaagatttatcttaagaggaattatcaattaaaatactggatcaaaaggtacataaattacggaacaaggagattcaactggtcaaagtgcaatggaataatcatggagtagaagaatctacttgggaaagagaagaagaagtcaaagacaaatattcaacactctttgccaatccataaggtaaatttcgaggacaaaattttgtttaaagcgtaagagatgtagaagcctaagaaataaaatgaaattagcatattatgttgtgatgatctagcaccaccagcctagctcattcaagaaacaagttatggaagctcaacccatttaagatttgacagcccaaaccataagtcaattaaaatcccaacaaattaagagattttgtttaagtaaatttgattacaaagatttaatgaataactgggttattacaatggtcatctacatggtatttcatataggcaacccatgttcgaatcaccatgtagatgtttttataaaaactttatggattatctttttaggcttaaaaactcttcaaattcttagttaaagacccaatttaacaaacttaaagataatacaactccctccatttagtttttcattaaaaagaaaggttacaagaagtgaaaggtcactttttcactacacccctcctcaaatccgaatttcctcttatttctctcaaaaagaaatatatttcatgtcaatttaagctaagggtataacaaggatgagaagaagaaaggcttcctacatattttgttctttgatatccaagaaaattcaaggtaggtagaggtgcaagtgtttatttcgttttcaaattatgattgaatgaaatggtaccttcgggtacgatgtttcggcactacaatagtttgaatgatcattctccggctttaagtgttatgacaatgctatagtaattggatttagtcggaaattcatctacgtacgatggtatgaatttatagtttgaaatttttaatttgacaatgaaatgtaccaatgatatctattgagtttcaaactcataggttaattcccttcctacaggttgaatggattttccttggggtgtagatgattgtaaaggatgatgcggcatgctatggagaagccggtgatttaatatctttagttgattatgaaatgtttacattttctttaaattagattcctatggatgtcgtgtgtggatctattctatgaacatttgttatgaataaattatatttgaaagtagtatgtgccataggaataaatttacaaatcaccgtttacaaaaaaaggggttggcgatttaaagttttgctgtctcgttaaaaaaaattcagattctgcctcatttttaaaaattcataactccttcgttactgggaattttcatacaaaatcagtggcaatggatagcctcataagttatctattgaatgaacttagaatcatgtcaatcctatgtcggtagaattttatatgttgcattaaagtaaactgcactggtagaatcgccgtttttcctgcttcttccttgacttcaaaaattcataactcaaccattacttgaaatttatagataaaaccaattgaatttaatagtctcatggattagatactgatttaattttaaatcatgtggttttgatgtttttggaattttatatgttattttaagtgaactgcaccggtttacatttcaatcgggtcgctctgagttttgaaaaatattttaatacctcatatgatggcgatggaagctaatttttgaatatgtcatattataaggagtttcctactgtaaattaaaattttaggaagttttgaggtcgatagctatgcaaacaaatttattttgataattatcgtttgaaacaaaaactaaaacagcaacattactttttaagttttgtcaaaaatttcacaacaatagtcgttacatgcatggaacccattctaagaaaatttttaaaattgttttcttttagtattgaattattgtttaaaaaattcttcaattaaatactaaaatttaatgtttataccttccactaaaaatatagtaaaaaaaattacgactaaagtacagttaatctcgtgatatttcgatccatgcgggtcgggacgttacatcatatatcagtaaaatacctgctatcaacgtttgagttctcctctgcatcctattgagtcattgtaaaagctcacgcttttctctttttgttatgatcactgttatcatccttcttttgagtaaacatgggacaatccttagcaatatgtcctggcttaccacaccaaaaactacattcttcccatacaagcattcaccatgatgagacttaccacacttagggcaaggcgcaacagccgctacaatggccttactgtcactatatttgagataagcctactatttttccatttgccttttcctttgtcttgaccatttcattttctctttctaacttgccctttatcctacaggttgtacaattgatggtgttgcactacagttgccttctgataccaaatagtgtgagctcgttccagcatctaatggtatgatgtgaaggtacgtaacataagaatgatgcttaggtctgggtttaacccttgctcgaacctttgagtcttcttaatttttttgtcaaccaagtgtggagcataccttgagagttgatcgaattttagcctataatcagggataagacatgaaatgttgtgtttttcatccattaatacttgcacttttgtgattaatggatacttaaatgtatttagtatccttatatattgatttaggctgcaattggatggaagtcgtgaaagttgggagaaaagagtgaaaaaggaccgaaatggaagcaagttaaagtacagcgaccaagttgcaaataattcatagagaagacgagcaatggaatgaagattcaagagtattaggggtcaattgaatgagaaaagaagtcagagaataaatatagtcgaagcgttatcacatatcaactttcaggcgaaaaagttacgctctaaatttttagccactgtttgagacccatttttggcctagtaaacttgaaaattggaaatttttatcaaaattgtagcacttttcgttatcttttcaatacaatttgaatcaccttaatcagacatcaggagagaaaggtatatccaaattactgaaagctatctagtgaagaaaatgataaaatcttgcaatcgcacaccttgctttagagaacttgaagattgaaaatagttgttctatgtgatcataataatttgaaccacaaggtcgcatgttttatctttgacgcacgaattctggtttcctaatttgagtcaaacacctatggaaacaactcgggataagtcttttaaaccctaaaattgttagataacatagagaatgcccctaacccacttttctctctttttatgctctagatttatggtactaaactcttatgcttaatcaaaggagatggaagccttggtacaattataactgtaagatccacctggtttttattgtttaatttatatgtttagtattaaatattcttctgcatgtattcttatggttgttgtgttcaattgctaagatacatacaagcctattatcctccacaatctatagctaggttaaacatcaaatttttattgtttgataaatttaacttgtgaagcaattaggattaatgatttgccgctttggaaattatcgaatgttcggaagaatattcatctagcttaaatgcaaccacttttgcttgggttatctagttcgttgatttctctagttcataaagcaagtattgaattaaatcttcgtgcttgattgggattgttcgataattaggattaattagatcgcttgtttctaattaattaaaactaaggacaaatatgaaatcgttttgaatggaaaattattttcaacaatgaatactaaaactgtgaattgatgattatttgtggatcaatggcaggttattaatttctaatggtggatgttgacttagatcaaggtttgttttgctgatttcatccaatttattgattagtattgacattaattgtttttcttaagaattaattgtttcaaaatcaaaacccccattttagttaatctatcatagaaaataaactaatcactcttcatgggatcgacccttactttcgctactacattaattttaagaagtacaggttctaagttggagtgtctacgatagcacgcaccaaatttttgctcctttgccgaggagtgatttagtttatttttgtgtgttttattagtttcattagttcttgtttaaaaaaaatttatttatttggttttttttttttagtttagtttaggatatatatatatatatatatatatatatatatatatatatagctttcttaattgttcatgcccgtaactcggtcctctaaggaagacaaattgcagtttgatccatacattaaaagaacttatgtaggctgaggagtgacattcagaggaattttgaaggacacaatctcattcataccccctcgtttacaagttattctgattcagaaagagagggactcgtggttggaaatcaaactttgaaggagcttgtagctccaaacttgaactaacaacctctctgcataacctttcctactttagatgctctactacttttgaacttatatatggactaatacatcttttgcctacttttcatggtcttgcacatgaagatccctaaagaatctaaatgaatttcatgtggtttgcacaaatatgaaacccactagagtaattgaagagcaaatcaaattgagagcactttcattctctctgaaggactcagctaaggactggctctaccatataccatctagaagtgtcataacatggaaagaaatgaagatgatgttcttagaaaaatattttacagatttaaaagtagctaacgttcgaaagaagatctgttgcataaggtaggacaacagaaaatctttgcatgaatattaggaacagttcaagaaattatatgcaagttgcccccaccatcagattagcgaacaatttctcgttcaatatttctataaaggcattttacctcctgataggggtatgattgatgctgcaagtggaggagcttcggtagttaaaactcccaagggcccaaggatcttgattgcaaacatggtagccatctctcaacaatttggcactaggcttgatagtccatctaaaccagtcaatgaggtaaatatctcatccctcgaacaatagatttcgagtctaactactctgttcgacaaacagctatggtaatatgcaaacagtgaaggtgtgtggaatttgttcgatgacagagtatccaactgacatgtggccaactcttcaagaagaccccaatgaacaagttaatgcaatggatggccttcctatacaatctcaaaagagttatgatccctactttaacacctataaccaaggatggagggatcatcttaatcttagctacgggaatcaaaaagtgaattggcctatgcaacaaactacccaaatttccaggaaaataagcagtcatatcctcctagacaacaacaaggtcaaacttctaactctggtatatcttttgaagatattgttaagtctctggccattaatactttacaattgcaacaggagacaagggcaagcatttaaagtttggagaattggatggctcaaatggcaacagtaatcaaccagttgatgacccaaaactagaggaaattaccttctgaaatagctgtgaacccaggggaaaatgcaagtgcaattgtgttaaagagtgacaaaaaagttgaagcaccggtaaaggcagtctccatatcgtcagaacaaggaaaggaggaagataccattgtagacaaaggtactaccaaaggtgatactacaccaaaacgtgagttttcacttctttgtgagtataaactagtaccattttttcctcgggctttagcagaaatctaggaaagatgaaccaaattgtgaactttaagaaattttccatgaatgtgaggtaaatattccattgttatacaagttcctcggtatgctaaattattgaaagaattacacttaaaagaaaacagaaagtcaaagggtgtgagaaagtgaaagtttgggagaatgtctctgcagtcattcaaaggaaacttcttgcaaaaatgcaaggatcctagtatgtttactatcccttgcacgataggtgacactaagtttgaaaaggccatgctagatttaagagcttctataaatgtcatgccatattccatgtatgtttctttgaaattggggtctttagttaaaactggtatagtcatttaattagctgatagatcaaatgcccatcctatgggagtgattgaggatgtccttgtaaaggttagtgaattggatttttgctgaattttatgtgcttgacatggaaaatggtgatcaaactagtcttatcgtgttatgaaggtcattcttaaaaacatccaaaatgaaaatagatatatttagtggcatactaaccatggaacttgatggtgaaataattaaattcaatatttatgataccatgaaattacctagtgaagataatgttgtttactctattgatttgattgattgcatagtacacgatgtttttgaacttaacggaaagggtgaattggagggtgctattagtgatcatgctgaaaagaagagtggggaattgactttgagccatgaattacaaaaaactattgcaacactgaacagtctttcaaagttacaacaaacaggtaatgattcatatgctaatttaccagtttctaatgaaaaacctaccttctattttgcaggatcctactctagatttgaagcctctccctaatcacctttaatatgcattccttggagatggaaacacattgcccgtgatcatctcaaacgaactgaatgcagcacaaaaagaaaaactgatgcaggttctcaagaaacatcgcataactattggatggacaatcgcagacatcaaaggaatcagtccatcaacctgtatgcatcacattctgcttgaagaaggattaagatctagtagccaacctcaaaggagattgaacctacccatgatggacgtagtaaagcatgaaattctcatgcttttggatgttggaataatttatcctatctctgatagcagttgggtcagtcccattcaagtgattcctaaaaagactgggataactgtgatgaagaattaaaataatgaattggttaccaccagtgttcaaaatgggcggcgagtttgtatagattataggaaattaaatgttgtaacccgcaaagatcactttcatttaccttttattgatcaaatacttgaaaggttagttggtcattcttactattgctttcttgatggttattcaggttatttcccaattgcaattgttccggaggaccaagaaagacaacctttacatgccaatttggaacctttgcatatcgtcatttgccatttaacctttttaatgctctggccacttttcaacggtgtatggttagtgtatttttagattacattgggtatattacagaactctttatggataactttacagtttatggagactcatttgataactgtttgcataaccctgcactagtccttaaaagatgcatggaaaccaactttgtactaaattctgaaaaatgtcatttaattgttgaacaaggtatcattctaggacatgtcacttcatctaagcgtattgaggtagataaagccaaaattgatattattcaatgtctgccttgccccgctagtatgctgaaagtctgttatttctttggacatgcaggtttctactgcaagtttggacttctccaaaatatcattgtccttatgcaaattttcacaaatggatttggcttttgagtttgatgaggatttcaaaaagtcatttgatacactgaaggatctgttgatgtctgagccaattatccaaccttctgactggaacttttcctttaagataatgtgtaatgcaagtaactttgtaggagtagtgtgtgggtcaaagaattggaagtgcttcacacgtcatctactatacctctaagactctaaatgatgctcagagaaattactcaaagactgaaaaagaactcttagctattgtttttgcgttataaaaattttgtccacatttacttggtgctaaagtcattgtttatttagatcatgcagctttgcgttatttgatgacaaagaaggaagcaaaaccaagattaatatggtggatacttctcttgagtgaattcaacttgaagttcaagggtgaaagaggaacagagaacggtgttgctgatcatttgagctgtctagctcatgtgggtgatgaacttcaattgcacgaaaccttttatgatgagaaattattctttgcaagcacgacactaccttggtatgtagacattttaatttctctagggctcgaaaggacaagatgaagaaggacgtaaaatattatgtatgggataatccatacttgtgcaagcattgtgcaaatcaagtgattagaaggtgtattctggaaaatgaaattatccctatccccatcttctgtcattcttatgcctgtagaggacactttgtacccaaagatgacagcaagaaaagtgctaaaatgcgatttctactggacatccttatttcgagatacatatgccttctataagttatacgagaattgtcaaaagataggtaacatatcctagaaaaatgaaatgccacaattacccatacttttttgtgacatatttcatgtttggggcattgatttcatggggccatttcttgtatcttttgattttgcttatattttgcttaccgtggattatgtgtcaaaatggatggaagctatgtccaccagaactcatgattctaaagttgttgcagattttataaagtctaacatattctcctagtttgggattccaagagctctcatcagtgatcgtagcactcatttctataactgaacagtggaagctttgctgagaaaatatcatgtgacccacaaggtgtcaactacatatcacccacagactagtggacaagcagaagtatcaagtcgagaaatcaagtctatccttgaaaagatgatctgtccaagcagaaaagattggagtttatgcttagataacgctttatgggcatactagactgcatataagatgcctattggtatgtcaccttattggttagtatttggaaaaccatgccacctttcagtggagcttgaacataaagcttattgagctgtcaagagctttaacatgacgatggacgagagtggaaaacacaggaagtgacaacttcaagacttggaagaaattcgtaatgatgcctatgagagtaaaaaaatttacaaggaaaagacaaaggcattccattataagatgatttctagaaaagaatttgaagttggtcagaaagtcctcctacactaatcgtggcttcgactatttccaggtaaactacgttcccattggattggaccctttgttgttactaatgtttttcctcatagtgtagtagaaatccaaagcacagcaacttcaaaggtgttcaaggtgaatggccataggctcaagcctttctatgaaggttttccaggtagaggacgtgacaacattgaaactcagagatccaatttatgatgattaaggaagaaagcaataaggctagccaaagacaacaagcagaagcattgcttggaaggtaacccaaggggagttcattccttcacttttcattttcatttttgcatccatattttaggttaaatttgctctcttcttgacattttactttacatgggggacaatgtaaattttaagtgtgagagaacaaaattaattttttttaatttttttatttagatagtgcttccatctcacaattacttttcactagaaaatttttttttttttgaaagattgagggaaaagctctggttttaaatgatttttggttgcatgtactatcagctagatgtaattaaaatttgacggactcataatatgattgaattaatgatcttccaacttagagttaattagtttagttattttctttgaggatagtagtaactaaattttgtaaacaaaaagcctgtgaaattttgagccattagactgacacattcatacaagtctcactattttctttcatgagtgatttttttcatgaaattgcttctctagaacttgccttgattctcttcaaggccatattgatacacgcatgcatgaacatgattaaggccatctttgttgcataagttagccaccttagccaaatagtctacttttatttaatttttccctttattgaacccctttaagtcttataacattttcttttgtaaactcacattacaagctttaaacccaaaaaaacaatattcttacccaatctgtagagctagtggagtattgttcatcgttttgatacatatgggagtgcgaaagaaataagtgtggggtgtctaaaattttggtaggattatgtggtgtaatggaacgtgttctcaattaaaattcataagttccattattggtgataatttgaaaaaaaaaaaaaagcaatgatgataaaaaagataaaaaaaaaaaaaaaaaggaaaagaaggaaaagaagtgatgaagttatattcgtgattcctcctaacatcacaagaacgggttgggttgtgtgaaatagatgcacagaaactggtcttgtatattttatatatacatttgagcttggattaattcatagtttcaatggctttagagctatttacccaaatatttcccacctagaccgtaggccacgttagaacccgtgaaaaagaccttatgatttatgttatgcatttgatctaactggtggagaatgagaagatatgcaagcatatggtagatcatttccattggaataagcttgaacgaaacacttaccctttaaacacatactgctaataccccatgaggatctacatgtttggtttactccatctttatatgagaatgcttgctaattgagtataagttgtgtgagattgtctatttatgatgtgttatgtgttttgaagagattgatcgttctatgttaatagcattgcaaccttactatctttgtgaaagtcaatttggattttacttgaggacaagcaaaagctaagtgtgggggaatttgataagacttgaaatgtcgtgcttttcattcattaatacttacgcttttgtgattgattgatactaattgtacttagtacccttatattttgatttagattgcaattggatggaagccgtgaaagttgggagaaaatagtgaaaaaggaccaagatagaagcaagtgaaagttcaaagaccaagttgcaaataattcatagatgagactagcgatgaaatggagattcaagagtgttagggatcaatcgaatgaagaaagaattcaaagatatgaaatatagtcgaagtgttattgaatatcaactttcaagtgaaaaagttatgttccaaatttgtagcctcgattttagacccatttttgccataataaacctgcgaactggaaaaatcacctcaatcaaacatcaggagataaagttataaccaaaatacttaaagttgtctggcagagaaaatggtataaccctgcggtcgtacagtacaagaccatgcagtcgcacaccttgcttaagagaacttgagagctaaaagtagtttctctatacgaccacaaccatttgaactatgcaattcctcaactactagcgaccacatggctcatctctgaggcgcaaattttagttttctaatttgactcaatcacctatgaaaacaactcggggtacgtattttaaaccttaaaatcatcaaaacatagagaacacctccaacccacttttctctctttttgtgctctagatttatgatgtgtaattggactcttgtacttgatcgaaggagacggaagccttggaacgattataactatgagatcttcctggtttttattgtttaattcatatgtttagtattaaatatttttctgcatgtaattttatggttgttgtgcttaattgataggatacatactagtttattattctccaaaatctatagataagttaaacatcaaatccgtaattgtttgataaatttaacttgtaaagcaactagatttaatgatttgctgctttggaaattgtcaaatcttaggaaaaatatttatctaggttaaatgcagccgcatgtgcttgtgttatctagttcattaatttctctagttcataaggcatgttattgaattaaatcttcgcgcttgtcttgaattgttcgataattaggattaattagatcgctttttcaaataaattaatactaaggagaaataggaaatcgattcgaatgggaaattattttccacaatgaatgctaaaattgtgaattgatgattatttgtggatcaatgaccaggtataagtttccaatggtggatgtggacttagatcaagattcgttttattgattttatccaatttattgatttgcattgatattagttgtttttcttaagaattaattgtttcaaaatcaaaacccccattttagttaatacagcatagaaaataaactaatcactcttcgtgggatcaactcttactttcgctactacattaaatttaaggagtatagattttaatttggagtgtcagtgatagcacgcaccaattagtcagggacatactaccttgctttccttgaaatcctttagagagtgagaaaaatacttgtccatcacttcttccttgaatggtccccaagttaatgccaattgctgctccagggtcatagttcaggacatcgaatcgcaccagtgacttgtattaccggtaaacataaacttcgtacactggaccttttaggagtcaatgcaatctatgaatcaaaaaatttgttctaacttacgaagcaattcctcaactactagcggaccagatgctccatcgaaagtaggggacttatgccttcgaaataactcaactaccgaggcatgagtcgagagagtaataagagctaatggtatgggtagagctggattctgattcagcctgccaagatcttgaaccgcttgtaggagatcccttatcaaattgttctgatttgctcgagacattttcttagaaataagatataatatctctcattaacttcagttaccattactagaatacttggaaaaaaaagggaattatttttcaacttgactaggattattttatattattgttattattattatgtttgcagatgctagtatacgcttcgtatatgattgtcaaggtctaaggattcgtttacctcaaaatctaggtaagctcggatatcatctcctattgattaatatgattccttctccaagaattttgttatcattccttctccaagaattttgtcttttcttcgtcatttgtggctcaaaacattaagttctaacccaatacatgtcctttaaatatcaaatttttcttcaaattactttcttctttatatgaaagatatacataaagaaaaatgtaaaacatagcgaaacatggaaaacataactaatgaatcataacatttttcataataaagattttaactttgcttagctaaacgtacctaggtcgtattatgagattgactaatggatgcgaaatgccatgaagtaccttaaatatttcattttcccatctttaaatttcctatttgtactgaaactaatatatttttaaaaaaaaacaagtctagagaatcgactaaactcatgttttgatactacgctgtaacgccccaacctgtatggaccaaaacatcactcaaacaactgtaacttagtctagacttaatattaatataacaatttagtttaattaactatacttttttcttcttttttttttgcggaatacataatgaattactataaaatttacctaagtattatatatttatataatttattctaacaatacaacaaaacacaatttaatacttaaaagaaacaaattcaaaaggtctttggagtgattttcatgcatgtaccattgacgttaacgttttaggtagaaaatataaatatgttgtttgacttctctttctcaaatggaaaatgttaaaaataaattcatttacatagttattaatctcaaaacttcacaacattttaagggatggtagcaaacttcttatattatggaatatctaaaaatcggattccgccagcaacatttgagaagttaaaatatttttcaaacaccactaacaataaataaaacaaacctgttttctttttctatcttgtatggcaagtgccaaaataagttagtttgcatagctattgactccggaaacttcatgaaattttaaagtaaattaggaaactccttatgataagatatatccaaaaattgacttccgtcgacaacgtatgagttattaaaataatttttcaaaacctcgtaccgactcggttggaaggtgaaacaatgcagttcacttaaatgacataaaattccacagatatcaaaataacatgatttcaagtttatttagtagctaatcaaatcccattggattcatccaaagatttcaagtaacgattgagttatgaatttttgaaaccgagggcagaagctaaaaatagcaacactatcctgtgcagtttacttttaagtgacatataaaaatctaccaacatcgcagtaacatgattccaaatttattcaatagaaacctgtgaggttatcaatcgccactgttattttctaagaattctaaataacgattgagttatgaatttttaaaatcaaggcaaaagctaaaaatttaaagaaatagcaacattaaatcgctagtacttttttttttttttttgtaaacagtattttgtaagttaatttctataacacatatctacttttaaacataacttattcataaagaaatgttcatagaatatttccacatacaacgtccataaaaatctatccaaaagaaaacataaacatttcattattgaattaaagacattaaattaccggctttccaatggcatgtcgtatctccagctatcatcatctatgccccccaaacaaatcaaatcaacctataataagggaactaaccatggtttgaaactccatagatatcatcgttgcattttgttatcaaattagatgatttgaactatagattcataccgttgcacgtagatggatttttggcaaaatccaatatctatagcattatcataacacatagagtaggaaaatgatcattcaaactgtagtagtgccgaagcaccgtacctagaggtaccatttcattcaaactttaatgaaaaatcataattcaaaaatgaaataacacttgcacctctacctaccttgaattctgtgaaaagccttaatttttcacacccttgctatttttttaagcttaacttgatataaaatatatttttgagagaaaataagagtaaattcagatttgaggagagatgtggtgaaaaagtaactttcctattcttgtaactttcttttttaatgaaaaattaaatggaggagttgtgttatcattaattttgttgaattggatatttaactaagaatttaaagagtttttaagccataaaaaaaataattcatataaaaaagttttacaaaacatttacataatgaaataaaggaaaatgaaccaaggcattcatatgttttgtaacctatctttatcaatgcccaataataaaatgattatttgatccaattaacttgatataattgttcttaatgtgcaaaatgaggagtttttaactaaaaaataactttgtaaaaatattttataaaaacatctacattgtgatttaaacttggattgtctatatgaaataccatgtagatgatcattgtggcaaccaagttattcattaaatctttataatcaaatttacttaaacttatctattaaattgttggacttttaattaacttatggtttgagcttttataatcttaaatgatctgagcttccatagctcatttcttaaatgggctacatcaaccaacttaagaataaaaattcgggaccttactttaaataggggaagaaatatataattcagtatggataattatttaagatatacatgtctatttgatgaaatataagcatgaagcatttaacttgtttaaaatctataaaaatgaagatgaaaattaaaaactcttagaagtgatagaggtgatgaatatatttctaatgattttaattcattttgtaaacagcaaggcattatacgtcagtgttatgcatctagagaccccaaccaaatggtttgaatgaaagaaaaaatagaacattagtcaaaatgataaatgctatgttatcttatgctaagttgctatttaacatatgatgaagctttgttgagtgcattagaatcttgaatcgaattccttcaaaattcacaaaggtttctccttatgaattatgaaaattaaggaataaattatttcgctacatatgaacaagcagctaaaacaacattaattaagatattattcgcattaacatccatatgtgacatacatgttcatgaaataaatatcaaaatgacattctttaacgaggatcttgatgagaaggtttatatggaacaatagaaaggatttttctaccggcaatgaacataagaagtgcaagtgagtaaaatcgttatataattcgtatcctcaagttttggttgaccaaaccctagaaaattatttataagacatgaaatctatacaattcataaagaataatatgaagagaatgaggtaaaactattttttggatggttgaatcaatcttcgtcgccaagttgtctatttttttttattttttgaatctcgtcctcttcaattctctttcaaaagtggcctttaggttcgtatttagaaaaaattgtagccgaggtaccaaatctttcgtttattagcagacttgacccaaaccttttgtttgtgccacagaggtaccaaactttcaaaaaattcacacctagagtccaaattgatgaaaactattattaatcaaaaatcaaagatctgaccaattgttgactggttttcaaaggggcaaatgtgtaactttacattttcatacaaaaaaaaaattaaataaaagaattttaaaaatagtcatttctccactcacccccacccctcccctctccctttccaaaccaaaaactaggtatctaccgataaaatcaacaattggaatcttgctgactttctcatcctcaccggaagcctcactaaaatctcaaaagttaatttcaaatcctgcaactcattttccttactcatcaaaagacctctggccaccaaaacacgctgcaaccaaacactagttttctcgaggttttctggctatgtcacttttccaaagaaaagaaagaagagatagagaaatctgactgtgtcttcataaaaaaataagggtacgagaaaggtgaagaagagactgatggtggggagatatgatatgagtgtatttttcttttctttttcatcacaaacgagatggaaagagtttttagggcaagaattactatgatgtatctttgattcttttcttgttaattttcaccaagaatgaaccatcaaatctgattatcaccttcttcagaaaaccacccctattaattatttacagcttttcaactttctctctcctatttactatggtggcctcatctttcatcttaaataatgcccaactgcccttcttcttttccctcatacttggtgctaataatccaacctttgcctctgcacatgcctttcttttgtgtgggcgtgtgagtaattaatttcaatggtaatttggtgtgttcttaattaggtcatagcggtttatcaaagggtttctcatagaatttattggcaaactggtttctggttttgatgggggtggaaagtggggatgtgggggtgagtggagaagatgactagggttttttttttttttttggtgttttggtttttaatataattcttttatttttagttttctatatgaaaatgtaaagttacacatttgcccctttaaaaatcagtcaacaattagtcaggtctttgatttttggtcaataacaatcaaactaacagtttctgtcaatttggactctagatgcaaatttttttaaggtttggcatctccggtgtcacaaacgaaaggtttgggtgaagtctgctaataaatggaaggtttggtgccttggctacaatcttcccttatatttatagtatcttgaagtcttggaaaggcagggattagattgggccaagaaaagagtctaaaaaaatcaaagatctttttcttgtccagcgatgcactggcgccacaagcgcggagctgcaagctgcgatgctgttgaaaattcagcaacaattgcattgcagtgcccactttagggtaaacgttcagcactgcatatcattcaatatttatttaataacttttactcacactatcaaattgaggtgattcagagtgcgttggaaaaataaagcgctacagtttactttagataggtttttccaactcaaatgtttactatatcaaacataggtatcaatctccagctaaaaaacttgaacatactatgcggttgaaaactgatttgtgaaaatattttgatcatatttcgctcattttacttcaaattgcatcccattgactcttagcactcttcaattatcattttgtggttcaaatcaactgttaaaatattgcaactgagtactcaaactttggatttcaccaattttcagtgttattcactcattactttcaatttagcctccaatcattaagtttcaccaaattcacatcaacttttccttgattcatgccaaaatcacccatttctccaggtttcgcatattcacatcaatttacctaacctgtaaaatagtacaaaaatacaaatcaaaattatctaaaactttaagaatcaaacgaagtatcgagattaagcagcattaatatgatgactgaaacgaactcatcacttagttgatacttttacgttatggcaaggtaaattaggtcaccaaggtattagtactatgaaaggaatgttaaattatgatatgatttcatataatacaaacaatgcatataaatgtaaaacttgtacagaatataaaatggtaaataagcattatcaaagtgtacaacggacttcgcaaattttagaatttgttcacattgataaatgtgaatcgaatgggctgtttaataggggaggaaatatgtaatttattattagtatagataattatttaagatatacatatgtttatttgatgaaacataagcttgaagcatttagcttgtttaaaatcgaaaaaaataaagttgaaaatcacttaaacaagaaattgaaaacactgagaagtgatagaggcggtgaatatttatctaatgattttaatttattttgtaaacaacaaggcatagtacatcagtgttatgcatctagagcactcgaataaaatggtttgaatgaaagaaaaaattgagcattagtcaaaatgataaatgtcatattatcttatgttaagttgtcatttaatttatggtgaagctttgttgagtacatgtagaatcttgaatagaattccattaaaattcacaaaggtttctcattatgagtcatgaaaaatgaaggaataaattattttgatacatatgcacaagtagctaaaccaatatcaattaagatatttttcgcattaacattcacatatgaattacatgttcatcgaacgaatatcaaacggcattcttaaatgaggttcttgatgaggaggtttatatcaaacaatcgaaaggatttttctacccggtaatgcaagggagtaaaatcattatatggtcttaaataagcaccaaagaaatggcctaaaaattttgacttggcaataatttctttcggcttcatgcataatagtattaataaatattttatatatttacaatatgtgacaaatattttgtttttatttgtttatatgtcgatgacaaatatgttgtatttacactctctaattctcattgaacatttattaccagcaaaaaaataaaataaaataaaataaaggaagaaaaaaaaaagaatggttccttgcacgtgaatcaacctcccttctttctgcgctatttgtacagcaaccatgcaatatatatgattcttttatcttctcagttttctgtccatcaaaagcttctgaacccttacaagagaaaatagaagcgtggaggtcacgttttatactccactttcgaaagttcatcaaacttcataaactggggaaaacatgaaggaaagttgtctcgagagagagaatactggaaatgataatgtaagaagcgagggtgaaaaaaagtggaccaagatgagagagaagcagaggagatccatcaccaccaagatcttccaaggcctccgcaggcacggtggctaccgcctgtctcctcgtgctgatatcaaccaagtcctccgtcatcttgcccaagaagctggatggatcgtcgagcctgatggcaccacttaccgctccgccaccaacactaccaccatcagcagcgtatgtattttttcatgtcaccctgtactatgtccttcacgacattggggtcaagttactccactattgagaatccgttaacgttgatgctaagtgctataactttgtgaatagcgaggcagcatttaattattgtaaaagttgtgttgttactgattatacttctatttttagaatcttagacacctattactgtgttttatgttctctcggatgtaactaactcataaaagattaataacattatttaatttgtgtaaatttactttagtaacaagatagattctttggtttcattaaactgaagatttttatttatttatttattttttttttttttttttttttgccggtaccctttaccctcttattcccttcagctattgaaataaccccttattttttaccctacggttaccaaatattaacctttttaatgtatcgtaccacaaaattaacattacattgcaataataaaagcatctgaattcatacttagccacatcttttatcttttaatggtttaattatgtaattgccacacgtatttggctaagttaataattgacctgcctcacaattgtcggtcacacgcagaataaaactgctaataaattttttacatttttcctgacgtgctattttgtgctgcaatgtgcaaaacatgtatgtgctaagttgatttcgtttcgacagggaattaatgtttgtcctctttgtgctcgaggaagaaaacgggctatgccagtgccaaccagcagcttcaagggagccaatgccggcattggtgctgtcaccaatgatgatggcagtgaatgtctgacggtggcctccccttgccacataggtcccacaaccctccatcactcctcctttagcctacccttttgtggtggattcagctcgagtaatactactattgctgcaactgctagttcttcttcttgtccatcgcattgtacagatgcagttagggctgctttcacttgtggatcgcttcacaggccctccacctatgatgccaccacttccagtcaggacacgcccgtgggatggcctcaatccctcacttaaatttcttaagccaggcacctcttaactacttgcacaagtactttcatgcttttcatgttatggttttacatgtaagacatattatttgacttcagtgtgactaaatattctagaatcttgggaacgtaaagtagccaatcctatatatctggattgcaagttttatgcactaggttcaatcaattttgggcataaacatttttaatatgattaatgcatttcgtttatggcagaactattatttaattgaattattattctcacgaattaatctaatagagtccatagattcaagtcttaataacttgttaatcacgaggagttgtgattgtgagaaaaacaaagtacatatgattttatcataaattatcagtggttgtaaataataatgagatatgaatatcattattacaaataaaccattaagtgcgacatttcttacttataaagaatagatgatctcacaagctaaaatgtagtaacatttaaatggatacatggatgtttttttaagagagcaaaacattggaaacatcgtgaagagattccacatggataattgtttgagtgtcgggggttaaatatttaatgtttggtattggaattgatcttttgacttgaggtcattatagtactttatctaaagacaatcatacttagatgatatcagatgttgctctggcaaaattttccaatacgatattgttcgtgtatgttaataattatatggagtctgtaaatgatcaatggaaaatttgtcactcttagttgatatcgaaatccttggacaatgtaaattaattagttgaaaagagtttcgacatttattgaatttagagtggggtgaagatatgattgataatggagattaacacactttcatatctcataattaattggatcatattaacgaagttattatagtttcatgataaacaaagaagttttgattttgtcacaccactcgatatttttcgtcacatcaattatccttacatgtaaatatcaagtagggacgatgaatgattgattggattggatcatattaacaatattattatagtttcatgataaacaaacgagttttgatattgtcacaccacatgatatttctcattatatttattgtctttacacattgtgaatatcaattagggacgacgaatgttaaattaaaagggagttttaattcattttgtttttattagatcaaaataataattaatgtcgtccgatatcgtcatcatgaacctaatgggccatacacaaaaagggaactagaagaatgatattatgaattatttaatttataagtgttgcacatttgtataattaattaattaattaattagattgtttattaatatgcttaagctaattgatttgattaattatcttatggaccaagtttaactaattagattaattaaatattgagctaacttatgttcaatagatgggataaatttacttaaatatccataaataaataattagggtttgagtttttcgtaagttatcacaatagcaattaaaattgctattgcaatttaacacacatctcacactatcatgatcgtcctagcacaagaaagagaaattctaatctcacattcttgttctcatgtgtggaaagatcgtgatagatcaagattcacaaaaaggagcaaagatcgcaattgttcatgaccaagattctcaaaggagattgagggtttaccaaaagtataattccaatcatgatttctagttaaatacaaagacgattgttgaagggaattgaaattattttttaatttcactatgcgaatatatgtaaattctaatagtggtattagagctgactttgtctttgttagaaattgtttttgaaatttgggaacggataagtagccaatcctatatatatggatagcgtatttttaatcgcaaacatcacataaaacatatattttgcttcctccaatatttactctcctcttagttgatctttttttttttcctcgatattctgatttatccccttcttgaattcatagtgctgaaaataagaaaagttggagaaagaagagagaagtgaagaatatttgcttattttcaggtgtgtttaaactatacaagaagcctttccttttataggagaaggatgagacaacaaaatgctctatcaaaaatgagatttaaactgatgaataaaatatgaaaagataacaaaattagttagaagtcagctaatcaatagatgtcattagcaaacagacttcaccattcccaagggtttagtaaacatctataaataggtagagtcaaaggaaggattaggcatgaaaaatatgaatagttttgtcccaaatagtcatttctcctcttgctccttccagagaatcaagttagtgagcttaggagggaaaaatcctagttatgtgagaagaatcatttagaagtcaagaaatttatgtcatttgcggaaactagatcaaagataaccacgatctcattgtatggagtgggaattgttcgctaaaaatacatgctgcaagtgcaccggtcgcgttaaagtaataaagtggatcttttgagtccaggttgtcgatccctcgaagatgtttaatttagattacacaactctaattaatttaattctaacaataaaaataaacacacacaattaaaaatatggttttgaaataaggaaattaactaaaaacctacaaaataagaaaatataaaaatcttgaaaatttcataagacaacgtggttgggatttatggtttcgtttaactgtcacctaattaatttctctacgagttaattaacaaactacttatgtattatgttagacccgatcttccaattttagttcattacctctctcgagcgaaattaaccctaattgatatgtttaacctactatatctgtatgtcgatttaaaccaaataatcgaattaaatctttgtgaaaatagctcattgggtcacctagggcaaggagtatatctttataccctacacaaacctaaagtttctaccatttggtctaaaatgcacaatattctttcaaatgatgtataactcactaaacacaatcattcattggccatataaatgaaaatgcatgaaatagaatcgtaaaaatacatgaaaataaacaaattaatatcaaagggcaaatattaaaatcaatcaagctagattaaactacaaccataaatcccacgacaattaacttagcccattttatacaaatgataaaaaagagaatattttgtacaatacattgcaaataggaaacaataatgaagaaaatacaagagtgaagataaaacccttttggatttgaattcttgatagcttgatcatgatttttcacaaaatttctcttccaaatatattctccttgtgctcttagattttgcccccaaaattatcgagaaaaagaaaaagaaaaagaaacagagaagaaagaaaaattaaaaggaaagtaaaaagaaagagaaggatgctagggttttccttccaagttgaagaataatggaaaaaatggttgaatttgcctttaaaagggcccaaaaatcgtgtttggttgctttcaaaatggtccccaattaaaaaaaatctagccaaacaggtcctagttcgtagctgcgatgacttgaagtggcgttgcagcgccatggctctataattgggcagcattgtagcgctgcggcgttgctacagtgccacctcccatttttcattatttgcaccccatatttgcactctagatatcttaactttgaacttgcacaaatttgatcctcgaattttgacttttctttcaatgtcaccctccaaaaattgcaatctgaagtccttgaactttcaatacttatgcaatttggtccccaacttcacgattttgtatggtcactttttactccatttgcattgttcttttaccttgattgatttttggcctgcaaaagtaaatgttacttaattgtgagtagaatttctttcatttcatcaataataatcatatttagatactaaacaagtgtaaaaacacacttatcaaatacccctgagctgaacttattgctcgtcccgagcaagattatctacaacataatcaagaatatctgatattgatcaacacattagataacttgcctaaaatatcaaagagtgtaaaattgtataatcaattcacaaatatgctccaaataatgctaacaaaaataatttgagcttatccaatgttcgattggtgtgtatgtgtgtaacgtcactttaaccattatttaaactaggaaaaagttgtcaagacgaaaaaatcttcaaattggctccaacctgacccattgtgatcaaatatttcctttcccactcatgagattcacactcctcaaatagctattcattttctttccttgggggtgtaaatctaaaggttgttcttagtcacgcatttctttttccgctcaagtttggtttgatctaactggcaatctcaacatctagtcatatgataattcttcactaatgagagcttccacattcaagctcatactaagtaattcaaactcactagttatcaaagcccaaatatcaaatacaatttcataaaaatatttttttttaagtcaaatcccatgttttaccttattcccttaagctttcttcttgacccttgtagtgagctttaggtcaataattctttggttgtttaggccaaagggtgccgagttttaagataccgctacggacttaataattcgagtaaaaaagcctacgaaagtgaggcccaagattcaacaagtgcaataacatttttttttattttttttttaagcacaacaaaaatgggacttagatccctagtatgtagtcattacctagcatggaatcacacactcctagataatatccttcactgactcgaccaccccaaacttgtctcacaatttggttaaatgaaagatgagagagtataggttgatataaatttttaagcaattcacaacctagtacttaccacttcaaaattctctccatcaatcaaaaattttccacatctagataaaaattaatcatgacatttgtgctcaaagtaattcaaggtcttacaatggataagcaattttttgaaaaaataaaaataaaataaaaaataaagagccccaaatagcataattggtcatgcatagctcatgaatcaataacaattttaaacatcaaaaccatgctaagccggtcaggctatctaacaagtcaacactatcgccaatttaagcacaatcacccccaaacttaaatcacacattgtcctcaatgtgtaaagaacaatatgaagaaaagaggagagggacaatgaaactttcccagttgtatatttgtgaagaggtaccaatgcttgacttggacttgtgatgctttcaatgactttggaaagtgaccttcttgtacacaatttgcccccaaacttgtgaggaaccatgtatatgtggtgcttcaaaaatttcctacaaaaaaatttatagctaattaaacaaaaggataaaaagtgcctcacaataagcacttttttataggctttagttcaactttggccatcgaatcacaggcatcaaaagaaggatttggatgccttgcccatttttcttcgtttggctttgttacactattcatttgatctccaaacctcgacatcgcccctttcaatgtgtaggactttaccattctatcctatacaaactcaacaatgtagatttctatctcctcatcagacttaatcaaaaaatcaattcctatgcaatcaatgaagtcgagtgaatgtatgttgattttatcttcattgattcctacatccttgatcagttcatttctgattaaattatcattcactttaagcccttctacaaccgttgatatttcttcggattgaatgatcaatccacaatttaaatcaacgggcagtgaaaagtcggtcccattgactccttcaagtggattgtaccccattgttgaaatccttcccaatacatgtaatcttccataagcataccactttcatccaacaaggcaagttttttggaatattttgcaagtaccatctcgttcaataggggaggcccatctcccacaagcttgatgtcctcatcccaattgtaaggtaccaaatctcccgcgagcatgtacccttcatcatttttgtcaatggattgttttcaacacctcaaatattttctaaacctcgaaagttttggcttgtataaactagtgtgtgaaaacaagcaattcccattacaatgcaccgcgtaccaattttcacaacttggatattcttcaaccatatcttgactgtgcacatagagatttgtcattgcaacaattttgtttctttaccaaagttagaatcctccaaatatttgaaaagtaaaatgagagaatacaagcacaagatagattaacaatatggaggctagccaaaatatacaaaaataaaagcaattaaaaacaaataaaaagaaattgttaaaattaaaattaactaaagtggtaatcaaagttaaaacattcctcagcaacagtgcccaaatctggttcgctaaaaatacatgccgcaagtgcaagggtcgcattcaagtaataaagtggacattttgagtccaggttgtcgatctttcgagaatgtttactttagattacacaactctaattaatttaattctaacaataaaaataaacatacacaattaaaaatatggttttgaaataaggaaattaactaaaaacctaaaaaataagaaaatgtaaaaatcttgaaaatttcgaaagacaacgtggttaagattcatgctttcgcttaaccgtcacctaattaatttctctacaagccaattaacgaattactcatttactacgttagacctgattttccaattttagttaattacctctctcgagcgaaattaaccctaattgatttgtttaacctactatatcgctatgtcgatttaaaccaaacaatcgcattaaatctttgtgaaaatagctcattgggtcacctagggttagggtatatctctatcccctatacaaacctagggtttctaccattttgtctaaaatgcacaaaattctctcaaacgatatgcaattcactaaacgcaatcattcattggtcatataaatgaaaatgtatgaaatacaataatagaaacacatgaaaataagcaaattaatatcaaagggcaaatattaaaatcaatcgaggctagattaaacaacaaccataaatcccaccacgattaacttagcctatttcatacaaatgataaaaaggagaatatattgtacaatacattgcaaataggaaacaataatgaagaaaatacaatggtacctcctttagttttattgatatgccctcacttgtggcagatgaataccgtggttacatgtgagattgaaaacaatgcaagcagtaaatgagaaagtactacttcccttacaattaattttacatagaataaattgaaagcagtaaatatggaagtactactcccattacaatacgatctaatacaagcaaaaataaaagataagaaatcaaaatcttaatgtctaaaatgaggtaaatcccagcaattagtacgcaaaataccacgtagagatatcggtacatggtctatagtagcataatccacagagtttccaaatgaagcttccttagaaagaaaatctgttgttgtattggcctcttggtatacacagttaaccgtgctattcaacacacgcaagagggccataatgtcatcccaaatttctcggaggcgccacaaagggtatgttccttgctttgtccattgaactaaaaccttggagttcgattccaccgtgacattctgtaaactaaggtctctacatggacgcaatccatcctcgagagctctaacttccgctaccatatttgttgtgatcctataataccatgcgtaacctgctttgaactgcccttttgcatctcgtattattcgacctcctccagatgacctggggttccttttgctactccatccacgttcagtttcataatctgatttggtggtttcctccaagctaccatttgtacacgattatgtttaatggaagcaatcgggcaattaagtgaatttagacaccagacatcactatctgaagttctcttcacattggagataacgcttgcgcattgagacaagtacgtttttaccatctatataactttcttccagtgaatgactagtccttccatacgtgctttgcatctagttttccatagagcccaagtaatcgtaaatggtgcaataacgcataaaatgccaatctgtaaggtagaagatgcctttgacccccatagattcatcctatttttccaagaatggacatacgacaaagcaagagtaagatgaagttcaaaataatcccatacctttttggccagttctccagtacacaacacatggttcaagagtctcaactaaaggagccgtacaacaatcacatttagaagccaatggtatcccaatggtttgaaccacttcatctattggaatgcaatttatgtttgttctccatgtgataaaagacatcattttttggaatttttaagtagcataaccactttctccaatggcatggtgtccccttttttcgaatcaattcccatgcttgggaggttgcatatgtaagagtcatgtccttcacgaataaaaatcccagaattctctatctcttccgcaaccttttccccagcaagttcacgtagcccattccaacaaccattcgtgaaaagatcacatactgtcaaattctggtttgttgccataaggcttgcataaataagatccctctcacccatccaattgtcataccaaaagctagaggagccatcatgtatacaaaccaatgggttctctaatatcaatggcatcacgacactactcccttccaaaattgagaatgtaaaggggatgatttcattttgaaaatagatttcttcctcgagtatttggctataaacaaatcagcctagaaagatcctccttgtaataatttccagcttactcgcatgtgcctagtaggttaccaccaattcgaggcattaagaaccaaatcgaccagcttatcggagcaatctcgagaagacaaaggagcttaagaggcaagttgaggagttaatgagcaagggttatgtcagggagagcatgagtccatgtgctgtaccagttctgttagtgctaaagaaagatggaacatagaggatatgcatggattgcagagccgtcaataacatattggtaaagtatcgtcacctattcctagggttagatgatatgcttgatgaattatatagtgcattcatatttagtaaaattgatcttaagagtggttaccaccaaattagaatgagggaaattcatgagtggaaaactgcatttaagactaaatacggactgtatgagtggttggtaatgccatttgaactcaccaacgcaccaagcactttcatacgtttgatgaatcatgttttgtgtgattttataggaaaatttgtcgtggtgtattttgatgatattctagtgtatagcaaaaacctaaatgagtatgtagagcatttaagaaaagtgcttgtggcaactatatgctaattttaagaaatgtacattttgcatggaaaaagttgtctttctaagatttgtggttagtgccaatggaatagaggttgatgatgaaaagataaaagctattaaggagtgacctatacctaagagtataaccgaagtaaggagttttcatgagttggctagtttcaataggcaatttgtgaaagattttagcacaatcaccacgccactcattgaggtagtaaagaagagcgtgggttttcgttggggtagtgagcaggagcagtcatttaatacatttaaagatcaattatgtaaagcacatattttagcgttacctaattttgaaaaaatgttcgagattgagtgtgatgtctcaggaatagggattggagcagtattgatgcaggacaggaggccaatagtttattttagtgagaagctgagtggagcagctcttaactgccttacgtatgacaaggggttgtactggcttcttcgagctttggagacttggtagcattacttgtgtcctaaagagtttgcaatacacactgatcatgagtctcttaaacattttcggtgtcaaggaaaactgaacaagaggcatgtaaggtggatggaatttacagaaacattctcctacgtcattcgctataagcaaggtaaagataatgtagtggtagatgctttgtctcacaggtatgtgttactatcttatcttagttctaaattacttggttttgagcacattaaaaatatgcatgtgaatgacttggatttttatgatgtgtataaatcatgtgataagggggctatagacaagttcttcagacataaaggctacttgtttcgtgaaaataagttttgtaatcctaagtgttcgatgggacactttggggttaagaaaactttagaaatgttagaggagcattttgattggcctaagatgaaaagtgacgttgaacggatatgtagccaatgcataacttgtaatggggctaaatctaaggttttacctcaagggttgtacacatcgttacctactcctagtgaacctcgagttgatatttcaatagattttgtgttgggtttacctaggactaagaaaagatgggattctacttttgtggtggtagataggtttagtaagatggtgcatttcataccgtgtcataaaattgatgacaccctcacatagcagatttgttctttaaagagatagtgtgtttgcatgggacccctaggagtatcctgtcaaatagggatgtaaaatttttgagtcgtttttggcgggttttgtggggtaagttaggtacgaaattgttattttccacaaaatgtcatacacaaaccgatgggcaaactgaggtggtcaataggaccatgactcaattattatgcactgtgataaataaaaatttaaagagttgggaggagtgcctaccttttgttgaatttgcatataatagagctgtacattctattacttcgttctcaccttttgaaatcgtttataggtttaacccactagctcccttggatttgttacctttacctgtaaatgaacgaggtaacctggatggaaagagaaaagctaagttggtgaagtcactctacgagaagttcaaaatgcaaattgaagaaatgagtaagcttattgcatcaatggcaaaaaaaggaaaaaagtgcatgacaattgaactaggtgattggtctgggtacatttcaaaaatgagcattttccagagcagagaaagtctaaattgcagccacggggagatggtccatttcaagacatcgaaaagatcaacgataacgcatacaaagtggttttttaggtgagtataatgtttcagctacatttaatgtgtctgatctctctcttttttatacaggtgcagatttgaggacaaatccttttgaaaagaaaagagatgatatgatccaagatgcggaagtcacaaaggcaagtccgaatcaagacccgttgagtattgaaggtggactgatgacgcgttcgagggcaaagcgggtaaatcaagcgatgggattacttgttcaatccactattgaagggacaatgttcgggatgcaaaactaggcaactttcatgttggggttgagagcgaaatcgaaatggatcaacgtaatgaagcggacgaagttgaagttgaaatttagtgctatgcgaccgcatagtacatcggcacatcctggcttgtggtcgcatagacccatgcagggaaatttttgggcagcaacaactcttctatgcgaccgcatagaaatactctatgcggccgcatagtacaaaattcgggacgtgttttcaatttttggcaacttttttagtttccataaaatttgattctaattattattttttggtacttggagcataatttccgtccaagacaatatttttagggttggtataaatactttctcataattattgtaagaacaagtttgacattattgagaattaatttgagaggcaattcttgctttccaatctttgttcttcttagaacaatttttgaacttatcaaggtgcttaattccttgtggcattcaaaatccgggtgtgagtctttggttgtgtgatcaagaggtctttcatattactattattgtggggttgcttggttcatcatcttgggattcaaattcataaactgggattaattcttggcttttctgggattcaacaatcttttatgggttcgttagtgatcatcctaaccgggttcgcatcactctacttgagtctagatatcctaatatggagaagttggcccttgccttattagtagcgttgtggaaaaactccaaccttatttccaaagttaaagtattgaggtattgacaagtttttcactcaaacaagtattagaaaaacccaatgtatcaggaagattgatgaaatgggttgtagaattaaaacaattcgagataaactgtaaatgacgatttgcaatcaatgcgtaagcgctagcaaatttcaaaattgaacttctagacgtccccattcctgagcttgaacatgaacaggaaacttggaaacaatttatggacaggtcttaaagagaaagaaatgctagattgtggataattttaacaaatctgggtggacataaattgaagtgtgcacttaggttcgcataaaagagtttgctagccgatttgcaatagcaaaggaaatgcatgcccagaaaattgaggtatagagtgattcgaagttagtggtagatcaagtcaacggaaggttcactaataaggaaaaaataacggttgcatacttgaataagtcttggacttgtcacatcacctcatttcattcaagctctcgtagatccctatagaagaaaaatggataaattatcaaaattagcaagcacgaacaatgtacagttattcaaaaccatatcgaatggaattattgtcaaacccatgagttaatcaaaaagggaggaaagtttagggatactaagcaaaatctaatggatataagataatatatcctacatcaggaatgaagtactctttaagaattaaaaagaggcaagaaaatcatgaataaaagtagccagatttgtattacttcaaacaagggtatacactccctttgccaagatgtgtgaatgattatgaagcaatatatgtaacgagagaaatctatggcggcatatggggaaatcacactgcagacattccttagcctaaaaagccttgaaacaaggctactacttaccaaccatgagaaaagatgtcataaattttgccaaaaaatgtaaaagatgccaaaagtccacaccgatacttgaaaaccaccacaagagttgactaccaccaatatccattggctcttcacgaagtagggtatcaattttgttggatcttttcctagagaaagatctaatatgagaatgatgatcataccaatagaccaattcaccaaataggttgaagcagaacctcttacaaacatcgccaaagcccatagttctaagttcatcttgaaaagtattattttttggttcggactaccaaactccattatattagataatagtagatagttccaaaggaaaaaaaattgagagctatgtacaaataactaggaatccgtagacatttctccacttcatattcatattatcttcaagctaatggacaagtagaatgagtaaacaaaatattgaaaaacatcctaaaaattaagattgattctgcaaaaggaattattgatgggccgacgaattaccataaattctgtagtcatattgcactaccaccaaaattgccacgtgagaaactcctttctctttagcatatagggttgaagctatgattccgatagaaataggtttgagttcaactaggaaactgaactttaacgaagaacataatgaagaagccgtgaatacttaggatctcttagaagaaaaaaggaaatacttctcaaatgaagctcacaatatatcaaagaaaaatggaaagatacttcaattctaaggttcacagaaaaattttaaggtggaagatttggtgttgaatttttattattattttttttttttaattacgaactagaaaatatgttcaagatactatgcccaaaatgttatgtcatacactataatcgaagtaattggtccaggaacatataaggtcatagatgaaagtggcaaacccttaaacacccatggagtggcttgtaattgagaaaatatcatcaataaaacaactttggttgatcttggttcggcagtcaacaaagttatatactttatccaattaacaaattaatgcctgtaacactattttaaatgtacattgacactgcgaagttttcaattaagcgggcttatcaacttgagctaaatatacaatactcatgtaaataatggatgaatttagtgaaaaatcccaaaattttttacaaggaaaagttaccaatgcactttgctacagtaaaaaaaggacaataatccaaatcaattaactgagtgaaaatcctacaaaaaaatgcaactagagttcttataatttctttagacttctgagttcacgtgattgcaagattcctgaagatgactaaggacaaaatgaagaggtgaaagactgaaaggccaatttattgaagagataaagtattggaagaagaagaaatgagaaatgaggtcaagaaatgagaagatggaatttgagaactaaaacacaaaaaaccattgaagatagtattaccatgagattgcatagtatgtttttccgtgcgactgcatggtggttttcagtaacttgaagcctggattttcttgaactatgcgactgcattggtttgtactgtgcagtcgtacagtactttttcggcgtatagtttttttctaagtttatctaatttgtcgtgaaagataagaaaggataaagggaccgtgtgttgattgtactctaaaagtaagtgaaaattttggcttttgtaattgattaaaactcttataaaaacaaatattgggttgtactttaaagccttaggaccgtcctaaaagagagaaggcattataacacattgatgaaggtttttagtggggagaatgaggcaaagacgtgaagattgacatcaagatgcaataattcgattcaagatttaaattggtgatgtctttttttcattattcagtctgttttcttctttgcattatgctaggctagatttgtttgtgctagtaaaacgatgaaccatgtgatatgaatctttaatctttagttttacattcttaacattaaaatacatttttggaatttgaatagttcatatgaatttattttctccacaatttacatacacgtgattatatgaatttgggggcttgcttcatgcatttgaaagaagggaaataggctcgacatggtataaatcgtcgtagggttcgatgggggatagaaatatactgttatctctatgtgaatctttaagtgttcataaaattcatacattcttaatattctcatccgtcatagaaatatagtcaggtcttatatgagaatagatttaatattactctagaaagattgtttaataaaataggaatattgattaatcaaaattcaaccgtgttgtcaatgtgtaaaactaagtttaaagggattattacatggggtttcgcaatcctagtatgtttatcattcattagaacatttcaactgctatttaaacacaacttgaatttacttaattaaatcacttataattgcatacgtaatttagtttagttataattttcatcaaacaaacactctcattttttattgtttcaattaaggtcacagtaatagaaatagatttaaatcaatccttgtgggatgtaattggacttaaaatctcctttattacttgttaacgaaccgtacacttacggtgattttacatcgaaatattttttcgtgatgaagtttttgacgctgccgtcaagaattgagttttagtttgattttatttactttgacactaattcaaactttttattttattaattttattttattattctactcaagtttatctaagtgcgactattgctcttcatttaagtcttgtatgcaaaggtcgcgtgatggtgaattgattcatgctgatttagaaattgaatgtacctttcattgtaggcaaagtgaggcaagagcagcgtagcaaaagagtaaaaatagcaagtaccaatggttaatcagcaaatcgagccagtgattagtcctacaaatccattagatgcagaggtagaagatggatgaaatatgatacttggggacttcagaacgccattaatcatccaaagccaatctagtattatgtattccccatttgggtagctaaacttctagcggaaaactaatgtgatccaagtttttcagaatggacatcagttctacggaatggctaatgagaatccacacacacatatatcttgattcgtggatatgtgttaaaatacgtattaagaaattttagacgatgttattagactaaggttgtttccacatactctacgggataaatcactcaaaaggctagatttactccccattgtgagcaaagtcacttggaatgagctagctcataaattctgcacgaaattcttctcactagccggggtagtgagattgaggcatgacatatcgatattcagtcagggtaaatctgaatcatttgataagtcttggagtaggttcaagaacatgctacggaagtgtcctcaacatggtttcgacaagaagacccaaatacaatttttctatactggattttacttccatctttcaaaagcttagtagattcatcatctaatggcttcgtatcaatgagaacagtcgatggagcattggtattatttgagagaatggctactacttcagccatgtggtcctctgatggttcaaaagaaatcaccgaaggtttatgaggaagatgtatagtcggccttatatgctaaaatagactccctatttcaaaagatggaaagcaattcacattcagaaaatgtaatacaaatacaaaaaccaagtcgtgaagaatgtggagtgaatcacagcatagtagagtgcataattttgtcacagaaaatggaataggtagagtacacgtaatggggttagcgtcaacaaacaatccaaattcatacacttacaatcccgtttggagaggggatcaaaatttctcatgggtcgtaaaaaaagaaatttggaaatcataatagaccctagatgcaatttaagtaggataagaaaattcagttggaagagaagtttgcaaagttcttggaaaagattgaaacaactctccaaaatcaaggtgctgcagttaagatcctggaaatgcaagtgagatagatggcactttctatgacagggtagacaccaagtactttcccgagcattaaagtgaatctcagggagcatgttcaagtaattacaacaagaattggggttcaattaccaaaaatacgtgcgaacagatcaggtgcaattgaagaaatggtgccttctttcgatgaggagtcgatgatcagacgaaagagacatctaccaaagagggtctagatacatcatgggctaaagcaaccaatcctatcaatccatacgagcccctattccattccttcaaagattgaaaaagcataagatggatcaacatcacatgaaatttttggatatcttcaataaacttcacatacacatttcgttggctgaggcaattacccatatatcctactatctcaaattcttgaaggacatcctatccaacaaatgcaagctggatgagcatgaaacagtgaagttgacagaagaatgcagtgctagaattcagaaaaagttacttccaatgctaaaagatctaggaagttttactgtaccctgcactatcgaaaattgctattttgaaaaagctttatgtgatttgggtgctaatattaatttgatgacacatctatttttagaaaactaggattgagggaagctaaggtaactatggtaatcctacaactggctgattgattacttactcatccacgaaagatgtttcggtaaaggtggagaaacttatatttccaacgaattttctcattttggacatggaggaagacaaggatgtgctagtcattttgggtcgatcatttttagctactgaaaaagctcttatagtcgtatagcgagatcaattaattctaaggtagggaaaggagcgagtctctttcaatgtgttcaaagccatgaaatatcctactaaatcaggcagctatttccagattgagatggttgacagagtaattcatgacacctttcatttgcgaaatttgtcagacacttgtaaggttgtattgtgaattctcaatccacttacactaactccaatgagattgaggtttgtgcaatatatatggagataaatcttccatacatgtcaaacgagattatgaggagatttaggtctacattgttgaatttaaaagaaaaatgagggatagtcatactacttagggaagggtgagattaaaatttggaggaaagttgacgtatgaaaaaaggtcatattgagaaaactaagtaggacctttaaggctatattcaaagtattataacatacttgtgccaaaagtcgagctctagactataaatcgagcgcttaataagaggtaacccattcttctatccatcttcacttattttgattagctattgcattaaactatgttcaaggattgcattagtattcaggaacatggttaagaacttatgcatttaatgatttttatcaaaatttaggtagtattttaagactaatattagtaacttggcatgtttacttattgaattcaatttacttaggctcatcattaacatcctagcattacattgagctacattgatgtgctatacacatttaaggctgcaactagatttcaatcttcttaatatcagaaaatcatgagaatacattacaaatatttaaaccttaatcgctctcgttaatatttattttaaatcttgcaatagaaaattgaaacttagcaataaagaaaaatggtagttgtcatgatatctactaactggaccaacctggtccttctacctatccgcatatacaatgaaaagtttatgttccttactaccttattgtaattacttttgcttttacattgaggacagtgttttgtataagtttgcaatggcataatctttacaacgacattaacattgatcgatatttgtgtataatttactgctttttgtatgattgtttgtgtgaaaaaaaaataaaataaaaaattgtggtctttatttatttttatttattattttgcgtgcttgtgtgggtttgatggccttgctggaaatgacgttgaatattggaataagtatgagataggaatagtggaaatagtgcgcgaatagagtagcaaatacttgtttatgataaacttaacattttctgtgcacaacatgttttatatgttaagttggagatttgattcattaaaaagaaaagaattgaacagaatagtaccttaaaaaacctctattatacttatccataatccatgtttcggtagttcagaataggggttccgtgcatcaaattttcttgtgtggattgtctaaaacaaatgagaagaagatgaagttaaagtcttaagttaggggttggttttggaaattaattgtctaaaaaaaagggcatagcatcaatttgtatgtgagtaacacttctctcaaagcttttatggcttgataagtaagcctgtaaggatatttgaaaatctggtgccctaaggtcaactgatttgggagtcagtggactgaagcttgctgaaatagttatatagaaagcaagaggtgaagaagctaataaaaatcatcttctcgagtctttataactcaagtgaataagcatggaatggttaaaaatctggtgccctaaggtcaattgacttgggagtcaccggtctaaactcgctacatgagttatatagaaagcaaatgaaaaaataccagagagagagaataagtataagtgaggaaaaatacaattgcattaattgagccccaaaacatttggttgctaaaactataccctatacatttaaagagatgcaaatagcttagtttaatcttaaaggtttgaagcaatcaaaaataggagaacatctacttagtgaatggtaaactacgtaatagtaagatctattcaaattaagagagtgtaaggattagaattaattaaacttcaacattagaacacaccccagaagagttgagtgaaaagaacatgtttgaaggagtgtgtatctcttgagtaaagaaatgaaatacttgaacactgcatgttggaagttgaaccaatcatgagcttgatatgatttgatgagtttacacacatacacgtctagtagtgcatataacaggtagggattgatttgattttgtaccattgagattgttcattgtgttgattactgaattttaattctgagacatggcaagttatgaaaccatgttttgtatggatgtaagctacacttttgtttgcggacaaactataattcaagtttggtggatttgacaagtgcgttttacacctatgtagatcacaaaatatgaacaattgttagtaaatgtgttagaatatggcctaattctatacaaattgtgttttgtaggataacattgatgaatatgactagatttagaagaaatgagcgaaaaatgatcaaaattgaagaaaataaaagttcagagaccaaagtgcaaatagtcaaaagatgacctagaagacaaaatgaagaggtgaaagattgaaaggccaatttattgaagagataaagtattggaagaagaagaaatgagaaaagaggtcaagaaacgagaagacaaagtttgaggctaaaattgtggaagatagtattactatgcggtcacatagtatgtttttccatgcgaccgcatggtgattatcagtaactcgagacctgaattttcttgaactatgcgattacattggtttgtactatttggtcacataatactttttcgacgtgaaaattctgatttttgtaattgattaaaactcctatggaaacaaatattgggatgtcttttaaagccctaggaccatcctgaaagagagacgaggcattataacacattgataagtgattttagaggggagattgaggtaagaacgtgaagattgacttgaagatgcaaatatttaattcaaaatttaaattggtgatttcttttctttgttattcagtttgttttcttctttctaccatattaggctagatttgtttgtgctaggaggacaatgaaccatgtgatatgcctttttaatctttagttttacattcttgacatgaaaacacatttttggaattttaatggtttatttaaatttattgtctccacaatacgtgattatgtgaatttagtggcttatttcatgcattcaaaagaaggggaataggctcgatatggtacaaaccatcgtagggtttaacagtgtatagaaatatactgctatctctatttgcatctttaggtgttcataaaaattcatgcattcttgtgtattcgcatccagtatagaaatatagtctggtcgtatatgagaataggtttaacattactcgagagaaattgatgaataaaatatgaatattgacaaaattcaaccgtgttgtcaagatgtaaaactaagtttaaaatgaattattgcatggagattcgcaatcctagtacgtttattattcattagaacactccaacttgcatttagttagttaaatcacttataaatgcatacataatttagtttatttataatttgcatcacagcaaacactctcatttttattgtttcaattaaggtcatggtaatagaaattgcactaaatgaatccttgtgggacaatatttgaacttaaaaaattttactttattacttgttaatgaaccgtacatttgttataattttacatcaaaatacattttagtgaatagcctcttcagtttagtaattcttctaagatgcacatatgtggaaaatgcaaataatgcaaacttgccatgtctgtaatccttgttaaatgattttgatgttacaaatggggaatcataccaatcccagaggcttgatgaatcacatatctccttaatggaggaaccatcaaagatatacctaaaaaacatatagtagtcgacaaggactacttggagtggaaaacgggctgggtcgggccaatttttatgcaaacccaacttgacccgacttaaccgattttgggctatttttataaatcgacccaaccagatcggtaatagaaactgaaccgatccttcccgactcagttcgggccgggtcaacaattattttattttatatttttttcttttttcgattagtttcaaactaccacatgaatccttattttcctgaaataaaattaaaaaaaattcaatcttttttcttccagttgatgatagtttgtcattttcataaacaatgatagcgtaaaaaattcaaccaaaacaaggtaatttaaataaactaaaaaaatactaatgaaactaaacacaatcaaaatagcaatcaagcatgaaaagaaaatttaaatattatagttatctgacaattaaaaatattacaataatccaaactcaataaataaaaataaaaatgctacaataatctaaaatcaaaactctcataaaacaaatataaggtaaaaatgttgcgacttccaagttgtcacataagctttaagcatcattcctacaatacaaataatagaaatagttagagaaaaagataaatattacattaataaagagttatgcatattaaacaacatatctacctcaaaaatttagaaatgaactaatcgcattgatttagcatttatttgatttttctgtttctaaaatctctacaaaaaataatgattaaattatgaataaatttgattaaatacatatttaacataatttatggaataactgcattaccttcatccaacttattatattcctccacatcttccatattgaatttctccaaggttgtagactctttaatccaattttgtgtacacaccaaaactttcaccatcctaggtgttaaagaactatgaaatggatcaagaattcttcctctggtactaaaagcactttctgaagccatcatagacacttgaatagccattacatctcttgcaagttttgacaatgtaccatatttgttttcattaaattttcaccaattaaaaacatcaaaagcatcgtcctagatatattcacaagcatctaacaagtatctatcacatcatttttcaattcaaataaatcttttgctgcttgtgttctcttaaacctagaaagacgagaaagagagacacttgaagtgggaccttcttttgcagaagaaacctcacttgaagaattcaagtcactaggtacttgattgctttcagatcttgtttcacatctcacataccaatcataaatagacatcaatttatctttcaaaatctttgtcatattacaagcaacttcctcatcaccataaatatcatcaaaacaaaaatcagcatatgccaatttgtatcgtggatcaagcacagtagcaatcaacaacagctgattaacttttccatttttcccaagtacttgtcaaactttttattcatgttaaatttcatctaaaagaacatcaccaattgaactcaattgttccaattcggttacaagtgaacatacttcatgaaaataaacattagagctaacatgcgttgaagtactaaacttctcactttaaggaattttacaaaaagagaagcattttcccaatcaaaagctgtaggaagcccactccttcttctgcaatcatcatacttctgaaaataatttacatactacacatcatcctcttctaaactttcaaaatcatttttaaattttaaagcgacttccaacatcaaaaatgtggaattccacctcactggtacatccaaaacacaattgatttacaatcaactttctcttcactcgcatactccttaacttttgttctctagcaggagaagatttaacatattttacaacattgtaaatactaacaattgaatcatgtgcttccctcaacccctcacacacaatcaaattaacaatatgcggatagtacttcatgtgcagatacttttcatctaaaacacacacatcaccactttgaccaatcatcttcctcttaatataagaaactgccatttcatttgtagttgcgttgtcaactgtgattataaacaatctttcaataccccatacattcaaacaagtctcaataccaatggtttcacccttatgattagcaatcacacaaaaggccaaaatccatttatgaagcttccagtcacaatcaagatagtgagtttgtgagagacatataattaatattttgagtggtactccaagtatcagtagtgagagaaactctttgactttggatgatctttttcaattgcaatttctaatccaagtacaactgataaatatctctaacaatagttttatgagacaagggatcaaatttaggacacactaccttacaaaattgtctaaaccccttaccttcggcaaagctaaaaggtaattcatccaatattatcatcttagcacatcaaagcctacactcttccttattaaagccaactagaatgttcacaccaccctcagttaggcttttttgtaatttaacgtcgaatcttcacggatacttcttacaataaataaccaattgattcctcaaggtactagtcccatactttttagcctcacaagcataatcctgcccacaataattccatacacacctaacatcttctttttccctaaacatgatggtggaagtggaggaaccaatgttgaaggagtttcaccaatagcttcaatttcactatctttatccatgttcatgtctatacaaatcaaacaagacatacatatataaataaaaaattgtagaaaagaaaaacatggtccatgaacaaataggccattattaaggataaaaaattcaatatcaaaatcacctccaaaatcgcatggcgatgcaagtaaaacgagataaataattaaaaaaatgaaaaagctagagaggacaatttaaaaagggttttaggttgggctggtaaaagaggaaaaaagacaacttttattaaacttggctttttatgtccaaatccacaataaaattgaaagcttcaagtaattacagtaaaatttacttttctattacattactaagtagttcagttctatattctgtaaattttccctacttaaaaaagagaaatagaagcaaccttttcagtttaggttttgcagcttctcgggtcttcctcttaattttttgctgcgtactttcaaaaaaccttctgtgcttgcattccagaagaacacccgccttcaacacctccccgtcgaacctgccaacaaatttcttttcaggctcacttacaccgataagaatctaaacattccaactacacttaaacaatatcggcttatctctgtataaataaatatattaaaaaaaacttgacacaaattgttaatatttatccatgtcttacataaatatactacatacacatataaggaatgttgattaatgaagagggaagtatatattaaaatcaaagaagaagaaacccacaattgaaggaagctttctgtaaagatgaaggagatggtctgaggttccaatggcgatacgtatatggcaagggaggctcaactttgaagttgagagagagacatcacgagaatgacaaggaaataggttttctcctttcgataacgggttaggtcggtttggaaaagtttgaacagtaaacctattaagggaataaatcccacatcgattaaatatcgaaatattgatcaatttaaatagatcttggatcactcctcttaataaggttgatcttattaagatgtatcccaaatcttaatatgatatcagagcccagtaagctccaacgagctattcgatccgattatgtttcaaaaatgagcacacgaatttcaagattaatcagctaaaaaagagccattatcttgtggaggcatattaagggaataaatcccacatcgattaaatatcgaaatattgaccaatttaaatagatcttgaaccactttttttaataaggttgaccttattaagatggaccccaagtcttaacaaaaccaacccgacctatctaaatttgaaaattaaaaatgaaccaacctgactcgttttgttataaccgattcattcatagtcaaagttaagaaaaatatttagtaaaagtccaaaattcaacgggtcaaagtaaaagtcaaataaagattcaagttgaataaattattttcatgagtcttaagttgtaattacaagtatttgagggctagaaataacataaattagaaatcaaagggatttagctttctgttactagaaattaaaggtttgaaaagtatatggcatgaagattggggacttaaattgcaataatttattggtgctccattaaggccctgtttggcactcatttttatcaaaatgcatttttctctctcttcttttcaaccacacattttttattaaaataatattacacgtaaatcaaaaactttttcttatttttcaaccacacattttccatcaatttactattcaaaaatgcattttcacataaaaattcctaccaaacaccctctaaataagttaatcaattctaaattgaacccatctttcatttgggaaaagaagaatcaagaagcagggagagaaaaggaaagaagaaaaaaaggaaagaagggaaaaagacaaaagtagatgcaagtttttacatgttttggttcttcatttcttcaacatgtccttcctttaaagagttatgttagttaaatttttagaatttatgaataattgtttatattcaatttaagcaagaactaaaggttattgatatgtatcttaggtattaaacaagaaggattatatatattggaatatttgtgttgaagggaaagaagtatgaaatgagtttgtaaattagagcctaaatctttatatctattgtgtatatatgatataaaacagtttgttttatgatgtattacaatgagagatggagttgatgttggatttttgtatttataattaattttcgggcaaaattcatgctcaggtgctattttccaaattcattctagaaagtgttatttctgttaatgatttcggtgacactttccaatatacaaaaaatggcgccacattttgatagcctggaaatatagtgttgtttttggtatttttttttattttcttggatttttagtatggaaatcaaatttagtattaaatattcgggattaagtgttaaaataacttatataaaggtagatatgttattagtgaccctaattgggattatgacgttacattgaaagtaaaagactcttgagttctttttggtaaaatatcatttctaataataggaaaaatgcttaaagcaccttagtgatgagatatgatttcttgggacgagtgctagatgtcataattggtatgtgaatgtgaggaggtgacgagaagattgaagtcaagatcaatttacaacttggtgagtggaaaagcttatttttcaaaaataagtatttattaaattcatattagatcgtaaagttaattattcatatagttggcttgacaacataattttcagaataaagtggattttattgcaagtttttttaatgttaaattatgtttagttaaatcctttctttaacatattatatgagtattatgaatagtagctgagttgagtagtgttgaagcatgttgatctaccaagttgagccacacattatcttaattgtatgactcgtttggttagtttatatagtttcatgattcttttgtgaaacatgcatgttaccaaaaaaaataaatttgtaattcatgtatccatattatgggctcactgcatttttgtaaatgttgtgtatttggagtcttttggcttgtaaaggagtgtaaatataattccaatacactatattttgaatagttgtgttttgaggggccaatatatcctattttaaattatatgtacatgtttgagaaaattgattattgttcagatgattttagtccatatttcaaagaatactctgtcaaaattcttttaaaaattcatcacggtcaaagcaagttaaggtcgccttggtggtgggttcggcacttagctggtatccactattggtgcaaaacacatgtcaggttcattagggtgatttgaaatgggtcgtgtcacgattgtcctcttttttaaagggaaaattaggcccaataccctaaaaaatcaaccaatttgattaataccctgttaacaaataaatcatttaagcacgtatttaatacgttctaaaaccacccaaaccccccaaaacctaaatcagtcctaattccaaaaatacactcaggatgaaattccgtcactcaatatcaatatagattactcattttcaggttgttatattgcaattcacttagggcgagaacttagcaatattcagtggcacctttgaattagcgatggataatgcaagttttgagaatggttcttctgtgaatattgcgaggtgcagtgtttcggaatgagtgaaggattatgagtgtaatgcttcggaatgatcctaattcgactgtgcatctaggtggagtggcgcaacgatcgcgttggctgtgaggataaaaaaaaatggttatgttcatttgggtaaagtgagctttggaggtcagtggggatctggtggaatatgaaatatgtttataatcctatattttatatttagttgcaagtgttgtatatagaaaaatcagaataataatataaacctcagaagagaagtgcaatattctaaccttcttgatttgtagaagaaccgtaataaggttgggatttatgctgtccaaaatcaagcctactgattagagtaattagagcaaataaatttgagtgtgatacaaaaagctttttgtatgtatgtgccactataaactctgacactactttataactttgattgctctgaagttaaaactaaaagcttttggttcaaacatagtgcacatatccctatagcaacttcttttggatgcatatagcaccatgttttgtcatctctatattcattcatttcattattagttcaaaagcgactgtggaaggaggggtggggaagaggaataaaatgagaagacaagatgaaaatgtatgtctgcagtgtttatgtcactcttagagtgacaaacataggttttaatcgatactttgtcactttgtttagtcttcgcaacatttggaatatttgccacattttttaatagtgcttgccatttttatttttattttttttgtttaagttttttgtcactttttattgtttgttacaatttaaaatttctgtttctttgtgtgtaacaaatataggttttgattggtgttttgttacttttttgtgtatttatcacttttttctcacttttttaaaacttaacttttttattgtttgttaattttttagaattctgtcactttttttgagtgacaaacataggtttttattggtgttgtcactttttttactaatgcttttcacttttttaaattttgttactttttttaaaatttctatcactttaagtgacaaacataggtttcaattggagattgattttttttttttttttttgtttgcgtttgtctttttttaaatatggtgctgggaaccacatttctacttcattgaccttaaatggaaagcacaatgtctcattgactgaggattctaatgtttacatatggagctacaatcgtgaaccatgttctatctcgcaacccattatatcatttgagtgtttctcgtctgacacttctgtgacaataccttggtctggcttaaagagtatttatggttgtaatgattgtgtttggattgaatttgaataaaatgaaatattttaaggttttgatcaatgtttcatcactttttttttttaagttttatcattttttttactgtttgtcactttttttaatctatgcagctttttttaatttgtgtcacttttttaaattttcttcacttttttaaatttttgtcgcttttttagtatttgtcactttttaaattttcgtctctttttttagtatttgtcacttttttatcaatcatgttattgaaatttttatcactttttttaatgacaaatattatattttaataaaagtgacattgtatgtcatttttttaataaaaaagtgacactaaactttcaaaagtgacattgtcacttttttagagttttcatcatcttttaagtttttgtcacttatttaataagataaaaagtgacatgatatgttatattttcctaacataattcgcgtgtggattgtcttggacatgctgattatgttaacaaccgccactacgctcgtgtagattatcgtgaatatgctgattatattaagaatattattactggttctacacaaatggatggtgctatttttgtgtttgtcatttttttgagtttgtgtgacttttatttgaatcgtcactttttaagcgtttgtgtcacttaaaaaaaaaattaaaaaaagtgaatttttattaaaaaagattacacagtattttttacttcccaaaaacttttcatatgatttttcaaaacacctctaatttttagcgtttgtgtcactttttttgtgtttattatttttttgaatttgtgtcactttttttcaattgtcactttttaagcgtttgtgtgacttttttttattttttttgaattgtcattttatatagtattttttacttccaaaaaacctttcatatgattgttcaaaacacctctaattttaatagtatttttgtaagttgcccctttttaaacacaaatcgtgggtttgcggtttatgggcccagcccctaatgactacggtaaaaatcaccattcctatgtaaggcccataaacaattaaattataagagttagggaaaaaaaaagaagtagtcttccaagagaacgattatcttaaaaatattgacagaaaaatgcataaaggaaaaaactaatgatagtagcccgatacatataagtttcaaacacggatcctggccgttaaatttcaatagaatcaaatataatcacaaatataatcatccaaaaatgaactaaccttagccattaaatacgaaagggcacatttatacaaaacaaccagatcagtcgcgtgcctcactcgcacagaaatgcatgcatattggaaaaattattaaaacgacaattatgaaggagtcgtttcaactaatgtgcctattgtcagtaatgcatagaaatttcaacctcatccacaatcgttgtggaacaacctcaacaaaatccacaaactcaaatttaggggactattattataattatccaatctcaaaattttcccccaaagaatcaatacaccaaatcggagtaaaatgttaagttctcctattgcaagaaatcatcaaagcctatacctatcaataaaatttaaataagtcattctttgatcatagaaaataggggtgtaagcagtccgattttatcgatttttgacagaatttcaaaccaaatcgtttaaatcggtttgagaaaaactcaaaactaaatcaaatcattttgaacggtttgaaaaaaaactcaaacctaaacctaaacctaaacctaacgatttggtccgattttaaactgtcgatttcgccaatttttttttttttgcatgtttacttttatatcattaattcattgaattcaatatatatttatagcttactagcaataaatctaaagtatagtaagcccctgtttgaaccaaatttttgggacaaaaaaatgaaaatttggaccgttatcccccaagtccaaccgcctttgttgacctgttattttatgtgtgggactcaacctcctctctaacgatcaattttttcattatgatgatatggaaaatatggctcaaacaggggctaaatatatatactataaatttaattaccaactaaatcaaagtaaaatcacgataaactaaaacataattttttttctatttttgttcacctttttaaggctaatgacgatacaataacgttacaataagagtctactacactagatataaggtccaaaaaatataatgatgttcaagaagaccttgtgatcatcatatctgaaaaaaggatgctgattagacaaagagaataatcaaccataataataaagaaattgtttataatatttaaacataacaattacacaagtttacgtttgtatgatattaaaaaatgcatttaatttcatattcttaccttagtttgcccccaaaaaaattattaatctgaaactttattcttagcaaatattatcatcaaaggtttaggatttgtttcggatttggtataatagacttcaattcaattttgaagaggcgtgaaaagtctgaaaaagaagtgtgtggtgccgatagctcaagactgtgttgggtgtcggctgaagttcatctaaatttggaagaggaaaatgacttttgataaattatgttaatcttgagattattaaatataaattataattattggatattaataatatatatgtattagaaaattagaaattatcaaaaatacccacaaatgacaaaactattgacttttatatatttggatgaattttcaaaaaatttcattttcatttttttatttttatatattttttcgtcagtctggtttgattttaaaccacaattaaaattctcaaatctaaatcaaaccattttggttaggtttaaaatcatttcattgatcaggtccatgtggcattaaatcaacggttttaaaaatgtgatttcggttcgatttttcagtttgacggtttttacctacagtcctaatagagaatgtaaattaagttctgaaactaacataaatgattagactagtacagctaggactattcgttatcaataaatatttagaaaggatcataatcgagcctttatacgtgagtgagcaccctaaaggaccacaatatatgtgaacccagaagtaagctgctgaccataatagcacgaattctcataagcaaccttgaatataaaaggtgatccaaaatacccgatcaaatatgtaaactaaattggtgaataaaatgtaaaatattagaatttgttagataattagtagctgtcatgtgtcgctagcaaaaatgacttaaatatcccaatgcctcatcagtaatttatgaatgaataggcatagcatgggaaggattaggcatgaaaacttgaatagattccttccaaatagccatttcttctcctgctctttcttgagcatcagattagtgaatttgaaggggaaaactcagtgttaggattatcgacccaacaccaacaaacaatcgtaaaacagtaaaaaataaaacaagaacataaaatcgaacacagaaattttcacccagttcagcctgaaatggcctaatctggggggctcagaggtaagcccgtcactagcaagaaaccttcaagagagtgtacaaccagttgaagaaaccacatcatacccactatatgatcatcgatccacaaggatctctcagtaactcgaaaacctagcctacaagactagacaaaaccttcccaagaacacactacagatttaccagccacaatcaaggcctaaaactctgtaccatagttctatcatcatcagatatcaacaaggttattacaataatcttcactggttcttcaattcaaaagagaaaagaagaagcagaaacatgaaggaacgagagagagagagagagaaacttgaagggacaatttctgccaaaatgaaaagaaaagtgccggctgacttcttctcaccaacccttaaagtctccttttgcattaattatatgagactaaatctcaaccatagatgtggatcaatggtccataaatgataagagaaaaaccacaactctagtgacattattttatccaataaccgaatgccatctgtccatagactataaagagtagaaaacgttttttcacttatggatgtgctgtttgagaatcacgacttcacactcaggctatgtgagaggaatttatttatcatcatttagaggtcaacaattgcaaggagaaaaaataaattagaaatgtggatacactctatgtttgagttcacatgtgaatactttgaaagtttgattttctacaaggcaatttcaagattttaattttgatttttaaggttaatagattacacctagtttttctctaattagtgttgtccatttactgttagtgtatatcagttacgaagcttctctaggactttattgatttggtctccaaatttatccaccaattataatttatacgtactatgtaatcttagttatacaaaaaatttgccttgtaaaaaaaatgatattttccttttttttttaatataaaaaatgattagtcttgcaaaatcttccaaatttggctaaaattcaaattcatcccccaatttgggctacaaatcaagattttttttaaatccattagttactgttccaaaagctgactatgttatcaattttacctgtttattcttaataccttcacaaattataataacaaaaaggaagataaatagtattgaagacaggcttatgatcagtaacaaggtatactagtgccaaaaaagcttctcagctaaacataaggtcccatttacgagatattttagttcaccaatttatatttacgggccaaggcacttacgagcaacgtaaaataattttttgagaagattatttatcaccgattctcaattttttttccttaattatcaatattcatccaattttgatgaattttcagaaagtaaaagcgaaatttatattatattataaaatagaaattcattgtttaccacaaagttaagcatccgagacattctacattttccgacaatttatttatcatttcggtatttgccctttttttatattttttgttgtcatagatattgtttcgcgcgggttgagtcgctaataattaaagaggatcagacgattgtgtaagggacgaaacctcttgagacaaagtcccaaaaagaggtgttcttttattggcgataaactttacaattggaaatgaaaaacagcgtgcctccaagaggcgcaagcacacgagttacagaaagaaaaatgtataagtctaaaagctaaggaaatgaaaattacatattctctgttcgagagttttggattcggtcctttgcttctgcgtcctttctcccttttatacatcatagacgatctctttgtgattaactaccctaaaaactgcttgatcgtcctataactactcactttctttgtagtggccattttgtcataaaactgccttttaactgctgccattatctttcatcgttcaaccgctttcgattgaattccttgagtcgtggaacgtgataaggctactttaacaactgccttgataactgcattccttgataaccacgatgcgttatgtttgttgatactttgggcgacttgaaggtttgggcgaaagtagaataacagctctgggcgactgtatgacactccattcgttcagattctgggcgacttgcaaatttgggcgatggcgttaccgcattcttggaccccttatttgggccttcaccttgattcgttcgattggacatcgttctttgggctatccgatttggggatcctccaattgggctttactccttgagctgttcgatttgggctgaatttttatgtgtcaacaattaccccccaatatggcagaattaataataattattgaattttgccatattcacttcatgtttccagcgacgttcgaaattcccaagaatttcaatcattgtttccttctataacttgaaaaagtgcgtcgttttgcaaacccttataaaccccaaacacgccatttcactgctaccaaaccacgcctcatattttctgcatctctttcacgattcactgttcatcttttgcttccttgttacgtaaccctgaaaagcttcgttcattctccaatggctgcttcacaatctcaagctagcgattcctttaatttttatgactttcagaaacttctgagtcgcccatacataaccccaagttttctcgcgcccgccgacgttggacataatgagttttatttgggtcctttcttcaacaatgcggaggcagttgaacaggcggcggtgggtcagctgtttccttgcactcatggccctccttttctaaactctctgccgctggggccacttcgcgaaagaggtattcgcacttggcctaaatctgatgtagcttttcgtaggtggcatgcttgccttgtgggtcatggtcctactaaggcactttttgatagcgctaggatttctgatttgttagaagtctctattcgtccccctacttttgattcagcgctctttccgattgctttgagtttttggtcccctgagtacaacacctttatttttcctcttagccccatgtctattacattaagggatgttagggccctggtgaatttgccacctttgggcgataccattttcccaggtatcttagtttctggtggcgccccacagttcggtaaaaactacaccgattcttattcaagcctgcagaccctccataatcattcgagcgctgagcctacccatgctgagcgagtggcctttcttttagtttggctttgtaaatatgttttgtgtgtgccaagtataaagccttctctgagttatttacctatagcgtacgaattggcgcgtggcaggcctttgaatttatgttctttgtttttggctgccctttatagaggtatggcttttcttcaagctcaattgaagaatgatgcatctcccactggcagtggacctctttggttcactcaactgtggttgagatcctattttccatcgcttggtgctccatccatttctcgtccttctgctagctgttacgggctagctatggagcccttaactcctgtgaatatgtccagaagggacattttttcattcttttattctttagattcaatttcttccttctttccttttcctccttttttgactccaaactatgtacatcccccttccactatagatagcgcgagcacctccctgctcatttggctccagttcttaactgggagggagcttttccatgatatcttaactgggaccaatgccaaagcaagggtagaaatttatgctccccaattttttgctcgtcagcttggttttggccaaacttggcctgttcctctttgctattcgaagagcttaattgaccgttttcataccattaataaggcggaagcagaggctataaatgctcgcaacctccatttatcaagccacttttcattagccccttttaattcttgtcatgctactcaccctctttttgaacaactctggccatcggtgaagcgtagattatttgcgactgaggccaatcgtgcctttccttcattagaccaaccgagtatttcttctcctcctcctgttttggtcactcctttgtctattcggagcccctctccttctcgtcgtactaaacaatctgctcgtccatcttcttctctccccgccaggcctactacggccaagagtgctccaagccgcaaatggccagcctcagcatctcccattctggaggatgatgatgatgatgatgatgctcctcttatcgtcaggaagaaggtaattaaattggtctgtttacaaatatgcttttccacatttgaaacttttctgtatactgatgatcttttggacttttcagaaaagctcagcctctccttgaaaggctttggcatcgacaactcttgctccatcatcctctgctgaggctacttcatccaaaccggttgatgaagggaccatgcttaaagatacatcttcagtcccagagtcttcatcacaacccatggatgagccaccttcctctcagggcgtcgaccccccaaacgtcgaagcagaaggtaattcagttttttgatgtcttacctttgctcgtgctattggtctttgatctgttgctcttgagctttgcaggtactcctatgagtccgcccgttgtggcaacatcttctcgctcggacaaggggaagtcctcacgaatggatgagtcgttggaggcgagcttggctgagggcgcgccatcttctacgattgtcgacgaggtagtttttctttttgcttcatttctatttccaccttgttcattgtagtgaggattttcaatattggtggtcttctttgcaggacgctgacaggattgtgcgttctatccaagacttgtttgcttcctggggacaaattcagacgtttcgccctgctccatccgatcgtcctgctacttcttccgaagaggatttgaagttcttgaaggagttggtatttgagtacgtatccttcatggatatggacattggaaaggctagtgctgccagacataaggatgaacttgagcacttgagtgcgaagttagagcaagcactgacgcttccgtcgctcaatctttctgccaactttaaagcgacgttgaaggtcattcactccgaggtcctttctatgctggccaagaatgctgaactaaaggccaagcgtactcaatatcttcgagccgtagctgagaaagagtctttgtgcatggagatcaacaaggctaaagacgagttgaaagaaatctcttccaaagtcatgattgaagactctttgatggttaacttggctgctcagatgagagaacttcaagccaaaatggacgattgcagggcgaggatggttgctaaaaagcacaacgcctcccagggaattgagcgaactaagtccttggtcgagcagtacaagaagttggaggttgatgatgatgacgtcgcggctgaattgaacatcacttcttctcgacagaacgaggattgggaaaaacttagggaacgaattcgttctttatgggttagactgtaattaagacatacgatgtcttttctcttttgtaattttgttcattattaacgaacattaactttttgtgcatttatttgacatttattttctaatcatcaattctttaagcacttaactgctttgcactaagaaccttgtccattcccttttgatattcccactactgttcccaagacttagggccatttaattccgtttattagatagaaatgtggctgttcatattctgtctcttcatcttcaccccctataaatgcttcgcatttttcattctctatcttcatctcttcattttcttcttcgaaaccaatttgctgccatttcttggcattctgacgatcaacctgatccaaaaatggactgtctagtccgtccgccttatacttaccttgatgtcacctttggtatgggaggtataggaaatattttctggccagcagcgaagttttttcctgcaaaattcttcccatcgtctctttgttcttcacaaggagtcaatgatgggaggcaatttttgggctgcttgtgggccactttgcttgctgagagtgcttctcagcttgcctgctgagagtgtttctcagcctctttgctcgccattgcagcgatgcatttaggaaggtggtgaggccagtacaccctctcactcggcaatcccaccattgcagcgatgcaattaggaaggtggtgggcccagtacaccctcttactcgtcaatcccaccattgcagcgatgcatttaggaaggcggtgtgaagcttactcagtgatcaaccgggagatactttagttgtattttgtagcacgtccatcatttgtatcttttgtattcttgtaatgaacgtttgataataaagaactttattcgaacgtatttcgctctgtctttattattttttgatcgtccagaatgtttggttatgtttttatctgttcacattcccataaagaaggaacatattttttcaaatatttgccgttaatgaatcttacgtgcttggtgccgtctagatcttccaagtggtacgctccattaggcaacacactgtttattttgtatggtccttcccaattgggcgaccacttcccgtactttggatccttggtatctaaagggagtatcgtcttccaaactagttcacccaggctgaacgacttggctatgacttttttattataaaatttagccattctttgcttttgaacttgcaacctatctaagacgtccaacttcaattcatctaaacttaataaattttgaactagtgattcggcatactcatcatcattcaacttatgttgcaagcacactcgaattgattgcacgttgatttccataggcaaaacggcctcctgtccataaacaagttgaaaaggagtaactttggtacttgaccgaggtgatgttctataagcccataaggtcttgttcaaacattcgtgccaatttctggcgttttcatctatcatctttctgatgatattttttagaatcttattagaagattccgcttgtccgttggattgagcgtagtacggtgtggagtttacaattccaaacctataaataatgtgatcacgaataaactctataacattcttctgggtgatctcttttaaaggtaccgcttctacccatttggtgaaatagtcggttgcaactataacaaaagtatgttgcttggacgatggagggtagatcttccctattagatctatcgcccaacctttgaacagccaaggtttaataataggtgtcatctctcgtgctggtgccctttgtattggaccatgtttttggcatgttaaacaactttttgcatactgaacgcatagttctcccatctttggccaaaaatatccactcctaataattaaccatctcatcctttggccagcttgatgagctccacatatcccttcgtgcacttcagccatgattgtcttggctttttgcaaacttacacactttagtaatacaccatcagagcgtttcttaaacaattattcatctattagtgtgtaattcagcgaacatagctttgtcttcctgctaatccctccattaggttctttaaggaaccctttaatctctgttctccaatccattgcatctccatcttgtatacagtgaagttcaattttcctcgcccttctttgaattacgggcaatatgattccatattcacaagtagacttccaattcaaaacctttgagtaccctgatgccatttgggctaactcatttgccatgtcattatatatcctattaacgcattggagttctacttgatcgaattcttctagtaattcttgggcgatctcgtactgacttataatggaatcactttggtatttaaaatcaccgatcaattgatggatcaccaattgagaatcgcccctaacgatcacatttcttattcccatatctaccattagttctaggcctacaattaaagcttcatattcggcctgattgttggtgcacattctgtctaaggtgaatgcaaacttgtagcaaatccctaaaggattaatcaatgctacccccactcctgcacctttagaggtttttgacccatcgaaatacaacacccaaggttttaattcgaatgaattgatttctaattcgatttcttcaggcatgtcaaggcatggatgatcggctagaaagttagccaaagcctgatttttgactgccttttgaggtatatattgtatttcaaactctgataaagctagtgtccaaaggcctaccctttggtgtaaaatagggcgcgagaacatatacttgactaaatttactttagaaattaaataaacggttacgggccgtaaataagcccttaattttgtacatgtgaaatacagtgctagacacaatttttcaacagcagagtaattacattcacatttcgtcaaccgtctacttaagtaataaattgccctttcttcaccaaattggtcttcctatgcgaccattccagctattgattctttttcagccgatacatacattttcattggccgtccctggattggtgacaccaacactggtggacttgatagatatgtcttcacgctttcaaaagccttttgatgttcttctttccagacaaattcgtcctgatttttcagctttaatagcggcgaaaagactttagttcgccctacacagttagaaataaagcgtcttaaaaaatttacttggcctagaaacctttgcaactcctttttattgttaggtggtttggcttctaagatggctttcgctttatttttgtcaggttcaatccctctcttgtgtactaagaaaccaagaaagttccctgcattaacaccaaatgcacacttcaagggatttaactttagcttatattgcctcattcgttcaaacgaacatcttaactgttcgaaatggtcatcttctttaatggacttgaccactatatcatccacatacacctcaacaaacttgcctatcatgtcatgaaagattaaattcatagccctttgataagttgcccctgcattttttaggccgaaaggcataaccacccattcaaaacatcctagagacccagggcatctaaaggcagttttgtgtatgtcttcttcagctatatagatttgattgtatcctgaatactcatccatgaaagaatacatgacatgttcggcagttgaatctactaaaaaatccaccgtgggcattggatactcatctttgggtgtagctatgtttaaatttctaaagtctatacacacccttagtttaccattcttttttagtactggcacaatattcgacaaccattcaacatatctggtgttcttataaaacatgttttcaataatcgctctatctctttcttaatttcagggagtacattaggagcaaaacgcctaggaggttgcctatgaggtttaaaattaggtttagttggtaatctatgttccaccaagtctctatgtaaaccaggcatttgttcatattcccaagcaaaacaatctttatactcttttaacaaagcgattaatttgttactaacctcttggtcgagcatctggctaatgaacgttgggtgatctcctccttcatcgccaatatttactttgatcagagggtcttgcgcttgagcgtatccaggtttggcaatccgcatcacttcgtcatccagttcatttgtaagtacttcctcttccaaacagtccaccttgttgacttctcggccaaggctttgctctaactcgaatactgtcaacttgtccttcagcgcttttagggcagtctcttccttcgctttgttattgcattccttattgaaagccatcagtctggctttgaaggcctgaatatcggccatttgcttttgcaactcagaatctattcaagattccttgattattcttttgccaatcactggctcttctagggccactatatttggcctcatctgtttgaacatctcagtgagtgcgtccactgagaatggttcttcgctttgcgcgacaacctgagtttcttccccgtcttgtaccactctgacaggtccatagtttccttcgtacatgaacttttccaccgagtttgcttccgcgacaaaaggcctatgatcggcctgtaccacctctgcttcgcctttgtcattccaaaaaatcaggcattgatggagtgacgagggtatacagcgactttcgtgtatccaatcccttcctaggagcacgttgtaactagtaggaccatctattacaaagaagacagtggtcctggtagtcgtacctatagttatgtccaatggcataactcccttagctgaagttgctcctccattgaagttagtgaggatgacttctgtaggaatcatatcaccctctgtctttgcgaactttctcatcatcctggatggaattgtgtttatagctgctccattgtcgacaagcacttttgccactgggacgccgttaactagagctttaacgtataatggcctcaggtgttttgtcaacttcatggctggccgtttaaaaacaaccttttaggcagcctctatttctatctcttgcttgttttctgtcgaattatccccttgtgataggtcgacgtgcagtatgtcacgctgatcctctgtctcctgaatttccttcttacttttttctaatgcttcctcatcagttatccaacctgtgggagggggcattattcttggaggtgacccatatttctcagagccaggcactctcttcttccttttgggtgtcccgtacagtacgtagaaatcgaaaggacgcccagatggctcccccaataagtctacttcgcgaactccctcttggtgtagttgcttaaacagagtgttgcgcgatactcccctctttttcctttctgcttctaggtcgatttcttcttcaatgtctgtcatcccatcgtcctcttcatcgttgtaggcctctccagaagtctggccttcttcacataccagcatgcaggcttctccttcgttgtcctccctctctttttccttttctttattcttgaattcattggccagtaggtaattattggccacgacaggagccaacgtaccgaattggatagcaaggggctgatctggatcttcttcatcctttttgtccctctcaaaccttgacctcccagaagaggtttctggcagttccttcattgattcatctgtaccagtctctttcctacctttgaggacgttctaattggctaccttgagtaatagaggcactttaggatgtggcattccttgttgctacctcattatccgtccatagtttcgctggaaacgcctttgttgggtcctagtcatctcatcgaagggtattgtccttcctgcgctgtactggaatgaatgccatacatttggccggcgaggttgcggcctaaatgttcttccagtatctgctggtctgaactgcctttcaaaaggcggtcctctataaaatgatgtacctcgccctttaccaggctgaatgtttgggaagaaagcagggcgatgaggatgctgccatgtccctggtttctccgtgtctccatttacttcccttttacaccttgcacacaggacgttttcgtccttttttggttctttccctttgattcgttcgaagacactgggatgtgttttagtatcctcttctccatcatctatgaccaacttgaattttggcaacttgttcttgaaccgagacgttaccatatttaccccaagtggccgtgggaaaggattctcgtccactgccatctttttcttatcgtcgaacgtaattcatcctgattcaatagcatcctgcaatacgtgacggaaaaccaagtaattgttagtcaaatgtgaccatgcattatgccatttacaatattttttaccctttatttgttcagggtttggcaatttgtgcttatcgctcagctttatttgcttatccctatataatttatcgaatataaggtcagctttggtcacatcgaacaagaacgttctagcctttatgtttccatcctttatgggctcatctttgcccgatggtctaggcttggccattatgggactagtatatgtatccccttttaccaattcggccaaacacatttcggcctgatcgtatgattcgtcatcgatggtatgaacgtcaaaatttgggtctctgtaataagtccctttactagaatttttcatttgttcttcttctcttatcaatcgctcatacctaatcacattcgcactcaactgaaaaaggtcgggaaattccttgtcctggaacttcttttttaaatcaaagctcaagcagccttgtgcgatcttgacaaattctttttcgggtagaggtacaaaacacttgcttcttgctgttttgaacctttggagaaaattttctgcccattcatttggcatttgacgtagattcgccaaatcagccaaagtgacttcagattcagttttataaaactgagcatgaaacaactgttccagttgttgccatatttgaacaaagttcgctggcaagttgatgaaccaggagaaagctactcctgttaacgaattagggaaaagtctcattttatggtaatcggttacatcaccactttgcaacgtgaatcgccctatgtgttctagagtagacacctctcctaaaccagtaaacagtgagaattctggcactttataccctctaggccatggatatgcttggtctacccaatcaggatatggctttgtgtatgtcggcctaatgacaggacgcaccccaaaggccatctgatcctgcacgatttccataatctggttcctcaacatgacattgggatcatatggaattcctacaggttgattaaccggttgatttgcatgaggtctgatgtttggtctttgattggcgacaaaattaccataattaggtccattaccgttagcctggacatctgttccctcattaccacgtggaatattctgtccattgtttaggacattatctctcacgtttgaattaccccccaagttaggcatgccactaccattattttgatttggcactgtagtacctccttggtttgaagtagagggaccagaaagcgattccaccccttgattcggatttaggacagagggattatgtcccataattgtcctggtttgaaagtggtttgtaagaggtatagccggttgacatatttggcctactaacttattcattgtttcgtttaacgtctttagctgtttggccatattgtcatagtgtccatttccattttgtgtaaatctttccatattatgaatacttcgaagatttacctgtttgacgacgtcttgcgtgagttctccaagcaatgcacgcatggttcgaggactcaactccgtcattggttcgtaacgactgttactgctctgattttgtccatctgttcgtggagaggcatgctgctcctcatatcgctcgattatagactggattcctccctgacttgctccttccttgttggatctctgaggcatattgtttcaccttttgtactttcaacacttaacagcactgtcccactgggcgtgccaatttgtttcgcgcggattgagtcgctaacaattaaaaaggatcagacgattgtgtaagggacgaaacctcttgagacaaagtcccaaaaatgggtgttcttttattggcgatgaactttacaattggaaatgaaaaacagcgtgcctcccaagggcgcaagcacacgagttacagaaagaaaaatgtttaagtctaaaagctaaggaaatgaaaattacatattctctgttcgagagttttggattcggtcctttgcttctgcgtcctttctcccttttatacctcatagacgatctctttgtgattaactaccctaaaaattgcttgattgtcctataactacccactttctttgtagtggccattttgtcatgaaactgccttttaactgctgccattatctttcatcgttcaaccgctttcgattgaattccttgagtcgtagaacgtgataaggctactttaacaactgccttgataactgcattccttgataaccacgatgcgttatgtttgttgataccttgggcgacttgaaggtttgggcgagagtagaataacagctctgggcgactgtatgacactccattcgttcagattctgggcgacttgcaaacttgggcgatgacgttaccgcattcttgggccccttatttgggccttcaccttgattcgttcgattggacatcgttctttgggctatccgatttggggatcctccaattgggctttacttcttggactgttcgattttggctgaatttttatgtgtcaacagatatcatttttttttttatgttttttcaaaactttatgttttccctagaataactttttcatttttcaccatattaccgacaaaataaagtatttaccaatggtttggttcccctggaacttttattatttttatttttttagttaccaatggaatcacgtgttgaaaaatcctcagaaaaatattaatttatttaattgttgaatggattatctatgaattttaacgccaaaattcttctgtcgagaaatcccttggtacttaaatattgatgtttgcaaaaataagaaaaagttattgtttattatcgtttggtaaattttcattaacaatagtgcacaatcaagctcattgaatagcatctgaatgtcgtgtttgtgttacaaatgatatgtgcatttatcgtgtgaactctatatacttaggccatgtgataagtgcaatttcccagccaatttactatgattttatgttttcaaagtattaaatttaacttaaattgggttaattttctcttgtttcagttttgaactcatttctaagcaattggaaaagagagaatgattaattggccattgaatgaaggtttggggactaatatgcacttgaataaaagtggaggatcaaaataaaagaaagaatgaagaaatagggccaaagctcaatttttggaaatattcgcatgactaggtgacagcacagttacttaggcctggggatcgcagggacgtgtgaaataaaaacaaatgcctgggcgaccgcccatcgcccaagcgaaacgcgaactatatatatatttttttctttcttaaatttcactccaacaaagaaacctaatcttgggcctttatttgcacaaactttagagacttttggaactccttgaagaggcatatgaatgtaacgtgtgaacacacacacaaacacaaaaaaagattgaaaaattgattgcaaaaaagacaaagaataatgcaagatcgaattcaagaaatacaagaattccgggtgatgagtaatctttatttcttttgttttctttccattaacatgttaggctaaagtagttttgtgctaggatttcgatgaactttgtattataaaactttaacttttaaatcttctttttgatataaaaggacgttttcaattctttaatggttgtcgtgaagttatgttactctacaattatatgcgtaatagttgtatgaggtttatggctttttctcactctcgaaagattgaaaataaattaggcatcgtgtcaattgtcgtagaatccaataggagatataaatacgtcactatctttatgtattcataaatactaaatgtattcttgtatgttcgcatctatcataaaaatatagtcatgtcacatgtaaaaatatgtttaattctactcgaaaaagattttaggaatattgatcttcataattcaattgtgttgtcaaattgtaagatttggggttaaaggagaatgatacaagaggatttgagatcttagtgctttttcatcattatattttcatcaaatttgcatgtattataattttgcattgatttttgttacatctggtcttgcatcatgagtagattatttaattgcgattaatttgagaaaaaaaaatcacaattttcattatttcggttaaggctaagttaattcgaaaataaactagtacaatctatattgatatgatacttggactcaaagatcattttactacttattaacaaaccgtgcacttgcgatacttaaaatgaacaataattttcgtaacaagtttttggcggcgttaatagggattgtatttgaatttaatttcatataccttggtacaatttctaattttttgcctatgagaatgcaatattgtagaaggagcgaaccaaaaaactggcatgatatgcttattcaaagaaggaagtttgaagttgggcaataagtcttgctattcaattcagacacaagcttttcctaggcaaattgaggtcaatgtggtaggggccatataccattactcaagtttttccgcatgggatggttgagatcattcatgaaagcaaatacacatttacatttaatgtacagaggttaaagccatattggaacgacagattctcgacaaaaaaagtctactgtcaccttgcaacgttaagtaaatctctcaaaatgtcaagctctaggctataaatcaattgctcaatgggaggcatcccattttcctatctcttatcttttatttcaattgttcattgcataatatatatagctttaggtattgcattagtattctagggtcatgcttaggaactcataatttgcttcgtttttaaaacattttagatgattttcaagtttatcatatgcacacacgaactaatttaggcttaagcatgtgaaataaatcataaaaatactttgccacacactgagggtgtttgggagtgatttttcaccccgaaaatttgtttttttttatcaatatttcactattccagccgtaaaatttgacttcttctctcacaggaagcccccacttttctcctaaaagtaaaaaaatcaattctcaaaatcgctcccaaacgggacctataactcattctaattcatataaaaaaattaaaagtggaggctggtaagcttggcacttgcccagctttaatagtcgagtactcgcccaacctaattaagcaagcccttaacaatcaaactagggggttttacactagatgaaggccccgtattaaagaaaggaggatttgcttaaaaagccttgtcaaccataatatttcgtaaaattgcctatacgaatgctttttgttcaagtagtctatagtctatttgatcatatattaaaagtcttaaatactcttaaattgaaatgactaaaatgcccaatttggagaccaatatttactaaatccccatatataaatccctaaatcctcttcatttttaacgtttccaaccatattttaatcatattaaacccacctttaaatccaactttcttattcttcatatgcattattcttacttataattaatgatcacattttgaagtttctttatttgaaccaagaacaaatcaaatagtgcaaattttgaaggtaggttagcaagaatcgatttcaaacagttgaaggtatgctttaaaaattgaaaattaacggtttcttgttattttctagttgtatactattaaaaaatcaattgagtaagaaaaatttgtcgtaaaatataaaaacggaatggtgccctttttcagtagatgggtgcctttttttgtagcttggttccattgtaatttgacattggtggtattaatacaattgttttcaaattagtcatttcttcattcttttatagcattttattattttaaacaaatttaaatggcacatacacattttaaactacaggatgccgatttttctgcttaaaatctattatgtaacaatatgggttgccttttgtttattattgaagatgtattttatagtattttgttttgacaattaatggagtaatattttatactttgttgttgaattacaaatatggactctagtgcaatgattgtcattcattattttgttgatttcgaaaagagtgatcaaggtggatggatttggaaatggatagaaaatgatgaaaacaccgcaacaaatatttttgtataaaaaactgtttcatgtatagagttgtatgatgaagtccgaaaagcagttaagattgatcccattatgtatgacatcgagatgaaatttctcattcccaacatggcaaaattatcaggtccaccaatgaagattatttacggtatggatgttagttggtttctctctttgcatgaaaaagttccaatctgtgtaacccttgtggaaattggttattttgatcaacaagacatgaagcttaattttgtaaatgtttaggaggatcatgaatacaattcaaacattgttgtagataatgtggaagacatggatgaattgaatatgcaaaaagataagtccgatgataattatatgggacggttgtctccatttaatcaaatttgggaactttacaagtgattgttattaggatgggatggaaatagtgcatggcaactacatagataattctcatgtgataaatgaagacaatgttagttacaatataccttttacatcagtagatgagattattagcatttcacaggttgttgcttgttcgaatccttatggaacatcagttaagattcctagcggggatgatatgcacgttagtcaatttttttgcaacaagaaggatctctaggcatcactacaaatgcttgctgtaagaaactattttgaattaaggtcactaagtaaaagaagagtacatatatagtagtttgtgttaaaaaaatttgcaaatggcatttgaggacaatagggttgaaggaaagtgacgagtttgaaattcgaaagtattcacattatcaaaatttttcattggatgtttgccacaaagatcataggcaaactagttgttggaagattgaaaaacacatcatgtcgaaacccaacatatatacaaacctacgaacattcaaaatgatatttgtcaagagttttgcatagatataataatttataagccgtggatggctagaaaatgtgctttagagctattaagaggttcacctgatcttagttgtgatagattcctggtatagtggtgttcattgtggttgacattgagaaccgtttcaaatacattttcatatatatatcttcatacagttggcattgttgattctgaaatcgatgtatcatggacttagttctttaataacctgtttcaagtaacgggtatgttggaagggcttggtcttttctgatcgcaagggtagcattggtaatgttataaagattgtttattcttatgcgcatcgtggatgttgtatgtgacatctataactaaacataaagtccaattatcatatcttcatacatttggcattgttgattctgatcatggacttagttctttaataacctgtttcaggtaacgggtatgttggaagggcttggtcttttctgatcgcaaggatagcattggtaatgttataaagattgtttattcttatgcacatcgtggatgttgtatgtgacatctataactaaacataaagtccaattatcaatatgactgatattttgccattgtttatggcaactacaaaggagtatagcttgattaattttgaaagatcataggaaaatctatatcgtaaagtttgatagctggagaatacatagaaaaaaagttgggtatgaattttgatctcgagcacatttcaaaggaattcgttacaatattatgacaacaaataatgtagaatctttgaactcattattcaagattgctcgcgagttttcagtacttgctatggttgagcaaattagaaagattttactgaaatggctttatgggagatacattgaggctgaaaaaaatgtgtaactactctaaccttacctattgaggatagcatgcgcaaaaagtatgatgatgcaaagggactaatagtggtaccaataaatgagtatgagttacacgtcggtgttgaaaatgaaattcatagtgttaacttggaggcaagaacctgtacttgtagagaatttgatttggaaaagcttccttgcaaacatgcacgtgcagtagcaaagtttaagaaaatatcttgttacagtttttgatcacttattaaactagtactagttggaaacaaccatatgccgatgcatatatctggtagcaaatgaggctgactggaaatctccaatcaaacaaaggtgttactacccctttagaattgacgacgaagtggacattcaaaaaactatcgaattccatcaacaatagaaggcaaaaaactcataaatgtagtaggtgtggtcataagggctataatcatctaacttgcaaaaatgttgtaaactagttgacagatcaatggaaccttttttgttgaatttaatcttgaaattgtgataaattatgattatttttgatacactgaaacggttttctcataaattcttaatttttgataaatatgacaacatcacaatttgttaatgccaaaatggcattaggtcactttaaacatacaggacatttctactcatttcttgtatgttttggtacattcaagcccataaacacttgaaagttgaaggatgaaagttctaactacatttcgatgttatggttgacacatttgtccaagttatagcaagtcactctataattcggttggaaaaaataaactgtactactcttcacttgaaaataaagaaaaacgtaattggcaagtgcgatatgcaaaatatagcacgtgtagtcgttcaactgtataagacgtatatgatgtttcaaacactattttaatagtttcagagtaaaattgatacttcctaacccaaaacggcaccaagtcattgtaaacgtacaggctatgtttctactcattccatattcgtttcaatgcattcaaggccataaactcttgaaagttgaagaatgaaaagttctaactacatttcaacgttacgatcgacgtatttatccaaactatagtgagttactctataattcaatcgaaaactatactacattaaacttcacttaactataaagaaaaatataagtggcaagtacggtatgcaaaacatagcacgtgtagttgttcaatgtgtataggacgtgtatgattgataaatgcattttactcacttatttatgccacaaaataaggacaattgttagtaattattttggaatatggcttaattctgtataaattatagttcgtaggacaacaatgataaatgtgacagaatctaggaaaaataagtggaaaaggatcaaaaaggaagaaaatcaaagtttagggaccaaaatgcaaatagccaaaagatgagcgaaaaacataaacaaggatatgagagagttaagaactaatttggtgaaaacgtagagtattggatgaagaacaaatgaatagaaaggtcaagaaacgagaaaatggagttcaggggctgaattgcaacttttgaaaagtttccaatactatgcggtcgcatagtataaaactccatgctgttgcacatctatttttagcaagtcccagggctaaaatcaattgaactatgtagttgcattgaaatgtactatgcagtcgcatagtataaacttggcgggaaaaaatctagtttccttatttaattaaaatttttatggaaacaaattgtagaacctatataaaaaccttagagcaatttcaaggaagaacacattgagaacatagagaacacattttgaaggagattttgagctaaaaacacgaggagaaacacgaaaattgatgggattatgcgaataattcaagagaaatattaaatcggtgatatcgttttttcaaatttctttgtgttttactactttccccatgttatgctagataattctatactaagagaacgatgaaccatgtgatgtaaatttttgacttctagttttacaatattggcaatagaacacgtttcttaaattttgaatattttatatgcaattaaattcttccataattatgtgcgcttgattatgagagtttggtggcttatttcatgtatttgagagaaggaaaatagtttgacaaggtataaaccatcatagggtccgataggggatagagatataccgttatgccctgcgtgaatctctaagtgttcacaaaatctcatacattcttgtatatttgtagccattatagagatatagtcggtggtgtatgagagtaggttcaacattcgagagagattgttggatagaataggagcattgattcttcaaatcttcaagcatgttgtcaatttgtagaactagggttaaaagtaagcgttgcatggggatttgcaatcctagtgcgcctttcattcgtgaatatcatcaactttgcatttaaacttcaattttcattttaattaatttaattcatacacattctcatatatagcctaggttagttataatcacgttacaaaaatcatgtttggtaatttcgtttcgattaaggccaagataggtaaaattaagcttactcaatctctgtggaacgatattcaaaactcttcattccactttattacttgttacgaaccatacacttgcggtattaaaattgaaataataatttcgtgaacaagtttttgactctgttgccagagattgagttttagtttgattttatttattttgacactaatttggacttctacctgtattcttgtatagttattttcattttatttttattttttttctcttttttatgatatataaatatcaaaaagatcaaaaacagcaagaacaaatggctaatgaacaaaataacgcgataatttgagctaatgaagaggaagatgtggaggagggaaatatgcttgttggggatttcacgaccccacaaatcattcaaagccaatccagcattgtgtatccaccgtttggacagctaaagaccaacgtcatacacttatttcaaaatggacatcagttttatggcagagttgagaaaaacccaacacatacgtctctcgattcttagatatatgtcaacacttcagatataaggtatatcaaatgacactatcagattgaggctattcccacataccttgtgtgataaatcaattgagtggctggattctcaaccaatcgctagtattaccaccaggaatgacttagagcaaaaattctacacaaagttcttcccgtccgccaaaatagcaaaatcaaagcatgacatctctatcttccatcaaggtgactctgaatcctttgatgaagcctggaatacgttcaaaaacatgcttcaaaaatgtccacataatgggatcactctaggttcaatatttctatgcgggactactaccatctttcaaaagtatggttgattctttgtctaacggatcgttgtcaataaaaaccattttcaaagcgttgaaactatttgagacagtggctactacttcagttatgtggggatcagaacgagttgttcaaaagaaggtaccaggcatatatgaaatggatgctattcaaccctatttgcaaaaatagattttctattccataaggagaaaagcgtatcacaatcagggaatgcaatatataagtgaaaacaaagttgtaaaaaatgtggagtgaatcataatatagcagaatgcttaattctatcatagggaatgaaataagtagagtacgcacaatggtgtcaatgtcaacaaaactatctgatttcagacacttacaatctcggttgaagagagcatccaaatctctcgtggggtcgtaaccaaaataaatttgaaaattagaatagacttcaggggcaatttcagcaagagaagacatttcagttggaagagatgtttccgaagttcatggaaagaattgataaatacatggaagcaaataaccaattcatgaggaaaactgaaattactctccaaaaccagggtgctgcaattaagaacatggagaagcagatggaactttctatgatgagaagggcacctggtactttgccaagcaatactaaagtgaatcccagggagtatgttcaagcaattattacaaaaagtggggttcaattactagaaatgaatatgaagagatcaaatgctgacaaaaaacaatacctcattctgatgaggagcagattgactagaccagagaaacaactaccaatgaaagttcagatacaccattggctaaagcactgctcttgtcaatccatacgagtccccaattccattttctcagatattgaagaagtataagatggatcaacagtacatgaatttttttggagatcttcaagaaacttcacataaacattccattcgctgaggcaattacccatctacccaactatgccaaattcttgaaggacgtcctatccaacaaacgcatactgaaggagcatgaaatggtgatgttgacagaggaatgcagcgctggcatttagaaaagttacctccaaagctaaatgatccaaggagttttattgtaccctgcactatatgaaattgctactttaatagagctttatgtgatttgggtgctagtattaacttgatgccactatatgttttcagaaaactaggattgtgagaacctaaggcaactgcggtgactctacagctgactgatcgatcactcactcatccataaggaatcattgaatatgttttggaaaaggtggataaactcatattttcaatatatttcctaattctagacatggaagaagacaaggcatgctgctcatattgggtcgatcatttttagctactataaaagctcttatagatgtgcagcgagggcaattaatttgagtttgggagaggagtgggtttctttcaatgttttcaaagagatgaaatatcctattgagtcagacagctgcttccagattgaggtggttgacagcataattcacgacaattttaagttacagaaccttcagacgttttatgaggcctgtattatgcattctcaatctactttcactgacttgaaggagattgaggtatacaatgttgagttccaaatgaatgataagggggagtcacacttcttggagaaggacaaagttaaaatttggagggaaattgcagcaggaaaaaaggtcatattgagtgaactatgcaggacctcgaaggctatattcaaagtgccatgacataattgtgttaaaagtcaagctcagactataaatctagcgcttcataggaggcaactcattttcaatcccttttcacttattttgattagctattgcattacacggatttttagagatcacgttagtatttagggctatggtaaggaactcatgcatgttgatgatttttaacacattttaggctgtattttaagacttgcattagtaacttaggcatttttatctatcgagttcaatttatttaggctcatcattaacatcctaacattatgttgagcttacattgatgtgataaacattcttaaggttgcacttacatttcaatttccaaacgaattagaaaaaacttatcatctcctagctatatgattttcgtacgctttgttagatttgtgaattcattgcaaatatttaaaccttatatgctatcactaatatctattttatattcttataatagcaaattaaagcctagcaacaaggaaaagtgatggttgacctcttccaggtgtgccaccttgatccttctacctgttcgcatatgccctggtgagtttcaaattcgaactactttattttgattattttttctattttattaacaacaatatcttgtatagtttggaggtggcaaaatcttcaggacactttcgacattcatcaatgtttgtgtagaatttacttcttttttttttgtcatcgtttatgtgaaaaaaatttgtagttttacttatattgttttatgtgcttgtgcgggtttgatagctttttcggcaatgatattgaatattggaataggtaaggactaggaatagtggaaataacacatgattagattatccaatacttgtttatgtgaaacttgacattctttgtgcacaacactaatgctctacacgttgagctagtgattggattcttgaacagagaaggataaaccctaaaaacctttattatattgacccataatccatttttagagtagttttgaaatgattgagcaattgcaggagaatattgagataagtaggggttccatgcatgaaattataccgagtggattgcctaagaccaagtagatgaagattaggtgaaagtcttatgttaaagggtggttttggagactgaatgtctagaaaaaagggcataatattaagttgtgctagaataatacctctcaaagcctttatgattgagcatgtaagcctgtaacaaatctggtgccctaacgctaactggtttgggagtcatcggtttaaaacgcgttacaagagtcatatagaaagcaagaaggagaaaagttaataaaaatcatcttatcgagtctttataacttgagtgagtaagcctgcaaggatttaaaacttggtaccctaaagtcaactgacttaagagccatcaacctaaaagctcgttataagggttatatagaaaacaaatgagaagatagcaaaacaataataattgaaaatcagtgaacaaagacgcaatgacagtaagtaagcccttagacatttggttgatagaactacatatttgatgcgaggcaaatagcttaatttagtcttaaatgttgaaacaatcaaaatatgagagcctttacttgttgaaatgcgaacttgtaatagtgagatctatccaaattgagagatagtaaggattaaagttacttaaactcctaacttcagaacataccccaggataattgagtgaaaagaataagtttagaggtgtgtatctctcaagcgaagaaatgatatatttgaccactacgggttgggaataaccgaatcatggacccgatatgttgacatgagttcacagacacacgtcaagctgtgcatttacaagtgaaggttgattttttttttgcactgtgaaaactgtttcttgtgttggttactgaattctaaacctgagacacagcaggttgtcaaggcatgttttgtgtagagttatttgaggacaaacaatagttcaagtttgggaggtttgataagtgcgttttacacacttatttaggtcacaaaacatagacaattgttagtaattatgttagaatatggtttaattctgtataaattatgtttcgtatgacaacattgttaaatgtggagagatctaggaaaaacaagcgaaaaaggacccaaatggaagaaaatcaaagttcagggaccaaaatgcaaataataaagaaatgaccgaaaaacataaacaagtatgtgaaagagttaatgaccaatttggttaaaatatatagtattggaagaagaataagaaatgaaaagaacggtccagaaacaagaaaatggagttcacggactaaattgcaacatttgggaagtttccaatactatgcggtcatagagtataaaactccatgcggttgcacacttattttcagagttttagggccaaaattgattgaactatgcagtcgcattgaaacatactatgcagtcacatagtacaaacccagggggaaaaatctggtttccttatttgattaaaattcttatggaaacaaatcgtagaatctatatagaaaccctaaagctgtaaattttcaaggaggaacacattgagaacatagagcacattttgaaggaaattttaacccaaatgagtagaaattattcttgatcttttatttaactcatatgattattcttgattttttatttaactcatatgaaaatcaactagggagtgatctcatacggaagataaacattgattgcaaagatactaaaagataattcttgataattgtttgagagaatatgtcaaaataatttgttggtatgtagagattatctaagcatttattgtgccaatttgtcaacaataaatcaaagtctttaacaaatcaaaactatttgtattacatatacttcaaacaagtgagaagatgaacactgaagaacaaaatgaaagatcaaagactataatacacattcatcaaagtttcactcctagctctagctaaaagtttagaaatacataataaaatgttacagagaaaatgaatgaaactagaatatgatgaagagaaattgatgccctcaaactcttagctagggtccccttttataggcaaaggaacatccaacatccaagtagataatttgcaacttgtttctatccagcttgaagacaattggaacatgcaacttgatactaattttcaaatatggtttgtagtgaatttggatttttgatcaataaataaattgttgccactcaagttatatttccatttgtgcaaatatcaggtccattgaatctctacaactccagatatagccaaaacaatgactgctactcacaatatggactttgcacggtaattttggctaccatatgatgataatttgacttcttagtaaacatgaaagttgtagatacatactttgttgttccaatccaacttgaatcaccttggttcaatatctatagctcatgttatgagcattttaccgagacagctgcatcttacttgagtcgactcatcattttacttttcaacattttttctccacttgctctacttgctctacattggaaatacatttgaaatacatcaaataaatactctttccaaagtataatactcatgtcgatatgtatgtaaatacatatttcgattaattgcgcttttaaccatgtatttatgcaaattgaatttatggcaagagaattgaaattagagactaacattagtaaatttatacaaaatgaatgtaaaatgtcttgtagatgatatattattgaagcacttttagatgataatcaacaggaactggttcatttaccaacaaattatatgctacttgtctccgctcattgccatcttcattcatcatttttcccttctactggaattggatcctcatttacatcatatgcctctttagtattcatgaatccactacgaagaggagagtgatatttgtaaggtattgatgggttagaattcttaattcaatgtacaacagatgatacattctcgtcaatttgtctatacaaaaatataatataatcaaacctttgatctacgtaagaaagtatctcatctattcgcctttcaatttttcctctttaaagtgtctaccatttgtactaatttcctgaacaaactcacctctagatggataaagagatggatatgatgtagacggtcctggatgaaacgtatgaacatatgtagaagtaggtggcctatgaaatgaagaaggatcatgaggagatgtagagacattaggagactgacaagtttgctgaggaaaatcaacacaaatggacgaatctgctccatatacattatccacaaagataataactattgatcatttacttcatccctgaatcgatgaatctctgtccaatttgctttagaagcctcttcctctgtaggctttagtgtgcaatgaacaatctatataataaaggagatgtccacttagttttcatgaagtacattatatgttttaatatacatttagaatatacttacatttggtttgtccaaacttgtacaaatattcttggagctaggcattttagaagaatttcatcgacatattttgagaaggtcagtcttctctaaattttcagaatatctccatccaatagatggtatggcttcataggcccaaatctatataagattcaaaatattacaatataaacaaaatgaataataaattgcgactttaaaagcattacctgcaaggctatcaaaaatccataaactgaacatggatatttttcattatttatcaagtatgacttcaccaagaatctccagtctctcatgaatatatctattgtgtggctaaaagcctttctcccccaaggataaatattaaaagcctctaagtaatcaaccattgacaagtgttctaaatttacgtatctgtagttttctttgtgcaatagtatcgtttccaaaatatatacgaacccaatctagtacttgtcttccatatacactttgcgactttcaatagcttccttcaaattgtacaccttatgcctttcttacactttttaaagaatttcttcaccaatctatctttaaagtcccaaatattttcatagaatagaattatttattttatctgctatattttaaattttggaaagtcaggggactgaagtgatatatgtattaatacaattttgtttgggccaaatagttagatttcgatagggcgaaaaagagtatatcaatatggggcttgttggatagttcgtaattaatcatatatattaggctcgagaaaaagttatttcggataagtgaagcttaagttattaaagtttaaaggatttttaattaactagtatttgatagttaaattggtcatggaatttaaaagtttggtagccacgttggtatctagataaaggaaaagcatcttttatttgattatgataagaactttttggaatcctattgaaatttcatattgttttacaggtagtttaggtgacctactttctataggatttttcataagaccaaatatatatatatatatatatatatatatatatatatatatatatatatatatatatatatatataaatgggagcaggtttgaaaaaaggatcttagagtgtccagggttgggctaggaaggtctcttaacgccttctttttcttctcatcggagttgtttcacaaagactcgtagggtaaagaagaaggggggttttctctttcatggccacatatctttccgactaagaaatggaaaatctttgtcctgttacatgaactgataaaggacgtatggattctcgagaagaaaggagccgtggtggtccctccaaatcatccccgcaggttattttctcaataaataagtaactgtaggagttcaatcttgatgtaatttgaaaaagcaaacaagaggtccaagacaataaatgaactactaaactcagtggttagagtattgctttcatacggggggagtcatttgtaccaagatttcgtgattcgctaccaaacttattccaattccaagagctcggatcaaatcggtatatccttctccttccttttttcgaaagaaaaggaggatccgaacaaaatcgatgaagcagaagaaatccgagtgaatggaaaggaaaaaaacaggatgaattccactttacagttagatacaaaattatctattcttgaaacaggaattaaagtagtagatcttttagccccttgtcgtcgtatttttccatagaaatatattcgttcaagaagagctccaaaagatgttgatcgtaaatgagaagattggttacgtagaaagagtatttagccttacaaggtggtccttgttgattcacacgggattccatgtgatgaatattctactatagtgggtattcaagaatcggtccaacgactggagtgggagattcagagtcgaaaagaggatttctcacttctttcgatatataaaagatccatctgtatacatatcatcatctacatccaaaaagtcgtatactttggaagaagcttgtacagtttggaaagcgtggagctaaaataattcaatcagaacgctttttaaaggattacgtgttagaaaatttttaccacaaaagcattatacctattaatcaaagtagagttcgcacccattaatcattattttcagattatagatacgagtgatttgagaaaaagatttcaaaatttaattgatccaacaaggtaggtacaaaggcgcagtcgcttttatcctgtttaaattgtttattttcatgttgttcaattattatgcttatgaaagtttacagatataatatgatatgtatgttatgaccatctgataccaaagatatgatgcttattgagttcttactgatttttaaagatatgatgaccatatgaaattttggcacatgtatttaaatatttttgtttgggattccaccatgatattttgtgtcctactaagtatcccttgtactcattctttttccctactcctccaaaattagaacatatcgttagttggcgggcgatgagatgcgagcgcaatgccagaaattatggaacccaataataataatttggtgaaatttgacagtggattttatttcaatatttgttttagtttcgttattgttgcgaaaattgctatttagagttaaaagcatgtttgtttggttatgtttcctatacgttttatttatcattggtagaacaaaaatttcatgttgggatgttgatgcgtttatttaaattatgtaatgaatttttagtaacgatttaaatcttaaaatttaggtcattacactatcattagtcacaatatggggctccaacgaaggctcctcactagctgttaacctcattatcaatgagaactcgtataataaaaatcctattggcttactaccaattgaaaaccagatctcattttgttttttggttacaatcattctcatttcaaattggtggactggctgggatgaaaaaggtatgcgattcattcgatatagttgtccgaaacaagattccatcaatatttcttggtgaacatcatctaacgtttctcaaacatagtcaagttttcgaaggaaacacttctgtgaatgcctgtctttaattctatcttcaatgagaatcacatactcaaatgagcattccatttctgtaattaaaaacataaaacgatcttgttgaattatcaatgaacaaatatgaagattttaagtaatggtaggtgatacttaatacaatccattaaaaaaaaaggataaaccacaaggtgacatttttaaattacataaacagcagggtgccatttttagatttgtttgtaagttatatactaaactatttaatttcaaaaaattggatcaacttcctagcttgcattaaatcacaagctgcacttttcgagcattttgttcatctgaagtgatttttgttggagcttttaagagctttatgaattcctaaagaagacatgaaaatttcaactgtctaccattattctgctacaatcagaagtttcttactagaactgtgttcaagtgtatgtatagattttagtttttgtcttttaagtagtttttagcatcatttttcaaagtttagcattctagcttctgccattgttcaatcataattgcgatttaataatcctcctatagaattgtgaattaaaatctcctttatctgaacatttggatcgataaactatagaaaactctaaaaagattaccaaattagctaataaatatattgaaaacccacatttccattgtgtaatgccccgaaaattttggtcggatggaatttaattttgtatgctatattttaatgttctgaaagtttagggactaaagtatatataaagtaaatttctattttatttgggttaaaatgtagatattgacggagcgataataagtctatgaatattgagctcgttggatagatcgtaatgaatcacgcacattaaactcgagaaaaaatcgatttggataagtcagcaacaagaaatttcaatttgaagaaattgataaaaattagttttcaaatcagtaaaaacttggaaggaagatgtgctgttgagacttgtgtgcatggaattatcttgattttgaattgtgtgcacgtgtagaaatggttatgaataaaaagaggtaggtttattttaatatttatttgctttgattttggagaaagaaaagggtgattctccttgattttagggattgcttattttagtattatttaattgcttgattttacggattgatagactccacgtgatgattagataaggggaaaacaactgtagataagtagattaaacgagattgaggcattttaggggaaaagcacgtcatggaataatgggatatagacggttacacggtacttcccttttctatttaagtaccgtaaataaatatgtatattatctaccatgaagagaaaaagaaatatggatgcatgtcatagtagcaacaacaaatacaaaaacaatagtttggaacgcgaatttggatattctctttcaaaaactgatttatctcacgaggtaggatatcgaggtgcagtgtttttctaccctgtctaaatatttttcatgttgatgaattttatactcatgaaaattaaagttatgatatgaatgatatggtcatttcagtacaacaatataatatgatatgatatgaattcttactggatttaaagatataagatgatatgattttctgatacatgttttaaaatttttatacgggattgcaccattaataattatatgctactgagtattctcatgtactcgtccttttttcctacttctcacagattagaacgagtcgtttgttgatgggcaaggaggtgcaatcgtgatgctagaaatcatggaattcaaaataaataaattcggagtaacataactatggacttttatttttttagcgcagttttatcttcatgtgaaatttgaaatttaagatttgggacatgttttagttaattatgtttttcatatgttttatttattatatagatggaactagaaagattttcatgttgaatgtttgatttaatttatttaattatggaataaagattttagtaatgattttaaatctttaaattttgggttgttatagtttggtatcagagcaaaggcttaattttttgcagaatcatatgtaatttcataatttgagtgttaaaataaatataaaaataataataataataaatttgagcctttcaatcactgttggtacactttcatataacatggttaagcatctttcactccccgtcaccaacctcatccccccttgtctaattcatacgacatcaatttgacctcaaattcgaacatgaataagaccaacatataatcttttatatatccggagattgcttgggaaaagtcaatattttttcacattttccggtgatgaaaatccttagtcagttctgggaaaaaacgcgaaattctctcttttatgttggtttagggagtatgcgccatattttcttcatctatagaatacataccctacatcgtgataatttctagagcatgacatgagcttttatactttggtgcatgaaaattggtatataatagtatagtttcgggggtgttctccactttatcctaattttctggttgttaccttttatgctgctaatttacattttcatatccatgtagatacaaattgctaccaaaaagagaagtctcaattcaatagaaaggaaagtctaaggttggtgagacattaaacgatcgttagaggacgaacaaaaatcttgacaatggagacatacttcggtttttaaactttaaaatcatgaaaattttgaggtgaaaaggaaggataaaaagctatatcaagagaggcaggttatatttggtgactttcagggaactctacttgcacgaattatacaacactggtaggagaaagatttttgaaactcctcatgcgacataacccaccttaaggagttcttcaccaacttcaacatagagattgataccctagagtcctccaacagaaattagacatgggtgagaggaaagtagatccagttcggcccagtggtgattgacaaatgttatgagttgaaccacacatatgtagagctcctatgggctgagcaagacatggcgctaggagtccaatttttatatggtggggatgttgaatggccacttcctacatctcatttcatgcataagaagttgatcccagagttgagaatcttgcatagcatcgtcgaaaccaatatccagaaagcttctgatgctttactcatttattttaattatttttgctcttatagtgtagacaatgtaattttttttgttttcggttgggtaagtattaggatatttagaatttttatttcatacttttcaactgtttactgggtctgtataactattttaatttaaaaaaaaaaatcaaaacaaaaaataaaaaataaaaaaaaagtgtctagtatagtgttgaatgatttgtcgctgatgatatctatttgtttgaatcaagtacaactttagctaaaattcgacaacatcgtatcttatgcttttatttgagtacttatctatggtagacttgtttacttgagcacatagccatattggcttagcacttatgttgggacatgacttgattatgtggatttaattgttgatgttattaacctatacttgagtgaatttctaaatccttattatagaaatcaaaatgctaaaaattagtttgggaatgagaaggttagtgcttgtattcaaagaagtttgatggtttggagttctcaaatcccgcattggatgaaggagtttgagtcaaggaaactagaatgggtactgaccagttttaacattcgaacctcatatcaaagaaaaatgtgatgcatcttgtacttctcatcgttgagtttttatgatttgaattacaaagcctagaggggtatctaaaaatctagtgccttatagtcatctgacttggaaatcatcgactaaaactcgctatatgagtcatttagagaagtttaatggagaaaggtcttgtatataaaatttaaaaatgacgaaaagaaagtatgatacattctatacttttatttgtagctttattactcgagcaattaagcttaaatggtatctaaaacctattgccctatagtcatttgattcagaagtctcaacctgaagcccgctacagggtcatttatcaagcctaatggagagaagtcatatgcaagagatgccaaaaggactagattgattgcgttctagtactggtgtgagttcaacgtcagctaataacacacatactaagtctaacatcatataagtaaaaaaattattttcgatgtttgattttttctaaagttataagtaaatttgaacctgaggtgtatgaaaagcagttcaacgttgagtcttttatacatgatttgtttagatagtcatatgttttatgcacaagattatttttgttttgttcgaggacaaacaaagattttggtgtttgataagtatattgtgtattaatctaattattaagattttatgtcgtcaaagtgttaaattgtacctaatttgggtttattttctcttgttaattttgggcccatttctaagcagttggaaaaaagagaaggatcaattggccattggatggaagtttggggactaatatacatttgaataaaagtagaggatcaaaatcaaggaaataatgaagaaaatgcgccaaagtgcaatctttggaaatattcgcttaaccgggcgacagttcagttatttaggcatgtgaactaaaaacagaggctgaatcatatgcctgagcaatagctcggtcgcctaagccgaaagcgaagagaatttttttttttttttttcgtttttaaatttaatccaacaaggaaacgtaatcttgggcctttatttgcacaatttttagagacttttgggactttaaccaaaaaactaataaaaataaataaaactaaaaaggtttgaagaattgatttcaaaaagaggcaaaaagaaaagaaaaaaaagagagagagagagagagagagagagagatcgaattcaagaagtctaaagaataaatccaagaatttcgggtgatgaattatctttatttcttttgtttactttctattaacatgttaggctaaagtatttttgtgttataattttgatgaaccttgtattttaaaactttgacttttgattcttgtatttggatgttaaagcacgttttcaatttttgaatggtagtcatggatttatgtttctctacaatcatatgcacaatagttgtatgagctttgtaacttgttttgctttcaaaagattgaaaataaattagacatcgtgtcaattttcgtagaattcaatatagaatagaaatataccactatactccacgtaatctttatatattcattatattcgcatctgtcataaaaatatagtcgggtcatatgtgaaaatatgtttatgtctactcaagagaaaattgttaaacagtttagaaatattgatattaataattgaatcgtgtttcaaattacaagattcagggttaaagagaattgatacaagggatcctaatgcgttttttatcgttatattttcatcaaacttgcatcaattataactttgcattgattttagttatgctcggtcttgcattcataagtatattatttaattataatttaatttgagaaaaaaatcacaattttattttttcggttaaggctattaatttgaacttgaactattacaatctttgtggacataatacttggactaaaaaattcattcaactatttgttaacgaacttgcactagtgatatttaaaacaaacaataattctcctaacactttgtttgaggtccttttttcgtgaaaaatgagttttgaaggaaaaattttgaatttctgtgaaaattattttattgggttaatatatggttaaaaataaatttgtataaatgagtttttagggaacgaggctcaaacatgggcttagtggagtctgcatattggtgtcactagaaagtatagttattttactgctgggaaagttcatttatactaggactaattgatcagaaaagctactactttctctagatcgtagagcataattatccacaaaatcgaccaaacctgcccggaaaacctcagtcttagggttgtgttgtaagaaaaaaattatttcaaaagtaaaataccctcaaaatcgacaaaccgaaccgatttgatcagttcgggtcagttttcagttgagatttcacccagccaaaactttcagtatggtgataggattgggtacaaacttggcccgtccccagccctacatgtagaaaaatgctcatgtattcaatcaatgaactatgctattcctgatcacgtgatgcatacaaatttactttctggctatgtgagattctatatataaataccattataagcaggcaagctatgaataacaagaagttccatgtaggtccttgactgatgttcatcattgttaggatttatgttgtattgacaattctttagacaaaatgactaatatgaaaacttgtaaaattcaaggagtcaattggaatattgtatagataaaataggtaatttagggttcaagtttggaacaaagagaaaagagctgccggatttactcaaacctatcgcccatttcatgcttgagcggctaaaacagaaactctattgcccgcctgtcgttgagctatcgcttgaatgatagaccatcacctgcctgccgcttaactctcgctcgagtgacggtgttatgcaaaaactcctagttcgcattttttaagagttttattcggcacatactacttaaatgccttctattataaatacccaagtcttaacacatatttagtggtggttgttcaatacatgcctcttcataacattattccaatattcaagaagacatgtaagcttgtgatatatccattgattattgagttcatacaaccacatatttggaaaaaacatcaacttcatataatccagaacacccacttcttatacacgtacgaaagatactttctcaatagcttttagagattattgaagactatgggaggttggaccagaaacaaaggaagattacaagaataaggtgttcttggtgatctataagagagacaatttcagaagatcgggaagaggtgagtgaaacatgttccagttggttttgaagattgtagaaagtagatcagtgaatctagtggaattttcgagactagattgtactgtaagtatatcatttatatagttaggtttctccatcaacaattcttgtgctatttactgctttattaatgtttgtggcaattcagcgtaggatgctttaacttattttattaaccatctagacgcaattaaaaagtgatttgttgcttttaataattatttttatttcgcagtattcacctattcaccccctctagatgatattagggtcgaacctgtaactctcaatcaccaatctctacaacgaagtttatcctactttgtggagttaggctagtggtggcaagccggctcggctcttaacctcacgaactcagctcgttttcaacgagtcgagcttgggctcggcttgttgattttgggcgagctcgtggcccgagccgagctttgcctcgtgggctagtcttttttttttttttttataaagagaaaaacacaaataaatgaaataatgtaatgaaaaaactttaaaaaaaaataaaatttgttaaaaaaatacaaataatttaatgaagacacttttttatttttttttatttatatcatattgtaatatttttttataaagtataaaatatttatataatgaagacgaattattttttgaaatacatttacaaaaaatatatttttttgatttctttttaaagtaaataaaatgtaaactctcctcctttattcgggcttggaatcggctacatcaattttaaataagcggagttaaaaattgtacacgaacaatttgttgtaacatgtacaattttttaaagaaaattaaatttaaagattaaaaataaagaaattttaattaatataattaaatcaaatatcacttaccttactacatgcaatttcagtgtatttatcttgtagtcgaaaatgagcgttctgtcaatccttcacgcacattaactctttcaaaacatcttctttcagtcggctcctgacatcggtcaaaactcttttacctgtactaaaagcatattctgaagcaatagtgctaaccggaggtgtcaggggatctttcgcaattacagaaacaattggccagcatcttttatactttcgctagtattcaattacttcttctgaacttgttttaattgttctgtatgttggcatattatgattgaagtaatcaattaattcggcaagcatcacattttgagtttcggtcgatgtttgatgagatgcaaatgtagacgacatagcactaaataaacgcattgcagttgcatcatatctaaatgtattaatgccttgaaataaattcattatttcggcattatcttcttcaatttcagccgaaggagtaagtgcagggggtactcgactaacattcgcacccattcttttcgcatataaatcatacattccacataatgtttgatctaaattcttataggtgataggtgtatcaagtattaaagttttattgatttgatcaattacgtatttagttcccgaaatattatatcggaggtccattgcgtatgctaaaggaaataatataggcagttcttcccaatattttctaaactttaatcccataacaattataatttcactaaaaataggatcatttttatatttatggaatatttttgcaattatataaaagcgttcaagtaccatacatcttgtgtgataataaacgctggataaaatttttgtggtctcataaaaagatgtcaaaatcgtttaacttccaaagttaaaatccaatcggattcatttaatataccatcgtcgtcacttctaatgtgtctattgttataaaagtcagttattaaattttcgaaacctttacatgactttaataacaagtaagtagagtttcatctatgacctacgtcactaacaaatgttttagcagtcgttaccccctagttcggcacaaaaatcttcaaattcttgttttctactaggagagatcgtaatatatactaatgcattcctaattctttgaaattcatcatttatatgttttaaaacatcttgcacaattaaattcaagatatgacacaaacaacgaatataaaacaaatacctaccaaaatcaggttgaagtgtcctacacaatttatcgacgactactttattaacactagcattattaaaagtaaaaaaatcgaattttagtctcacaattatattttctaacaatactgataataagattatatatattattagcattgtaaggaaactcaataattctaaaagcaataattttcttatgcatgcactaaagtgggtctatatagtgtgcagttgcagctatatatacttttttattaaccccttcccatttatcagaagttaaagatataatacccccatattgttgcaaatccataattaattgttattttgaattattgaaatattgtattgtatcggcacgaagagtgtttcgacttaccccaacgtaccttggctgcaaatattttttcacaaacgagacgaagtgttggttgtctgcaatagccagaggcaactcaatggcggcagcaaatttcaccattccggttcgagtattgttctccgaatacaccaacatggataggggtgaagtcatagaaccggcgcatgaactgcaaaattgcaattatgtttgaccagctggaagaagtctatgtctggccgcacatgctttgtagtggcggttgagatgagtggtaccaattcctttttgccatgtcaatctttgttggcagtatttacatactgctttagattctgcaacgccatcaacggctttttccgttgaaatcaacttaaagtgatctcaacattttgcttgtttttgccctttcgctttccccttgcatctgggatgtttaattcaatatcttcgtcctcatattccgcttcgggaacgttaatattatctaaatcaattggattgtgacttccctgaccatgaatgtgttcaatcttcaggtatgagtatgtcatttagaccgacaaatttatttgaaaattaactttgtggcatcctagacgattcgtcatgatgtggcccacatcccgtatcgaataatctctcaacaaatgaacgtcggttcatttgtttgattgtttatgatgaaattcaaatataataactagaaaaatataaatgtagtgagattgtaagaattgagaattggatgaattgaaattgtaactaataaaattataaaaattgaatcgatattgtatattttgcagaacaagagagtaaaaactcgataagagagttgagagagttgaagtagtgattgagtaattgatatgaaaagaaagggtgagtcaaggggtttttatagtagaagggaaaaaaaaataaaaaaaataaatttcaatgatcgtttggtcactaaaaaaacggtcactgaaaagttttagtgaccgaacggtcacttaattataacaagccatgagccgctcgtcccagcgaggctcgctcggctcgcgctcgggctcgtgattttacgagtccgagccacccacgagccctatttcgacgagctgagcgtcggctcgacccttttgacatccctaagttaggctattgattgtaattccacaaatgcatggtataatagccaaatagtaatgtagtaaataaaatatcactttaaggactgagtacttggtatagttctaattactactaactctaattgaatagtttacttgtgaatcattaattttatgctaattatctaaactaatttaacgaagcaattatgaagcgtttgtaaaatcaaaatcacactttattaatccatattaacataaaagaccatgataacacttctttactcttgtcggtcaatatttctattttattcaataatctctcttgagtagaatttgaacttttcccgaaatatgacctcttatgtctcaatgaaagatatgaacatgaaacaatacattaaaacaaaagaacatccatttaaatcatacaaagctagttttatatctctataccaaattgaaaattacaatgattgttataacgtgctatattccttattcattctctcaaataaaataaagataacacatcatcaattcatttggcgggcaattaacgtaaaaacattaaaacctataataattattcaagataaacaaatattaaatgtcaaaattttgaaattgcattgaaatgtatatgttttagaacagtttaagtatgaattcattcttaattgcacttatggttgattatgagttcaattgtgtaagttagctaccttaggttcttttaagattgttgaaaattttattactaatcacccaattagaaccctattgaaactccatttagaataagtttgggggttattagattcatctaaaaccatgaacatcataactttattgttttttggttcttatagttggcctaaaatagttaaacatattgtaatagtcatggcacgtagaaaaaatctacatacattgtatatgaagctggtctagattaatttggtcgtactcgctaaaaatgtccaggagataacatatcaggaaagaaggttacccacactaagagtgaaaactatattaaaaaattagaaagatattagaaagagaagaagggacaataaagggaagaaagtaaaatatatctaagtgtgttgagacagcaccaaaacaactataagtattgtcttagcccaactagtctttgtcattgattaagaattaaaagatcctcactaaaataaatataactttttcagcacttaaaagacaacattcattaattgaatgttgcaaaatgtgtctactacaacgttaaaatatgtgaatgttgacattagtatgtgtctattacaacgttaaaatatgtgaatgttgacattagttaaaataattgagatttgacaacatttttaagatgttgttgctaatgtcatctttttgcaacgtttatttagtgttgccaaaagttttatttttcataacgtttaatgtccgctgttgaaggttcaactttttgcaatgttttctaaacgttgagaaagatttatctttttgcaacttatgaaaacgttgcgaaaagataaatctttcgcaatagtagacgaacgttgcaaacagatatattcacaacagaatataaacattgcaaaaagggaaccttttcgcaacgtctactaagcgttgcgaaaatatctttcgcaatgttttctaaaacgttgtgaaaatatctatcacaacgttttacagcgaaagatcaacctacacagacccaattaaaagatcagcccacaagacccaaactattttatggcccattaaaagacccaattcaattacaccctaatctcacacacacgaccgaagaattcagcttttgtggcacttctcatcgccttcttctacctgcaacttttcattgccttcttctacctgcaaactcgtccctctcacagcacaagctaatctcaactcgtttagcacgctcacaggcagtgaggaaggcttcgacagttgcaattgggtaactgctttacatttttttttggtcttcgatttattgctggttctgcttctattcgaaccaagtgaagagtgtaccactggtagcaagatattggattcaatgatttgggaaaagatggtgaggaaacctgatactcaggacctccagtttacgattaaacacaatgactgttgaaccaataattttggggctacattaaaagaaatttcatggttatgtctggtctgatattcaggacctgatgtctggtctgttgaaccaaaaaactaattaaatctacttttggtagtaaacaagcttagaaagaaaagttggaagatttcaggcagttaactggttgggaagcatcagcaagcagtatttttgtgcggtttgatgatttaatctaacgcctattttttggtttctcttatttttgtgcggtttgatgatttaatctaacgcctgatttgcaacatagggcccaacgttgtaaaaagtcttattttgttgtagtgcctatctcttttttcttttgcctttagggaaattaaaaaataaactgagcagaacaagtgatgagagtatatttgcataattaggatttgatattggttagaaacagatattccggaagttaaatcacataattccattcaagtggtgttgatgaaatatgattaacacacacattcgaaagctgaataaaagatttgtaaagaaataattcttcgttctcgtgtttcattaacttgtttaaattttgtgaattagatatgcattttgaggaaacattagttacttaatttgagttgagtatatttgtgtagagtcaagttaattgtctattatgccttattcgaggaaaaaaagtttggggatatttgacaagtgtaaatattacatttatctacgccatcaaaactcacttttgggagcatttttatgaacttgatgattaattatgtgtatttttggataatgctaggaaaaaacccggtattggaaaaagtgttgataaaaaggatacaatttggaatttttttattacagttttggaatcaaattctacacttgaaatcgaatgacttgacatgaaataaagaaagttttgaactgcacaataaagtggatccagggactataattgtaatttcctaaagaattgtggctttggtgagattacaagcctgtttgggagtgattttgataattgatttgttgaccgttaggagaaaagtggggtccatctgtgaaagaatatgtcaaatatgacggctggaatagtaaaataacgattaaaaaatcaattttttgggtaaaaaaatcgggcccaaacagcccctacatcatcaattggcccggaaaaattgaatctggatgggagtgaataaattgccgggaggaatttaaatgggagtaaaattcttggaaatagagaagaaagctggcggcagaaattagggaggaactaaggcacaattactcctccgttccatttgtatgagttgattttatttttcaaacggattacaaaattttaatgttattgaaaagaaaatttttgcaaacaattttcctgatttatcttatttaattatcaacaactagtagtagcataaaaaataatggtgattaaattattgttggaacttggaagtattaaagaagtgggaaatactatgaaccacttaaactttactccctttgtgaactctgtgcatgtatttggatgattccagggagtatgtaaattaaaatctgtaaaatttcaagattaaatgggaaaaactgattataattaattaggcaaattaaataagggtatattagtaaactaatgaaataagtatattttcaacaaagaaacaggactataatttgggacaagaaattaaagaaagtcattttatataaatgagaagagggtgtacaagaaaaaggagaagaaaatttcaaaatttgcatgcaaaaatcattgacaattgtgtaggaaatttaggatttaattatggaacgtcattaaacttttgggagatcataataattaatgaaggagaagacgaactattgttacgattcatataacgaagaataatacgaggagtaatttttatcttgttctttgtagttgaaccatgttatgtcttttaacctttatttgattaattttgaattggctagatacatattgttaggatgaatgatatagattagacttttagtatttatttaaattcaaatgtttcgtgtgactccaatatctattaattatttattgcatttttgttgctttctaataagtgcatttgtgcacttattcgagccaaattactaaactttcatgtcgttaaagtattaaattttacttaatttgagttctcttgtttcagttttggaacgattcataagccattagaaaagaaaaaagaataaattgatgattgggttgaaggtttggagactttttgcacatcagaagaagttaaaggatcaaaataagcataatttgtactggatgaccaaaataaaagaaagaatgaagaaaatgattaaaaagcgaattttgaaattcattatgattgggcacctgcccagttataatatctgggcgaccacccgacttgaagtttcaaaagcatggatgaattaatgtgcttaggctgtaggcactcacccagtccaattgatgcaaagggtccatttttcgtttcgaattcttcgccaacaaggactcttcttcttgggccaattttggacatttttgaaagctttttggagactttcgaaaggcctataaaagaaatttatcagctctaaattagagggataaatataccattccattcatcttatattcatcataaaaattcatctttttggagccaaaaactagaattttcattggacaactcatcaggattgaagattaagtgtgaagacagagttataccattagattttcttcttctccaggttatgaattccatcttttgtattagtttttccctctttatcatgctatgctagatttatttctgatgcctaggttttcgatgaatcttgtactacgaagctttaggccatgttctcttttctattttcaatccgttttctattttcgattttggaaaatagtgaaaacgcgttctcttttccgtttttgaaaatgaattttggaaaaaaaaatttgtaaagaaaatgcaaaacgtcaaaatcgacattttggacgttttctgtacaaaatccaaaaatggtcgaaaacgcggaaaataggagagagaaaaccattcaagccgtgtctcttccgtctccctttctctcttccttcaactgtctcttcctcctcccttctcgacgccggcaccaacttacctgcaccatttgaattatagctttcctcatgaacacgacgctacaaccaagctcttttattggggtattcatttttcccttgacgacattgttcaagcttcttgccgtctcgacagtgaaatccaaatactcaaggttttcctgtctttctcgctcttcttgcgtgagaaattagattataactttgtcttgttaagtgatatacaatttaatttctttaggaagagttgtagaaaacgaatctgccaatttgagtttttgtaggttaagattacattctgtgattttcttttaatgctactaaaatgagctaaatggtttccagtttaccaatagttcagggaataagtaactggtgtaacgtggggaattttggttgattttggcggtgacaatggttgattgttcatgatggtggtgttgattttggccgtggttgatggtggtagtgactggtggtggcgttgtggtggtgttgattttggtcggctttgtggtggttatttcaataaaacattataaaaaacttttctcaaaatttcaaaacaaatgcgcttttcatttttgtgttttgagaaacaattttgcagaatgacagaaagaacgtatttttaacaatttcaaaataggcactcaaaacgcaaaattcaaaatgaattcaaaactcaaaactacaaaattgaaacacaaagaaaacaacacattaacttttgaatcttatttttgatgttaaagcacgttttcaattcttgaatggttgtcatggatttatgtttctcttaaattttatttacaatagctgtatgagttttgtaacatattttaccttcgaaagattgaaaataagttagactaatgtcaattgtcgcagagtctgataaggtatagaaatatacaagcacgctctacgtgatctttaagtacttataaatccttaatgcgttcttgtaggttcgcatatgtcatagatatatagtcaaaccacatgtgataataagtttaattttgctagagagagattgtaaacaattaaatataaattagagttcaactctaattttaaaacttaagacggttgaatttcattaaaattaaattttaattaaataacaaaattagaatccaactctaaggtccagatattagggcgaacttatttaattaaaatcaaattttaattgaatattaaattagagtccaactctaattcataagtatattaggatgagattatttaattaaaatcaaattctaactaaatatcgaattagactctaactctaagtgcaattgaattaaaattttaatttaggataaaattcctaaataaaataaaattcaatttatagtcaaagttttatatttaagttaaactccaattttaatgaaaatataaaaaggtcgtccattttaaataaatttttcaaagggtcaaagttgaaaatatgggtcaaatgattttcaaaatcaatttaaaaacccttatcctttttgaaaaattttatttgacccaatttaaaattataaccaaatccttccactttaaaaaattgcagaataggtccctgcagaatcagcttgcgcggttgcgttgccacagccattatcgctgctgtatatgattgattacaactttgcatttattttaattaaattaggtatcgcattcattacaactttacattggttttagttaagttaggtcttgcattcgtaattagattatttgattacaatttagtaattgaaaattgtcaattttcatagtttcgataaatgcaaagttaattcaaactcgaactagtacaatctctttgggtatgataattgttaaggaactgtgcacttgtggtatttcaaatgaaagaatatattcacaacactttatattgtctacgcatcaactaattgattagggataatactaagattgagagataatttactaattaactcgttcaataaatagcataggtattataagagatttatggataattatgggctatggaattttggtcgaactttgttacttgatacattcatgtgtatgaatttaaatagaaatatattaaattcgtgacatacgaataaagttagttttgcttgaaagagatcattaactataattggttaattcgattgtttgatagatataaaagggactaaatgaattgagattagatgaaaattaaatgacataagtgaaatcgaagtttctaactatttaatcttataatcttctcaaacgttatataagtagattaccttagattaatttggttcattttacagaacttaaaaaacaataataataataataaataaataaatgaaataaaaactttgataattgattaccgattaaaattgatgaaaatttatattgaataatagtctttgtggtactttgactcaattttctactttattacttgttactatccctacacttatggaatcatgtgacacataaccaagatgaaactaaaatagtgtaattgcgccctgaagtgtcaaagcatttgtcacaccttcactgtgagaaaagataatattgatatagaaaaattaaggcaggacagtatatatatctggcctgaactaaagaaacagtttgtgaactctttctctgggaaccaacacagagaagctcatgcagcctggattcatgatattagataagaagaggtagggtctctaaaaagatatctgaatacttttgttgagaatttaatcaaaattttcaatttccaccaaaatcttctgtgttgagagataaaatttgataaagaattataccttttgatgactttcttaaagagcatttctgatctgtaatccacaactatctaatcctccaacctccaatggaatctatataggaaacaagattgaaagaactatggttttcttttcttgtgctagcaaaaatatgaattgtattccctacaaattttgaaaccctagcatcctattaatataagttttggttaacttggtccgtatcttaattttaatccagttcaatatttaattaatacaattaactaaatttggtctatgaatgaataaatgaattaattaattaatttaggcctattaacaagcaaccaaactaattacttgtccaacaatttttaattaattaattggtaaatctcatttttctagtttcccttttgtgtatgacacattaggtttccgatcacgatacgcaataatgtgaattattattttgatcaattcaaaattgataaattaaaatacccatttttaatttatcatcgattcacatccgtcatcccaaattgacatatagcaatgtgttaggacaatatgtatgacgaaaaatgttacgtgatatgataaaatcaaatttatttatttatcgtgaaactataatcatttcgtcaatatgatccgatcaattatatatatatcgattatatcattcatcatactattaagtcaacgtaagttgaaaattgactttttcaacttatgagtatacattgatcaagaatttcgttatcaatttaattgaatgaaatatagttcataatctcttactatctaaaagtgacgaatcctttattgatcattcataactttcatatgattcttaatatatgtaaacgataccgtattggtgatccttggcaaagcaacatccaacatcatcaaagtatgtttgtcttctataaggtactatgatgaactcaagtcgaatgatcaattctactactgaatgtaaggtatttaccaatgacactcatatagttatcaatgtaaaatctttttagtgggtctccaatattttgtcatacaacgaaacatccatttgctcatataagtgtaatcgcgctttagtttgtgagatcaattacttatttcacaagaaagaaatgacagtttatccgtaataacaatatttgtatcatattattacttacgaccagggatgatttaagattcagtcatatgttatttgtatttcacaatcacaaccccttgtgatgagcaaattaccaatacttgaatctatgaattctattatttaatttattaaaatattaattaaattaaataattgatttgtcataaatgaaatgcatcaattatatattaaaagtctttatattcaaagtttattagatatagggcataatagttacacatatttctataaacaatttatcatgagaaaaacaacagatttttttttttttttttttttttgtagaatatgagctctagatagaaacatcatctgggaggatgtgtgcaataagaaaccaccaaccactagcggaactggaggggtcctcgggtgtttgatgacccccaacttttgagatttatttttttggataaagttacgtttggtatggcttgaaatttatattttaatttaaattaaagttaacgattaattttaatagtcatggaatccttaactttttaaattatattaaaatttaattttaattcctaccaaacagagacaaaatcacaataaatttgaattgttctcttttctcttgctatatcttactctcttcctcacacattttaccaaaatcttaatccttctaattttttaaaatttatctataattttctaaaaattatcacatatacaacaaattttcacttttcaattaattagaaccttcatttgcatactttcctatcctattggtgtatatagaatgtgcctgagttgactatatctaaatttaacttatatttaaggaattgtatttatttgattgattactagtattgaatattgattatacattttttctttcgattacttgaattaattctttatatcaaatacaatgtaaattttttaaacgcaaatatgcattttcttgttatgaacaaaatataaataaaatgacagttcgaaatcaaatggctgaaaatgatgagcataatattaatgaagaaatgtttttttaaatgaaaatctacattttctcaggtgaagtatgaattgttcgaaaatcaagaacaaattattcaatttatacagagtttaattgtgcccctaactcaaattatctacgtctgcccctgccaccaactatgtcaaatcgtagagattataaaaaatgacatttagataagtaacagaaatttggaaaataatgtccaacccaatgaaaaaagcgtgactcctttgcagtcggtagtacaacctcctagaaactgttacccgaggtgcaatagatataattgagatgaggtgaatattgtaaataataatgttatctagttctgttagtgctaaaataccagtttagttgatgttaagtgatagatttaatgaaatgtagaattaaatgattcatttaattatactctcatttaatgccagattagtattacttagatggattttttaacaccattattactaaataggattactctattgtaaatcctgcaccaactctcaagtcaagcatcaaacaggggcttcatttgactaatgggagatataacagatggggaacatgcatattggtgttattattccaagaactcgaagaatacacaaagtatacttcaaagaatatcattgtaaaattacggactcaaaaaatctattgacacaaagatttcatcgactcatgggctcagtaaccattgtacccttctgtacaaactaagagacccaaaatatacccaaaccctacacaggaaaatcgaacgcagttgcttcgacggaccagtagggaaaacccccctttataatagcaacccttatccctttcacaagaatcactaagattcccacagaattaactctgaatcactaaagaaatcagaaaaaatcacaaagaagacgactcagaaagagaaccagaaagtcgacctttctagagagttcaggaggcagaaagagagtgatcgaatcccttagggcaaaccatcagccttttatttatataaaatatcatcaccgttgatattacttaggagatccaatggtccggagcaacacacgtggccaaacgttgggctagggttttgggcttcttgtttgagttattgggcaatgggttgtagtatctacaatgggcttagcccgatttatcatcatagcccaatgttgagttataattccaaaaattggcatcacaactctaacactctctaccttgatgccaatgactaaaacaggaaacttcacataaaagaaaataataactccagtatgtccctccttatccaggtcccttatattcactgcatcaagatggttcacatactacgtgcaattcacacagaatttacccagtatcaatcttcagaattttcaaacaagatttaaacttgttaagagggagtacctttgtccccatgtcagctggattgaattcagtgggtatcttttcaagtgcaatagtattattatgaattatatcacgaataaaatgcattctaacatctatatgttttgtcctttcatgaaaaacagggttcttgcacagatgaatgacactctgactatctgagtatactactacaggatgtgacaaaacatttaattcacataataaacctttaagccataatgcctcttttatggcttcagtggcagccacatattctgcttcagtagtagatagtgcaacaatagactgtaattgtgatttccaactcacacaagtgtcacacaaagtaaacatgtaagatgtggttgattttctattgtctctgtcccctgcataattagaatcaacaaagccctttaacacaataccttctttacatggattaaaacataaacccaagttagaagacccttttaagtatctaagtaaccacttcaaggcagtccaatgtttagggccgggattggccatgaatctacttaaggtactgatagcatgagcaacatcaggtctggtacataccatagtatacataacagaccccacagcattagaataagggacttttttcatatatttcacatcagattcatcaacaggagactgatctttacttaatttaaaatgacttgcaagtggtaaagtaacagacttagattcatgcatagcaaatttagataacactttttccacataggaagattgtgtgagaaagagagtctgttgagacctatttctcttaatatccatacctaggatccttctagcatggcccaagtctttcatttcaaattcagaagataaagatcttttaatgtcattaatatcactcatatattgacctattaacaacatatcatccacatacaaaagcaggtaaacagttacagaatcattttaatcctttttaaagtataaacaatgatcaaatgagctcctaaggaaaccaactgatgatacaaagttatcaaaacgtttataccactgtcttggtgattgtttaaacccatacaaagatctttttaataaacacacaaaatcagatttcttagactcaatgaaacctggtggctgacacatataaatggtttcatccaaatttccatgcaaaaaagcagtttttacatccatttgttcaagttctaagtcaaaatgagctactaaagcaagcatgactctaatggttgtatacttaaccacaggtgagaagatttcattataatcaatcccaggtttttgtgtaaaaccctttgccactaatctggctttaaacctaatgggctgtttcaaattattaccctcttttatgttataaatccacttacagtcaactatggatttgtcttttggcttggggaccagggtccaggtattattctttaacaaagagttcatttcttcttccatggctagctgccactcttttgacagctcacaactcatagcctcatatgatttaagttctttaaaagcaagatcttgaaataacaataaggctagagatagatagtctctcattctaagaggttccctaatttctctcctttctctatccctagctaactgatagtcttctaagggattttcttctccacctacttcttgaacagatatattttcttcagttttagcttctgaaacttcttcaattttagcctcaatttcatcagtgtgttctgaaggtgttttcagctccacctgcagcctggtttcctcattttttatcagttacaggttcaggtttttgatgttttccagacatgcagggcatatcacactcattaaatgtcacatttctacttgtgatcatcctaaaccccttaacactcttatcccatagcctatatcctttcacaccctcaggatatcccataaaaacacattttatggatctaggttcaagtttaccaatactttgatgagagaatgcagcacaaccaaaaattttaaggtgactgtaatctggagtttttccagaccacacctcctcaagggttttaccatctaaggcactagaaggagttctattaatgatatacgcagctgtcatagctgcctcgccccacaatactttagggacagcagaactgatcatcatacatctaaccttgtctagaatggtcctattcatcctctcaacaactccattttgctgaggggtataaggtacagttttatgcctaaggaccccactaactttgcataattgatcaaaatcagcattacaaaattctagaccattatcagttcttaaaattttcattttcttccctatctgattttcaatcaatgttttccaagctttaaatttttcaaatgtatctgacttctgttttaacagaaaaatccaaacctttcttgaaaaatcatcaattaaagatagaaaatatttgttttcacctcggctaacagtagaagagggcccccataaatcagcatgtacatactccagaattgaagtagtcttatgccttccagtattagaatgaagtctatgttgtttaccaagtgtgcagtgttcacaaaatggaatttttgaaatattattttttccaaagacaccttttttattcagaatacgcagacctctttcacttacatgagctaatctgttgtgccattttaaagtggcatcaacttcagcagttgaggattcagcaatgtgacatgaaataacttcagctccagtgacatatattccattgcttttggcacccttgaaaattacaagtgagcctttaattatttttaacaatccattgcctagtttggcttgcaggccaatgtcatctagatttcccattgaaattaaatttctgtttaagtcagggacatatcttactctttatagagtaaagatatatccattttcaaatttcaaagtcacactaccaattcctaaaactttacatgctgcattattacccattaccacctcaccaccatttatttctttaaagtcttctaaccatgaccttttagaggtcatatgaaaggtgcagccagaatcaagtatccactcttgactctggtcattattaccagaaaaataaacagtattcaggtcagatatggattctgtaacaacatagacatccatagttttatctctttggggctctactacattgccctgatccactctcttttctctctgttcattctttttcttgtagcagtcttcaataaaatgaccagtttttccacatccataacactttctattttcagtcctagaccttgacctaggtcttcctttccatttcttctttatattgttactcccttgattatattgattttcatgactaccaccttgcctagtaagtgatctacctctaacaaataaactttcaggttcccttccatgcctttcagatttaagttttaattctttacttcttaaagaattaataacaactttaggggttaactcatccccactatacttaattgcagttttaacatctttataggtttcaggtaatgagtttagaagaataacagctttgtattcttcagaaactttatcacccgcattagttatatcttgaaccagtttattaaagatgtcaagattgtcttctaaatctttggaagggtctattttaaaactgaaaaaactttccaaaaggaatattttatttggcaaagattttgttaaatatagttcttcaagtttatcccataaatctttagccttatcaagttttccaacctttcttaacacttggtcagataaatgcagtatgatagaggtataggcaagttcatcagattctgttttttgttcttcagtcatagtctcaggaaaatcaagagttatagcttttacaactttctgttgaacaaaaatccctctcattttttgttgccaaatggggaaatccccttttccattaaaaaccccaagttcaaacttagtagttgacatttgaagttcttaatcaacgcaagaaaaattattgaaggttcaatgttcagcaagaaagtagatacagaataagaaatttgacaatacttaaagtcagacaagttattcaataccaagaagtttcaagaatcaaaggaaaaagtataagtgcacaaagtattcacaatatcaagaagtagcagtatgttcaatgcaatacacttcaggccttaaatgcccaagttcaccaggattccgtgaggatcatgtcctcaggtcaaggctcaacttagggcatcaagaccaaaagcaggaaatgatattaccaatgtttcacatagaaccagaacacaaatgcagtttacaaattgtgtaactacagatgtatatcatatgtacaacacgaacaaaaaaaattgattaagtgttatgctaggtcaaaactgcaaaccaaacaatagtagtcgagtcaggactaccaattcaccaagaatgcctcgagtctgatgttggtcacccgatgatagtcgtgaaaccctcagttcgctaatcgggagctgcaagaactaacagagacaacacgaagttaaccaatatcagttgagaaaagaaaacaaaaaatatggaaataaactcagagatataagatctgaaatcaatcgaacagatctaggttcggtcacatgagactcttaagatctgactgtgaaaataaatttttcacaaccagatcacaatcgaaccaagtcaacatgccacagctggctctgataccactattattccaagaactcgaagaatacacaaagtatacttcaaagaatatcactgtaaaattacagactcaaaaaatctattgacacaaagatttcattgactcatgggctcaataaccattgtacccttctgtacaaactaggagacccaaaatatacccaaaccctacacaggaaaatcgaacgcagttgcttcgacggaacagtaggaaaaacccccctttataatagcaacccttatccctttcacaagaatcactaagattcccacagaattaactctgaatcactaaagaaatcagaaaaaatcacaaagaagacaactcagaaagagaaccataaagtcggcctttctagagagttcaggaggcagaaagagagtgatcgaatcccttagggcaaaccatcagccttttatttatataaaatatcatcaccgttgatattacttaggagatccaatggtccggagcaacacacgtggccaaacgttgggctcgggttttgtgtctcttgtttgagttatcaggcaaagggttgtagtatctgcaatgggcttagcccaatttatcatcatagcccaatgttgagttataattccaaaaattggcatcacaactctaacaggtgtgatgtaatgtgttttgaatataaagagaaaaaaacgtctaaaaaggagagtggatgtttaacactcgaagctctagggactcgtgacattattgagatcttaaatttgcacaattctatctagattgttcataaaaatgtggaaattaccttgtaccagaagcacttagactttagagaatccattgtaaaacaaaagaaattttcttttaaaaagaaacagattttcggcttgtacaactttctgaaaaaaatctgttcggcaatcaaatgaaatccagaatttacaaaattcaaactctaggcaatttacacataggaaaattacagtttaaaatttcctatgcaaattcaatagctagataggtcaaaattattttcataaggggatctcccttttttttttttttttttttttccgtggtagtccttgggaaaacgtcaataacatgatttttacacaatcaaaattcatgattccgattccgagagataaataatacatatggcaccttttccaactagaattacctcaaaccttttagtattttggtcggggtgaatttttaaatttaggggcaaaaactgaatatttcaaaaaatagtcttgccacacaattgaaccaaattaaccacaaaacaatatccgatccatcttaaacaaatttccatttcataattaaatctttaatcatgcgaaaaataccaaattaaaatatgtcagaagtttaaataattatttgaacccaacttgacttaaatgatgatttttggagttcacatcaaggcaccactgctctcctctactctgccatcagtccattaatctgaaattagtagggggttgagtttttcatagaaacacccaatagactcatacacatgctaaatccaaacatattatactctaagcatatatacatgtcattcaaacttttaatgagtaagcatatcgatggttaggatacatacaaacatttggtgcactactgtgccatcaacttcacatttctagtacactaccatagcaccatctcatatttgaaccccacaaggagccatatataatatataatcacatttatacacactaaaatatcccaaaaattgaaataaaacagggtttaagtctacctcttttgaaacaaatgttagtgtttgagtatcgtgtatgtctcctttacttgaattttaattcgtaaactatttgatttgtgtgtgtatatctttgttgttgtgttatcaagggaaaattgaatgaaacaataaaatgtggagatgattgaggacacaccatgcatgagatatacttatagtatcggacgttgagataggttgtcatagtacaactaaatatactaataactaaccattaattcaaattctccagtaaaaacttcgtcaggataaggataattttaaaataaatcaactgattatggatagtccatttagcactggccaaaaatcaaaacaaaaggaatgaaattccttcaaaattcaatgacatagtcttaattttactttctctaacttggttctccttatttgaatgacttcttctcgagcctaatatacatgcttaattataaggcattaaatgagcccaatatcgatatagtaattctcacaactgcaataatttaataataaatattgcaatattgtgcgtttgatagaaacaagaaatcttaactagctctaataagaattaagtgataaaacataacataaatgaactataatttgtaacaaaatatttcaaaggcaaccaagtaactaacatggactaaaataagtcaacgtacttaattacatgaccacttagtgaacataaattggaaaaatttacaacgacgcgaatttatctcttataaaattttggtaaaaaaaaaatatatatatatacactatcatttttaaatatgaaaatctttcgtttgctacaaccctttcctcttaatttgatttcgtcctcaaaatttaacttacttgggttataaatctctgtgtacttggtctcaatttcttcttctctctcctaagtagccttttctatcgtatgattaaaccaccagacccttagtaatggcacttctctatatctcagcttgtagaccttcctttctaatatctcagttggttttttctcatacattagtctttctataaatcaatcgacggacccttggccacttgactagagtcatgaagatattttctcaacacagcgatgtgaaaacatcatgtacaattgatagttctggtagcaatgccaaacaagacgccacattttcaactctatctagaatttcaaatgggctgataaatatcaatctcaacttccctttcttttcaaatcatattacatccttcattgatgccacctttacaaaaattttatctatgacctaaaatgctagtgctttcattctcttattggcataactttttctgactattttgagctatcttaattctcattctgatctttttatagcctcaactattttctcaacaaggtcaggatctagcattttccatttactcacttcatcctagtataccgacgaatgacacaataggccatataaagcctcctacggtgctatctaaacagtagcataaaaactattattgtatgaaaattctataaacaacaagtgaatttcccaatttccaccccaatctaagatacaagctctcaacatatcttctaaaacttggatggttcattccaattgcccatcggtatgagaatggtaaacattactaaatgtcaacttaattccatcgtcatttgtacattcttccaaaacttcaatgtaaacctcgaatttctatctgatatagtcaatactggtactccatggagtctgaccatctctttaacatagagatgtgcaaattgatctatattaaaattcattctgaccgagagaaggtgaatggactctatcaatcaatccatagcgtcctgacccttcattggcctagggaaccctaccgcgaagtccattgctattttctcccatttctattttagtatatttataggattctattccccaaatcgcctctgatgctcggttttaacctgttgacaaacaaaacactttgatacgaaacgaactattctacctttcatgttcctcgaccaaaatgaataatgtagatctcaatatattttggtcctgccttgatgtgttgctcaagggcaaagcgagcttctgttatagtctcactacgaagtccttcatctctaggtacatagagtcaacatatatatattaacatcttatcctcgactatctcaaaatctttcattttttgtgtttgatcgtagcccgggtcatccttttaggcctttatcactttggccttaagtgttaagctttagagttaatgttgctaacctcaccacttttttaactggtggcattagtacctcaatttttaaattttcaaaatccttaattaactgtttttgttctactctcaaaattgataactaacccttatttgtcctacttagttcttctgctactacattagccttattaggatggtaatggatagtgtagttgtagtccttcactagttccaggcatcatctttgtctcatatctaaatccttttgagtgaagaagtatttaatattctcatgatcagtgtaaattttgcactcgctcctataaaaatagtgacgccaaattttaagggcatgacctactgctgcaagttccaaatcatgtattgaatagtttcatttatactacttcaaccaccttgatgtataggctattacctttccattagcctcaacacacaccccaaactaaacttggatgcattgctataaataacaagtccatatgaacctttaggcatagctaatatggagcagaaactagtccgctctttaactcttgaaagcttttcgaacttaacttatttacaggtcaattgtgtcaaaggccctgcaatttttgagaaaacttcaatgaatcgttcacagtagcaagctaaacctagaaagctcctcacttatactacagtagtagataccagccaattattcacatcatcaactttagctgggtatacttcaattccatgggcaatcaatacatgacttagaaatcctattctatctaaccaaaattcaaactttttgaatttagcgtaaagtttttcctagcttaaagtctccaacactgttctcagatgttcttccttctggttaaaatcctttaagtaaagtaatgtataattgataaacataatgaaaaactaatcaagatactgctaaaatacttgattaattaagtccataaacaaactagaggtattagttaagctaataggcataactgtgaactcatagtgcccttagtaaattcggaatgccatctttaatgtaacactctatttaatctttaactgatggcagcttgatctcacattgatctttgaaattgttgtagtttcctttaactgatcaaataaatctctagttcttggaagtggatacttattcttaatagtcaatttatttaactctctataatctatgcacatcattatcgacccatcattctttttaacaaatagtacaagagctccccatggggacatgcttggccttataaaacccttactactcaattttttgccacgcgtcttctacaatgtgatttatactgcaagtatacggtgtcaagttttgtaatatagtaatggagttaagagagtcaaacccatatggattgtaattcaatttctaataattacgtagctccactttatttagatgagtggaatttggaatcaatggtttaaacaaagttaatgcaatgaatgtggtgacaaacttaataatcaattgcaagttagaagaataatcaagatgaaaaagcctagggttgtgatttcacctaactatcaaatatgattctcaaatatataattatttctaatcaattttttaatgtttataagcaaaaactaaaaaatatttctatctcttctctcgagtgtcggctagaaattaatcctagatttcaactccaatatctctattccgaattaaaatcaagaatttatcaaattcatagttcttttatggagtaagcttcatagatcctatactttcactcaaaacccataaaatctacattgtgttaatcatatgatcgtgtctaaattcccctttctcgagtgccagaattgactagtatctattcattcaattagtggccaattaactgaaagcattaaaatcataatacaaataaacagaaaggaaaatttcatagaaataactataacaaaatcaaatcatagtcttaagttttggctaatcatatcctagaagaattatttagttcatgatataatctatgaaaaatactaaaattcatataagaagacatagggaagagaatagaaaaaattgattgtaaatctttaatttttttttcctgttcttctttgccttgttcttgaatcttttggtattttgcctccttgccctcttgaaatttttttttcaaaatttacctccatattgtggtctttaggtttgtatttatagtaatttgaagtcttggatgtataggattgaattgggccaataaaagagtccaaaaacatatttaaaaaaaaaacacttttttctacaaggtggtgtcgtggcgccaacttcgggtagaaagaagagactatgcattctttaatattttttatcataacttttttttttcgatatccaattgagataattcaagatgccttgaaaagataactcaaagggatgcaactttgcttcaaatatcattttcaaatttgatagttttctatttcaaaaatgggtttcaatatgaggctgaaaatatgtgcataacttttttcggttagaaattgatgtgtgatcatattttgattatatttcatcattttgatatctttctttatccaattagctttgagcattcttcaatcttcatcgtgaggtttgacacaactattgattatttgcactttagtccccaaactttggatctcttacaacttgctatttttcccaatttggttaacttttgcttatttttttcaatatcatcaacctatacaacaacatcaaatatcctcaaacttaatattttgcttgtccttgagcaaacaccaaactaaaaaaaaaacttacatacacataagcaaatgaatacaaacaaaatcacttaaaacaatgtgctatatatcttgcctttatagctcaggattgaaaacataacattaatttcatgaatcactttaagattataatgtacaagctaaattttcacctattcaatacaaaacgggtgtgtgtatgtagagaaccgagtacaacgttgtacaataattagttgatccagtttctgaccttaaaaatcaaatatttacttacttcgctcgtgggatttgaacacccccaaacttgttttcttttcacttcccgagatgtattctaatgttgattttcaatactaatttcttacaccactcaagtttggttagatttacaaattgcagctcaacatatcaactgatgaggattctccttatttttgactgcttcaaccttcaagaatcaaccaaattactaaccctttgtcaaaagcctaaccctctaaaacaagtgtttggagcttaattaagacatgtgtgtgcctttctcctctctttctctctctctctctctctctctttatactcttttctttttccttcatatatgtatatttttaatgaatttattggcagaagtctctccattaagctttctgaatgactcttgtaacgagttttaggtcgatgacccctaattctaattactttagggtaccaagttttaaacccttacatgtttattcatttgagtcataaaggttacgaagagacgtttcacaatgaattattatgattgtcctcattgagcttttttcattagctttacaacaaggcagctttttttccttttatgcagtgattagtgtaatgccctctattaaacactcattctcaaaaatcaaccttcaacttaaggttttcactcaattttaatcctattagtctcagatagtccacacaaaacttagcatacacagaatctacatccacgcccatgtctctctacaacagttcaaacatccaagctatcctaaagttggttaacgggtatggatttttgtttagtggttgtttggatttagcaatctaagctctctatttcaaccaataaatatgaatcaacctactcatgtataacgcttcaatcaactcacgtgcataaatattttccatttcacattaataagcaaaaataaactcaagcacataacttttccacaattcataaaccaacacatgtcctcaattacatacatcaatgtcgacaaggcaatctaactcacacaagcatgcaaatttttttattttttttttggtgtgtaaaaaaatgcacacaagtcacacaaaataaaaaaaaataaaaaacaaattaggccaattagacaatttataatacactcctccccaaacttaaactagacactatccccaatgtgaagttaaaggaaaataaggtgaacttccctgaattgtctatattgtcaatgacgttatggtgctatgatgctggatttgattgatgcttcttctatcttctcccctaaacttgaaattattcagttttttcttgtcaatgttggtttgattgtttcgcagttcatgtttcagaaaaattaaattttagatattagaaatacagaacaagggttagttagctcaaacatctaataacaaacttaattactaaaaaaccaaaaggaagacaggatatagataatgattcctaaataaactgaaaaaataaactaaattatcccataactcaaaagcaaaatgaataaataaaaaagagaaaaacttgggttgcctcttaagaagcacttctttaaagtcattagcttgacttcgacaaatgatcacgggcatctaaagaaggctttggatgccttgtccatttttcttctcttggctttgctccactctttgttatttctccaaacctaggcattatccttttcaattaagtaggaattttccatgccatccaattcaatttcaacaatgtagacttcagtttcctcatcggacttaatcacaaaatgaatttctatacaatcaacgaattcaaatgaatgtatgttacttttatcttcattgatttctacattttcattcagttcgttcgtgatcaagtcgtcattcactttaagcttttctacgatcattcaaatttcttcggattggctgatagattcgtactctagatccacgggcaattagaagtctttgtttttaacctcttcaagtggattgtatttccaccttttgaattcattctagtttacgctcttccaacttggcaagtttattatagtattttgcaattattctctcgttctcacagcaatggttttgattcttttgtcaaatccgagttcttcattcaacagatgaggaccatttcccacaagtacgatgtcctcatcctaatcgataggtacataatctcccaaaggcatgtagtcttcatcaaattttttaattgcttcttttcgacattttgaaatattaggtgtgtaccaccaaaggcaacaaaaatgtgtgaattagacagcacaacatctaccaatgcatagattgctttaacaaaacaggtagagttacttgtaaaattgcaaacacatggagcaaatgcaatgatggccagttcagcatgtgagaattgtgggagaaatcacgctacagagaattgcatgatgctcacttctttagaggaacaagtaaactttattcaaaatagctcctataattgcaactcatatggtatcaatttccagcaagaaagaagaccaagtttgggggagatgtttcaacaatatgtgcaaaagacggacaagatattccaacaaattgacacgaactttcaaaatcagcaatcatccatcaagaaactgggacacaaattggtcagatagcacaacaacttaaagaacgtccacaagggacattcccaggtaatacaatgataaatcttaaggaacagttgatagcaattaaagtagtggagaatgatccacccaggacccccgtaaaagttaaagcatatgtacttccactttcgtttccccaaagacttcaaaagaagtcgatggagcaaaatattcatgtcataaatacaaagagtgaggtacaatcgcctgagatcactacagagagacccaaaagaaaagataaccaagaggtgattgatgaagctacaattgtagaaaaatctgcacagaatgcaactgaaaatggagaaagtacagaaacatcagctgccaaagaacaaagtctagacaaagcttacatgcctcccattccctttcctcaaaagcttaagaagaacaaacaagacagaagctctagatcaatgttccgttcattgatgcgatactccaaatttcaagctatatgaaatttttgaaagagatgttgataaagaaaagaaagctgtcggagtttgaaactgtggcattaactgaggaaagtagtgcaagagtccacagaaaattacctcatagattgaaggatccagggagttttactttaccaatttcaattggaaattcatattcaattaatgcattgtgtgacactggtggtagtatcaatctaatgtcgtattctgctaacaggaaattgggactaggtgaagtcaactcaacatcaataacgctacaactagctgatagaacaatcacaaggtcacgtggcaaagttgaggatgtactcataaaagtaggaaatttaatatttcctgtggatttcattgtattggacataccagaagatcgagacagtccaattatattgggtcgttattcttagcaacgggacgaacccttattgacatggagaagggagaactaatcttgagggtggaagacaaacaggagatattcaatatttatatgtaatatgagaaaccttccaataaaaatgattactatagaattgatgaagaagagccacctgatcaacgaagctgtcagaacaaaaaaaaaatttggagaatttcttggtgaagataagaatggacaaatcaaactttggagagcaaaaaaggattgcatcaatgaaaattgcacaaagtgcaatgatggaataacttggtttgagccaccaagataaatcagcgacacaattcaagctaatgacttaaaagaagcgtttcttgggaggcaatccaatcttttattttatttttattaattttgttttcaaagttctaggatagtttaatttataatttatttaggaatcataacccataccccttctacccataggtcttggagtaattaagttggttattagatgtttgagctaagtaatccttgttccatgagtttaatttttcaaatttaatttttcaggaacatgacgtcgcgaaacactcaaaccaacatggacatggagaaaatgagacaaatctcaagtttgggggagaatgtagaagaagagtcgatcaaatgcaacactaagacaccacaacatcataggcaatactgatatttcagggaagtcctcctccttctcctttaaatttcacattgaggacaatgtttcaattaaatttgggggagtgacatcatttgcttacgttgttgagtttctcgaatgcttatgtgtgattttcttattttatgtgtttgtgtttttattcaaaaaaaaaaaaaaaattcatactcgtcatgcttgtatgagttagatagtcttgttagctatgatgaatatatttgagagcatgtattaatttatggattgtggatgaatcatatgttttaattggactttctacttatacataggaagcggtataacatttatgcacgagtattaagttgagcgtcgcacaggaacatgagggctcatacacataggttaaagagatgacttaggtgtgtaatccctaatctatgaatgtcaataccccttaaccgtacacattataatttggggcattctaaccggcgaaagaaatgatttaagattgtgatgattccgtgcatgtgaaaaagattgtgtggagtgtatttaattttttggtataagcttggtgatgaccgaatgctagaaatctaacccctataaatttcgcttctttttattagagaagaagcattgcacattttcagctgagtctcacgcctgcacctttttgactcgagttatgaagtctgtaggggtctcttgaaacctggtacccttggtatacaaaaaaatcggggagttaccgacctaacacatgctacaggggtcaagaagtggaaaaaagggtgaggtaaaaaaattaaataaataaaaaaataaaaaaataaaaaaaaaggaaaagaaaaaaaagaaactgatcttgggggcctagataactagtgggtttgaatcactaagtataaactaaattgttgaaacactcataaattgggagaatcactacatgaatgaattgttgacgttgccggttgaagttacccaaattagagcggtgtgaggaaatcttaagtaaaactgaactttagaattacaccatagtaagagaataaaagaaccaagtttgggggtgtgtgaatcttaagagtgaagaaaggaaataattgaccattgagggttgggaagtgaatcaacttgtgaatgtacgacacacacacccgcttcgtattgtatgagtagaagtttggttcttgcattgtgattttaacaccattcataaatataatataatgttatcaatgctgagccaaaaagacaagctgtctaatcgactagttgtgtgtgtatcgtctttggatgattttattgtttggtttgtttgtttgctcgaggactagcaaacggtgaagtttgggggtatttgatgagtttgtttcactcatgatttttgcacaattttggcttgattaaatgttagatcttgtgagtatagaacgtttttttatgtgtttgttagtgttgttttgaagattaggagaggctatgtgaaaagaggtattaaagtggacgaagaggccaaaaacatggaattggggcagaaagacggcgctgcattcatagcgcctaggcgctacaaaactgaaaaaagatgaaatttggacccgagaggcagcgcttaggtgccacaaccacagtgcccaggtgctaccatcagcccctaggtgctcaagacgtagggcctaggcactgcgattgaagatctagagcacgttttttgggctgtttttaaatccataaaaaccctacttctacataaaacggaagggcacctataaatacatatttctcatacttttgaggggttctggacatattggagagaagacaacaagaagggagattcaaaagaaaaattcaagaagattaacaccaagcaattgaagattagaagcattcattggaggaggaaggagatcttggtgcaagaattctactttttcttctacatttttattacaaactcggtgatgtattctaagacaatttgctatttttcttcttgcattatgagtagctaaattcattgttagggggaataatgtaaccaattgagattctttacattctcttattaaaattctcaatttttaatttttccatgtgttgattttgctatgagttgaatgcattaaattatctgatcaataatttgatgatttttgtgaattctttacaaatagagatatgagtttaagatttagaccatgtagtaaaatccagtacattggtataacgagtagagatacctatactatttattatagtcataattgaattcctaggacatagaactcgtttaactaagttgaatttgcatagagatatgaaatttaattagttgaataggctcaatgagaattcgagagaggtaaattgaatacaataggagaattcgaccgagcactacattagaattgagttttaatttaagatgtaaaaatgatcaattggtgaagttattctacccttacatccattcattatttgattttccaaccaattgtgtgaacattcatttattttctagaaattagattaaaatccagatttaacgacctttaatttgttttagtcaaatagtagttaaaaaagattgaattaagtgctagaaaatagtccttgcgggatcgaaaattcggactcttaggtccactattacttgttacgagtcgtacacttgcgaaacaaaattttacaacagtatcccacagcaaagtcgacgaaagatgccttctacaagcacatagtttgtatccatatcgagattaattattgcaattcttctgctctctagcaattgttagaatcatgtttatactattgaatagtacgttaaaattaacaatataagagaaaatctgttttaaaacaagagctagttgggaataatattagtcaaaatcaaatcaaacaatctttggcgacggcgccaaaaacttgacgcgcattttctacaacgcaatttatactgcaagtatacggtgtcatgttttgtaatatagtaatcgatttaagagtgtcgaacccacatggattgtaattcaatttctactaaatactttgtgttgatcttattatcgtggctaaattttttctctcaagtgccgaaattaactaatatctactcattcattagtagtcaattaattgaaagcattaaaatcataacacaaataaatgaaaaggaaaatttcatagaaataactaaaacaaaatcaaatcataccctcaagatttttctaatcaaatcctagaagaattatttagttcatgatatcatttatggaaatactaaaattcatataagaagacatagggaagagaataaaaaaactcgattgtaaatcttcaatttcttctcttgttcttctttgccttgttcttgaatctcttagtgctttgtctccttgccttcttgaattttccgttcaaaattctcctccaaattgtggtatttaggttggtatttataatattttgaagtcttggacgaattagggttgaattgggcaaagaaaagaatcaaaaaacataaaaaaaaacactttccgtgcaagacagtgccttggtgccattgtagccgtgctgcagtgccacaaattctgtattttcagcatgttgggcattgcggtgctcacttcgggtggaaagaagagattgcacattctttaatatttttatcataatttttactctcaatatctgattaaggaaatacaagatgccttggacagccaactcaaaaggctataactttactcagatattattttaaaatttgatcattttctatgacaaaaatgggtctcaatatgtagctagaaactggtgcgtaacttttttcggttgaaatttgatgtgtgatcatactttgattatatttcatccctttgatgtccttatttatccaattgacttcaaccactcttgactattcatcgtgacgttcgacacaacttttgattatttgcactttagcctccaaactttggatctcttacaacttaaccattttctccaattttgtcaacttttgcttctttctttcaatctcatcaactcatatcacaatatcaaaacacatattaaaactctctaaaacactctcaaggataacaaaataatgaattaagtggcacaaatatcatgagtgtggagccctcatcgtttttccaactgtattttcaactcttgaagctccttaggagccattttgtaaggtgctttagatacttgtgtggctctagggatccagtcaattttaaattctacctagttggtcatcaaggaatacatctagatattcttgtgctattggtatgctatccatagttgtctctctttctaatgtgtcgtaaggttaacttgaaatccttggtagcattcattttttatcaatttcttagcttgcatggctaaaatgaggcgggaaggtgctttaatcttagaccgataaaacctaaattctttttcaccagttattcgaaacactaccctttctcaaaacaatttatggtttcttgatgctaccgaaccgatccatgtccaatatgacatagaagtccttcatcttgattacgtgcagatccacttttaagactagccaatcaaagtctatctctactgctttagctatcttatccgtatatatggttcttcctgatggtatactaacttctagtgcactatcattgctttcatatatcacaccaattctagctaagcttgtagcagatatgaatgaatacgttgcacctgaatcaataaagacaaatatagggttgctagaggtagatagtgttaggaccttcttcttgctgctcacggtgattttcgggctcagttaaccattaaacatcgaattcaacatcaaaaccgaagtccccaactcgccggcgcctcttcttcctatggttgctttcttctcttgctttgttgattcaatccacagacttaggatggataccactcaggtaaggttcacaaagactcaagcaacagggatggagaagaaatcacgaagaagatgaaggcagaagacacggcagtttcttatcaactcacggcttcaacttggttggacgggttcaacttatggaccttgccaacaagggtgaaaacactaatatatatagtaagtcaagtggccaacataaggtaagtagggatatggtaagtagggatatggtaagtaggctcgacaagggttaacttccaatggaaagaatcaacaagccacaaagagtattagccgtccaataggtaaggcaacgtttggtcggttcatccattgtccgatgttgaattatcgttcagtcattcatgtcaactgataaaattggttctcatcatcgcccgggaggtcgtttgacaacataatgtctaacaacctccaccttggtgtcaaaggacctgcaaagaaaaacgtttttccattagtgacacctctaacagaaaaactgataaaattgaaatcatttacctgtaccgatgtttagaagctctttgcaacttctaaactttaccagtggcagactttcgtgcccatatctgaaggattgtactgtgtgtgaattttttcaagtcttactacttcttgtgatattatatccctaatgaagtgtaacctaacatcgatatatttagtgcgttcgtgaaagacaggattcttacacaaatgtatggatgattgactatcagaatacacaaccacatactcattcaagacactcagttcatgaagtagacctctaagccatagagcctctttaattgcttcagtggtggcaatatattctgactctgtagtggatagtgcaactatgtgttgtaactgtgatttccaactaacacacgaatttgataaggtgaatacgtaagaggaagttgatttcctaccatccctatctcctgcatagtcagcatctacaaaaccttttaatttcacgccttctttattagcactgaattttagacccacgtcacttgtacccttcaaatatcttaaaagccactttaatgcttcccaatgttcaggacctggattagacatgtacctactgagagtactaatagcaaatcctaagtccggtctagtgcaaaccattaaatacattatggaaccaatcacatttgagtatggagttttactcatgtattccatttcacgttcattgcagggagcttgttccttagatagaacaaaatgatttgcaagaggcaacgtgacaggtttgcagtcactcatattaaactttttcaacacttttgatatgtatggggactgatgtaagaatacgatggaatttgacctatttcgttctatttccatgcctagaatccttttagcctttcctaggtctttcatgtcaaattctccactaagatctgcttttatattgtttatccacttaggagatgatccaactaaaagcatgtcgtccacatagagcaacaaaaacaaataattgttatcagtctcgttgtgttgaaagtataggcagtgatcgaatttacttctttgaaatcctatagtgagtacaaaagaatcaaacctcttgtaccactgtctaggtgattgcttcagaccgtatagggatcttttcagaaaacacacataatcaggttttaacttgtctttaaaaccttttggttgattcataaagatttgttcatcaagctctccatgtaaaaaagcggtttttacatcgagttgttcaagttcccagtcaaagagcgcaaccaatgcgagcatgaccctaatagtagtgtacttgacaactggtgagaaaatctcgttataatcaacaccttctttctgtgtgtaaccctttgctactaacctagccttaaaccttaagggttctgaactactagtaccttctttaaccttaaagacccacttgcaatcaacgattgatttattcttaggtctcggtactaactcccaagtttgattcttttctagagaactcatctcttctttcatagcctcaagccactccttagattgaccactgctcatagcctcttcaaacgtttctggctccctatcaactagttcttcgtaactagcgtatgcaaaatccaattcagattcatatccgaatctcctaggttctctcgtttgtcttctctctctatctctagctaagttatagttagctagtagattttcttcttcaggatgctcttctatcactacttcattttcctcttcaggttcttggacctgaatttccacctcactcgaagtactaggtactgatgtgttaaattttcctaactccaccttaaaccgacttctttcttcacttgattcagtttcacttactggttcggtttcgttctttagacaaggcatctctttctcattaaatgtgacatccctactcacgatgatcttaactcctttttggcttctatcccatagcctatatcccttaaccccttcgggataccctagaaagacacactttctggctctaggttctaactttccctcactttgatgagaaaaggcagcacagccaaacgctttaagcatcgagtagtcacccaattttccagaccatttctcatgtggagtatcaccatttaatgcagctgatggagtcaaatttattagataacaggcagtgacaacggcttcaccccaaaatgacttaggaaccccagaacttaacatcatgcagcgcactttgtctagtatggtcctattcattctttctgccacctcgttttgctggggagtataagggaccgttttgtgcctcgttattccactttctttacacatcctatcgaattcagtattacagaattctaggccgttatctgtccttaaaaatttgatcctcttgctagtttggttttccatttgtttcttccaattgttaaagttatgaaaggtttcagttttgtctttcaatagatagacccacactttcctggtgtagtcatctatgatagataggaaatacttattcccacccgatgtgggattactagcaggaccccacagatcagaatgcacatattcaagcatgcttttagccttatgcgtactggtggaaaatgacactctatggtgctttccaagcacacagtgatcacagaatgataggtcagacacacagtcattaccaaatgcacctttttcattaagtagcttaagtcctttaatgcttacgtgtgcaagcctactatgccacgtgtgtgtgtgatcgattttggcggaagaaatagaagagtttaatcctctaatcacttccccagtagtgatataaatgtcgtttttcttgattcccttaatagagattaacgcacccttcatcattttaaacataccgttttcaattttaccggtgaagttgtctttctcaagtcttcctactgaaattaaattcctagataattccggaatatatctaacttcttttaacacgtacacaaagcctgtgttaaattttatctttatatcttcaattccagcaattgtataggagaagttatcacacagaactacttgcccatcattagattcttgcaagttttcaaaccagttcttttcagatgtaacatgaaaagacgcaccagaatctaatatccattcatgcatgtgagaattggtagttagatttaattcagtagtgtatgcgactggactagtgatcacatagacttcaccgttttcagtatcggaggtagaggataacacatttacctcatctcttttcttaaccttctgttttcctttttctttataacagtcttttataaaatgccctgtacctccacagccatagcattttctgcccttagttctcgactttgatctaggtctaccattccccttctttttccaactattactacttgattcgccactactttggtatccatcatgactggcttgcctaaattgtgttctaccccgcatcatatgcaactccccactcctcctatcctgtttttcagccttcattttcatctctttacttctaagagaatctacgacaatttcaggtgttagcgtgtccctaccatacttaatagcatttttaacttctttataagagtccgggattgaattgagcaagataatggccttataggtttcagacacggcttcgtcacaattgacaatatcttgcaccaatttattaaatacatctaaattgtcgtcgagatcctttgaaggatccattttaaagctgaagaatcgttcgagtaggtagagtttattcggtgtagatttaagcaagtataagtcttctagtcttttccaaagttctttggtggtttttagttttcccacttttcttaagacggcgtcagacaagtgtaatattattgaggtataggcaagatcatcggcttcctctttttgttcttttgagatatcaggtgcaaaattgccttcgatggcttttgacaccttttgttggactagtatgcctctcatcttttgttgccagatagagaagtcccctttaccgttaaaaattcccaaatcaaaattatgtgttgtcattgattaacaccctaattaaaccacacaaagtagtattgggaaacgtgataaggtaatgtcttgttaattattagcaaaggtaataatgaacctaaacgctacgtccaccaaggaataacaagcactttaaattagaagaacaaaatacttaattaacgcaagtaatcctaattctagcacacgcaatggttaccccttcacggtaaccccaaaacctaacgatcaccccacacgatgatcttgctattgctgaatttaaatggattaagccaatttaccagagcggacctatctgagtctgtaaagtggagaaaaacgagcttgctgttgaatttcgatcggcgtcgtaccaaagtgcaaaatcgtccaactttttctgtgtaacctgaaacacaaaacaaagtatatcagcgcgttcaggagatcgaaacaaacaagttacctgaagactgcgtcgtcggaaaattccccacgcgccaccgccggaggcccacgcgccgccgccgccgccacgcgccgcctctcccggagcgcctcggcctgctgatgatgggtatggcctccgtttgtccaaccgagctctagtttgtgagtaattgcagattttcagattcgggttctaagttgaagatgcgaaaatcaaccgattttgagccgttttttgccacccaagctctgataccagatgttaggaccttcttcttgctgctcacggtgatttccgggctcagttaaccattaaacatcgaattcaacatcaaaaccgaagtccccaactcgccggcgcctcttcttcctatggttgctttcttctcttgctttgttgattcaatccacacacttaggatggataccactcaggtaaggttcacaaagactcaagcaacagggatggagaagaaatcacgaagaagataaaggcagaagacacggcagtttcttatcaactcacggcttcaacttggttggacgggttcaacttatggaccttgccaacaagggtgaaaacactaatatatatagtaagtcaagtggccaacataaggtaagtagggatatggtaagtaggctcgacaagggttaacttccaatggaaagaatcaacaagccacaaagagtattagccgtccaataggtaaggcaacgtttggtcggttcatccattgtccgatgttgaattatcgttcagtcattcatggcaactgataaaattggttctcatcatcgcccgggaggtcgtttgacaacataatgtctaacagataggatattatatcgagttcaacttgatctatatgtgaatttgaatagaccttagttaaacactttaaatctctgagaatgtatgtaactaactagaaaatatatctttacacttttatacatcttttactacgtggtctaaacaaatagcccacctctcgatgtaattgtctcttacaaataaatgaattattggccaattaatacaaagcattaaaaatagaaataaaaacaattcacaacatcgattggagatttaaagctttttaatgaaaattaaatttcaaaactaagttacaatcgttcatcctaaataataacttaatcatacatcatgagaggaaaaatacaggatgtaattaaattacataaccatgttttaaggagaaagggaaaaaatgaagattttgcaccaaaattctcttttcttcttgtaaaaaccttgaaaccttggcttctttgttcttttttccttttgtggtctcttttcttttgattgatttgaattttttcttcccaaaaggcatcttggcttgattaatatttgtccaataaatctccaaaccttcgcttgaatatgtgtataatgaaatgctacaggcctcatttaattgttggacaaagccactacctttctaggccataagtgcatgtttgctgaagaggaatcgtttagaaatgaagttcttagtacgaagaacttctagtggcaactcgtaaatagcccaaacattggccactcttcgagttccaactgatcaactgtgactgtataaagattgagttagcaaatatcgaagaagagagcagaacggacacttcggaaatgaaattcactaaattcattgcattgggttgacagggtgaccttagcgatcacattgccatcaacggtttgccaaattattctagtcgaggaaaattgaaaatattcaagattttataatttttcctctttttctttatatatttcaaatccaggtgatatctcagtattcatacgtattttatttaaactttgtgatgttaagataaatttttagtcaccaagacatagatgaatcctttattatgaaattttaataatattttcatgacgtcaacattaaatatttaattttcttggataattgttagagtatttaacgattttcaactaattgatcactatttggatcgacgtgcgattttattattattattattattttattttcaagaaaaatattaagaaacatatcacatcataacaattgttatgagctctggtaggggatagagatgtaaggttatgttttgtatgacttcacaaggtgtctagtgcttttaatgcattttccatattcgcatatttcatagagatatcggaagatcacatataagaatatttgtttaaattattctagagagattgttaaataaaatatgaacattgattaataagagtaaattaataatatcatgattttgaattgtattaaaatgaattaatagagggggattctaattcttaatgcctgttttaaccgattttacaaaagcttttttgattgcttatattttggtcaagggtaattagcacaaaacatccttatctttcacttttattgtgggaaacgtccttatctttcatttactgacattttgacccttattttcccttttcattgcacaaaagttcattttcattatttttctcatttaagagttgtgaaatgatgaatttaaataaaacaaaaaagaaaaagaatgaactaattgcaaccattgtccttatttttcaaaaaagtgtaaacaagtcccaaataaattattataagggtaataacataatctccctacctttcactattattataaaaaaagttcatatctttcattttttggcattttcacccttagttacagctttaattgtgcaaccatcatttctatcattttcatccaatttctcaataaaagttgcgaaatgatgaatacaccgtcctacttaaatgaaaaaggctgtatttatttaaacattttcggctcagactatcctaagtagtgatgctatgaggtgggaaagtgtccaaccattacctagctaaatctctcaaagtatatggaaagagtctcgatcgaattgcaacaatagaaactctcaaatatacaattgatgcacatatatcaaaaaatctcaagttgtgagcatttgaatttctagtggctttcccaaagaattgtaatgcatgcttgaacatgtttatcacatccatccacaaagaaaaattagcttgctcaaatgctagataaactatgttggatcgaatttctaccaccggtggaagcatgtattcctccatcagtctttcattttcattaccaaaagctacaatcggatgtactgtatcttcattcaccccaatggttactcgattttgtatattttttggcattgattctgcttgatatttggtatgcttctaattgttcttttcttctcaacttgaattttcgttcgatttttgggtcaaatggatccagatcaacgtatcttgaacttcacaagtaagatcctgcaaagaaacaaagaataaattgtaactctctctctctctctctataataataaactaaaaaataataaagcaataaaaattcatattaaagctataactaactaaaaactaattaaatattacagttttcgacaacggcgccaaaaacttcatcatacgaaatcccaaaagtgtaagtattaataaagtgaagaatatgatattgtttccatgagaactacatacttattctacgatcaattaatgttaacctcattcaactaggaaacttgtatgaaggttttatattaattatttaattaaagtaattattctaatgagtgaactatgaagcctttgtaaaactatgtaagatggttactatgaccttgaatccacttattaacccgttttaatgcaattcatagcaagacaatatgcacgcatttttgttgaccaatgttcctaagttaattaatagcctctctcgataataattaaatttatcatctcatgtaaccttcttatatttctataaaagatacaaacatgaaagcatgcattaaaaatactagaacatctatagaaattatgcacagcatagcggtatatttgtatctccctattggactttacaatggttataagcaggggcggacccagacgacttgacttgggggggcaaaaataaaatttataggatatcttctaataaaaaaactaaggaaaaaaaaaaaaaaaaaaaaaaacctaagcaaaaaaaatttttccccccaaaatctaggggggcaattgcccctataaaccccccctaggtccgcccctggttataagtgcaatctattgtattttgactttggatgacagtaaaattcacatagcattgcgattagtggccaattaattgaaaagcattaaaacatataactatcgtctaataataaatacacattggccatcttaaacttttattaaaacatcgtaacaaagttcatcaattcctacattgcaaaatcattagaattcataattaattggaaaaacataaccctaatttcggataaattgagaagcaaaagaataatcttgaaatttcaaatctcttcaatgatttcctgatgcattaccaattgtgacttctcttctttgctcaaggatcaaattagatgtctcgtacttattagctttgttaactggttatatatggctattccaattgctagaggaaccacggatgacagtttggagaagtctaggataatcatcttttattttttctctttgaaggaggtggtcaacccatcttatattatccttccatctccgtttctacattaaccttattcaacaagagtatgagagttccatgcttatttatttggcttaggatttcattatgcagcacttaagctctaatatatcattatctccaatcagacattacaatgattattatgagtgtaatctatcttttatctctctcgataataataaaatctacacaacgttccaattagtttccaattaattgaaaacttaagtcctatagtaatcattcaaaaataaacacaatttggtgttaaattattgaactttaataaaacatcattacaatgactcatcaatgctttagtaattggaaacctagtctagcattccaaaatcccacaaattcataataaattagaaaaacatgacttgaatttttgataaattgagaagaagaagaatgatcctgaaatctcgaatgtcctcaacggtttcttgatgaatctttaattgtgccttctcttctttacccaaggatcaatgttgaatcttcaatttgtagaaatcttgtaaattgccctttattttttttattttattcaagaacaattgaatttgcctttcctttataatgataattgatgtataatggagtatgagaggtgtcctcaatgatgtgcccatgttctctatttataatggttgaaaataggttaaaattcacgtccaaaatggttccaaagaagagtttttattaaaatagaaaattgtggttgggtcctcgcaaatgccttgcatgagcgctttgttcatgaaacggatgccacttcaactttttgctttcttattcttttggaacaatggctcacacgtgagtaacgtatttaacagaatgtgaggcatcttccatttttgggaccaatttcctgttggatattggtaaaataaatcgagaattgaaaatcgattaaagtgacttcgtatcgacttcgaccaaatactcaaaagctcgactcaatccgtttaggcaaaattatttgccacttcgccgcttcggggcgcataaacaaacggggatcgacctgcccggtcaggtcgcgggggtcgagggggcgacgccccccatgggggctcgggggcaacgcccccgaaagagaattttgatttctctgcatgtattgaagggtatatttggcatttcgaaaaccaatatcggatgaatgagaaattacgaaaaaagacgaaaatcaggtcaaaatatttgactgtgcgaccgcacggttgtccggtgaatagacaccttttcataaaggtgcattgtttggaaatggtgcatggtttggcctcaaccattttgtccacaccctttcatggtctataaataggaccctttgggtgtcctattcctcacaatttgatatgcaaaacatctctcatcctctcttctatccaaaatcaaaattatttcatttattttgattttccttcatttcatccttggagtacataagcctaaatttggttcgttgtacttgtgttttggagtcctacaaacacaagtgtaaccgttgtatcttgagagtcgattgccgaaatccgtaggcaccgttgcggggcaaattcgacttaaggacaaagagtccaactcttgcctcgactttgtccctactttcttcttcttcttgtttgtattttctttgccgttactctgtccaattttcggcacggatttacaaaccatcattatacttattttggcgtcactattcacaaaattcctccaatatttccaacttctcaacggcgtttttaggtaatttcttcctgcaattttattcatttaacttcaattgcatccaaatgaacctgtataatcttcaatcatctttgtatagtcccaaacaactattgaaaactttcaatttagtcctaaaactttggatttcaccctttttgttagttttttctcctttcttccaatttcattttcaaatcaacgtgttttacctacaaattaaatatacgagagattaggccaaaattaatcattaaaacttttaaatgtctatatttgaaggtccatataagtgtataatttgttattatcaaacaccctcaaacttgaatatttgtttgcactcaaacaaaaatataacctaacttaacaaaaaagcatgcatgcagtaaagttttggttagataacaagtcgttttgttttttggattgaaatcattgtattaaattaataaataattccaaggtcacaatactaaaatcaatatcaactccaatgcaaaactaatgtgtgtgtgaagaattaagtaaaacattataaattctcacttcaatggtccaatttgttcttttttcactcgtatgatacacacacccaaactaatccttttgactcttaaggtgtgatctaaggttgaatttttatattattcccaaccttctctagtttgaaagtactttactaattgcaagtcaataactcaacaaataagaattcttcaaaattttgattgttttaacttctacgactcaaccaggctaataattccatgtcaaaagtctagttctctccaataatttggggcttattcatggtgtgtgcgcatcatctattttacgcacctacttctttgagatttcatattctgtttgatacattagcttgatccctttgagatttctttctgggattttctataattgctcttttggagatcttttaaggtagcctcacaacttgacaacttttttccttttatacaatgattattacaatttccctcatttaaaactcattctaaaaaactaacctctaatttaagatttttacctagtttttatttcattggtcttaggcaatccacacaagaattcacacacacataatttccattcatcttcctataacaattcaatcgcccaaaaattatgctaaacttggtttaataatgcatattattgtatcattggtttaacatttaagttctactatttcaacctattaagtgtatgaatcaactcattctttcaaaaatacttaacttaattcacatgtgcaaaaaatatgatgttttacatgtattatgatcacttaatcaaagtgtataacctattcataattaataaatcaacacataactcaaaaaaatattcataattgccagcaatgctacctaatctacataggcaaactaaagagaaaatatttttttggaatttctaattttattttttttcaattttttctcatatataataaagaagtaaacacaaaatcatacaggaataataaaactaaaaactcaatatctttcccacccccaaatttaaagtagacattgttatcaatttcttaaagtataattaaacactgtaaagaggggaaacagaggaaataggtgctccccgagttttttttttttttttgtccgatattgaagataagtttgttagatcagttcattccattcttcaacttgttaaactgccacccgtttgataacattgtatatgtgtttgtgtatgtgtgtaagagtaaaaaattagtttaaaagctacaatacggtgtgtatgatagctaatttttgatgaccctagagctttgaaaaacgtgccacgtgactctttaacaattttggactcaaataaatggctttacttttactaggatataataaatgcggacatgactactttttatataaataaaaaatgcctaaaactgatgcaacatattaaactctatgcaatgttaataacagaaagctaatgaataaaagggtaaaagttttggttgcctccgaataaatgcttaatttaaagtccttagctagattacttggaggagtcaatcatgatgattcaacttagaaattttcagctttgcattctttacaattttgagctctacatccttttctctctctctctctctctctctccaagtcttgaattcttcattgtcatctctactaaggattccatcaagtttgggttctctcttatgatggcttggtagatcatcatatttaatccagttacattccatgaggtctgctggttgcttgggtagattgtgtaatttaaaaaattcttatttatcctttactcttaaggtcaactcacaatcttttatgtcatttaaggcttgaccgtttgtgaagaaggatcgactgatgattattggaatattttggtcttcttctatgtcaagaaggatgatgtccatcaagaatatcaattattcaactttgatgagtacatcttcaaccttgcctcttggatatttgatgcttatatctactagctacactgacacctttgattcttttagttttccatgtcctaattcctctacacatattgttgaccaccgatctccgaactcatttaaaatgtacttcatacccatctaatcaacatgcaagtttgggtttttgagctcggctcgatctcgtagccaccgtaatttaaatagaaatcatgattacagattccttaaaccttgtcaaatcacccaattggttaagcacacttggaaaaatgacgttaggaccgccaaaacccaccaattaactaccataaatccttatcttggaataggtcatgatttcctgataagatgggatattattatgatttgattggaaccaacctcgtaaatcaatcaaggaaaggatggacgacacacaaatcaagctccgctatggttaacaacattgacaagacataattacctggaaaataaacttaaatccaggggaaacagctcctgttagctggactacagaaaaaaatatacttgtaaccttcaatatcaatagaaaatacacatttcactcaaaaagttggccaaaaattacacttagcaatttttgacgccaacagtttggtactagagaaaagacctcattgtgcgagaacagccccactttttcccaaaacaacaaccaaacaaaagctatgagttgcagttccacattgggaagccagtctcacacccatcccaatgaaaaaagtaccccacatagttttcgaaaaaagcaagatcaaactgatacagaggtagagtcccatctagggaaagccagtctcacacccattagtaggttgacaaatgcagtcagtaggttggaaagaaatcagactcatgtttccctacttgatatcgaggtggagtccccaactaggaaaagggccacgtgattcccacgaggagatccctccttgaattgaggagatcagaagacccctctactgatggagccagtcaccagaaaggctggcagtgtatttgataggttgggctctcagtacttcctaacacctctaagagcactagttgagcctaaactaagcactttgaaaagttgtattactgatctagaggacagaagtgaaggagtggtggataagtgtctctcccagcatcagtccctgttcacagaagacattcttattgaacctatacctaaaaaattaaaaataccacagttgattgtgtatgaagggaaaggagatctacttagtcacctgacaagagtataaaatataatattttccccttttaattattgtattcgtgtgattatttgataccaaaatgtactcattatacttatgttttgattcaggctgtattttgatagaaaaggtggaatatagaagaaaagagcgaaaaaggaccaaagtggaagaaaatgaaagttcggggattaaagtgcaaatactccaaacttgtgtctaactttatgatgaagatttgagagtgttagaggtcaaacatatgaggaatgaagtcaaagggaaggaatatcgtcaaagtatgatcatacatcaattcccaatcgaaaaagttacatatcgatttttagcctcatattgggaccctttttgacatgtcaaacaattgaattggaagatgacatctgaaaaaaggttttagttctttgtgttagctttccaacgcaatttgagtcacctaaatcggatatcgagagaaaacgttatgaccaaaatactaaatactattcggcccatacgattgcataattcagataccatgaggtcatatagaaggtttcagggaacttcagggctgaaaatatttgttctatgtgaccgcactatgcgatcacatagaatgcttccgaggcgcgagattttgtttcctattttcactcaaacacttatggtaatctaattttccatgacttttaagccaaaaatcatcccggaacgcaatcattgatcctcatatcaattttctttggtttttggttgaagaaatcaatggagtactaaattctttgatgaaaccacaaaggatcttgatcgaatttggggatttcaacgtcgtttcattcatgtatgtgatttttattgttaaataattccaggatttagatttcatctttatattacactttgaggtttgcttaacttttattaaatctatcatggattcaatcatgttttttccattgattgattacaatatttgttgagtttaaattgtttgaataatttattgacgttatttgattactgctttatgctaaggtatattgtcatttttttaatcttgtttcaataaatcaagtcgaatttgcttttaggaagtctaaattctaggattagaagtgaaacaaattgatctaggtttctccttttatgaattggttttgaaattgatttaacttttattagattgattatagattcagtcatgctttttctatcaactaatcaaaataattgttgagtttgaattttatttatgtcattggtggattaattatttccttatatgcttgatgtatatggacgtctcttaatcttattttaatgaaaaatgtgggaatgtattatagaaagcctagacttttggagtaaaatgcatgaataattgatgttgattgacccaatccaagagagtaaattttggtgctctactaatctcacattttgatattaaaatttcattcaaattgataaattcctctcacagtcacgaaaaccctagtttgtcaaatcctttaaacaatccgtccatctccctatggaatcaacaccccaaagttgtgctacaactactgcgttattctttggacaaaatcaaattttggcgccgatgtcggggagacggtacaaataattgaaggattctcgagtaaaatgatgacttcgttcctcttctacattttttcaattagtttagtttattttcttagttattttgttatttctcatctaacatttttttatgttttatgaacatgcatcgagatgagcgaaggcgattcaatgcgcagcctcaaccagtgtttgaatcactttctaaccctctctcctaatctgcatctattggcactaacatcatatttcacaacacaatgactgataatgagcatgatgatgcgctctataggactttgcatgattaccttaaccccccacacacatttacaccatcatgcatcatctttccgcctaacatgccacatataggcctaaagctgggaatgattcaatttcttcccaattttcatggtcttgaaagcgaaaaatcatatgtgaatattagggagtttgaggaggtggtggcaaccttccacaatcaacatggtacgttggatgtagtcaggctaaatttttttccattttcactcaaagaacgaggaaaaagttggctgaattcactgggaccacgttcgattgggacatggactgaaatgacccaagcattttttagcaaatactttctccatcataaaatgactggtttaaaaaaaacaaatttcctcttttgtccaaaaggatagcaaaactttatatcaagcatgggaaatgtacaaaaaattgcaagccctttgtccccaccatggttacgaaagttggcgtatgttgagttatttttacgaagggttaacacctaaggagcgtcaatttgttgaaatgatgtgtaatggtgaattcgtacaaaaggatccagttgaggttattgaatacttagatgacctagcagaaaaagcccatacctggactagacttagtgacattgagagtaacaataggtcatgacctcaaggaaattctactagcacaggcatttattaccttagagaggaggacaaccttagagccaaggtagaatcccgcactagattttgaagccctacgagctaaggattcaaaacccatgcaatctatttcccgtgttgagcctttatggctttgttctgtatgtggcggtattgatcatccagcgcaaaagtgtgctatttaccttgagatgaggaaagtctatgatgagcattgtaatgctttaagtacatatcaaaagccctacagtctatattctgaaacttataatccaaggtggtagaatcaccccagttttagctggaagtctgagaatcaacaatctccccaataaaatcgagcttacaatatacctccacatcaacctacgtcttctaggagttccttagaagacatcttatatgcattcattgaggtacaaagtaaaataaataaaaaatttgagactatgattaaccaagtggttgaggaaaacaaggagataaaaaatcatgtctaaattggacattgccttaaatgtaggagaacatggaaaatctcctgtttaagttcaaccaaatcctaagggacaacacatgtcacaaacctcaagatcaggagaaaacagtattagggaagtaaatgccatcaccattcgatctgggaaggttatacaaccaactcccaaacttagggaaaatgaaaaggagtctaatgagtctgaagaaagtagccctagtgatgagggagtaggaaatccatcaagagtgcccttccctcaagctcttaagctcaccctgaaatctgtcaatcaacatagtgaaatcctagaacaccttaggcaagtaaaaatcaatctacctctcttttccaatgtacaataaatacaagtttcacacggaagtgcacactttgatatatgaaaaaggttttcaaaaggaaaaaaaaaaacatgaaagaagagcaaatttcttaaaactttgggtgccatcgtgaaacaacattcatcatccaactttatccattcaaagcttcaactttaggaatgtagaggtgcaagtgatttttttgttttcgagttattttttttgttaaaagtatgaatgaattgatacttctgagtatggtgcttcaacactactatagtttgaataattattctccagttctatgtgttataataattctataaaaattggattttgctggaaatccatctacccgcgcaatatgaatctatatttcgaattttctattttgataagaaaatgcaccgatgatatatattgagtttcaaactcttgggttaatttccttactacaggttgatttgatatgcttcgagagtagaagatggtaaatgaagatgcaatgtgctatggataaatcgatgacccaatttttaattcgaatacgaaagtttacatgtttttcttaacaaatggatttctatgaacattatttgtgggattgttttaagaagatttttatgaattagttatgttttaaagtagtaatgttttataaaaattaacgtacaagttaccattcattacaaaaatgtgagggataagacttagtgtttttttttttttttaattagcttgtccttggcttcaaaaattaataacttaatcattacatgaaaattttggacaaaatccgtaggatttgatagcctcatgggttatctactgaacaaacttgaaatcttgtcaattcgatgactgaagaatttaaatatcattttaagtaaactgcatatggtttatctcccaaaccaagtccctgggggattttagaaaatattttagtactgtatatgttttcaaagtaagtcgatatttgaatatgtcatattataagaagtttcctagcttccctcaaaatttcatgaagtttcgagattgataccgcttgagaaagaaaagtaaaatagcattttatttatttattacccagaatgttcatgtcaataatgttatgtgcatggaaatcattcaaaagacctttttttttaatttttttcttttagtattaaattgtgctttattgtaaaaaaaaataaaaatagatataaataacacttaaagtaaattttaaagtaaatctttatgcattatgtgataagtatagttgattaaactaaattgtatataaactttaattctacaactaatgtacaattgttctagtaacatctcagtccatacgggttggcgctttacaatagcaacacactccaatttaactagttcataaaaaatccgaacacatatatctccagatttctctgaaattataagaattttcatgctccagggattattgtctctatcaagtcgtggttattttgatgcaacattggagtgatttgatgccaagcttaatgaaagtattactacctgggaggatctaattagaaaattctacaataaattcttcctaccaacaaaaatagcaaaaatacgattggaaattctaacattccaacaaagagatggacagagttatcataaggtgtggaataggtttaaggagctaataagagtgtccaaatcatggaatcaccataggtaatcaagtgcaatacttctgcacacgacttccgacactatcaaaatctcatatggattcctctattggtggatcaattgtcgaaaaattagttcaacagtgtatggattttgttcgagtgaatcgccactacacattaaatattctcatcagaaagagtgctaacacaaactaactggaatttataaattagacattacaatatttaccaatgcataaatagctgctcttacaaaatagtagagttattggtgaaatagaaaatacatggaacacatgccacaatgacccatcatgtgaaaattgtggagccaatcatctcacagaaaattgcttctctatgggttttccagagaaccaagtagagttcattgaaaatgtcacccttaattttaacccatacggacaaccatataatctaggatggagacaatacgcaaatttcgaatagtctaataatcagccaaaagaagttcaaataatgcccagtaagagaaaaaaaccaagtttaggggagatattcaattagtacgtgtaaaagacagaaaaagtgttcttgcaaattgatacaaatttttaaaatcaacaagcacccatggaaaaactaaagatataaattgtttagatagcttaacagcttgtagaaagccaacaagaaacattgtcaggcaatacaatgatcaatctaaaagaacaagtgcaagctattacaattagaagtgcagtacaattgctaaagatacatgtgaagataccaaacaaaaaagacagagatagaagttgaacaggcaaatgaaaaatctacaccaaccacaaaagatgaggaagagagaaaataaaaacacccaaagtaagagcaccaagtcccattaaagcttatcactacaagaattttatacttcccctacaaaatttggggagacaaattgatatttgtaggtggaattcacttttccggacaaatatgacagtttgtagggacatgatttgctttaaaattttcaataacaggaagacttgtgtccacaaaaatttatattttttccaatagaaaattttgatgggtaaagatatatcttttgttacaaaaaaatttgacctatttgtaggccaatatttggaagaaaaattttcatttttacttgtatttttagtccttataaaatgtaaattcgaattgaaaagaaaactgaaaagaaaaactgaaattaaagaaaattatttccacatttttttggcgttctttttcttttattttccttctgttttccctttcttttcttttactttttcttttccgacacttctttcttctcctcccttcgctatttccccctactctgttgcaacttccgtcaccaaattaccgtcccgccaccttcaatcagccatcagtcatcgagcccactagcctaacgacccaaatcaacgcttgagacagctaagaggtatcatttattcatttttttgtaggattgttaccggatttgcaggggaatattgtgtgaaatgtaaattgggttgtttatctgctataaattcatttacttggtagctgtcaatttatttatagggttatagagaaatattgtagatctacagtaaagtgaaggttcatactcaattgaaaatgttacgtgttcaaaattatgataatgttttgtttccttgactttagattaaaattttgctttatccaatttattagatgtaatcattgttcttatcaaaattgtgctttgaatctttagaacttcctgtcccatatctaataatgttaaagttaagaataaattaatttgaatttccaaaattttgataataattgctgcattcatcaatgacgatatgataaaaacctgaagtgtggatagatttcaaattaaaatttggtttcttctgttgtcattagtgaattgatttcatcaaaagccatccgtgatattttgttttttgtagatggtgtcaattgttatctctttcacgacgctagaaagttctgttttatgtctttgtggggaaaaatggaatgaaagaacatgttgcaataaaacatacatgattgcttgtttatcttcccaagggtgtgtaaatttctccactgctgtggttatttcatttgttttgtgagaataggagtattaaggggaagtttgaaatcttttgataacttggattagatcttgtaacatgagtttaattggttcttttattcttagaaaaataacatagaattttatgatttgtgatttttattatcttcaatgattagactaatcaaaaatgttatttggtattaattttgtatgaaggagtagctgccccaatggcatttgtctcccaacgcgttcatacaagaaacacatcctcactgtacacatggtatctttatactcccatcgagtattttcaaagatgtcgatttttacacgaattgtttgtttcataaataattactaactcaagaaatatactaactttttaggtgtctttctatttttatgatgaacgaagttactatgagaaaagattaagaagtatgaaaatatagttgcttgagaattggatctattgggtttggcttgtgcttggatctattaggtttggcccgtgcttctgaatacacattcttcgtctttgcattcctggttgggaactattttaatgttaattctctttttttcctttatttctttcactttgttatgcccttttttcttcatttataacatcatgcagcatttgagtaatcatcttggaatatttcctaacaggagggtatgacacccttgaacctatatgctgaggatgaatttcatcattctgcttgagctggggctggaggtgtcaaaagaattacaaattatgctccggtaaaatatatgctggatgatcataataatctcgtatttcctctttcacatttttgacgttttattgctttgtaaaagattttattgcattatctttggtctaatcaacgagttttgtaggttttgaaatcgttaaacagagcaaggacagagggttctcttatgccttataccttgattcgatgaataagcgatatattgaagagttctcttcttgtaatgtcttcattttgaaggtattgaactaatcacatttcatattgattaatacgatatatttcttcgagaaaactgtggtttattttgtactcagatttacaagtaattactaaaatcatataattcatcgacttgtatggggaaatgttctttctacgccaacaaccaatggattaagtttcaatgagtgaatctaaaggaattttactgcatatgttccaaagtcattttttttcctagcttgctatcctttgtgtattcgaactttcaatcaattcgtacttatcttcatagattagagctcaaagaatttttcccaaatgtgccaggttaaagaatgtccaattccatttgaagaattacttgatgctgacgaagttttctgcacaggttattttactctttaacatctttcttaaatagagtttgaatcacatctctcaatacgtaacatcttttcctagtgtaggtgctacctggagactacaagcaggatcaatgattgtcatctttgggttggagcaataggattagttgtatgatcttccacctgatagaatagaaggatttgctgcatatctaattcatgatgatgaatagttatatttttttaggtgcataataatagatatagagcatgcttgctatgatcttttatatttagatgtaatgatactttgtaaacggtttttatttttgttttggtgaaatattttaaattcaatgttatattgattgatactatctttttgtgttttttataatattttgaataaggttaaaaaaattattacaatataaataaaaaataaaatatatgaaaataatttaatttttccctataaattctttcataataatctacaaatatgttttccccaatttttcgtagataaaaataggtttagcccataaaataatatttactgtgttttcaaaaatattctttccacataaaaaattatttgtagggaaaaatacaatttagcccacaagtaatttgaagggaaaagtgaaatatttcgtaggcaaaattaactttagcaaatgaatgattttgttgggggaaagcttacgcggcaaattgtatttgtcttcaaagggtttgtagggaaaaactttagcccacaaatttcaaaaatttgtagtcttttatctatcctctcgatgtttgccctacaaatatgcttacagaatatttttgtctggtaaagttttttcctacaaattattacctttcccatcaaataaatttcatagagaaaacataaatttcttgtagtgtatgcggcatcaactccttccctcaacgactatataaaaagaagttggacaagctttttgctaaatttgtagagattttcaagaaattgcacatgagcatccccttcacatatacattaacaccaatgcctagctatgacaaaattccaaagaaaatgctttccaacaagagaaagatgaaagaatataagatagtctacctgaacaagaaatgcagtgtaattctcctgaagaagctacctgctaaactaaaggaccaagagagttttaatatatctcgcaccgttggttttaactactttgagcattctttatgtaatttgggtacaaatattattttaagaccactctctaattataggctctcttggattgggaaaagcaaaaccaacaacaatatctttgcaactgttgaactggtacatcaaaagaccaaaggaaataattgaaaatatgctaatcaagtttgataaattcatcttccaagatgatttcattattttggacacggaagaagattcaaatattccttaaatcttaggaagacttttcttggccactggaagaacacttattgatgtatatgatgtataaatgatccttcgagtagacaatgagcatgtgatatttaatgtgttcaaggtaatgaaatacccattgacttagatacttgttgccaaataaatgttcttgaggagcttgtagctgatacatttgaggagaatatacatcgaactaatatgaagtaggtattgcacaatcagaatgagagaagtcgacaattgaagaatctgctttatagttggtaaaatagaccatgtgaaagagacattggcaatatgagtttcttggtaccaatccttcaccaccagtaccttcagtggatacggtcctaaatcttgaggccaaacctttgccatcacatctacactatacttatttgggaaattccatcacactttcaataatcgttacaaatgatataacagagaatgatgagaaaaagttattgttcgaggtactatgggtcatagaattgcaattggatggacaatagctgatattaaaggaatcggtcctattctttgtatgtggaaaatcttaatggaggatgagtcaaatccatcagtggaaggttagtgcggattaaatcaattttgaagaaagtagtgagaaaagaagtgttcaaattgctagatgtagagattatctatcccatctcagacagttcaagggtgagtccagtgcatgtgatgcctaagaatggtggaattaaagtggaaaagattgagaacaatgagctaataccaacacgattagtagctaagtggagagcatgtatcaattacaaaaagctaaaatgccacatgaaaagattattttccattgtccttcattgatcagatgttggaaaggttagtcagtcgctcacattactgcattttggatgaatatttaggatacaaccaaatagtagtttctccagaagatcaggagaaaacaacattcacatgtccccatggtacttttgcctttaagagattgtcttttggtctatgcaatgcacctccaacttctcagtgttgcgcgatggccatattttctgatatggtggaaaagtacatcaaggtatttatggatgacttttcaatatttggtgattcttttcttgaaacatctatctctggtgttataaaggcacaaagaaatgaatatggtgtttaattggaagaagtgctattttatagtaaatgaaggaattgtgattgaaaaattgcagtgacctaatttggttaaggagatcaaaagccttttgggacatgcaaggttgtatagaagattcattaagaacttttcaaagattagaaaacctctattcagcctattggagaaggatgtgccatttaacttttctgatgagtgtttaaatgcctttaatactttgaaagaaaagttaacctctacacctgttatagtggcaccgattgggaattacctttcgagcttatgtgtgatgccaatgactatatagtgggaccaatgcttggaaaacattggagaaaaatattgtacgtcatctattatgctaaaaaaactttgataggtgcttagatcaattatgcaacaactgaaaatgaggtgtaagaaaagtattttcctttaacaaatttcacagctatctaattgggtcaaaggtgatagttaatatatatcatgtagtttaaaacacttgttggagaaaaagaatgcaactcaagttgattcaataggttctgttattataagagtttgatataattcgtgctaaaagggaacataaaatcaggcagcaagtcacttattgaggttagaatagtcgaaataattgaaagagatagatatcaatgaaatatttctagattagcaattattgcaggttgagaaagcatcgtgatatgctgacattgtcaactactcagcaagtggatatttgaacctaaactttacttatcaatagaagaaaaagcttttccatgaagctaaattctattattaagatgatccaaacttgtaacgaagagggacagatcaaatcattagaaagtgcatgataaaatatgagatgaagccaatcttgtcatgggttcgtgcttcagcatatagaggactctttggccaaacaaaaatagcagcaaggtgcttcaatgcaatttcttttggccaacattatttaaggatagttacaacttttgtagatcttgtgataagcactaaagaacaggtaacttttctacttgtcatgagattccacttaacaatattctagaggtagaaatctttgatatatgggatattgattttatgggaccatttgcatcgtcctataacaattgatacatcttagtggcaatggactacatatcaaaatacgagaaagctaagacattgcccacctatgatgcaaaggtggtggtaggcttcgtaaacaagcatattttcaattgataaattacctagagccataataagtaacgttataacacacttctacaatttgctattcaaactagtacttcacaagtatggggtacaacattgaatcgccgtacattatcaccatcagatagtggagaggttgaaacttctaacagatagctgaaaagaatctcgaaactcatggtaaatgcatctcgaaaattactccaagattttggatgatgctttgagggcctattgcacaacttacaagacagagattggaatgtcaccatactgtatggtgtttgggaaagtgtgctacttactagttaagtttgagcaaagaacatactaggcgctgaaaacagttgaacatggactaagagaaggttagaaaaatgagaatcttacagctacatgaattggaaggattcagaaaagagacctatgaaagtgtttacatctataaggaaaggacaaaacaatggcatgacaaaatatccaacattgagttttcaaaatgggagatcaagtcctcttgtacaactttagattgaaacttcatctaggtaatttgaaattgagatggcccgaacctttcatagtatcacaagtgttcctttataatacaatcgaattacgtcatccaataaagggaaatttcaaggtcaatggacaactcatcaaacactatgtagtataatttttaacagctaaagaaagccttaaaatcatggttccagaatgatagcggcacaaaatctagttaatgactttagagaaacgccttttaggaagcagcccaagatctatcccttacatatatatatttttttaatttttagtttgtttcttttattgtttataatattctcgttgtgttttgtaaaacaaaattcaagtttggggtgaaaccaagcatcgacaagatatttgaattcaagtcataaagtttggaggagtaaataaaactcaaaatggaggaagaatgttgaaaagtatcgaaaggactcaaaaaaccaaaataaacaaatgtccctcaccaaaagaaccaactcaggtgcctcgatgctacactcggccgcctacttctatgattttttctttcttttctctttctttctacattacaactcccatatataaaatcctcacttcttctttttattttacaacttcaacacaactctcacatagcaattccactcttccccaaattctctcaagccctaacaaatttttttctcttcattcttcaaattctcttcatataacaacacatcaacacaaaaatatctctcttttttccttcaaacttaccaagatctacacaaaactcaaattatacccatacatcacaattcattctgacctccaagatttacttccatcaacttcaagctagtgggttactttatgaagactacacaaggaatggtaagtttctaaacttttctttggaattttgagataaattgtgtttcttacacttggtggtaggatgtgaaagaaataaaaaaagttattttgggtttttggtatattgtggggtattggcattttgagacgtgaatttatgaattgtacaaagtatttgttgcaagtccttagagaacttaaattatttaggtgatctatttgatatgtttgttcacttccattgacattgtgaaatatgcaacattgttgtggtgttgagtagagactgatgaagtgaattgttgttggtattttgatattaagaaattcatcatattacatggaggttgtagtggttgaaattgattgactttgttgccttttgaagttcacaatgtcatctaaaaagaaatcaaaatcctcagcctcttcttccaaccttgtgacaaaataaatttacgagtgccaaagcagagaagaaatatcaagacatggtatttcacaagagttgtattccataatcttaaactttaaatgagagagtagactaagggtcaacatttgttgttatttacaaaacaaccacaattggggttgatacagtggtacgagaatttcacatgctaagggccacagagatttaaaagtctatgtatggggcaagtggatccttttttatagaactcaatcaataggttctatagattgccagatattgataatgataacttctccatactgcgtgaagaagggacagtagaccagaaggaaataatacgagagttggataacccggacaccacatggaaatgatcgagcacagatgtcactaattttcggccacagggatgtatgctaaatgcaaagtgtgacattatttcatatgtgctaagcttttgcccagcagcaattttagtgaagtgataaaaaggggactttattgaactatgcgattaggagaagccccaatattgatgcgggcacaattattcaaactaatttattgcatattcttaaaggttccacaactattgatttgggttctccttcattgatatatgctctatgcagagaatgggaaattgtgacctccctagcggggaggtagtttatccaaaatcactgattacttcatttgtaagcaagactccacaagagccccaccatagaaaaatagaggcacgaccatcttgctcccgtcgagccaaatgaagacattattagtcagatcgaggccatgctgttatagctcacaaagaaacaagatgagttggaattgaggcaaaaacagagacatgattagatcccacataaactgaattaattgcaggcatctatgaatgatcaatgtcaacaattgcagaattcaatgcattcacaatatcaatatccgaatgaatttttcacggtgttgtactttgcatatccctacatgacattctctcatcaggcgacattcccatatcatccagccaccaagacccacctcaccaggatgatggcaatgacactagctgatgtattcaggaaagtcctatacctcctttgtatttatttttacattggagacaatgtatattttaagtttgtaggcgaatcattttttattaattggttttgaatcatctgatattaatctcttttgtcagttgttttgtattttgtgaattaatcatgtgctttagttgaattttcttcttatccatgtgaagcatgacaatagttatgcacaataattaagtttagtgtcatacaggaacatgtagatttatatgtataggtcaataggtgatttcatgcatgttaaaaagattgtgtggaatgtttttgactttctagtataggcttggtgatgaccaaacgctaggaatctaacccttgtaaattttgctttattttatagacagttattcagtttatgttttacgcctacactattttcactcaagttagtgagaccgtaggggtatttttaaacctggtaccctttggtattcaaaaattggggtgttaccgactcaaagctcattacaatgatcaataagaataaaaaagggtgaggccaaatgtggagaaaataaggttattgtcataaaccgagtaaaaaaagagcgaaagggcaaaagagtcaaatttctacattaaaggatggaaaaaggaggtatatgatggagagttggcatctcgtcgccatcattgtggcacctatgcacgacaacaagaaaaaaatttaggaaggtgatgcccaaaggatagaagacagaggtgtggcaccatggcatcacacaggaacttcacgcggaaccactcctatggtgtcgaggcacaacctggatgtaactagggcatagttttgtccatttggaaggccataaaaactctaaagccaggaaaaatataacgggaaatataaatataagaatggaagcacttttgggggttccacacattgagagacacaaaatacaacttgagaattacagagcaaaatcaaaggagaagaagaattacttaaagatttagaacaagaagagaaacttgatgcgaaattcatccatttttctacatctcaattcaaaacccagtgatgcacttcattattatttattgttgttcttcatctatcatgagtaactaactttttcattagggcaagcaatgcaatctattgtgacactttatttcttttattcaagattcaagttctttcatcatatatattttgattttagttatgtatttaatgctttgaattacttgatcaataatttaaagattttgtcttttactattctagaggtgagttttagatttaaaacacatattaaatttcgataatttagtataatgtgtagagatacgtatgctaattcttactgtcttaaatgaattcttagaacaaatagtgcgtttaactaagtttgattcacatagagatatgagagtgagttagttaattacgcttaatgagaactcgtgaagggtatattgaatacaatacaaaaattcgatcgaactatacatcagtttatgaatcttgaattaagaattaaaggtgatctttacatgaaattgttttgccctaatatccattccgtatttgaatcatcaagtcaatctatgtgtgcaattttgatattttcaattagttagaagaagttagataaaaaatcaccaaatcacagttttttgtttgttttcatcatattggagttagaaataataaatttaaatattaaagtgtaatatgtgtggaaacgatactccagatttagaggtccactatatcacttgttatgatatcgtacacttgcgatataaaaatgcaacatcggttcctcactttatcttcacattttattttatttacttcatgccattttcctttgataacacgtcaacaagaatatatacacagatcaaattgtccaaaaattaaaatttcagataaaggagacacatggtattcaaacccgaatatttgtttcaaaagaggtagactctgactcttgttttatttcaaatcatattacggttgagcatgtataatgtgattgtatgttatatgtgtctctttatggcgttaaaatatgaactggtgatgtagtagtacactagatatgtgaaattagtggcatagtagtgcaccaacttctcaataaagccactcatcttcagtacatgagcactacctgaagatctttatgtcattttacgctagaaagctcatgtctgattgtacaatttttggaggtgaaaaatcatagtgcaagcatccgtaatctcgtgttgcttttgcaactcaggtgacatagctgctagcatgacacatgttgtagtattatagtcataactatatttattgtaagtagctacctctttcttattcgaatcctcagtcgatgtctctagaaaaggctcctcaagatcataactaattttctcatactcgaaaacaattctcagattgcggtgcagatagagagaatttggctcggttagtatgttggtatccaatatgtctttcaaattcatatggttacttggaattcaaaaactttaaatgacgaaaaataaagaattaacatgtattcaaatgcattgcataatatagtatggactttaattaaattaaatatgctcccaatatttaaaataaattcgtaaccctcacatataaattaatgtaatccatacttgatttctagtggattggtatcccatttattatattaagaccttgagtatattaaaaaagccttcataaaatttgtgggtagatactattatcaattgtattattatacaactctcaaatcattaatctaacaattctttatttctacacatcttatatgttaggttaacatacatttggaatttatttccttaaaagtactcaacaaaagataaattttagttaaatcaaatcaatcattcaaaaatatctaatatttcaactgtgaaatatatccctaataaaccagccttgagtttactcaacaagttaagatcgatttaggactcttatttttcactataatgatggaaagagaattataaatttacttaatatcttagcaaatgatttatcatgtaaaggtctcataataataataatatatattttatcgtacatctagtatacaaataaacatagatataataatatggacaattatggattaattcaatttaactctgctgaaccaaagggaaagctagtttgtcacctcttaggggatattgtattgacttagtatcaatgtaccatttccatggtctcctaatcttcttccatctccaactaaaacctgcattctattctaattggtaggtccaactgaatttgatacgcatgcccataataataacggactcgcatatctaaaataaataaaagctcataggcccacaaaacagcaagaataatattaaccattcaacacatccacatgattgagtccataattatccactaattaaatatatatcatattaatgtattcttatataatacataatattatatgcaaataagtttcaagtttcgagcaattatagttgtctaaactaatttagatagatggatcaaataattaattaatttaattagcggttttatttaattaaaatcatattttaaataaatatcaaaatagagatcaactctaattccaacaatatattagagtgtataatttgattaaaatcacattttaatcaaataccaaattagagtctaactctaattctaattgaatgaacattttaatttatgataaaactccaaaataaaataaaattcagtttagggtcaaagtttaatatttaagttaaaatccaattttaaccataatatagaaagtcgtcaatttttgataaaatcttaaacgagaaaaaatcctctaaaaattaaatttaaaaccttttcaaaatttatatttaaaacgttttgaaaattgaaatttgacgcctagttttaaaactacgaacaggtccttcacgtttattatttgcacgataggtcctgtactttaaaattgcaattttaaccccttgaaatgaaatcactggaaaccctagaattctcttcaaatcttctggccgagtagtgtcgtgtgctactgttgcagcaggcccagcacggtcgttccaagcagcagagatgaatgctgcagacacacatcagtgtccaacgctacggcgctcgcgaagcatcctatgtcgccgaccattcctcccaatcccatttttgacaaacaattaattttctttcaaaaacatatttttaaagatgaaaataaattttctaaattgctagattcaaaagaaattatgaataatcaacttttgattgtcccaagatgcaaaatgatttctaacaatcacaaagtagactctaataccactgttggaaatttactctatcataaatagcaaaatttaaaacattttcaattctcatcaaggatttgctttacgtttagatagaaattatgataagaattataactttagttaattttcctaagaactataacaatctacaattcgcagatgttcaattgcttagcctacaatgaaaatccaaacaaggaagaagatgacagaatcgaagtttctcttttcttgtgatagcaaaataaattatgttatgttttctgaattacaattaaacttggatcattaattaattaatttgtcccattaattagtcccaataaattaattgtgcaaatgtccaacgtcgatcaattaattaattagcatcatcattgttctagttcttttttgtgtgatccattggattcttgatcatgatgcctaatgatgtgaattattattttgtcctaatcaaaataagataaattaaatcactcttttaatttatcattaattcacctagatcaatcaatttgcattttttatccaagattgagatctaataatgtgtcggtgaagcacatgtgacagaaaatgtcacgtggtataacaaaactaaagttgttcttttatcccgagactataattcatttattaatatgatccaattataagacatgaaatgtgtcaatctcaattatcgaattatatttttcattccactattaagtcaatgtaagtcaaaaactgttttcgacttgagtacacattggccaaagatttcattatcaaattaattgaatgaaaatgtagatcataatctcctactatttaagtgtaatgaatccactattgattatttacaaccttcatacgattcttaacatgactggatgacgccgtattagctactcttggacgaacaacatccaacattatgaagtcattattattctcatataaaacactatgatgaccttaagtcaaatgatcaactccactatccaacattggagattaatcaccaccacttagatagttatcaacgtagaattattctagtaggtctccattgttttattattttaacaaaatatcgatgtgttcatctaaatgacaccatattttaacttgtaaaatcagttactcactttacaagtgagaaatgacacacttgatggtctattcatgataacaatatccgtatatcgttattacttaagaccattaataatttaagattcattcatatgtaatttatttatcactaacacaacttcttatgattaacaacttactaggatttgaatttacggaatctatcaatataatttatatgaaaattaattcaataaaataatagatcttgccataaataaatgcattaaatagattaaaagtgtttacaacctaaatcgattggacctagtacataatactaatacgatttgcattcttaagttaggctctggattgtgtagaggatgacagaattagatagtatttggtttgaaaacaaacactacttgtccagggcccatctggccgtagacgtatggcctctctcatttggtttcatcgatagaattagaatgaatttttttggtttcaatcaagctcccaaatgcattttgaattcctaacgattttccacgcctgcaaggtgttagttgaaatgtctcaactggcataagttgattttgagtcttagttttcgtacaaatcatatgtggtccactacattgcattccgttgtacaattttgaattttattgcataatcacgatgatgcattgacatgaccacactacacatggaaggtttccgttcattgcctccatccattatttctgtcccatatttccatcctcctccgttcacgcacttgttggtctgtttaagttttaatgcgcttgtcatattctttatgtataactaatttcaagttgtctatcttatttgaatgtacaatggcatccaaacgaagattatacattgaggaaaatttatagtttagatttgttggcgattgacatcaatatttaatatgacgtctatatttaatattttacgataattagtattttgtgtgatttgatttgcttgttattgttttccatatataaaggaaaatatgaaaatattgaaaaaattcaaaaaaaaaattatttatttattgtgtgcttaagtaaaacatgtgttgtcatcttctagattgtttttgaaacatattaataaaaagggattcgaaattgaactggattattcaaaggagattattcaagaacaatcacgattcaaggaattaagtctttttgtcttgttcttcgtaaaattaaaattcaactaatatctcattattcaaatatgtattttgtaacttttatgatgctcgtttaagtttatagtcactaggatgaagatgaagcctttgttatgaaaatatttggtgtttgtttatcctcggtggttgttataagtttaagacttccgattacttagctaaaaattgagttgagttgtaatcattattttattttaaagaaacaataaagacatagcgctagatataaatcgttatatggtacgataggagatagagatataccgatatgtcttgtatgatctaattgaacgtcgagtaattgaatgcatctacaaatgttcgtaatcttcacagcaatatcgtagatcatgtgtgaagatatgtttagttctaattgagaaacattataaaattgttacattgatcattaagacaaacatgtgttgtcatcttgattatttttgaaacatattaataaagagggattcgaagttgaagtactttttggattttgagttggatgactgaatcgtcttattggccaacaggtttctcaaaaagccccagcctattatcacccaacatagttttattagctaaattcttgtactcagaccatgtgaattcctcataaagttcttcttctccttcttccattagagaggataaaggtgtaatctttgtactcaaaggtggccctccaaagtataccattgacactcttgattttaacctatgagccaatactctatgcttcacgcttctaaacctgccattggtaattacctgcaccaaaccaatttcataataaccttgtcagacttttcacgagttcatacatacacgggagcattaacatggattataagaagaatagatatataaaaacatgacacttagtataataaaaattactataagacagcatacaacgaagcaaagccggagtactgtctagctcaacgaagatggtataaggtatatacagagaggatgcagtaaagataaattacagcaaattaagatatacggaaagcaaaatctcttaaagtggtacaagtaaaatacagtgataattaatttcccttgatcttgaaaaataaaaaaaataaaaaaattctcttccaaacctaatttatctaaactcattttattgagtgacaaatgaaataaatggcaaaatgtacggttacctgcatggaatccccaacattgaagaaaaaggaggattgatcaggtgggactgagacccatgtaccgtctctcatacagatttgaaggcctgatgtgtcgttagaccttacaacagaaattatttgtgggtctgtatgttctccaaatccgatcaagttttcaccactcaatgcttgacgctctgggcatggtggataatgattcacccgaaaacaagaatcacttttttcatcccttatcagactactcaagacatccttcggtcctattttgagttcttcaattatcatttccaaaatagaacacgtcatgttttttactgctgagacgtattcatttattagagacctacacacacaccccgacatacgaagattaagataaatttttactttttactacgtaaagaaaaaaatagataatattgtgtccgaaagttcttttaccataaaatttctgaacttcctggaagcacgacttgagcatcctgtgaaataatctccggcctagtgctcaggagtatgtactcaacccaacccacatcattgtttgggccaatttttctgtaaccatagccgaaagcgttaggagggccatatttttctttatccagtcggggtagattgaaaaacttaatggcttcacattccaatctactcatgaactccattgggacgctatggttgattactttgaaaaatccaatctctttgcaggcctcgactatttgggtcttagcatcaggatctagtagatctaccacaggaattccgtggaaagtgcttgaaatgggcttgcatgtattgttgcaagctaagttgtcaactgtctgagataaaatctccatgccaattgcacagtgcttgtaggagggaggggtagagagaggttaatgaggtgtacttgttaactggagttcaaatgggcaaaatgctcatgcacaaaatgatataagaattcacggggcattgaaaaataaaaggatattgttgggttttgatatccaataaatttggggcgatgctgtaattttcattgactgaggccaatgacaaattgattatcaacaatcaagtctaaaggctcgacccaagaacaacatggaccgttggaagtagtttaaggaattaatgttacttacggcctatatatttaactattggatggctcttgagttttggcccatttatcccttatttggcccaaattgataacctaatgttagactatatagcctccttcatttgcattaaaacgtatgtgatttgtgagtaaaagaagagaaaaacgtggcttcccaaattgagggcgaaaaccagcaacttgtgctccaataattggtggctacctctatgtctttggcctcctcttctgtgccttttttcattggttttctcttacctttgtggcttgaaattcaacatcgatatcttgtcctttgtaggtaagattgagaagcaaccataggtgaatatattggctgagggtcggagtcgcttggttggttgtttggtagagaaagataacgtgaaactgaacttgggaatcaccattttgaagatcttggagcgagcttccacaacaattggtatcagagctcctatgtttcgacaaaatcaaacaaaaaaacatatccaaaacccaagggaaaaaacaaaaaggcagaaatgaaactctccagttttttgaaatctgattggatatgttttcttttttttttttttggccaatccagtgacttgttggtgaaatggagaccactgacacgatgtgtagatggaagcgatcccgatggtgtggagcatggcaaccacgcgtagaggttccttgtgccgcgtgaaggcgcgttcgaagtttttcaataatattgtcgtcaagcaatttgttcccaacatcatttgacattttgtggtgttattattattattattattttttgtttcaggttatacagtgtaatctggacaattctgcccattgcgcatttggaattcaatcgtctttgatggattgcattagttgttggagctttagggtgaatagtggtggccctaaagtttgataaattcacatccatcattatttatagattgtagattgaccctctccaatatattagtttatcccatttaaatttcagcataacaaatcatcgtgtgagatgacattaggattgtgattatcgtgtcgggataaccattgcattgggtgaaaaattgcatttttgttgacataccttcatgttgcatttattattatgttaaaatacctagacttgactcatttgatcattcctttcatatagagatctcgaatattacaaaatcctagaaatctagaacggtttatactactgtcttaggattactttgtgtgacttattgtgcactttagctattctatttgcaaaatgtctttacatttcgaagttgaaatttttaatggaaaaatggattttttgatttgacaataaaagatgaaggggattttagttcaacaaaaagttttgaaagatgaagatgacaaatttcttgttgctttgacaaaagtacaaaaaagaatatgatgaacttacttccacttaattattttacacctatctgatattgtttttagaaaaattgaaaattttgattttacaaaagaactttgaaaaaggttagacgacttatatttggttaagaatgcaattaagtatagtagagacatcttaacacccgagatcgtcatagattcctttatgagtaagtggatggagcttaaaactaaaaagatgataagaggagtggtgtgatatatatgataagaagtagaatgaagtttaagcaaatgagtctgggtaagactcaagatagtagtgacttgaatgatgagggtgataaaaagaagagcaagggttgggacaagttccgtggtaagcggtgttacaactatggaaagtttggacacttgtgagggattgttccaagaagaaggataagtagaaggctaaaatgacaggtgaggtgaatgttgcttttgggctgaatgatgaccctagtgaggtttgttaaaaataaatttagttactgcatgtgcatctgaatataatcctttctacatgtgtgtgattacttaattcagttgcatggttatatgttgcattttcaatatgtttgataagtgcatttgtatgaatttgagatcagtccaattatttggtgtaatgtgtttgcatgcatagtaagttgggatgcaattgcagtaagtttgttgcatgtcttcttggtaagctggagtacaaatacataaggatacattgatggtttgtatcaaggatgtagattgtgacgtttagacatgagtggagatgtgattaaatattgaaatccattatctgtaaaaaccctgattaagtagagtatgagagtggcaagtccatcacttctattaggtggagacccattatctacttatgttggaaaaagtgaggtggtgatagaggattatctcgtgtacttagtatctattgtgatttacttgtcagacataagttagtgatcaacacagtgagcatgacggatgatgagaagagatatgtgctctcgggatgtgagcaatacagaatgtgataggatatgacatgaccagtctcgaatcaacctaatggacctgacacgcgtcgtgcgccgatggtagatgctagctatgtgctgaatacaccactaaggcaaccttgacctgctttgactgtgatacatttaaaaaaaaattggcagagtttcttttaagatatggactaaaaccacctgaataataatcaacttttctcaaacatatacacataatataaaacagggtacaccaaccctcagaataccaactattgagaataaagtgcacaaaaatgaaatttacacttctgaacaaatcaaaacactctaaaagcccaacataatcaaaagataccaattgtgcaatgagcccatgttatggttacattttttgacaaaaatgcttgtatccaaaaatatgaactatctaaactggcaaaatgagtcatacatctgatgacaatgtatggctcaatctgtagatcaatatgctccaatgttgctcaactatgctactatctaataagaaaaatggtgataaaacatatgaacttgtagctcagtgagtggataatttgcaaataagtatattttttccatatatgtataagttctgaaaattcttgcttcattaaaactttgagaaattttgaaatctagtatcactttttaaactatgacataattgtattacaaaattcttcgtcctttattttagataagtagctataaagtataacgaatataaataatctgatatttatgaaaatctatgaaatattattgttgttcaatactctaagttgaagctttattctgagaactgaataaactgaaatttgataaagtatagaaatatagaaaaatcatgccaaaaagctacacataataaccttactcatgtattgattagtgccaatatacatggcaaagctattcaattttgaaattctgtaattcgagtcatgggtgtgcgctacacaaaggctataatatggtcatacactatgaaaacatttacaatagtgcaaagtgggtaaaatcatcataactgatcatacacagtgaaaccatattcacaccaatgcagagtgggtaaaataaccatatgaggtcatacactatggaaacacattcacaccagtgcacgttaaggtaaaaccacctgggtactttctagtgttttttgtttttaaattactttggatatactaaaacaggtaatactcatataacatggtaatgaaataattttactgaattgaatttaacttttgaaaagaattaactataaaatccactatattctaaaaatcattctatcaactcagcttataaaataggtaactttaaatttaatggatacttctttctaaaaaatagatttttccactcacctaagacaagctataagctatgaaaggcgataagcttttccaagctttcacgtcactaactcttgaaatagaatagaacaaatgaagaatcttgtacttgagtccatatttcatcttcttcaataaccttttttcttcatcttctttttttctcttattttcttcccccttttatttcttttctttttcttccatcctttcttctctccttcttttttctgggtttctagttctttccaaaaagagaaaatggattacttatcctttaagtggataaatattgtatacttacaagtcaagtaccaaacatcagcacataaggtaacatttagtcctttaattaaaataataaaacattgactctctaaatttttatttgatattatttctgaccctttaatcctgagtaattacaaattaggccccatgaaattattttacttaatttaagtcctcatttgactctgactttgaccaatagaatttttgactttaagtggataagatgcaacaatcttatccccttcaaagaatttcatctttaaaattcaatcatcttgaattcaaaatacataaaggtataaagtataggtaatgaatgaatttttttagcaacctttaactggaacaatttcattctttcatagcttgcatctcattttgttttttctaattgagctatcgttgacttcactagtaatcttaaagcaccaggtaaatctgacatttacttactaagcctttgaaatagacaatacattcattcttaaataccagatgaacccattgtaaaatccatcactaaccaattgtacccaagttctaaataacatatcaaagactagcttgggcaagagaataaaaaaactgaccaaatcaatcaaattgaaccgacttaggtcggttcaacacaagtaattgttaggattggtttggttttcttttaaacaaaaccatggtagatcaattcagtcgtggtttaaaattttaaatagttggttaactgaaccaacccaacctacttatgtgttcaccatttaaaaaaaaaaatttaagaaaaataaaaatcaagaattaaaactataatctcataactatatctcgatttctccaatttacgatgttgtcggtaagtaatagtattgaaaattttctttcacaagctcaatatgttatacttagcatttttctatattcaaacaatcataacacataatacataaaaacaataaaaattttaaattttctgttgatccatctctattaacctgattttatttgttaatcaatagttcttataatataaaattatttggttattttagttctagtaatttaagagcgcctaaaaggctaaaactagaataatttcttttaaaaaaatttaatttggactaaaattccaaaccgattaaccaaaccgtttggtttggtttggtttaagaggtaggttagttggtttggtttgaaatttgaccaaaccgactaatttgattttggttttgggttggagtcgaaatcgacccaaatcgaaccacgctcaggtctatcaaagactactatataatattttcaatttttcattttaccaattcttagaaaattcaattatttcccaatctaaagttgaggaaattacatttcatgtcctccaaatcttcatcttatatcatgatttaaactattctcttatcaaagtctttctctgtagtaatttaatttataactttcttttgcatctttcatcccaataaacaagtctttggaatatgctaatatcatatataacctcaattatcgtcacttgtatttggttcttatacgtcacctccttgaaaaataaattatcatccaaattcccttcaattaagaaaccatagttgaaacctcttctgaacttgttttcatagtgtctaacattctattaaaagaaactacacaatgtaatttaattatataactccctacaactaagccaaaaacggatactcaaactccaccacataaataacaattttacatatataaaattgtataaatctacctcataaattgactatatcatttgaaaagaatcttgtaaactttatagatctatcaacaatgatccaaataccattttgtgtacttggaaccccaaatgaaaaatatttgaggttaactacttccattcaaaattaacaacatttacaataattcaattgttcatgattttctaaaattctagttatccccaacaacaattgagattgttcaatatggtgctctttttctttaattatatatcacccaatgataatatatacacaatttcaatttcaaccctttcaaataaaagatataccttaattctggtgatcgataagtattcatttattttttattttttattttttgcaatgtgataacactacaactcctaaattcaacctcaatataatcaactttacaaattgttttaatcatgtctcttctgaaatcttacagcataattcacaatttatcattttactttagaacacattctaaactctaacataactaattatcataaaccaagtcctcatcagctttagatacaagagcaaatacttcctcaaaatttaatctgaaaacaaaactttttacacttctaaacccatacaattttggtgctcctttttctatgaagagtcaataataacatttaagccatgataattctatacttttattccataaagaggtcattaacttatcacttatcaccaatgcataagccttcgtgtatattacataaagacctttaattaatattataacctaaagataccatttcacaattgaataaaatttacatttgatgattgtcttagactttagactatccaacatatcatccatttgttccatagcatatatatcttgataagaatggaatactttatttgtgagatctttacattattaaaaattcattatcttcaccttaactttcaaatttaactcgaagcctccaaattgtatgtaatataacataataatcgaacaaatagccttggcaaaagtaattaacttaataacccaaatatatcatcacattattttgctattaaaccttgccctgtcccactttttcttttctttctattcacaccttgtaatacttaattacacaccaatttcttaaataaaaaaataaaatacaatacctaatctttatttctacttccttttttaatggcattacctcgatcaactcaattgttcaccataactaaaattccatcttcctggtaatataatatggggacatattcctattgacttcatgtatccacaagaagcctgtgtttagatgacatggctaaaaatgcaatcatatccaacataatattttttgatcattctaggctctaaaatacattacatgtcgtccataatttcttatccacttgttatattacaaataaaaatattctattcaggagatccaaattatatgtgaaaagatagtaatccaaatagaataacataaatctcccattgtaacctaaatatatcatcacattaatttggcataataccaatcacaactttcttttatcactatctccaagatcttctcacaatcatataacctttttacatgaacatcatcatacatattgccttaaactttttatcatatcatgtcctataagttgcacaaatatttcatcatatctatcttgttaacctttattgaatgaatatcatcatacccttatcaaatgaacaattatcgatgagactgtgcatccaattcacatccttaataaatattaatatatatctttttactatttactttcttattcttcaattcaagtggccgctcaatttgtcctactcatttttttctcttatacttctttgattctgattctttgtcacctattctttctatacttgagaaatgaaatcaacgctattcacgtgtccctttttttccccagattcacataaacatgcctcaatgcacatatccatttagttatatttcttaagcaaaaaattgccatataataagtaataattatgaagtctatccctatatttcttatatcccttagtataatcaaacaactcataagtaattgaaaaaaaaaatttggaatcatttaaacgtaatctcatcgacgcctaaggtatattataacacattgttatcaatccatcaacaaattatcacttttccttctacaatttcttatcatatagcattaatatacaccatcgtgatttctatcatcatctcatataagtggccacaaattaccgcaaaattttgataacactaatgacaatttggcttcccaacttagttaaaacttctcgttgactatcaccaattacacagataatatcattcctttttacttataacgccaaaccttaactagagatttttctatgtatacattaaaaattattgtaattctacatataaattgatacttaagtgactgtgcaatctatcactttaaatgcctataagtatttaacctgcaaaaccatcaaaactttcacgtttaaactagcaatctgttcaactcttaataggctacatacacaacaattccaacccaacaactaataacaatttcaaccagcagatcattgcaattgacatacatactattcatttctaaatatgttaaaagtatttttcaaccattttaggttccaaatattctagagcaatagcttgagagcttatgatttctgccaccacgacatatgaccatactcactgaatatgcatgatatgtcaatgtatgaactatgaaactttataaaaatgctctgataccaattgacacgacatgtcccaaatcaacataatggacctgacatgtgtcgcgtgccgatgatagataccagctaagtgctggatcccccactaaggcaaccttgacctgctttgattgtgactaatttttttttaaatgacagacttccttttgaaatatggactaaaaccatctgaataataaccaacttttctcaaacatgtacatataatataaaacagggtacaccagccttcataataccaattattcaaaataaagcacataaaaatgaaatttacacttctgaacaaataaaaaaaactctaaaagggcaacataatcaaaagaaccaattatgcaatgaggccatgatatgttacattttttgataaaaaatgcttctatcccaaaaatatgaagataaaatgagccataagatgacaatgtgtggctcaactcggtagatcaacaggctccaatgctgctcaaatcagctactatctaataagaaaaatggtgataaaatatatgagcttgtagcacagtgagtagggctggacaaaactctcgaatcgaaccaactgaacccgacggttcttctcaagttaaatacccgaacggatatttgaattgagaaccgacgggtatggttcggttctcggttctaggccaaaatcagaaaaatcgaataagaaccgaatttccctaattttttaattaatttattttaaataagcaaaattattttattttttctaaataaatttgttaactagttaatttagttcaaacaaaaaaaatatgatttttctatttctaattttcagttcaaagtcaacttaatcaaattgacctcaattttatctaaatctgttactctaatgtagtgtcgtttctattgaagaaaatcaaattaaagctttacaacatctcttttaattattttgagctcgctatctttctcttcatgtgattttaataatcaaatttatgaagaactcaacaaagaaagacgtaaatgacacataagattggactacgttattttgtaagagctaagattgaacatatcattaattaaattaatataactttgtatatattaaaaaaattaattataatacggaatctcagaaccgaatggaaccaagcccgaacggttccataattaaatttgaacacaacggttccacttactaaatacccgaaaatttcggatcgggtcgattcagttctaagaaccaaaccggaccatgtccagccctaatagtgagtggatagtttgcaaataaatatattttttccatatgtgcataagttctaaaaattcttgctctatcaaaactttgagaaatttgaaacctagtaacacttttcaaattgtaacatagttgtattataaaattctttgtcctttgtcatagataagtagctgtaaagcataacgaatataaataatcttatatttatgaaaatctatgaaatattattgttgttcaatactataagctgaagctttattttgagaactaaataaatcgaattgtataatctgaaatcttataagctatagaaatacttacaattcacaccaaaaaggtactcgtaatgaccttactcatgtatcgattagtaccgatatacatggtaagctatttaattctaaaattccataattctgtaattctagtcatgcatgtgtagagctgtccaatggctataatatggtgatacactatgaaaacacattcacgataatgcagagaaggtaaaatcatcataattgatcatacaccatgggaatacattcacactagtgcagagtggataaaataaccatatgaggtcatacactgtggaaacatgttcacaccagtgcacattagggtaaaatcacctgggtactttcctttttttttttaataactttagatgtgctaaaataggtaccctcggtcggttgaaccagcagcttccccatcacctcctccaggtcaggatggtcataaattcaaccattcgatcttttccaaatgaatcgaacctcgataagtcacatcatctgaagcagcagcctcaatttgagacctaatttgatacgggattggcgactgtttttcttgcatttatccttgcgggtttttttgatggaactgaggctgccccaggtcaagattcaagacttctcctatcaagtcaatgttcaaaatgaaaattgtaagaattgaataggaagataaaaggacattgttcagagtgaaactaaaccaaaggccctctctctgtaggactcgctatctatgccacaaggctggcaaaagaccctgattggctacttcgttggccaaaaatagcattttttggtactcatataacatgctaatgaaataatttagttgaactaaatttaacattaaaaagaattaaatataaaatagtcaacttttaatttaatgaatacttatttttgaaaaataaaattttccactcacccaagacaagttacaggttatgaagaccaataagcttttccaagctttcacatcaccacctcttgaaaaataatagaagaaatgaagaaccttgtacttgagtccatattttgtcttcttcaataaccttttttttactcttattttctttcctcttttctttcttttctttttcttccatcctttcttctcttctgcttcttttctcggcttctagttctttccaaaaagagaaaatggattacttatcctttaagtggataaatattgtatacttacaagtcaagtaccaaacttcacataaggtaacatttagtcctttaattataacaataaaacattgaatctctaaatttttatttgatattatttctgaccctttaatcatgagtaattgcaaattaagccccatgaaattattttacttaatttaagtcctcatttgactctgactttgaccaatagaattttcgactctgactaaattgagtgagatgtaacaaaataagtgttatgagatctttttatagggttattaatgtatttgttgcatatgtattgaccatttgattgattactttattttaatttgttgttttgtgtgaacacgttctgaaaagatttgtgttatcatattatatatcttcatcagaagtttatttactcttgattgattattgtgaaacacgaggtaaggtatacgatcccaattttattggttacctttatcatgcaagtattaactttgtatttcattacccataggatgattgggtatcaaagtggagatttattggattttgataccaaataaatcctaaatgataatttaaaacgtcggaatatatttttacaagcatcagtcagtggtgaattgaataccaacaaccaaatctaaatgctcgacctaaaaataacaacatggaccgtttgaaataacttaaggaattaatattgccatggcccatgtatttacatattggatggttcttgggttttgtccatttttcccttatttggcccaaaatgataaataatgttagactgtatatagcctccttccttagcattaaaacgtatgtgatttttgtgtaaaataagagaaagggtatctgcccaaattgagggagaaaatcggcttcttttatgttcaaaaactggtggctaccttcgtgtcttcggcctcctctctgtgccttttttcattggttttcttgtgcctttgtggcttacaaatcaacaccgacatcgtttcctttgtgggtggattgagaaactaccgttggtgaatatattagttgtgggttagagccgttttgattggttgtttggtagaaaaggggaacatgaaactgagcccaaaaattattgttttggagatcttggaatgaggttccgcaatagacgccatctatgctaggtaatttagtgtttaaaaaaataaaaatactaaaagttactttttgaattcaatcaaatataaatttcatctacaaatttatattcttcatttattaagcacacacgtcttgggacccgatcgatactattcctcctaaaaatttagtaatgattttacctcgacacccttctatgtcctctcattgtacaaatttattgtctaaagtagttaaaagttcaagtaagtagaaaggagcggaatctcgaaagtgacaaattggatgccgtaactctcttttatacttgttattcatttttctgaaaatatgcgggaatatcttaaaacatcaatggaaaatttcattcttgtccgatttgtaacatcccgactcattgacatacaaaaaggaaaatttactaatacaagttattatgtctatatatgagtggatgattgcggaaccaaaatcatagattttactccaacacgtggcagcattgctttacaattccatcctcaaaatgctaaatcaaccaaataacttgtcagttccataaaagtttcagaatagcgacaatcggttactacattttgaagaacgagattcctaacaaagttagtttatgaattttattttccttcgttgagagtaaattcctactagggtcgtgaatgaaatattaactttaagcatgccatattctattatttttacgtatgcttggagaacataaacgaatggaaggccgaattcgcccattccatgaatttgtaaacagaataaaagtagagctctaaagagattcactgcattaattcgcacttataccaatgtagagggttgctatactgtaaaacctattcaggatagaattttttttggttagttgaatattcgataaccagtagtttttcctccacggcacaatatactttttcagacgataattaatagaaagttattagaaataaaatatatttgaattctttaaaaaacttacggaatgactgttgcgtttaactcaaaatagtaaagttaaattctgtcaaaatctgattaaaaccctagttcaacaaaaaagagtgatcaattttacactacactgtctagtgcaaatttggagcaagaaaaggaagataacttcacgtgcagttagattaattattatgaagatttcggtagttgtatatgtgtagtgaaatggttgtttgttatttgacaaagtattgctcaagtttaattcgtaggagtgtaattaaattccatgcaatatagaaaagaaaagaagaagaagattgaaaaaaaaaaaaaatagtgaggaaaagaaatctgaggcaagtgattaaaaccctttttttttttttttttttttttttttggcacttcaaaccacaagttagagcgaactctaacgaaattttttctctctacgagaaactaattttggaatgatttttagatagtttttacaagagattttgatgtaatactcaatgtaaatgatatatgattcataatggacgtccaaaggatcctatttatagaaactgagaggtagtaagcgaagaaacactgctgttaaagaaacttttcacccgcgtgctgtagcctatatctcgaccaacagcttctccactcgcttggccctggagtggcagtactatatgattttttcctcttcttctcctagtttatccttccaaatttgaaccacgatttctcattgatccgtaattggttttgaaatttcaaatacactatgacgatctactcggcaaggagaacaagttagtcttttaatttttatgatttgactatcggatcaagtccaaaaatttggtcgaatttggcacaaagtcacttttcaaatttatacttaaccaaatttttttaatttttaaaccaaattcctacaataagtatacttgtcactaaaatctcgcaactgtatggttaacaatcaagtaatagagaatgagtaaattaccgttcccactaggaccatgtactttgcccctgtgttgttgcctattattttgcaaaaaaaaaaaaaaaataataataatactaaaaaaataaaacttgcatagtattttagaaaaacatgtggttgaaaaatagaaaaattttggatttacatacaaaatatattattgtgtgaatatgtagttgaaaataatcctgtagcaaaaaaagttttaaaacaataggcaccaaacaagggcataatttagtgtgtatatatataaattgttgcattttttctattgcatgtgtacgatatagtaacaaataatataataaacattcaagtccaaattatcgcttccacaatgactataatttaatacttgatttactatttctaacttctatttgataaatgaaaacaaatatgattttggtgattgcttgatctaactattaataataactagaatgtatctaaatgcatctaaacttgaattagggtttcaaatatggaataaatattaggactcacaattttatctattgattaccttcaatttttaaatcaagattcgcaaatctaatgtaatgcttgatcgaattcttttatcgtgttcaatttatctctctcaagttctcattgtgtctatttaaataagtaatttcataatcaattttaggcaaacacaattattgttataagaatccaggtaacgactacaataattagcataagtatctctacgttttatactaaattactgaattttactacatggtctaaatataaaaccgacatctcgattcgtaatagatttacaaaataattgaattattacccaaataattcaaagtattaaattcaaaaataaatttaacgcatttgttctgaaagaactagaatcttgaataagaaataaagtgtctcaagtagattatattttttgtcctaataaagaatttagctactcatgatgtaggaagaaaaacaataaacagacattgagtacattatcgaatttttattaaacataatgataagcagatgaatcttgcaccaagatgattttcttttcccctccatcaatattcaaaaccttgagttcctgatgtttttctattttgatttgttctcctaatttacaagttgtattgcttgttttgcaaagtgtggaacccttgtcaagtaccttttctcttgtgtttatactttccctaacgtcttcctcgaattcgtcaacttatagcaggcagcgtttaggtgccatgtgagtagcgccacaacatcgtgaaattatgctcggtggcgccatgtggtgccacagcgttgcctctcgggaacaatttagcattgcacatcttttagtatttttatcataactttttcttccgatatttgattgaggtgattcaaatttgagttgtaaagataactaaaattttacaattttaacagaattagaattttatcaaatagaaatttactaggtcaaaaatgggtttcaatccctggctaaaactttggaatttgcttgtgcaattgaaatggatttgtgtacatattttgatcatattttgctcctttttgacttcttattatatccaattgatgcctagcatcctcgaatcttcatcttgaggttcaacacgactttgaatatttacactttagtcattaaactttggatctcgcccttttttgccaatttttgtttctttatttcaattccacttccattcgtagaatttcacctaataaacgaaatatacaataagttaggctataattgctcaaaagaactaataaatgtctatatttttagtccaaataagttataaaatacacttatcatacatccaaaaactgcaacatttgtttgtcctcaaacaaaatcataacttaacttaacaaatacaaaaacatgcaaaaggttttggttagataatttgccgttttgcaacaagattgaaataattttattaaatctataaacaactccaaactcacattactaaaatcaatatctacttttccaatgtaaaactgatgtgtctatgtgtgaagaattaagtaaaatactataaattcacgagttatttcaattcttgacactagatggtcaaattttttactttcatcactcatatgattcgcacattcctaaacttattcttctttactcattttacagtgtatgatctaaggctaaatctttatactaactcctcaacctctctagtttagatgtatgtcacacttcgacaaataatgattttctaaattttgattgcttcaacctcaaatacttaactaggctaataatccattgtcaaccatctaatttcctcaaataaatgtatgtagtacataaatacataattattattttttcttttcctacgtccaaacttttctcctttaaactttctaaattaccgtagtaatgagctttagaccaatgaccacaagtcaaattatcgtagtgtaatagatttttagataccgttgtaggcttaattacatgagtcataaaagcctacgaaaagacgtttcacaatgaggtagacttttttctctcctttctttttttttctctctctcttttcccccccatgattagtgctatgctccccattaaatatctattctcaaagattagtccctaacataagattttcacccaattttcatcatatcggtattagatcttccccacaagaatttacacatatgaaatccccattcatatccatatctttctacacaataaaatcacccacgatgtaatgtcccaaatttttactattagttagatttaaatttaggaattaagtgcactattattaaattttaatgacattattgattattggcctagtctaatgaacttattaattattgaccaatagtttggcagactaagtagaaagttattttggaagttggatgacatcatgcgtaaaacataagtaaatatgccggttggtcttggttaaagatgatttattgaccacatgcattatctacaccacaattcaagcaatgccattgatttgaccactatataatggaaaatggtttgactgtatacattatttacaccaagctttaagctaaatgaattgatttgaccaagtaattaaaggtattgattgatttgactattttcatgacaatacaccatttatgcattaaccgtacctaacatctagccatttacactacaaatagatgataaaaccaatactaaactaccccagaacaactatttacacactctccctctctacctcctctctttctcttgtaatttttgtattaaatatagccatacacttatacaatcacacgtgaatgatcaaccccacacgcaattcaaggatctctttccaacaataacaccttttaccatcttgaattgttagtgaaaaggtaagttgtgctttatgtttatagtggctaatgtttatgtatgtaatatttccatgactatgttatgtttggtccatgttatgcacgttttattaagaatggatcggagtttagtagcacaacgcacgagaatttagcaccatataagttccgtctaattttcacgtttccctatacaagtcttgaaattttcataggaatacatacatgaatttattatccatgtacgcttattaaaaattattttcaccctattatgtctctacttttcagataattaatgattcgaggtggttagtatggagatggcttctggtggcaaaagtttcaaagatagaattattacattgtcaaactattattatttcatttgattttaaatgttctaatgtatttctcatttcaagttaatttattaaactcattacattattttaattttggtaagtactttaataatttatatgattgtgttgaatattctttaaattagttttagtttatgatttaatgtcactcgagtcgttaaggattcaggtcgtcatagttggtaccagagcgtgtcaatttccttgtagactctgatttaaggaaaaaaaaattatgtcactgttcacaaaaaaaatatattttttcattattttttcgtttttctttgcaaggaattttacaattcaaatactattatttaaattattaattcgaaataagttgtttgttttaaataaataatttttaataagaattaaatggtttcttgcacgcaaagctatactccaagtcgtcacccctcgtattaggtatctcataagtttcatcgctatatataaaatctttagtttatatgcacatatgattatgttcattatgcaaagaatgcaatttatcaacgcacgaataagtatgagttgctataaaaattaaaaattgttggaactattgggaatctacttatcatgtgcaccgaaaaattaatacatatttcaattccccaccaaatatctctttgtatttagataggaattgtgatagaaaaggtaccttttacgagatctgcaacctcctttgcaattcttgcttcgatttgtaatctcctttgctattctttcgtcctagtaaccttgatctatcactcacagctgtccaattgtccagtctccaatgatgatccatacagagaacaagattgtaggattatgattttcttcttatgctagcaagaagaataaagaaaaaatctccacaaattgaaaactctagtgacttatttatataagtccaaatgggcttggcctgacccggaccaatatttaattaacttatttaattaaatctggcccgtaaattaattaattcggacctataaataagcaacccaattaattaatttatccaacgcttgttaaattaattaattgacaaatcacaatcttctagttctccttttgtgtgcaacccatcaggttcttgaccacaatgcccaacaatgtgaattattattttgatctaatcaaaatcgataaattaaaacacccttttaatttattatcaattcacgttcgccgtcccaaattgacatctagcaatgtgtcaggacaatacatgtgacgaaaaatgtcacgtgttatgacaaaaccatactcgttcgtttaccaggaaactataatccgttcatcaatatgatccgatcaattaggagatatggaaatgtgtatatctcgattatcgattatatcttttatgccactactaagtcaatataagtcgaaactccttttcgacttctgagtacacattggccaaggattttgctatcgacttaattgaatgaaatgcagatcataatctcttactatctaagcgtgatgaatcctctattgatcattcacaactttcatacgattcttgacatacccgaacaatgccgtattagctgcccttgacagagcaacatccaataacatcaaagcatgattgtcctcatataaggcacaataacgatctcaagtcaaaggaccaattccactgccgaacattagagattaaccactacactcagatagttatccaagtggaatctctcgttggttctccaatgttttgttctataacaaaatatccacgtgttcattcaagtatcactacactttagcttgtgagatcaactacttactttacaagtaaaaaatgccacacgtaatggtctatccgtaataatgatatccgtatctcgtcattacttacgaccatggatgatataggattcaatattatgtaatttatatctcacaatcacaatttcttgtgtttaacatattactaagattagaatcaatggactccattatttaattcaattgaataggaattaattaaataatagatcggccttaaattgcttcaactatatactaaaagcgtttatatccaaagtcgattggacctagggcatagcacttacaaattcccacttgcactagatccaaccacttttgtatctaatatcataagaagttacatgacgatcatgtttatactgtgataactctttgtcagtggatttgcaatattattaattatgggaattcgttcttctgtttacgtcatttctatgtattatctctccgatgagattataccaccttaataaatatttggatcattaatgagaccatagttcctttcgcttgtgcgatggcttcattgttatcacaatttaatggcatgtgatcaacaatgtaaggaactattcgaagttcattaatgaatattttgatccactttgcaattccgtgctacttctgaagtaatcatgtattaggtttctttattgaaccaatagatgtttcacatttagaacctttccaacacatcgcctaagagttaaccagtttctccatataaaaatattctcaaaattttatctatgcagattgggatgagtaaagcaattttctagatctatttctatagattaagtcgcttctctcatatcgttcatgaataaatcatttaacaatcattatttcaacgatcgaaatataggaatgtcattttctataataacaggaatataacaatgctcctactatttcttgcaaacacacaattcatcttcatatttgataaaattaaacattttgacttttctatcaaatcgaagattttagctccaagaggcttgcttgaacccataattatggtatgtaactattacgaccaaaattcgaatgaacttcagcatggctacatgcgaaaggtgtaattaaggtcaacacttaaccttttgctactagtcttactttttatgttcggatattcccatccatgtcgaccttttccatataaaccatttacaacctatgggttttatcccatcaggagggtcgaccaaggtccaaaccttgttcacatttgtcgagttcatctcgagtttcatggcctcttgctatctcttttaagttaacacttgactttattttcatgcaatcagtaggtttatcgtcctggatcagcaatgccgaattagtaatcatggatttgcaccttcttgaaggtcgaatgatcctactagatttaaatggagctgccatgtcattaggagttctacttcatgatcaagagtaatccctcgtcaggtgtgggaccaaactcggattcatttacttggtcaactatatgtgtggacttcctcccctatagtaaacatttttgtaagaagatgatacgtcgtgagacaaagactttcttcttaatgggataatataattgatatccaaatatctattttggatatcccacaaatatgtatttatcggatatagtctcaagctaatccaatttagggcacttcaaataagcgtcttagtcccaaactttcatttgagaaaaattgggactattccatagctcgtatcaaattttgttaatcgatttaaatgagacatgttttagtgtgacacactaaaataagtacatgacctcaaaacgattttaggaggcttgcatggcttattattaatcgtactatatctaatagtttacgattcctctttttagatacaccattatgttgcagtgtatgttgaggagtccactacaagagaatcacattctcttttagataatctaaaatttcatttttaaaatattcccacttgatcgaatcttagtgtgagaatctctttacctaattgtttctctacttttagcttgaatcccttgaacctttcaagagtttcacgcttgaatttcgtcaagcatatattactatttctgtaatagtcattagtaattttgatgaaataagataaacatcacatgacatcaattgacatgggtccatatgcatcagtatgcattagaccagtaattatgcacaccttttttctcttcaagtaataggagatttggtcattgtgccaaacatgcataattcgtacttgtcaaaatcaatggatcccaagtatacatctctatataactttggaatttcatttcatctatatgacaaagtctaccatgccaaaattaggtaataattagattatcgcatttatgcctcataaattctatactcattatagaatgcttagtattaagaacacaaacattgttttgtaatttaccataaccattaagatctttatcaagataaacaagaacaacaattgtccttagcagtaaaatggttcatgtccaaacatgaaactcatttaatattccagttatggttggtacaaagtaacatttctctaattccaatattaagcctaaaggcaatagcaagaagtacgctcctacaggcaatacaacaatctttgctcattttcaacgtacatgtcaacttcttccttttgtaccagtctacttccatttagtttctccatatttgtataaatatgagatctacatctagtatctaatacccgagaagattttttcacaaagtccctttagattttctcttaacatcggtagatgaatcaatagtttacccactactaactttgatatcgggcttaacagtcttaagcatgttaaacaactcaacgagtatgtattcaagcttattcatatcataattcataattagtataaataactctctgacagaaattgcagaacgaagtcaatacttagttcacagtttatcactaaatttaattgagatgacttctcaatgccaatcatctttagtacgtaagcattgactgaagattcctatgtcacttttcatcgggatagtttcttggaagtctcatgtccttccatacatgattattatcatataattctttgaaatgaaaaatcatacattaacatctatactttcaagttgctttcgtaactcaggtgacgtaatgcaaacatcacacatgttgcagtactattgtcaccactgtgttattatagcagtcacctcttccttaaccgagtcgtcaccaggtgtcactagaaaaggactacttatggacaaccaactttttcatgcttgagaacaattctcaagttacgatgccaataaaaaagattcaatttggttgttggcatctagtatgccactccaatacacatggttactcacgattcaataaatataaatgacgaaaaggaaaaagaataatatataaaatgcatcaattaatttaacatagacttttattaaatttattatgctcccacaaatcagtagccgttggcgttggagcagcaggagcagctgcgggcggtgatttagttctttcattaaaaaacccgtcggtgcttttgttgttgtggaataagaagcctttgtatcttaatgcacatatttaattaggcgtattgtgccagttcttttgagtaatatatctagaaatgccccttgataacttcttaacatcattttggacacaacgattattccctagatacacacgtcgtgttattctctttttcaaaaaattgaaatgattgaagtttttctaattatgctcccactatttaactcaaatttatgacactctcatataaatttatggagtccatacttaactcctagtgggttgggatcccatctgttataccaagaccttgagtgtactcaacaagccttaatataacatttgggtagatactattatcaattgtatctcaatacaactcctagatcattaagctgaaaacttttttctttatacatcttatgtgttaattcaacatgcctctaaaatttatctccttgagtgtactaaacaaaggataaaatttagttaagttggatccatcattcataaagatctaatatttcatagtgtcagacatatctttaatagaccagccttgagtgtactcaacaagttaagacgatttgggactttgatttctcactataatgatggaaggcgaataataaattgacttaatattttattgaggggttttgcattcaaaactcttatcaacatcaatataatttattacgcatcaaacatatatgatgatgatgatgataataataataataataataataataataataataataataataatagtgtggacgattatgaacttttactatctagtcttttggagccataaggaagactagttggtcaattcattggaggtatagcattgaatcagtatcaatacaccatctccatggtttcctcctcttcttttggcttcaattaatccagctataacatatatcctatactagttggtatacaggcctaaatgaaattgaactcgcaagcccataatacgacaagaataaaaccaaccattcaacacatccacatgatcgagttcataatcatccactaattatacattcatcccataaatgtaatcctatataatatctaatattatatacaaatatgtttcgagtttctagcaatgaaggtcgtctaaactcttttagacaaatggatcgaaataattaaataattaattaatcatattaatcaattaatttaattagcgggcatattaaattataatcaaattataattaaatatcaaattagagtccaaatttaattccataattacagggcggggttatttagataaaataaaattttaattaaatactaaattagagtccaactctaatttcaaattttaaggtggtggaatttaattaaaataaaatgttaattaaatagcaaaattagagtccaattctaattccaagattttaggacgaactaatttaataaaaatcaaattttaattaaatatcaaattagagtctaactctaattttaagaaagattttagggcgaaacaattttaattaaaatcaaattttaattaaacatcaaattagaattcaattctaatttctagaatttattcggatgaataattaattaaaatcaaattttaattaagtactaaattagagtcaaactctaatttaaattgaattaacattttaatctaggataacactcctaaaaaattgaaattcaatttagggttaaagtttaacatttaagttaaaatcaaattttaacaaaatatgaaaagtcgtcaattttaaataaattttttgatttgggtcaaataggacaaacccatttaaaatataattttaaaattcaaattcaaaacacttttgaaaattgcaccttgacccattttggaaatagtaacacagccctcagtatttctaaaatttcacgaagggcccctatttaaaattgcacattgaccttattttctttaattgtaggtgctaacccgaaattttgtaaattgcagggaagtccccatccccaattcacctcacccgatttgcaaaaaccctaaaaaaaatagaactagggggcgtcgccactcgacagtaagtaaagcccgtcgccaatggcgacatgcattgcccttgcagcaatgcatacactgctgcaacaacgagcaacaatgcgtgttgctgcgacatcctagagcggcggccattgtggtcgtggtcatcactacttccaaaccttgagccgcagtcgtgccactaagtctccgtaggcgaaccattgttccaatccattttctatcctttttatatttaattttttttacaaatcaaatttcaaaaatataaaaatcaaatttcttcttaattgccagaaataagaaaagaacaaaatccactttcgattgttcccaaaaatttaaaacaatttctagcaaacacaaagtatgagctgataccactgttgggaatttacttatcacgcgtagtggaaaattaatacagatttcaattcccatcaaaaatctctttatgtttagatagaaaatataactttttcgagatctgcaaactctttttgcaattcttgctttgattctgtaaactcatttgctattattccattctagcaaccttgatttgtcacccacaactatccaattatccagcctccaacgatgatccacacagaaaaaaagattgtaggattagaattttcttctcgtgatagcaagaagaataaagaaaaaatctctacaaattgaaaaccctagtgacttatttatataagtccaaccgggcttagcctaacccggaccaatatttaattaacctatttaattaaattcggtccgtaaattaattaatccaattaattaattcgaacatataaataagaaacccaaataattaatttatccaacgctcgttaaattaattaattgacaaatcacaatcttcgagttctccttttgtgtacgacccttcagtttctcgaccacgacgcctaacaatgtgaattattattttgatctaatcaaaataataaattaaaacaccattttaatttatcatcaattcatgttcattgtcgtagattggcatctagtaatgtgttaggaccatacatgtgacgaacaatatcacgtggtatgacaaaatcatactcgttcgtttaccgtgaaactataatcccttcatcaatatgattcgatcaattacaagatatgaaaatgtgtcaatctcaattatagatatatctttcatacgactattaagtcaatataagtcgaaaacttcttttcgacttttgagtataccttggtcaaggatttcactatcgacttaattgaataaactccaaatcataatctcttactatctaagcaagacgaatcatttattggtcattcacaaatttcatacgattcttgacatacccgaacattgccatattagctgccattggcgaagcaacatccaacaccgtcaaagcatgtctgtcctcatataaggcactatgatgacctcaagtcaaaagaccaattccactaccgaacattagagattaaccgctgacactcagatagttatctatatggaatctctcgagggtctccaatattttgttttatagcaaaacatccacgtgttcattcaagtgttactagactttagcttgtaagatcagctacttacttcataagtaagaaatgccacacatgatggtcgatccgtaataatgatatacgtatctcgtcattacttatgaccatggatgatttaagattcaatcatgtgtaatttgtatctcacaatcacaactccttgtgattaacaaattactaagatttgaatctacagactccattatttaattcagttaaatataaattaattaaataatagatctgccataaatcgcttcaactatatattaaaagcgtttatgtccaaagtcgattggatctagggcataacacttacaaactcccagttacactagatttaaactgtttaaggagagcttgggatttaaacggtctacttgtaaccccctcctctcctcgaagccttttagtttagcattattcaaatcaacatgacagaaattcacatctaaaggaaaaaatttcttttttcagaagcttttaagaaaatttcatttttagaaatatttattccaagaattcttatagaaccctccatttcaagaaatcctcctttcaaagaaactcttttttctaaagaaactcaaattttacaaatttattttaaataataataataataataataataataataataataataataataataattaatatgttaattttttgcttgtctttacttattgtaatgttaattttgaacagggtttaagggatgatctaaggtgcctatcgtggtagtgtttgaactaggaacttaccatgaattattaacaaacgcacaactggcagatttcaggggtcgctccagtgggagaacaagcaactatatgggcatatggaaaagtgcaagtggaaagataacacgagcaaaggacaataaaactatgataagaaaggaaaaggagacccaatttgaagtgatagagcttcctgctttgcaagaaatgtaagaaataccatttgggagcttgtctcttagggacaaacacatgtttttggtttggataacaagggcacatggccaagttttgcactaagatccagcagaaacagataatcacacagcatatgtaagaatatgtacccaagggacaagtaagaatctttgcattgactgaacggaagaggatcaagatcgtaatattttgacaagtaatgttttaatatccagcttatatgcttatgtattaatagattctggtgccactcactcctttatatcccttaaattcgtacaaagattagatgtggatattatacttgcgagttcaccctctggataggtgctgaatacagataatgtagttaaggtagtaaggatagaaatcaattaggtctttagagatggagctttatgtattggatatgggagatttcaatgtaattcttaggataaattggatatccaagaatcatatgacaattcatttttcgagaaggaggtggttttcccaaaacttagagaagataaatttcaattatcagtgactaagagtaggtccccatccagtcttgtgtcttcattacaagcatgacagatcttacaatcaggaggtagtacgagttttcctattcaacaatagacaaagaagaagagaagaagttgacagtcgatgaagttagagtggtacaaaaatacccagaggcttttccagatgatttacccaacgtcactgtaacgagaaattgagttcgcaatctatctcacctcaaggccttacctatttctaaggccccttatagtatgacaccaaagatgctacaaaaattaaaggcacagatagaagaattgctagagaaaggattcatttgacccaatgtatcaccatagagagctctagtttgttttgtcaaaaagaaagatggatcgataaggatgtgcattggttaccgggaactgaacaagattactattaagaacaagtattatcttccaagaatcgaggacttatttgaccagctttgaggtatattggtatttttcaagatcaatttacgatatggataccaccaactaagaatcaagacatgtgatgtctagaagacgagttttaggacttgacatggtcactacgagcttttacttatggccgattagtgtcaaaaagtgcttcaaagatatatcatttacaagttattttaccttcattttgtatgaattcactaattttagtctctaatttcaattcatttgccataaatttaatttgcataaatacatggttaaaaagtgcaattaaccaaaatatgtatttacataaatgtcggcatgaatattatgctcttgaaagagtatttatttggtgcatttcaaatgtatttccaatgtaaagcaagtggagaaaaaattgcttaaaagtaaaaaaatgatgagctgtctcaagaagatgcagatgtctcggtaaattgatcataatgtgagctatagacaccgaatgaaggtgattcaagttggataagaaagataagatatgtattttggaagaagtcaaattcccatcatagagcagccaaaattaccgttcaaagttcaaggttgttacttgtcgtatacaacttttctacctatgagtagcactaattattttggcaatatctggagttgtagagatctaatggacctgatatttgtatcaatggaaaggtaactcgagtggcaacaatgtatctactgattaaaagtccaattttgctgcacaacatagctaaaaattggtatcaatttgtatattctaattgtcttcaagctggatagaacacaagttgcaacttgtccacttgcatgcttgatgtttctttgcctataaaaagaaaccatggccaagagtttgagggcatcaattcctcttcatcatattctagtttccttcattttctctttgttacatttcattatgtatttctaaatatttagctaaagctagggttgaaactttgataaatgtatagtattgtctttgatctttcactttgttcttcaatgttcatcttattacttggttgaagtatatgttctacaaatggttttcatttgttaaagactttgatttattgttaacaattttggcccaataaatgcttagataatctctacataccaacaacttattttaacatattttctcaaacaattatcaagaactatcttttagtatatttgcgatcaatgtttttatcttccatatgagatcactagctagttgattttcatgagttaaataaaagatcaagaataatttctactcatttatctgaagtgaatccccaatgctcgagtgttcttcttcatcgtatttccaccaaccattcaccactcatagactagtttatttctttccaattcactatggttcaaccttggacttccaagtttactatttgagacaagctgcacttgggcttgcaaccttaaagttgtagtaatgccattctggttgacaaatactccggagtactcatggacttggtaaaccgtgttttttgtgattttcttgactgatttgttattgtatttattaatgatatccaaatttattcaagaagcgaagaagatcacgagaaatacttaaggattgtttaaaaatgttgaagaaggagaaattgtatgcaaaatttaagaaatgtgaattttggttggaacaagtagtgtttctcacgcatgtcattacaactcgaagaatagaagttgattcaaaaaaaaaggaggcaattctaaattgggtgaggccaatcattgttgggaaaattcgtagttttttgggtttagccagatattacaggaggttcatcaaagggttctcaaagttatctggaccattaacacagttaactcgtaagggtgcaaaatttgattggattaaaagtgcgagcatagttttgaagagttgaagcagaatcgatgaatgcatcagtgttaaccacaccagaaggggcaaaaggttttgtaatctttaatgatgcatctaagaatggtttgtgatgtgttttgatgcagcaaggcaagttgtggactatgcatcaaggcaattaaaagctatatgagtagaactatcctacccatgacttaaagcttaccgtaatcgtttatgctctaaaaatttggagatactacctacatgggagcaagtgtgacatttatacagaccataagagtctcaagtacattttcactcataaataattgtatgtgagacagaggagatggattgagttagtgaaaactatgactgtaaattccattatcacccaggcaaggcaaatgtggtagcagatgccttaaactggaagacaatgggtcaagcagcgatgttgaccacacaaaagcctttatggaaggagtttgacatagtcttgagattgtcatgttatagcttaattctacagctagaatgacagcattatcagtccaactaacacttgtgatagaattaagagtcatcagaaggggcgaccaatcctttgagtttattaaggttgatatagagatagagaaacgaaaggacttcaccatagctgatgataagtcattgtagcatcagagacagctatgtgtgccagaccacgaggtgttgaaaaaggaaatgtaggaggaggtccactttgctctatattcagggtatccaggaagtcccaaaatgtattgggatctaaaagtagtgttttggtggagaggattaaagaaggacatagccatatgtatgttgaaaggtgttcaatatgctaacaagtgaaaggctgaacatcaacgaccatgaggattactgtagccattagatgttccaaaatagaaatggaaacatgtgatgaaggactttattgtaggtttatcaaaatcagtaaaaggtcagaaggccatttgggttatcattgattgattaaccaagttttctcatttcttatcaatttgcatgaccttttctatggaccaatttgcacagttttatgttaaggaaatggtgaagttgtaagtgtgctagtttcaattgtatcggacagagacctaagattcacattgaacttttggaagagtttatatcgggctattggaactaaattgaactttagtatagctttccatcctcaaacaaatggtcaatctgagcggacaattcaaacattagaggatatgcttcgattgtgtgttttagagtttggtggacattggaaaaagaatccacctttatttagtttgtttataacaatagttatcacaccactatcagcttggcaccctatgaagcattatatggaagaaaatgcagattatgagttcattgcgatgaggttagcgaatgtaagattttgggtctaaaggctattgaacagactgtataggctatcgagaagatttacagtagtactgaaacgactgaagacagatagaaaagctatgcaagataagagaataaagggcttggattttcttgaaggtgacaaagtattccccaacatggagcctatggagggagtattacgttccgataaaaaggaaaagttgcaacaaagattcatttccctaattgaaatcttaaggtgcattggaagtgtagtatattaattggctttaccccctgaatgctcagcagtacgtgatgtatttcacatgtctgtactcaggaagtacgttcgtgatccatgccacatagtgaatcatcaatgaattgagttataacacggtttgagtcatgaaaaagtaccattcgaaattatcaataagaaatttcaagcacttagaaacaaggtgattcctttagtaaaagtgggatgacgtaatcactcagttgaagaagctacttgggagcgagaagtagaaatgcgagacaagtacccacaactcttcgaggaattccaatgtcccaaatttttagtaattagttagatttaaatttaggacatagcactactattaaagtttaatgaccttattaattattggtatagtctaatgagcttattagttattgatcaatagtttgagggcctaaatagaaagttattttggaggttagatgaaatcttgcataaaacatatataaatatgccaattagtctttattaaagatgatttattgaccacatacactattcacaccacatttcaagccaattcattgatttgaccacgtaaataaagaaaaatgatttcaccacatgcattattagggctagatatggtccggttcggttcgattctaggacccgaaatttttgggtatttagtaagtggaaccgtcgggtccaaatataattatgaaactgttcggttcgattttcaggttccatattataattaatttttgtaatatttacaaagctacatgtcacaccccattcatatagataactatccattaacccgtgtgggagtgaaattgatgactcaacctagacatagaatttcacagatttttttcatttgataaaatgacataaactatacctctaaaccaagatcatattgccataatcaacacatatattctgaagttataaacatgtctacatgccatgtcaaaagatatacaatataggatctccaacatacagcacaataggccataagctcaaaatagcagcccaaaaaataaccttacaggtcgtcatccatgtacatcaaattctggaatctcgtaagagctccatagctagccgtgctctctatgtaattccaacctcacctacaatgcaagaactacataagccaatgcttactaagcaaaaatcatgcatgtcatgaatatcaataataacaatatatgccactatgccatttactttaaacatcacgataaagaagcatcatattccaatattcttcaaagtcgactcgaagtcatttcattgggcccttgacctgcccattatgcactggatagagctctatataatatcaatatcaataatcaataatcaaatagccaatatgaaatcgacgtcgacgagtggaccatcctctcgtgaccactagaggcccatcccctaactacctctatgatcccccaagaagtatcccaccgacagcgccaataatcataatatcacaagggcatagtcgagtgatccaccctcccgtgatcaccaaaggcccatcccctgtctacctttgcaatcagccaagaagtatcacccgcgatgccaaaacatatcacataagcatgtcttacatgccttagtgtcctagtagtggtcaataaaatatttataaggaaaactcaatttgaaatcatgtttcgcatgtaggattttcaatcatgatcatatgtcgtgcatgcaaatgaaaatgctcatgaatgacatatttaatgaaaatcactgtcaataggtatcgtaacctcatactcaatgaccataaccatgatatgatatgcaatgaacctcttgtcaaagttatctaaatcttccaatattaccacatcacaattagtaagttcttgcatcgtagttgcaaatgaatttttatttacctttcgcctttgtgtgtgcaagctcctacggagtgtatatcaattctctttttcgctcaatgtcgaaaaatcacctatattaccatctaatattaaagacaatcctccatttaataatcttaacacacacaatcccaaaatacatccattcacgtcaaaacaatttagatgaaatcattatttcaagttaccgatggcatcacaaaataatcccataagtctcgctatttctcgagtccaattatgaacatcaatgtcatccaattgtttaagaccatctagtactcattagaatctattttctagggctaagagataattaatggatatataaaggttaaaatcacattaaaaacacaaatgggcagaatttgttttcagatttctattaccatccaattatttttctaatcctttttcacccccttaactatatccaacgactcccaaatttttactaaaattctataacatgtatttgaaggtaatcacgatctaaatttgtgacaaatgaagtgttttcagcctaaaaaatcgtccctttttcaccacatcaaatcaggcagttttcttttcttgtgactgttttcggtttccattttactagcatgtcaccaatcagattccaggctattagaagaccatttatattcttataaccctcatataaaaacattcatttacatatatacaagttatatcttaagtattatccaaaatcaaagtttaaaccattcaaatctagcaaatcctcatctctgtccagattactttctttcaaattcttgtaattaattacacctattttggcatcataaaatcattaaaaacactccaacctaatcacaagaaagttcatatgttcaagaaattataaaccccttaagaaataatggatacgaacctctgaaccgtgaagtaataaagctgtccagaaattccagcttcctgtttctatttctctttgactctttcatcctctttttcacttggaatcacttagagacgagctaaaggagttaatatattttctaggaggtaaatgagtggtattttagtggttgaggtcgtgcatattacttaaggattaaggatattatgggatgcagccacgtaataagtaggagccggcatcttggctgcaatatttgacttttttaccattagttttgtatccatttatgaattataaaatatatattcatcttatattaagttcttagggagtatacacaagattgatgccttaaggttgaagaaattgagtgttagaagaaactgagtgttaaaatgacaaacatcccaagcacaaggtgttcaagcatgaggtggtcacttatagtataatctgattttatatttatctttgcaggtaaaaatcaagtatccttggcttattttgacatttttacaatccatttcacttgccctaagatcccaaaatatattatagagctaattcctcaaccgttcatataatgacctacgtgattgacacccgatttcaacaatttgcacctcaatatttatgacttcatatgagacatatattattgcattgtgatcatgtcacttcatgcctcatgtctcaaatatggcaattacctatctaaggtttaaggtgacctcgatcaactgactggaaagctggaacctttgtcaatactaattttcgaccttcttgattttccattacttatcaaaccaattcccaacatttagttaaactcattttctatcatagctcaatgtaaaattcacctccttggtcgagaagtcgaagattatcactatgtaaagattttaaagtctcgatgatcgaatgcaccattttaagagaaagtagttaggaaattgatacaaatgacaatgtaattagcatgaaatgcatgaatcatattggccgtatgtacaatgtgaagctcggggtattacactacattaattcaattaatgatatgttcaattttagcttcttacaaaatagtccaattttatgtgtcttttgtgtatctttttgtcaagttcttcatagatttgattgttaaaatcacaggaagaggaagatagcgagctcacaataattaaaagaggtgttgtcgagcttcaattcgatttctccagaatggtagaaacgacataacggtagagtaacagatttggataaaacttagatcaatttgattaagttggttttgaactgaaaattagaaataggaaaatcatatttttgggtttgagctaaattaactaattagtaaatttatttagaaaaaataaaataatttggcttatttaaaaaattagagagatttggttctttagctcttgatctagaactgagaatcgaaccaaactcattggttcttgattcaaatatccattcgggtatttaacttaagaagaatcattcgtatcatttcggttcaatcggttcggttcgggagtcttgtccaaccttatacattgttgacatcaagttttaagttaagtgaattgatttgaccacatgattaaagttattgatttgaccattttcatgaaaatacaccatttatgcattgacggtgcctaacatctagccatatcctttcacttttctgcacacaggcaagaatttacactctaaataggagacaaaccaaacactaaacaacctctcaataattacttacacactctccctctctacctctataactttctctatccacctcctcactttctcttgtcatttgtatattaaatataatcatacacttatacaatcagatgtgaataatcaaccacacatgcgactcaaggatttctttccaataataacttcttttatcatctcgaatgtctggtgaaaaggtaagtgtactttatgtttatggtggctaatatttatgtatgtaatatttctacgactatgttatgtttggttcatgttacgtatgttttattaataatagatcggagtttagtagaactatacatgagaatttagcactatataagtttggtctaatttttgtgtctccctatgcaagttatgaatttttcatagaaataaatatatgaattcattatccattatatctctacttttcagataattgacaattcaaggtggtcggcatggaggtagcttatggtggcaaaagtaacaataatacaattgttacgttgtcaaactattattatttcagttaattttaaatattttaagatattactcatttcaagttaatttattaaactcattacattatttgaatttgggtaagtactttaataatttatatgattgtgctgaatatttttaaaattaattttagtttatgatttaatgacacttgaatcattaaggatttgggttgtcaggcatgaatttttctaaatttgatcgaatgatgtatattgtagtaattttttggtttagcaactaagtgctactatttcaacccatcgagtatatgaatcaacacattactttataatgctaaatttaattaatgtacgctaatattattgagttttaaatgaataagaatcaattaatctaagcatgtaatatatccacaatttataaattaacgcatgctcccaaatatgctacctaacccacacaaacacacaacaaataagaaaatctttgtgaaattaaaaaaaaaatcaattttttacatatataataaagaagtaaaaacacacaatcacacaagtttttttctaagatgcctcctgtatatatatatatatatatatatatatatatatatatatatatatatatatatatatatatatatatatatatataatcggagaaataaaatgaaattaggcaattattttgtgatgatctagtactacgagcatagcccatttaagaaacgagctgtggaagctcaacccatttaaaattatgaacgctaaagccaaaagttaattaaaagcacaacaatttaagagattaagtttaaataaatttgattacaaagatttaatgaataattgggttgcttcaatggtcatctacatggtatttcatatagacacccaagttcggatcaccatgtatatgtttttataaaactttttatataaattatttttttatggtttagaaactcttcaaattcttagttaaagatcaaatttaacaaaactattcctccatttaattttttattaaaaaagaaggttacaagaagatgaatgtcactttttcacaaccgctcctcaaatcctaatttgctcttattttctctcaaagaaatatattttgtgttaagttaagcttaagggaataacaagggtgagaacaaaaaaggatttctacacattttggtcttttatatccaagaaaattcaaggcaggtagatgtgcacgtgtttatttcgttttcaaattatgatttttttcataaatgtttgaataaaatggtatctccaggtacatttcttcggcactacaatagtaattgagttttgtcagaaatccatctacgtgcgacggtatgaatctatattttgataacgaaatgcaccgataatatctattgagtttcaaactcatgggttaatttcctttttacaggttgaatggatttccttggggcgtggatgatagtagaggatgatgcaacatgctttggaggaagccggtgatttaataattttaattcgatcatgaaatgtttatgtttgtttcttttcatatggatttctatggacgtcatatgtggaactattctaagaacttttcttcatgaataggttatgtttaaaagtggatatgacgtaaaaaagaagtgttagtaaattaaagtattgttgtcttttaaaaatttcaattttttgtcttgattttaaaaattcatagctcactggttacttagaatttttagacaaaaccaatggcactggataaccacataggttagctactgaataaacttagaatcttgtcaattcaatgtcagtaggattttatatgtcacttaaagtaaactactctggctagtgttgctgttttctagcttctgccttgatttcaaaaattcataactcgaccgttacttagagtttctggatgaaactaattggatttgataatctcatggattagctactgataaattggaaatcatgtggttttgatgtctgtgaaattttatatgtgattttaagtgaactgcaccggtttacctttcaactgggtcactgctggattttgaaaaatattttaatacatcatataatgtcgacggaatctaattttttactatgtcatattataaaaattttccttattagcattaaaatttgatgatgtttcaaggtcgatagctatgcaaaagaatttattttaacacttaccctatgagatagaaaaagaaaatagcttgtttagttagtgttagcaggattttgggaaatattttaacgcctcatatgtcaccaacggaagccaaattttggatatgtaatattataagatgttcactacttttccttaaagttttatgaaatttcaacattgataactatgcaaatgaggttatttttaaaacttaccgtgtgaaaatgtgaaatcaaaacaggttactctctttcttacttcctaaagtagttcacaaatggaaaactgtcataccttttatttgttttatagatatgtacttgccactaatcaagtaataaaataggcatatgcatggatttgctcgactgttttcttctttattaattaatgcctttagaattatgttaatattatgttactatctaaaaatatattttaatgggaaattcaatggtagttattttaatatatatatatatatatatatatatatatatatatatagttcttaaggaattttttttagcttaagttcttaaattaaattattattttaaataatttctaagtctaaagataaggtacaattgtttgagtgatgctttcataccaacgggtcggggcgttacatatatgtatctttgaaaggtaaaatatgacaaatataagagttaagaagtaatttagaagcaaaaatgtggtgcgcctcccattagttcttgatttatagtctcaagctcgactttgggaagtgatttttcgtggaactttatatatataaggttttggaagtttttcttagctagcctaggttctctttggaccacgtttcacacatcctccaagatcttactttgccatcacaaatatggtatgacttgcctagattatccaattcaaactcaactaagaatacttcgaactcttcattagctttaatcaaaaaatcaataaagtttgaggtttgcatgctaatcccatcttcttttaattccactaattagtttggctcttttatgattaattcctcgatttctacacgttttttctattgcaagtgtacgacatcataacaaagaatataatggatctggattgttgttcccacgatgactataatttaaaacttgatttaccatttctaacttgtttttgatgaatgaaaacaagtatgatttttgtgattgtttcatctaattattattaataattagaatgtatctaaatgcagcaaaacttgaattaggattcaaacatggaataaatattagagatcacaatttcatctattgcatacctttaattcttaaattaagactcacgaatctcatttaatgttcgatcgagttcttttattgcattcaatttatccctctcgtgttctcattgattctatttaactaagttaattccatatctctaagtgaatcgattttagttaaacgcacttattgttctacggatccatgtaatgaacgcaataaataacataagtatctctacattttagactaaattaccgaattttactatatggtctaaatctaaaactcacctctcgattcgtaatagattcacaaagttattgaattactggcatagtaattcaaagcattaaattcacaaataaaatcaacatatgtgtattgaaagaactataatcttgaataaagaaataaattttttcaaatggattgcataatctgtcctaataaaggatttagctactcatgatataggacgaaaaacaataaatattgattgaatacatcatcggattttgaataaagacgaagataagcaggtgaatcttgcagcaatatgttgtttttcccttttgattttctctcctaattctcaagttgtattgcttgttcttcaaagtgtggaacctttctcaagtaccttcctcttgtatttatgctttacctaacatctttcccaaatttgttgactttatgcgcttaaaacgggacaaaaatccccaccctagacgattgcaaatggtgcctaggtgccatgtaagtagcgctacgacattgcgacgtatgctgagtggcaccacggtgcagcctctcgggaaaaaattagtagtgcacatcttttagtatttttgtcgtaactttcttttccaatatccgattgaggtgactcggatggggttgtaaagataacttaaagggtttcaatttgaatgattgtagaatttttgtaatttgaaaatttattaggtcaaaaatgggtttcaatatctggctaaaaatctagatcatatttgtgcgatcaaaaattgatttttgaacatattttgatcacatttcactcctttttgagttcttattgcattcaattgacctctaaaattctcgaatcttcattgcaaggttcaacacgacttttgagtatttacattttagtccccaaactttgaatcttgccttttttttttccaattccacttccattcatagagtttcatctaataaatgaaatatacaataaattagactataattattcaaaagaactattaaatatctatgtttttaagtccaaataagcatataaaatatacttatcaatcaacacaaagttgaaacatttgtttgtcctcaaataaaaccataacctaacttaacaaatacacgaacatgcaaaaggtttttgttagttaacttgctattttgtcacagattggaatcattgtattagattattaaaaagtttcaagatcatattaccaaaatcaatatctacattttcaatgcaaaaactggtgtgtgtgtgtgtgtgtgtgttaaaaattaagtaaaacactttaaattcatgagttgtttgcaattctagacccttgatggtcaaatttttttcttttatcactcataagattcacacacttccaaacttactcttcttaacactttttcccgtgtaaggtctaaggttgaagtcatcctctcaagtttaaagggatatcactaattacaagtcaatacatcaataaatatggattctctaaactttgattgcttcaaattcaaagattcaacaaagctaataatcctttgtcaaagatctatttttctcaaataagtgtttagaactcagtgtgtaaatacataattattatttttcttatcttatgtgtggacttctctttgttaaactatttaaatgacctttatagtgagctctagaccgatgactcccaagttagatgaacatagggcattagatttttagatatccttccagacttaatcacatgaggtataaagtctacaaagagacatctcacaatgaggcagcttttttttgtctcctttcatttttttttccttttctttctccttttttgccatgatttgtgcaatgctcacgattaaacatccattctgaaaaatcaatccctaacttaacattttcacataattttcatcatattggctttagaaaattcacacaagaattttacacaattgaaatcctcattcatatttatatctccatacacaataaaatcattcccaaactattctaaatttggtcgaatgatgtatgttatagcaatttttttgtttgacttctagtttatactatttcaacctattaagtatatgaatcaactcattactttatagtgctaaatttaattcatatacgtaagcagtatcaagttttacatgaataggaatcaagtaatctaagaatgtaacatatacaatattcataaattaacacatacgtcaaaatatattcgtcgacaaggttacccaacccacacaagtacacaataaacaagaaaatctttttgaaatttattaaaaaaattgttcacaatcacacaaggatagtaaaattaaaaactcaatgttttgtccaaccccaaacttaacgtaaacattgacttcaatgtcttaaagtataatctagagcaaaaagggtggggaaaaatagaaaagatactacccaaatttttttttccaataatggaagtaagcttgttagatcgtttcattccattctttcctaagatgcctcccgcttgatatccaagtacatttgaaagataaaagaagacaaatataaaagtcaagaagcaatttaaaagcaataatatggcgtgtgtggtaactattttttttaactactctggagctctgagagatgtggcacatatattttctattgtttttcactcaaatatattattttcttttaatgaacttaacatagatatgatgaccctaatattgaaacagaaacatgtttaaactaatgcactttaatagattgtatgcaatgcaaacacaaagagcataataaataaaagtgtaagaaattgggtttgcttcccattagttcttgatttatagtctcgagctccactttaggcaatgatttttcatagaacattgaataagtctttggaggtcctgcttagcttacgtagattgtatttgcaccacgttacacacatctccacaatcttactttgccatcttgtatatggtatgactcgcctagattatccaattcaaattcatctaacaatacttcgatctcttcattgactttaatcacaaaatcaataaagttggaggtttgcatgctaattccatcttatttaatgccacaaattcaatttctacacattttttctattgcaagtgtatggacctttaagtccagggtatcgttcccataaggactacagtttaattattgatttactatttctaatttctatttgatgaatgaaaaccagtatgatttttgtgactgtttgatctaacaactaataataattagaatgtatctaaatgcaacaaaacttgaattaaggtttcaaatatggaattaatattagggctcacaatttcatctattcattacctttaattcttaaatcaagattcacatatctaatgtagtgttcgatcatcgtattaaatttacctctctcactttctcattgaacctaattaactaattcaattccatatctatatgtaaatcaatcttagctaaatgtaattattgttctatgaatccatgtaatgatcgtaataacaagcataaatatctctgtgttttatactaaattaccatatttcaccgtgtgatctaaatctaagaatcacctctcaatttgcaatagattcataaaatcgttgaattattggccaagtaattcaaagcattaaactcttaaataaaatcgatatgtgtgctttgaagtctagaatcttaaataaaagaaataacaggtctcaaatagattacattgtttatcctaataaaggatctagctactcatgatgaaggaagaaaaacaataaatattcattgggtacatcaccagactttgaataaaatgaagataagtggatgaatcttgtaccatgatgatcttcttaccctaagcgatcttcaaaaccttgatttcttgatgtttttctccttttatttgctttcctaattctcaagttgtattgcttatatttcaaagtgtggaacctttctcaagtgcctctcctcttgtatttgtacttcccttaacgttttctcccaaaattggagactttattcgctttaaacgaccaaaaatcaataccctagatgacaattggcatcgcttagcagccatatgagtggcatcacgatgctgcaacattatgttgggtggcaacgtggtgccgcatctcgaaaaaaattcaacggtgcacattttttagtatttttatcataactttctctctcgataccgatggaggcaatttaaattgagttgtaaatataactcaaaaagattaaaattttactagaaatagattgtttccaatttagacgtttactaggtcataaataggtctcaatttttggctaaaaattttgaacttgtatgattgaaaaaatttatttgtgaacatattttgatcatatttcacattttcttgacttctaactacatccaatttacccctagcattctcaaatcattatcatgaccttcaacacaacttttaaatatttacactttagtccctaaactttgaatcttgcatttttttgctaattttcgcttctttctttcaattacacgtccattcattgagtttcacctaataaacgaaatatacaataaattagactgtaattgtttgaaagaactattaaacgtctatatttttaggtccaaagaatcgtataaatacacttaccacgaacaatttaattcctttgctaaattaatcagtttagttaattaatatgagaatcgttatgaaactcaagtactcgataaatactaggacgtttaatcccatttagtattaattcctctatttagacacacacattcggatataaagatcaatgttccttattcatttaataatctcactcaagtacaactaaatatatcatcacaggtaacctttctatatcgctatgaaaggttcgaacatacgaagatgcattaaaatcacgagaacgtcaaaaagtattcgtaagaatatacccgtacatctctattccctatcaaactttataatcattgttaatacgtgctgaattcctattcattctcttgaatatcaatagaaattcgaagacaattcaattagtggctaattaattcaaaagaattaataccaaagtatggaatcaaatatcaaaacttcaaaattaaggtttgttggaataaattctgtaagcgtatgagattgttgataagtgataatgcgatgagaaagtatcatctcacaggaaatacttcttaaatgaattgtactagttcttttaataaatttgaatgttgtaacacaagagatgaataatttattatatattattctacaaattatctaaatgcgttggtttgtaatactagacttatgaatccacctattgattttctatttccaatttttgacttatgtaatttagtgtgatttatgcattcattacaatcgatgattctttattttctatctctttcaaagtaagttaaacatattctaaatacaactcgatcatattcctatcccgaattcatatgtgaataatacattaatgtatacgattatttacatgattgcacataccatacatcttattcctaacatctactatccttgtattaaccttgtagtgttctaaatttatcatgaaactccttgcacaattacaagaaattaattatctaattgatgatcaaaaactcaaataatgaaaattcataaaagattaatcaagaacatatataaaggagaatttagcatagcatgaaacgtatataattataaaaaaaattcttttgatttatacacttattcgaacaaaaaatatagatatttaatagttcatttgattaattatagcttaatttattgtatattttatttattaggcaaaacttgataattggaagctaaattgaaataaataagcaaaaaatggcgaaacctaacgttcatggaccaaattgtaaatatccaacgattgttttgtatcaaaaaatgataattagtgattgctagaagtcaattgaatgcaattagaatttaaaaagaagtgaaataggttcaaaatattttcacaaattaattttcaactgcacaaatagtattcccgatttttatctagagatttagacccatttttgacatattaaatgtttgaattgaaaaaaaatactatttctagaataattgtagtcctttgcattatctttccaaaacactttaaatcagctcaatcaaatattggatgagaaagttaagacaaatttattgatggttacgtgttgacataatcatgcacgatgcatagacaacttttcttattcgattggaactcaatttggatgtttttttggcctattttcaccatctatatatacaaaacatgggtagctattgaaggatacctctcatacattattttcatcctttattagaaaaaaatggagaccatttcatagatcttttaagggaattaagaggccattgcaacatttcaattctatgaagattcaatcttgatcattgaacaaagaagagaagaaacagttggagattcatcaagaaaccattgcagaagttcaagatctcaaaattcttcattcttttaatttatccgtaattcaggttatttttttccaattaattacgatttcttgtgattttgaaatgttaggatagggttttaattattaagaaattgatgaaactttgttatgatattttaataaaaattcaataatttgatgccaaatatatgtttattcttagatgagcgttataggatttcataaaattttaattacttgaccactaattggattggttgtgaatttcattgattttgaaagaaacaataggatagaaagtacttcataacagtcattgtaaagttcgataaagaatagagataatgctatgcttctttgcatgatttatatatatgttctagcatctttaatatatgctttcatgtttgcatctttcatagagatataggatggtcacataagataatagatttagttgacatcaagagaggcttttaatcaactttagaatattgatcaataagagtgcgttgttttattcaattgcattgaaacgaatttaataggaaaattcgaggtcatagtaaccttctcatctaaatttacagcagcttataatttgctcacaatatttgttagtttaattagaaaaagtagtataaacaattcaaataaaattggctattcaattaaagttgaaattcattgaccgttggttaagtacgtagtccttgttggaacaatatctcattcatcaatctattacttgttctgataccgtatacttgtgaaaaattaagtgatcaaattttaggtattgttgtcaaggactatagaatttaattattgcgtgcaaatttcgagacactatgatcttgttccatttgatctgaagattgatcaaacatttaggttgagaagaaaataacagttaaaagcacaccaaaaatagaaagccgaatcaatggcagaaaaatatacaaaataaattgcagttcaatgggagaccaacttaccatccaaatgctcatatcttgagttttatcttattttattattttttatatgtgtgtgcgacaattgaatatttatgggtttctagtgatacaattcaattatgactcttcctatacaatttgagaaatgaaatcactacatttctcaatttgattcaatatgttattcaaaggtttgggaattgtacaaaggcttgcttcatcagtgtccacaacatggtttgtagaaatagctccaagtccagtatatttacattgggttaaatctaacaagcagggctaacgatgactttgctcgtgatagatcaataacaaaaaggacaacggatcaagtccttcaaattatggaagatctagcgtacaccagtgcactaatgccaacaaaaagattatgtggaaagaggactatagggatacacaaggttgatacattgatagttatttcaaaatagctagaagcactggctaatctctcttagaataataaccagtcctctcaaggtttaccatatcaaaatataccattacatttttggtagtaaaaaaaagcccttatgggaaaaagtgtttaacaaaatggtagcatcatctactaaaacatttgccaagatggctcaagcatcaactaagtttatacaacaggttgtgaaaaattttcaagttcgaaggattgctatatagaatttggaaaatcaaatagggcaaatagccaaagcactttcagaatgacagtacttacccaaagctaagttaaactgaaataaataccaaacaataggtaacgatattaagtgttgtggaaaatgagctagttgaggcagctactacttggagtgaggttcacctaccaaaaactacagttaagagataagtggtaataaacgaaaaggtaccttctacacatgaggaacaagtgggtaaatctgaacaattagcaaaaatagttctaaattagaagtcaaataatccacaagttaagacaatcgttcctatcaagacacatgtgcctcatgtctcatttcattagagattatagaaaatgaagctcaaagaacagtttgcaatgttctttgacatatttaagaagcttcatgtcaacatcccactaatttaagcatatctccaatactaaattatgcaaagcttttgaatgagatcttaccaaagaaaaaacgctcattaaatttgagaccatcaagttaaatgtagagtatagtaccatctgacaaaacaagttaccttttgaactaaaagatccagtgagtattaaatacattgttcaataggaaataattttactttcacttgtttatgtgatttcggagcaagtataaatttaacgcctttttctgtttacaaaaatattgtttagaaaagctaaaagaacacaactaacttcatttaattggtgaacagatcaatcaaatacccttgtagagtggttgagaacgtgctcataaaggagataagttcatattcccaatagatttcattttcgcaataaagacacagaagaaccaagagatgcatcaccattattcttgagtcaatctttcctatcaacaagttgggttatcacagattttgaataggcaaatcgacctttagagtggatgatgagcaggaaaagtttaaaatctataccgctattaagaaaccatcccatgaagagaatagcagaaatgttaaggaggtaaaagtgaaagagtatttaaagtgccaaaaaaaattgagttggtgttacaattgggaacctcatggatgaaaagaagagctcttcaagcatgaagaatcaaacatggggttggtaatgctaaatactttgatcaaagctttgccgatgaagtccactttcaaccaccatgattaacgcaacaaagtctagctaaaaactttaaattatgagcttatcgggaggcaacccaatttctgaccttttatttattatgctttatgtattttcattgcatgtagtttgataatttgcattagtttttggcatatttttatatatcatgttcacatcaagcctatattaaggtaacaattttatttgagtcaaaaatagtaaaataatcacgtggcacattttacaaagctccagaggcataaataaaactagttatcatacataccaaattacaaattttatactatttcctcacttttatagtgatatttttgtttcattttttcaaaggtacagggatatcgatcaggatgaaacttaacaaattaaagaatgaaatgaattgatccaacaagtcgcctcaaatataaaaaaaaaaaaaaaaaaaaaaaatttgataaacaccatattcctttcaagacattaagaatactgccaactttaagtttgggttttattatataagagaaaaatagaagaaattgaaaaaattaaaaagtttcaaaaataccttttcaatttacttgtttgtgtgagttaggtagccttgtgcatagataaatatatttggaattatgtgttaatttatgaactatgaatatgttacacggttaattgattttcatcctaaattttagcactgtgaagtaatgagttgattcatatgcttgatcagttgaaatagttgaatttagatgctaaatcaaaataataatgataataataataataatatacatccttagaccaatttttgtatattttgagagtgattgaacttatatagaaagatattgatatgaatgaagattccgtgtgtgtaaatccttctatggattgtctaggaccaataagataaaaattgtatgaaaatcttaagttaagggtctagttttgagaacaagtgttcaatatggggcattacactaatcatggcaaaaaaagttgcctcttggtgcaacgtttctttgtagctttgtagctcgagtaattatttctgcaaaggtgtccaaaatctgttgccctatagtcacctgactagggaatcatcggccagaagttcactacaaaggtcatttagaacctttaatggagagaagtttgcagaaaagatgaatgagaaaaaagtaaaattatgtgccacatgccttgatcaagccttaaacacttctctgagataatgacttttaataaaaggttattggcctagtcgagtcttgagaaatccttcttcattgatatattgacttgcaattagtgacatctatctaaactagagatgatgagaagttagtataaaaaattaacttagatcaaaccatggaaaaagagtgaaaaaaaataaatttggggtgtataaatcttacgagtaaatgaaggataaatttgaccatcaatggttaggaattgaaacaacttgtgaaatcatgatattttacttaattcttcacaagcacatttcagttttgcattgaaaaagttgatatttattttaatgttgttaccttgaagttggttatgaatttaatacaatgattctaatattgagataaaatgaaaggttatctaaccaaaattttattgcatattcatttgttgaattagattatggttttgtttgagaactagcaaacgtttaagtttggggacatttgtatccggttcaaaaaatatagatatttaatagtccttttgattaattattgtatatttcatttattagtaaaactcaatgattgtaagctaaattaaaagaaagaagcaaaattggcgcaaaagagcgaaattcaaagtttgaggaccaaatttcaaatatttaatgattgatttgaatcataaaatgatattaagattaaggagtcaaatggatgcaattaaaagtaaaaaggagagaaatatgatcaaaatattgtcacagatcaatttccaactgcacaagtcatgctctaaaattttatccggaccattttttacataataaatgttcgaattgaaaaaattctatttctaaaacaattgtagccttttaagttagattttcgatgcaatatgaaacaactcaattgcatatcggatgaggagtttttaacaaaattcttgacaactacgtagagacataagcattctcgactcgaatgaatctttccttgttcgattgaaactcctttgaaacccaatttggacgtgatacctggcctaagttcactctctgtatatacaaaacatgcccaaccatcgaagaatacctcttcatgaatatattttatacacttatttgggctttaaaatattgacgtttcattattcttttgataaattatacactaatcttgtgtatattttgtctattaggtgaaactcaatgaatggaaactcgatgaatggaagataaatcgaaagaaagaaacaaaaaatggagaaaacggtgaaaagcaaaatatgggaactaaaatgcaaacattcagtagttgattcggagcatgaacaaaagattgaaaatattacaagttcaattggatacaattagaagttaaaggttagaaattgcaagaaaaagggcttaaaaaatcaggaaatgaattcgagaaccaaaatgcaaagcttgaaagaaaatataattggttagctgcccaagttgccccgcttgaaaaatcaaaagcaagggcttaaagttttgcctgggcaacagcctagcaaattaggcatgtctctctcatttttttttcctccaaaattctacatggaaaccactttcttgtgcgattttgatgtagctctcatatgcatctcatacactaaaattcatcaattgacattatcaaagagaagccaatccattgttcttgtgagagtaaaatgcaattgtaagaattcaagaattggatatttaaatcatgatttttggagaacaaaaagaggaataattaggatttcatcaataaacaattggagaaattcagcaatataaaattcatcatcttctacttcatcaacttgaaatctcgattatgttcttttcaattaaacatgttttcttgtaattttgtaatgccagccgaggttttcaagtactaagatgtagatgaaccattattatgatattttaatataaattcaatagtttgatgcccaatatgtgttaatttttggatgaatgttataggatgtaataaattttcaattgattgatcactaattcgattgtttatgaattttattagttttgagagaaatgataagatagaaatcacattataacaaccattataaagtccggtatgggatagagatataatgtctgctttgcatgatttctatagattttctagcatttttaatgcatactttcatgtttgtatccttcatagaaatatgggaaggtcaattgagatgatatatttaattgacattgagatatgcttttaattaacgtaggaacattgatcaacaagaaaaatgttcatactgtcatgtaattgagttatactaaaattaattaataaggccattcaaaatcttagtatcgtctaatctgtatttacaaatgcttaataaattgctgactagaaaattagtttaattagataattcattataaaatgattcaaacacattttactattcgattagggttatggttaattgaatctagtttatatatatatagtcctcgtgggaatgatactttactcttcactttattatttggttgcaatattgtacactcgcggaaagtcgaacaaccaatttttttggcaccgccaatgaggactattgcatttaattagttttttttttttaggttttcattgctatattggtttaatcatgtattagaaaaaatacgctgtttcttctctttcttttttagaatctcgtatgtaaagtttcgaagcacggtgatcttgctcaatttgatctgaaaattgaacgaacattcagcttgagaagaaaaaatagaagaagtacaacaataaaaacaagcaaatctaatgacaaaaaacatacaaaatcaagtcaacattgggatgaatgaaattgtagcacgtcaggttgtagctacgggagatgagagtgagagactgttaggggaatacatgattcgaccatggtaagaagtaaatctagtatagcttatccagcatttgggcaagctaattccatttacaaatgaacttgatcaacatgttccagtatgcactgtaattcttcaagaaagccactaaaaattcaaatgatcacatctctaggttttagatatgtaccttgtaagtgttatgccctaggtccaatcaaccttagacataaatacttttaatatataattaatacaatttaatggcaaatctattatttaattaatatacaattaaattgaacaatagagtccgtagattcaaatcttcgtaatttgttaatcacaaggagttgtgattgttatgtacaaattacatatgattgaatcttaaatcgtctgtggtcataagtaataacgagatacagatattgttattatggatagaccatcaagtgtgacatttcttatttgtgaagtacgtagctgatctcacaagctaaagtatggtgacacttgaatgaacacgtggatattttgttatagaacaaaacattagagacctgcctagagattccacatggataactatcggagtgttagtggttaatctctaacgttcgttagtgggattggtactttgacttgagatcgtcatagtaccttatatgaggatagtcatgctttgatggtgttggatgttgctctgccaagggccgctaatatgtcgtcgttcgggcatttcaagaatcgtatgaaggttgtaaatgaccaatcactcttagatagtaagggattatgatctgcattcaattaagtcaacaacgaaatccttggccaaggagtactcataagttgaaaaggaggtttttttacttatattgacttaatagtggagtgaaagatatgattaataatcgagattgacacacttccatatttcataattgatcggatcatattgacgaagagattatagtttcacggtaaacaaacgagtttgattttgtcataccacgtgatatttctcatcacatgtattgccctgatacattgctagatgtcaatctgggacggcgagtgtgaattgttgataaattaaaattgtgttttaatttattaattttgattagatcacaataatatttcacgtcgttagacattgtgataggaaacctgatgggtcgcacacaaaagagaattggaatattgtaatttttcaattaattaatttaacaatcgttggataaattaattaattgggttaattatttatacacccgaattaattaattggattaattaattcacgaaccgaatttaattaaatattggactgaatcaactcaagcccgtttaggcttatataaatacatggctagggttttcaatttgtagagaattcattattcttactagcacaagaagaaaatcctaatcgtgcaatcttgttctctatgtggatcatcgttgaaggctggataattggacagctgtgggagatagatccaaattgttggaacaaagataaggaaaaggagtttgcagatctaaaaaaggcacaacctctatcacattttctatctaaacacaaagctaattcttggtagaaattgaaaattgtttgaatttttcactgcgcacgttaagtagattcccaacatacccgtcaactaaatattcaggagtttttagtgaataatcacattgagagatttagctaggaaaggttggacacattctcacctcacagtatcactacatgggatagtttgagccaaaaattcttagacaaatactttccaccaaagaggattgctaggttgagagatgaatcactacattctcttaacttgatttagagtacgagttatgggaaagatataaaggtctgctacgacaatgtctacaacaaggtctgcaaaaatggctccaactttagtactttcatattgggctaaatctgggtagtagggctaatgttgactcaccaatgatgggtcaattacaaagtggctacaggttgggattatctaataatggaagatctagcatatgccagttcattatggccaattgagagatcaagtggaaaaagagatgtatagatgcacgagatttacacattgatagctattttaatacagctagcagcattaactaaaagggtagatggttggacaatcaatcaagtagatgggttgatttgattgaagatcacatatgagcaattggatgcaactggaggtcaaaggattgaaatataggaaaatactttcacaactcagttttcaatcggaaaagttatgcctcaaaatcttcaaccttagattgagacctacttttgggtagcaaacattcaaattagaaaatttatagttttaggagatttgtagccctgtgagttatcttccctgtgcaatttaaataaccccaattggatatcaggaaagaaagttaggatgaaaataccaaaggctgcttagggactaaacaatgtaaactgacacgcataagacctgttttcaccaactcaagggcaagaatgttgtaagtcgtacgtagggcttagatgcttgtgcgcacgcaatgttaattcttggtcaaagctagcaatttttgtctgtgacttaaattccttttcaattcaaattcttcacgcgtttaactttatttttggtttcttataaacacaaaacttggtcaaacattgagaaactctctctagtctctagatacataataatatcataaagttcatcaagaacaagcagttagttactatattttaagggaggagatcaaactttagcaaggaattgaagtcaattacatcaagatttttaaaaattcaaacttagaattaaagatcaagatttcttgcattatttcatgattcgggtgatatttatcattatttttctgtaatttatttaaaaacatgcaaggctagatttgttttgtattgaatgaagatgaaaccgattgtttatttattttaattcaagattagcattttagtgtttttgcacttcttgattaatttcacataactattgcattatttaattatttaaccatcatttagacaattagttgcttgttgtagtactaagaggctcacaataagtttagaatgcagcaaaattaacataaatgcaataaatgttaggaatgatcatttatcatgtgtataattgtatagataatctaaaattaaatgtattctattcattcaaattaggactatgaatatattcgggtcacgactagagtagatttgatttgtcttgaaaagaaagtaaaatatattagctttattcattgtcaagaatgcacgaatatgattagattacaaatcatgaattgaaatagataacaataggtggattcaaattccgataatatcatccataatttgataaaaatcaaacttttacaactttcttagattaattaagtatacatgaaatcaaactctcttttgtgttatatatttgaattacatacaaaactagtaaacatgaactgaatttgcttcctagttgatgatactcttaactcattaattatattacatgtcaatgatatcatatgcttgtgggattttatcaaacactagccaactaggaatcaagtacgcatttcatgaatttatgtgagagtgttataaatttgagttaaacaatgagagcataattaatttaataaaaatccatattattctacatttattaattccttaacattcgttacttatagtttttaaataatgagaaactatatgaatttcagaggaatattggatgccaacaaattgacccaaccaattttttttgattgacaatgcaatacgagaattgttcttaaacatgaaaaaattggttatgtccttaagcactcctttcaagagacatcaattgaggactcgactgagaaagatgaggctatttataataaacaagtgatgacgataatactatagcatgtgtgatgcctgcagttatgccaactaagttgcaaaagcaaaatgagagtatagatgctattatcatgatttttcatttgaatgagttgtataatgaacaatcacctatggaaagaaatggaattccaagcaactaagtagatacaaaaaggcagaaggatcttcaatcagtactcataaattgaagatgattggctatattgagaagttgtctcaattgggttcaattatagacagttaaaaaagtatcgacttggttctacagtctctatcagagagctattcataattaattataaattttaatatgcataagctcgattgcaccatctttgagttgttgaacttgcttaactattaagcctagcatcaaagctagtagtaggcaagtcttggccattggtttctctaagggaactaagagatagtgtaaaagaggctttcaaaaagttctaaagtggctaagtcaatcaaagaaaacagggacattcaagtctggtgacccttgatgtcattgtggaatgaaaggttattcaaagaaaaactacaaggtttatgtttgcttcattagcttcttggtattagatactagatatggatcttatatttacataaatatgtagaaactaaaataaagtagacaactacagaaggaaaagttgacccacaagttgaaaatagagcaaagggtgctacattatctaaagaaacatacttcttgttattttcttcaagctcaatattagaattagagaaatattgttttgttcccacctttacgaagaatattaattgaattagtgcttggatataaattactaattaatgttaaggacagactttgttccttttatttagatgaggtcttttatggttgtagtacattacaaaatagcatttacattcttgatgccgagtcttctattatgagtatagaaaataaaaagcataaaagtgataacctaaataatacctatatttggcagtgtagactaggctataaatgagatattaaggagaaagggttgtacaattattgggcctaatacatattgatgcataggacccatgtcaatcgctgctaaaggtggtttcttttgctttatcacatttactggtatggttatatatacttgaagaagcatgaagcactgaaaagttcaaaaaaatcaagctaaaagtagataaacaaattggtaaagatattctaacattaagatcccatcaaggtggagaatatcttaaaatgattgtttttagattgtctaaaagagaataggattctcttgcagtggattctgccacataccccataaataatagcatatctcaacggaggaattacacactattagatacagcgatcaatgataagccatgcacacctccttaaatcattttgatttcatgtaataatttcagcgtgatatactcaaaattgagtcccatctgagtcggttgacaaaactttctacgatttatagagaggtagaaaacctagcttgtcttatactaaagtttgtcgctgtcacgcttatttcagcacactgaatcggaatagtttgaggccaaattcgataaatacatatttgtaggatatgtaaaagagacaattgaaaatcatttctataatttcattgagaagaaatattcattcaagacatgttatcttttagaaaaagagttcattttagaagaagacaatggagaaaattaaaacttggatgagttcaagaatctgtataaatagttgaccaaataaatgaacttgagtcggatcccacacttgttgggggtaaattcttgatcaagaagtagagactcctaaggatacgtcaactctacataaatctagtagaatcatttgagctcttaaaaggtatgaattcaaatatacgaatcaaggatgatgaatctactaattatgtagaagtaaagtcaaacattgactcaaacaaaggtaggaggccatggaatccaagatgaactcgatatatgtaaaataatggtgggaccttggtcgattcacttgattggagcttacaaggaagatattgacatggatggaaacgtccatacatacgaagtaagcctagtagcaaaatattataagtaaagacaatgagttgactttaatgaaacctttttccatgtagctatgctttagtctattcgaatttcgcttacaatagctacatatcatgactatgagatttgtcaaatggatgtcaaaactatattccttaatggaaacttgtaagaggatatgtacataaggcaactcaaaggttttgaatccaatgatgctaacaagatatacaagcttgattgatccatatatagattaaagtaagcctctaggagctaaaatcttcaatttgatgagacaatcaaaaggtataatttcatcaaaaatgaagaaaaattctatgtttacaagaataaaagtgggagcgctatagtattcttgatattatttatagatggcatattataaataggaaatgatgtgcctatgcttcaatcgatgaaattgcggttgtcgaaattttttcatgaatgatctgggataagcaacttatattttaggaatcaagatctattgagatagatctagatgatttcttgacttatccaaatctatatgtaaaatctaaagaagattttatacggaataacaaagcagttaggtgaaaaggttcccagtaggagataatcactgatttaataacagaagtctaatacatcattgcttcgaaaaatagcaaaagttatggtttggatcaagaaattcattaatgaacttggagtagttctaaacattgttgatcacatatgcttgtattgtgataacaatgaagccatcatgcaagcaaaagaactaagatctcatcaataatccaaacatccattaagatggtattatttcattagatagatcatacaaaggcatgaagtaaagaaagaacgaattaccacaagtgataatattgcaaatccattaataatgagtttttattgcataaacattatcgtcatgtagactattatggtataaaatagataattgattggatctagtgcaaatgaaatttgtaagttggaagtgttatgccctagatccaatcgattttcgatatgaaaacttttaatatgattaatgcattattattatggtcgatctattatttaattaaattactattctaataaatcatattaatagattccataaattcaaatcttagaaattttttaaattaaagccaattgtgatagtaaaaaaataagttacgtatgattgaattttaaattatacgtggttaagaataataacgagatacgaatataattactacaattagaacatcatgtgtggtacttctcacttatgaagtgcgtagttgatcttacgaactaaaatatagtggtatttaaatgaacatgtggatgtttagtcataagaacaaaacattggaggcttgcctaagagattccgcatggatagctatcttcgcgttagtagttaatctctaatgttagtgggataaaagttatgattagaccaaatcaagtataatggatggattgattaataatctgttagggtttgagaaatcaaaaaatacttcgatcgtaatctcgctagcacgagaaaggagaaccttaattttgccatttttgttcccttgtatgaattaccatggaagactggataattggatgattgtgatgtgtattttgtggtattcatgttccaatattgtcaaagaatttcgcagaattaactaaaggtataatttttattacagcttttatctaaacgtaaagaagatcatcaataagaattgaaattgtttaaattccactatgtatgattatgtaaattcccaacattatctctaatgtccttcatgacattgggtcatgttactccactattgagaatctattaacgttgatgctaagtgctatgactatgagaatagtgatgcagcatctgattatcgtaaaagttgtggtgttactgattatactttaattttaataatcttagttacctgttattgtgttttatgatctctcagatgttactaactcatgaaagattaataacattatttaatttgtataaaattatctttacaacaagatagattcttttgtcgcattaaattaaagatttttgggtacccttgcttacacccttattcccttttgctattgaaattgccttctagttattatcctatctagagcaatttttattaataagagtttcatattaattatttttatgcaagataattaacttggagtgatcggtatcctatggttaacaaatattaacctttttaacatatcatatccacaaatttagaaactaaaacaaggataaccacgatctcattacattgagtgaaggaatcactaaagtctgatagaaataatgctagtgttcatagaaatcccacaagtatatgggttcattgtacaagtaataattgtgatgggagagttatcgtcccacagggaataaggtctaattctagtataattgatatatttaaattcgtgtttgtaatcaatagttgatttgcgaatagctaatgaggttttgtaactaaaacttataaaatcgatgaaagtttggctcaaaaaatcaaatgagtgaacgtattatattttctacttcactgatcaattcttggttctaattctcaacaagtgataattatctcaattcatgcaattgtgacgatcgataattctacttttatttattattatttttcaagatataataaacctatgattactacaagatgatcctattcctagtccaaattcatatggtaaacttgcattgacatttaggatcatcacacatgatcatattatttctaacatttattgtccgtgtgttccaataacagtgttttgcctaccttgagttttccaacactgcgaataagcaacttattatcctaatggcgcgcagacattaaaacaatgtaaatatgcatattaatggaatcacaatgcaagaatcaagataaaaacataaggtctcgaattaaaaactaagaatcaaatagttttgtcatccatccaatacaaaggaatttagcctagtatattaaagtgagaaatacatgaaaaataaaataaagtcatcactcgaatcattaactgtgaagaaaatttggaaatcttcaattaatgccttcaaatctagaccaaagcaatgaattatttgttcttcaatgtatattctctctatttctccaaaagtcggcttacaatttgatgatttaggtctggacgtgcatatcttattcatatggtaccaaggagactccttaccaaaaaaaaataaggaaacctaaatttttcccaagtttaacattgaggcgcacgccttaccaaggcactccgttttggccttgaggacgtgcctcacctgtaggcgacgatgtgccttgggttgtttcttggggctaagtttacaactttgtcatttaactttctccaaggtctttttttgtctttcttcactttttttcttgtaccattcacttattcttcattctaatagagttcttgcatctcgaatcttcgttttgcattgtgcctaacatgtgtgttgttgcattttagtccccaaactttgtatttgatgcaaattagcccttttcttgcttattctccttctcccgcatctttcatcgattgttacctacaaacaatatatacatagaatcagatcttaaatagaagcattagaatttgatgagaatttcactaaaatgatcctgagggtagcaacaattcaaaaaggtactatggggaatctaaagaagaaggagaggaaaagctcaaaagaaataacaaagctctcactatccgattgaatgagaaataaggcatcaagatcatgaaaaaagagtaaccaagtcggcaataatttagccttaaaaggtatagaaatcaatgtaattcgaaatctataatttctttgattgaattttttatacataaaaatgaaaccatacgcccttagatgacataatagtcatatggaagatgatagccggagaaaattttgatcacatgcttttagacgatggaaacgtgataaatgtcttgtttgaaagaacatttattaaatactaacctattattcatggatacctattttgaagcctcgcaatttcatcaaaggaggtctagcagctccagccgcattgacgatagactttcattgtgacttagattacacgatccctcacggataggccactctgtttgtgaatttaggacaggtgcctcgagtatattaaggatatatgaatttcgacataaagtgcacttacgatgatatccatggatgacctactacgaagcaagagaatatcacaatatgtcttcaccagttatgcatgaaattccccaccaatataggaaagattgtataaattatgatcaaaaagttttacgagaaattcattttagtaatctaagagagacagccctacgagttcccatggaaaatgtgatagcaatagtggaagcaggtaaatttggggaaaagtttgaagtagataattcaattgacccttgcattatcgattgtatttttgaaggtgtagtggttgaagaactagtgagttttcttgtaagtaaagaggacacaaataaagttttaaagactagcatacgttgagcctatgaaaagcctactaaaaaacttcttaaaaatgaattttgatgttcttataaatgcaggccacttatcaaaataatagaagtacatattgacaacatgctcgttaaaagcctttgggctaaaaatcaccaaaaaaaaaaaattctagaagaagcctttaataaactcgactttacatgtgtataaaatgaaatttgactacgcaacttagatatttgagtgcaatttttttttttttgttgaaaaagttacattgaataaacaccctctccgtaaatccatgcatatccacatggtaacttgtaatgttcatataatatatcaagaaaaatacactctattcaaacatgttactttgaggttacaaaagtgttaccattctatttcacaactcatatatacgcaacacgagtttccaaaatatagtaaaaagactataagaataaaatgacgaatccccaacataaccttacaaatcatcatccatgtgcatcaaccctcgaaaatctgtaaaagcttcacatcccgccacgtcttctatgcaagaactacatatgctaatgctcaataagtaaaaatcacgcatgccataaatatgaatgtatgtccacaaattttttctgccataaatattatttgattgaatagttaacccaatcccttgtagtttgaagaaaagaaaaaaagatgagacgagagataagaaatccaatgttttactataattttaaataacggtcccggattcaagttgattctatttcacctcttcctaaaagaaagacaatcaaataattttcaatcatggtccttacaaattggatcatccatataatatacaaataataataataataataataataataataataataaaatattgtggctgtttgatatattttttttttttaatttttaatatgacctgaattccaaagacgatttcattagctatcttacaaccagactcctcttttttcattccagtttctccacaatagtgaaccctagttagatttaggcatgctatactttttagttattgggagaatttaaatgttagaaaaaaattttgaaagatgtcaaatgaattagaataaacaaataatcttggtagctacgccacccagagaatttaaagaacttaaacttctgcagaataccaatcttaccaaggttgcatgtcttcattcaacgtacttaaggtattcgatgtaagtctttctcccatttaaaccttacccttctaaggctaggccatcctaacgtgttatttaatggatgggccttgatacagtgctggaactgctaactatgatcaatatgctaattatagatatgatgccaaaaatagatctattttatatcacccttcaatttgaattaacaaaagtaatatgtcattgtataatatgggttccaaatatttcatgatctggatattaatgactcgaatctctctcaattcaaaaatcctggttttgaattgatatcattttacttattcctcttatattgtattcatttatcctaaaaatttcatttcaatagaggtttgcccattttttatgtccgtaacttactagagcctcaaggaaataaagagaagatgtgtatgaacaacatatcaagcaaatccttgtaataattcttcggaagatgatcctattgcaggaatagccttaggtacgccttttacaattttcatcatccaatggaaatggctctcatcttgtgacttggacgaaaggtttctctgtaaagaaagggaataaaaatgtgtgcattaagaacgggcggatgtatagagaagatagtttttattcaactccctcaaagtggaatccattccaaacatatatgctatagttccttatcaaaatgagggttatctgctaagcactacgatagagagtgtatgaatatcttcatggtagacttgattttacaaaagacgataagaacatgaactttcagccgtttatgcgttggagagatcatttctaattttgtgtcgaagcaaattataaatcacaattgaagtagatgaaattaaagggtattactttaatgctacaacagataaatgggtcttgcaatcaagcttcattctacttttgcacaagagggccaatctccatttagcccgaggaaacctttgcacacttctattaacttttgaaggttgagatgctcaagcactgctccttaagagcaacgtatctacaaatttcaccatatcggcttgtaatataagcattggatcacctttcttatctcaaataagaagggtaatgggaagaatacattaaaaatcatgatcaattcctttttcaaatcctgctgcagctgtgacccatggaaatgctagacttaataatttattcagtaaactactaggcgctcatgtagctaatgcctgattaacctattgtaggttgaaacgctcactaatgagtatttcattttcagaattgtaacctttctatgatataaaagccagcaatacattcttcttcaatataagtttgccaccaacctaaaattgaagatatagaataagaattttataagttttataggtcattgctcagggtttgacaagaactatataagttcgtcactaacactgatagaggtttcaagatacagaacaagaactttataagtttgtactaacactaattcaatattctgtatgtcattgaacattgtttgacaaaagaactttataagtttcctaaacttaaagatatagaacatgaaataaaattctgggtttgaaatcatcttctatatgaatcttatgcccaaataataatcgatgatatcactaatatcggtaatagaccatccaattgcaataattacctgcaatgtagatgctttccctaaataagtattcttcaaatgttctagtagaggttttgacttaacaagtaggtatatattgaatagatggaaacaatttggcagagcctttaccaagttcttcaaagtagtctttatatatatatatatatatatatatatatatatatatatacacaacttttgttgatacttttaaattattggcgtacttctcaatttcaatgttctatattgttttggacttagaataaactaggaatgtttttagtggttcactagattgtttatatttaacggattctgtacaaattagtcaaaaatatatatttggaagtaatagttagcttcagacggataatttatcactttgaagacattgaaagtgacttttcatcccgcaatcttaaaattactcccttaatatacatcaatcaaagctattctcgtagcaagaaatggtcagccatattaaatttacatgtctcggtctttctctgtatctaatacaatgaaatctagagggtaaatgaacatttccaccattgttgaaacatcttcaataattttcctcggacgctttatagaatggtcatccagttaaggaatattatggttattttggcctctcctaatggcattaaattgatacttgcactcagctaacataaatcatatataaagtaaatattttctatggtacaagttacagtaaaaatccctggatccttgaccttatttggcaatttattttgcaaacttgttctgcaaccctcaattagcatcacagtctcatgttcatcaaggttcttggtacttattagtttgacccctaaaattacctagaagggagtgaacaggggaataccgtggaattaaagttaccaattaacattaacaagccacttattgattgttctagataattaatccaacaagtctaattatcctaagttgaaatgacacaactatcaataaaatagtaaaaaatataagaatcgttgatcaagaaatccaaatgggtaaaaacttcaggaccaagctccattatggataataatgaacttacaatacgatccaatctaaaaactccactaggctcgttgatcaaattcctacaatctccaagacccattggaacgtgcatcactcatacctgtttccgacattttggaattgtatatctcccatagatcaccaagaactccttattcttttattctttctgtacttctagcccaatctacctcaatcttcaacaacctctgaaagctattgagaaaataccttcctgtatgtgtataggaagtgagtattttgtattacatgaatttgatgtttttcctaaatatgtggttgtgtgaacataaaaatgaaaagattgatcaaaggcttgaatgtgttcttgaatctaggaatgatgttatggagaaagaatacaatgaacaaccacactaaatttcatgttggggggttcaatatatatagtagaaggcatttaggtagcttaggccggataaaactcttgaaaaatgcaaactagggttttatgcgtaataccatccctcaagcgtaggctagcgaacggtgtgttgctcaaacgatagctcagccactattattttcctttcaagcatcagatgggtgataggctagcgtaatccgatggctttttccttccttttacaaactcgaaccataagttacctatttcatctataaaacatttcaattgaccccttcacttttacaacttttcatatttgtcattttatctaaataattgctaatacaataaaatcctaacgaactcccctttggtattatgtgttaaaactattcaatacaagtcatggaagtaaacttaaagaagctatgcattatgatataaaatgccatgattgaaaaatacaattatctctccccttgcaatcatctctccgccttattgcaaactttatcaaaaatacaatcaaatgcaaatgcaaatctcttttcaacctttctcctcatttttgtcacaaatgataaagggaagtttatcaattgaacatcaatacataataacttaaatatacagttgataacatgtacaagcataatccataatcaataaacttttctacatactcaattcaagttaagatggaataaactgtataaataacccatgtgtgtgaaatgtctctaatccgttataagcaggattttataccttaattttgtcagaaatgacatactatccatcactgtcaataggataaaagttcatccccctactgacgaatgtcaaaccaaaagtagcatatagggcctataaaaaaatctcattttgcatgcatattattcttttctccccatatttttgagcgtatatatttttacacaacatctatattttcaagctcatcatttttcttttcaatttttatgtcttatgtgctggctcttctctattaagcgactaagatgatctctatggtgagctttaggtcggttaacccaagttagttgaacataggcaccaggttatgagatatcccctcatgctaaattgttcaagtcaaatgggcttcgaagaagaacataagatattgagccttttttagaagggagtatagttgagttatgtctactaaaataaggtcacttcatgttcaaggtcaccttaccaacacgtgactaccatcctgaatctcacacatgcggttaagtcccactcacaatatcatagtgtgtgcaatgcagatgatagatagatgaaaaaaacctatactaagtactccttacaaacctaaacaagtaatagaaaatatgatactatccataattaaactcatactttgtcacaacgtgtactttcaagtactagtaacattgtgatcactctccttatatcctagacctcccttattacaagcaatcttacccattcctaagatgctatcaagctttgctaaatcactagagaatgcaaagagttgggtgttggaatcctcaagatcgctcatcaaggtcctaaccttattttataaagattcttttacaatgctcaaatcaccaagtctctcaaaggacatctaaagatcactcattagattcttaacgtaagtatctaaagattcattcacagggttcagcttactcagggataagataaattcttgaaggtgaactaaaagtttttattttgctaagaaattctcgaaatttcttagcaaaataaactatatcctcatcattaggtgacttcgaatcagaacactcattacagttttccctaatagtattcaaggctaaagacttatcttttgtaggtttagctaaagttaattcataagtctagataaatccaatcaactcttcaaacttaatggtatctatgtcctcaatctcctttataatcgtgattttaggcctaaatctctaaggtaatgatctaaggatttttcgaactatcttaggctcacaaattctttcacctaggttgaaactagaattaactatctcattcaagctcgcataaaagtaatcaaatgcctcatcctctttcatcataatctcttcaaatctagtggtcaacatctgtaacttggagcttttaatagcttgagttctttcatgtgtggtctataaaatatcccaagccactttcacaatctcatacatagacatagatagtcgcctaaattattcaaggaataatgtaataaataaagcatgtagggctttactgttccaattacactcatttaaattagatttcgaccaattagcaataggtgtagggtaatgtcagcattaacagtgctagaagggacagtccaaccatttactatgctcaaccaaacatgctcacccattgacttagggaaacctctcattctaaccttccaataggcgtaattattgccatcaaaataattaagaacggatatgactgactcattttgactaatagggtcaaggatcaaatttaggctctgataccacttaatagttactaggtcgaccctaaattacgtagagggggtaaataggtggataccacgaaattgaaattacaaattaacagcaacgagccacttattaattgttctagataattaatcaaactaatccaattatcctaagttgaattgccacaaatatttataaagcagtaaaaaatacaagaattgttgacagaaaaaccaaatgggtaaaagcttcgggatcaagccagtaacctctaataaagacaataatgaacttataatacgatccagcttagaaactctgctagactcgctgatcaattttctgcagtctccaagcctggtggaacgtgcttttactcacaactattcccgatcttttggaattttctatctccagtagatcaccacaaattccttgttcttgtactcttcctggtcttcttatccaactttcctttatctttagcaacctctgaaaactattgagaaaaacctttatgtatgtgcataggaagtgagtgttttggattataagaatttaatgtttttcccaaatatgtggttatatgaactcaagaatcaaaagattaatcaaaggcataaatgtgttcttgaatctaagaaatatgttatggagaaagaatgtaatgaacaaccacaccaaaattcgtgttatgggttgggtatatatagtagaaggcattcaggtggcatggggctggataaacgccttgaaaaatacgaactagggttttacaagtaacactatcactcgagagtcaggctagtgataggcaagcgatcggtgtgtccctcaagctgcaggagggcgacaaggttaatgtttttttccgctcgagcatcagataggcgataatccagcgtaaatcttgcgacttgtacctctttattccaaactcgaaccccaagttacctattttatatatacaacatttcaattgactccttgacttttacaacttttcatatttgtcctttcgtgtaaagaattgccaatacaataaaatcctaagattattcttgctagtgagaattttcttcataaagtttgcatagttgggtatttgagctagggcatctacacatgaatgtcgacatgcatcttcttaagcacctcaagtaagtttgaaaactccttgtccagtttatatcttcgtaaccttggtgggaatggataggaggtacatgttctctaacataagcaatcgccttagcttgtggattgtctcaattctctttcaaatttttctcatttgatttttcagattgagttggcactttatttttatttgcaacatttctattaattatgctttcaggttatcatactccactttttttgtaattgcttgctaagtagggctccttgtcttctttcaaatgtagtacaaccagccgacctatttaagtttccaatccttttacggttgccgaatgaatttgtaaaattattctggtttttgtcatatattggtaagttttctgtatgaatttacccatattctgagctctccacaattaccacaaaaccatgaattttgattgcactgcatttgtagaattatttatagtcaagtgatctattatcttcttttccgaagatgacatctgagcacaaaatgtagaaaatacatctatctcatgtacacctgctgccttcatttatatacttctttcagaagaccacaaagcattatttgctaccatggtttcaaacaacttaacaacttcatttggtaacttcaatgtgaaggatccatttatagctgtgtcaacgagtctatgacatgaaagtttcaccttgtgttgaagtattggacttgcaatgctttcttgatactatggttgtacactttctaatcacgtccttaaatctctcccatgctttgtaaaatactctgatttctgaaatattgagatcccattattccatttagttacttttgatggagaaaagtactttataacggaatcatgtatgatatagttcaaatgcttctcctagtagggaatccaattatcctcttgctccatcttgaagtgtatgcgagaagaatcttaattagatagcttcgtatgacacaccattcaaattgtagttttggtagatgtccaaaaaatacgatacatgtatgtcaattctcatttggctttccataaaatgataatccacaataaaacagtacaatgatgtccgtcctcattggaaagtctagttcccaaatgccagataaacaatacttgactagtttggtacaacatgtggtgcgatgaattttctgagtgacaagtgatctccatcaattttaatagacttttcaactcatgatggctgcattactccgttctattctcccatgaggttctgctgctgttgcttaattctcaatataaaagtgcttttcaatttcgaataatgggtacaagatcatcatccctcgaacttcgcaccaaggaaacgttaaaaaagaaaaatatataagaactagaattcgggccaaggttagagttaattaataaaaatgaaagtaaataaattagtctttgacaatggctctaaaaacttgttcgcatgatttcacaagtatatggatcgtgacaagtaataaagtgaaaaattgagtccaagtatcatcccacataaactactgttcactatcaatttttatcttaacttggctttgatctaatttaaatcagcgatcaaatatcaatttttagtcttgtgttgtaactagattgtattgaattactctaaggaaatctaccaatataacgaatccagagtcattggtagtaattcgacgtttgagaagattatgagattaaatagttggtgattaaaatttcacttaagttatttaatgttcatctactcccaattattgtagcctgttttcatagatgtcaaccatcaaatttataagttatggctaatgatctttctggagcaaaactaacactatttatagttgaaatttactatatctatatgtaaatccatacacatgtgaatgcattaattaaaaggaattctttcatgattgtataacccataattctctctcaatctcttttaatatatatcatttatttcacaagctaaattaatgcatcacctctcggttttagaattatccctaaagcaatcgaatatacctagacatttgaaagcaattcaacaagcaataattcactaacaaatattcgagtggcatgaagtctttaaaataactaaatattaaaaatattagcaatattatacatcctaacaaaatttatctagtcacacagagatttaaacaaatataaaggttaaaagagactggattcaattacagcgaacaagataacaattgctccaagatattgttgttcttcctcacttgaatctcgataatggctcttcgtttccttcattaattatcgtagatctcctagtaattctatgacatttcattattaaatcccaaatttcttacacaattgttaaagatttttgcgcataaaatatggaacttgttacacccccaactaaatcacttcagagaatcagtcacgccaccccccgaagtgccatgtgtttatccgaagtgatgcccacttctgacaacctcaacatggtgagccgcaatgtgacgagtagatccactgaagtaatcgaagtgtccctcaactccgaagcgctgaacatttcgaggcacttccttgatagatccctccgccgccactgtcagatatctccaaagatcaattgatgtgacatctccataggtctagttaatgtgacgtattgactttatatcaacttaactcagaagaactaagtgcccgcccactgtaaacacgactgattgatgcctatgagcggacgcctcacaccgtcagatgcatacacgtgtctcacatccaacggtgctctacatctataaatacccaaggttaggaaagagaaagagataatgaaactcttattaacttagctttccatactaagaaatatatattctcttccccactcttttgcataacttgagcactgtttcgatcacccaacgctgacttgatcatcggagtgtatgcagccgccaccaccaccgctagttccgatcgtgtgcttctgaccgtgtgttgtgcacagggaggattatgtggagtagctatccgttggccacatggagggtccaattctcaaggtcaatagattggcaccgtctgtgggaaactttccttccaaaagttccacattgtccagtgaaaaatccaccaacaaaccaccgatttaccctgaaaagggcacgttcttgaaaaagaacaaagtcaacctacaaagttcttaaaccccttgaaagggtaaacaaaatgatttatagtaatgaagatgcaaattttgaagggcacagggatgtctctgaaaaaaagataatcaagaccaatgtcacgcatcagagaccccatcaccggcgtcaccaaggcaacgggacaacagcgctcactgaagggatggctcaaatagctgtcaaaatgagggacatcgtcgctcagaatgtggcgatgcatgaattcttcatgcaagcccaaggtcattagggcttccagatgcctcaaggatcatatccagctcaaattcatgtgcctcatggctaaggccattcgagccagcaccggaaacacccctttgaaagagaaataggtacggatgtaacatcctacatgtagggaagccaaccagcagagccaccactaggagataacttcccaccagaatacgaaccacaaaggtttgttagtgtcttcgatagaatagggtagaacctagcaatagggttcgctctgtacaaagatcagtgcgacaagagcaggagcaagaacaagtacctccttcgcctagaaataggcgagagaggaaaaacctagtggattgggatagtcgaggagaggcacatccatccctccccccctccaaaatacatcagagagggaaggctctaaatggccatgtcgcttctacaaaattgatgataatgatgacaacctccccttctctagagaaatccgaagcttcccgatgcttgcaaacttcatgctccctaaaatcccaaaatatgaaggaaagggggacccacaaaaacatttgactaagtgcatgacgcagatgagcctcgttggcactgaaatgtagggcctttcatctaaccctcactggagctgttgaagtgtggtatagcagattaccacccctgagcatcagaagctggccaaacttaaaaaaggcatttctgaaccaatacctttcatgaagggaatgggagccccagggcgacgcctgcaagacatgagtcaagctcctgacgagatgctgaagagctatcttgccaggttcacaaataaaatcatgtactgcgagcaaatcactaacaaagaggcccttttagccttaaaaggtggcctcaacatgaacatactgttctagagggatgtacacagcaagaatcccaccacctatgacgagctagttgaaatgatgagggtggaaattgtcaatgaggagatgattaaccaccggaaccatgcggctcaaggactttcccctcctcagaggcagatgggtcaaggaccagctacacacctcgtcaccaacaatagacctaggccggtcacacgatagcccccacatctagataggcattagcttcagccactctaaatgcagtgccagtgctagcatatgaaaatgttcttgccgaagcaggaccatctggaggaacaaacaacaatcgaaaaaagaagaagaagcgatcaaacaaaccctggaaggggcaaggttttgcaccttttaccaactttacggacacgacaccaccgaatgtaaagatgctcctcgatcctcgaatcggagtaaccaacactcctcgagaagggatgaatacccccacaggtccaactccccgaataggggagagaggcgatatagagaccaattgcccaagaaaagagaatccagagacaaaggagaatccagacatagagatcaggccccatctaaaggccaagttatcaaggaaattgatacaatcattagaggacctcacatcgagggaaacaccaagaacgcccagaggaactacacaaaggaagcaaaggatccaccaatgattactcacattgtcaatcagacccaggtggctagcaaaatagccccgatcactttctctcaagaggatgcacaaggagttcaccacccccattgtgatgaattagtggtaagagccgtagtggcccgaaacggactcaaatgcatgctcattaacaatgacagctcggtgaatatactgttcggatccacctttgataaaatacaaattgaacacgagttgatccccattaccaacccgttatttggatttactggtgacatcatcgtcacacgagggtgaattactctacctgtcgagatggggtcagtccccctagtggcccaccacttcatggagttcctgtggtggaccacaaatcagcttatcacggagtattaggctgacctaccttgaaagatctttggacagttacatacatccagctcttatgtatgaagttcccaactaagcaggggattgctacagtgcgagacgaccaaatgggttcaagggcatgttacctcaactcccttcaaaaattcgaaccccgcactattaatgtcatcataacgggtaccaccaaaaaagctggcatggacatagaaatgattgacgcccctaaacaacggcgtacctctgaacaggagaaagacgtcgacatgatagaggcccctgaagaaaggcaccctcttgatgagttggatcctcgaattatcgagtccgaaccaaatgctactccaatggaagaactggagacttttcccatcaaccctggagaacccattcaggtcttgcagatagggaaagcactaccccccgaagtgaaagaaggaatgatgaacttcttaaaaagaaacctggatgtcttcgcatggaagcacgaagacatggtggaaatagacccaaggatcgttgccaccaccttaacatcaactcctcatatgttccatgatatgatccaagagtcgagctcgatgaaggcaagtgcgagacgagacccgttggtagtcgatggcagaccaatgacgcgatcaagggcaaagcaagtgaaacaagcaatgggattgctcgtttaagaaaccattgatggaaccatgtttgggactcaaaatggagcaactttcatgttcgggtcgaaggccaaatcaacttggatcaatttgttatcaagcgacgaaactggaggctgaaaataagcctgtgcggccgcacaggcaaaaacaccatgcggccgtacggtggcataccgaaaataaaaatcgcatttcttattgaaccatgcggccgcattgaatacatcattcggccacataagccaaaaaaattcgcgaattttccaaagttcgtctcaaaaaatatcatttgcaggttcggcattccccactctttagtgtctgataactggttagaggcatccagagccttagtggcgagccggtggtgctcattagaatgatcaatcctcctcatcatagcagccacctgacactccacttcgtagagctccttcttcagcctctccacctcctcattggccctcactagccggccctctacctcctgctttgccttctccgcctccgaggccctctcttcgatagtctacaccgtattcccatagtgcaatatctcctccaggcgcttggccagatcctccctcttggcgtcgaggtccttgaccaagccttgaaattggacacttgtactcagagcccaggtgatgcaagcactattagcagcaaccaggtcctctgtggtgcaggaggaggtgtggtctttccactcctcgatccaatacttgctgtggacttgagctatagccaccgtctccggaggcaaggcttccaacacctccctcactggctcccctttgttggtgcccagaaagtccacctccttttctggacgagccctttttctcctttactatcccgacacttgtgcaactggaatggcaatgataggaggaccgatcggggcagcaggagacatcgacctctcccttatggccacaccagtggggattgttgtctggcggaggaccggggcaacccttgctactataggctgctctgacaagctggcagcctttttctcttcctttggacagctgcctccggctccttctccttctcctcatcctctgctataggctggagttgtttgctcgcagtcactaggtcctttgtttactttttataagtaaagaaggaggtcttcaaggcctttgcctcggccatcatccactggatagttttgaagtcgggcctcatcgacctcttcttgttgaaattgtctacagcaaaacaaaatggattaacataagtacaataagtctggaaacacattagaataagtacactccagatagttaccttgggaggccatcaattcgtgcataacgaagtgagtgttcttgataagctcgttataagacctcatcttcaacaaaagctgataaacgatacagattatgttaaactccttggcagaaagctcgcacagaggaagagtatctgcaagaataacaaatagttaattaccgagctgatgcgaaacacaaaaaatcacaaagctcagtactcactaagtgtaaaatactttgtggggaccgtaagaggtgccagaaggttcctctccattgtgtcccatctcccaaaagcccagcaccatgaactcttccattccttgatggagcttggcagatcaagtacaaatggagtgtgggaaccccatgaagtcaggtagtgccaccctccggtgttatcaccccccgccgctaccttagggatatacaaagtttgaaacactaaaaagggcatctctatcccaaacgactcctccttccatagcatccatgaccccaccatttgactccaagaattggggttcagttgggtcagggccagaccacaagtcttcaaaacataacgaaagaaagggtagatcggcaacctaagaccagccctaaataatgcttctctcacagctacacagcccggcctagagtaacaggcccgctcatcaagctctggcaaaattaggcccacactatccgggatcttatatttcatcctaagtctatcaatgtcggcaggcttaagtttggaagggtaatcatacgcctcccagcgtatggaagtgtctatcaggctatcaggccgcctccaaatgttttccccgtttaatatcaccccaaacaatttcaaggaggtcgccaacactggatggtcaaccctcactatctccaactcccttcccgaagcgttactacccttagaagccaacttcaaaattcaaaaaatgcgaagaactagaaaaatacttactgaaatgaatggattgaggttttctatagttggaaaataagaaatgggccactgtacttgccaaagactgaaaatgccataggaaaacacttgaaaatcgccgaaaatcgcagagaattttaagagcacctagagcttaatttcgcaaaagtgaaaacctctaacaatgctcaagtcctccttttagaggaagcccaagatgattcccaccgttgaattcaaatgatgtcaatctaaattgttcatctcatcacaaatttggattgttgaaataaaacgccagatttgatcaacacttaagatctgattgtgcccctcagacacgcataaagcccgtcacctcgaacaacaacagtcgtcatccataagtggctgcagcagccctttttcttggaacatgcaatatatccgactgtcgccttgaaaatacgcgacagttgtcgcatcgattaacgtcataatcagacgcttcagatcagggacagtccatcccaatatacctcagatgaggtactcagctttgtaagcttcgacgtacctgacgcagagatccctgtgggtcatcacctcagacgttacattttctcagctttacaaagctttggccattttccaacacgtcgccccctgtgggccaacgcatcggtagcagatgagctcttcaaccaactttacaagcttcaatgcacatgacgcagagatccctgtgggttatcacctcggacgctgcgttttctcagctttacaaagctttggccatctcccaatgcatcctcccttgtggtcagagcatcggtagagctcttcaactagctttacaagcttcaacgtaccttacgtggagatccttgtgggtcatcgcctcagatgctacatttcctcaactttaaaagctttagccatctcccaacgcgtcgtcccatgtgggttagagcatcgatagcagatgggcgcttaacccaacttcaaaagcttcagcgccactgacgtagtccctgtgggtcatcgcttcgatctcatgattcctcaactttacaaggttttagccatctcccaatgcatcgtcccttgtgggtcaatacgcccgtggcggatgaactcctcaacctactgttacaagcttcgacaaagccgagagaacgccctacctactccgccttggtcatcacttcgcttcagccaacacctattcggcacgcatgcttattccatcctcccacatcagcacttcatcagaatccacaatacttactctaaggctagcatacacaatcgggaaagcaagtccacccataataagaatattcatgcctgaatttggggggaaccactgttacacccctaactaaatcactttggagaaatagttacaccactccccaaagtgccacatgttcgtctgaagtgatgcccactcctgacaacctcaacatggcacgccacagggtaaagagtagatccactaaagtaatcgaagtgtccctcaactccaaagcactgaacacttcgaggcattcctttgtcagatccctccgtcgccattgtcagatttccaaagatcaattgatgtggcatctccataggtctagttgatgtgacctatcgactttatatcaacacaactcagaagaattaattgcccgccactctagacgcggctgattgacgcctatgatggacgcctcacactatcagacgcatacacgtgtctcacatccaacggtgctctacatctataaatacccaaggtttgataagaaaaagaggtaatgaaactcttattaacttagctctccatactaagaaatatatattctcatccccactctcttacataactggagcactgtttcgatcacccaacgctgacttgatcatcggagtgtatgcagctaccaccataccactggttccgaccatatgcttctgaccgtgtgttgtgcgcagggaggattacgtggagtagctattcgttggccacgtggagggtccaattctcgaggtcaacagaactttcttctcctttttgttgtactttttctgcattatgtcctctctaattcttatgccaccagctttcttttctattttcaagaattttactcccatttaaattcctcacagcaagtcattcattcccgtctgaattcatattttctttcacaacttatgctataatcttactgcggccaaaattaattaacaaagtgaaattcagtccctgaatccactttattgttcagcttaaatctttatttttttaactcaagtccttcaatttataaattttaaatttgatcgcaaaactacaaattctatccaaatttcgtccttcttaatcaacactcattctgataatggttttctcctaccacaataaaaactatacataattaaacaacaagttcataataacgctcccaaagccacttttaataacttagataagtataatgtttactcttatcattttgtggtcttttaatgatcctcaagatttccacgacctatacagttagaatcttggactggacaaatccactggaatggacttgtttttgatctccttagaaaagaaaagatcttcttcattatcacgttcgaatgatctaaattaggctgggttgtcatagtgagtttcgtcatgatattttttagactcgtccttaattgtcatgtaactcttggtgccattataatttgtttgcttccacgtctagtctatttatctcttgttggaaaaaattagttgagtggctaactttggcacaaaatttgagtggaacccggttggttattttggaagttcaagattgatttgtgttcttctctatgaaaacatcgaaatcttgtatttacaagccagaaatgatgttcgggtgaatgggaaatcggagctaaaaatgtgccaattgaaaggagtttatcggagctaaaaatgttccaattgaaaggagtttatcttgttggaggaaaaacatttaagtttgtcccacataagaaaattatgaaagcaaactccaccttaaataggattgcactcttgaatggtgtgatcatatgtagtatagaagttctctctatgtgtgctgatacgatccaggagtcgagcccgacgaagggatgtgcgagacgagacccgttgatagtcgatggtggaccaatgacgcaatcaaggtcaaagcaagtgaaacaaacgatgggattgctcgttcaagaaaccattgatggaaccatgttcaggactcaaaatggagcaactttcatgttcaggtcaaaggtcgaatcaacttggatcaatttgttatcaagcgatgaaagcagaggctgaagacaacaccatgctgccgcacaggcaaaaccacatgcagccgcacacatgcatatcaaaaaccaaaagtgcaatttcagttgaaccatgcggccgcatgtggttttgcctgtgcggccgcatggtgttgtcttcagcctccgctttcgttgctttttgataacaaattgatctaagttgattcgaccttcgacccgaacatgaaagttgctccattttgagtcccaaacatggttccatcaatggtttcttgaacgagcaatcccatcacttatgtcacttgctttgcccttgatcacgtcattggtccgccatcgactatcaacggatctcgtctcgcacttgccttcgtcgggctcgactcctggatcatatcatccccttcctcttcaaaaggatttgtccttgaatctgaacctacatcaaacagagagagatcagatacattaaaaatagccgaaacattgtactcacctggaaggtccaacttgtaagcattgtcgtttatcgtttcaatcacttgaaatggaccatcgcccctcagttgcaacttggacttcctatgctccggaaaccgccctttcctaaggtgcacccaaacccaatctcttggctcgaatgtcacgcgcttcctacctttgtttgcctgcgacgcaaccaacttacttttgttttcaatttgtgcttttaccttttcatggaatgacttaatcaatttcgccttctttttgccatctaaactaccacgttcattcacaggtaaaggaattaaatccaaaggagttagtggattaaaaccatatacaatttcaaatggagaatatgatgtagtagagtgaacagctcgattgtatgcaaattcaacaaatggtagacactcctcccaactcttcaaatttttattgattactgtgcgtaacaattgtgtcatagtcctattcactacctcagtttgcccatccgtttgtggctgacaagttgtggaaaaaagtaacttagtgcctaacttaccccacaaaactctccaaaagtcactcaaaaatttgacatcccgatccgacactatgcttctagaaaccccatgtaaacgcacaatctctctaaagaataagtcagtaatgttcgcggcatcgtcagttttgtgacatggtataaaatgtgccattttgctgaacctatctacaaccacaaaaatagaatcccgacctctcttagtcttaggtaaacccaaaacaaagtccatcgagatatcaacccaaggctcactaggtgtaggtaaaggtgtgtacagaccttgtggtaaaaccttagatttagcctttttacaacctatgcatcaactacaaattcgatcaacatcacttttcatcttaagccaataaaaatgctccttcaatacatctaaagtcttttgaaccccaaagtgtcccatcaacccaccactatgtgcctcccttactaacaactcccgaatagaacaattctaaacacataacctattttcccgaaataaataccactcatgcctaaagaacctatcaaccgccccttttatgcatgaaaaataaatatccgaaaattcaacatcttttttatacaattccttaatatgttcaaacccaagtaacttagaatcaagagtagttagcaatacgtaccttcacgacaacgcatccgccaccacattttccttacctcgtttataccgaatgacgtatggaaaggtctcaatgaattccatccaccgtgcatgcctcttgttcaatttaccttgtccccgcaagtgcttcagtgactcatgatcggtgtgtattacgaactccttcagccataaataatgttgccaagtctccaaagcttgaacaagtgcataaagttctttgtcatatgtaggataacttaaagcagctccactcaatttctcgctaaagtatgcaataggcctctgatcctgtattaaaactgctccaatccctattcctgatgcatcacactcaatctcgaatgttttgtcaaaattaggtaatgccaaaacaggtgcttcacacaatctaccttcaatagtattaaatgcaagttcctgttcatcaccccagtgaaaacctacactcttattaactacttccgtgagtggtgcggtgatagtgctaaaatccttcacaaatcgcctataaaaactagccaaaccatgaaaactcctaacttccgttatgcttttaggtgtcagccaatctctaataacctttatcttttcatcatctacttctaccccattagcactaaccacaaatccaagaaaaataactctatccatacaaaacgtgcattttttaagattagcatagagttgttctttccttaaaacaattagcacacattttaaatgttccaaatgctctcctagatttttgctatagattaagatgtcgccaaaataaaccacaacaaaatttcctataaaagcacataaaacatgattcattaaacgcataaaagtgttaggtgcatttgtgagtccaaacggcataaccaaccattcatataaaccatatttagttttaaaagccgttttccattcatcaccctcccgcatacgaatttgataatactcgctttttaaatcaattttagaaaatatgtaagaaccatgtaatttatcaagcatgtcatctaacctaggtatagggtgacgatactttcccgttacgttgttgatagccctacaatccacgcacattcgccatgttccatccttttttggtacaagcaaaaccggtaccacacaaggactcatgctttccctcacatatcctttgctcatcaacttctccacttgcctttgaagctccttagtctcctcgggattacttcgataagccggtcgatttggaatcacagctccgggtatgaagtcaatttgatgttcaatgcctcgaataggcggcaatccacttggtgcatcctccggaaatacatcatcgaattcctgcaacaaagacttagccaaactagggaggggtgggttagtttcctcaaaattgaggagtgattccttataaactaacaagatcatctctttcgtctcaactaccgccctcctcaaatcactctcttttgcaaaaaaattcgctcgtgttttctctcttctctcggggcactctcttttttctctctcttgtgattgctctctcttttcctttctaatggctatctcaatattttctctctttttctccaactcactatttgctctcattttttctaactcttttgctctcctctcttcctcacttctcaattttaattggtcctcatagacttgcgccggtgttaatggcacaagagtaatggtccttccatccttaatgaaactatatcgatttttgtacccatcatgcatagctttcctatcatattgccatggtcgccccaataaaatatgtcccgtttgcattggcaccacatcacacgctaactcgtcctgataactcctagttgacaaattaagtaacacccttcgattcaccctcacctcgccactctcattcaaccattgcaatttataagatctcaggtgtctcaacaatgttaaacccaatttttctacaagagatacgctagctacattagtgcaactaccaccatcaattataacactacataccgtactgttgacgtggcatcgagtgtggaaaatgttctcccgttgcaactccaagtcatccgctttgatgtgagtagtgagagctcgccttgtgactaatagatccccaaccggcccttcaactttttcttcttcactaacaccctccaacgtcggcagtcatcaaactcgccatcactatcgctcacaatctctccattatcccgcaacaccatcgcccgtttgtttgggcattgagaagcaatatgccccgttcccaaacacctaaaacatttgatgtcccgattgcgcgacggttgtgcctccgattttgatattggtttgctagcattttcatccttgcccttttgccaatcatttttacctctaggtgcagccccatttttattattgtcatcccacttcgattttcatgttggattaagagtcgaagtacctaacggttgctagacgtccccttcctcttcaattgcctctcgaccttcattgccacatgtaacatgtcctcgatttccacataatgttgcaactctacaatgtttgcaatatcccgatttaacccattcaagaaccgtgccatggtagcttcccgatcttcctccacattagcccgaatcataagaatttccatctccttgtgataattctctacgcttttcgatccttgatacaaaccttgcaatttttgatggatttccctataatagtgactcggaacaaacctccttctcatcaacatcttcgactcatcccaagtgctaattggcctttcccgacccctacgtcgtgatgttagtacttgttcccaccaagatatcgcgtaatctacgaattcaagcaccgccaattttacctttttctcctccgaataattatagtactcaaaaatcatttcaaccttcctttcccaatctaaatatgcttccggatcgcttctccccttaaattgcagaatagtcattttaatacttcccaaatttccatctacttcatctccctagttatttctaccccgtctttccatcctatcgcccctatgcctcgctcgtcccatatcaatgtcattttcatcaaaatcatcctcatcactacgatactcatcccgccttcctctcctagatttacgcctacctagccccctaacattagacatctccacttgtccccggctaagattagcaattgtagtacccatttgtgccatcccttccccttacctatccaccttctccctaacatcaccaagtaccctttcaaacctccttatcatgtcctccgatgcattgttgtcattaccatttcggcttgaattagaaccttctctttctgacatcatatcacacaattttttttatgcctcacaaagatttcactcggaaaacactcactatggctttttccctatattaaactcacccctcggccttttaccactcaaagtctccctccaagcacttcaaagaaccaagtgaactaaatcaattgttttaccggcaattcaaacaaaccgaatattaatcaaaaaccacgagactgacttgaataagtggaatagatgaatgttttgacactaatatgtgaatagactcaaaaaaagaatgacagactcgaacccaattgaatatcccaaaaatcaaacacaatgtaggaattgttgttggtaggaaaaaaacacaaaatcaaacaatgatatcaaaattttatatatatattttttgtttttttgtgaacaatacttcgagatgaacagtagctcaaatgtacagtaaccctttttttcgtttttgtactttttttttttactccttgataaaagaaggtgagtaaactaccaataactcaacaaaacgatgaaaagaaagcaagaatgaagaaaaactaagaaagaaaaattaacgacccaaacaaataaagaaaagatataactttcaattaatttggagccaaagctctgataccaactgatgctaaccccgtagcaacgttgactatgaaacccacaatgagattgacgaacccaagaaagccaaattaatccaaaagtttaggattaacccaaaagaaagtcgaaccaaaaaacccaacaagaacgacgcttgaaagaccccttgatcacgcaatccaagaattaaatccggttgtttgaacaccacaagttatcacttgataagtttgaaattgttcaatgaagaacgatgaagagaagacaatacgcctcactttaattcaatatcaataatgtcaaaggttttttaacaattgaatggaaactcctatttatactaaacctaaaaactaggtaaaaatcgtgcaaaagtcgagcataatctccaaaatatggaaaagaatcaaaatctaacaaaatatggaaaattgccaaaattggaaaattcgccaaatttttggcttgtgcggccgcatggtgtaaatccatgcggtcacatggttcaactgaaattgcacttttggttttcggtatgcatgtgtgtggccgcatgtggttttgcttgtgcggccgcatggtgttgtcttcagcctccgcttttgtcgcttgataacaaattgatccaagttgattcgaccttcgacccgaacatgaaagttgctccattttgagtcccaaacatggttccatcaatggtttcttcaacgagtaatcccatcgcttatttcacttgctttgcccttgatcgcatcattggtccgccatcgactatcaacgggtctcgtctcgcacttgctttcgtcgggctcgactcctggatcatatcatgtgcacagggagagcaaatcgaacataaataagcttcggatggggaatttggccccttagaagagcctacattttgctaatttttttcctccaactgaccgtttaaattccaaaactgttgaaactcctatattcattgtcattacaatatgagttaatgatattcataatgttgaaactatatatatgcaacccaatttcaaacaattctacacaagagataaacaacacggcatacaattttttgcataatttatgtaacacagtttctgcataattttagtctgcatagtcacacagtcccctatctgtctggaagtattttgttaatattgttcagacacaaattctatatggcagagtactatttgaggtgctcaaattttactattcctccgtcatatttaaagagacaaacgtcctaatcaaacctcaagcacctatgatgagggggcgaatctgttttaaggaaactatgttctcatttaactcggttaaaatttttcctgcttttggctaattagtatacttgttctattttattggaatttaatctgctatattttttatagtatccaagttcattgcatgtacggtatatgcaaaactggtatgtgcaaatttagtagctatgttttatatatggtaagctgcaaatactatgagtggtaacctgtatatatggtatgtgtaaatacggtatgttccgatatattgcatatacgatatatatcattttggaatatgttcatccggtatttgctaatccgacattcatccactaaattcagtccaacaagcttaaaacaggttcatttagcaaatatatatatatatatatatatatatatatatatatatatatatatatatatatatatatatatatatatatatatatatatcttatattgttgattttatagactaattttttgtttgtctttcagaaatgacaactaaatcaaccaatatggatatgtcccaaaatgttgctactagaaatcaagttgcgggctcaactgtagcttaaggtccgagtatgttgtggcttagactgtggctaaattaccaagttatgttgtgaggcaaactgtggctccaacaactggccatattgttattgttccagttaatcatggagaaaaactggagaaatttaataatttgaattccaaaggtgacagcagaaaatgttattttatctgaccaccttgaatcttgtgagattctggactgaaattattccagaactcaatgaggatgagggagatgttcaagcgactagtgtacttgatgcatggaaacattcagaatttctatgccgaaactacattatgaatagcttagtagactaactatacgacgtgtatagtactttgaatactgctaaggagctatgggagtcattaaatcgaaaatgtaagactgaagatgccggggccaagaagtttattgttggccaattcttggattataaaatggtagactccaaaatagtaatcagttaagtgcaagaattacaaatgattcttcataagattcatgtcgaaggggggtgattttgagtgaaactttccaaatggctgcaattattgaaaaattgtcccccgtgtggaaagatttcaagaattatgttaagcacaaacgacaggaaatgaatgtcgaagaactgattgttagacttcaaattgaagaagacaatagaagttcagaaaagaatgagttcaatcctactgctgataaagacaatgttgttgagcacggtcaaagttctaagactgtaaagaacaagcataggatattttgtggcaaaggtgctaagctgggaccgaaaggaggcatttctgagaacaaatttcaagaaaaatgcttcaattgtgatcaagtaggccactagtcttcagagtggagattactaaagaagaataataaaaaagcaaatgtggttgactacatgacacatgatgtgtcggaaatgaatctcacagcagtcatttttgaagtgaacatagtaagttctaacccaaaagattggtggattgacaccgatgctacatggcatatgtgatctgataaagagttgtttgttgcattgaaaacaattgagaatggagagaagttgttcatgggaaattcaacaaattctgagatcaaaggtcaaggaaaggtgattctgaagttgacttcgggaaagaagttgacacttaataatgtgatgtatgtgctgaaaattcgcaaaaaccttgtgtctagatcacatttaaataaacatggttttcgcattgtatgtgaattagacaaagttattttgtcaaaagatgaaatgtttgtcgaaaaatgttttgtttttgatggtaagtttaaactaaatgtaatgttgttaagcaaaaaatgaataaaataaactcttctgcttacttgcttgagtctttcaatttacagcatggttagactaggacatgttaactataatactttacatagactagttaacttgaaatgcatacccgcattccacattgattccaactataagtgagaaacttgttttgagacaaaattaacaaggtcatcctttaaatcaaccgaacaaaatacagaaccatttgatttagttcatagcgacgtatgtgacttaaaacttgtataaacaagaggtagcaacaagaatttcattacttttgtcaatgatagcacaaaatactattgtgtatctgcttaaaaacaaggacgaagccatagagaaatttattctctataagaagaagttgaaaatcaacttcataagaaaattaaggtgttgcgaagtgatgaggtggtgaatatgaagcaccatttgctgaattctgcgcacaacatggaaacatacatgaaatcactgcatctaattctccgtaacaaaatggtgtagctgaccaaaaaattcgtaccttgaaagaaacgatgaatgcaatgctaataagttctaagttagctcagaatatgtgggggaagactgtgttatcagcaaattaccttttaaataaggtgccccgaaagaaaatggaaaagaccccttatgagttaggaagaaagtcctcctataaatacttacgagtgtggggtgtcttatccaagtggctattccaacaccaaataaggtaaagataagcccgaaaactatagattgcatctttattggcaatgcacataatagtagtgcttatcgatttcttatgtatgactctaaaatcccagacatacacaaaacatacgataatagaatcaagaaatgcttcattctttaaacatgtatttccatacaggtctaaagaggaagcaagcttttctaaacgaataagtgagactatgaatgaaaatagtcaagactaaaagctagaataggagattgaggttagacaaagcaagtgagaaaggaaagaaaaaccttatggtcctgattttctaacctatacgctagagagggaacctcaaaattatcaaaaaatgtgaactcttcataaggacctcaatggaaatatgccatgaccagtgaaatcatacataagagctagtggatcttccttcgaaagtaaaccactagactacaaatggattttcaaaagaaaaataaaaacaattggaactatcgaaaagtataaggatagattagtaataaaaggtcaaacaaatggaaggacttgattactttgatatgtattctccagtgacgagacttgttctaagttagtcatattatgtggacaaaattttcgaaaagttcaataaggataatactggcttgactagaacaccgatagggtaattggcgcaaaacgtccctacctttcgagtgcattgtggaaaacgtcatcacctttcttttttttggcatttttgcccctatttccacctttctttgcgttgaacgtccttttcacctatttttgacataaaatgatcaacttaccctcctatttaaacaaaacaaaacaaaaagaaaagaaaaaaaatgcaactataggcctagactttttatatgtgtaaatgagcccaaaattgaaaaatttgtcttctacacaccacccacactccactgccggcttccacctcaacaaccaccaccgaaacgccgcctaaaacaccagagctcacaccacaaacaactttcatcagcttcgagccttttccaccctaatggccgcttagcgtagccgcatatgaccaccagcaaacttaaatcggaccaccttaaaacatccatcaacggcaagtcctgaatagtacggtctacaaccaccaccggcacgcaacccagacccatcgccttcaccatccaaaaaaaaggaagcggaatttactggttttgacattccccacctgatctgaagaatccctttctatagcaacaagaaatcagcatctttcttcaattcttccgtgaaatttgactcatttctccatcccattttaaataacccagaaacaacatcgttgatgcattcgctggtttggaaaagatgatgctagtggatgggttcagtggaggtaaagtgatgtccttatgcgcgataaagttaccggagataatagggaaaacagaaatttgcacagaatttttcttcagctcaataacattccggtcggctaaataatcaatacccgccggtgataggaaagaaatgatcagtaccaagtgtacgattccaaaaaggatgtttactctgaagtctttgacaagatgcgcaagaaaacgcctgaaggtgttgggaaaaaagggtacgaagaagaagtgagcttcattggggtcttgagcgttaaaggggcttttcaggagggaattgtaaaagagagatgcaactggattttggaaagtaaatggtttagctggggtgtaaatgaaaattttgaagttagttagcatgttttggtagttctggaaaaggggtgggagagaggtatggtgaaggtgaggcggcagcattggagaagagggggaggggggaaaacaagggtagctagctatggccattgggatggaaaaggctcgaaggttgtgggctgtgttttttcaattttgggcttatttgcatatatgaaaagtctgggcctatcgttacaattttttcttttctttttgttttgttttgtttaaatatgagggtaaattggtcattttacgtcaaaaataggtgaaaagggtttagcacaaagaaatgtgaaaacaggggcaaaaatgccaaaaaatgaaaggtgggaacgttttccacaatacactcaaaaggtagggacattttgcgccaattacccaacaccgatagctacaagtcaacatctatctaaaaacaaaggtgaaagtgtttcttaagtagagtactcgagaattattggaagtctaatgacttgatgagttgtacaagagtagacatagcctacacagccaataaactgagtagatatacgagtaatctaggagctaatcactggaaatgaatagtaagagtactaaagtacttaagatatactcataactttgcactatactataccagatatccagtggtcattgaaggatatagtgacgctaattggatatctgatataaaagactcaaaatctaccaatggatttatgttcacattgggaagtgctgcatagcctaaaaatcctataagcaaacatttctaatcgaatctactagagaatctaagtttatggctttagtaaatgtggtgaaaaggttgagtggttgcgcaacttcttagaggatattttaagatggtcaaacccgtgcaagtaatttgcatatattatgacaatcaatcagtaattggaagggcatagagaaacatacacaatggtaagtctagacatatacattgtagacataataccataagataactactctcaactggagttatcactattgactatgtaaggtcaaaagataacattgcaaatctactaaccaaagggttagattgagagttagttggaaaatcatcgaaaggaatgagactcaagcccttgaacggataagttattacaaaggaaatccaacatagttgattgaaaatcccaagatctaggttcagaaggacaacctaattgtaaataattaagtaaatcactgtatgggatgttatctcctgtccattcctatgatgtaatggtgatgtcgataaggatgaagataagcaataggattttaatgattcctatacgccaaattttgagccaagtaatgcgggttacttgtaataaaaaatcacttaagtgaaacagaagtggggtcgtttctaagagaattgcgtggggctcaattcttagaaactctcatagaaccaggcatatggtcatggccaaaatgaacataataatgagaactaattgtgttaggaaagaatcatgtccgaagtatatcatcgcttacacaaatgacagaaaagttcaaagacaacatatctactggtcagctagtaaggtaaatatatttttacgacagaatgttcaaagggtaatacctacctatcctatgcaggtttcaatcattgaactttatcaccaagtctctttgtttcattatcttgtgtctcttccaattttcattcatgtgggattgttggaaaaaatgggttgagtagctaactttggcacaaaatttgagtgagatctggttggttattttggaagttcaagattgatttatgttctcctctatgcgaacatcgaaatcatgtatctaccaaaattgattttcggatgaacaagaaattcaagctccgagtgctccaattgaaaggagtttatgttgttggaaggaaaccatttaagattatctcacataggaaaattatgaaagcaaataccctcttaaataggattacactttggaatggtgtgatcatgtgtagtataacggttctctatacatgcacgcgcagggggcaaatcaaacagaaataagcttcggacgtagaaattggacccttagaagagcctatattttgctaatttttttcctccaactgatcgtttaaatttcaaaactgttgaaactcctctattcattgttattacaatgcgagttgatgaaatttatggtgttgagcctatatatatgcaacccgatttctaacaattctatagaagagataaacaacacggcatacagttttttgcaaatttacataacatagtttctgcataattttggtttgcatagtctcacaatccctgtctgttcgaaagtattttggtgatattgtttatacacaaattatgttcggcaaagtagtatttcagatgctcaaattctgatgttcctccgttgaatcctagaagacagaatccaaatcaaacctcaagcaccgacagtgaggggacaagtctattttaaggaaactgtatttacacaggcctcggttaaaaattttctttgcttttggctaattagtttacttgttctattttattagaatttaatctgctatattttggctaagtagattaatttgctcagtttattgcaatttaatatgctatattttgggtagtatcgaagttcacttctatatgcgatatatgcaaaactggtatgtgcaaatccggtatctatgttgcatatacgataaattactgtgtatacgataagctgtatatacggtaaggtgcatataaggtatgcataagatatggtttgttgcatatacgatatgcataaatccgaaatgatgcatatatggtatgtatcaatccatttatatccatctagtatttgctaatccggtattcatccacaaacatttagtccaacatctctattagtggtttatctagaatctattgttgttgtaaattgacttcctcaacaagcctctcaaagaagttataaacctattttataatttgaagtttcatcttgaaatgtcaatctggatataataagttatcaaatatttggttaatacttttatatttacaactcagagttgaacgtgcattgcacgttattctaaaatactttataaatgctataaaagtaatatttgatatgataggccctgattttgatctgccactgcataaacagtatatggaagaaaataaagtttagggtaggaatttaagagaagaaagttgaactctcaaaacttaacttctatgtttcaaattttttgtcacgatgaaatactacaaatgagcaaccttcttacactatatttggttaaactgtatttggtacataagaattaatttctaataaatgaatttaaacacccattaaaatttcaagatatatgaatagaaataaattcatctataataactcaaaatttatgttagactcatcaagtcaagatttaatgagtctagattaatgtgaatattaattaattgagaattaataacatgaaattcatacatgactaaggattttgttgtattgattacatattgaaaaataaaactctaaattcatgtaaatcaagattcattgagtcaatattaattgagtctagattaatgtgaatattaattaattgagaattaataatatgaaattcaaacattattaagaattttgtagtatttattacttattgaaaaataaaaagtaaagtactatggaagtaattgaattgcagggttagaatcgtccaaaaaaatgattctcactttttgtgatatttaatgtattatagatgtgtagtacttattccttaatatgccttcaaaacataatggttcatttgataacaaaaagcttgaaattcgtgcgcatttgacctttacacaaatcaaatctcttgttggagtttgatattgtttaataccagactatatcatggggatccatattaaaatatcaaccttgttaaggggagtagttcgaattgttataagttaggtaatatcttcatattatccgatatgggatttattccttgacaacctataggtctttgttctcagttgtatggattattattactcacatgtagagggtcatttgaagtttgtagcgtggacttttgggacgtcaataatactatgagtgtaggcatagcttatttctgccccatggttgattcctctaaattccacaagagggtcgttctggttatccctatttttaccctgagttggggattggtttatcaaattctcgagcatggctctcatggtggcatttttatcagaaaggcaccacatattcaaagacggatctggagggagactagaccaagctgtagcccggtctagtcccagcccaagtccaagttgtttgtggtaatttttaattttttccttgaagtagccaggttaaatatttagttagcccggtttagttccagtccagccaaagtccaaaccccattctttatattttctttgcaggccaccagtccaatatctaaatccacttcaccaattttttaaaaccctcatattggctgaaaaattctctcgtctttctcatctctacgggcctcgccgagttgccgacacactttattctaggaccaggtttgcctcttaatctctttcactctttgtccttatataaattttcttcttgtcatttattctattttcaatttttgcaatatatcttaaggtttaagttggcagtgggcttcgagctaagaaattgaaattgaaattggagagtggaggtttttttttcatttgtgaattaattttaaattctttgaatgaaatgttttgctatgttttaattttattggttacatttacagagagttaactttctatgttttatgtataatctttagaagaaataatttattctttaattttttttctcagtttactttgtcaatgcccaatggggaatttccaaatctatgagcatgttgattgatggttgattatgtgtagaatggaaaattgtgttgtttttcctcctttttttggcgggtgggttgctagacaaaaataaacatctgcttagcaataaggaaggtttatgggtgagattcaagaaccatgcccgaattgaatcaagaaaacaggaccactgactaatttgcaatactattaaaagaatatttattgcattggttattcaactaacttagttaattataattaattattctataaagatctccaagaaatttaattaactagcttaacaaataaatattcaggttgaacaatctaaaatttgatcaagtaaaagtggacccgtgtgatgattttgcattatattattgttgccttgtctcatttttttatgtcccctatttttagcacttacaaatggaagatcaacattcatcgaagagaataaagacacaattttcattctttaaaaagaccggcagtcaatttagtgaaagtatatctccgaaaattgaacacccctcagcctcaaccccatgcaacatcctccaaatccagctcaagaaattgaacattccttagtctcaactccggaattgcaatcatgtactagtattgaacgggatccgagaaaaagaaagcaaatgtttgaacatcctggcaatctacgagatgagattagaattgcatatataaaagttggaccttatcagttgaagcttgaggagtatccaaggatagaagaaaaaaaacaagctcgtcgctttcaaaaaaaatgattcactgaatttccatggttggagtattctcctacaactgaaaaggcatattgcttttactgttttctttttcagaaagagggtaattcatcttcttgttcgggattgattactgaaggatataataaatggaagagggtgaaagatggaaataaatgtgcatttcttgttcatgctaattcagcatatcataaactgtgtgagactagagcaaaagatttaatcagaccatctcagcatattgacaaggtaatgaatactgtatcgaaagaagaaattcgaaaatgtcatttacgtataatgccttcaattaaaagtgttcgatggctagcattttaaggtttagggttcagaggtaatgatgaatctccatcttcacgtagtcgtgggaattttatacaactaataaagtacgcagcatatttgaatccagatgttattaaagttgttttggaaaatacaccacaaaatggccaatacattgctccaacctttcaaaaagaaattttgcatattatggccaatagagtttgacagatgatttgacaggaagttggggatgaatgctttttgcattcttgttgacgaagcacaagatgcatctaatcgagagtagatggccatatcttcaggtttgtgaatagtcacggtagtttgatagaacatttctttgcaatcaaaagagtcagtgatactacttcatcgaatctcaaaaatgaaatatgtgatgttcttgctcagtatgaactttgggtaaacaaaatgagaggacaaaggtatgatggcgctagtaacatgcgaggtgcttggaatggacttcaagtattgttttttagagattgtccatgtgcatactatgtccattgttttgctcatcgattatagttaacattggtcacggtagctaaagaagtccatgtcatttggaacttctttcctcatttggacaagattgtcaatgttattacttcttctcctaaacgagttactgagttgcaattttctcatagagagaaaattcaacgtatgttggataccagggagcatgaatctggaagtggggctaatcaaatggttaatatgcaacgatcgggagctactcgttggagctcacattacaactctataaagagcttgatagatatgtatggtgcaacccgcaaagtgcttcaatagatttgtcatcattattcaaatggtagatctcaagttgaagctcgtggtgcttgcaaaaagttggtgagatttaagttcatatttatcttgcatttgatgcatagaataatgagaatcaatgatgttttttgtcaagcccttcaaagaagatcccaagacatcttgactgcttgaaggtttgtgtctacccctaaacaattgcttcaaaaattgagagatgacgattgggaagaatttcttcaagaagtaaaatccttttgctcaaagaataatattacattacccgatctagaaggtttgtataaaactggccattttagtgatgaaactacaattgaacattattattactatgatgtttttaatgaagcaatggattttgtaacgatggagttaaatacaagatttaatgacatatcagtagaactcttttctctcagtgcagctttggatcctaaagattcatttagatcgtttgactgtcgaaaaatttgcacacttgtagagaaattttaccctcaagattttttgaagcaagatattattacattggaatatgagttgccacattatgagttagatattaagggtgagtctcgatttcaagtatctacactttctgagttatgcaaatagttgactgagagtggaaggtcggagatttacattatgatgattagattgattcgtcttgaattgacattacatatttctaccgcaagtactgagcgagtattctcaacgatgaaacatgtgaagacgacacttcgcaacaaaatggaggatgattttcttgctgattgtataatactttttatagaaagagaacttgctgagaaaatagatctacattctattatagatgagtattatgtttcaaatcctcgtcgggaatgacttaaataaataatgttatttaacaagtttttttagtatgtataaattttattatattcactttatcaagtacttccagtcccctctatgaaaaattccagatccgtccctgcacattcatacccatatctgaccagtctatgtcagacaggctaccttctgcttgttcatgcagtgttagaggattcgctgtttgttttccaggacaatttgcttattatgctgccctttttggttaacattactctccaaacgggtcacacaaacatacgttgttttcattaaatttcataagaacacttccaatgagatgtaaaatttgattttttctagtgaaggagaaaactattgaaattgatatatatctatcaaatttcatatctcaaaacccaatatccatccaaaatcttactcaagtatctttttggaatgtcatgcatatcttagagatacttctctttcttaatagacttatgttcccaaactctattatcaagaacttatatagtcgattataagtctaagataaccaatatttggtaatctacacgtcaaaagtctatatattcagaaggtgctaacattgagagaactccattaactgacaggttgtagttaaccaacattctttcttaaaaaaaagaaaaaaaagaaagaaacatgcacaaattggactgcattatctcaagcctcatcatactcaacaatatcccattctttttacccaatacgtcatatagtttttcatgaacaagttggtgaaaaagttatagttaatccaataagaatttctctttcattacatagattattgaacccttgtgattgagatccacgctcaaatattcagaaggtgctaaattgagagaactccattaagtgacaggttgtagttaaccaacattctttctaaaaaaaaaaaagaaaaagagaaacacacacaaattggattgcattatctcaagcctcatcatattcagtaatagcccattctttttacctaatacgtcatatagtttttcaagaacaagttggtgaaaaagttagtcaatccaatgagaatttctctttcattacatagattattaaacccttgtgatagagatccacgctcaaatagttcttgatgccttcatttccataatctgattttccactccacttcaaaagtctaaatcaatacagtatcttcaacctaacaaaaaaaaagaatcaaaggcacaactgaaatgtgtaaatccatctataaatgtaatgaaaaatgatgttccatctctatcccttttaatcatagaccactaaaaaaattcaaatggatttacaatatggaagtttagcctttgcaactttgaccattgcataaatattcaaaaccataataaacatcgtaactgtgaatatgaatagaattaccgtacaatctttgatagtctcttaatatcaaatatgaggtcagtttctccattttgcaacactaagttgcggtgtcaatcatataaatctccactccatctttattatttgtatatatctaatttgtatcaagtcaaatactcgacaatagactaaaaacactctaactcttgaatccactatctacccaagataaaattcaatatgtacaatgctaagacataaacaacactaaaaggaaaatattcaaatgcaatattctttagctcaactaattccaagctaagaaatttaaaccatatgatagaaacacttgaacctttataatattagatctccaccaaaaccacttttatgtactatctatatgttctccttggtttcttttctagtcttgtcacctattctgcatttgttttagcttatttaaaacttaatattggaagttttatacgaactaaaacattgccacacaagtatgtgctcaagatttagtaacatcaagttgcacttctttttaacttgcacaatggatagtgtctatagagaaaattgatgcttcaatttgtaaatcacaatgacgctcaaggtttccatcattgagaagagactaatttgaagttactactcatctaaaaaaaatatgaccaacgaaaagtcaacactatgttaaccatctcaactaagtcacatttcaaaaaaaatcatctataatataacttaacaattcaaatgctcaaacattagaatctatattttctcgtaattttgatctttattctatgaagtaatatctttgtcaccttaagagatacttgatccatcaatctaaactttattaagagttatagaaactcaaccatcctttgtgacaactagcacttataacttaagggagagaataaaagaataattaagtgctgaatcttaccgaataattcattttttccaatagaatttcagatattgaatccctaattcattcgacttttttttatttcagctaatgccactaatttggattctataattgagtgagtaatacatgtttctttcttgaaaatccaagaaaccgcacatcctgtaagagtaaacacccaatctaaggtggatttattctcacctacacttgatatccaattagcactggtaaatccttctaggcttgatggaaatttagaatattggagacctatatccttggtttcctcagataaccaagaacacttccaatagccttccaatgtttttcatttgaatcactagtaaacctactaagtttactagtttcaaatgctatatcgggttttttacattgtaaagtatacgttacacttcatataacactttcatactcaagttgtgctattgctcttccatcattcttaacaagtctcaaactttgatcaaatggggtcttaacctctttaatgtacgagtgtttgaacttattaatcacattctctatataatgtgattgactcaacattaacccccactagtcttggtaattttgatacctagtattatatccacttgactaagatttttcattttaaatgtggaaaatagaaacatctttgtttctttattccttgcattctgattagtgtctaaaagtgcttcaaagatatatcatttacaaaggcattttacattcaatttgtttaaatacactaatgttagtctctaatttcaattctcttgcagtaaattcaattttcataaatatatggttaaaagtgaaattaaacaaaatatgtatttaaatacatgtcggcataagtattatacatttgaaagagtagttatttgatgtattttacatgtatttccaatttagaacaagtggagcaagtggaggaaaaaaatgttgaaaactcaagaatagtgaactgtctcaagcaagaagcagctgtcggtaaaataatcataacttgagctgcagacatcgaaccacggtgattcaagttgggttcgaaagtaagatacgtatctacaacttttatgtctgccaagaattcaaattcatatcacaaggcagccaaaattatcgtgcaaagttcagcttgttacctgtcggatacagcttttctacctgtgaagcagcactcattgtttttgtcatatctgaagttatatagatccaatgaacctgatatttgcaccaatggaaagctaactcaaatagaaataatttatctgctaattataagtccaaattcacggcataaggcatctgaaaatttacatcaagttgcaggttctagctgtcctgaagctggacagaaacaagttacattgtccacttgcattttggatgttcctttgcctataaaaggggaccttggccaagattttgagagcatcagttcctcttcatcatattctagttttcttcattttctttgtaacatttcattaggtatttttaaaccattagctagaggtaggggtgaaactttggtgaatgtgtagtattgtctttgatctttcactttgttctccaatgttcatcttcttacttggttgaagtatatgttctacaaatggtttttggtttgttaaagactttgatttattgttgacaattttggcacaataaatgcttagataatctccacataccaacaacttattttgacatattctctcaaacaattatcaagatctatcttttagtgtatttgcgattaatgttttatcttccatatttcatatgagatgaataaaagatcaagaataatttctacccatttatccgaagtgaatccccaatgctctagtgttcttctcaatcgtatttccaccaaccatttaccactcatagaatagtttattccttccaattccctgtggttcgacctcggacttccaagtttactacttgcgacaacctgtacttatgtttgcaaccttaaagttgtagcaagttttgacgctgttgccggggatttgcgtcaaggattattttctgctgttttctatgagattttcttctctttcataatctttataaatcaggtacactcgttcctttttcgatcttagtacattagctattttactttaaaggaaggcggagcctccttcgttttttattttctatttgttttctttctttaaagggaaggctgagcctcccgaactacctttcctttattacatggttggccatgccacctaattttcgttctttacatctagtttatgctattttatatcatattggtatcgtgaatttacttctcatcgtttagttaaagataattgtgaaaccttctttagtaatttatttgactcacctcaagactcagtcacatcttccaccatggctgataatgaaaatgtacatgatgaaaatgaaaaccaacaagcacgaaccatgcgtgattacttgcaacctccttgaaattctgctccttcatgttttattttccctcttaatgctaataatattcgattcaagccaggtatgattcaattacttcctaatttttatggcttagaattcgaaagtccatatttgcatcttaaagaatttgaggaagtatgtgccacatttaacgatcaaacttgcccccaatgaaatttttaagttgaaattgtttcctttttctcagaaagacaaagcaaaaacttggcttaactctttaaaagctaggtcgattggcacatggcaagaaatgcaaagtgagtttctgaagaaattctttccagcacataaaactaatgatttgaaaagataaatccaaattttttctcaaaaaaccaatgaagtgtacttttaatgtttagaaagatttaaagatttgttaaatacatgcccacatcatggttttgaaaaatggcatactataagtttcttttatgagggcttaactcctgaaacaaaacaatttgtagaaacgatgtgcaatggtgaatttttagataaagatccagatgaagttttagaatttctagatcatctagctgaaaattctcaatcttggcaaacagtaaaaccaatcgaaaactcaatcaaatctagtcttgctagttctagtggaggaaaatatcaattgagttaagatgatgatctaaatgctaggattgctagtttgtctagaaaggttgaagctgcggaattaaggaaagtaaaggaagttaaacccgtgcaaaatgatgaaatttgtagcatttgtgaaacttttggtcatctaacgcatgattgtcctaacatcccagttttcaaagaagttttacatgatcaagccaatgctatgaacacttttaaaaagccttttccttctccattctcaaaaacatataatcaacaatggagaaatcatcccaactttagttggagagatgataatcgtgttcatatcacaacctcaagggctttcaaaatttccttcttttccaatcaaagactcttgaggaaacattgcagtcattcatgcaaggacaagcaaacattaataatcaaacttcacaggccatcaatgaaatcaagaacaaactttcttcattgacctcttctttgagttctcaaaagaaaggcaaatttcctgctcaatctcaaccaaatccttctgggcaattcaatgtaaatgcttctagttcctctgaaagtcaacaagaaaatgccaactccatcacgactcttcatagtggaaaaattattgagaaaactatttcttcaaaaaaactaaaatcaagtggaacttcaaagcaagaaaatgatgtttccaaaactgaggaaaaaatcatttctgaacctagtgttgaaaaatgtcccgttccagctccatttcctcaacaattgcaaccaatttcaaaactcaaccaaaattctgaaattttttaacttttcaaacaagtcaaaattaacgtaccattattggatgcaatcaaacaagttccttcatatgcaaaatttttaaaagacttgtgcactgtcaagaggaaacttaatgttcaacaaaaagagtttctgatagagaacgtgagctcagtcattcaacaaaacactccacctaaattcaaagatcctggttgtccaacaatttcttgtgtgattaggaataataggatagaacgtactttgcttgatcttggtgctagtgttaatctattacctttttctgtgtatgaccaacttggtttggcagagcttaagccaacaacaacaacacttgaacttgctgatcattcagtaaaagttccaagagggattgtagaggatgttctagttcaaattgataaattctattatcctgttgattttatagttttggacacacatcctgttttaaattcaaatacacaaatacctgtcattttaggacgtccctttcttgctacttcaaatgcattgataaattgtagaaatggtatcttgaaactttcttttggaaatatgaccatggaaatgaatgtttttaacatttgcaagtaacatggagataaagatgatttgcatgaagtaaattttattgaacaatttgttgatgatcagtttatcgctacatcttcatctaatgtgctagaatttgaatttaacgataattctaaaaattcgcatataatttctttgttaaattctttttaggagaaaaacacaagtgattggaaatcaaattttgaaaaattataacaacaatctaatatgtccatgatttcaagtgttcaaatgttaaagctcgatttgaagccattaccatctaatctgaaatactcctttttgggtgaagatgaaactttttcagtaataatttcttcccaacttgatgcgcaccaagaaggtaagttgttaaaaactttaaaaatgcataaaaatattttaggatggaccatagctgatataaaggggattagtcctttgatttgcacacataagatttatttagaggaatatgctaaacctacaagagaaatgcaaagaaggcttaatcctgttttaaaagaggtggtaaaaaataaagtcattaaactcttagataatgaaatcatttatcctatttctaatagtagatgggtaagtccaaccaaagttgtaccaaaaaatctagtgttaatgtagtcaaaaatgaagaaaatgagataattccaactagaactgttactggttggcaaatgtgtatcaactataggaaacttcaacttaacgagttggaagaaattaggaatgaagcttatgagaactctcgaatttataaggaaagaatgaaggtattccatgataaaaacattgttagaaaaacttttgagccttcccagaaagttcttttgtacaactaaaggttacatttatttcctggaaaattacgctccaagtggactggccctttcattgtcaaaattgtttacccacatagagctatagaaattgaaaatccaagtaatggaaatatttttaaaagttaatggacatcatttgaaaccattttttgagaatttctcaagattaaaagagtccattgctttacatgatcctaaagattgatatcattttctcattgttttattttgtatgtttgttttcaattttataatgttgtgtgtttgttttagatgtgtttgttttattatcattttttttcttctctaatgaaattgaaggatcatttaggctaagtttatgcagactttccaagtaaagctcaaaacccatcccgttgctcaaaattttgctccttactgtccttcatctattttgcacgtttaatctttgcattgaggacaatgtttcatttaggttggggggaaaggaatcaaaaagttcaaacaaaaaaaattcttaccaaccgatgataatatttgaaattgtttttatattattgtgactaggggatgctgctttgatttagtttaagcttgttcatgttagattgatttacattgagcataataatcatgaaaataacatattatttagattggatcaatggatagaatatgtagaattaactatgaccaaaaaaaaaattcctactttaggatagtttgggatggttgagctgttgtagggagacattgagataaatatggattccatgtgtgttaaattttgtgtggatcgcttaagaccaatgagattataattaggtgaaaatcttaagttaaagattgattttcaagaataagtgtttaatgaggggcattgcactaatcattgcataaaaggaaaaaagctaccatgttgtgaagctaccctaaaaagcccaatgagtataattatatacataaaaagagattaggctagtgcaagaaacagaatacacacggcaaacttgaagggaaaaaaaaagcaggtgtatgaaatagaagacgcactacatgctttgattaagtcccaaacacttattttagagaattggacctttaataagagattagtatcttatttgattcttggaggttgaattagtcaaaagtaaggagaatcctcatttattgatgtgttgagctacaattagtaaaatataaccaaactagagagggtgagtaatagtatataaatttaaccataaatcacaccatgggaaatagttacaaaatcaagtttgagagtgtgcatcaagagagaaacaattgaccactgaggcttgggatgaatccaatttgaaaaagtatgtaattggttgaattgattatgcacacacacacgttggtcgagcattgaactagttagattatgttttggtagcaaaccttagatgtcttttgttaagcattttcaaatcctgagataagtgcgacaagctatttcatttgaagtaattttgaaattttaattcaatttccataaatatatggttaaaagagcaattaatcaaaatacgtctttaaatacatgtcagcatgagtattatatatttgaaagagtatttatttgaggtatttgacatgtatttccaatttagagcaagtggaggaagaaaatgttgaaaagtcaagaatagtgaactgtctcaagcaagaagcaactgtcgataaaatgattataacttgagctgcagacatcgaaccacagtgattcaagttaggttggaaagtaagatacgtatctacaacttttatgtttaccaagaagtcaaattcgtatcacaaggtagtcaaaattatcgtgcaaagtccagcttgttacatgccggatacagcttttctacctgtgaagcagtactcattgttttgtcatatctagagttatatagatccaatgaacctgatatttacaccaatggaaatctaactcaagtggaaataatttatctgttgattataagtccaaattcacggcataaagcatctgaaaatttacatcaagtgcaagttccagctgtcctgaagctggacaaaaacaagttgcattgtctacttgtattttgaatgttcctttgcctataaaaggggaccttggccaagattttgatagcatcaattcctcttcatcatattctagttttcttcattttctttgtaacatttcattatgtatttctaaaccattagctagagctaaggatgaaactttggtgaatgtgtagtattgtctttgatctttcactttgttctccaatgttcatcttcttacttggttgaaaaccaagtaatttagttcttaatgaatttaaaagcacataccttcgagacaacgcatcagcaactatattttcattaccttgtttgtacttgatgacgtatggaaatgtctcgataaactccatccatctcgcatgtcttttgttcaacttaccttgacctcacaaatgctttaaagattaatgatcggtgtgtatcacgaattcctttggccataagtagtgctgccaagtctctaatgctcaaataagtgaatacaaatccttgtcatatgtcggataattcaatgctgccccactcaacttttcgctaaagtaagcaataggtctcctttcctccattaacactgctcctatacctattcctaatgcatcacactcaacctcgaatgttttatcaaaatttggtaatgccaaaacaggtgctttacataacttatccttaattgtgttaaatgcaatttcttgagattctccccaatggaaacctacattcttctttactatttcgatcaacggtgtggtgatggtgctaaaatctcttacaaatcgcctataaaaactagccaatccatgaaaactcctaacttcagttatagtcttagatgttggccattcttttataacttttatcttttcttcatcgacttccaccccgttagcactaacgacaaatcctaggaaaacaactctatccatgcaaaatgtgcactttttgaaattagcatacagttgttcctttcgcaacacaacaagcacacaatttaaatgttctaaatgcttatctaggtttttgctataaattaagatgtcatcaaaataaactacaacaaatttcctaataaaagcattcaaaacatggttcattaaacgcataaaagtgctcggtgcattagtgagtccaaacggcataactaaccattcatacaatccatacttagtcttaaacgccattttccattcatcaccctcccgcatgcgaatttgatgatacccactcttaagatcaatcttgctaaaaatgcaagcacgattcaactcatcaagcatatcatctagcctaggtattgggtgacgatactttaccgtgatattgttgatagctcggcaatccacgcacattctccaagtcccatcctttttaggcaccagcaaaataggtacagcacatggattcatgctctccctaacataacctttgctcatcaactcttccacttgcttttgaagctcctttgtctcctcgggattgcttcgataagctggtcgattcagtatgacagctccaggtacaaagtcaatctggtgctcgatgcctctgattggtggcaatgcacttggcatctccttaggaaacacatcgtcgaactcgtgcaataaagacttaaccaaactagggagggatgtgttagaatcctcaaaattgaggagggactccttgcacactagcaatatcatttgcctattatcgctcatagcctttttcaactcactctcctttgcatagaagttgacctttggcttttctctccgctcagctgactctttttctctcctctcaactaactcattttctctcctctcatgtggcttctctctcttttctccactctcagccacctcactattttctctcttattgatggtttcactattgcctctcctttttcctgactctcttattctcttgtcttcctcacttttcagcttgatttgatctccatacacttgtgccggtgttaatggcgcaagagtaatagtctttccatccttgacaaagctataacgattcctatatccgtgatgtgtgccccttctatcatattgccatggtcttcctaacaagatatgacccacatgtataggcaccacatcacatactactttgtcactataactcccaattgagatattaattaaaactcttctattcaccctaacttccccactttcattcaaccactacaacttataaagcctagggtgtcttaacaatgctagtcctaatttctcaactaaagttgtgctagctacatttgtgcaacttcaaccatcaataatcatactacataccttatcgttgatgtaacaacgtgtgtggaatatattttcgcgctgctgctccgaatcatccactttgacttgagtgttaagagctctccttgacaccaacgatttcccaatagcaaactccaatttttcttcttcttcaacgtcctccaatgcaggcatgtcctcaaactctcattcactttcactcaccacctctccattatccaacaacactattacccgtttatttgggcattgagaagcaatgtgccctgaccccaagcatctgaaacatttgatgtctcgattccttgatggttgtgaatttgttttaggtgctattttgctagtactttcttctttccctttctgcctctcattcctgcctttaggtacaactttatcacctttgtggttgttgttccaccctggcttccaagatggattaacaatcgaagttcctaacggctgcctagctgcccctttcctctttagttgtctctctaccttcatagccacatgcaacatgtcttccaactccacataatgttgcaactccgctacattggcaattttcctattcagcccattcaagaatcatgccatggtagcctcctgatcctccaccacattggccctaatcatgagtattttcatctctttatgatagtcctctacacttttcgacccttgatatagaccttgcagtttttgatggatctctcggtaatagtggctaggaacaaacctctttctcatcaatgacttcaattcctcccaagtgctgattggtcttcccccactcctacgttgtgaagtaatcatttgatcccaccgtgaaattgcatagtcactgaactccaaaaatactaacttcacctttttctcctccgagtagttataacactcgaagatcatttcaaccttccgttcccactctaggtatgcctccggatcactccttcttttgaatgaaggaactgtcatttttatatttcccaagtttccatcaaactcctccctacgatcatttcgaccccgtatgtcgaacatatcgcctctattcctcatccttcccatctcaacaccgtgaaattcatcttcgcccctccatactcctctcgcctttccctcctaggctcccatctatccggtcctctggcattggatacatccactcgatgctcccgactaagattagtcaccgatgtatctaatctattcatccaagcctcctgcttctccaacctatctctcaaatctccgaacgctctctcaaacctctgcaccaaatcctccaatgcattgttattattaccttgtcggcttaagtttgattatgccctttctgacatcctaacactaaaaattttattttactacctcaccaaaagtcactcggaaacacacaagggcttttaccctctattaagctcacctatccgccttttaccactcagttctttcaacaattgcttctaggaacaatcaatgaactcaatcaatcaatcaaatcatgtagaatttcccaaaccggatgtgactcaatatttataacaaaggactcaaagaaaacttttaaaacttgacttaagttgaaggaatggaatgattcaatgtgtccaagtaatttagaaacgatattgaataataatagttgatatttgacggattaataatatttaaatttttttttactgtacgaatgaacagtaaaaaaattttcagatccgaaaatcaataacaaaatcaacaaagaaaacgaaaactgatttgggcgaaaattgagcccagaaacgaaatttgaagattttttatgaaacttttggatcaaaggatcaaaaaaaaaaccttctggacacaagaacacaaggaattgaaaaaaaaaactagaaaacaaaggatataacctgattaaattggggccaaaactctgataccaactgatgtgaaccccagagcaatgcaaactacgaaacccacaacgagattgatgcggaacccaagaacgccaatacaacccggttttggatcttgaaccccaagaattgaactaagaaatcatagattagcgaagaacctaaaaccccttgattacatttaaaagaacccacaatctgattgtttagaacgccacaagaaattgaatcttgataagttccaagattgtttaagaagaacaagaaattgaaaaaacaaattctctctctataatattactcaagcaaaagtcaaaaagtccttacaatgaaaagtattttcctatttatactaatgagtaaaaacgtcaaaacccatcaaattatggtaataatttgatttcataagaattctatcaaaactagaaaattcgaccaaaattagaaaattcgccaaatttttggcttgtgcggccgcatggtgtatttccatgcgatcgcatggttcaacaagaaatgccatatttattttcggtacgccaccgtgcggccgcctaatgttcgcacaggcttgtttttagcctctggttcgttgcttgataacaaattgagccaagttgattcggccttcgacccgaacatgaaagttgctccattttgagttccgaacatggttccatcaatggtttcttgaaagagcaatcccatcacttgtttcacttgcttttcccttgatcgcgtcattggtccgccatcgactatcaacgggtctcgtctcgcacttgctttcgtcgggctagactcctggatcatatcagaatgtcattttaacatacatttgatgtatatgtaaatcacagatataacctaaagtgaataaaattcgaattgatgttatttgtgcaaccagtgcacacatgtcaaagtaatatattccttcttttttgttgatatcatttggccactaacgtagctttaaaggtattaaaagtacatctgcattgtacttcttcctaaatacccatttgtagcctatagatttcaatccaaggagtaaatcaactaattttcgagtatattttgacattgttgaatcaatttcatcattcacagcatctttccaaaaaatgctatctagagattatgttatttcttgataagttttaagattgacttcttctcaaagaacatacggagtagttattgtgatactcttctcatttccctaaaccaaatagaaagaaataagttgagagtcaaattcatccagtcctagcatttaatcctttatagctcttttgcttccatgaagttcacttattccaacatccttgaaagatatttctactcatgatattgcaaaactaggaatctccactaaaggctcccttaaagaattattatctaaagataacaaattctcaaatacatcacaagattcaataatgacatttgctttcaagtttaataaacgatatgccttgctattttgggcatattacaaaagtgaatttaatccctctaggatccaacttagtccttttaggatctcgttcttactataagcatgacacatccacactttgaaataatcaaattttggttttttctatttcaacaatttataaggagaaaccttaaatcatttaaaatgaatcctattaactatgtgacatgcacttaataaatcttcatctcacaaattatatggctatttagcacttaataacatagcatttatcatttcaactaaagttctattctttctgtcagccaaaccattttgttaggggtgttttaggtgtattatattgatatattatgtcgtgttgttcactatgaagattaacttcactagataagtatttacctctcctatcatttctaagaattttaatctttctatttaattaatttttctacttcaaatttgtatatctttaacatgctaaagggttcatccttatgtttcactattaccttctctgattaacattccatttaattcacatatgtcaaaataaaataagtccaataaattagatgtccttttaacactatgaaaaggtttattaatcattttagacttaacatattattcactattattatgcaatttgcttccacataatctaatatcattcttttaaaactagaatatctaatatgtcctagtttatgataccataaagaaatagacttatcaacataattcatttgtggctttgttaatatcattgccaatagtataaaatttaaatattccacactagaatagcgttttccaataaatacaccattccaagaaagtacaagtttgctgaaatcatatgtggacttaattcctggttttcccaacaaatcaccacttataagttttctattcatatccgatacatgtaaaacatttactaacatgatcttcttgtcagatgtgaattgtaagtctacgcttcctttgctaacaacttttgatttaattttattccctatttgaatgtcttcattgtccacctcttgacatattttgaagagggatttatcatagcacacatgtatggtggtacaagtatcataccactgtccttgaacatttcctctgaccaaattctcaatgctcacattagcaatgatgttgtgaatggagtcactttgaattcttgtattggccgtttgtcatgtctacaatctagtgcataacgtccaaattttctatacacaagaaactttgaatttgtttttgtttttgttatctttgttggggtttgagaattttctcttcttgaaatccttgttgtatttatttagttgatccatggcattggctttaaaagtgctctcatgagaatgttcattctcatctcgtgccattgactcttcatcaatgcgaagatgtttttgaatatcatccaaagaacaatttcctggacttgtcctaacgaaggcaagttatcaaaaatttgaaatcaaaatatttagagattagatatttttggtaccttctttctcagcattgtatttgttttccaacaattcatatatctccattgttgaggtaatgcttctatggacgtcataaaggtgatcaaaaagagtgtttaaaatgtgtcctctacctattaacttaactttttgtctcttcttccttttcgcccttatttcatctgtgtcattcgaggttagttcctacaatggtttcaattttgaatctaatatgtagaagatattcaaagttgggagaagaaattttaacttgtcattccatcttataaagttcgacccgtccaatctatcaagcctcaaaaggtcatgattcatcatgtttatcatagccatggttgtctcgttttccatattaagaatatcgtttgagattgttgaacaaagttgatgaagaatgaagaaataaccaacaacaaaaaatggccaaaattgaaggttcgaacatgattataaattgttgtcctcaaacgatatttattgtaattgggataagtgattcaatgctttaaaatataaatattatgtaggagtagccaaaaccttaatccaagtttgaatcaagtaaaaccaaacttggaaatgaacttttaggacaaatatcgaaatttggtttgatcttttgatttgaaagttagcatttgtttttctcccgtgaaattataatttatttttctcttcttatcgaccacatatcccccaataaaataatattacaatgaaacccaaaacttttccttcattttaacctcacactcttcaaaaaattaccgtttcgaaatcaaactcgtgggggctacaagccacaaatgttcaaattaagcagccttttatgcattgaagcatattgaaaatacatatgttacaatacctaatcatgaaaagaatcatgtgcaaccttttgggagtgtaagaattttccctgatttggttatagataatgtgttatttgttacccgactcaagttcaacctgctcagttagtgctttaaccaggaagtcaccgctatgcatcaagtttctcattgattcatgtgtaattcaacatctgcacacattgaagatgattggcaaggatagaaggactgtagatctccacgtcatttatgttagtttctgattcagttcaactttcccaaagtgttaattcttattcttattcgatagtcaataatgtaactgatcaattttggcaccatagacttggtcatttgtcattttaaaagttgaacctgttaaaagatcaattatagtttgttttaggcaaaatgatggtgttgtaactccttgttttatttgccttttggctaaacagaggaggctatcatttatctcaaacaatcatttatctgctaatgcattcaatttgattcattgtgatacttgggggcaatgtcacattccaacacatgctagccatagatactttcttaccttagttgatgattgcacaggttttgcctagatctatgcaaaatctgatgttaattttattattccaaagttttttttttctctctaatagaaactcaattccacaaaaccatcaagaagtttaggtcaaataatgctcaggagttacagtttacagattactccaatgccaaaagagtcaatcaccaattttcatgtatagaaagacctgagcaaagttctgtgtttgaaagaaagcatcaatattcttaatgtgacaaaagccttattttttcaatctagggtgccaatccaattttagggagaatatgtgctcacaacctacttttttattaatagaaccccctcaccaattttgaaaaacgtgacttacttctctatgttgtatggtagtccagtagattacactatccctaaagtatttggcagtctttgttttgcatccacactgctatcccacaaaaataaattccatccacgagttagagcttgtgtctttgttcgctatcctcaaagcatcaaaggttctaaattgtatgacatcttttctaagtccatctttgtttctagagacgttgtaattcatgaaaatcacttcccatttcacttcataactcatacagcttaatcattgacccatttcctgatttagtcctgcctcacattatgccaaatttgtccatccttcacttatattgtaacaccccaaattttcataaactttgaagcatcaccaaaagctcacttttgtttgttttaaacacaaaatgataaaaataatttttttaaaaaaacttaccaaaatatctataaatttaaactaaagatctcaccacacttatcttatctcattccgtgttgctcacacctcgaaaacacatatctcttatcattgccaaccatactcacttgactaatcactcaactcatgtctgactggcaggtcacaatagttcctgaaaaagcaatagttcgacccaaccaacacctagaggggggtgaataggtgtttatgcggaattaaaacaattaattaactgatgcaacaagtcacatcaattatgcattgcctagattcattcacatactctatctacctaagttgaattaccggttgaaaaataaataacagaaagcagtaaaaacacaacaaaatgttgacggagaaaacccaactgggtaaaaactccgggcacaagccagtaaagatccactatagaagatattgacttacagtacgtcagacattattgattctaacaatattctgacctccttactgtatcgaccacagctatcctggattttgcagatctacgccaaaatcccagctttgaatatcttctacctcctgtgaatcaccaagcactctagcttttcaagcaatttccttcccggattttcaaacagatgatcttctggaagtttatatggagatatgaaagggtgttttggttttgtgagggttgatatttttattcaaagaatcatgagaatcaaagatgaaaagaatgaatttattttggctcttgatcctttggaagttgagaggaattgttgttttaatgtttgccaaaggtcacctaatgaaaatcggacgttttgtttatatagtaggtcgaatttggtaatatggagcgttaaaaattcgcgaggcattaaaattaccaaaggccagataacacagtcgctcgagcgaggtccttgcgaaactcgagcgacgtaccttcgctcaggcgatagaccagcggaactccagcgaggtcagttctgcaatttttgctctagcaaggtcagggcgaaactcaagcgacatcaacgcgccgtttgcatcttcaaagcatcccactttaccctagacctatgctatgacctttactaaattgcaactttagtccctgaactatttgacctgtacaatttagtccttgactttacaattttgacaaataggtcctttggtcacagattgccaattacacattttcctaacagttcctaagtccacgggataatcctctatcactacatcacttcttccaacctacgtagataatgggtctccacctaatagaagtgatagaagcatctctctcatactccatttgatcagggtctctttactgataaaggattccagacatttaatcacatctccacccatgatctaaatgtcacacaatacatccccgatacaaaccacaatgtacccctagacatctatactccacctcatcaaaagacatacaactcaccactaatgcatctcaaactcactatggcaaatcaacaccgtttggagaccacaaaggttagggctcaatttaaattggcctacgtaccacaggttactccaatcaccaatgctcaaaaaatccataaaggaaatgacgaaggtagcactcgtaaaggaaagggttggtcactacaaaagatgaagaagataaccctacatggctacctcaaacaatctcacaaaccacaaaggctcataaagataaaggataaaacggctgcccatctttcttctcactactacgctcacacaccattcatagagcaaatagagtacgtcacaaaactcaacccactatgcatgcgaacaattacaccaagtaataagatcactttaattcataaaattaaacacatcaaatgtattgaaagtgtaactcaccaacgtaacaaacttaagcaatcacatgcatgcagaaagaattacacacatatgcaaatgcagtaaccaggtttactctaactaaacctcgctagagtcatcactcgaccctaaagccaaatttgtctcacctctcatcttatccttcagcttatccttctagttgggacagtctctaataaagtgtccagacttaccaaagttgtaacaccatctaccactaaactagtcccgtcccttgtccttcttcttacaaccataatcactcgaatcactactgtcttgagttctacccaaattcatttgcttaaactttattctattactcatcatatgtacttcgccactcatctaatcctctatttcagtcttaatctccatctcattacttctaagcgagtctatgacaatttcgggtattaaggtgcccctacaacacttaattacattcttaacttatctacataaatcaattcttaacttatctacataaatcaggcatggacttaaataagataatagccttattttttagagacattttcatcacaattaacaatgtcttgaactaatttgttaaagacatctagattgtcatcaagatcatttgaagaatccattttaaatctaaaaaatgtttcaaacaagtacaatttgttaggagtagacttaagcaaatataagtccttcaactttttccaaagttcttttgtagaattaagttttccaacttttctcaaaatagtatcagataaatgaaagatgattgaagtgtaagaaagttcatcttactcttctttttgtgcttcgattaagtttgcaggaaatttgccatctattgcttttgaaacttttcgtcggactaaaatatcattcatcttttgttgccaaattgaaaattctcctttcccattaaaaattccaacttcaaagtgtgaagacatttttaagaaaaagaacaacaaaatgcacagataggtcacacaaagtaatcctaagagtgcaatatacatcattctagattctcggggtttcatacgattcacgatcttagatcaagagaatgtttgaatgggtcaagttcaggtgttctaacagggtaatcaatgcaatacgaaggtatgtaaacaaaagttcgaactctcacacaatgtagtaaattaaacacaaaagcagttattaacttgcaattaaattcaacacttcaaatatggtaaataactcttaaatttctaacacaagcaatgttaccccttcacggtaaccacaaacctaatgtcaccctacacgatgacacgctaatgctaaaatttaaactgagagagccaatataccagagcggaccaacctaagtctgtaaattatgagacacgcgaatttatcactttaggaccaccactatttgtcataaagtctcaagaaactatagcaaccaacaaaccacaattgaatcccgaacatttaaataacaattgtgtccaaattctactgtacaacttgaaatagaaaactttcaacacagaaatgctagaaatattgttaggaacaaaatgtctgaagacctcatagccagaaaagtgtcacacgccctcatgtgtcgagaagctctgtgcgctcattagccacacgtacttaaccgtcaggaccacctcaacatacatgtcatactagtggtctctgtttccccaaactcctactagattggtcaaaaaacacgaaaacacgggttgatttttgacagtattttggacagtttcttcaatctgtttctgcttcgttccagccaatttactggactattttactatgtttcacaagccaaaaccaatactttgaagctctgattccaaatgttgtggaagctctctctccaagaatcttcaattcggtggttttccagattcagtccaacatacctttctctacaaacaaccaaaccaaccggctccgatccacaatcaatataattcacctcgattgctattcagtcttacccacaacggacaagaaatggtgatgacttatggctaaaaaggctgggagagaataccataaagataggctgcgaaggaactaccaattacacaaagtaaacaattgttttggacacttctaggggccctttttcacacaccaaagggggtatccgaatttctcttatttttctcacaaaccacacttgaaaatagctagggttgaagtcttatatatattctagggttaggcttttaattggaccaaaagagaagtcaacggaccaaaattcaaaccatccaagagaaaatacgattgaaccgagtggagctcatggacttggttgttggacttatttcattcatcggcctatgcctatgaaataattaactcatgttaacatcgtagtccaagatttattggatatcaaaaaccaaacatgtacaattaaattttagtttaattggaaaagaggagccgtataccataagtcgtttcggataaggttgagtttaattagtagaattaggattttgtcaaaatgatgatttcctagttaaacacgtgcacgttcactgctaagaaaagacggaaattgggttattaatgatcagcttaaaccgtttttataattacattaggattgaatctccaaagtttagcataatcacaactaaggattaatattaaaccaaataaatgattaatatccatcttacacgtttcaagaaagagaaattgaattggattataactcatgtagaatttcatttatcccattttctttaaattgggtctaacttaatgtgttcttatccaaaataacattatctcgagaccaatacttctaattaattacgatctgcaaaaagggtccaatattgatatacttatctttgcactatcaaaatctaattatttgacccaaaaatatgagaatttagaatatatatcacttaggtccctcaatttgaaaatataaatatataacatatagaataaataaatcttatgctataaaattttcgaggcattgtacatctgtaacttcaacttttggtatgcattcagatagcaatatcagtgatcatatgcccaacgaattgcctgccattccttcacaaggactagatttcgaccatcctttctttattccaagaagatctaatagaatcagcaaaccaccttcttatctttgttaattcgattacaatcttctatcaaacacacttcctctagacaacagttcagtatatcctttgtgcaagcacatatcatataaaaaattctctccctcgcacagaacttacttccttaagatatcttcaaactttaagcctcaattctattataaagctgtataatttgatcattggaaagaagttatggcatctgaattggtagccatgaaactaaacactacttggtcagtaaccacattatctaaaggcaagcattccattggctggaagtggttttattaaattaaacgtaaacctaatggaagtatagataggtacatagcccgttgggtagccaagggttacactctgtaagagaactatgatggtattgttcgatatttttcatcattttgcatgtatttatttttttgttttgcgaatgatttgccgctctgactagtgtttgccgctgcgcaacagggatcgacctgttcgtttgacagttacttccaacagatgtgttcttcatttcaaaggacacacctattcaaacggttgtctcaatttctataaattctgggcgaattctcgtttgcaaaacacattaaaaaaaaatattcttctctatttctcttggcatcatcagttctttttcgagtgtatttttggtttgatcaaataatcacaatttgaatcaaacgcctcaattgtatcctgagagagattttttatcataccacagtcgtgacttcgttggataggggagaaacatctcttaaaagataacgtttttcgtgccttggagtttattaagttttcagattttcctatatttttcgcaacaggtatttcttgctatgatgatatttcttgctattgctgccattcaaaatggcatcttgtccaaatggacgtcagcaatgcatttcttaatggggatctatttggagaaatctacattgatttgcccttgggatattgtaaaacaaatgcaaaacttgcaagggatggactggactgctagtgcacaaactccacagatccatttacggctctaaacaagcatctagactgtgattttgtaagttttctcaggctcttgtttttcgtagttttcatcaatcaaaattagattattctttatttgcaaagggctctatggtgataattttgtcgctttatttgttgatcatatcattattacaggtttgaatcattgtatgatcgtctctttgacgacatttttgcacagccaatccaaactcaatgaccctagtaaactgaaatatttccttagtttgtagatagctagaactcacgaggggatattcttttcccaaagaaactaaacattatagcttctataaaaatttggttgcatgggttgcaaaacaactgctctatccatggaccccaaagctcgccttagttattttgaaaggatgttatttgataatgcatgaatggtgggaaagactgaggttggctggaacaagcgaggtagggctaggagggtgcaagcctcttaaaggtaaaaccgaagaaactaggtcaaaaattggtttcaataaaaacagggaacaagccaaagcttacctgttcgttagtgtagtcattggtactattcttcccgtagtattctacacatctatggcagaaagacacattcctaataccgcactcaggaaacatatatataaacttagccatatccttttttagctagaattatcagcttaatttacaagaaagcaaccttatgatttatgaatgaattgagtctctatccaaacgttttcattttctagttgtccaggtggaaaatctcccaggctgatagcaggtttggatacaagaaagcatcctctaaaggtcattcactctattcagaagtgcttacaatagttttggcaatagaaaagtgaatgaagcacaaccaacaagttagacattttttccagagtgccattcaaaattttcgtcaacttctaagaatcctttatttgatatgttacgaaatcaagaagccactccgattgtggtcctgctaccacgtcacagaacatgggttatcccaataactaaaggagcttcacttctgcatcctttggttgtaagtgtaagtgttatgccctaagtccaatcaactttggacatgagcgcttttaatatataacggatacgattttatggcatatttattatttaattaatattcaattaaatcaaataatagactatagattcaaatcttggtaatttgttaatcataagaagttgtgattgtaagatacaaattacatatgatcaagttttgaattatctgtggtcgtaagtaatgacgagatacggatatcattcttatgaatagaccatcaagtgtggtatttcttatttgtgaagtagctgatctcacaaagtaaagtgtagtgacacttaaataaacacgtggatgttttgttatagaacaaaacattggagacccactaagagattctacataaataacaatctgagtgtctgtggttaatcgctaacgttcaatagtagaattggtcatttgacttgagatcatcatagtgccttgtatgaggactgtcatactttggctgtgttgaatgtcgctttgtcaagagtcactaatacggcatcttcgggtatgtcaagaatcgtatgaaggctgtgaatgatcaacagaggattcgtcactcttagatagtaagagattatgatccatatttcatccaattaagtcgataacaaaatccttagacaaggtgtaatcagaagtcgaaaaggagtttttcgacttatattgatttaatagtggaatgaaagttatgatcgataatcgggattgacacacttccatatctcgtaattgatcggatcatattaacaaaaggattatagtttcaccgtaaactaatgattttgattttatcataccacgtgatattttttgtcacatgtattaccctgatacattgatagatgtcaatctgggatgacgaacatgggttggtgataaattaaaatggtgttttaatttatcgattttgattagatcaaaattattatacacatctttaggcattgtgatcgggaaccgatggatcgcacacaaaagaagaactggaagattgtgatttgtcaattaattaattgaacaagtgttggataaattaattaattgggttgcttatttataggcccgatttgattaattaatttacggatcaaatttaattaaatgggttaattaaatattgggtcgggtcaggccaagtctgtttgggcttatataaatacgtgactagtgttttcaatttgtagagctttcattcttgctaacaaaagagttacaatcttgctctctatgtaaaatttcattggagactagacaattggacagttgtgggtatcaaatcaaggttgttggaataaaagaaaagcaaatgagtttgcagattttgcaaaaggtataatttctattacaatttctatataaacacaaagaagatcctttgatgggacttgaaatctgctttattttccactgtgcatgttaagtaaattccgaacagtggtatcaaagcttactttgtatttgctagaaattatttaatgtctttgtgtaaccaaaagttgattgtcacaccttttccagtttctagcaattgacgaaatttgatgtttatattttgaaatctgattttgaaaataaaaaattttaggtcggagatgggtgggccagcaatactactagcgacaacacttgttaccatcgtgaaagggcttaataatggtggcagcgcggcactttcaggtgtagcactgagcgctgttgcgatcatcgctgcgatcacaacagcggctactgtacctatgcagtgttcaacactgtagcttgctgcggcatcgaacgttgttgcagctacagcctttgacattattggtgtgtggcagcatctcacctacaaggtgactcacgtcgccgctgcggctatatgcttgtttgtgctactgaggagcggcaccgcatgattccaaattctagggtacttcattcgcacgggctaagaatttaaaagtgacaggccctttactgcaatttcaattcgagttcattgtgtaattttaattgaaacgggcttgtttgcaattttcaaaattgtgaggccgtgcttataatttttaacttgggtcaaatttcaattttcaaaagattttgaatttaaataatgaaaggttttaaattttattttaaatgggtttgaccctaaaatttcaattttgacccttttaaaattttattcaaaattcacgacttttatgttatggttaaaattggattttaacttaaatattaaattgaccctaaattgaattttcttttatttaggagttttatcctaaattaaatatgttaattcaatttagtaggagttggaatctaatttaatagttaattaaaatttaattttaattaaataattcaccctagtatttcttgaaattagaattggattctaatttgacatttaattagaatttgattttaattaaattttttcgccctaaaatttttcttggaataggagttggactctaatttggtgtttaattaaaatatgattttaattaagtaaattcaccttaaaatcttggaattagagttgaactccaattttgttatttaattaacatttgattttgattaaattcaatctccttaagttttaaaattggagttgaactctaatttgatattcaattaaattttaattttaattaaatagttccaccctataattgtggaattaaagttagactctaatttggtataaaattaaaatttgattttaattaaatatagccgctaatttaattaattaattaatatgattaatgtttattagtggatgtttattaattaattagtggatgtttattaattaattaatatgattaattgtggaaaacatttatatgatgactgtttattagtggatgattatggactcaaccatgtggatatgctgattggttaatgttactcttgttattttatgggcctgcaagctcttaatttggatctgcgagtccattattattattattattattattattattataagcttgcgagcttttaatcattttggacctacgagtccattattgttattgttactatgggttgggagtccaattttatttaggcgtgtatgccaactagtataggatacaggttacagttggactaattgaagacacaagaagagaaagagaccattaagatagagcattgaatgatcaatgcaataccccctaggaattgaccaactagtcttcattatggctcgggaagattagataataaaagtccataatcgtctacactattatattatattatattatattatattatatatttgcctatttgtgtgatagatgtattatatatatgggattgctacgatgagacctttgaatgaaaaacccctcaataaaagattaagtcacattttatattcacctttcatcattatagtaaaaaattagagtcctcaatcgatcttggcttgttgagtacactcaaggctagtatattatgaatatatttgacactatgaaatattagatatttctaaatgatgggtccgacttaactaaattttatcttttattgattacactcaaggaaataaattttagagacatattaagctaacacataagatgtgtatagaaaagaagttattagcttaatgatctgaaagttgtataaagatacaattgataatagtatcaacccaaatattttattaagacttgttgagtacactcaacgtcttaatataacaaatgggatcctaccctgttgggagttaagtattaattccataaatttatgtgaggggataataaatttaagttaaacaattggaacataattaatttaataaaagcccatgtgaaattaatcgatgcatttatatattattctttttctttttgtcatttatattgaatcttgagtaatcatatgcatttaagaggcatactggatgccaacaaccaaaccaaattttcttgattgacactggaacctaagaattgttcttaggcataagaaaatttgttatgtccttgagtggccctttccagagacacctgctaatgactcgattaaggaagaggtggctgctataataaacacaattgtgacaatagtactgtaacatatgtgatgcttacaattatgttacttgagttataaaagcaacgtgagagtatagatgttaacacatgatttttttattttaaagagttgtgtgataataatcatgtgtggaaggatatgagactttcaagcaattatacgaatgcaaaatgacaaatggatcctcaatcgatgctcatatactgaagatgtttggcattgagaagttgtttcaatagtattgagctatgaactaagtatttacttagctatgcaatctttgtcgaggagttatttatgcgaattatgaattatgatatgaataagctcaaatgcacattcattgagttgcatgcttaagactattaaacccaatatcaaagttagtattgggcaagctattgattactttaagaatattatgagaaagtctaaaggggtttttgggaaagcatccaatatggctaagactgtcaaagcaaaggacaataccaaatttagtgacctttattttcattatagaatgaaggacattcaaagaaatattgcaaggcttatgtctacttcattagtttcttaggtatttgtaccggatgtggatctcatatttatataaatatggagaaactagatataagtagaccactataaaagggagaagttgacttacacgttgaagataagcaaagattgctgcattgcctgtaggagcatacttcttgttgttgccttaggcttagtattggaattagagaaatgttactttgaacccaccattaccagaacattaaataaatttcatgtttggacatgaagtattttaatgttaaggacaattgttattccttttattttgataagatcttaattgttgtggtaagctataaaaatgacatttatattttaaatgctaagcattttataatgagtatagaagttgagagacataaaaatgataatctggatgacatctaaatctagcattgcagacttggtcatttatatgaaaaaaaaattccaaaattacatagagatgtatatttggggtcaactaattttgaatcatttgacaaatgcgaatcttgcccattaagcacaatgaccaaatgaacttttacttgaaaggaagaaatatttgcatgattattggtctaatacatagtgatgtatgtagacccatgtcaattaatgctagataattttctcttatttcatcacatttacttatgactatttcgacaatggccatgtatattttatgaaattcaagctagaagtagataaaaaatatatatgtaaaaatattctcacactaagatccaatcgagatgggaatatcttaaagatgaaattctagattatctaagagagaatgagattctcttacagtgaactcctccatatacactataacatagtggtgtatctgaaaagatgaatcataaactattaaatatagtacgattaagaacaagccatgcgaacctcctaaaattattttgaggtgaactccatacaagctatggaaaggtaatagtccccatttatcttatacgaaagtttgagactatgacgcttatttaaagttcatttaatctgataagcttgagtatatatccgataaatacatattttgggatatccaaaacaaatatttggatatcaattctattctcttattgagaagaaagtcttcgtctcacgacatatcgtcttattggaggaaaatgtttactctaagaaatgatagtgggagcaaaatagaacttgaaagagtgcaagagtccacaaatatagttgatcaagtagatgaatttgagtttgatcccataccttatgagggattactcttgatcaggaagaagagactcctaaggacttgacagctccatttaaatctagtaagattattcgaccttgaagaaggtacgaatccacaattactaattaggcattatttatcaaggatgatgaacttactaattacgtagaagtagagtcaagtgttgactcaaatagatgtcaagagaccatggaataagacccatatgaaaacaaggtttggaccttggtcgaccatcctgatggaataagacccaatatgttgtatatggctttcaaggaaaagattggcatggatgaaaatatccgtacatacaaaaaaaggatactagaaaaaggttacaaacaaagacaagtgttgactttgatgaaactttttgtctgtagtcatgctgaaatccattcggattttggtcatataccataactatgggttaaagcaagcctcttggagatgaaatcttcaatttgatgaaaaatcaaaaggttagattttatcaaaaatgaagatgaactatgtgtttataagaagataatgggagcattgtcgcattcctattattatatgtaaaaaatatattattagtggaaaacgacatccctaagtttcaatagttgaaattgtggttgttaaaggatttcttatgaaagatacgggagaaacaacttgatctatagagagagatctaaaagattgcttaactcatcccaattttcatagataaaatcttaagaagattatatatggagaaattggtttactcttaagcaatttgtcggaatgttccaaacgtgaaacaaccattggttcaatagcaaaaatctaatacatgattacttcagaagcagcaaagagttacaatatggatcaagatgttcattaatgaattggggtagttcctaacattgtcgatcacatgttattgtatggtgagaacaataaacccatcgcacaagcaaaggaactaaggtctcatcaatgatccaagcatgtattagggtagtatcatcttatcagagagataatataaagaaatgaacgaattctcacaattgataatattccagatccactaacaaagagttgtcacagtataaacatgatcgtcatgtaaactcttatgataataaatacataagtgattagatctagtgcaagtgggagtttgtaagtgttatgccctaggtccaatcagctttggacataagcacttttattatatagtagatgcaattttatagcgatttattatttaattaatattcaattaaattaaataatagagttcgtagattcaaatattgtaacttattcattacaaggagttgtgattgtgagatacaaattacatgtgattgaaccttaaatcatcctagtcgtaagtgataacgagatacgaatatcgttattatggatataccatcacgtgtggtatttcttatttgtgaagtaagtagctgatctcacaagttaaaatgtggtgacacttaaatgatcacgtggatattttgttatagaacaaaacattgaagacctgctgagagattatacttggataaatatttaagttttagtagttaatctctaacattagatagtgaaattagtcatttgacttgagatcattgttgtgccttatatgaggatagtcatactttagcagtgttggatgttgctctgccaagagccgctaatacggtatcgttcgggtatgtcaagaatcatatgaagattgtgaattttaattcaattaagtcgataataaaatcattggccaaggtgtactcagaagttgagagggagttttcaacttttattgacttaataatggaatgaaagatatgatcgataatcaggatttacacacttccatatctcgtaattgattaaatcatattggcgaagggattatagtttcagggtaaatgaacgattttggttttgtcataccacatgacatttcccgttatatgtattgctctgacacattactagatataaatctgggacgacgaacgttagttggtgaaaaattaaaatggtgttttaatttatcgattttgattatatcaaaataataattcacatcgttaggcatcgtgatagaaaacctgatgggtcgcatacaatagaagaactagaagattatgatttgacaattaattaatttaacaaacgttagataaattaattaattgagttgcttatttataggcccgaatgaattaactcacagatcagatttaattaaataggttcgttaaatattgaactgagtcaagccaagcccttttgggctaatataaataagtgactaaggttttcagtttgtagagattttcattattgctagcacaagaggagaaaatcctgattcctaaaatcttgttctctgtgtggaattcaattggaggttggacaattagatagttgtggatggtaaatcgagattactggaataaaagaaatgcaatggagtttgcagatttcacagaaaggtgtaatttctatcacaatttctatcaaaacacaaaaaagatccttggtaggaattgaaatatattttatttttcgctatgcatgttaagtatattcctaacagtgagccctgccatgagatgcaggaatcaaagtcaaattcacacattcgaacttaatagacaacactagaacacttgaacaaggatccactttcttttgctccagctcatatagaaattgcccctagattccttgatttttctttcatcctccctgaataaagcgaaggtcttgatctagagtcaaatttttggcttgctataaattcgacacaggctctaccggaaccaagcataccttgggaacaagaaaataccatcgtaatttggattgaatcccttaaatgtcagtgatgaacaaaggaagatgattcttttcgtgagactttttttctagcgattgaaccccaagacctttccgtgccatcataagaatgaaggacccacctgcactgcgattttttggggaatctggtcgaaaccccaccttcataaagataatattatacaataaatagttggctggggcaatgatgtggattattcaagatccaatttgtccttctcttcaaagtttgataccaatgatttgaattcaaaatctcgggacttgaacaacgggaaagatatagcttttgactcaatgaagtacaataccagtggagaagcttagctggatgattgattacttaaccaaccagatcctttattctaagagtaggctactgaagttttgatctgatttatgtagagacaacaattgcttgcttcttctttctagtggacatcctgagcaagctatgcagaagatgggaggcttgccattttcattttgttatcttttcatccatttaatttagggaagagtatttcattaaaatgaagaaatatagcagactcaaggtgacttctaaggagataacttgggagatgttagagctttttggttgcacttgtacccagtttgggtagccgcacttcgccattccatatcttctccttttcttatatcgttagtctgtgaaatccaagaaaaatggcaataggtcacttacataggaaaatggattcttctttaattcattcaaatagggtcggagccaggattttagttcagtgcgggcaaaaaaatttcgacaccaaactttaaggtttttgttatggatttaatgacaataaaaaaataaaacaataatgcgacaatactaaaaacaacataatttatatattacacttttagtccgattactagtaggagtgggagtattttataatgacaaaagaatcacaaatactggaaacaactcacaaaattcattgcaattcacaatttcacgtaatcaattcaaagtgcatttcacaaatttcacataatcaattcacaatgcaattcacaattttacaaggcaatataaatccaatagggcagtaacagagtaagcaactcacaatcgcagatggccagaggctgaggcaataatgaattagaagtatgtctcacttactgtctggtagaaaaacaattgaagagcaactgtaggaagcaattgaagaacaaagcactaatttcatatgttatatatatatacacaaatctaaaaaacaaaaaagaaagaaaaaaaagcttcaaaatcagggtaggtggaaaattggaaataagggattcaccttcttcttctgctggctgcttattgctggaacttggacgaatcttctacggtcgattttacctccgccctcaaagtcaaaggttaactggagtggtggaggcgtggagctaccattgcagagaaagcaatatctcttatggactatggagcaaatctgatcaaggacttaggaggaggaggttgagtgacttgagtcagagaagggcacggttgagtcgacaggcggagagtgaagtgccaagtgctatcggttgaaattgaatgaatcgaagtgcaattgccaattgattcaattgaataggtcatgggttggttgtaaatggatcgtgaggtttgattgggctaatgggttattgggctagtgggcttctctggggtggatagggaaatgaaattatactgcaaacaaacaaaaagtttaggcctagggttgggcccaaaagtttaacccacactggacttcattgggctctgcccctggcttcaaagagtcaagaggacttctgcgaacattccattagttcaacttctgatagatgttactagtttataaaaaaatcctgccctttttttcttagcccacagatttaaatgatcaaactaaagtgggccttcgttctcacactttctatggtccagcaaccttatgcattaagctgtttagctaggctagtgtgaaaatatggccaagtaaagtagaggacgactgacagtgtgatcttcttccttttttccaataagttatttcaatggataatgatggtggatggacatacggaaatgggattcctaatagcaggaggcaatttgaagtccttgctcatttaatgcaaatccaagggctctatacaagaaagcgaaactttacaaaacaagcaagaaagtcctttctatctcattagtcaagcagttcagtagagagagagagatctgtgcgttttctaggcctatttctgtcctggtacgtatcctaggtaagccaagaggtttacacatcaccaaaaaatctctcccaagcagctggtcagtacatgattctcgcccagcttgtcccctaagataaaatcacttttctctgccgattggattgttgacatcgctgaattgaagctggatccttgccaacttggccacctggacaccttatatcccatctggagaacctgaagtaatacaatagatttgctttcttcatcaaggaaaatccaatgacgtatagtcaggcttggaagcactaccttttcggtctttgacaaagaatgaatagaatcatgactttggaatgtcgggcagggatgactgtccataaatatagaataaatgaagaattccctgctagtgcactactacatttactccgttggatggatgactgggttaccagatgagctactttgctcattggcttacttttagttctgactttcacgttgcccaactcgaatcagttggcaagtcgaatcccacaaacaggtaagcatctttcggcttgagattgttgttccctcaagcgttcatgcgaactgtgacaactagaaaatggtggctggatttgatccttcgcgatggaaatgccctctcaaaatgaagaaagacttgtcgaaaatggtcctccatgaatactttgcctgtatgaaaagttcgacaacacattcctcagcctgatctgaaatttactgttatcaattagaataatttatgttggcttggtaccacaaaagcataagtatgaacaaggattaatttggcttatacgctattccctctttgtattaaaggaaatctataatgaagacttgttggttgcctactttacttaactatctcttggccagacataatcttcacattacacaagctcagtcaatttgtttctcaacctcgccagccgcaccttgatgctgctcatcaccttttacagtatctcaaagccactccaagtcaagaattaattttttctacttcttctctacaacgtcgagcttttgctgatgctgtttggggaacatgtcttgacccaagaaaatctagcataggtttttgtgtatttcttggaaagctaagaagcagcaaactatatctagatcatctgtgaaggtagaatacagtgctctcgcttccattgccagtgaacttatttggattcaccagttacttcatgatttttaggttccctccttagctccagctttgattttttgtgataatcaaactgcacttcacagtgctagcaatcctattttccatgaaagaacgaaatacatcaatattgattttcatttcatctgtgataagtttactgaaggtttcttcaaacttttaccagttcgttcccaacatcaggtggcagacatcttcaccaaaggtttgccaacctctcgacttttttcccttgatgtctgataagtgtgttttcacacacttatttagctcactaacatgatttaaacatggaaaaaatagtcgaattatgacttaatcttgttaaattcatgctatgtaggtgtttctatggaaaaaatggaattcagaagaaaagagccgaaaaaggaccaaaacggaacaaagcgatagatcgaggaccaagttgcaaataatccatagatgagacgggaaatgaaatgaagattcaagagtgttaaagttcaatcggatgaggaaaggagtcaagaggtgaaatatggtcgaagtattatcaagtatcaaatttcaggcgaaaaagttatgctcgtgattttgagtttctacttgagatcaaattttggcatagtaaaaatcagaatttgaggaagcctatttgtatcaaacgtgtacatctttgagttttcttcccaatgcactttgaatcacctcaatcggagatcaggagagaaagttatgaccaaaatactgaaagctgtccggaggaaagattttataaccatacggccgcatggttataattccttgcggccgcacagggtattgcagggatccaaatgagctgaaaaattgaaccatgcgaccgcatggtttaacaccatgcggccgcatggctttaagtgcgataaaaaattctgaaatcccgtttttaattgaaactctttcgaggctccgtggggacatgatataaaagccaaaattcatcagaaaaagggcagaacgttcagggagaagaagaatacaacttttggagacaaggaacacaaacttgaagccgatttcacaaggattcaaaggggtttttaaggttttgttcaagaattcagatttcaagaactttcatacgagtgttattccttctagtcattaatttcgttttgttttctgtaattatgaatcttctaggctagggttttaattactaggtgatcgatgaaccgttgtttgttattttaattctatatttcatgaacttggtataaagattcgttggatattttgattgatttacatgcattaattttcttccgcaattagtggccaatgactgtgtgagttttgatgacttgtttcttacattcgagagaagtggaataggttcgataaggtgtaaattaacatagggtccgataggggatagaaatatacccctatgctttatgtaattcttaaattgttcacaaaactacatgcattcttgtatgtttgcatcatccatagagatataggctggtggtgtgcaagaataggtctaatatatatcgagagagtatattggatagaataggaacattgaattggcaaattttcatcgaatcattaattttatgaaattagggtttttataacttcaattggggattcgtgatcctagtgactttaatttgattcattttaataaattcgcttttaaacttgcttaatttcatttacttgagtgtttaagtcgtttaattcgagaaatttcgaaattagggttttcaattgaaattagggttttgaaattagggtttttagttgaaattggggcttttcgcatttagatcacattttcactcaattagattcggttaaggctcgattaaatagaatttaactactcaatctctgagggacgatattcggacttttaaaaatccactttgttacttgttacgaaccgtacacttgcggtagttttaaatcgaaagaattatttcgtgaccaaatttttggcgccgttgccggggattgagtattcgttaattttattcaatttagcactaattcggattttttttttttttttaatctattttagttcattttattttactgttattaaattttattacataagtgcatattttagttaattaagtctttaaattgaatcctactgcagaagtgcatgccaagatctgctgaaggagatctactcccagccgacccagagatcgaacgaagctttagaagaaggcaaagagaaacagagcagcgagaaatcagatggagaacgtacaacacaatcctgttgtacaagccaatggaagaggggaagaagacgaaggaaacatgctcgttggagagttcatgacccctcaaatcattcaaagccagtccagcattgtgtatccaccgttcgggcagccaaatttccagttgaagacaaatgtgatacaactgttccagaacgaacatcagttttatggaagagttgaagagaacccgcacacgcatgtctcgcgcttcttagagatgtgccaacacttcagatatcaaggaatctctgacgacgccataaaattaagactgtttccacatactttgcgggacaaggcgattgaatggctcgattctcagccgatagccagtattactacttggaatgacctagctcagaagttctgtactaagttctttccaccggccaagattgcaaaactaaagcacgacatatctatcttcaggcaaggtgaatctgaaaattttgatgagacttggaacagattcaaaaatctactaaggaagtgtccacaccacgggattagcaagggacttcaggtccaatatttctatgcagggctacttccagctttcaagagcatggtcgactcttcagctaatgggtcattgtccacaaaaacaattgatgaagcattgaagttatatgagacaatggctacaacctcagcaatgtggaccatggaacgagcagtaccaaagaagacaccaggagtttatgaagtggatgtgtattcagcgttatctgccaagattgactccttatttcacaaggtggaaaatattacccagtcagctaattcagcgcagacaaagaaggcaaattgtgaagaatgtggagctgagcatgtgacagcagaatgtccaattttgacacaaggaaaagagcaagcagattttgctcaatggggacaacgccaacagaataatgtgtatggagagaccttcaacccaagctggaaaaagcaccccaacttttcttggagcaaccaaaatcagaacaggccacaagggcaataccaacagcaagagaagaagcctcaattggaagaaatgtttggcaaattcatggaacaggccaaccaatatatggaggcgaacaaccaattcatgaagaagacagaagctactcttcaggaccagaatgcagccattaagaatttggaaactcagatgggacagatggcagttgcattaacaggtagagcaccaggcagcctgccaagtaacacagaagtcaatccaaaagagcatgcaaaggctataacaacgagaagtggggtggaattgcctgagagacaagtgaataatcccgtgacaaatagagaagaggtgtctcctgaagtagaagagaatttggagcaagaagaacagatagaagagccaacaccgagagtaaataaaggaaactcaagggataaagaaactgtagctgtaaacccctatgagccacccatactgttccctcagaggctgaagaagcaaaagatggaacaacaatacaagaagtttctcgaggtcttcaagaagctccatatcaacatcccatttgctgaagcactggttcagatgcctagctatgcaaaattcctgaaagacatcctgtcaaacaaaaggaagctaggagatcatgagacagttatgctaaccgaggagtgtagtgccaggattcagagaaagctcccaccaaaattgaaagatccagggagtttcactgtcccttgtaccattggtgaattatattttgataaagctttatgtgatcttggtgcaagtattaacttaatgccgttgtctgttttcaggaaattaggattgggagaagcaaaaactaccacggtgactttacagctagctgacagatcattaacacatccacgaggaataattgaagacgtgttggttaaagtggagaaattcatattcccagcagactttctgattctggatatggaagaagataaagatgttcctttaatactgggcaaaccattcttagccacaggcagagctttgatcgacgttcagaatgggcagttgttactgagattgggagaagaacagatttcattcaatgtcttcaaggccatgaaattgccaatagagactgacagatgtttcagggttgacatgatcgacaaaatgattgaagagtcatttacacagcagaatccatctgatgcattggaggcctgcatcgcatattctaaatccacaacttctgattctgaagacatagaaatgtgtgcaagatttttggagtccaacccaccttacacgcggaaacgatactttgaggagcttgggacagggccagagaaatcacagccatctattctgaagccaccaaagttggaacttaagcagctacccccacacttaagatatgcatacttgggggagtctaatacacttccagtgataatttcaaacatggttagtgaagtggaggaggaaaaactgcttagggtgcttcgagataataagcaagcaattgggtggaccatagctgatatcaaagggatcagcccttctttatgtatgcataaaattctcatggaggagaatttttgaccaacagttgaaagtcaaagaaggctaaacccaaacatgaaggaagtagtaagagctgaggtgatcaaacttctggatgctggaataatttacccgatatcagatagtaaatggactagtccagtgcaagttgtgcccaagaaaggaggaattacagtggttcagaatgaaaagaatgagttgattccgacaaggacggtaacagggtggagagtttgtattgattaccgcaaactaaataccgctacaaggaaagatcatttccctcttccgtttatagatcagatgttggagagattggcaggccattcccactactgctttctggatgggtactcgggttataatcagataccagtggcaccagatgatcaagagaagaccaccttcacatgcccctatggtacctttgcataccgaagaatgccatttggactttgcaacgctcctgccacatttcagcgatgtatgatggcaattttctcagacatggcagagaaattcattgaaatctttatggatgacttctcggtctttgggacctcatttgatgagtgcttggatcacttaaatttggttttgcaaagatgcagagaaacgaacttagtattgaactgggagaaatgtcatttcatggtccaagagggaatagtcttgggacatagagtatcggcaaaggggatagaggtggataaggcaaaaattcaggttattgagaaactaccaccacctacatcagtaaaaggagttcgaagttttcttggtcatgcagggttttacaggagatttataaaggacttctccaaaatcactaagcctctgtgcaacttgctaatgaaagaggtaacgtttgagtttgatgatgaatgtttgatagctttcaatactctgaaggaaaaactcacaacagcgcctgtgattgtgtcacctgattgggatttgccctttgaactaatgtgcgatgcgagtgatcatgcagttggtgcagtattgggacaaagaaagaataaaatttttcatgtcatatactatgcaagtagaactttgaatgacgcccaaatcaactatgctacgaccgagaaggaattgctagctgtggtttatgcattcgacaagttcagatcgtatcttgttgggtctaaggttatcgtctacacagatcatgccgctctgaagtatcttatgacaaagaaggatgctaagccgagattgatccgttggatattgttgttgcaagagttcgatattgagatcaaggataagaagggcagtgaaaatgtggtagccgaccacttatcaagattggaacgggatgaacctgagatatcagtggacatcaatgaaatctttccagatgagcaaatttttggagtagaaatagtcccatggtatgctgatatcgttaactaccttgctaagtccatcccaccaccagactattctagccatcaaagaaagaagtttttcgcagagttgaagtattacttttgggaggatcccattctctacagaagaggcgcagatcagataatcagaagatgtattcctgaagatgaagtacctgagattctagaacattgtcactcttctgcatatgctgggcattttggagcttcaaagactgctgcaaagatactacagtcgggtttctattggcctactttattcagagacacatttgagtatgtgaagagatgcgataaatgtcaacaaaccggaaatatctcaagaagaaatgagatgccactaaattacatcttggaggttgaaatatttgatgtatggggaatagactttatgggaccttttcccccgtcatactcaaatcaatatatcttggtggccgttgactatgtctctaaatgggtggaagctgttgcattgcctactaacgatgcgaaagtggtgacagagttcttgaagaagtacatatttatgagatatggtacaccaagagcaataataagtgatggaggcaaacacttcataaatcgtcaattagagcagctgttgaacaaatatggggtgaaacataaagtagcaactccatatcatccacaaactaatgggcaagttgaagtttcgaacaggcaattaaagagaatactggaagttacagtgaactcatcccgaaaagattggtctaagaagcttgacgatgcactgtgggcttacagaatagcatttaagacaccaataggaatgtccccataccgcctgatttttgggaaagcgtgtcatctaccattggagttggagcatcgagcatattgggctatgaaacagttgaatatggatctcaaggctgctggtgaaaaacgactgctgcaacttaatgaattggatgagatgagaatggaagcttatgagaactcaaagttgatcaaggagcgcaccaaaagatggcatgatttaaacattcagaggcgagagtttgaagttggtcagaaagtgttattgtacaattctagactcaaactcttcccaggaaagctaagaacaaggtggtcgggtccctataccataactaaggtgatgcaatatggggcaattgaagtaagtcacgagaccaaaggcactttcatcgtcaatgggcaaagactgaaacactattggggctgtaattttcctaagcagaagtccactgtgcaactcaataacccaacatgaagaagatgcaggaaagtcgagctatcgactataaactagcgctgggtgggaggcaacccaccgtatcctttaatttattttattgcatttattttggaatttgtttacatttcaaatgttttattaggtcatcgatcactcacacataatagtctaggcactacacgtttatagttgcatgagtcgaggttaaagataatgttttgggtgtttgagtgtaaagttaagaatttcggggttcaaagttgttaattttattttttttaatgtttatttgaaaaaaaaaattaatatgtaaagtcgagtcaattttgaaaaaaaaaaaaaaaaaaaaaaaaggtttgtccatgcggccgcatggacaaggggtccatgcggccgcatggacccccaccgaaagttaagtgggggtaacaaattacaccatgcggccgcatggtgtaactccatgcggccgcatggagcaaaagtgacgggttttaaacccgtcacttgccaaaccaacccatttcttccccccatttccctcccacacggtttccccctccctaatccattttcactcaccaccactcttgcacattttcaacctaaccccaaattaatcccaacattggcatacattctcaaggattttggatcaaaaacttttactttcctttcacaaagatctcaaggtaagaaattgaatttctatgcaaagtttaaaattcttctttgaattctttacattttcgaattgggtaagctttaaattggattgatttgagatttttggactaggcctaagtgcaaatcaaaagcaaagtgaaggaaatttccaatgcacacaaggtgtttgattaaatgtcaataaggcatatgattctaaattttgaacttttcatttgtgtgatgatttacattgttaatgtgaggcatactagacgaaaaatctcatggaatttcattggaaaatgttaacctcacatatatgtgcacataacctcataaattgctaagccatgtcaactcacgtcactaacttcgtccatgtattttcctaaccaaacgacccccgattgtagtgaaatttggatatatgctagaccacaatgagtactttcatatgcccggaccttgtccggggaaattttaatatttctcgatgatgctcggggcggaagttggtcacttgatcatgggtcaaattttaaaaaaaatgcatgttagagtcataattttgaatttttctcattactgcaatattgatgttacattgacttccatgcattgaatattgcacatattttgaagaaagttgggggatttgtgcttgacatcgatattcctcattgtttccttattacacgaacttgatacacttcgttctttatttgtgcaggatgccgccgaagagaacatcaaaaggtaaagaaaaggttggttcctcctccggcacaacccgcaccagagagctagtaggaggtgtgcgaagattctatgatgccgaaacgttagctcgatatgagaacataatacgccattggggcatgataccagagagacaggtccggttagaggattttcctggttttgagttaccaaacctgatacaaatttgtggatgggagaagattgtagaaaagccacacccagtttatgaaagtttagtccgagaattttatgcaaacttcaatagtgaaattgagactccgggttctgaacatttacaccagacatgggtgcgaggtaagtggataatgttatccccagccgtcattcatgacttctacaatcttaatttggacaatgtggtcccgattcccgcccaattcaactggaatgaagtggcggaggttctcttgggaagagagaatgcttggcccctacccactacagagtggcatcaaattgagcttactccctccatagccatcctttgggtcttcatgtgccataacatcgaacccacatcgcatcggacaactttcatggatcaaactgctgggttcatatatcatttagtccggggatgcaaagttgacttggctactcttatttttgaccagatacacaatttgggaacctggggagataggcggtctttgatgattttccctagtctgattagcgggatatgtcttgatgccggtgttacagttgaggcaggggagatgcctgagaaatcaagcccattgataaagctcaccacatttgaagctcaggaacgagctagggtaaggaagagagaacaagaaagacttgagcagcaaagacaaaatgcgcaggaagaaggacaagctgctgaatatttacccttaccacaagccccgccacaaccagttgagatggattcgcagctacttcgacaaatatttgccacagccactggaactagcagagacatacaaaatctccagcagaggttcgagacaatgaccaccacagttgacaaagtgcagagagacctctactcctcccgagcctacacaagaagtgctttgaatgcagccacagctgcgagaagggtagtggagactatgaacggtaggttgaacatgtacgctgggagaatggatggcatacagtggcgtgtgaacgagacttgggatcgtttgggaaatatggaaagtactcttcaggccattcaggccgagcaagtacagcagtccgagttgctgagacaagtcctatctcgcttcccacctcctcctgaagatgatgctgcaggtcccagcttcacaccacaaccaccgcattgatcaggggagtttggttaatctcttattgccaatgtggtccatgttttaaattctgccattttaactttacattttacattgaggacaatgtattgtataagtttgggggatggtagcataatttcaaacaaatattcggcatgtaattatttgcatattcacactccatcgttaattttgacaagtttttgcatgatgcatgcttgatgagtgaatctttatgaacgtttgcatgcttgtgtggggtttggtagccttgccggctatgatgtgattattggacatgtataaactagaaactgtggatttagtgcaggatttaatttgctaatacttgttgatgcactgcttgacactcttttgcacgccactcatgtcacgtgttaagttattgattggaattttagaataaattagaagaaacctagaataaccctctataacattaacccgtaatatcactttaagatagtttggagatgattgatccattgtagggaaacatggagataagtggggactccgtgcatgaaattataatgtgtggattgtttaaacccaaaaggtgagaaataggtgaaagctttaagtgaggatggttttagaagtcaaatgtctagaaaaacaaagaaggggcataaagtaaaaaactggaaaagtatcacttctctcaaaaagcctttatgactcgagcaagtaagtctgtaagggtttaaaacctgatgccctaaagccaactggtttgggagtcatcggtctaaagctcgttacatgggtcatatagaaagcaagaaaaaaggagagttgataaaaagtcatcttatcgagcctttataattcgagtgaataagactgcaagggtttaaaacccggtgccctaaagccaactggtttgggagtcatcgcctaaagctcgttacatgggttatatagaaagcaaatgagaagatgacatgccaaaaaaaaaaaacttaaaaataaaagccctcgttggacatttggttgatagaactataacctcaatgcgaagcaagtagcttagtttaatcctaaaggttgaagcaatcaaaaataaggagagtctctacttgttgatatgtgaacttgtaatggtaaaatctatccaaactaaaagaaggtaaggattagaattgtttaaactcctaaccttagaatacaccccggagaaattgtgtgaaaaaagaatacattttgggattgtgtatctctcgagtgacgtaaggataaatttgaccactatgggtttgggataaactaatcataagcttaatatgttggcatgagttcacacacacacgttgagtattgcatttgatgagtaaaggttgattcaattctcgcactcttgatattgtttctattattattactaagtccaatcctgagacacggcaagctattaagccctgtttgtttagcattaagtcactacattgtttgaggacaaacaatagtttaagtttgggggatttgataagtgtgttttcacacacttatttagctcactaacatgatttaaacatggacaaaatagtcgaattatgacttaatcttgttaaattcatgctatgtaggtgtttctatggaaaaaatggtattcagaagaaaagagccgaaaaaggaccaaaacggaacaaagcgatagatcgaggaccaagttgcaaataatccatagatgagacgggaaatgaaatgaagattcaagagtgttaaagttcaatcggatgaggaaaggagtcaagaggtgaaatatggtagaagtattatcaagtatcaaatttcaggcgaaaaagttatgctcgtgattttgagtttttattgagatccaattttggcatagtaaaaatcagaatttgaggaagcctatttcaatcaaaagtgtacatctttgagttttcttcccaatgcactttgaatcacctcaatcggagattaggggagaaagttatgaccaaaatactgaaagctgtccggaggaaagattttataaccatgcggccgcatggttataattccttgcggccgcacagggtattgcagggatccaaatgagctgaaaaattgaaccatgcgaccgcatggtttaacaccatgcggccgcatggctttaagtgcgataaaaaattctgaaatcccgtttttaattgaaactctttcggggctccgtggggacatgatataaaagccaaaattcatcagaaaaaaggcagaacgttcagggagaagaagaatacaacttttggagacaaggaacacaaacttgaagccgatttcacaaggattcaaaggggttttcaaggttttgttcaagaattcagatttcaagaactttcatacgggtgttattccttctagtcattaatttcgttttgttttctgtaattatgaatcttctaggctagggttttaattactaggtgatcgatgaaccgttgtttgttattttaattctatatttcatgaacttggtataaagattcgttggatattttgattgatttacatgcattaattttcttccgcaattagtggccaatgattgtgtgagttttgatgacttgtttcttacattcgagagaagtggaataggttcgataatgtgtaaattaacatagggtccgataggggatagagatatacccctatgctttatgtaattcttaaattgttcacaaaactacatgcattcttgtatgtttgcatcatccatagagatataggctggtggtgtgcaagaatgggtctaatatatatcgagagagtatattggatagaataggaacattgaattggcaaattttcatcgaatcattaattttatgaaattagggtttttataacttcaattggggattcgtgatcctagtgactttaatttgattcattttaataaattcgcttttaaacttgcttaatttcatttacttgagtgtttaagtcgtttaattcgagaaatttcgaaattagggtttctaattgagaaattagggttttcaattgaaattagggttttgaaattagggtttttagttgaaattggggctttttgcatttagatcacattttcactcaattagattcggttaaggctcgattaaatagaatttaactactcaatctctgagggacgatattcggacttttaaaaatccactttattacttgttacgaatcgtacacttgcggtagttttaaatcgaaagaattatttcgtgaccaatgtccaagatggctattactgatcttcatcgtccatcttgagggaagagtattagaatattagttagttagctagttagctaatacagcttgtaaatcagtccattagttagttcgtatagctgtcaattacatcgcacactctatttataatcgtatccatctgaataagatttccctccattttacaattgtcttcttcagcacttctacttcgatacatcttcttttatcaatttctgaatgtgtacaacttgcttaacgagaatgagtatgtaaataatgatgtatttacatatactatccattatcatctaaaggctaagaatataagttctggtggataattgcaggtttaggctttgacaaattaacgtaggattatgaggattgtgagactcgaaccacggttttttgcttccagaattttatgatattgagaagtcgtgttttgtgaaaatgcaactctattaatttgacactttcaactggatggagacacgtggctaaaccatggctgttggattgaatctcgaaccttccattattaacgtgtcatttcacttggcacacccattactccattacacatttttgactcttggtctttgagagagagagaacccctcgtttggttagggtttgttctgctcgattctgtggctcaaatctctgatttgaggccttaaacgtgaaagtcttagtgatttcgtttagatattctgagtgattatctgtaatgtcctgtgtcttcttgagttgtgatttttgacagatatgtagtgaagtttctttgtgattcttcgaaggtgttgagtcgatctggagagataagtatatttgcttcatctcggtgtattttgttgaacatttgtaacccttcgttgccatttttggctattatagtgcaaccgagcataatccaacttgttggatgctcaacgggagatgtaggcgttagatgttgtcaccgaacctccggggcttaggcagaaagaaatcttgtgttgattctttagggggtgttctctttgtgtttcagttttgtgttttgagttttgtgttttgagtgtttgttttgaaattgttgaaaatgtgttctttttgttagtttctcaaaataaaaaaaaaataattttttttttaaattttgagaatcacaacaacaccacctcaaaacaccaaaaaaaaaattaattaatttttatttttttttttgaaattttgagaatcaccacactatctcctcaaaattttttttttaatttttaattttttttgaaattttgagaatcaccacaccacctcctcaaaaaaaaaaaaaaaaaaaaaaaaaaaaaaaagtgtttcccgcgttttcaattttttcaagttttacactgaaaacacccaaaacgacaaaaaagtcgttttgtgttttcttcacaaattttttttcgttttcgaaaacgggaaagagaacacgttttcaccgttttgaaaaatcgaaaacagaaaacgacccgaaaacgataaagagaacagggccttaattttctgcacagtttacttttggccgatttcattttcttgcttctcgatttaatattgtgtgacctctaccttacagtggtatcagagcctaactgaggaacacgatacccggatcttggagagaaaggtggatcttcaacagattttgaatttatggagctgctgaaaagcagatgtgaactgcctcgggttattaaactcactgggtgagatcttttaaaatttactgtgtattacacttgagaaatttgcgtctcttgaactttcccggattttccagtacaccgttgaaacctccttgagactaatctttgtccagtagcttctacgaggccactgaaatttgagataaatcaagtacgagtgtgtaacttgggagaatcttgctggagggatctatgaaaccttacaatctcatctcattaattgttttctgttgataaatcaagcctactctctctgttgatatttttttagattactgaaatcttgtattactttgtgatttactatgatttcgaagttggcaacttaggttttctatctcaactgttctgaattcttgctaaatcctgtttgtaataacttgcatacattatggctactgcaaaatttgaagtgagtcaatttgatggtaaaattgatttcgatacctaaagtcagaaaatgaaagccattttgatgcaaatgaatgtgctgaggcattagatgattcatggcctgagggtttaacacctaataagaaatctgaacttgatgaaattgcctggagcactatattcttatacctatttgataatgtgataagagaagtgggtgaaaccaccattgcctctgatctttgggaaaaactcaaggcgaaatatgaaactaaaacaactccaaataagtgtttcctcttaaagcaattcttttcttttaaaatgaatcctgcagttgacttagaagaaaatttgagtagatttacaaaaattacccaagacttggccaattatgatgaaaaactttcaaaagatcaattggctgtaatcttgttaaactccataagtgataagtataaaaacattaaggtttcacttgaatatgggagagatgaacttgcacttgatgttatgctttaaggaataaagcattagagatcaaggctgagttatgtatcagtcacactggtactagttttttaacaaaaggaaaaacctttgaaaaacctactcaaaactttaagttttcgaaaactaacaaaaattggactgacaggaataagaccaagaataatgcaaaaggtaaaaaaatgttattattgtggcaaacttggtcattttgcaaaggattgtttcaaaagaaaaaatgattcaaaagaaaaaagtcttgatggaagcaatgccttcgcctatgataaaactaaaactgaaaatggttttgttttggtaagtactgaaaaatgtcaaagtgatgaatggatacttgactcaggctgttcctttgacatgtgccccaacaaaaattgtgtttataaatcttgaaaaaactaaaagggggcaacttataatgggcaataattttgcctgcaaagtgattggaattgggactgtcaaattgttattggaaaattgtaatgttttgttccttgagaacacaagacatgtccctgatttgaaaaggaacttagtgtccctaggaatgatagatgataaggagtttaacataatcatgggtcaaagacatataaaaattcttaggggggatgacttggtcacttcagcccctaagaaacatggtctctactgtttaaatgctaaacccttaattggattaactgcctctgtcatgactaaaaaatttactttggctaaattgtggaatcagagactaggtcatattggtaaaaagggattaaatctttgacattcaaaatgtgtatttggaaaccataatcttggtgattttggtacttatgaacattgtatttttggaaaacaagttaagcttccttttccaactggaattcataaatcaaaacaaaaacttgagtatttacatgctgatttatggggtcctgcctctgtctctacattgactggtttcaagtattttttacttataattgattatttttcaagaaaagtctgggtacacttgctaaaatcaaaagatgagacattttctgttttcaaggattggaaaactcaagttgaaaatcgaactgattttaaaataaaatatttgagaactgataatggtttggaattttgcaattatgaatttgacaatctttgtaaaaattatggcatcacaagacacaaaattgttcctcacacaccaacaaaatggaatggcagaaagaatgaatagaaccctattgaacaaagttagatgtatgcttttaagttctggtcttcctaagatgttttggggtgaagcagttaaaactgcagcctacttgattagtaggagtccctctagtgctttaaattttgctgttcctgaatctgtgttgtcaaatagacctataaattacacttatttgacagcgtttggctatgctgcttatgctcatcaaaatattggtaaattagaaccaagatcattaaagtgtgtactcttgggttatgttgataatgtaaaagggtacaaactataggttaaatcagagaagggttatagtgtaataataagaaaggatgctatctttaatgagtcattgatgccatgtcctgagggaaaagagaaatttaactgaaaaagatgttcaaattgaggtggagtccctttgtagtaatgagaatgcctctgggtctacaacaggggataatgaaaatgaagaacatgctacagaaccagaaattgaaattgatcaaactgaagagactgattctgcagctctttccctgatgagtatcaactcacaagagatagggagaggaggcaaatcataccctctaccagatttgatactgacacctttgtttccttattttcttaccaaaatatgtctaaaaatgagccaaattcttttgaagaagccattaaatgtaaagaaagcagaaattggaaactggcaatggaagatgagatgtcttcattacttaaagataaaacatggattttagttgacaaacccaaaggtcaaaaattgattaactgtaggtggatttataaaataaaactagggaaaggtgatagtaaaaatgttagatacaaagccagacttgtagcaaaggatttcacacaaaaggagggtgtagattacactaaaaaattttctcctgttactaagtatgtcaccattagatgcttgctttctattgttactcaatttaaatgggaacttgatcaacttgatgttaagactactttcttgtatggagaattagatgaaactatatatatgaaacaacctattggttttgaaaagggtgatcctgaaaatactgtttgtttgctcaagaaatctttgtatggcctaaaacaagcacctaggcaatggtataagaggtttgacacctttgtcctaaaacttggtttcagaagaagtcaatatgacacttgtctatactgcaaaggtaatggagttgaaaactcattatatctagtcctttatgtggatgatatgctgttagctagttcagacaaatcagaaattaataatatcaaatcaaagttaaaatcaaaatttgatatgaaagacctaggtgatgcaaaaagaatattgggcatgcaaatatggagggacaaagataaaaatatattatctctaaatcaatgtgattatgtgtcaaaagttttgaaaaaatttaatatgtttgattgtaagcctgtgacacttcctcttacaaatcattttaaattgtcttctgaattttgtcccaaatctgaagaaaaatatgctagaatgtcaaaaaatcccatatgctaatataattggttctgtaatgtacttgatgatacgcaccaaacctgatcttgcatatagtattagcattttaagtagattcatgagtaatcctggtgaagaatattggcatgctttgaagtggttattgaggtacctaaagggatcttcaaacttaggattagtgtttaaatcagataaaaatgggatatgtttaaaggctaaattgactctgactttgctggaaatagagcaaatagaaagtcaacctcatcctatttttatacactatgtggtactgcgattagttggaagtctcaacttcagaaaatagtagctctatcatctactgaggcagaatacatagcagcaactgatgctgttaaggaggggatttggttaaatggtttattgacagaaatgggctttaatgataatcttactgtgctattttctgataatcagagtgccattcacctaatcaaaaatcccatgttccatgacagatcaaaacatattgatgttaagtatatttcataagagatataatttcaaaaagtgaaattaagattgataaagtttctactcagcttaatccatcagatatgggtacaaaagtaattccatgaaacttttatctgttgatactttgtgatttttttttttttttgtgtacaggtacatagagcaaatgaagatgagttaaggatttgctcctcgctgcactatagttccaaaaattatggtagcaaggtggagaatgtgagactcgaaccatggttttatgatattgagaagtcgagttttgtgaaaatgcaactctattaatttgacactttcaactggatggagacacgtggctaaaccatggctgttggattgaatctcgaaccttccattattaacgtgctgtttcacttggcacacccattactccattacacgtttttgactcttggtctttgagagagagagagaacccctcgtctggttagggtttgttctgctagattctgtggctcaaatctctgatttgaggccttaaacgtgaaagtcttagtgatttcgtttagatattctgagtgattatctgtaatgtcctatgtcttcttgagttgtgatttttgagagagatgcagtaaagtttttttgtgattcttcgaaggtgttgagtcgatctggagagaataagtatctttgcttcatctcggtgtatttgttgaccatttgtaaccctccgttgtcatttttggctattatagtgcaatcaagcgtaatccaacttgttggatgctcaacgggggatgtaggcgttagatgtggtcaccgaacctccggggcttaagtcgaaagaaatattgtgttgattctttaattttctgcacagtttacttttgaccgatttcattttcttgcttctcgatttaatattgagagacctctgccttacaaggatcaaaactactacttttttaattgggtaatcatgacggaaggattaatgtgataataaatgatagatttaaacattaaaaaatttaattgccgcaaacaatgaaaaaccaattttcttggaccatggaaggttctacagctggtcaatttgtcaggtaatagatatttgttttgatgtttgtcacattgaaatatgttttggcttataattaagccaaaaacatgtgaacaacctcactctggttagattgcattgtgctttttcattcattcattaccttcttattttgatcctagacaaggaatggactaatgcagtttcattgaaaacattgtcatgcagtcaccgtaactgaagttgaggcactgtatgaaatatttaagaaaataagcagcccaataatcgatgacggtctcattcacaaagtaatattacattttttttttttatcaagaatttgatccctaattatttgttgtgtatggttctgaatacatcatttttgcaatgttgttgccttaaaacatttagcaacatatgtttaaatttgaagtaactaatgcttaacacaaataatttatttttatatctacgctacacgtacgatgcatgtgtgtctctctagtagtagtcataagagtcactatccccaaataaacaagtcttgagagactctgtgtgcaatcattggatgccactgtgttaaaattgttggataaataaaaaaatcatgcataaaaatatgataaaatcgtgattcactgatgcaaaatattggatacagtttcaaattatcgaaatcaacatatgtgcatcaaaatgtacacaaaatgggatttactgaaacgctaaaattagatggacacgaaataaaatgacgtatgtgagtgtacagcttcttaagacaaattttgcccacaggtcttaacatattaaatggatgtttgtctcctaaaatacaacacactttcaaaattattaaagcaagaaaatacttttgtcagcaaatttaagtgatgatagtattcttcactaataggataggaacgaattaaaattgttcggtctgaattttatttctaataataattggatggaatttaatttcactaaaataataaaaaacagattattttgaaaaaataagagaatttagaaaccaaaatttcttgaactgattttagagtaaatatggaattaggggttcctatctatagatttacgattgtatttttgggatgattggatcttttgacataaattaatgaggattattaaatcacataattttatatttaatggtctaaattgcacctgtaaaaaggtcatgacttttcgtaatgtagatttttgaatactcacattcaatttgaaacaatatgactctatgatgtgcactcttttcattagaaaactgtgactggtcatcgcatcaatttaaatttttttttaattcgcacctataaaaattatctcataaattcaacaatatcccagatgaatgaaagaaatcaactcagaacatgaaagacaaagaatagtattattgaaatataatgcattggaccgataacttttgttttgaacctttcttagtaagaatcttttgaactcacttaattaataagtaaatgcaacattttgaacttttgacggtaattagaagtctggacaatataatttatcacttatatcaaactttgatcatctattgaatatttcagtcttaaaccttttttagattctataaatatgctagagaattcaccttattaaaattttcagagaactagccaagttcatacttacgaaggtgatgttcataaagagtacactacaatactctacttttactgtttacaggattcctaatcaaatatttggtagcaacaattctttccattatagaaatgaaaatgaacttcaaagtgcttatcatcgagtcatgcataactatttttcctattgaacctactccataggatctctagtcttcaagttaggtttccattaagttgactcattaatttaggcgttaaacccattttctttgatgcacgatctcttctctctagacaacccttttctaaatagattcattaaaatcaatattgttgcatttaagagaaactatcaaatggtattatgtctactacgcatatgtcgagacttaccattatatatatatctcgattaaatcacatattgtcactattagaattaggatatgacttgaattttatttagaatgttatttggaatcctattcagagtctatttgaaaaattctagttaaagttctatttgaaaggtcaattgagagctgaaatttgtgtcgaatttgaaggttcaaattatggatcggaaagttgctgcaatttcgctagttggccgctagcttggcaatagaacagcttcatcaaaatttcaataaggacttaatgcttgcctagccctcaagcgattaaaccgtcgctatcctagagttcgagtggcatagttatccgacccaacccatttcacagtttaaagcattttaatttttttctttccatctagaactatattattagggtttggatgtccactacttgttctctatatatatatttagctcttctttacaatttagttaaggtagtttaacctcattagaagttagatatatcgtaaacatcaaatctttgtattatttctccatattatattaaaaacttcattctcgacaaattactttattcttgtgtttttgtgatctttatttgatattgtgcccataatctcatattttcttcaacaaatcggtattggattaattcgattcaaattttcctcacaacaaactggtatcagagcttttggttttgcaaatcgtacaaagcttgaggttttgatcaagttaagagctcaacttgaccttttatgatggcaactatagagtgtgacattccactattagatcgcaatacaggattctgtttgtggtaaagatgcgagcagcacttgctcaaatggatttggacgatggattgttaggatttgagaagacgaccacaacttggactccgaaggagaaatggtggaagggttgaaaggcccgatctcaaatacatcttcatctttcaaataatataggatgttttgaaagagaagtcagccactgcattgtggacaaaatttgagcaattatgcatgatgaatcttactagcaaattgcatatgaaacaacttctatattctcattgtatgaaagaaagtacatctcttgaagatcacctaactatttttaaggaaatcgtcactgattaggagacattggaggtcaaatgtgatgaaaaggattatgaattgattttattgtgttcattaccgattttatatgcgtcttttagagatacgattttatataaacgtaataatcttaccattgaagaagtctataatgctctatattcaaaggataagatgaagcatcttgttgcatctaaggttcatagagatggcctcattattgatggtggcatgcaagggattaatcaaaatctaacttcgaattttgtaattattgcaagaaaaatgggcacttgataaacaattatcatgagttgccaggataaaacaaagttgactacaaatcaacaatttgaaatttcagggaaagcaattattgcagaaaattctaacaataatggagaactttcatttacgtctgactacaactctaaacctaagaaggtttgggttcttaatagagctttcacttttcatattttccaatcgggatttgatttcaacatatgaagaagtttcaaaaggttttgtgatgatcgggtagtaatataccttatcagatagctggtattggctaggttagaataaaaatgtttgatgagatggttagaacacttgatatggtaagatacgctctatagctgaagaaaaatctcttcttcataagtactcttgatacaaaaaggtacaggtacactgttgaaagtgaagtcctaaaggtcagtaaaaggagctagtgttttgttaaagagacataaaaaaatatcatttatagatcttgatttgttatatagagtttttttagcaatcagcatattttaaaaacttaggtagattaggagttgaattccgtaacattggagtctagtttgtgatctttttttaaagaatatatctcatttgaattcaaaagttacaagtaaatccaccttgccacctttatcggtagtgttattgaattcagttgctagtaacagacccatttttggttataagacttcaaataggtacatttttgctatttagttaatgttttgaattgagttaatagtgttgattctgatcaagatccttctttttattcattcaattacaattctattatagggcttgtttcagccttgtctggtgcctagttggggtgacagaggtagagaatattttcaattggaaattttttttcacgaagaatttcatttttatttatttatctatttattttttatttttttggttagagagttgaagtttattctttgcaatagatgaagtttgttcactgcagtggaattcgtgtcaaggttgaatttgttaaaatttggttgtgaccttaattctatttggaatattatttagaatcatattcgaaatctatttggcaattctagttgaaatttcatttggaagtctaattgggagttgaaaattgtgttgaatttgaagagatcaaattatggattgagaaaagtcgcttcaatttcacttactatccctagcttggcgctcgagcggcgatgtcaaaatttcaacaaagacttggcgtctgcctggagctcgagtgacataattatctggcccttgcccatttagtattgaagcattcatttccacctacaactctactattagggtttggacgtcccctacctgattcctatatatattcggctcttctccaaaatttaattaaggttgtctaacctcatcaaaagttagaaacgttgtaaatacaaaatttttgtattctttctccatattataataaatcttcattctttgcaattatattgttctcgtgtttttgtgatctttattcgatatgtacctataatctcatattttctccaacaaattggtatcggattaatccggatccaattttccgcagaacagtcaccaatttgaaattttatataagaaaataaataaaatttgaagtctcatgcttccatctgattttatttaaacctctaatttaatcttcccattttcaagttgtggaagattttcacgaaacaactacaatctcaatagtaaaaaatattgactaataaattttgaactcttgtattgaatattcaattttcaacatcgtttacttcttaagtttaatagagtattcattgcaatgcagtttatcatttcaaatattctttatacattctaaatgctaatttgaagtaaaaatcgcgagcacgcacaagtcctggggtgcatctaaactttaattgagaatatgacgcaaacaataatcctacccctacaatattgaataacactgagtttagcaacataatattcattaactatataaagttcaatcttttcgttaattacatttaattgtcagataaattttttcgacctctagccaaaatataaatgactaagaatgttcatgtcttataaaaaatcatgcactttcatatttaggaccgccgacgttacccactttttggttaagaatctcatctttttataactttatcgtatgtgcaagggctttcaacattttcatcgtcatacaaaattttctatgacatgtaatcttaaactgatttggagcggaaatatggaagtaagaattcatatttatatattttctcgtgtcttttcggaatagttacatcttttgctataaatgtagatcattacatcacacatttttatatttaagtacccaatcaaaaggtcttgactttttgtaatgtaccttttttttatagtcacattacaattcgaaacagcgtgactctttgattcgcacaatttgtattcaaaaagttgcgactagtaatcgaatcaatgggaaactttttcaattcacacctataaaacttatcccgtaaattccaacaaaaatcactttatactcgcgacatgaaaaaccgctgcgaatattcgagcatgtatatattcatacatgccaatttaaaaggcggctgggcactagtgatagtaaggttctgcatatcagttgcaaccgcaagtttgttcaatttgataatttatactcgaatactatccactatctgggatggaaagtaggaaataatttggaaataaatttgaggcgattctacgcgtatgatctaattgtaaacaaaataaataaataaatatcattccaactatcagctggcaggattgtccgtacagttttccttgttcaattaacaccttttcttgtctgattaaggatcacgcgcagcaacttggttgataaatatccatttttctcagcttacgaagtatttcttgaaacagaagcttatgtaattcttaggtaaggacgtccgctgttgacttccactggatacaaacagttcttaaatcactgttgttcatgcacctttcagcgagaacgagcactagtacattcatttgcctgttagcaaagagtagtcacctccttttagtcctgaatgagagaagtcaagatttgcttatttaaagcaagctctctactattgcaacctaggatagtgcaaatggcaagtggaatggtctggtttcacttcaaccatccaaatccgcgtacatggatgaaatgttgatctgcttttacatgctttgatctatgggaccattctcaatctttacaatttttgctctttttctctctacataaacttggttagatgcagggaggagcttgtggatgtagcttagtccatcactaatcttatcctcccaattgtattcctcatgtttattgcttctgtgaacgtagtagctaaataatcccaacatgttacataagttaaatattgtataatttttcgattttccacaattttcttcattcttttgtccgccatcgtctcactggccaaacttgacccctgttattttgaggtctatctaatattcagagtttcactctatctactgtactcgttgccaatattcaaatttgaagaaactcattagtgtctgtcccattaaatcagtggctgtgattagaaggccgaaatagggctagcattgatatatgcattttcgttcactttccacttgaactgaagaaggtttgtttaggattcggggtggaatctctgcagatgagcaaaacatatgatgtttaggtctttgtatatatatttacaacatgtactgatccatggcaatcaattcaattctgatgacatggatgcttggttttgcacaagcgggtcaaactcttatgaagtaaaaatcttgctctgctctgctctgctctgctcagctgatgataactacagaggaacgaaatcgaaatgtaaaccaaagctgccatgaatgatagtaaatcgaaggtgatatttagattgactacaatctggataggaagcatcagctaatagtcaataactaaattgtacaacatagtttgaaaaatatatgatatacgaatcagaactcaaagtaaaagtattgctaaaaccattccagaacttacgttgtcaagcagttatctgttttgattaattgaaggaccttgaagccttacacactgatattatccagagagcgaaccatcgtttctgccttattttcaggtgctaaatgtagcaggaaggaattatgacaggccatagtagccaaagacgctgaaaaaggaaaacttttactaacttgaatctttatttcttcattttctgccaggaaccctcccatttaactaaataagttacaccacaaaatttcaataacctctcaattgaaagacataagtagcttcaagtgctggcttctggtaggaactatcctagttaaccaagtatgtagaaaaatttaagcaacctcccgttggagggcataacttggagaaggtaaacatcctattcacttgtctgaaaagaaatagctcttgcagtcctagcttccatcaattgagaatctaggtatcattctggcaaacaaacacacttctgtacattctcacttcgatcaccaaaagttatggcaggagcacatcccatcatggaaatggtgaaatctcatattatccctgactataatctcccgttgagtaacttgagaagcaccacacacaaataaatgacagtcctcgcatatccttagatttttcacaattctaataggaaggccatcatcagtagtgagcagcgcataagccaaagctcgcttctcactgtgattaatcaaaattcgctttttttcttcatcactcacatgataaagcacacagcttagattcggactataaccatttaattttagtctgtcaacaagatcctccatggcctggtcaatttctctagacctaggatgggtcaaatcacctgcatagaattcatggatcacccctttgcttccctcaacccagctaaatgccggattctttctcaaccccttttctctaatcaatttccttactttcgaaacatcttcccaccttcctgctcttgcataaatatttgaaagcaagatatagtttccaataccatcaggttccagcttaaataaatgtctagcagcaacttccgcaacatcagggtttgcatgcgtacgacaagcaccaagcagagctccccatatgctagcattgggctctatcggcatgcttcttataagcttcagtgcttcctccaatcgtcctgtccttccgaggagatccaccatacaattatagtgatcataagatggtttaacaccgtatgatttctccattattttgaacatgtgttgacctttatctaccaatcctgcatgactacatgcagtaagaaccccaacaaaagtcacatggttgggcatcacatcctttttgaccatctcctcaaacaattctagggtggaactagcgcaaccgtgaattgcaaaaccaacaatcatcgaactgtacgtatacacatttttttcctgcatcatcttaaaaacttcatatgcactctccgcacttccacactttgagtacatatcaatcaaagccgagccaacaactacattgtccttgggactatatccagaccgctccgcaacatccctcacccaatttgcatacttactcgtgcccaacagtgcacaagcattaataacaccaaccaatgttacctcatcagtctctacacctgctctctgcattctctcaaaatagtccaatgcttcccttggctttgcgttctgtacaaaccctgtcaccattgaagtccacgccaccatatccttcacaggcaacccatcaaacaactcccttgcagaatccatatcaccgttctttgtatacgcaacaatcaatgaggtccacgaaatcaagtccctgtgaggcatttcgtcgaacaccctcctcccgcaatccaaccatccgcactttacatacatatcaatcaaagtgttgccaacaaacatatccaagccaaacccacctaactttacactctccccatgaatctgccgtcccaaatggacattcatttgactagaacatgcctttaacatggccgtatatgtgaacgatacgggcgtaacaccatccttccgcatggaactataaataagaactgattccttgaacagcccgtcaatcgtgagccctcgtattaaagccgtgtagaggaaagggtttggatgtttcacttgggagaacactaaaactccataagcgtgcatggggacattgattttagcgagaactcggaggagctttgctatgatataagaacactggccgaggcctttgcggattatgtagccgtgggcttgcttaactttggtgaggcttgtgcagctgtcgagggtgtgagtgagttgagattctaattgtttgatttgttggagccgtgaaaatggtatgaatggcgttttctcttgtcggaatttggtgggttggcgaatgacgagtggaggtctgataataggtagaatcagcttccgagagagtgaaaccatcacatatttctgtgcagccacggttgacaactacatgtaagaccactctcggacttcaatttgaattgtatttcaagttcacgtacactgtaagagatgtgactgcaaggtccagtagcccaccctacgtaaaaactgatataaaatttaaaaaaatcgagataaaaaaaaataataataataactgctacttcacccccgtttggcccccatttcgtagaattaaaaataaataaaataatatttttttgaaaaatgagcagttaaaaaggaaggaaaaagaaaaatgtaatagaaattaatgtaagccaaagaagaaattttttccccaaacgaagtaacagtttaaacaaaaaaaaaattattattaagataataattaatgagtaatattagcgttgaggatttactgaagttaatttttaataaagtttttattcatttggttttataaatttgaaacatagttaatccgcttcaaattcgttactcaactttcaatctctaaaagagtaatctcagaatctcaacggtacttaagtttgtgaaaatattgtgtgccaatgagaaattattggttggccaatcttcttcatcgtctacacatgatacacgagatagtcacttgatattgttaaggatatttagtcggccaactaggtaagatcacttttttagttcaaaaatgggctataccccgcaacccccccccccccacccaattcaaaatccagaactcatgtcaagccattaaattagtcaaaattaaaacttaggttaaaatcaaaatttaaacccaaattcaaaattatataatccaccaaaattgcctctcgacccaaaatcagaatgtgcacctcagtcccaaattcaaaatttgcaacccaagtccaaagcaacaaaaatttcctccaagaaacaaaatccttagggtccgcttgattgtaatgatagaatttgggtggaaagaaaacaaattgaaatgaattgaattgtctagaatttattttagtggaaattgcaaattaatagtgtttgattggtataattttttacctgaaaaatattaaaataaaagtgtcttttggtgttcatttgactttatttttcatgaaaattgtcaatttaaggaatatccacttctataattgttcctgaaatttgtttccattaccaaaaaggaaaaaaaaaaatatttatattttggtattcgtttgactttattttacatgaaaattatcaatttaagagatatcatcttttacaattgttcctataatttgttcccattgctaaaaaaataaaaagggcaaaaaataaaaaggttttggtgagaattgattttccaccaaaataaggaaaatgcacatgtgtgagcaaaacatagaaaatgaattccatgaaaaagaaatacaatcaaacaccaaaaaggttgttccatgaaatttaatgcctataaaacagggcttattctcgcaactgctggaatacacagtagaatagtgttgcacttagtagtgtcgggcatctatagcacaatctataacgatctttatcgaacttgcacaattggtattgtgcaagatctcactattgtatcaattcattgcaatgcttcaagcactgccctggcttctatctatgatgatgttcaagtcctaacgtaataatatggaaggtggaaaatttccgtattaagatgcatttattcatttccaaaaataatttcattaacgatacaaaacaattttgtacaaactagtcatagtttaacatgctaaaaacctttataaatgctataaagtaatatttgaaagtgtgtgaattttaaaaagaattaatgcaatttgtttttatttaatgaacttttgatttaaatgaaataaaaaccaatttgtgaaaacaatttaccctttggataagaactgaacattcaaagaatattatcctttcttcatattcgattaatgtgcattgaatatatcaattgaaaatatttattttagagccacattatgtacccccgtttaccttatacgtacgtatctttatgttcattcaataaatcaattgaaggaaaattttaaaaatattcatcttttgtttcaaaaaaattttaatgaatttaatttattatccaatcaagtgaaatggaccagtcaaataaacattgatcataactaaataattgtcaaaataattcatgataatattgttcaaatgactaaataatcaaaaatatatattgaaaaatgaaaaggtgatgaatatgtcaaatatagttaaataaattaaatacatattgaaaaaagaaaagtaatgtaatgaatgtatcaaatgtattcatcaaaaataaatagttgacaaataattaatgatgatattgtttaaatggttcaaataattaataaattaaatacatattgaaaaacataaaataggatattattaaaataattaaatatatattgaaaaacgaaaagtaaggtattattgaaataattgaattatagtaaggataatatcgttcaaaaaatggttctcacttgatgtgatatttaatatattatagattaaaccactatttgaaaaccattatttcataactctttaattcacatactcattaattttcaactactcatttatacaataaaatattttgcatgtaaactcaaaacttttgctttttttttttttactgcattctcaaaaaaataataataataataaatcatcttctcaaaataatgtcagcaacaattacacaattatatttagattccataagttattctcaatggtaagccatagcaaattttattaaacaacaaagttgtctttgataccacagatttacttataagtgccatagaaatttaaatatgtttaaaatccaaaatttgtatcacctttgtttataggtagaaaatcgttataggctgtgtactttgggatatttccacaagttaggacgatttttaatttgacatatcacaattttagcatgccacatgtaacgccccgaatattatcgatttaaatattggggtgttaccgatattatttcgtaaacatacttgaagcgaaaaatatttaattgaaaatttaaaacctttaatttatttgaaaataaaataacagtgttgtagaatttagagcactaaatggaattaaagaaaaaaaaatcctaacaaaattattcttaaatgttttcctaaaaattttctttacttggcaacccgcgccgctcagccaccatctccgtcgaccaacctaacctaagatgttaaaattgaagaagtgagtaatttatactcagtaggatacgtgcgtccaaacaatacgatgacttttaaaacatgaatctataacattccataccattatttcatcaagagcaatcgatgatcaattgaaaactctaacacaattgaaaagacccggaggcgatctcacatttcatctcatttcatttcataaagacccgtaggccaattagtatttcatgaaataaatcacgtaagaaaaattataatattgaaatgacggaataacttgcacataatatcataccttgttagataaaacagtttttaaaaagtcaaatccaaaatcacgttcaagatctttatttttgcatagtgtcgtgttgagcagattttattatttggtgaaaagtgaaaacatctattgtacacctatgatatttataaaaacaaaagggaatattggaggcctagatatatgcaaaatattgtgttcttcccttaaaatcctcaatcccattattccatgatgtgtttttccccttaaacgcctcattctcgtacaatttatagttattttcccctatcttattatcatgtggaatctatcactataaatccctaaaatcaagcagttaaataatattaaaataagaataattgtcaagtcttatcaatccccaaaatcaagctttagagaacaaatgagcttctatattcaattattttatttatagtacgtgatagggttggacaaaactcccgaaccaaaccgatcgaaccggaatccgacgattcttctcaaattaaatacctaaacgggtatttgaatcaagaaccgatgggtatggttcggttctcggttctaggccaagacctaaaaaatcgaataaaaatcgaattttcataatttttttaattaatttattttaaataagtaaaattattttattttttctaaataaatttgttaactagttaatttagttcaaaccacaaaatatgatcttcctatttctaattttcagttcaaaatcaatttaatcaaattgacctcaatttatccaaatttgttattctactgtaatgtcgtttttaccggagaaaatcgaattaaagctctacaacatctctcttaattattttgagctcgaaatctttttctttctataattttaataatcaaatttatgaagaattcaacaaagagaggtatgaaacatataagattgaattacattattttgtaagtgctactattgaacatatcattaattaaattaacgtaactttggatatattaaaaaatttaattataatacggaaccgaatggaaccgaatcggaccaaatcggacccgaacggttcggtaattaaatttggatccgacggttccacttactagatacccgaaaatttcgggttggttcggttctcgttagaatcaaatcgaacgggaccatgtccagccctagtacgtgatctactaacactttcaataaatacaacagatcggagtctacttttaatgcaagtgaaaatattctatcttgctaggacttatggacaagattacatgtcataatatgaagtagtaatcacaacataagaatacattgtcaaaccctaattatagtgttaaagagggaaataacattaaaaaaaaaaaagggctcgtggaataagaaaataattttcgatgtgctagtctaacgttgagtgagcagggggtttgcattgagcaagcaccaagcttcctggttttagtgctcgagtaggagcttggagcgcagcaagcaaaaaaacgtccacataattccttggtccatatttttaacgtcttcaaggcccacttctactgatccaccaaaacccaaccaaatttagtttcaaacttcaacgaatctccacattaaaccaaatttcaatacgataaataaatttcaaagattctccacctaaagacaaattccactgtgaggcataaaattgaactctttgacaaaacatcaaacaaattctccaacgaacaaaacctctccacctctactaaaaaatctagctaagataaacttaaaaactgaatgtcaatttgaatccaagcattgctcagtcgaattaccttaggtaccaaagtagttcgaattattaccatgatcaacaaaattacaaaataactcaacatcactaaacaaggcaaaaacacaccctgtaatagaatcaacgctacaaactactgtgtagaagtttctttgctagacttgacaccttcaaccataaagcatatgttactaaattagctttccagtacctttgtggaggcctaatatctctcttgtgtctatctctaataatagaatatgatggtaccgttggaggtggtggcaaagcgacatttcccgtaacttctaaactcaggtgagatgtattttttgttgtagataccaaatcaaactccaatggtactataccaaactgaatatctatcaaagaacttaatttttgctcattggcctctaatgatctatagaatcctacaaggcatataattgagaccttctatctccatacaatacaaccgagcacctttactaacctttaggactccacttttgaatcaattgtacttaagaagataatatttctcttcaaatctggaacattcctcacttcatcaagtgtcctaactataatgccctaaatgtctaattcaaattgttacgagtattaatttcataactaaaggagaattttatccaaatagttttaaatatgaactaaagaaaaaaaaatcaatactttcaaaaacaaaacatcttgacccataggaaattaagcataagtttccgtactttaaattttaaacacttgaacgtcaaaacaaaaattaaaattacttctaaggtccttccgtcaatccacggcacagaactccaattaccatcatctatccagtttgctttaatctgtaaatgaaatcccagaagggtaggtatttaaacagttaaacgtcaacacaaaaattaaaattacttctaagatccttccgtcaatccacggcacagaacaccaccaattaccatcatctatccagtttgctttaatctgtaaatgaaatcccaaaagggtaagtatttcaaaatatagagtgagatacatgtaactaaacctcgaaataatagtaatcacaatactcatacaatctataccacatttcatagtgagaaatcgaaccatatcaaacagaaagctctatacatttctgtataacattaaaatcaaacagacagaaccatatcaaaatggaaagatttgtacatttcataaatcaccaaatccgaaccatatcgaacggaataggtattagcatatcatgtaagactattgtaaaaatattatatcaagatgaataaacactttgtatataaatttcttgccttaccttttccttaaaattctttggaatcaagcacttttcttgatcttcaataatcttcctttctttcttttcttttgtgtataaaactttgatagaattttgaaacgaaattataagaactctgatattttttattaataatttgtgaaatcagattttgtgtatagggcctctttaaacatgatgaaaatgctttattttggtcttaataggtgcaaatgaagggtcttcaattccccattattgaataccccattatcctcaaaattcaactcatttaaaccaatcaaaaattatattttaacccttaatttctgttggaacccgacccctcatcatagaaaaaataattttgccaaatagttcatttatcacatagattttttatagccgaaaataccatgaaaattacttttaaccatcttatgatcgaaaactttcaaaagttataccattgaattttttttacatttttatccttcattcctcatatctttatgtctgaaatctcaacttcaaaattcgtgaaattgtgaaatgacaattttacccttctagcctaaatcatcacaacataaccaaatctttcacaagtctctttacgattaaaaatacttaaaattcttcatatgaagatcatataaattatattttctctcaaatgaatatttaccttatttgtacttgagtcctcaaactttcaagatgttgcacttagtccttatttttccttgaaatttcaatcaaaacccaaattatttattaccatgcaacaaccacagtaataaatataaataattttcatatagtatattaaaaaatttcttggatattaaatcccttcccccttaaaagaatttcgtcctcgaaattacctcagttaaaaatatttatttcatgggtccattaattttgaagttgagatttcagacataagatatgaggaattaatggtcaaaaactaaggaattcaaaggtatatatgtgtgtgtgtgtgtgtgtattctaaaatgaggggttgatctagcaaaaattaagggtcaaaatataatttttgattggtttaaacgagttgaaaatggaggttgatggggtattcaacagtgggggggttgagaactcttcatttgcacccattaagaccaaaataaagcattttccatcatgttttaggaggtcctatacacaaatctgaatttcacaaataattaatcaaaattttcagattttttatacagaaaagaaaagaaagatatgaagatttttaaaaaatcaagaaaaaatgcttgattccaaaagaattttaaagaaaagataaggtgagatacttataggcgaaatgtttattcatcttaatataatatttttacaatcttacatgatatgctaatacctcttccattcaatatggttcgtgttcggtgatttaagaaatgtacaaaactttcagttcgacatggtttaacttatctgttttgaatgttatacataattgtatagagctttctgctcaatatggtttgtttgctcactatgaaatgtggtatggattgtacagtattgttgtaatattatttcgagtttgaattacttgtatctcgctatgtatttttcgaattagttaacatttttgggatttcaatcacagattagagcagacctgatggatgatggtgattggtggtgttttgtgccgcagattgttggaaggatcttgaagcaatttaactttttgtgttgatgtttaaatgttttaaatttaaaatattgaaacttatgtttaattccctatgtgtcaagatgttttattttagaaagtattgaagtttttttctttagtttatatttcaaactattcagaaaaatttttctttaagttatgaaatgaatatccgtaacaatgtgaattaaaaattcagagtgttacagttggttggtgccagcatataatttaagtcattcttaaatgtcatgtgtttgaattctaggggacgcaatagaaagctgtgaaggataaaatggtatatacccttccaaagcaagcagtacgtaaacgaacaaccaagcacgaggcctaagtcgttacactaactatcccatcaatatcttaactctaatctttcgaatatcggctatcttacaaggttcattgttacccattaccacaacaccttttgaaactattttatatgttgaaaacaaatcccaattgaaacacatatgaaaagtgtaagctgtatcaagaatcaaatccttgtcacgtttgcaatttgtcatcaaaaataaccaaaagtactccatttaccagtagcaattttctataatatagcttcacctgaagtttctggttgcttcccttctgattttcaaccaattttttctcaattttgtaacttatagcaattattctttatgtgccccttcttgcaatagttacaaattttatttttgaagttagacatcgaactacacctcttataatcatcatgaacaaaaaggccttctgcttgagcctctatccaaaaagatgcttcattttctcttttgaaaataaagtatcataaacttccttaatagtaagagtattacgactatatactattgtgtctctaaacgacatatatgaagggggcaacgaacacaacaaaatctgtcccaaatattcttcatcatacttaacctccatggtttctaaatcgcgacaatatcttaaaaaacagctaggtgatctacaagtaatgtattttctattatatgatgagaacacaagcactgcttcaaatgcaattttcttgttaaactcttcatcatgcataattacttaaatttcaaccataatactactgcaatttgatcctacattgtttttttctccattgaccaatttaaggacatcttgttaaatcccaacagagagtcatctaaatctatctgagcaacgcatcttcatctctcacaatgagaatccagtgctacaattcaaaaacagaatatcataattcataattcccatcataggaacgaaatcttggcgaatcaaatcttaacttctgataccgcttattaggaattatgaatgagattatatgccacaatatgaagtagcaatggcaacatgagaacacaaaaattcaacagaggaaaggaaaattcactacaatatagataaagaatacaaaaatattatgtttacaatattgtctaacatgttttaacttgttgagccaactatatataggatacatttccaaaccctaattatagtgttaaagatagaaagaaaatcaaaaaacgtatagaataaagaaaacaatattcgatcgaaaaacaacagagttagagtgacaggttggcagcaagagagcgtctgctttgagtgctcaagcaagagcttggcatgtagcgagagaaaaaatgttgaaattattccttggtccatattttgacctcttcaaggcctacttcagctattccactaaaatccaatcaaatttggttaaacttcaccatattttattaaggatcaggacttaaagaagaaacaatagagatcttgatatgtttaaataacgcagaaatgcacagttcttaattcaagatagagtaaaaaattaatagttgacgatttaaaagatcaagctcattataatttgtaagtattgtgcacattaattttcttttaatattccttaatttttagaaaaaaagtacacttgacaacttattcatgtataactttaactacacctacattaaaattaaaattaattgatttcaagccctaaaaaaggagagtttctaaaaatttaaaaaataataataatgcgacctctaagagttcttaattggctagttgccgaaaggcgtagtcgattgacaataggtgaatattcccatgacatacttgcgcttacttgaacataatttctttccaaaagaaaggttaattccacaaaacaaaaaagctggggtcgtgctctatcaaagcgaaatttctattcaatgtaaaatggaagtatgataattaccgctcaactcaacccatcctatgggcctaaatcgagcggcatctttcaacacaagcaaagatcgagccaagctcggctcaacccattgctatccctagctccgtttcctttgcgaaaatcaagttaaataagtgataagttaaaattttgatgattttgctcatttttaaatcatgttgtatttatatatgcgtatcaattgagtataagttagcaagcaacttcccctcggtcggttgaaccagcaggaagaccgagtcaaacgaaaaagctaccttgaagttccaagcatcatccatccccatccgagagcacccaacttgtttgttgacacgtgaggggaaataggagtctgaggtggtaggatttaccactatagacctatatatttatatgttcttatcaaccgatttattgagcataaactaataatatgaactagatcatgtaacttcgtccgaatatgaaactcttcttgaatcaatcaaaaaatcattttgttttgatcatttcttagatttttgaattgaatcaaattctttttctattttagagtgaacagtaccttataaaaccgtttagaatgagtagatgaagagaaaagaaaatttccctaaagggagctaagttgtctctccgcttgaacaatccactattacactttgtgctctacatactatattcctaaaaaaatttattcgatgtgataaagaaataaatagtttgtcaaagaaaatcttcaaactattataaaattgaatagaaaaataattatatatgtaattgaatttcaatttattaaattatttatgactagagcaattgtgatatttaatcacattcattcccctagctttcatatcacaatgtatagtgttggcccaacagagcagttttgtcatcggtgttcttttaatctttactcatttcactgctcaatagaaatttacctctacccataccatactctagctgagtagtttccacctcgtattcaagattgagtccagaaatttgacaatggactaaaatgtcacctataagctttacatcttaacattccagaaaaacacatttcgttgtatcataaagttatcttttttgatggagaaactggaaaagagaacgatttaatatcatctgtatattccatacataatactatggatcataaaagaaaaatgtggagaatgtaattctcaattttagttgacgataaacacgtggactcgaagttatattcggcccccgtttggccccattcttgccaaattttaatggttggaatagtgttttttttttaaatgtgtggttaaaaaagaatgaaaagtttttttatttgcgtataatactattttatgtaagattgtgcggttgaaaataaaagagagaaagaatgagaaggagaatgggggtcaaacgggatttcgatagactgtaaaatgaatcacgaataaatttagagtggatgtactagtagactaaggtggatggaaataaatttttttttttttttttttttttttgggtattcaaaacaatattatttgtatcgaaatttatacggaatgaggagttgagcttaaaactgaataaaaaaaataaaaataaaaatagtgcaagtgacattattttgaatgaaaacttataaatgctatctaccaagtgcgatctcctctaattttatgcataatttcttgtacgttttaatccatatgccaattgtatcttcaatgtttaataaatttgcagtatgaccatcaaaagttactgaacaaatttgggaaattaaatttgtaccaataaacgaaaaaataaaaataatataatctttagatagataatagaatcaacgtagtatcaaaatagccacatatttaagtatgagaggaaattacatctagtggcggcccacaccactataaacgggatagtcgatcacctaaggctccactttgattagggtgcctaattatgtaaaattaattgattggttgaagaaaaatgaaaattatatttatggaattctataaaataaaattatcatatgcagacacaaaaaattaataaaaattgaaaatacaaaatatttaaatataaataaatggaataaaacttatcacacacatttatttatcacaaaaattactctcttttataattaatttaacactatttttcgaacattccttttatttttctttatcaaacaaaatgtttctttgtctcatcaaatttcacatccaactgccacccactataattttttttcaacccaacaagaaataaattatctccctttgaattaaaattttaaaaattcaatttaatggattggtatgatttcaccgtcattgttacagccttacatgtttctttctttctcttttatcttcaaaacatatactgcaaactacataagcttttattatattttgttatactaattcttacagtcaacattatccaattttatacataaatcactcaaatgtatattcaattttgtttgaaatagttgaagtgaaaaattatcaaagaaacgaatggatctctttgtcattgcattgtaattctgtttgccgaacttcacttatacaaattatatattgaaatttaacatttcgttatattcctctttagtttttgggacttaattgtctgtaatagattcttcataattatattaaagtggaaattacataatctaatacatttaaagatttcatttcacaaatcatatgttaagttcactttttcaaaagtcggattttttaaattaatgaatatatttaaaaattaattaaacaatatatatataaattaattaattaacccaaacacaatttcaaaccctaatttatttttcccccacttccccccactccccctccccacgcctctctctctctccattctcacatctaccggaaacctcatttttatctctatattttgtagcctctctctttcttgaaaaaagacctgccgaagtgaagtcgcgcgaagcagcctgacatcgccaccatcatcacaagtcgcttcaaggccaagctcgtcgtttgaaaagacgagtcaccgccacaacgagatgcccccgatcaaccacttccatcatctccggtgccgatcaccccttcattcactagtgcttccacgcatagcgccattataatgaccgctgtgagagcttgctacaattcggcacgatctatgttcttcatttgcatttgtgatagagatagaggagatggtggacttgaagaggtggttgtggtgattgtttatgcatgcgactgtagtagtagcgatggcggtaggtggttgcgctcagtggtgtgcaacagtgatgatggtgagtgagacggtggtggagacaagtctggtgaggttgtggtggatctcggatgtggtggtattttcctgtgacgtgaagatttgtttgagacagtcgtggtagtggttctgatggtgacgacaatgattgtgctattggagtcgatggtgatgtggtggtcacaagttatttgtttgatcggaccattaaattggttaatatgtgagcaataaaaaatatgtgacaaatgaaaatgataaattgtgacaaaaaaataatgtgtgagttaaaaaattattaatttgcaatcaataatttgaaataagttttgatttataacatttataatatgtgactcgtaaataaattgtgacatattgatttgtgaccaattaacaaaatatgacctataaaaatttttatttgtgatcttgaaataatttatgacatacatagatttgtgaccttaatatatttgattaataaaatatataattaattaattaaatcataaaaataataataaatatctgatttttgaaatttgaaacctttattcttaattttgaaataaatgatacttaatctcttaattatgaatttttccctttacaaaattgaaaaaactaaagaaccaaattaagtgatactacaatttaaaattgaaacgatctcaattaaatcaatattttttctccaaaataaaaaatttatggttgtatattgcagaatttttggtgcaaaacagaaaaagataaggatttctgctttttggagattggcgatgcaataattaataccatgaaaattcgattgaggaagataataacataacacaaattggatgagagttgtgctgcttgtgcccgagattgaagaagtgcaagaatggaaggttttgggcgtaataatggttttcaaaatttaaggctgaaatgtgggattggattggatttatttattttgcacttttacttaaaaaaaaaaaaaaaaaaaaaaaaaaaaaaaaaaaaaaaactagtatttttgaaataataaagaagggaaagtaaaaatggtattatgaatttaattacggtggcaggtgtaattaggactattgtaaattctcagagtttatcaaatcacgttgtattttctgttagtatatgtttgtctgtaaaacctacatgcattctattgttcgtgaatgtgttggcattattccagaaagtattgttctctaagattttactagtaagatcaatttttgaatgtatttttctggatagaacttctatgctgaaatgagattcagtagattatgtattttgctataaatcttgatgctcaattaggatagtatagaagtagcaattatatgttcagttgcatggttgttgccgaatgttcaaaatcttgggatgtaataattcgaagtaaaacattatagcaatcaaataaggcaaaacctgtctaagcaattatctttcttcgtaatacataatgttatttttttcaaacgagtatcatttataatatgtaaccgtacccattttataacatgctattaaagtgaaagaatcttagtatataacatacaatactttatggcaatgtatgtaatgtggttttttataataatatatgtagcaacaagttagaagccacttaacatatcattgaaaagaattcgtaacaagccaataatctataaaatttacaattttgctcatcttgttacatatcaatattcacatgtgcctcacaatatggtgtgtattgaatctgaaatattaaaagcacgatactataacaaacaatgatatgcataacacaaatagcaatgataagttcgactggatctagaagttcaaatgcttgtaaatatgtcacattcatgctgcttcttcaccattttcatgtacacttatgtggtcaaattaagaagttgaaacttactaacgtgaatagccaaaaaaaacttattaatattattgcacaaagttttgaaacaaaataaaatatgaataatattgccttaaaattcagaaaaataattctaaattgtttaccgattgcaatagtttttattcagtatggtttaaatgtaggagttgtaatcaagatggtagttgtttattggttgttttatttataatcaattacttaaaatagactgacatatcaacaattttagcaattttatttttataaaatacttagcaatttgggatgtcattaattgtggacatgttaactgctattgaagtgtttcagttaaaaaaaaaaaaatcagagaaattacggagagtaatttttgttatgaaaagagaaaaaaaagagaggagaatatcagagtcaaaactcaaatgtatattattaaaaatcaatgtcctatatttatagggttcaaaataagagttacattaagaatgaaattgatcttctagataagataagacttatttatgtataatgataatacaaaataatcatcaataattatctcattattttacaacaaatttgatttattcttatataatatctagtatttatagtatataaaatatcatgtaataattcatgaataattattttttccttggttgtatgtgaatttttccctaaatatgatacagttaaatttcgttacttaatctctctaatttttttatttttttttaactgaaacacttcaagagcagttaacatgtccacccacaattaatgacatcccaaattgctaaatattttataaaaataaaattgctaaaattgttgatatgccagtctattttaagtaattgattataaataaaacaaccaataaacaactaccatcttgattacaactcctacatttaaaccatactgaataaaaactattgcaattggtaaacaatttagaattatttttctgaatcttaaggcaatattattcatattttattttgtttcaaaactttgtgcaataatattaataagttttttttggctattcacgttagtaagtttcaacttcttaatttgaccacataagtgtacatgaaaatggtgaaaaatcagcatgtatgtaacatatttacaagcatttgaacttctagatccagtcgaacttatcattgctatttgtgttatgcatatcattgtttgttatagtatcgtgcttttaatatttcagattccaagagaaactccacctcacaaggaaaaataaattctgctgctatcgtaccaaatatgcattttcatttaatattggcattgcatcaaaactaatgaacaatctgtctctgttctctccctttattgacataatattccatgtcatatatttttttaatcaaaatttacagaacttcaaaaatgtaaccaattcaaataccaaagaatacataattaaatgaatgcaaataaacatattctccgatcaactgtaagcacgtaaaaaagccaaggttaagcacataattttcttcaaatgttgtattaattttcaaaaattaggcacaagaatcaagtgtatcacaagtcctatgatttcaaaaaataaattcaatttgaaacatccgaatcactctagttaatgacagtatttctttagtgagaagtactcattccacgtatataacagttacctcgtctgaagggaaaaatgaccgcatgtcttcttgacctctgatttttaaccaacaatccttctggtatgctgaaaatacaatatgaacagcttgccagtgcattatccatgttcttaatttcagtgcacgtctgagaattcttcaatgaggatggcagcacacaaagctttccagatgggtactaacattgtaataggaggatgtaattcctggaaacaaagccaagcagtataatatgaaggtaaggtacatgcgaaattatgaaaactatagattatcttttttttttagatttaattaattaggcataaaataacctatccaatgtttatattttgaatttatatgctttattttgcccaaaagttcaaacttggaacatccttaccttgaaaactagtaagagttcttcttcttcacgtataataagagacaaactccagtaacaagtaactggggtcacgcattcatttaagacaggtttcaagatcttgcttataggaacaaagcagcgaactattctcccactgatttgtaaaaggcattaaaaaatactctgattagcgttgtaggaaatagaacccaacttagtcatgctatctatagttgaacaaatagaacatggataacaattacaggggaggaaaaagaaagacaaataatttaaatttccttctggaccattaaaaaaaaaaaatcatctggcgggaggaaataatggatactttgtaaaaattctctctaagaacaatagaccttatttttctaatcacagattacaatagcaaagaacttaaggtcaatggtggatactcaaatccaagtgacaaccaaatagcacgtaacagtgtgaattggtctttacaaagaccaaaaaacactatcttataatatactcttactgacaacataatacactgaagagctcacgcaaccccatccacacccaaaataaaatggcaacatggaaaaaaataaagctcaaatgatttcaaataattattacaagcatagctggaaaagaataaaagaatgatgatgttatacaaattacaaggtaccttctgtaagtagtttcaagctgaactccaaaggcaggcaaaatcgtaaccgactctgttacacagaaacatgtaacacaatattgagaaattagatgccactgcctttcccactctttcctgagagagagtactttgtgaatagcacataagattgcgttacacaaacaaaattgtactcagtgcacttataaagaacataatgataaaaatatcgcataacaattaagattcaaacacttggatagcgggcaacgagacaaataactctactttgataagggccaatcatccgacagtttttttttttttttaatataggaaatcaaatattttattaatcaaagataatacacaagaagtgtattatcaatttaaacaaaaaagaaacaatataaaattggacaatccatctacacgagcagtagccacagcattaacccaagtatacaatgtcaaacaaaacaattctctaatctactctgttgttcgtgtgtgatcattaaaacagcgactgtttctctctctccatacacaagtcatacgatgcaacccagaatagggtctcaaacaccgactatttctctttctccacacacacgccatacgatgcaactcaaaacagggtcccaaacaagtttactatccttattacaaaatgttctcctccatgcctttaacacatcttccatacgtcgcggcaacaaccaatccatgtgttgagaagttagaatagtgtttcacagcaaacggacatcgtcacaataaaggaacaagcagtcaatcgtctctcaattcctcctacacatataacaccaatttgtattataaaacccctaattcgaaggttatccactgttaacacgtccccttacaataatcctatagtccctaagttacaaaagatatcttttgtctctgatgttcaaatttaacaagatagcccctcaagttgtaatctgaagtcataccggtccaatttgtaagtcataacttgcagttaatcttcttgtggcaaagaaaccactgaaaatcctataaactaacatgtttttaacttttgattttgatttttcagttgagtaaattaaattatcagtcaattacaaattggaacaacttgctaccaagttgaaacaaattgggtcactgtatagaaataggaatatcaggaacaaaattagaacatcgtgaaagctaattacctatagatgtgatttacttgtatagttccaaagttctaataatctgaaaagtgaaaagtactaataatctgaggttgatacattatccaaacgtgtatattaaaaaaactccatcggtggctactgcagattccaggctatatcagcaatccattcccacaattaatttatatgaccagttatgccaaaaaaaataaataaataaataaataaataaataaaatgcctatagtgctcaacaattaaataaggtcttacatcgaagtacaggatcaacatttacttaataaaatctatgtaaattcgaatatttcctggacaaaatcctacaattcctagatcctcacctttctcaacttgtttcccttgccatgatttcacaaggcacgccgctaaagaaaagctaaaaagaatggccattgacaggtcctgcaatcatgataggcacctgtcatgttttgacaaaataattacaaaatagtgaagatgaagtgcagttttgacatcccccataaaaagttcaaaggaaaaatgtataaatcctcagaatttatcttgggcagttggcggttatataacaaaagaaacatccagaaaacatatgcatattcatttaagtgttagtggttgagacaaacttcaattttccctttttcctttcttgttccttgttttagtttcttgtatttaagtatctttaattatgcaaactaattatgaagaagcaaatgttattgaatcattaaaatacaggaatttattcgtagaagacaacaggggatatttttcaatagataaagaagccaataaatctttataacagtgtaacacaaaatctcgaagcacaagtaactactattgatatttgagcacaggaatttgtataaacatacctgtgggagaaggagaaagcagaaagtggctgaaagcagaataaatatgtagaaaatgtaacccagcgcactgcttcttgaaatgatgatatggtgaatgtcaattgcatcaggtggacccttgtttgtatcatttatatacgtgtatcgtccttccgaaatggtggctaatgactccaccatcttagactacatcaaaatcgaactgggaaaggacttgtaatgagttttatctccagttacctctcttcattaatcaattatagaccattcccaatatataaattgcaacatcttcagggaggattgaaagtcgaaacaatccagaatatttctcaactaatataaatgctgataaaaatttggccaaacttgatgaatttcatcattaaattttgtatttgttgtattcaccattgaaattaaaagaataaagtttatattagaagattgaaattactgtgcagttgatttactagggagtgtggtatattagttatattcaaatatgataataagttaatattagcaaataaactttgaatggtaaacatcaaagtgttgagttggtcaagcaaatatgacataacatgttataattaataactactccctacatcccaaaatgttgagttggtcaagcaaatatgacataacatgttataattaattattactccttccatcccaattatataggctgactttccttattttcttatcccaattttataattctttttctctatggagaatattttgttttattcgtttactaatatacccttgtttaatttgcctagttataactaattttccccactcaatcatgaaattgtacaaatataaataagggtagactagaaagtttttgacaaaaattgcttttcctataacattaaataaaatttcttaattcatgtgaaaacaaaacccgtttatataaatggaacggagtatatattaaaatgaatactaaatcagtttgatgacgaattttgtttttccagattcatctttcaaagatatgcatatttaagtttttcaatttacatgttaagctctatctaaagtaatgacaacttaccttttaacaagaaacgactttggataagataatgggaatcagaagttattttatcttcctcttgaacttttgcaaaatctggtacagcaagtaaaatccttaatactattgcagattctaattctaacatttggatcaccaattcacaagccagtgatcatagggccaaagaattcaattttcacttataccatacgtaccctctctggaaacaaaaaataaaaataaaacggtgtaatttttttatggaagcagtactcctgtttggtgccgaggaaatgtacctcactttcacattacaataggacaagtggcaaaaatgtcatgtaatcttcctcaaaataatttaagcaacttttttccctaaattgttttgcttttcataacctcacttcaagaaagatgattggcagcaattagaagagatatatcctttgctacatagataatgaggaaggaagaaacccccaggattaccaaataaagggaactacagagaaagaagccatataatagtagaggctagcacattaaatattagggcatccaaatttattctacttacaatgttatatcctaaattttgggccgagtggaagtaacgggagcactggaatttgtcggtgttctgctgcagaggaaatcagcctggtaactgtagatgtatatacttgagaagaagtatatgcattgcacctgacgttgaaataggctcacgagttggagttgccactgtggaaatggactatgaagcaggttaagatggcgtggtgcggggtgaagatctcgcaaatgaccgtgttgtaggtgtagcagaccttagagtgtagaggtggcagactgtggcgattgtgactcgaagtttggtactgaactgagttgggcgatctgggtagacaaggaggatcgtggcggcaggcgaatttctggacttgtcgtggtgacaggtggttgggtggggtggttatgcaaggctatgaagcaacggcgtgtggtggctaatggtgttgagaggtgccgggcgacgggaattggtggtggtgagcagcggagttggcgacggggaacggttggtgtgggtctgctggataagtggtgtttgccgtgcgatcatggtggatacggcaagaaactggtaggaggcggcactgtttgaggctggtggtatgggcgagacaggtggcagaaatggtgtgtgagtaattgcggtggttgtggctgtagacgggttgagaatgggaagagacgtctgcgccacaggaagtggccggtgagggtcaatctagggttggaaaaggctggtgtaggttgatcggaggcaggttgatggcaagtgaatgcagcggcagatcggctctggtcatagtggctgccgacgagaggagcggctattagatcagggttttggagacgtaagttgggtgtctaggattggaccgggtatttggttcgggccttgagcagagtcagttagtggactgttgggcgggtttgagttgtgggcactggattacagtttgtggtaggattgaaatgggctgtacggatatattttgagaaaaattcatatataagggattgaggaacaatacacaactaccacactataataagcacatttcataaataacaattttacaaaataatttcataaattaggtgataaatgataatttaaattaataaatttaatgatatataatatatacaaccgtgcaccctcactatcacatatttccacctcccaacccatattttttgccacaatagtctttacccaaaaaatagacactctatctccacatcaccacttatcacccactacccatcgtcaacgaatcgctctccttttctaactatagagtgactatcctcccatcactatgcgtcctccatctcaaatgccactgtcaccaacactatcaaacccactttcatccctcccccctgtcacatcccgaagtaaagtcaggtactgtcattggggctgaaaatttccaacataaaatctcgccgaaggaaattatagtgacagaatctttaagcaatacactagcaagaatggtgtctattcatagacaaaactcattaccaaaaaacacaaaaattattaccaaggagttgaggaaatttctactgctgcttatgattctgccagagttttttttttccttttttttttttttttgagtaaatggcatcaaaaaatgtttgttgtaagaagacgtttttatagagaatatatggttgaggtgaggatggggtgtggttaatctaatctgtcgaagttcattcaagtaaatggcatcaaaaactgtttgttggaagaatatattttataagggaaagggtttgcagtggggatggggtggggtggggtaatccaatgtaaatgtttagaaagtgggattgtggttgtagtgggatgatcttcattgccaagcacataatgatgcatttactcatttcaacattcgctgtctctctttgtactacgtggtgacaatagtgatgtgttgtttgtgttcaaacatgtgttatatgtgattaactgtgatcaatttattttcagtgtgactatttgtgattgagttagtctaaatcgtgattgtatgcagttcactgttaatttagccacatatgatcacaattaacatagatttgatcacaatcaatcacaattaacataaacttggtcgcaaaggatcaccatgaacaaattcgcacacaccgcagattagtaccgtaatgcacaactatcacctccaatacaccactccctaccaccttcaactcaatcctatgaccataaatattaccttcaccttaaatccacgacaacaatcatcaccgccatcatcacttccactaacaatcaacataaagatccccaatttctttaattttggaattcttctgaggatgtgctcgacaaatttaaaatttagcacgatggataactattaggccaattatgtagtcagagaaactacatatcactattaacacagacaaacctggtaacaactgataacaattaataaagacttagtcatggaatgtcacagttaaacatataaacggtcaccaccaccggcatcactactgatgccaccactctaccaccaccattgcatcatcaccaacattgcacaactattataaatgatgttttacccacttataaactttgaaggcttgacaaaacataaacaaaattggtctggtgaaaataaataaggtaaagggacgaaagagatttacataacatttatcattgcaatattgtcatatggcttcggattatggatgaccacctggtcatgagagacaaaaggcacaactgacaaagaactcaacagtgattggttggttttggaaaagactacttttacaatggttctttacaatggtggcttccaatgtgagctgaaaagggagaaaaccccaaaataaataaattaaaaaaattaaacgaaaaagcaacaaagacaggaccacaataattgactttgctacatcaacttaaaaaagggcggcaaaatggaaaagctctcttcatacaccccgttgagaaggacgaccacgactaacattgcgcgaaaaagctctcctcccccaacaaatctgtacgacttcgtcgaaaactaaccttcctagcgacagcatccggcttaacttcggcatttacaaaacattgtatctacaaaaccacccaaaatttttggtcgacattacactacatcgtcggagactcaccttccggcgacagcatacccatccaacttgagcccaccttttacagatgcatgccaacattttccccaacaatacaaccaatttagcagaataaggcaacgattgcgattgcgattgacgtttggagaccagcgtaaggcacaataattaacagaagaattgaacattgtttgaagactaccatttcatctacccaacactgtatctctcattcaacaaccattggtaataagaaaaaatctagagtatgtgaacatatgtgtcattaacttggatattattatttgctaatgttaaatcacttgcagtaatcctgaatccctcattttatctatgttaaatcccttgcagtaatgttaaaccttcattttatcaatgttaaatcccgaatgcattaatttgtaaccaaatgataacttatcatccacgaacgttaaaaaataagaaaaatgaaatatcgattattattaaattttttgatgcaaaaatgaaggtatacttacaactttgagtagacttaacccttcataatctgttgttatttaaaactctaagattattgttttttgaatgggacatttcattttgacccagtctgtgaaattatggaagcaatggaagatgtcacaagatcggaattggaaaatgcgaatgtggaagacaattattgtgaagatatttatcatgaaattcgatattatcaattgctaatgttaaatctcttgcattcccggtgaaaaccgtagataatgttggcatgaagaagggaaaaaatgagtatgtgaagatatttgtcatgaaattcgatattatatcccttgcattgtcaatgaaaaccgtagataatgttggcatgaagaagataaaaaagtatacttgctaatgttgaatcctgaccgaattaatttgtagccaagggttttcatactattcaccatggtaccttaaagttggaaaaatggaaaattatttattattacattttttgatgcaataatgaaagtgtacattttttcataatttgcatttttggaacaactttggggttattggtttttgaatggaaaatttaattttgacgcaggctgtgaaattatagaagcagtggaagatgatgtcagagtagaattggagcatgtgaatgtggaagacaatatgagcgtatgtgtggatgaaacgagaggaggagatggtgtgattgtgcctgaggtgggtatgaagttcaaggacgaaaatgaagtttacgatttctatgagagatatgcatttgaggatggtttcccagtcaggaaaaggaattcgaagaaagatgacaatggagttttgcaatatgtgacgttgacatgtagttgtgaaggacgacgaaacagttctacgagcggctctttgaagccacaaccaacaatgcagacaggttgtaaagccaggatctctgcaacttttgattatcatggtttatgggtaattagaacagtacaccttgaccacaaccataagacaggtccttcgaaatcaaggttgtatagatgcaaccgagaaataagtgcacatgtgaaaaggaagattgaagtgaatgacctgacagggattccgttgcacaaaaagtttcaactctgcagttgttgaagcggaaggttatgagaatcttacttgtgtggaaaaggactataggaactatattgaaaaagtgaggcggttaaaacatggggaggagatgccgtagcaatacaatcttacttttcagaaatgcaagcagggtgctcaagattttacttcagtattgatctggacgaagattcaaggttgaaaaatatttttttgggcagacaatcagtgtcgtcaagcatataaggagttcggggacgttgtcacgtttgatataacgcacctcactaataaatacgacatgccgtttgccccattagttggcataaattaccatggacaatcaacactttttggttgtggtttgttatcaaatgagaacacagatacttttgtttagctatttaggtcatggcttaagtgcatgcagggtcaagcgctaaaaggaataataactgatcaagacagggccatgcaaaatgcaatacaaatagttttccctcatatgaagcacagatgatatttatggcacattctaaagaaattgccaaagaagtttggttaccatgtggacaggggatcgatattttcggctatacacgtattagtgtatgattcgtagaatgttgaagaattcaaggccggttggaaaataatgatagataaatatgagttgcaagatagtgaatggttgtcaggtctttagaaaaatttaggtcaatgggttccttgctttctaaaaacatcgttttgggctgaaatgtcaacgacacaacgatctgagagtatgaatggctttcttgatggatatgtgcacttgaaaatatcgctgaagtaatttgtggaatagtatgaacatgcactacgaaacaaggtggaaaaggagttccaaactgatttcaagaaatttttgcaaatggttcagtgtgcaacgacgtatgaaattcagcagcaatttcaggcagtatacacaatttcaaaattcaaggaattgcaagcagagttcataggaaaggtatattatgacatcatatctaccgcggatgtttgtccgaggacgacctacgaggtatgcgacaatgtactatgcggggatcgataaaaaagaaaaagattcgtagtgttatttaatagggagaactatgacattatctgcacttgtcacttgtttgagtttcggagaattatttgcaggcatgcaatcgtggtacttatttgtaatgacgttcgtgtactcccagacaggtatgtacttcgaagatggaggagggatgttagtagagcacataccagggttgctgttaactatagtaggttggtcagcactcccggacagttgcgttatgatagaatgtgtcaggctttcgccattgcaaatctagccgcagaagatgaaggtcagacctatgcgataatggaatggataggcgttcaagagaaggaacttatgagttcgagatcaatcagcggaagcaatgttctactccaacgtactactcaagtgtcatcgaacaacataagttcgcaaaaaatgtaaattgcacagtattggaccctaacacagtgaacaagaatggtgcacctaaaagatttcggagaaagggctcattagagttgatgtcaaagaagccaacggtaagttcacgtgttaccttctcaagtgaaacggattcctaacattatatctcattttttggactatacatgtaggctccatcgaaaggcaaaagaccaactgcaaggcgtacttgtccaccagatggtgcattgtccattcaggctcatcaacaataagaatcgtcgatgcccattcgttctcctactcgcagctcttgttggttagtaactttaatttatcccgttcgtatgtttgttgtgtcatttgtgctttcttattttgatgtagggttaccatgaaagctaaatgtttccacaacaattaccaacttctacaccgatccattcgtcgtcgacccatccaacattcaattctcgaggtacgcatttatattaaaccacgttccttttttatccataatttgtgtgcatagattaatgtcgtatttcatgcacatccttactactatccagaggaatggcatcaagttggcaatgagttttgatccagtttaatgcatttaccagttgaatataatccctagagaagtgaagagtcaggagaaaattcctccaattacataattcattatcgatgaaagacaatgattttcaacttcagatcttcaacataataggtaggtacaatcactgaacactgattagtaaccccaatagtgacttccctctgcagccactcatttgctttacaagtagctaataaatgaccacttgcggaagtttggtagtatgctagagtgtatatatattgtattctcattttgttgatttagctaattttttgttgcttgtgcagcaatgaagctacttccttcaggaggaatcgcagtctcgcaaaggagctcactatagggactgtggcatctgtcttcttgcagcaatggcaaacctttttttcaattggcaaggttttggatccttgttcttgctactttcttccagtatctatgtttgattagtttttgtattaaatgggacgagattttgttgagcaaattaaaggttgaaccccaaccttaagggtcccccactgcccctgccctggagcatcgtgagcgaggtaaatcgcaggttatgcctccaagagtacagagtggaaggctgcttgtacacttgcacttacccaagagccaaaaaattattatttcagaattcgagcccttgacgcggcagcctcaagcaaagctggatttctccaccctccccttttaccacttggagatgtgccctgggggcgattttgttgagcaaattaatttacatgacgtgttgcttatttgaaattgtgggtctgagctatagcttggtttcaaattcgatggtaacgtctataaatgcaatttattcgccttattctcatttttttcctgatattttttaattggtttcctagaggaatagctttggttatttgcacaaacttgtgacttcttgcacttggattttgcttctgaattatatttttcctcccatctatctttagttatgttttaatgaaatctaaatatgaaacaagacgttctacaattataataatttgaatttttggaacattatcataataatcaaccacataattggacatttcataatagtcagtttttcttgtttggtttagccgcagcctatattagtctactgaagctattatttgatgacattgtttctcatatagtgatcacccaccatccaaacaagtgaccgaagaccttgacaaaggccattgtataaagttttgtaatgtcgagcatgggcatataagtttcttttcatttaccaaagtggaactttctgtccttccatgaccttctcgggaccggccatatgcaggtgttctcagtagtttggttcagattgaaaatcataagaaagacagagacgttatcatcttattagggatgtcaattgggccgaactggctcggctcgtgaaaaagaggctcgtgggcggctcgggctcgtgatttcatgagttgagcgggcccccctggctcagctcaccgtgtagacgagccacgagccgagcagctcgtggctcgtgagcctgtgaccgttctggtcactgaattcagtgaccgtttggtcattgaactttttttttcacccctcctcccccattgttttactataaatacccccttcccccaaatatttttttttcatatcaattgctcttccaaaattacaactctctcaactctcttttattatatcaattatcgagtttttactctcttgtgctgcaaaatatacaatatcaattcaattttttcagtttattagttacaatttcaattcatccaattctcaattctcacaatctcactacatttatattcatctaatcaagatttcatcataaacaatcacagaaatggatcaacgttcatttgttgagagcttgttcgatacaggatgtgagccattgccacatcatggagaatcgcctaggacgccgcaaagtcaattttcaaatgaatttgtcagtctaaatgacataccgatatctgaagatgttcacattcacgatcagggaagccacactccaattgatttggatgatattaatgttcccgaagcggaacatgaagatgaagatcaacaattaaatatcccagatgcgaggggaaagcgaaaggccaaaaaacaagcaaaatgttaggatcactttaagttgatttcaacgggaaaagtcgttgatggccttgcagaatctaaagcagtatgtaaatactgccaacaaagattgacatggcaaaaaggaattggtaccactcatctcaaccgccactacaaatcatgtgcagccagacatggacttcttccagctggtcaaacacaattacaatttggcagtccaggcgtcggttctacaacttcacccctatccacgtgggtgtattcggaggacgagactcgaaccggaatggtgaaatttgttgccgccactgagttgcctctagctattgcagacaaccaacacttcatctcgttcgtaaaagaatatctacaaccaaggtacgttgggataagtcgaaacactcttcgtgccgatacaataaattatttcaataattcaaaacaacaattaattatgaatttgcaacaatatgggggtgttatatccttaacttctgatatatgggaatgggttaataaaaaagtatatatagctgcaatcgcacactatatagacccactttgatgcaggcataagaaaattattggttttagaattattgaatttcctcacaatgctaataatatatataatgctattatctgtatttttagagaatatcaatatgagagtaaaattcgatcctttacttttgataatgctagcgttaataaggtagtcgtcgataaattacgtaggacacttcaacctgattttggtgggtatttgtttcatattcgttgtgtgtgtcatatcttgaatttaattgtgtaagatggtttaaaacatataaaggatgaacttctaaggattaggaatggattagtatatattacgatctctcctaatagaaaacaagcatttaaagatttttgtgtcgaactaggggtgatgactgctaaaacatttgttagcgacgtaggtcatagatggaactctacatacatgctattaaaatcatgtgaagatttcgaaaatttaataactgacttttataataatagacatgttagaagtcatgatgatggtatgttaaatgaatcccattggattttagctttgaaagttaaacgatttttgacatctttttatgagaccacaaagattttatccggcttttattatcccacaagctgtatggtgcttgaacgcctttatataattgcaagaatattccataaatataaaaatgatcttgcttttagtgaaattttaattgctatggaattaaagtttagaaaatattgggaagaactgcctatgttatttcttttagcatgcgcattagacccccatataatatttcggaaactaaatacgtaattgatcaaatcaataaagttttaatacttgatacacctatcacctataagaatttagagcaaacattatgtggaatgtatgatttatatgtcgaaagaatgggtgcaaatgttagtcgggtaccctctgctgcacctattccttctgctgaaactgaagaagatgttgcggaaataatgaatttatttcagggcattaatacatttagatatgatgcaattgcaatgtgttcatctagtgccatgtcgtctacatctgcatctcatcaaatatcgaccgaaactcaaaatgcgatgcctgccgaattaattgattatttcaatcataatataccaacagacagaacaattaaaaaaacttcagaagaagtaattgaattctggcgaaagtatgaaagacgttggccaatcgtttctgcaattgcgaaagatctattgacacctccggttagcactgttgcttcggagtctacttttagtgcaggtaaaagggttttgactgatgtctggagtcgattgaaagaagatgttttggaaacattaatgtgtgtgaaggattggcaggacgctcattttcgactacaagataaatacgctgaaattgcatgtcgtcaggtaagtgatatttgatttaattatattaatcaaaatttttttattttttaatcgttaaatttaattttctttaaaaaattgtacacgttacaacaagttgttcgtgtacaatttttaacttcgcctacttaaaattgatgtagccagtcccaagcccggattaaggaggagggtttacattttattaactttaaaaagaaataaaaaaaacattttttgtaaatgtatttcaaaaaataattcgttttcattatataaatattttatactttataaagagtattacaaattacaatatgatataaataaaaataaataaaaacttgttttcattaaattatttgtattttttaacactttttatttttaaaactctattctttattaactttaaaaagaaatcaaaaatatatattttttgtaaatgtatttcaaaaaataattcgttttcattatataaatattttatactttataaaaagtattacaaattacaatatgttataaataaaaaaataaaaacttgttttcgttaaattatttgtattttttagcactttttatttttaaaactctattctttattttatataaaaaaaaaatagcgcgagcccacgagccaagctcgcccaatttcaacgagccgagcctgagctcggctcgttgaaaacgagccacgagctcggctcgccacaagcacgagctgagctcgtggggttaagggtcgagctggctcgactcgacccattaccaaccctacatcttatgtagtgcaacctattaccatgtaatctatgtattttaagtgcgtgtgtgttttattttattttattttgctgcagattggtttctatttttacatgttaaaattgttgggatataagtcccaacagtgcattgaaggaaaaatgcatttttactgtgttttattttatttgatttctatgtatctttagtgcgtgaaagtgtagaaacaatgtaatatgaaatggtagaatcaacagcgcgttgaaggaaaaatgcaaggtttgaacagacacacaattcgatccattgcactaataacaaaaggcattacattacgataatattgttcaaactagaaaacctccaacctaacattgattctgctaacataaacaaaagatttgacataactaaacacaaatgcaccgccaatcaagtcggcctcttgcccttggtgttccattcggtgcttgaatttcccattcggatcgtcacattcacataaatgtggagttcttgtttatcatttagctgaacttgctactaaaacatgcgggacatatcatcaactaattcggtcagatccggcttcggcaacataataccaaagttcttggctttgccctttgattccccttctttgcaccactcccagaaaccacatttaagactgcaaaatttgaagaatttgcctttgttggctgtagcccattctacctcaaagcatttctgaaagccttggttacacattgggcatcgaacttttattaggcattcggcaaaaaagtgggctttactcctacagctgtgacatatttcggagttctttcttgccattctaatatgagattcagacaccaaaaacataaagttataagatagatgtgaagtatgatcgatcattatgaacacttgttttacaacaacagcatcaacaaatactacattcatgcacccgaatacttgccaagcttctattgcattaatatttactatctctaggaaataatatttagagtgctaaaacatgcatcatagccaaaacagttaatagtgatttcacttggaacatttggagtagttagttatatatgctaaaacatgcatcataaccaaaacaagttagttcatgcctctagttttctgagattcatatatgggccttaggatttacatatgaagcttttcaaccccagaaccagtttgaacaaaagtaaaaaatttatacactttggaacattagtcaagtctcagctatgcccagaaccgatttgaacaaaagtaaaaaatttatacactttggaacgttaatcaagtctcaactatgaagtttttcaagcccagaactgatttgaacaaaagtaagaaatttatacactttggaacattaataaagtctcagctatagatattttgggataaaagaataaaattaacaatccggcacatgcactcatcacactaacaacaaaatttatacaatagccaacacaaacaatatacttctccatgcatgaaaattcgaaaaccaagcaattcttcaagaaccacttgtatgaaaaaacatagatattataaaagcccagaccccaaaatcatccaaagataggaaaaattcccaaaattttaactgacccagatattcttcaacaagaacaacataccccgaatgcaagtgtgtagtacatcaaacggcaccataaagttttttaaaccacgtaccttcctgtgaagccactttccttaatattttcgttgaattgatacttcaaatctgagtagatgagtctgcggtagtcagacttctatggaaacggtatcaattttctagctttgtatgcgatgagaaagtcggaggtgatgcgtgcacctgcggcggcgtgcctccgacgatttgaaaagaatagcagccgttcaccacaattggggagaaattagagagagggctttttcttttcctgtagcgtaagagtaaagtttatgaattagagagggctatttcttctcctgtagcgtaagagtaaagtgttttcatacaacaaataaataaagttatttatttgacttagctgcttttccttttttgcccttgacagttcacatgcaaggcaacattgtacaagtagcgcggtcgattggtttttcatcaaaagtgcattccctagcattgttggaggagaaataatcgtgttttttattagacatcatcaaaactcctttaacccatctttgtcagtcaaccaaaaacgaactcatcctcctagccacaatccccaacaactacactgtcaaacacagcatctttagttgccaataggacattagaaccccattaatactccacttacgtggcattaaaacaatcactatttccctagcaaagccccataaatttgtaaattttcaccttatcacaagccccatcatcagttgccaatagtaattttgaaatttcattcaactccaaaatgtcattcaactcccttgtacgtagcgcgccatgctatgtctagcttttacttccaaagccccataatagcaacagtcgccggagtaaattttcttctttcttttgtcgtcggagctagctatttttgaggatgtattgtttatgtgagaaggagggagaaaaagttgagatgtggttcctatgttaaggagagagaaatagtgagatgtgggattaataaatgttaaataaataattaacccctaatttgtgaaaagaaaatttttaagatttgatatttgaaatgtatactcaaaatgtaggtttttgggtaattttctcttataaatattacccatttcaaatttaagaaacaaggtttaaaattttaaaaatcaaatattaattaaaatttatttataaaataattaattaaaaatatattttattaattaaatatttcaatatcacaattctatacaatttgatcacaaactatcaaattaattggtcacaaattatttgtcgatcacaaatcaaaaattttatagattacaaataaaaaatttatacttcataatttatttatcgatcacaaatcataaattttataaatcacaacttattacacggtcacaaattatcaaatcatcgatcacaaattaacaaatttttattttacacattatttttttgtcatgatttatatatttcattagtcgcatattatctagtgttatatattaagcaatttattggtcacgatcaactaaataatttttgatcaccacaacacttgcgactaccatgacaccactgtctccagtggggcctccaactccaccgccaacaccaccacctcttgtagcaacatcactatctctaataaaccaacaccgcctcctccaactaactagcattttcaacttcaaaacaaccactactagcaacaagatccaccaccattgccacccacaaaaccatagtcaccaccagatccaacataatcaacgcaaccattggttccaacaaagtcacgaccacctaaacaccaccaccacaaaacctccacccactaattgaaaacataataaaaaaatcacattagaccatggcgctgcaaatcccgaccatagcatacaatagatcccaaccacgacgtgcagtagggttaaatcagcaacaaagtaagaggcaagggtcagcagggttgaactagcgatgatcttacctatggtggcatgacactcccacttggtttcacacaagaagcaacactacacatagctattccaactagagtgcacgtagcggtgcttgcttgtgttattgtacacgttgtcgctcagcatggcacagcactcgtggccatcgctctagttgtgctcgttgtcgtcactcaatcgctgtgtagagaaataaataagtgattgtgagggagggggtcggttgtaacctgtatagagagaggggggattaggaaataattatgttttgataggtagatggtagtgggtggatatgtaaaataatatttataatattattattaataattagaattttaattatatttgatttttgaaagaaaaatttagggtccatttgattgcaaagatggaatatgggtgaaaagaaaacgaatttcagataattgaattgtctagaaattattttcctgggaattgtaaattattgttttttgttggtatatttgttgaaataaaagtatttttttgtgttcgtttgactttattttacatgaaaatcgtcaattaaagaaacaggttttactggtattgggggtgaaatttggatccattaccaaaaaaaataaaaataaaaataaaaaaatcaagaaaattaatcatctatatttttgtgtttgtttgactttgttttacatgaaaattatcaattaaagggaaatatttttttacaataattcttagaatttgtttctagtgcccaaaaataaaaatactacagtagccgagaattggaattctcaccattccaattcactgaaaaggtgaaaattggcttatgtggcaagaaaggtggaaaatgaattctagggaaaattttgccaatcaaacaacataaaattggaaagataaaatttcaattctattttccttggaattccatgccaatcaaacatggccttataacttttaattatgaattgagatcttgaaaatatttaatccatgtaatttccaaatatattttttgggtaggcaatggactagtggatagtttttggaccactaggcttgagtatataggttttagatatagtggaaattacacccaagcagattttctaagatccaacttcaaaaatgagattttaaagttttttttatacaaaagttagatgatagtatatttttctaaataatattataaaatttaataaatctactaacctaccacccactaaaaccctcatccccacccaatttttaacactaaaattttcatctcctctttttcctcccctttccttccccctctcccttcctttctccattgtttatgtcaatggcacatctccattgtatatttgtcaacaatgcattgcatctccattttcttttgtcgataacacatcgccatgcaccaccatcataagaagtggcttgaacccgaccttgttgatgagtgtgttttacttacaagttttgtactattttaacttagttattagctagatcttataagtattgaacatttgaatatgtttattaatgttattttatagattttgtgagatggtattaatgacagcaaaagtggaaaagataaatgacttggaattaaaggaagagaaaataagaagaaaattggcaaaagagtaaaattaccatatcaaaataaaggggggaaaaagaagaagactacccaagaggtggccctgatggtctaaggaggcaaagctatggaacctcagcaccacaggaaaagtagcaatgacagcatagggccgcacattaggtgctacgatcgccaccttggctggtgacgtaacgccacttccaagtgctaaggcgtagcctgagagtaactagggcacggaatttttggctttttaaggcccacaaaatatctaaaaagttgggggaatgaaaagaggcacctatagatacacgaaatgaagcaattgaaaggggtggaaaacgttgagaagaagaacatacaattggagattgaagagctcaaatcaaaggggaaaaaaaaacatagaaattcaagtttgaagtcttgaatggacaaggaacaaaatcttagcacaagagtaatctctttttttgcatctttattcaaattccgataatgtattcaataacaatttctaacttttctttttgcattatgagtagctaaatttcatgttaaggagaacaatgtagtatattttggaccatttatttttttattcaagattattgttgtttttatcatatatatgttgattttattatgagtttaattggttgaattatttgattaataaattaatgattttgtgaatcttttacgaatcgggaggtgaatttgagatttagaacacatagtaaaatttgataatttagtataacatgtacatatacctatactaattaattgtggttgttatatgaatttttataactgatgtttcgtttaactaagattgattcgcataaagatatatactttaattagttaaataggcacaatgagaactcaagaggagtgaattgaatacaattgaacactacattaggttattgaatctagaattaagatttaaaggtgatcaacagatgaaattgttatgcccgatatccattccatatttaaattctaaatcaatctttgtgtgctttcttttattttcaagtagttagatcaaatatcacaacaatttttgtttgttttcatcaaatgcaggttagaaatgttaaattaagtattaaattattgtactcataaaaatgataatccggacttgaaggttctatatataacttgttatgatatcgtacacttgcgctagaaaaacgtaacacctgtgcgcagctaaaagtgaaacctctatagcaacgttatcgctacactcactctcttcctcttccctttttccatcttctatctgttgacaaagtagccccactccactatagtgtgaagcggcctgtgaccaccacttattcacttcgatgtggtttcttccttatcaatgtttttgtggttttttaaccgtaatgttttctttcactgctcaattgttgcgatgctttatgctacgactgttgcgactttttttagtggtctctatacggtgctagttatgtctagtagctatagtgcgccttgtgtcttctgctgtagcaacgtcaaatgttgtaggtagctacaatcgacgttgtatcttgaagtagcggtactcctagccgagcaacactctgtagtctcgtactacagcgcatattgttgcctatccgacgacgatggtcgttgttttccctaactcgtttagatccaacatttttaagcgaaaaaatttattttctttcaaaaacaaatttttaaaagatggaaaatgattttatttaattgatagattcaagaaaaaaataaataatcaaattttgtttgttctgagatgcaaaatattttctaacaagcacaaggtagttttgataccactattgaaaatttacgtaatcatgcacagcgacattcaaaacaacttcaattcccactaaggatttactttgtgttgatagaaactatgataagaattatacttttagttaattttgcgaataacaatcacgatctacaatcaatgaccgtccaatgttcagtttccaaaaaaaatccacaaaaggaacaaaaattagagaattatgatttttctttcttgtgctagcaagataataattgtcttttttttttttcaaccctaacatcttattattagaagttcaatagacttaggccatcacttaaacttaactcgattcaatgtttaattaatctaattaattaaacttggtccatgaattaatttttttaaataattaattttgctcattaataagtaagttaattaattgaatgtccaacacctctcaattaattaattagcagcatcatttttctagttctcgatgtgacccgttagattcccaatcatgatacccaacaacgtgaattattaaacacctttttaattatcattattttatctaaattaatcaattcacatttgtggtctcaaattgacatctagccatatgttagggtagtacatacaataaaaaaatatcgcgtgatatggcaatatgatcaaattaattacgagacatgaaatgcgccaatcttgattaacgatcatatctttcatcctattactaaattagtctaagtcgaaaactcttttctacttatgagtatatcttggacaaaagttttattattaacttaactgaataaaatgtaaattgtaatctcttattatttaagagtgacaaatcttctattgatcatttataatcttcatatgattcttgacgtatttgaacgatgttgtattagtgactcttgacagagcaatatctaatatcatcaaagcataaccgtcccatataaggtactttaataaccttaagtcaaatgaccaatttcactatcaaatgttaaagattgactcctaatactccgatagttattcatgtggaatctctccaacaaggcaccaatattttattcttttaattaaacattcacgtgtttatttaaatgtcacatattttagcttgtgagatcaattactcacttcacatgtaacaccccaattcttattattatttttttatataaaaactggagtgttatgaaaaactcaaattttcttttaaataaatgcgaaacgacgcaaatcaaagaaattctttacttttaaccataaatatcaatttatacgcgagatttgagtttctaaaaatttgaattaattaaacaaatgagtctttaaactaacaattaaatttagagacataaaaagaaacaaactaagtattcaatatattttttctttttttgattcacttgacagtccacatcaccatcatgttacaactccaatcgaccctaactaacttgtaaaaatttgtaagagtgagtattccaaaacacccagtaagatacgtgctgttttcataaacaattatataacaaataaaatctacacttcataccactctactcttatggagtatatcggtgaccaagcgatacatccatcttaaatcatcttattatcccgtaggatttcatctctctttttatagaacccaaggctccactggcaatccatgcatatttaattgaatataaaagcaaaagaaaacaaaaacacttgcttaaaagtatcctatctcgctaaataaaatgaaaatatgaatgtatgtgctcaaaatcttttctctgctttagtgaataatggttgcaaattggcttcttttcttgtaactcccaaaagtatccccgctctctctctctcacgtgtgtgtgtgtgtaaattttttggtgtggtgaaatatgagacccttgcaaagtatttagagtaataaaaggtggttgagtcattattaaaaacgtgtactacctattggaaattgaattgaccaattattctaataaaataagatagaatctaatggaaaagcaattgtagttgtagccactcacgtgtggtaccaaccacctaactaattaacaactcttgataaagacaacatctttaaacttattaatctttggtctaacttatttaaattaactttttctcaagtcaaagacttctaattaattatgacctttgaaatgagaccaatatcgatataccaaatcttgttccatcattatctaattattaaatctaactaaaatagaaattaaaattctaccattttagtccccaacttttaaaaatataacaaaaaatttctttttttaattatattatattatttttttttggggttgctacaatctacctaccttaagaaaatttcattctcgaaattacctgcattcgggtcttccgtgacctgtccttgggctgaagtaaaaactcccacctttctcttattttctagcttgtcattcttcttcgaaatgtcctcttgtagtttttggaaatatgccctattttacagcatcgatagcacacatgcttcccaaacagacgttcacctctatgcattctgttgcactttgggtagggtgaaacgacttgtccaaaatttgatccaaagttaacctttttgttctgtccttatcctttctcttattggaccaattccatttcctctttcctaaaggctcagctccttgctgaaaagtttggtaaatttccaacatatttgagattgtttgggcagtctgcagtattcagctgtaggtggtagattgatgggatgccactattccatcaatctcatggtacaatcccaactcgaacctccatgctttctttacttctgtgtccactagatgtggtgcgtacctagagagttgttcgaactttctctcataatcttcaagcttcatctttaccggtttaagttgaaagaattctgtctcttttcgatctctcagagcttgtaggaagtatttccccatcacctcgtctttaaattgtgtccaagttctgcacattattgtacctctgttttggtgcgtgatgctgactcccactagtagcctacatcatcaactgacatgaattgtgcacataataccttctgagcatcagtgtaagatagatatttgaagattcgctccaaccctcttatccatttctcagttgctagtgggtctgccttaccatcaaaggttggaggcttatagcgatgaaactggtccacaattgagctaatgtttgcattttaggaatcagcttgtgcttattatctactcagatcttgtacaaccctcaacaaatccctaatgattgtagcttggtattgttgttgtcttgccatttttttaacacataaaattttaatttagaaatatttaataacacaaaaataaccataataagaataataattttttataacggtgaaaaacttaaaagttttcaaatcttttatataatattttgttttcaaatataataccaaaaagataaacattccctaagtaagcaaataacatctatttctaattttttttttgtcctaagaaattaattttggtggagtctcttcgtctgaagtaatgcataattctagctcagaatccgaaatcgaatcaatgaaattttgtggctcgaattcttgctcaggttcttccgactctagtttgattctacctctaggtcctcttcaagctcttcctctgagtcctcattaggctcttcctctggctctggttccgattcaagctcgggcttaggctcaggctctggcactagctattgttgtttgtggttccatgggattatgatagcttgacaatatccattaaaatatatcatatcccattcttcttacgaatacagcccataattcatatccctcatgaagtaagccatgtctctccattggggctgcataatacttatgagatgtatatcgagaggattgtcccctcattatatccaaacgattttgcttctcctacttaaaaaggaaaccctcaacatgttcaataaaggtttgctcccattttactttatagtttacgtagttttcaatagcaatttgagcacgttgaaggggtgttgggctatttccagtcattctggttattttccaaatcctaattatgtgacaaacataatttaattatgttagatttggagtgacggctagtttcaatcaaagttcgcatagaccatattcaaaaattcaacttataagtcacgcgtggtaatatacttatacatttcatgatatgtagaaacataactcataaccatgctagaaaaaaaattgattcatttcatactcgggatcaactagagagtggtcgaataatgagcgccacgtgccaagtattcttataacatttttcttaacaatacacacacacagacacacacatatatttatacacacacacacacacacacacacacacacacacacatatatatatatatatatatgtgtgtgtgtgtgtgtgtgtgtgtgtgtgtgtgtattgtaaaataataaaataattatcgatgactatttagtgttatcatgatacctagataagtcctatctagtttagaatatctattttattctaactgtaactcttattttggaccctataaatatagggcattgattcataataatacacaattgagttttgactctctatttattctcttattttatctcttccctttagttttataatacattatcagcacgatagtttaaattttttatataactcaaaattttctttgaaacaaaaaagatccatttgccactcgttctcacctatcttctagttctcgcccttgccatcaccatctagttgtttctattatcacttaatgcttccatctacctctgcccgtcgttggatttgatcaaatttgacatgtttccatccattgtcgaaaaccagaccaaagcaacaccacgggctgacgaatttaattgcccccccacacacacacggagtgctctcctagagaaagaaataggggaaacttttccttttagttaattcttcttcttcttcatcacaatatttatagatgtaagtgtatatgcaaacatatatgcatacacgtatgtgtgagaaattgttgttgtgttattgatttggattttgaaataggactggtttgataatactaaaaattgtaagtagatcttgatgtgggttgaagtttttgtttttgttaatggttttaattttcagaatttatgcgaaacgtccatcaatattaggtcaaaacgtgaaaaatgcatttgggtgattgattgtacatgttttgagttgtttgactagaaagggatgaattccaataaaattgtttgccactatacatttttttaattcatttgtaatcattatgcaattaatttatatttttatttgctaccaaattttcattttgtcaaattctgatataaaataatcatctttatagtaattatgcataattattttaattaaatactaattattcactaatcttaattagctatgttttccccgaaaatattcgatgcaattatgactttgattttactatgaatacccttatatggattaatatcatctgggtttaattaaatattgatatttttcttataatttgcactcgttaattctttttttctattgaacaaaattttaaattagagttattgaatacaataagatacatctagtttatagtaacatatgatctataaatattctcaaagaatatttattgttatttttaaggtaatacaacattataattaatatttttgaagaatattacttgctcttgaagagcatgagctatttttttaatactctagaagaatattatttgatctcgaagagcataaattataagtttcaatatttcagaagaatattgaaatatttttcatgaaaaacatgaattataatttttaatatttcaaataaagatattaattaattgccgtcgaagaaacaatagtaaaatataaagtattcttgaaaaagtacagctctaaaaatattaatatttgtttaaaaaatatactcatgaagaattaatatttttaaacaattatttattagtgctcgtgaagagcaccacattattaatattttacaaggaatattatagcttttgaagtagcacactattattgatagatattttaattagattttacttgcttccaaagagtataaatgaatgtgatctaacgtaaattatgtttttacttctaagagtaaattcttatacgatttattatttcaaatgataatatgttattgctccagaaaaacataacactatgattccaatatttcagaaaaatattaatattgctcttaaagaagcgataataaaataatacgtgctcttgaaagagcacatgttttgaaaaatatgttatgtgtaatttatgaatttgtgcttatccctaaaagataactacttatgttatgtggacattgatcattatatgattatataatgttcaatcatattcttcgaaattaaataattgaattatatattatattgaaccaaaagttcaatttgattttattatttggcatgaccggttggaccatcttggatcaataatgatgcgaaattaaaattttttaatgaaaattcaatgaagaataagaagcttattcaatcgaatgaattcctatatatcatttattaactttatcgacaattgattattaaacatcactagataaaatatggattgaattctttatatttctaaaaataaattaaggtgatatatggggccccatcacccaccacgttgaccatctaaatattatttgtatctaatagattcgatgcaaatactagatgattacatagtgttcgcaacctaaagtttgtgaaattattgctcaaattatgagtataattttcagattatataatcaagaccgtgtcttgttaatactagtgggtgtaaatctcaacattttaataagttttagttgagatattgataaatgatgcaacattattgtttgttaaatgtctccaattaatgtaattgataaagtactttctatttttatttaaggaattatattacgtatcatgtcaaaatcatagttctccctattataatcaacttatggtcagatcctaattttttcatctaattattttgatattgtcatatatgtaaaaattgaacaccataatgaactgagatgaaaaataaagagtgttgagaataagtgcgtagtttgaactattatctcatatggatgatattttgtaacactgagaaaaatgatggtcaaattaattggataattctctcagcattcagagggagaggttaaaaaattgaaaaataatgtataaatgcatcatcttctaaatcctcacataatatcattcgaaccagaagtttaaaagataatttatttagatgcatttactgatcaaagagataaacaatatctcacgcactagttttaaatgcttcaacacgaattgatgtcctatgagaacaatttgttagcattgtatttgatatatctatggcacgcctaaagcgtgatagtgttcgattctaatacaaaaaattttcaaattaaaagggagcaattaacaaagatggtctcattaaagaggcatatactcttaatgagtatttagacataacaaattgtaaaatcttagaagaggctcaggtacctgatatgttgaaacttgagatatctcaataagttatatcattgtgagaaaagaaatatatagaaccgagaaggaaaagaaaagttgtcaacaatgcttctacatatgatgtactgtatcatattatgaatagggaagaatcaaaataaatgcgtcgaaatatatcgatggaaataatgtttggctaaataaaagggatacaatcctaaatggaatttactagagaaatgtgaagtttttggacatgtagtccgaaaatctaaaggtatatacttatacgaaaaggaaatgaaaaaaatgaagtcgtaatgtataatgcacgactttcaacatagtgaatttcgcaaatattgtcgtggatgaaatcgcgagtctatatcatgttatcttgacgttatatgaaatttgaaatatgtgatagtcaactcatctgacataactattaatgttatcttttgtaagatttaatacgcctgaagtataactcaaatgatacataccctagaactatgttcttagatcattataatgattgaaacaatctggatgcatgtgacattatcgtcttagcgagtatttgttgaatgaatgctataaaaatgatgatgtccgaccatgtgttttcattaaaaaaacgaatattgaatttacaattatggttgatgatttaaatttaattggaactcctgaagagctcaacaaaactgcagattatttgaaaaatgaatttgaaatgaaggatttgggaaaaactgaattttgtctcagattgcaaattgaacatttcgcagatatattatttgttcaccaatctacatatgcagaaaagttttaaaatatttttatatggataatgcacattcattagtaacatctatggttgttcgatcatttgatatgaaaaaggatacatttcatccacctgaagataggaaaaaatttcttggtcctaaagtgccatattttagttcaattggagcattaacttatcttgcaaattgcactcgacccaacataacttttctgtaaatctccttgcaagatacaactctacaccaactcaaatatattggaatagtgttaagcatattttattctcaaaagtcaggatttgctttagtgagatatgcagatgcagattatctatcttacccacataaagttaaatcacaaataggttatgtgtttacacgtggaggaactgctatattatggagatctatgaagcaatccttgacaattacatcctcaaatcattttgaaattattgcaatccatgaagcaggccgagaatgtgtatgattgaaaaacatgacccattatatccaagcatcatgcgggttaacttcaataaagatagtccaacaattttgtatgaaaacaacgcaacttgtattgcacaacttaaataatgctatatcaaagttgacagggtgaagcatatttctccaaatttcttttatacagaagagtttcaaaagaatggcgacatcaatatctaacaaatttgctcaagtgataatgtggtcgatttattcacaaaaatattgataatatctacattcaagaaattggttcaaagaattggaatgcatcgactcaaagattttcagtgattttctttaggcggagtagatatattctttttccttagtctaggttttgtcccactgaaattttctaacaaggttttaatgaggcaacatcttttctatactccaaaatattgacaatcaactgtatcttttttcctttgtttgatttttttcccacaggatttttattaaacaaggtttttaacgagacaattattgtacaaataattaccaaagagggagtgttgtaaaataataagataattattgatgattatttagtgttatcatgatacatggataagttttatctagtttagaagattcattttattccaataataactcttattctgaatcctataaatgtagggcattggttcataataatacacaattgagttttgactctctatttcttttcttattttatctcttctctttagttttataacaatatatatattttaaaaagaaataggtttttttctcaaaataatgtgtccaaaaaatagatcccttttccttttccttttttttctaaatgtttgaaatattgttttctgcctcgtcaatttgaataatgcacaactaaaagactttcagataagaagggggggggggtcatagacggaccgcttaaatcccaaactcttcttaaataggttaggtcttttttacaaaacttttcaattttgcaattacgcaaaccagcaaaactcaaacaataaatcgaatgtgaaatctcttaaaatatgaattttaaaattggtacattttttttttaaatatcaccaaaggataaagctaaacacaattttttttttttttttttatctcatgtgaaacttaaactatgggcattaaactacaacaatctaaatcctaagctattattattcaaaatcaatttaaacaaacagttgtccttcaaataaaataaacaagtttttttttttctttcactcaaagactaaaattaggcacataattatttataacatgtccatgagcgttaaaatcactttaatttctaaactactatcattcaaaattgatttaaacacaaacatttaactttcaaaataggaagaaaaatgtttaaaatttttttttgtgctattgctcatgcactgttcactttttttttatgtctacagaaaagtaaaatcgggctttgataccaaactgtaacgccccatttttttatatataaaaattggagtgttacgaaaaactcaaatttcctctttaataaatgtggaatgacgcaaatcaaagaaattctttactttcaaccataaatataaatttaaatgcgagatttgagtttctaaaaatgtaaacacaatcaatggactaattaagtaaatgagtccttaaactaattaaattttgagacatgaaaagaaacaagctaaatatttaatatctttttccttttttcgattcacttagcagtccgcatcaccattccgctataactccaattgacccaaactaaccagtaaaaatttgtaagagtgagcattccaaaacacccagtaaaatacatgcagttttcatacacaattatataacaaataaaatctacatcttataccactctgctcttagatggagtatattggtgaccaagcggcacatccatcttaaatcctcttattatcccgtacgatttcatctctctttttatagaacccgaagtccactagcaatccatacatatttaatcaaatataaaagcataaaaaaacaaaagcacttacacaaaagtatcttacctcgctaaagaaaatgaaaatatgaatacacgtgcccaaaatcttctctactttagtgaataatggtcgcaaattggcttcttgtcttctaactcccaaaagtatcatctctctctctctctctctctctctctctcgcgcgtgtgtgtgtaaattttttggtgtagtgaaatatgagaccttgtatagtttttatagtaataaaaggtggttgagttattctagaaaatgtgtactacctattggagtttgaattgactaactattctaataaaataagatataatctaatgaaaaagcaattgtagttgtagtcactcacgtggggtaccaaccacctagctaattaacaaatcctgataaagacaacttctttaaactttaatatctttggcctaacttattcaaattaattttttctagagtcaaagacttctaattaattatgaccttcgaaatgagttcgatatcgatatactaaatcttgttccatcattatctaattattaattctaactaaaatagaaattgaaatcctattccattttagtccctaacttttaaaaatataacaaataaattctttttttttattctattattattataattatttttttcaggttgctacatcacaagtgagacaatactacacgtgatgatctaatataataagcggaacctacaaaatgtattcaacaacagtgggtattaaaaagtagtggatcgtacaaatgtcatcacattgcttaattcaataaacaatggatcctacaaaatatgctaataataagtgaatagtaagttgtgaatgttacgaaatatgtcaataaaaagtttatttgaccaacataagtaaaaagtttaagcagggccaaacctatcataaaagtaaaacttaccctatgagaagacatgatgagaggagacacttcttatgctatagtcatactttttgtcaccatatgcaatgatggatccagaaattcatcagagctagcacgaatcttctgaactagagaggatactcaacagtcgcttgagcgatcatcaagtgattgtccaatatatggggaaaaaaaaaatttgtcgtagccaacaaggtggccgccatggctagcccggtgctagcttcgtcattgaccatatgtcgagtataatatctatctagctcatagtcactttcaaactcgcaacccagggatttcatcttgaaagattaacattattgagatgaataactcaaataataataagctgattattatttttaaatgtattcgatttgagattttcccctcaatactcaatcatcttttttcttatttgcgaacatgatctaatctcaatatatatatatatatatatatatatatatatatatatatatatatatatatatatatatatatatatatatttttttttttttttatttatttattttttttttgacatagaatcaaacgtttttcagggaataataataataataataataataataataataataatagaatcaagctcttttaagttcatacctcctagtgaagctgttgtagataggggtgggcgtgggtcggttcggttctgttctctttagaaccgaaccgaaccaaacttttcgggtatctagtaaatggaaccgtcgggtccaaatataattatggaaccgttcgagttcggttccgttccgttcggttctgtactataattaaattttttaacatttataacaacgttatataaatacgactaatgatacattcaatgattttggaatgtcagagattagtaaactaccttgttcaaatgatcgctacgatcaaagcttcagtcgacgaaagtcacggcttcgatcggaggccagagtgtcggccgacgattgtataggttttggaatattaacgaggctgtgagagtcgagacaacgttatgcactttattgtaggtgtttagggttatttagtggatttgatcttgtttggctaagaaatgaaacaataaaatgggtaattgggtcaaaaattaaaaaattagaaatgaaacaaattattaggccaaaaatttggatttagaaatcattaatttgttaatttgtttaaaaaaattaaaattaaaataatttgatttactcaatataaaaaaaaaaattagaaagattcggttcttattcggttcttcggttcttggtctagaatcgagaaccgaaccatacctgtcggttctcaattcagatacccgttcgggtatttaatttgacaagaaccgtcgggttcgaattggttcgattcggttcgagttcggttcggtcggttcggttcgggagatttgcccagccctagttatagaacatcccaaatatgtacattggccgattttattatccattttcaaaactcttactctggctagctataataactatagttaaaaatttacattttcttctacaaacgatgcggaattttacgacggctacatggggcaaattttctgagatatacatgactcctcaagccacgcatcaaaggtaactgtactaaagactttttaatggtctatgctgcttaattttcactttgccatttctacttaaacattaaattttccagaaaaaaaaaactaattggtggtctgaattcattccatatcatattcattaattactttctatcaaaacattccacaaaagttatttttctagcatcaaaaacagcaaaataaaagagagaaatttttattttgagttctctgtttccttgaaatttgaaatacttctactataaggaggaatcgttgtatcttgggagacgcttgtcatgattccactagcatcgtcgtcgtacaaatccatcataatgaagtgttgaacacttgtctcaattttgcattcttcatttttgttcttcatgttctgcaacattattgacattccaagtaagcttactttgatttattgtttaatttagtttcaaatataattgggaaacacacacacaaaagaccccaacattgaatgtgcttaccagagaaactaaccatatattcctataaacaccataaaaatgtagcttattaatttccgtaagttggtttaaagttcaacactggaactcaacctaaagcaagttggaattattgtaccacgatcctctgtatcaactgccctataaccgtagtaaaccctacgtactacagtcctttttaatggtccttgaattagcttcatcatttttattactttcatgtgcttctaattaacatgccaactgattgcactaaagatccaactctctctctctctctctctctctctcgtgtatgtttgtgcagcgcattcgtttagacctcaaacttggctaaacgtaggttatcacttgcctcacagtgcccccttgagtgcctttaaaaggcgacatgaccatctccaagtaactctaatggatgcgaaatatgacattaaactactgcttttcatttttgttttgcagccatgaacgaggtcaaaccattagttcatccatgcatatacttaatttcattattaatctgtaaaaaaatttatagaacaaattccataaagttgcaattggaattataattcgattaaaattttgattgacaagggcactgggtcgcagagacaagcagcagaaagtaaagaaaagtgaatggaatattgaaaaatcaaagtatggactcatgcagaagaagagttatgaaggaacatttttgtagctcgaggaaatcttgaaaataccaggaaagttgaagccatagatgttgttgtcatcaaattatgacactctttcaattattattattaaatatttctaccaaagtaaattagtcgtacggtatcagcattgagaaaggaaaactttcttctcctttcggctacatgtttccaaaataatgagactgaaattcatgtacaatgttttctttatgtatttgtttaatgagtcatcatacgatattttctttcatctcacagtggagtaaaaataaaaatatagatcaatatataagagtttgaactaatcatctttatcaagttgacattttaaaatgaaatttcaaggtttaatatgatattagagtccattaaactctaacaaacttgcaaaaacatattaaaggataaattcatatgaaaatataaatcaacatataaaattttgaattaccacttttaataaaattaatctgttaatatgaaatttcaagtcttaatacttaccacagttaagtacagataattaatcaaagtgtcgttataagttctgttgaagggttagatttgttagtatggatatggacagacaatgacgagttttgacgagggtaataattatgagaatgaccatgaaaagcaaagaaagaagaatttttgcacgttgcatgatgacaaaaagtatgagaacatgtgagataatatcccttatcttattcttccctactaaattttagtgtttttaaagaatcttaaaaaaaactctttatttataaataatatcttatgcattacaaaaataattttttaattacaaaacgaaaactttatgcattctaataatactctttattttgaccttttattttgcttttctaaagaaatatttattgattttttctcgtattttaatttaacataacttttttatttgttaatgaccaatcaatttaaatatgatttgaatagtttaaagagttgagtattgaaatttgtgatttattaaatacaatattatataccaagaataaaagttagtttgtgtctaaatttagaaggcaaacctactctcaatttttaaaaagttaaaataaagagtatcttttactccctccgtcccaattataaaggcttgtttcgtttttcatacggattaagaaatcttctttaatgtcattaaaaaatgaattttagtcaaaatctttcttaatttacacccatttaatttttaatatacagtagtaaattattattggaattagtaaaaaatttgaatgatttaatttgaagaagaagaaataagagttattccttgttttcaaaaagtgcaaaatgtgcgtatttagatgatttcaagaatttggcacattaaatggggaaaattaaataatgatatattagtaaaggaacaaaacaaaatattctaaattagaaaacaagcctatatatttgaaaaaaatgaaaaaggaaactcaacatatatagagagtttcttgaaaatgctcttagtattaaaatgttctaggaatttgaactccctaaaaatcaattacaatagcattctacttggtgttttgctgcttggacagggtttatgaccaagctttggaaactctcgtatttttttttcttaatctgtccaataatcagatgacaattgtcatctggttccaaaccctagattttagccctgttagagtagaatagttcttctacttgagaaaagaatagaaaatacaccaatagtaaattgctgctcaactaattcttggacagaattgttaaaggttaatggctttcgaagaagtggtaggaaattagagatcccaaataataacataactctaagcttgaaagcttgacttatattactccacagttctaaggagaaaaataaaaggttaaaatcttatatagtgtgaagtcaatcttgttccggtcctctacacccaaagatgctataaagggttaagaaaacaagaaaggaaggaactgaaggaaaatttggcagcaccactcaataagaccttggtaggaaagattttcttacaccttggtataatcatattatagaaataatgaaggtaattgttgagaattagaaaccctaattctaccgccaaaagcaataatgagtttgtaaaaaaaaataaacacgaaagcacacaagatttatagaaatacgttatcttccatcactgcagtaaatcactatcatgaaaagaaatttgtaagagaaaatcactcaacctatcttctttaacctctctattatgatggtaatttaaaacactaatgacgactctctatttataagataaatgaggacaaaatcaaaattacacgtgcaaaatgccataattgtcctttatgaaatttatttgaaagcataatgcatgcactctaaaaacgtatgaatggtaaaatcccctctccactggtgaagaaaaatttcattttactcaaatgagaccttattttggaaagcacagtggagaatgtattagcaaaaactatacagtcctatttgctattttgcttcaaatcctcttggtttctctcaacttttggattcaaataaattaatgccaccatctaattacatagaatctagaccatttaatttacaataagtgcttaaaagaactagaatatacaaccaaaaataacaaaagtgaaagaaaatgcaaaaatgtataaatattctaaatgacgcaccaaaactagacaaagatacaaacagctagacaaccttttaattattaaaggctcaaggttgaagaaaaaacgtctgttttgtcccactatatgctagaaaaacatagattaaaacacataagacatatttactcaaacagaaaaagatatcttacatttctcgaaccataaaacgtcgaaaactaaaagcaggaaacaagcatacaaatttcataattagattcttttggaatgctactgctaatataatttgcctatttattgatttctagcattcgtgaaaatatatcctcaatcattgctggaaacaataaaaatctctagtaaagctctttattcacacacacacgatgaaacatggacacgtaaacgcataacatatacaagatttttctaccggaagagagtgaccaggcaagagatattgaaggaatgaaagaggaccaatttttggtagaattttctacttgtacattctctgtgtacttaaaatcaatggcaaaactgtgtttcacatctcagtgtcaaaaaaaactattaaccatgatgtacaccaaccataacattgtagttaaggtgtgagttaaggagaatatatcttccaaaggatattatgtcattattgtataatgtagctaatgatgacaatattaaaaaaatctccattttcatccattgttttctgggcatgctgttgattaatgattattctagtttccattttctttttgagtcatatatttagggatactagtacttatgaagttcataattatgattataattttaaccatgctcatttgttcagtatcaaagattatataagttctacaaatattatgattatatttccttaccttgcatcactgtatctttgaacttgcttcatatatttactcatccattatgtaaaactagagggaaattttcctgaatcttgttgacctaatcaagagaaagatgttaatcaagaatgaatagaaggccagaatgaagaaaagaggaacaacgagaatttctactgataatttgcaactgtttgactttatatgttcatttcagacatgatgcaacaatctttaagtaggtatgcataaggtattgttttgaaaatgtttatgttttatgtttttaatctaattctcttcctttttctttttttaagttctagatatcctatataaacccatcattttggtactgctaccacttcccaattaaacttcattattgaaacaaatagaaaaatagagaaaaacttttagcttcgttttgatcctttcctctccttcacaatatgaaattcagttttaattactgatcatttatttttacatacctcctctaaaatttcaccaggtaataaaacctagcaggaagattttcattttacagacttattaaaagggaagagataatatccaaattaagttactattattttttattgtgaggatatgacttttgaattctcgtgcatgtctgggtagccatgtaaataatatttcagaggcaattgctgctcaaacagagataaaatcttggcccccaatgtgaatcgcgctgctcctcatgatgcacctcggcctggattgaaacccgggatttaatccagggttctgaagcactcctctatctcagattgtccaaaaaagaagcaacctctttgagtcaccaattcaaacaggcaattatagagcagctcgaatttcaacacaagctagaaaagcaaatagtgaaattcaacaaacaattttaaaatttgccataaaaacagcacgcgcattttttatggtggaatcaaactttatgcatttcaaagggaagaagaatagttcaacgttgcgcatcgaaatttgaagtacaaatcaagcataatgagatgttaatttccacctctctttctcctatatttaagcactatttttcttaatatctacctcatcggtgtcaaatattgcttctcgaacagaaagtaattaaggttgttgttcaggatcttggaggtgggaagaattgcgtaccagctatgaaagtgttgagcggagctgggtataaagaaggatcaagaaaaggcgaagaaccaccgccaccgccaccagcggcggaggttgtggcggcagaattggccgttccagttattaaattaagttgttgaactcctgcactgacacttccaccaccagatgagttgtctccggcgatatactggctttcaaggccttgatcgtatagaattcccttaaatacatgtccactaatgttcactgccgtctgatatgcatactgatcctcagcatcgtcaatggcgcttactctaacgcagcgaaaaaccgcctctgaattcacttccgtagggaaattcccaagttgtaaccctacaaacatcagacacaagtaaggtcatatgatctaaaattatttaaaaaacattgttaatataaaaaatacaaatacaaaaagaaaaaagaaaaaaaaaaaagttgacaaaatatcattgaggtagcgtagggttggggggaatagggtcttccttgtcaggaatacctaaaaatagtgtttcaaaagaaaagggaaatggaaaaggaaaaaggaaagcctgataatgggttttggtttttactatggaggtcgatttcaactttaaacgatgtctaatttagttgagtttacctgattcattagtgtttattctagtgcaaacaagagaggaagaagcatttggattgtctctttgtctttttgcagtgtctctttgttcttgcaaagcagaaagctgttgttgtctctctcttctttttgcagcaggaacccaagtgctcttaacatgagtttggcactgaaaccctcggctcttacagcaagttctacatctcatataagaacaatctttcttagcttgattcccacaatcctggcagctaattccaccaacaccacctccgccgccgctcctcatcataggaaatcccgacctcggagaatcgttcgagatttcgaagccggtgcgactcggcccaactccaacggctaatcctccggccgatgcatagagatcttgaagcgagttctcgttgggatggcgttggaggaaatgttgattttcttgctgatttggatggttctgccaaagttggaaacttttatacggtatgtcttcatttctgaacaaaaaccagctttctgggttgatttctgggggtgggttgttgtggttgctactgctttctcgttcttgattgcttctattggatccgcccccgccaccaccaccacctccgcctagtgagaaaaagccagccatgttgacgccaactctaatccttttctagacttcaatttgagactgacaatccataacataaccgccaaacagagatgaaaatgaccccaagaataataaggcacgccttaatttacccgggtactgttttgatttcttgaattgtgggcataggaggtatataaatataaatcaattctgtggcagtgtcgacgcagaattacagttctgccacgccgccattaccgtggcttctaaaagcattctgctttctctttgtaaccaccaatttaagtctgtcttaccctcagaacagaaagaacctttcgatcatcgcttctattccatttattattacacacacttacacacagactcgctcactctttctctctctacatcatatcaacttgaagagatgaaatccaaaggtgtttggacatctgcatgcagattaacggctatgactactgccacgtagctttttctcctttgctactttatgtcgctgcccatataattaactaattaatcttgatcccgagctcaattttggaataattgcattatacatccccaagttaatttccaaccgtgttttaaaaagagtaaagtggatcctatcatgaaagtcaaatttcaagctagacaggctaagactcaaaattaataaatatatatatatatatatattgcttaatttatattaagtaccgataatatgatacatcatttaattagtgaatcattaaatatatgaaatatatcattagcttattaatcaattaaatgacatgccatgtcaccggagcttaatattagctaaacaccaatatttagaaaatcattttcgtatgtatgtgtgtgtgtatatatatattcttatttttaatgttataatcattctaaatttatttaataattaaaaataatacatatcaaacatctaaattgataaaatactatagttacttaatagtttcgataattagtcaattatgcaatttttaagctttcaaaatgcaaaaatcaaactattttttcaataatttcaactttcaactaaacaaatcctacttagcctctgtttgtctaagagtatctccaaccacaacaccattgcaccattttttggtgcaaaattgctccaacccaacaccaaactttgcaccaaaatggtgcaaagtgtaaaatatccattttgcccttatttaatattttccaaataaatttgttgagggtatttatgtaatttgtgtatatattttttaatacaataaattattattattttcattaatattaatattatttgtgtttaaaataaattttaaatgtaagacataataatcaattaattaattaaaagacgaaaacaatttaaaatacatcaaaaacgattatttattagagttaacatgaaatatattaaatagcaatttatgttctatgtttattaattgtatttttattaattgttctatgttttgtatatttattaatgaatttaatctttttcgtaatttaacgtaattatttatttagtaatttatgtatttatgaaataattaaataaataatatttcaaataagtagattataaagaataaaaaagggaagaaaatggttaaatattattcatttaatgtaatttttggtgtaatcgttggagatgaattttaatttggtacaaaatttggtgtaaaatggtgcaaaatttggtgcagggttaaagatggcctaatattctctgaaaactctctttcttttcctaaaattattttcaaccaaatattctcacaataaaaatatttttcatataatttcaaaaattttctttacttttaactacattttctccaaaaaaaaaaaaatcattattccaaaattaattttccaaaaatagaaactcctttctcattaacttatttaacttttatgaagtaagctgtgtgaaagttaatcaacaactaaacaatgttttggatgatgagttttgattatgcaattacaatgaaaagacgaagatcagtttgtaaaacttgtaaaagatgattatggtataatagaataaggatcaataaagaattttcatcagtcgtattttgcataaataattttagattaactacaagtttgaattataatgtagaaataaatctagggtcacaattattttcaaatgctatcatgctttgacaattaagagcatctccaaaatactctttgaatataatatacttttaatttaaaagatttaacccttaaaatcatgtttcaataaactctttaaattaacattttaatttagagagtctgtttagttttctaaatttggagagtcaaattcactctctataattatatacatccaaaatatttcaatttttgatgtataaaaataatctagatagaagcaaattaaaataaaagatagggaaaaataataaatatttttttagagtaataaaattaagtgttaaataaaaaatagggatttctttgaagatgctctaaattctaaataatttcaccacccgactcatgttagaaatggatccttagatttgagactttttttcaatatttggtttcttcgagggtgactagacgagatttaagtttaaaacaagcatctccttttatttaatactctattcatctcatttatataggttgattttgttttcatacggattaaggaatcttatctactattatcgaaaaattaatttttatcaataactttactagtctacccttatttatatttgtacaattttaaaattaagtgaaaaaattggttatagctaggaaaattaaataaggatatattagtaaatgaaaaaataaaacatcctcaataaagaagttagactatataactgggacgaaaaaaaaaataagagaagatagtgtatataaatgggatggagggaaaaagttttaatcatttgaaattttatttaataattaaaataatatatatcaaacatctaaaattataagatactacatttacttaataattcaattatacaacttttaagtttttgatatgcaaagattagacttttttatagttttaactttcagctaaacaatcctacttgaaattttctaaagtgtttttatttttgacttttatacacataaagtcaattaaaattttgaaattaaggttaaataagagggcttttaaaaaattaagaaaatttaataaaacaccactagatactcattgctaagcccgaacctcgcgcctagatgaattatatagaacactatcatcactacaataatcaatgttgagctcgtaggtgcaaacatgtgccactgttagtgagcatttataagttaattaaaattctgatcattagcaaacctatatcatcgtcatcgagcaattctaatatgaaaaacacaaatttaatcttagtcatgaatgacaagctcacaaaaacatgagagccaaattgttgaacaagcataaatacttttatctattttaacatgctattccacaccatcaaaaccactattgaaacacacgaaaatgagaatgctaaatcttgtgaaattaacatcacaatcgacgaataacgacacatggcacgacgaataaaaggtgaaaatgtaacaaattcagttagaaaatcactaatcaatgatcgccatgcatcgctaaaaaaggattggattaccctcttgattttatctgatatttataaatagtcaaaaattcaagcaaatttggaaatagaaaaaaattgaatatacgctattttcaaatagtcaattctctctcaaactcttattttcaacaaatttcatttgagtttagggagaaaaaaaccttgactagattaaaaaaaaaaaaaaattgttagcctcgattttgaggtcaacaatatacgttttattaagtttttccttacttgaatcattccctattaaattctattactttgaatatagaatacctcgatcagattcctactagccaaaactcaacgatagtgatcatttacaccttctcctagaaatggaatgagtgaggtgaaaatgtacgttgtgccaccataaaatgaggtcgaagaaaatataaggtgccattatcaataaataacatttgacattagtcgaatgtcattttgataaacaaacctaatacacaattcaataggagtgaagttaggagggacaaaaaaatttctactggactgatacgtaggaaaaaattttaccattaaaaaaaaaacaaaaacaaaaaaaaaaattgcttgagggcaagccccacaatcctactaaaatcttaaacttttcatatgtttaaccatgtttaatttgtagggcgatcgaatcaaattatacaatatatattgtacaaattaattagggctcgtatgaaactaaaccaatttataataattgaataatttattgcattattaacaattggtaagtgatatgacaatcccaattagagtgatttttaggggaccattttggttagcaggttaggagggcatcttcttacgaataatttaaactttattaattgaggggttgactataatattaaagggcatataggccatttaatacagtgattagtagttaactcgtatacggaccccgccggcctcaaactccgccgtatatgacctactataggcatacctatttgttaaatttgcaatttggtccctcatcttttgaataaattacagtcactgaagatatcattattttatgcccacttgcagtatctttgaatactcttggatcacacggaattttataggcatgttggaatagatgccttgatgcatgagagcacgggaatttagaccatgtctgagcctcatttgggattaaaaaaaaaaaaaaaaatatttagaatagtttttttttttttttggggaatatgttgttaaaaaataatgatgatttttacgtttatatataatattattttgttggaaaatttatagttgaaaataagaaagagaaaaaaatgtattttaggattaatggagtccaaacatggactttctttcaaaactttctttttctcatattcattttcaatcacgtattttccataaaatattcttcacataaatcaaaaaaaattccatattttttatcgactcattattaaaaaaattactttttaaaaattgattctttaaccaaaaatggctgtcaaacaggggcttagcgtttaccaataagaagtttaatcatactcccaaggttttgtttaccaatactcataggtaatttatattctatccgcctataaaaatagacttattttcctttttgtcttttctaaattattagttattttccttgttgctggtgtccttaattttctaatataccactatttaacatgtttttttttacttttatttaaatcgttatttaatgtaaaaatatattagaaaaaatcaagaaaaattgatgttttcaactatattaattacatatttttattctaaacctatctttgtaggatgaagggagtacctaattatgcttctaaatattttatgactttttgtcccttaatatgttctttttaaacaaatttcatatgtaattttatcacagtataaataaaatagatgcatatcagttatcattgccgactaattattttcggtaaagtaactaaatttgttactgcacataagtaaatgccatcatttttgtgacaatgaactaacgacgtttggaagcattaccgatggtgaaaatatttattttcagaaaaatttaccagtgcggcattaaaatcttatattacctcaattattttattttaataaatatgtaatttttaatttaatatattttgttacaaattctattaaattgtgagaaaacaaaattattaattaggattgatgtgtttaaagcaaaatataaattgctttggaataaaagaaaagttgaaaactaagggcatgtttgataggctacattttccatgaaaattttccacccaaatggtatgtttgattgccaaaattttccatggaaatggtttttcaccaacccccatgtgacccctttttccaagttttggtggaatcggttttctttaattttggtggaaattggttttctaggtgcatttttttttttttttttttggcaattgaaataaattctatcctcaattgtaacaagttctatccttttaattaacaattttcgtgaagaacaaaaccaaacgaatattaaaagatagaaaatttcaacatttttcagatgaaaaattatataaatcaaacatatttaattgacaattcacaggaaaacaagttctaggtaatttaatttcctagaattcgttttctttccatccaaattatattcttacaatcaaacagaccctaaaagttgctggaatggatcccaggtctaaagataatagccatttaggtacaagtatatttaacaattgaatgattataagctacttaaaccacaaaaataaggagagatttggtccttaggaggcaaagttggaaaacctaaagatagagtaaaaatctagtcgtgaataataaattataaagttgaaaatgttgttgatttttgttcaaacttaattacacttcttaatctctagcaataatttcacttaactaactgctagacccctcctacatcacctacactacttcccacatctacttgtagatcttaacgtgttaatagatctaatcatatatgttagaaaccttttaaacaagaaatgttgcgatgttatgatacgaaacgcatatttgaattttatcaagttattgtaattttaatacatttataatttgttagataatgtagattatacaaaaacaaacagtgttaatgaaaattaaatttaaattttgtctatcatattattcatcatacacaaaatatattattagagacgtgattagagaacaagtccgttcatagatgcttatgtttatcctacttgttgattaattctatgtttaaatttaatttgttaaaaattaattcgtagcaaaggaaggatttcatattttaattctcaagacttctcataagccttaatttcttgtaattactaaatgttactctcaaaattcaaaataaaactaattcattttatctcgagcattcgtctttataatcttaataggttaatttataaggagacacatttctcgttgtagcttgtttgttacaaagatagtacctaccctagtctttccctcacttactcaagttgttttcctagatgattgctcgtattcctcaatttttatactttttatgcttgtatacttgtaggggtccatgattgaccccctcctttgcatccatatctactaaaaaattaaactttaaatacatttttgatatacggtatcacaattatattggatagccggatgaacataattttatttttatttttcattctaaatattgtttatgcattagatccactttaataacatatttcataatgatttatttggtgaactggctatggagtaatgtacaatatttcattgagaattatcaaaaactattttaaaacagtataatttgaaatcattatataagtaaattctcattgcaagcaactgcaagccatttagagattttctaaatacaaaatactccttattttagagaatcttataaagtcaatacttaaaccaagtttaaaaaaactctctattttaaatttttagaatagacagtgaggactaaatcttcattctttattcttacgttttaatggttgcactcattaaattacatttttcaatactcttgttcttaaattatttaaattatatttcaattaattggttattgatatacaaaaaattaagttaaataaaagatgagaatcaatcaattaaattttttgaaaatattctcttacaatttaacaagaaacagaactcataaacctctaaaatattaaaataaagtaattataatatttgtacactaataaacttactaaaaatactcctgtataaaataaatcattgaaaaacaaaataagaaaattacttattatatgttcaccaaattaatgcttgtgattattctacctatacttttgactatcctgttcatttacaaaattaattgccacagtaaaaagtcagatgtctataatttaaggaaagattgtacttatgcccctaaacctttcaattaattatcctttatttttacaactatagttctaaatatttcatttcgattgcacttgaaggacaacaactctaaatatttcattttgattgcaattgaagaacaaaaggaccattggctgatagtcaatcccaaaaaatcaatttatttacattttgactaagtctacaagaacaaaattataatttcatatttcttcaataaaataataaagatttaaattaaaaaactaaaaataaaaaggagttgtaaacggttcatcttccaacccatcccacacccaccaaccatcctacgtaacgaccactgtcggcaacactctcattcactaaatggactgctctatctcctcctcaatcccaagatccactgcccttaacttttgacattattgtgctggaagcatccgccactttatgataaaatggtgccgatttctttgtttcagttgttccaacattttgcgcattttcttacgttgtttttgatataggtttcatgggtttcgatgctggcttttgggaattatgacattggtcatgctacatctacaatcctagttgacaatcacatatctgaaagggggctcacgatgaataaaaaatcttggacctcctcctatgaggaggttgttaatcggggttgacaaccccaattgtacaagtagcaaaaaattttggacattccttatgatcactgtatccaagctttgaagttaccatattcctggtagagatgaccttttgtaggggttgcatatgataatttaccaatcaacgtgacgtgtcgtctattttcttaggatttaacttttcagagctgattcaagattttttggacttgatactattctaattgtattcaattccaaagtaaactggttcctagctatattggatgagaagcaaaccgatgttgttggcgatggagatggcagagagattttaggttgatttggtgttgcgcgtttgttgggatagggttgggaacgaagatgaaaagttcacaatttttgttttttttattaatttaattttttattggacaaatatcaaattataatttttcagttttaatttgttcaaaatgtgacaaaattgattttttgggtagattaagatcaaatgcatgggatacatcctcaccctgtaattgaaatgaaaggtttgagtaggggtgtcaaatgagtcgagtggcttgtcggctcgactgcttggctcgtgggcggctcgatctcgtaattggacgagcttgagcatgaacctaatgggtcagctcgtcaggcaagttggacccgctcgactagccacgggctagcctacagacgagtggctagtcggtgagcccacgagcaatggccaaaaacgatcactttaatattttgtatagtacagattatcaaatactgaacaagccctcaaacaaatgactgtggatccgtttgtgaactgtaatgaaatgtgtagaatatatattgtaatttgtataatatagactgtatagtataagtaactaagtaaataaatagtatgaaacgaaatcaagagttcaaataaagtctatgtataagattgtaattgtaaatttcaagtgtggtaaattggtaattgatattgaataattgaaattgaagatagaaatgaacgtagtagattgtagaatgtggaagagaatgagaattattgttggaatgttgtgtgaacaaatttggaaatgcgttggaacatttatagagtaaaaaaagagagagaaggaaatgaattaaagtgattgttttggctatttaagtagacgaaattaaaaattgtatatgaacaacttgaaacatgtacaaagtttttaaaaatttaataatagtattataaaataacagattttgattaatatggttaaattaaatgtcacatatccgacgacatacaattttggcatatttatcttgtaattgaaaatgagtgtcttactaatctatcacgtatattaatgctttcaaaatatcttcttttagtcggctcttgaccttgaacagtaccttcttacctacactaagagagactccaaagctacagttctaatgggaggcgttagtaggtctttcacaatcgcagaaaccactggccatcgtcgttcatactttcgtcaaaattcaattacttcttctaaattttttaattattttgttattaagcatattatgattaaagtaattaattaactctgcagacaatgcatttggacttgcatccgatatctgattacctgcggtaaacataatactaatagaggaacctattgcattttcagtatatatagacgtattaatgccttaaataaatttaatatcttagcatcgtcttcttcaatatcagcgggagaagtgggtgcagagagcactcgactaatatttgcacatagtcattctacatatattcatatactacataaagttttgttctaaaattcttatgagtgatatgagtgttaaaattaaagcttttaaaatctgatcaattacatatttagtacctgataaattatatcggggtccatgatgtatgctaaaggaaataatatagacaaatctttttaatattttctaaactttaattccataggatatataattgtaccaaaatcgaggtcattttggtatttataaaatgcccttacaattatataaagatgtccaagcaccatcaactaatgtgattgtaaacttcaaataaaatatttgtaatcataaaaacttgtcaaaattttttaaatttcataagttaaaagtcaatcggattcattcaaaacagtattatcatcgcttctaatatgcatattgttgtaaaatttagttattaaatgttcaaatccttcgtatgattttaataataaataagtggagttccatctatatcctacgtcactaacaaatgctttcatatcatcaccccaaattcggcttaaaattcttcaaatgcttgttttctgctagatgaaatcatgatatatttctgaatccttaattctttgaatttcattcttaatatgtttcaaacaattatgcacaattaaattaaaaatatgacacacacaatgaatatgatataactaatcaatgaaatcaggttgtaatatcctacacaatttatcgaaattggcatattagaactcaataatttcaaaagcaataattttttaagcatacaccaaaatggatatatgtagtatacagttgcaactatataacttcctttattaatcccttcttatatatctaagcgaaagatgtgacactcccatatttttgcaaatcgttaatcaattatttctttgtattaaagaaatattttattgtatcagaacgaagagtgtttctacttaccacaacatatattgattgaagatattctttcatatagaagacgaaatgttagttgtccgctattgctagaaacaactctgcattagcaacgaacttcaccattcccatttgagctttctcctccaaatacatccacgtgcaaagtatcatacaattaaaaccaacgattggattaccaaatttcaattacatttgatcggcagcaagagacccatgtttggccacacatacattgcagtgatggttcatatgtgcccttttaccatgtcaatcgttattgatagtatttacatactactttagaccatcaaccacacaatacatttgaatcaatttatagtgatctcagcatttagcttgttttaacccatttcgcttccttcttgcatcgaaaatatctaatttttgttctttgaacatcaacttcatcaaaatcaattagatttctatttccatgaacatccaaatctggaatatttttgggaatgggtacttcgttgagatcgacaaattcattctgagattgactttgcagcgttataggtgattcacctccaatgtcgaacaagacaaattagtgtgaatccatttatgaattgtgatgaaatttgtagattatattttgtaatttatatagtatagactgtatagtgtatagtaagtaactaagtaaataaataaagagtaagaaaagaaatcaagaattcaaatgaagtttatgtataagattgtaattgtaaatttgtagtgtgaaaattggtaattgatattgaaggtagaagcaaacttagtagattgtagaatgtggaagagaatgagaattgttgttggaatgttttgtgaacaaatttggaaatgggttgagatatttatagagtaaaaataaaagaaggaaaaaatttaagttgtaggtcccaaattcggataaaggaaaatggttttatctgttataaaaaaaaatttgacaagctcgcgagccaaagctctgctcgacccacgagccaccagctcgaggaaggagtactgactgggctcgtgggcaatagggctgagccgagccaccattttgtttgagtctatggctataaaaatggaaggtttgggtatcaattacaactaattgaaaagtttgggaccctaactacaatttttccataatttaatgcaaaattagtactacatctttttttttttttttaaattcaaaaaaggtaatgatatttatcattaggatatgccattatcagtttacggggtattaaacctcgaattcattatttaatggagttgtgtacatttcattgcaatagaaatgacttaaagagtacactactacataaacatatctttgtttataatgaataacagacacatcttcacataaattatatattagcaatttgacatgcccccggggcataatcaaatggtgtaaaggacaggagtgaggttatctcacgccttgctggcaatcgtagtgtgggggttcgattcttgagacatggaattggattccttgtaagcgcagtgtacatgcagctcttgttccctgacctgctaaggcacatcccgcgatttatctccctcacaaagttctaaaagcgggacgatgggggccctcaaggttggggttcaaccttttttttttttttaatattagcaatttgacatgacttatcttgaatcactgtattaggcttgaaacgagacgtgtgctatgatagaagtcaactaggtgttagatccaccctcaaggctaatctgttactaattatggacaaacagtcattatatgtcaagctgaaaaaatgaatatggggattcgtgaagcattgttttttgcttattcaaatttggagatgatataaaattaatttatttttcatattatatatagttagtgcatttatcttagttagcaattcaagctacatatcaaggtcaatggaccataataatgtatatacacacccaatttaaatgagacaaacaaattatgcccatgtttgagccacattctaaaaaaaaatgtattattcatgtcaaattaatggaaaatgtgtggttaaaaaataagaaaaaagttttagatttgcttgtaatattatttcattgaaaaatgtgtggttgaaatgatgtcaaatattgttgaaaaatgtatttttttgaaaataatatggctcaaaatcaagaggttcttgaaagctgtaaaattcaaatgttatgatgagaaagacgcttgaaagtatatgagatgattacttggtgctaatttaacaaataacttggttaatataattacttttttttttccaagaaagattgtgctttcaatttatggaaaaattcgtatttgcatcattacgaaaaagatttcatattatactacgttatggtaatataactaaaaatactggataatatgtgaattgtaattataaatactaatttctaaaaatagatcccaagtaagttgctagaactgaaattttttgaatttaccaaaacgttatgcttctcatttaatatccattcaaaaatcaaagaagaaattcaaaactaaagatgggcaaagacacggagttttatttgaggcataattatactgtgcatcctcattactgcagttatcaagaactcgtcggtgctgtaacaaatctttccagttttgacaccaaaatttcaaggcaatgttaggttttgaacacgttcttcaattagatgtaacccaagcagattgtttcaattttcccattttagtatgtatatgacggatcattgattctaaaaacacaatctttaatccaaattgtatcttttgactatttgcaaatctggtgacgatttaagaaattgaggataagaaaataattctgtaatgtgtctattttaggcattgtgaaattacataaaaataaagacggattatatccttttggaattctgtattttagctcacataatatggtgttatatatctcagttgttgcttatttgatgatttgattatatctgtaacattatagatgcatgtttcaataagaaaatatatacatcagtttatttccatctatatacaaatgatattcacccctaattttggaatacagaaatggatcatgtcagtatctttgtaataaatgagataaataccttttgccttcttgttcttttgattgcaagttcgttgagctggttgaaatgattacaaatgaattgaaggttaacaagagagtttccattctgaagatttagtacattgccggtgtagaaatgtctttgatacgaataatatatgacagccctctacatttctacatggagcttaagcatagggatgcacatatgacctcctatgcattgtgtgttggagtggttgaaatgttgcattctacactagcagaatacgatctaactacaacaaaaggatgtattgtgcatcaaatcaatatcaatatacatatatttcctcacgaagatgtcaaaggaaatacgaaaaatgaaagattttattcaagtattgatatatcaccaattgatacatgtgacaatgacattgatgaaatggacagtgtaatcatgtagcctaatctggaatgtattcgcgagaaataatatttcatgacagtttatttgttgaagacaactgttgccttgtacactaaccaaaaataagctaatctaaggtcacaagttggacactatgaagtaagtgttgaaatgtgaagtgttaagctacaaatgaaaatttagagccttaaaaataggtgagatggacatgtgaaggatacgatatatccataatgtttgtagatattctttggataccataacatgtgatcacaaccaagaaaatagtgctttaataggtgaccatgtaaagcaaaagtacacatttacacaaactaaatgtacgatttgttgttgaagtatggaaaagcttggagggtacaagaacatgtacttgaggttataatggaagatcttgatcatgcatatgcagaccttccgttgttcatgaacgagcttcaagaaaagaactttgggactgtaattggcatttaagtcaacgcaaacaaaagctttagatatgcttttatgactttaggagcatgcatacgaagaatggtagaactacaagcttgttgtagttgttgacgcaactgtagtgcccaacccaaatggatcgagatgtcactaaataattgtaccttagttgtagacttaataattaactatacttttaacaataggcatatatatttaatttaagaatttatttaaaaaaaaatatatttcatgcatgttatctattttattacatggaccgtatgtatgtatttaccaaataaataaaaagtttaaaataaattttaaataaaaagtttaaaatagatttttcatgtatgcatatctttaaacagtaaataaaactaagttttttattttttttccgcaggtgtcaaaagaaatttgtctatatagttatcaatctcaaaatttcaggaaattttaagggaatgtaagaatcttataatatgacatctaaatattggcttctttcgacaacatataaggcactaaaatatttctcaaaatcccgtagtgactcggtttggaagataaattagcgcagtttacttaaaataacatacaaaattctacagacatcatagtaacaagatttcaaatttattcagtagctaacccatgaaattatcaaacccaactgttttttttttcttcccaaaaataccaagtaatgattgagttacaaaatttttaagtcaatagtagaagatgagattttaaaaacaataacactaaatcttattgcttacatttataacatgaacggtaacttgtacattaatttctataaaacgtaactacttttaaatataaataattcataaaaatcttcttagaatagtgtcataaattatgttcacaaaaatctatttatttaaagaaaaatacgtaaatgtttcataattgaataaaaacattaagtcactggtttctccatagtgcgttgcatcttcatctactaccatccacgcctaaacaaatcaaatcaagctgtagaaagggaattaacccatgagtttgaaactcaatagatatcatcagtgcatttcgtcattaaattagaaaattcgaactatagattcatatcgtcgcatgtagatgaattttcaacaaaatctaatttctatacaattatcataacatatagagccggataatgatcattcaaactgtagtggtgtcatagcactgtaccgaaggtaccaattcattcatacttttaacgaaaaatcataacttgaaaatgaaataaccacttacacctctatctaccttgattttcttgaatataaaaggagcaaaatctgtaagaagcctttctccttcacacctttgctatttactttaacttagctcgacgtaaaagatatttttgagagaaaataaaagtaaattagaatttgagcagaggtgtagtgaaaaagtgactttcttcttcttgaaatctccatttttagtgaaaaactaaatgagagagttatattatcattagccttgttaaattgagtctttagctaagaatttaaagagttttaaatccataaaaaataattcatataaaaagttctacaaaccatttatataatgaaaaataaaggaaaatgaactattcatataatttgtaacctatatttataaatatccactaataaaacatttatttcatccaattaacttgatataattgtgcttaatgtgcaaaatgaggaattttttttactcaaaaataattttataaaaccatttacatggtgatctgaacccgggttatctatgtgaaataccatgtagataagcattgtgacaactcaattattcattaaatctttgtaatcaaatttatttaaacttaatctcttaaattgttgtgcttttaattaacttatggtttgggctttcataaccttaaatgggccgagcttccataacttattcttaaatgggctacttcaaaccaatttaagaatataaaattcgagacttcacattcctcacatctaaaataaattttgtcctcgaaattaccttaaattaaataaaaaatgttggagatttgactttaatttctactttttgttttccaagtgtcttcctctatcctttgatgtcaccactttcaagaagacctttttaccaacttcaaaatttaggtctgttcatcgaatgtctgcataactcttttgtcacccttgagctacttttatgcgatttctaatcttatcgattaccagaactatttactcgatgatcgcaacctaaaattctcttttcctcgacttcatcccattttctaacatagagagcctcgtatggtgctataccaatggtggacagaaaactgttgtcataggcaaattcaaccaaaggcaagtatgactcccaactacctccgaggtctaatatataagtactcaacataccttctaatagttgaatagttcttttggattgaccatctgattgaaggtggtaagttgtgctgaaattcaatttctttctatagccattataagctcttccaaaacttagacgtaaatcttagatatctatcagacacaatggagatgggaataccatgtaatcttacaactctctaatgtacaactgtgacaattgatctaagctgaaatttatttttacatgaagaaaatgagctgactttgttagatgatccactattacccatatagcattatatcctcttgctgacttcgaaaatcttactataaagtctatcgtaatatttttccatttctatttaggtatgtccaatggatttaacaaccctattggtctttaatgttctgctttaacttgttgacacactatttattttgccacaaataggcctatatttcttttcatatttctccatcaaaatatattacgaaggtgtcgatatttttttgtaccaccaggatgtgcggtctacgggggtgaaatgagcctcttccaatatctcattcctcaaaacttcatccttaggcacacaaattcttcctttacccatcaatgcaaaatccgaagatattccaaaatcttttctcttaccagtactagtttcattcttgatcttttctacaataatgagtctttaccctgtgcttttatgattcgatctctaaaagtaggttgaaccactaaagttgctaaatgggcaatgacttactctggtgtggcaaccatttcgatttacaaattcttcaagtctttgatcaattccatctgagcaatagataatgatgtcaactatcctattgactttctattaagcactggcaacaacattagccttactaggatggtaatgaataacgtgaccgtaatcatttactagctctaaccatcgtctctatctcatattcaattcctttcgtgcgaagaaatatttgagactcttatatgattcgtgtaaatgtcgcactttcctccatataattaatggctctatatcattaatgtatgaactaccacgaaagttctagatgatgcgtaacgtagttctactcatgttgctttaactgtcttatgcataggcatcacctttccatttttcatcagtaaacatcccaaaccttgtttggatgcatcagtatatacaacaaaccttttcgaaccttcgggtgtggataacacgagtgctgtaatcaatctttattttagctcctaaacactttgctcacatttatttgcccattgaaactttactcatttccttatcaattgtgtcattggtccaactattttggaaaaaatccttcgataattctaaaaaaattttccctttttctacaacaaatggttgcataacagtccaaccaatccatgcctaaaatcacatcaaagtctttcatctctatccgatacaaatcagtttctaatgtttttccctcaatttcgagattcaccaacctaactaactaacatgtatttaatgtttcaccggaggaatgctaacttttagtgtactctctgacttatcaaaagtaatactaaatttagtaatggaagatgttgatacaaaagaacgagtagctctcgaatcaaacagttcataagcaggtgtattagatactagtaaaatacctactattacgtttgagttttgcgcttgcaccattttgcacgctattatccccgacagctttcgatagtttgttcataactttctctctcagtatccaattgatgtgatttaaatgagttgaaaagctaactcaaagagttacaattttttagaagtacaattttttcaatttgaacgtttgttatttgaaaaatgggtttcaatttgagactaaaaatttggagcataacttcttcgactgaaaattgatttgtgaaaatacttctatttttgaccatatgtgattgggacatgtggaagccttgtgtgtacacacgtcacattaattaaatgaagaaagggatgttagctaaagcccaactgtcaaagcactctcctttaaataactgaggcccaactattgaagtgctccccttccttagccaaagtggttttctcctttctgccgagctccttcacattcgaagtccataacttctagaagtggatctgataggtgtatctttaaaactgactgatgtgacatcatcataaaatagaagttgggtatgttagcctatgagtgtaggacgactgacccattgtcaaatgtctgtcaatgtaaataatgtgagataagatgatgcgacattagaacctagcatatgaggccacgtggatctaatccaacaatgaccacgttggcctgaatactataatagcagtctttgtaacattttaaaagtaatgaatctttagacatataaaggacattgtacttttttctctctacatttattttccattctacaatcttttcctcatgagtatgtcttatttatcaactcgaacctatttgatcatcaactgaacattcatttaagccgacaatcaacatattgaggaatacgtccacgtatgcatcactttgattgacacatgttgacacatttttggaggtcgacagattgacgccatctatagaaaaactaagacaattaactacgaagatcccatgacgaaaggcctataatcctactcaaggaaaaaaagagtacaagggaaacaacttgtttgggacacaaatcctatttcttgaaataaagagagcattgattacaacaaaaagatattttaggaatagcatgagtactagtggagaagaacctacgccttgaaggactagggaataccttgaagaaggagaaccctcaaaaactgtcccaacgtcttgttacagattctacccaccaaatagacgaggtggattgtgagacaggtcacgaggaggctctagactggctactaggctcacccaagagagagaaatggggatagacatttcgacaaattattcttcaaatcaatattaggaagccctatttagtttcccacctgaatgttacccagaagatgtacaaatgaaattagttagcatttttgataagctaagtccaggataacctagaaataggaacaaccgatgccctcatccgtctagaaataagcaacacgaggaacctcgccttgggttgtaaaaagagccattggtggcaatatcaaccgtgcacctagaaattggagaaagagaagagctgagcaagcaagacaatgacaaggtcatctcaacctccttaggaggtcccggttagagaagaaggtgattttgaagaaccacaacgtcatgtaatcttgatgacgatgacgaaaatctgtcattttcacaaaaaattagaaatgctctagtcttgaactactttacgctacctaaaatacctaagtatgatgggaaaggagatccagcgaagaactttaacggtttcaaaacccacatgggattgagaggtgctatgcctgccatgaagtgtagagccttccatttgagcctcagtggagtggcagaagtgtggtacgccagactctaggtgggaaacattcgaagttggcctgattttaagaaggcttttctcaagccttcgccacttgcaaagaaggtaaagggctaatacaatgtttacaggacacgaggcaacaacctatggagctgttgaaaagttttctcgcccgctttatagacgaaatgacctactacgtagaggattagacatgaattcactcttttgaaaagatgtacaaaataaggatctcaccagttatgatgccctataggaaatgattaggcaagagattatcaatgaaaaattgaaggatcaccggaatagggtaaatcgaggtctttaccttctcaaatgcaaagaggaagaggcccaacatctcacttgatagaccaacaggttggacagtcaactcttctcaacccgatcaagcgttagccgtaactgtgcttaatgtagtcccaactttggcgtacgaagaaataaatcccaatgtcgacgtgtatcaagaaatgccacctcagtgaccagctcacaaaataggaggcaaaggacaaggtacacaacctagaaatagggatgaagcacccccatattgcacataccaccatttctataatcacaatacggctgggtgttgggacatggtgaaatacctaaataaccaaaggagaaatgatcattcctagagggataagacttctcaatagggttggcaacaaaggaatgaagcagactaccattaaaatagggataactcacgcagacgtggagaaaattgtgcaaggcttgaagaaggtcgaagacgccgaaggagtcccttgcccaatactggatgtgaacccatttgataaattgatacaatatttggaggtccattcgtgggggtgaactagaaatgcccaaagaaattatgcaagggaagccaatgactccccaatagcaagctttatagttatcaatggctggatttccaatcacaggggatttcaacccattacatttacccaagatgatgttgtaagggtacattatcctcattatgatgctcaagttgtaagggcagtagtggccagaaatggccttaagagaatgctggtaaacaacgggagttcagtcaatatcatatatggagctacttttgacaagatggaggttgacaatgagctgaccctaataacctcacccctgtatggattcacaaatgataaaatcattcttcgaggcaaaataactttggcaacagagatgaggatggcatctttgacggcccataacttcacggaatttctagtggtagatcatcactctgcttaccatgggatactgggaagacctgctctaaaagaattatgggcagtgactttgatcaaccacctgtgtatgaagttctcaacaaagaatggcattgctaaggtcaagggtgacaaacgaagtgccagagagtgctattcaaaatttatatggaaggttgaaccaatgagtgtgaatgtcatattaatggatatcgacgaggtcaacaaccctaaacaaggatcaaaccctgaacaatggggactttaaaatggtagatgcttttgaagaagcggctgccatggagatacagttggaccctgacgaaaggagaatgactgaagaagctattcattttgataaactgaacctttgtatagctgatgacgaacctcagatagctccaattgaagaactggagaattttatagtgaatttcctcgatccacttatgtttctgtaagttggcaagagactgtctctagccttgaaggagaagttgaaatgcttcctatactgcaacttgaatgtttttacttggaagcatgaagacatggtcgggatagatccaaagattagttgtcaccatttgaaaatcaaccccaagtcaaaccctcacaagcaaaatatgagagccttaaaccccgagaggtatgaggccttgaaagttgatgtacagaagttaattgctaaccgctttatctaggagtcgacctatccgaagtgggtgtcaaacctagtgttggtaaaaaaacataatgaaagttggaaagtatgtgtggattttaccgatttaaaccgatattttcctaaatacaacttccttcttccctagatagatcagctcattgactccaccatgggacatgaattgctgagtttcatggaagcatattcgggctataatcaaatcccaatgtatccaacaaacgagaagcatatatcttttattactaatcgaggcctatattgctacaagatgatgcccttcgggctcaaaaatggcggagccatcaaagattggttaataagatgtttgctgactttattagaaagacaatggaggtatatgtagatgatgtgatggtgaaaagtttaaaagcatatgatcacatacgacacttaaaggaggtcttctagactctttgtagatatagaatgcagttgaaccctttcaagtttaccgtaggagtagcctcgaaaagttcttgggttacatggtgaaccagagggtcatttaggctaaccttgataagatcaataccttggctaaaatgaaatcgctaaagaaacctaaggaggctcaaagcctcacaggtcgagtggcagcattaagctgcttcgtgtcaaaggcgatggacaagtgtcccatttttcaaaatcctaaaaggtgggaataggttcaaatggacaaaggaatgcaaggaggctctacaagctctgaagaagcagaacatggaatttgtttgttgatggtcatcgggagaaactggatttgtggctgggatagtttagatttgcccagaagtacacaagctcaattgcgccgtaagttttgggtttaaggcaacgaataatgtggccaaatatgaagctattctagctggtcttcaattagccagagaaatgcaagttaagaggttacatactagcagcgattctcagctggtggttagccaggttaatggcagttttgtagccaaggataagagcatggctgcatactttaagtaggtcatggagctccatcctacctttgaaagatttgaccttgtacagatctcacattgtgaaaattttcatcccaatgccctttcgaagttggaaaatagcaaggactttgagttattcactatagtcgccatagaacacattctgaggccttcaatttctaaaaataaagaccctctatgggccccatcattgtatttaaacaaaacgacattctgtcctctaaccaacaagaggcacagaaattgagatgacgagctgcccactttatcgtttgagatgacatactctacaagcgaggcttctcaatgtccctgctttgatgcataggtggataggaaccacttatatactttgggagatacacgaagggatatgtgataaccactcaggaggatgggctttagcacaaaaggttctaagggaaggatactactggctaaccttgaaaacggaagtccagcagtttaccaaaaaatgtgacaaatgccagtattttgccacaattcagagacaaccttcccacgagctgagtgttgtttctagcccatggtcattcgtcaagtgaggaaccgatctcattagacctatgctcaaggaaaagagtggttcctgtttggctaatgttacaattgactactttactaaataggttgaagctgagccactggccaaaataatcgaagtaaacacgtaaaaattcatgtggaaaaacatcatttgtaggtttggcatccccactcgattgtctcaaacaatggacgtcaattcaacaacagaaaggtttggaacctatgtaacgaattggggatcaagaaatacttttcctctccacatcatccacaagcaaatggaaaagttgaagctattaataaaaccatcaaatatacgtcgaatagaaagcttgatgcttcaaaatgagcttgggttgacaaatgcctcaggtttgatcggacatcagaacgacgagttggaccgctattggccaaacctcattttctgtgacttatggggtgaaggcaatgagcccaattgaagttggtctatcttcacctcaatggctgcacttcaacgaagtgtcaaacaaggaactaagaagatgtgagctagactttcttgaagaaaggaggaacagatcacagtccatgttggccatgtacgaaaggaaaatgacaaggtactacagctctaaagttaagaagaaatctgtgtgaacgaccttgtccttagaagagtgttcttttctataaaggagccatgggtagaaacttttggatcgaacaaggaaggtccatatagtgtaagagaagaagttcgacctgggacctaccggatagaaggattggatggaaaggcatagcctcatttgtggaacgtagaacatctgtgaaaatactatcaatgaatttgtacacgaccttgtatttgttatttactattgaaataagtttggtcttagctttatttacttagtaagttttatcttgtgaaataacgagctggatcccgaaatagaccgccttataaatggatgaagaggtaagtacaattccaaaatgaattacgcataagatattcaacctcacacggaggaaagcaaataaaaatggctaaactactaacacttgtgcaaaaaatcaattacgagtacaaacaaagcacaaatcaaacatgaagatgaggtattcatacataagaaaagtagcaaaattaacaagatagaaaatttaactttcattaatcaataaaatagttacaaaatgggcctcaaaggccaaaattacaaaatgaaaaataaaaaattacaaaaagccctatctaaacaggttgggaaaggaaagaaatggggtacaaatgtaattatggcattgggagcaacctcttggactttagcctatttttcattggtttcatcctcgatttctatcacttggcttccctctactgaagtctgaggctcatctccctcctccgaaaatttcgacctcaaaggtattgactggttaaaggttagcctcaatccactccaccacctctgtgtaggcatacttccatcagatggaagttggtaatatatctttttcggcttcactttcaatagactcagcttctcttttaacactctccatctcatcaaccaagccaggaattcttgaattcagctccttcacctgctctttcagagcaacattctctttattggccgcctccagggcctcaacagtgaacttctgatgggcatcaaatgtctccactcgcttcattagggttcttcaagctctcaatctctgacattgtagaagggagcttcattagcttttcttcagggcttcaacctcgggtaatgctttcttcgtcgctttctcggcctctgaagctcgggctataaaccctttatttttactcatgaagtttttattgagggcctccgtctcaatgacagtcctaaatttcctcgtcatttgacttaccctagtggtaaaaaggtctacacattcactggactcgacaaaggattgccaacgatcagtccagaattagtagaaaatagctcatatagtttgtacttctggaggcagcatcgacaaaacctccagagccagctcatctaggcctaggcaaaaatatcgaaaaactgatcaaaccaatcaaatcgaacctactcgggtctgtttaggtcggtttaacacaggtaattggtttggtttagtttgggtttcatttaaaaaaaccatggaggtttcgttcgatcatggtttgaagtctcataccgctagttaaccgatccaacccaacccaacccatttacatgtctaacttcttttttttttttttaaaaaaaagctagaaatcaaaagataagctttaatctcataactttatcacgattccctcaaatttatgatattgtaggtcaataatagtactgaaaatttcctttgacaagctcattatattatacttaatcttttttcctacttaaacaatcaggctacataatgtataaactggcaacgaaattcttaagttttctattgatttatttctaataacataattttatttgttagtcaataattcttataatataaagttatttagctatcttagatcttgtaatctaattgggccaaaacttggacaatttttcttaaaaaattcaatttagactaaaagtctaaaccgactaatcgaaccgatggtttagtttggttcagcttaagagctagagtgggttggtttttgaaattcactcaaactgatttggtttggttcagtttagtttaagaggtagagttcgttggtttgggttgagattcactcaaaccgactaatttggtttcgattttaggttggagttgaaaccaacccaaaccaaatcgtgcccaggcttaagctcatcactccattgaataacaaaaagcttaaggctcggggctgcattggctaagaaagacccactggagttccttgccttctttgacaaactttgcttgggggcttcgcattagtggacctcttctggacccctctagcaacagctataaatgctgccatcaacttttctccagctagggcttcggggcgaggcgattgtgggttggcaactgacctacctactccggtggtagagaagtgatgtttcttcttgtggaccctttccactttgcctttatccttgtctgccaggggaagtctcccagtagcttcttttccacttggtccctcacttgttttccagcaacagatgaaggctttaggcctttccttccaattgtagaggtggcgaccaatatggtggccatgtcaggaatggggcacctcatcttctcgaagtctacaaattaaatcaatgagtgtataaaaacacaacgcaaagaaagtatcaaagtaacgcaaagtgataattactcagtggtcgcagaagtacctcttcgagcgatcaagttaaattcttcaaaaaattgtttggaaatgataagcctctcgaacttctttgaagaagctggattcaagtagatgtcctttataagctcaaggaattgaactcaaatagatcgactcctcctgcaaaaaaagaatatagcatta